European Patent Application EP 4 141 103 A1 - sequence listing, part 2

SEQ ID NO: 4 - DNA, 648565 bp, Chitinophaga pinensis
  source 1..648565: mol_type = genomic DNA
ttgctaaagcaagctgacattaactatttattctcttaaaaaacacctgatcatcataatgattattaggccatcttttggctaaaacaaagaagctgtctcaattaattatgagacagcttcttttttatgaattcacttttacagctggagataaaaacaccgaacccgcctgtgacagcgggttcaagtcaactaaaacaaactttagccattgggcatccggctattagcatacccaaaaagtttctccgcaggagataaactgcgtggtgggcaaagtacgttctttgcttttctcctgtggcgctttactaaggctggcaacggtaatttttgtaagcttcagctttgaagtgattttctttttcatattgatacagatttaggttacttcaatctacgataagaatctgttaccatcaatcacgtaaaaaggggatttatcactgctgtgctcctttgctgatcttgttattaacgatacgggcgttgccgtcgatatccagactaccattcactgcttcggaaatcactgcacctgtattgcgggcgggtgaattgggagcaatgtgcaggtcaggtattgttgtactgataagtaaaggatctgtaccatacacggagctggcatcggtgccggaagtgcttttccaggtattgaaatccgtaatgatatttgtattggtaccattccagatccattgcggcgtaccggtagtgaagtaaaggttgttatcgatgacattaccggagccggtaccggtatatttatgcacaaagatatctaccggcctcgcatatacgatattattacggatcacgttatcaaagcattgttccgtgagacggatctctccttctatttcgccaaaagcgcccggctcgcggtcgttgaacaacaaggtattgtttaccacgtagcaattgcgtgtaccgccggatgtataaccgaggtagccgccgagatagatgccggtgcgccagcagttagacacaaaattattcctgacgatgcaattgctggtgggatatgcatcattttcactgacgataccgatgccgcggtcggcttcatggatgcggtttctttccacggtaatattccgggcgccgtctacataaatagcgatagcgccgtgaccatgcgttccgccaacggggccgcgtgtcatgtcaatgttatacaattcattttcggtgataaggccatttcttgcatagttcaatgctgggttggtattggccgcgtagccaccggctgcatcgataccaatgttttcggtgttgtagatcgtgtttctcctgatcgtaaatccatctacataaccattgatggtgaggttttcgctgtacccggttttagtgtcatgaatgatattatcttccacgaggatgttcttcatcacatcggcggtgttgccgataatttcgatgccatgaccgctcctgccctgcgatggttccacgttatgttctatgttataaattttatttttccggatgatgatattactggcacctgcgtctgctgtaatcccattcacatttgcccatgctgcagtacttttcaaattgcagatatcaaatccctccagcaccacatagcttgtattactgatagtaaccagcgcttccctcccggtaacgatcatgccggtgccatcaatcaccgccttttcaccgggataggctttgagtgtgatgagtttttccagccggccggcgcgtggaaaaaccaccctttccccgtaagtaccggctctcaccatcacggtatcgccgggaagcgcctttgccaaagcgatgttgatgctgcgtaccggtttgctgatagttcctgcagccgagttatcgccattagcggcaacgtagtaagtgtgggtttgtgcggcatcaacggtagtaacagcggtagatcctttactacaggcgccggccagcatagcgaatagaaaaaaatacatgttcctgtttaacatctttttaaaaataaacggcggcagtaagtgaccgccgccgtgggtttgcatatagtttattctgaaattattttcctgaccctgttattattcttatccaacacatatacgatcccatctttgtccactgctacgcccattggtgcattaaacgaggcggcagcgccgataccatctttaaaaccagcgctgttgctaccggcataggtagtcacgttccaggtgttagcggaaatagcgcggatactttcatcggcattagcgccgtaactgccattaccagccacatatatattgccggtaatgtctactgccagcccccatggatttgcgaatcgtgcagccgtacccgtgccgttttcataacctgccacgccggtagcgccggcaataacagtaggctgccacgtacccgctttaaactggataatagtattgcccgtgttactggatatgtaaagattgccggctttgtcgaagtccataccacctggcgccgtaacgccattaataatagccacactgctgccatccggcttcatttcaaaaacgccgccgccgccggtactgcaataatatattttgccggatgttttatctactgcaacattccagggttcctgtactgtacctcccagggtagtggtagtaccatccggtgtaattttgcggatgctccaggtgcccggatccgcggtatacacatttccctgtgcatccagtgccaggccgtatggaatctggaaacgcgccgcagcacctttgccatcatcgcttccgctgttaccggggctgccggccaatacagtcgcatttccttcgctgtctattttacggatacaggcgttgcccggatctgccacatatacgttcccgttatcatccgcaccaatccccatcatccggtaccagctttgcccgttaaaactaaacagtgcgtcagcgccttttccgttggcaaatccggcggtaccgttgccggcaagtgtggtcactgttctggaaaacacataggtaaacggcgtaccgctcaccacactgtcttttccaactttcaccacgaggttgccggtgccgcatttcttcggcactattaccataatctgtttcgtattggcgttcacgatagcacaacgtttaccattgatcgtaacagtgatatcggatgtatcagcagagaaattatcacctgtaatcagtacttccgtggtactgccgccggtagcgggaatgaagtcggtaagcagcaccggttgcccttccgcgtgtttcagatcgtcgtcttttgaacatcccgccaacagggcagacatcagtaaacaacctttcagtatatatgaattcagtggcctgatcatagcagttagttaagatttaaataaagaaaaaattaccagcccgggttttgcactaatgcgcggtctctttccaggtcctgttgctggatagggaacatatacatcttattatcccagtatcttttctggaaaagtgtgcgggtataaaaaccggtgaaagaaaatccctggtcattatctttcgcatttatattcatgccgtaaatcgcctggttttccggtttactcatcagcaaccggcggatgagcgtgtaataacgatcgccttcaaagcaaaattctacttgtctttctctcaaaatatatttcctcatttcttcctggttacctatggcacccggatatacggtttcaatgcccggcaggcctgcgcgtgttcttacctggttaaggtatttcacgatatccggattagccggatcatactcatttaatgcctctacatagtcgagtaaaatttctgagtaacggataaggatatacggagaacggtaggcgtcggtagacatgctgcggaggttatcgttcgggctcagtaatttagcgggaaggtagccggtgatgatgttgctgcccattccctgcatgcctgatttaccactgtagtaaaactcctggcggccggtaccatctttatttttttcagaagagaaatagtttttatcatctactgataccgctgcaatcaccgggcggcggttgtaagcgatgtaagcatagaaccttggttcacgctttgcgtacatgttccagtcgccttccttattttcccagtaatgctcaccatcctgtgcagcaaagcctgtttccacatagttggaagtagggtccgtaatggttttaccattgttcatataaaaggcatccaccacgttttgtgtagcgttgtacaggttgtaccctgcagggccgggagaggaacagatggtatatccccagcgttgccagttcatggaagcaaggataatttcatcattccaggaagtaaggaatacatcccttacagaaagaaacggatcgaaggtagtaccgccgttatcgaggttggtaaacagtttatacttgttggaatcgatgatcgcttttgctgcctgtgcggcgatgcgccatttatttacatcgtagccggcgggcgccagtggtgtaccatcctggtttttgaacgcagcaagagcgggattaccgttccacaaggggcttgccgcccactgtgcaacttttgcttttacagcgagacaggcgccacgggtagcacggccattattacctgaggagctccatacgaaaggaagtccggccgccgcgccgtccatcatttcattgatgaactttacgcaggtgtcgaaaggcgctctcgggtatttgttcatgtcttcatcctggctaacagtaccggtgagcttcacgaatggtccgtattgtcttagcagcatccaataaaagtaaccacgcaggaaaaggttttccgacttgtattgcgctttcaattcgttgctcaactgatctccaggcaccttatcaatattttgctcgaagatgaaagatttccggatggcagtatagtagccgccccagttgtagaagtaccaatcggacgcgctccagttgccgcccaccatgtaccttaccgtggtaccgggaatggaaacagagagttcatccgcggcgccgatgccggcatagtcgccgccagcctggcgggcgctgtagatattactcaggtatgcttccgcgttagccctggtttgccagatctgatcttcagtgagaaggttatccggctttttgtccaggtacttgctgcaggataccagtgtaatggcaatgataccgatgaaaaaaagtaacaggtatttatatctggtcataacaataatctttttgatcttgattaaaactgtgctcttacacccagggtaacggttttcggataaggataccttgccgcgaaattgcccagttccggatcccataatttgaacttcgtgaacgtgagcatgttggtagcagtggtatatacctgcagactgctgatgcctttgcgtttcatatccggtgtgataaaggagtagctgaaggtggcctgtttcaggcgcatgaaactaccgtctttaatccaccagctgctacttaaatagttattgtcgttggtattagctacggtaagacgtggatagcgcacattctgactgggattttccggtgtccacctgttcatcatatcttccaatacactggcggaatattgccccatgccggcgaaaggaataacacctacgccatcggccccggcgccattaccggtcacccctgagccattggccataatgcctacatctgccacgcctgcaaaaacagcagagagttcaaatttcttatagccaaaattaaagccgtaaccgtatgaccaggtagggaaactggatttacctaaataggtttggtcgttaccatcgatcctgccatcgttattgagatccgcatactttatatcaccgggatgcactaccctgaactgttgcgggcttttctccacatcatcctgactggtgaataacccgaggctctggtagcctttgaattcgccaaacttatgtccttcctgttgtgcataggcatacagggctatgggattatctgcgtagatgatcttgtttttggcgtaggtaatattgccgaataaacgaatcgaaatatcttttccgatatgaccggtatactccatgctgccatctattcctttattcaccatttcaccgatgttaccatagatactgctggagccgtatcctgcaatgggtgaaatggatttgcgggcaaccaggatcgcacttcttttatcctggaatccatctatgataatattcagtttattccacaaacccacttccaggccgatatcggttttggcagatttttcccaggtgaggttttctgtaccgattacatctgcattaacgcccccattataggaaggcgtaccggagctgccgaaagacactccaggcgcaccgctattataataagtgagataaccaaaacggttcccgtcgatctggtcgttacctgtcatcccgtaagacccgcggatcttcaggagattgatcactttggtataaggcaggaaaaagttttctttggaaatcacccagccaacggaacccgccgggaagtaaccccatctttttccctgttcaaagttttcagatccggtggcgcccatattcatttctgccaggtatttatccatataggaataagtgacccttgctgcagcgctctggttacgataaggaatggctccctttacatctccggcagaacccaccagcctgttgcggatgctacctaccagtaatccaccgaaattatgtttaccaaagctatgatcataggtgaggttaccttccaggtacatcatgcgttcgccggtggaagaggcgccatagcccaggtaagtactgcctatcctgctttgattataaaagagactaccatcttcgtttctgccgggcgcataaaacaggtcatttacaccggttctgctgttatcaaattcgctgtaagtatcaaaagaaaaccgggcattggcgctcagtccttctgtaattacatccagtttctgattaagggataacacggattggatggaaggtctgaattctgtggagtagccagcgttttgcaccaggttaaacgggttggcaccaccgttgttaaccgggcctgcccatttaccatccgggtaggataccgggaaagagatgggattggtagcgtaagtggaataccagatagaaccggcggagttacccgggtagcgggtgtttaccagcatggaagccaggttgagggaaagcagtgttgttttggtgacgttcaggtccacgttactcctgaaatcatatcttttgaaattgaggttgggattgtagccgatgttattcactttgtattgtccgtcctggttgtaaaacgacatagacacatagtagcgcatggcttctccgccgccgcttacattcacattggcgtttgccatagtggcccagtccttataaatagttttgatccagtttacatttggatagatatatggatcgagtccgctggctgttttacggatcaattcatcagagtataccggttcatcgccggcattggtacgggcttcgttatacaacttcatataattcacgccgtccagcattttcggcatctgggttagcccgctgaaacccgtttctgctttagcggatacctttggtttaccggccacccctctgcgggtggtgatgatcagtacgccgttggcgcctttcgcgccatacactgcggtagcggaagcatctttcagcagcgaaatactctggatatcttccggatcaatgttattaaaagcgccgccgtaggtgctgtttacatcttccctttgcacgccatcaacaatgatgagcggggaaacgcttccctggaaagtaccgataccgcggatggtgaagttgggattgtcataacccggttcccctccggcgctctgcatggatattatgccagctaccttgcccaccaatgcgttagttaaggagcgcaccggcgtttgcatatccgccatatttacagtggatacagcgcccgttaccgttacttttttctggctgccaaaacctactaccaccacttcgttcagcttatccacctttgcggttaagcttaccttgagtgttttctgattcaccacttttacttcttcgggattcatgcccatcatcgccactttgatgatgtcatctttgttggccgcaatggaaaatacgcccattacatcggtaacagttcctttcttactgtcttttaccgtaatagtggcgccaggcaggggatttccatctacatccattacctgcccgcgcaccagccactccgattgtttctctgccgccgcggtgaccgtggtttccggcgccgctgctttcttgtcgagtacaatgcggttacgctgcaatacgtagctgatatttttatctttaaaaataaaagccagtacttcctccagttttgcctgctggaagttgagcgacattttttccccatcgttcagcagttgattgctgtacaccagggtaagccctgtttgttttttgatggcccggaagatctgcaggagggttacctcattaccggtaaccgtgacgattgactgcagtgaaggcggcggtgtttgcgccttcacgctcgaaaaggaagtgcatataagggcacagagcaccaacatgcgcactacgtttcgcatagccagctggcagtggcgtatactttttctcattcgggaatgtttacaagttaaaatgatggtacagcaaatcaccgtagcaaatgctttcatcacaactacatcgtttttcagaaaacgggtgacaaggagtagtaaaaatattttttgagagaagaaaaatctatctcagggtaatttcattacctgataaatggtattcgatatgggcagttgttttaagatcggataagaaatcctccagccggttacggtccatcaggcccgttaccacctgtccggcttctttatttttgtccaatacaaagcgcattccatagaagcgggaagcggcggcgataagggttgtaagcggcatgcggtggtaatagtaaaccccgttacgccaggataacacttcttcttcatcaaagtggctggtaacaaatccctgtccggcgttgtaatcggcctggatacctggttgcagggtttggcgttcgcccgttttccctttggtgatgacgctgccctgtacgagggctgtttttactgttcccggctgataggtgttaatattaaaagctgttcccagtacttgtacgctggtaagtgctgtgtgtacaataaaaggcttttccgcattggcggccaccttaaaataggcttccccttctacatatatttctcttgccgccctgccgaaatgaaaaggaaaacgcagcctggtggcggcattcagccacacttccgtgccgtccgacaaggtaagtttgtagctttcgccggcaggaacgtcgagggtatttaatacggtatcggcagaagtatattgcagggcgccgttgctggtgttcagcgtggcgttgctaagtgcgatggttttggcgctgctgtctttgctcagctctactttttcgccgttactcagcaacaggcgaaccggttgcttctgttgctgcatggctaccgatggcgaagttaccggtgctgtgcgggtaaagaaatagtacgtaccgctgcctgccaagagcagtatagcggctgcggccagcccctttttcaggtgtatgaccgggcggcgtgttgttctttcttccttaatgcggtgcagggccgcgtcagaatcaatctgctgaagatacctgtctgtatgaagagtcatgctttcctgttccagctgatcccactgcgctttgaagccggcatcatgccgcagcatttcctggacatactcctcctcttctgcggagagtgttcccgacaaacgttgtagatataattcaaatattttttcctgtgcctgctccattgttaacaaaacgcgggctaataccccttattagtaattgcatgacgtaatactttcagccctcttttcaggtgggttttgaaagaattgatactgatgcccatttcatccgctgcttcctggtaccgttttccctggatatacaccatttgtatagccgatcttttttgtaccgccatatcgttgatggccgttaatacctgtttataataatccggtgaaacttcagtgtttaccatacaggtttcatcctgtaactgggtgaatgccactttattttccagttccgccttttgctttttaagatacgtgaggcaacggtttttgacggcctgatgcaggtatcccttgatatcacctgaaaaatgaaggtataattttttgtcccaaatgtccaggaagaaagtctgtacaagatcattggcttctgcctcattccgcaggaaccaataggcattgaggcaaagcagcttgtgatacttcataaataaagcatcatatgctgaagcatcgccttcctttaaccgctgcaccaatactatgtctgaagaatgactcatgtaaccggaaccttattggtaattattcattacaggtagcttaaacacataacatatctgtaacgctgccaagtggcaaccttattacagtgactttgattaaatgatccggaagaaatttatttcttccattgttcacgttgatactaaagattttggctaattgactattaaactggaatcaaggtaaataataaaatcggaaaattatacgggcgcggtaaaaaaattaaaagccccggtaaaggataccggagctttgttttcatgggggtttcagtagatagcctataatttaaagaagatcttctttttaaacagccagtagcacaggccccattccagcgccagtactgcaaaggcggataatatttcccggatgctttccgggattccggccagcgcggtaaatccttttacaaagatgccggtggtgggatttacccattgagcgcctaccgtttcaaagaagaggtaaataaaaatggcgttcatacccactacggtggctatccaggcgtaacgcacattttgttttacatctataatccaatacagcagggccattaccagcattacccatcccccggaagccagtgtaaaagaggcagtggcaatccgtttgatgatcggcgtgatgcctgccaggtccagtccgaagccggtgacaagccctatcagccctgcgatcaccaggatctttattttctgcgcccgcggccggtcgctgatcagtaacttcccggccagcgcgccccagatggtatgcgcggcggtggggataaagttaatggtcacccatccgtcagggttgatcttacccatcagcacagtatccataaaagctccgaagttatgaccttgtataaatggctcttcgaaaccgggcaataaaacaaaccggtacattaaatcagttgccagcaacagtaaaaggcttatggccagctggaaaccaaaggaacggcgtatgataaggtaagcgatcagggtggttacagataactgcgtgagcacattccataactcccatactaaccttcctgcatatacgcaatggagggcagtaccaaatataaacaactttaaacaacgcagggcaatatgccggaaattttgtgaccaggtaatacccttttgcgttttataatagtaagagatgaacatcgcagcaccggccattgtcataaaagcaggttgcaccaggtcccaggcccgtagcccgttccaggggtggtgaaaaaactgcgttatcagactgccggctacccccgtggggtgtaaatgtgctatcgactcatagatgcgagcgctttctccggccaggagaatcataataaggccacgcatcacatccagggaaatcaatcgttgactgacattggttgtttggctcattgtcctgtttgtaggcttaaattaataatttattccggcatatttaataaaaaagcggcagcgccttcatcggggatggtgcccagctgtgtggaccaatcgctggaagtggccaccatgcccagccgtatagccgttcccgtaaagccctttatttttgagcggtccagttttccttcaaaacggatggtccccccttcttctttaatggtgcccatcgtaaagaaatccgttcctgattgtacatcgaaactgaagctggtttgcggtccgttatgataatacatcgccatcgggataggcgccgtgttctgattgagcagcagctgcccctccagcaatacatcgtaagccgcgccggtaaacagggaagtgatcaggcccgtggcgtcactgttgtcgctgtcgatatacacgtcgaaaatagcgccatcggccagtttaccgctcatctctccatagaaatacataaactgtccgtcgtaatcgaatttcagctttttgaaaacgccgcctgccggaccggcagtgatcacattctggctgatggtatcccagtcggccaggctgttatcagtgagtttcaccggtgaggttttggagatccggatcacggtagacccttccgcggtaacccctgcagcggaagtggcgtacagggttggcacatatttacccttaccctggtaggtatgcaccgggctttgctcggtggaattagtaccatcgccgaagtcccatttccaggaggtagcaccggtagtagtgttattaaaagatacctggttcccttctacttcaatggtatatactaccagcggcgccgggttggtatcgtcttttttacaggcggaagctgcgcacagcagcataaatatatagagcagttgcttttgcataatcaggtggttttaaggattctgtacgcacagtttattggtttctatttcatcgatggggatgtaatagatgatcttcggattatcaggctgcactaccatgccggcataaccggaaggatttaccgccaggttgatatccgattctttcaggcccggtaaatgatacccccagtaggttctgttcatgggcttcttattgcggtacacatcataggcgcggtgaccttcaaaggcgagttccagtctcctttcctttagcaccacatccagtgcggttttcccggcaggcaactgttgatgatacaatgcacccgacaagccgcggttggtgcggatcatatccaggtcgtcgagcgccgcggctgttttgcccgctttggcttcggcttccgccctgttcaggtacatttccgcaaggcggaaaagaatgggtgagctcagcgtaggacttcccccctgaccagagaatttggagatatagtagatatcgatgccattcttttgctgcaatacgccattgtcatctttcaggggtataatatatttccagcgtacatcctccgggttagcggacatggtatccctcagcgacgcggacgcaaattcctctccccagccggagttaccgttggaatagatcatagaggcgatagaaccaaacttaccgtagtcgtccagttgcgtaaaggccacacagaaaatggtttcagtaccggcggctgcgttggcaaacagatcgggataagtagcggaggtagccagtgaatagcggccggatgaaattacctgcgatgcgaagtaagtggtgctgtcgttgttcccttcatacaggtatgcccgggaaagcagtgcccatgccgcttcgcgggaagcgtactgtgatcccctgctttgcgacatcagttccgctcctttcctggcgtctgcaatgatctgtgcatatacttctcctacgctggcccgtgccttttgtgcaggatcgctggtagaagtacgcaggattacaccgggagcgccggggttctgtgcgtatggcatggcgaataatttcaccaggttaaaatgactgaaagctcgcagaaagtagcattcacccaacatctgttgcgtggtagcatcaggattggcctgcttttccaccgcttcaataacggtgttggcgtcgttgataattttataggaaatataccagaaatagcgtgtattcgtttgcgttggcgagtggccaagtgagaaactataaaacaggggatcttctgttgtttgtccgcatacaatatcatcgctggcaaaatccgacaactggaaatactgccgcaggtacatattgttatcatcggtggtaccattaaacggcacgtgatctttcagcagtgaatatgctccgttcacggcatttttcagcccttcgggagaacctgtaatggtttctgtggtgagggcatcgcttggattcacatctttcatacaacctgtttgccataacaacacaggcagtagtattaatattataatcgctgatctcatgacaggcattttagaatctgaaattaatgttgaacaggtactggcggttgttgggatacttgaaatccgaaacgcccggcatcacctgtgatccgggtgtgatggtagtttgcggatcctgtcccaggaaattggtgaacgtatgcacgttatcggcggtgaagccaacggttacaccatcgaggcgccacctgtttaccaatgcttttggcagttcgtaactcagactgatgttacgcaatgcccagaaactgccgtctttcaaaaagcgtgtagacgtttgcgtgctgttggcagaattctgcggactgggctccgtggcattgtcgccgggctttgcccaggtactgctgcctttgggcaggttcacctggttatagtaaggttcgttgccatcattttccacaaagcgaaggttattactgtatactttgttgccggaaaggaaatagatatttgcgcttaaagagataccgctataggtaaaggtgttggtcatacctccctggaacttcggcagcgcggagcctacctcctggtaggtggcgctggcataatccgaggttgatgacctgctgccatctttatccaccacttcccacagaggtgcgccggtttgtttatctacccctaaccacttgggcatataaaattcatacaggttaccgccattgcggtagatctgtgaaatactccaggtagattgtgtgttgatgatactggccgggaatttttgcagcttgttagtgttgaagttgatattaaaatcggtgctccattggaatttccggccgcggatattcaccgagctgatgcctagttccacaccgttattcaccagctcccctacgttctgccaacgtgtttcaaagccaaccgacagtggttgtgatacctgcagcagcaggtttttggtgatattgttatacacatccacactcaggtcaatacgcttaaacaacccgatatcgataccgccgttccactggtatttgctttcccacgtgagatccgggctgggcagctgtgatggtgttgccgctatttgtccgttgtactgactagccagtgaaaacaacgccaggtagcgcgatgaccctatgtcctgtgtaccggtaacgccgtaactggcgcggagtttcagattagtgaacaccgcattatctttcagaaaatcttcattactcattaaccatgcggcagaaacagatgggaaagatgcccagcggttaccggatgggaaattggaagagccatccacacggaatgatcctgtgaggaaatatttatccaggtaactgtagtttacctgtgagatgaacgactgtataatggcttcattgatactaccattcacgatctggctgttagctactacgttcagcacttttaacccggcgggcagtcctttcccggaggcgcccagcacgtcagtattgctgccttcaaacgctacgcccgcgaggccgctgatgcggtgatcgcccatacggaaatctactttcagcaggttgttggagatgtatccatagttaagtgtactgaattcactgaggtaaccggtactatggtattgccccgccacatccggcgaataccaggttttatttttattgtatcccagcgaaagccggttagtactggtaaaggtgagccagtcggtgataccgatgttaagccccatgtcataattcacatcaaaatttttgtagggatgctctgaattattaatggtgtgaataggatttaccttatcgcgtgaccaccatttgaagggcgagttaccatctacatacaatgctttaccggagctgtcgtacgggttatcccagggcatgttgagataagcataatacatatcgttgtagtcgtatgttttaccaaaggagccgctgaggttgatgttgttggttaagctgatacgtttagtgaagtggtaggtagaattggctctcaggtttacgcgctggtagttggtattcataaaagttcctttctcgttgtaataagagaggcccaggtagtagtctgatttttccgacttgccactggcggagagatatatgttctgcatgggtgcgcgttggaacatatcggttaaccagttgtagttctggttgcgcaggtcgagcggccgctcattataaaatttcagcaggtctattttgtaggagttgttggaagcgccgggaatatagtcgcggtaatattctttctggcgttcatacaattcgctgccgttcatcatgtccatggtgccaaagtcgggtgtgcggaagccggtggttacttttgcctggaactgtattttacccgaggcggctcttttggtggtgatgatgatcacacctgcgttggcctgcgagccgtacatggcagtggcgccggcatctttaagcaccgttacgctttcaatatcgttggggtcgtagttgccgccaatgataccatccactactacgagcgggctttgcgacgcgttgaccgaagaaatgccgcgcatgcggatttctgctgcggcgccgggcacaccggaactgcttaccacctggaggccggctactttgccttgcagcatagtacctacatcgttggtggtaacgtctttcagttttgcggcgtctacaacggtaacggcgctggttaattcgcttttctttttatcggagtagcctactaccactacctggtccagctgactgttggcggttcgcagggttacctgcatgccgttgcgggcgggcagttcctgtttatcatagccggtgaaagtgaataccagtatttcgccggcgttggcggctacagtgaattgcccgccggcattggtagcgttgcccctgctggtgccttttacgattacggtagcgccggggagtagtgtgccgtcagggccacgtactataccggtaatacggccagtggtatccactggcagcggcgggggatcggactttgggcggataacgaatacgccgttgttgatagaaaacgttaccggctggtgttgcaggcattgctccaataccgattgcacggaggcgctgcttacctgtaaggtaaccggggtggtatttttgagggcggattcattgtatacgatggtagcccccgattgcaggattatttctgcaaatactttctgtaacggcatatttttcacagagagggtaacctgttgtgaaaaactcctggcgcttacatgtaggcaggcgatcaggataagccaggtggtcattttcataacccgcaaaattttggttaataaaagtccctttgggagaaatggtatctccttaaattttaaatgcatacttttaataaggtttagaattcttaaatgatcgtcgctgatcttacaggatgctgagctgctgccgggggtgtgtcaccacctccggcttttttcattgttcaatgtgttacttcatatgctttttttacaggttttacggtaataccactactttatttccatctgttttaaagtgattagttccgttttcttctaacacgcgcaatacggctgacaaattaagattccggctgattccgccaccatacagttctttaccgggtggggactgatacacaatttccacatcataccagcgggcaatttcccgcagtatggttggcaggtccatattattaaatacaaagagtccgtttttccaggccataattttattgacgtcggcatcgcgaacggtgagctggtggcctgacagggccagcacggcctgctgaccgggatgcaggatcttatcctgtacttttatttttccatccaccagggtagcgttgatcgtaggttcatcggggtaggccatcatatcgaagcgggtgcccagcaccagcacttccatttcattggcctgtactttaaagggttgtgcggcgtcggcggcaatttcaaagtaggcttgtccctgcaggatcactttccgttctgctccctggaaacttgtagggtaacgcagggaagtggcggagttgagccataccctggtaccgtccggcaataccagctggaattggccaccacggggcacggtgagggtattatacaccacttcgccggtggcatcacctgcctggtaggccagttgtcctttttcttttttgatgatgtttgcgccgccttgtttaccgagggcgccattggctgcgtcatcgagcgtgatagtgctgccatcggccagggtaagcatggctttttggttggccggcgctttatctgttgcggtggcgttatccgccatcatatttttttgtggagatggataccggtgctgccaccctattttcccggctactgctaccagcgccagcagggccgccgcagcggcataacgccagaaggggatctttttcactttgggcgcctgcatcaccggcttcaacctgttcagcagccgctgttccagcatccgtcggtcttcccctggctccactggcagctgcacttcgctgtcgtcgaagctatcataccactcgtgaagcgcttccacttcttcgggtgaagcattgcctttcaggtaacgttggatcaggtcttttaggtgctgcataataacagagtacagaaattctgctgttacccttagttgtttttagattttttttcagaagaagaaagaaagatagggatacacgtctttcaggcgaacgcgcaggtgtttcagggcctttgtcagatgggcttccaccgttttttccgacagttgcagggcggcggcgatttctttattgctgtactgatcgcggcggctgtataaaaatacgaggcggcatttttcggggaggtgggcgatttcctgtcccagccgctcctggaggcggcaataatccaggtggtccatatcggggttttgcaccagttgctgcgccatatcagccgtatccagcggatgatccggcaataaacggctgatctgccggaacacggcataccgggtagctgtagccaggtacccggaaagatggcggatatccagctccccttttcgtacccacaggctggccagtacttcctgcactacatcttccgctgcagcgcgggtacgcaggcggttgtatgcaatagcatacagtttctcccaataacgatgaaatatttcggtatacgccgattcatcggattgccgtagtctttgtaatagcgctatgtcactttgttcctccacgtgtggtaattggttgatatccgggtgcgctataaaaataagtaaaatgcggcggattttgtctttatcaggattacgctgattatactgattagtttgatttttacttttggattttttttagatttttagattaataacattaagggagataaaagcgaatatatccgcttatatctcccttaatcctttataaaatcacaaaagtaaaaatcaaactaatcagtataatcagcgtaatcctgagaaagacaacctccgcgtgatcgccgaaggcgatcctcgctagagggcgtgtacgctcgctccccagcggcgatcgggcgagcgccccatttccagctccagtgtaccgccctgcatgagttgctggtgggtgaaaaagggagaggtaagtacttctccgttcaggcgggcgctttggatatatttattggtatccgaacagtggttggcaataatggtgaagcggcggttttccggaagggtaatggtgatcctgctgaatatgggactgccgatggtatagatggggataccgggcgtaacggggtaaaagcccatagaggcaaacactacaaaggcgctcatgccgccgccatcttcgtcgccggggataccgaatacattgtctttaaaccagaggtccagtaaaaagcggacgcgcttctgcgttttccagggggcgccggcataattatacagccagggaatgtgaaagccgggttcgttgcccatagaaaattgtcccacgaggccagtggcatccgggaacttgtgccatagttcataacggggcatgccgggatctttgcggaacagttcatccaacctggcttcaaaacgtttttcgccgcccattaaactgatgagcgcagggaggttatgttgcacctgccagagataggtccagccgttgttttcatcgtaatagtcgcggccaccaggcccgccgtcgaaagcgggatctatattgatccagttgccggcagcatcctttggcataaaaaagccattgcccgggttccagaggtggcggtaattttcgccgcgcgcagcaaacagccgggcatcggcatcctgctttaatgccgctgcgaattgcgacaaggcccagtcatcgtaactatgccctaacgtaacggctaccgcctgccgcttttcaaaaggatgtacggtgttgacggtttcactgtcgccgggtgataaagcaggataatatccgtgggtgtaataaaaagaatcgagcggaccattgggtccattgcgccagggcagcatggtagccatcaatgcgttcttcttcatcccggcgtatgctgtatccgggtctgttaacggaatgcctttgcgcagggcatcgaggaaaacaatggtgctgtgaaacccgttcatacagggatgatcgccatacaaccggggaaaggtcggcatccagccactttgccggtacatttccgtataggactgcagcatgtcggcttcctgttgcgggtggaggatcatgcgaaggggatgcagcgcctggtaggtatcccaggtggcgtcatctacataaaacgggcgggtagtatgatttacttttttattatacccgctgtagtaaagcgtatcttctgcgatatccaccatccgctcgtggcagcggtacagggctgtataaaaagagcggcgctgcgctgtggtgcccccttctaccctgatctgatcggttattgccttccatcgctgctgagcattattttgtactgcggtgaaattcctgttacctatctcccgtttaaaactattttccgcactcgccatgctaacataagaaatggcgtacttcagggtaatgatgtcagtggtggtatccgggaaggaaaggtattgcagtgtatccgtgagcgttataacgttaacgggcgtattaaattctccatacaagtataccggtacatcatcatgataaaatgtttgtgcagtaagggaggttccgttggtgtgatacccggcgctatcgagcaataaatatttccgcatgccggcaagataggtaaaacgatagatccctgttttacttcctggcgtgaactccacagtggtattgctttccagcaaatcggcgtgataataccaggggtgaataatttcccggtcgtaggtttgtttttgttgccaggcggcgggtgtaagtttaccggtagcaggttgtacaacaaacaaaggcccgctgttgtgtgcggccacctgcaatggaaatccgctgacctgatcatcggtgtgatctttcctcaacgggtatacgcggatcatttgattgggcagctgcatcacaggcctggtcggctgcaataacgtggaaatattgccgatagtagggtcgatatactgttctgtactaatttgcgggttggtgctgcaaccatatagaaacagtaaggcgattaccggcaggtaacagaaaggtgactgcatagaatgcctgttcataacacgggcccgcatcagcaggcccgtgttgataaaaaagaggtgattatttacggtattccaccgtagccattacggggaagtgatctgacggctccctggcaatatattttgacatacgcacttctttggggaagttggcgtttgcctcaggagtggcgccctccgggcgtttgctgcgataggtatcggtaaggataccataacggctcactttaaactgtttggtcagaaaaatatgatcgatacgactgtccgttttgctgtcggttttaaagctgttgaaggtaccgttcagcgcgtagcggatggcggtggtttcatatgcgtcttccaaaacaccggaggtgtgcagtactgcatacgaatcactggtttggtctacgttgaaatcgccggtaaggatcaccggtttgttaccggtcatctcttttatttttgcaaggatcagttttgcactttctgagcgggcaaccacacccacatgatccatgtggaggttaaagaaataaaaggtaaatcctgttttaatttctttaaactcgccccaggagcaaatcctgggcagcacagcatcccatcctttattgggccggtcggtaatggtggacatccagaaatcaccttttttcagcagtttgaatttcgatgttttatagaagatagccgagtattctccttttgttttgccatcgtcgcggcctatgccgatataatcgtaaccgggcaggctgtttttcacatcttccagctggtggtataaacattcctgggtaccaaaaatgtcaaagtcgtggaacgcaatcagcgaggcgatcaccgggaaccgctgtttccagccattgcctgcaatggaatcgtctttgttgttatcattgcgcatattgtaggtggctacattaaacttttgcgcttttaccccgtaggagaaaatgactacacaggccattaccagcattatgcttttcttcatctgttgctatttatacggttatcaatactactcttcccagcctggattctgcagcaggtttggattgagctgaaggtcgttgtaaggaatgggatacaggtacttgcgttccagccattcttttggtacgttatccagccaatgcagttcaccgtaagtgccatgcgacagctgctgtggatttactccgctacccagttgaggagatacgttgatataggtaactccctttacaggattggccggcatcgtttgatagaagcaaacatccaatacgccatcgctgtcgagatccatcggcacattcagcgccggcacgtacataccgttccaggaaccagtgagcaacggcgcctgtctccatcttaccaggtcataaaaacggaagccttccagtaccagctctatgcctctttcccgcctgatttccagcagggaaggatcggtaatatcgttaaaataattgctttttaaatagctatcaatgaccaccggtttactggcaataccaccggtaataccggcacgggcacgcagtgcgcctacggttattttccagtcatcatcgctgagcagcttcagttctgcgcgggcctccgcatagttcagcaggatttccgcatagcgcatgaggctaatagcgttgatgttgttggtaccattatcgtaataagtgtcgtccaggcaccatttaataggcatataacctgtataggtatacgaaaataccggcggtgcagacaccacagttccgttgctggtgcgcttgtatcccggcgtgcggatggtttgctgaaggcggttatcgcggcccagtgtttctttattaaacggcagcgtatcatatcccggtgtgctggtaaaaggcgtaccatccacattgagataagtgttcacaaatttgcgggtgaaactaagccgggagccataggttgcgctggtataccaccagttggcatcgttaaaggcgccgagactggcattggcaatattggccagcatcacttcagcggtaaccggcgccgtgctggtaaataattgccgatatgaggccgtggcgccaccgatctggttcaaactaaacgccttactatcgatcaccgttttagcggcggcggcagcggcggtcaggagactgtcggccccacccgccaagcccagctgcgtctggtatttgcggaaggtgccttcaaacaggcatacgcgcgatttaaatccgtacaccacatttttagtgatctggctgcaggtaggatcattggtgagcgtaatattggcagcggcgtagtccaggtcggcgatcacggagtccatgatctttgtacgcggatcacggcctgcatataacgcgggatcatctacttcaaagggtttaccaatccagggtacattgccgaaacgttttattttatcgaagtaaaagtatgccctgaaaaaacgggccagtccgaggtagttatttcttattgcttccggtacgcgctgatcagtacagttggcgataaaataattgatgttgcgcaaatttttccagtcccatcccgtagcagtcctggaagtatatccgccctgtcgtaaaaaatctggaacggaattcacggcactgtaatcggccattccgtctgctttatagatatcattgataccgggtagtacgtcgtagaaagagttagcatagagtttcagaccatcggcacttccaaacacggcgtctttagtggcggtggataccggcgattgatccaggttctttgcacaaccggtcataaacatccctgctgccagtatcagtgccgcccttttccggagtaatgcagttatatattgttgcatagcttttcctttttatttatcagagtgtgatgttgatcccgatcgtatagcttttcaaaatgggataattattaccattaccggaactgttctgatccgttacagcatcggaacggcggatactttccacatcaaggtcgcgggtaactttatacagcggcgaccacgaccagaggttttccgcggagagataaacgcgtgcggacgtcatcctggcacgcgataccagcgagtgtgggaggttataacccagctgcaggtttttgagccgtatgtatgccacattttgcaggtattttgattgcggcgggtttaattcacccgcgccgttttgcgccacatacccgcgatagcgtgggaagtatgcatccgggttgtcttccgaccagatctttccctgctgtgatttaggcataaagttatagggcctgttatactgtccccagaatacatctgactctgatcccggccaccaatcctgttgtaatacaccctggaagaaggcgccgataaagaagttattccagtcggcgctcaggttgatgccataggtataccgcggcagggtatcaccgatgatggtaagatctccatgctggctaagtgtatttgcaccattattaatattaggatcgccgtccaggtttttaaaccggatatcgcctggcagccattgtccgctgttggaggctttaaagagggcctgtgttttggcggcctgggatacgttatcttttgtccagtagccatcgttggtataaccccatatttcaccgaagcgctgccccacataataatccgtgagtttattattggtgttgttgtatttggtgatggtggctttataatcggccatagaaacgcttactgcgtagtgcagtggctttgctgctacattaaactggtctttccaccccacagttacttcccatcctactgttttcaggtcggcatagtttcctttgggtacatctgtaccaaatacagcgggaagtgtttgtcctacggtgaacatatttttggtgattctcgtataggcgtccccgctaatggtgagatggtcattgatagcagagaggtccagtccgaggtcgcgggtggtggaggtttcccaggtaaggccatccggcagcaccacaggttgtgatgtttgttgctgctttacaccgttgatcacgcgggatgattgtgtgatggccagtttttcctggtaggcgtaggatgccacattaccattacccagggaaccataggatcctcttattttcagatcggaaataatttttggtgatactttccagaaaggttcctgtgctacccgccagcctgcggatacggaggggaagaaagcatagcgctgatcggaaggaaatttcgacgaaccgtcgtagcggccgttcacttccacgaggtagcggtctttatatgcatagttcaaccggaagaattcacccatgatggcccagcggtcgtagccgccggtggtgtttacattggtgccgagcgcgagactgagatctttggcatcgctgtacaccaggccgttgcgggtggtagcgaatcctttgtaggtcgactgctcatagttgaacccaacgagggctttaaagtaatgcacatctcccccaaaacggttttcatattcaccatacagattagaggcgaggtagagggtattgtaattgctcatcataagatcgttgtaggcgttgcccacataagcaattacacctggcgctgcgctgtaaggtacgggtacgcgtaaacgtttctggttatcggcggtattctggaaggtaaagtcgcctttcagcctgaatttatctttataaatatttgctataaagccggtggtgtttctgaatacctgtttgttccagtcgagtccgtttttaccataatacatatcccctaccgtgtaagcggcagaggcggtgagggtaccatccgggttgagcagcatggaagaaggatgcgcttcatcggccatattgcgccagataccacccccttcgcctacgttgagcgggttgtgataatccctgttggaaaattctgtattgttatacacctgtaaaaaggggaacagctggatgtttccttttgcgcgcaggttatacattttataatcgtcggtgttaaagcggaacaacccatcctggccataataacgacccgtgaggtagtagctggctttaccgctgctgccggaaacggtgagattctggtctgtagcggtggtatggtttttatatagcaggccgtaccagtcggtattgccataatactcatagttacctgcggcattcacgattgtttttggcagggagggatcatcctcatgcgctttcagggcatccaggtatgctttggagaagggttgtgttttattgatgttttgcggcgactgggaataatcattccaggcgctccaggcctcattgaagtttttggcatattcgtaaccgttagtcaccatatcgggaacggtagtaggctttttaatagagtaattagaggagtagctcacactcagcctgtctttcaccggtgtttttgtggtgatgagtaccacgccgaatgcggctcttgcgccataaatggcggcagaagatgcatcttttaatacagtgacgctggccacgtcggcggggttgagcatagccggatccccttctaccccatcgataaggataagggcacttcctccctgtccgatagatgttgtaccgcggatattataggcgggcgactggatcggttttccatcgccgggtaccaggttgaggttggggatcatgccctgtaacccctgactgaggtttggaagcgggcggttttccagtactttaccggatacctgtgcaacggccccggtaagatttgctttcttctgcgtaccgtatcctaccactaccacgtcattgaggttggatatattatcttttaatactacctggatattagtttgattacctacggcgagggtatccggtttgtatccgacaaaactgaatatgaggcggtcgccggcagtagcattgatactgaaattacccttggtatcggtgttggtaccggtgcccgtgcccgacagtttaatagacacccccagcaacggctggccggcgtcgtcgaccaccctgccctttaccgggtgcgattgcgcagtgcttctgaatgcgtagcctagcagcagtagaatgcataaccatctcttcatggtgattctttgattttgtagatcaggaataataaaatgtctgctgcaaataaggaagtgcgggttaacgggcgggttaactggtgattaatggcgtgaattaacccaaaataaattatgaaatgcgtgtataatcgcctaaattaacactagaaaagtttcttaaactaaagttaactttcagatcggagataatacttatttagcgagtaatttgccacgttattgaaagccggtgacccgcttttaccataggataattgaaaaattcttacagcaataattgtaaggccgccaatgtacagatctactcttttgttattaacgttactgactattactatcatcagcaaagcccaggaagcttacggactggagtttgcgtgcaagaatatcccgcaggaatcgcgcacttcccttgatcttttccccgggcaacctttggttgtgaaagataaatatgccctttcgtttgacctgtctttccttcctttttcttcttcctatttcgggtatattttccggataaccgatgaaaagaaacaaaatattgacctgatatataatgtacatacgtatgcgtttaatgtggttaccggtaatgaattttccgggatttcttttaagatagaccgggattccctgtaccatcaatggaataacatccggctggacattaacacccgtgcgcatacgctgctcgttactgtaaacgggaaagcagtaaagagtatccgtcacccggttatttccggacaccagctgaatatttgcttcggcgccaattaccgcaaaacattcaaaacctttgatgtagcgcccatgcggctcaaggatgtgaaaatttccgccgggcaggagttgctgcaccactggccgctggaccaggtaagcggtacggttgcaaaagatgggttcaccgggcaaactgccaccattaaaaaccccatttggctgcggccacaattcaccgaatggcagctggccgactccttttctattaacagcaatgccagtgtagcgatgaaccccgctactgaaaatgtgtatatcacggggagggattccatatatcaatacagttgcagttcgcacacattggctgccagtacgctcgggcagccacaaggcactcccgccgggatccggtcggcatacgacattgcgcggcatcaactgtacaatttatttcccgacaggcaacaggtggcccggtttgattcgggtaccgccagctggagtcagtctattgatgcggatgcagtaaccaactactggcattccaatattttcttctccttatacgacagcgccatttattcactgggcggatatggcgacttccgctataaaaatgaggtacaccggtatgatcctggtcatcagaactgggataccgtacatgtaaccggcgactttttcacgccacgctacttagccgccgccggcgccaacaacgcgggggattctgtttatatactgggtggctacggcagtattaccggtgaccagctgctgaatccacatgcgctgtacgacctcatgctgtttgatgtaaagcgcaggaccttcaaaactatttataagctgaaggaaccggaagaaccttttgctttggccggtaacatgatcatcaacagcgcgcaccaggaatattttgcactgacatttcccaatgaccgcatgaattcttccctgcagctgatccggggttcgctgaaaaaccctacatatgttaaaatggcggccagtttgccgtacaatttctacgataccaaatcagctgcctacctgttctattgcccacaaaatgataagctggtagccattaccttcttctctccaaaaaataacattacaaaggcaaaaatatatacgcttagtttttcaccttacggccttgctgtaaaagcccccgccaatgagcgtatacccgaatacgttatgaggctgctgctggcaatagccattgggttttccctgtttttgctggcggctggaatttctgctgtaaaaattaataaaacagtaaaggaagatgatgagccggtaatgcccactgagccacagcaggaagcgccagcgccgccggtaccggcaacaactatccttcccgcgcaaccagcatcggctgtttatttattcgggcatttcacggtactcgacaaagaaggcaacgatatcacccggttattcagcccgctgctaaaagaactgttcctgttattattcctgcattccttaccgggtaaaacgggtatatcttccgaaaaaatcaatgaaatactatggccggggcgctctgtgaaagatgccaaaaataaccgctctgtaaatattgtgaagctgaaaagtattctcgataaaaccggcgcctatacgctcgcaaaagaaaacgataaatggatctttcattttgacgatccgcagatacaggttgatctggccgagtacctgcacttattgtccgttattacaatcgatggaagcaatattcaccgggttgcagacattgtaaaaagaggcgcttttttgcaggaaacagaatacccgtggctggacaaattcaaagcggatatttccgcgcaggcaattccgctgctgatccaccacctggaggaacatgcagcggagccggaagaggtgatcagtatctgtgattgtattctcaccttcgattcgctgtgtgaagaagcggtgatgctaaaatgcaaggcattggtaacgctgcggcagcatgcgtctgcgaagaaaatatacacttcatttattgccgagtatgaaaggatttacggagaaacgtttgagatagaatatacgaaggcgatagagcaatattaaattaagaaggtgtaccatccgatacaccttcttcttacaaccgttggcggatcactttcaccgcatcccctctttccagttcattatgctcctgccagcggtcctgctgctgttttaccagctcgtccgtttgccaggcgaggaactttgcttccagccgttccaggcatagctgtttattctgcagttgtgagcggctgtccattgccagcacctgtaatccgctggggcggtggataccacgtacggcggtttccactttattcacatgctgaccgcccggacccgcggcccggcaggtttccagcgttacgtctttcggattccactgcacctgttttttgatatcgaatacagatacgcccacgaaccagtttttacgtttgtgaaatttacggtagggactttgtgcaatccactgcaccgtaccttcccacgatccgcaaaaagccattacatttttccccttgagcagcagcgtagcagaaagcagggtaccgttaatatctcctttgatattttccaatacctgtatgctgatgcctgctgcgcggccttcctttatcattatttcctgcacctttgccactaccctgcaacattctgcagggccgcggcccgaggtgatctgtataatcatttgttccatgttgttagtctttattcattcttacaatggcgggcataaaccggccctgtatgtctactaattcctgttgtgcgctgataacatcttcaatgtctttatacgccagcgggttttcttccacgctgccgccgatgagggtaacacctgcagcggccagcatttttttcaaaccggatacggtcatgctttctttggcccttttgcggctcatggccctgcctgcgccgtgggaggcggagtataaagcattgtccacgccctttcccattacgaggtaggctgcagtgcacatgctgccgggaatgatgcccatttcgccggcatgagccggggtagcgcctttgcggtgaatgatcacggactgaccgtttgccagagtatcttcccaggcaaagttgtggtgattttccacttttgcgagcgactgcaaacccagcgccttcatgaggttgaggtgaatgcggtcgtggcacgctttggcataatcaccggccaggttcatggccagccagtattcctgccccgcttcgctgttgagatccagccaggccagctgttgcgccgactttggcagcttgcaggtgtccatagcgatgcgcgtgtaatgctgcgcgatgttagcgcccaggccacggctgccggaatgcgacagcaatgccaggtactttttgggtggcagctgcaaggcattgtcttccttcagttctattaaaccgatttccacaaaatggttgccgctgccggaagaacctaactgccgcgcagctttggcttgtaatttccgcaacaattctgtcgactggaacgctgtgctgtcgagcacttcatgttcttgtggaaattccaggccgccttccatgccaaagtgcgtgtattctttcaacgccacttttacctggtgggagaagcgttttaaaaagctttcaccttcatcaaagatggtgagcgccattcggcagccaatatccacgcctactgcaaacggcagcacggcattatctgtagccagtacgccgccgataggcaggccgtagcccgtgtgtgcatccggcatgagggcgccctgtatggtaacaggcaaagacatcgccgtttccatttgttgcttggcggagcgttctatttctttggcgccgtatactttcagctggcctgttttttccagcaggtcgtacgactgaaaattgcattccaccggttcatccataaaggtatcagctatttttcccagtatttcgtgggagcgatagctggccggatcagctttgatggcggttaacagcgctataagatctgtcttcgtttcgtgtttgaaatgctttgatataatattgatgacgaggcttctggcctggtcgtttgtataacctattttactaagttcttttgtttttatactgcccataaaaggtaatgtatgtgccgtgatgcggcttttaaaggcacatcacggcggcgccggtaacccggtgcggtattaaatataaatgaatgtaaatgttgttccgtgctggaacacaccttccgctgaaaggagagataaagcaaacggaggcactaacgtatccgtatatacgaaatgtatttatacaaaaagtataagatccatacaagtattattccggcttatgtaaaaggtaagcagcaacgtttgcctgatcaggcaaggagcgaaaggagcgatatgtgggtacgttctgtcatgattccttgtattttaaaaagatgaagaataaggaattcgggtgcaaagatatagctattttataaatacagccgcatttttttcacataataattttagcgcagatagtcgcagattttaacatttctccagcctataaaaaagggtttataactgtgcatgacgtaaatttgtatgtacccgcatttttaacctccggaacccgctccggacgggctacatcaacattataaaactttttcttatggacaaacagctcatccgcaacgcctataaagtgtactggctggaaaacggcaaagcgcccgtttctgtttatgcgctctgcaaacttgtagacgtttctgaaaccgaattctatgaacaatacagttcactggaagcggtagaaaaagatatctggttagctatcttccaacaaacattggatcaactgcatgcagatgaaatttatcagcaatataatgcgcaggaaaaattgctggccttttatttcctctgggtgcagaagctgaaggaagaccggagttacctgttattgcagcgcaaacacttccggttaccggacctgtaccgcaacaaactggaaactttccgtcacgcgtttaacaagtatgtaagcgacctggtaaaagaaggttatcaatccagcgaaatcaaggaaaggaaatatatctccgaccagtatgtacatggtttctggttacaggccctgtttgtgctgaaatactggctggatgataccagcaaccagtttgaaatgaccgatgccgccattgaaaaagcggttaacctgagcttccagctgatcaaatccaatacactggatagtttgctggacttcgggaaatttatttttacgcggaaataagcatcatgaaagaacaatccaatattcccacttccaaagtggaaagggcaggcaaattcgttacgacaggatttaaggtaggtaccaactatatcaaacactacacccgcaaactgatggatccttctaccaccaaagaagagcttcaccaggacaatgccgcggatatttacgatacgctgagtaacctgaaaggcagcgcactgaaagtggcgcagatgctgagtatggataaaggcatgctgccgaaagcctataccgaaaaattcgccatgtcgcaatacagcgctcccccgctgagcggcccgctggtagtaaatacttttgtaaagacattggggaaatcgccttcacagctgtacgaccagtttgacctgcaggcttctaacgccgcctccatagggcaggtgcataaagccaccaaagatggtaaaaagctggccgttaagatccagtatcccggcgtagccaatagcgtaaagtcagacctccgtattgtgaaaccctttgccatccgcattgtgggcatgaatgaggtagacatggacaaatattttgacgaaatagaaagtaagctgctggaggaaaccgactacaaactggaactccgccgttctatggacctttccagggaatgcgcgcatattcctaacctgaaatttcccggttactaccctgaaatgtcgtcggaccggatcattaccatggactggctggatggtcagcacctgaaagaattcctgctgaccaccccctcgcaggaagtgcgggataaaattggccaggccctctgggacttttaccagttccaggtacacagcctgaaacaggtgcatgcagacccgcatcccggcaacttcctgatgcgcccggatggcactgtcggcatctttgattttggttgtgtaaaggaaataccggaagatttctatgagaattacttcctgctggttgacaaagaggtgttaaaagacgagaaacgccggcaccagatctataccaacctggaaatgattcatccgtcggacagccccaaagaggtggaattcttctccggccttttccagcatatgatcgatttgctgaccctcccctttacgctggacaactttgatttcggcaacgaagtttattttaatgaaatatatgcctacatggatgaactctacaatatgaaagagatccgtgattcaaaggtagcgcgtggctccaggcatagtctttatattaaccgtacctattttgggttatactccattctgagcgacctgaaagcgaatgtgatcaccggccccgccaggatacaggagctgatgaccgccaggaaaattgcttaacaggctttccggggaaaatcccggaaagctttgttcttttccatgttagtcgtagaattatcacaattggtcgcaactctgccttgataattacacaaatcccctaatttgccgccatgaaacaggaatggtaccagcagaaatgggcaataatagcgaggcatgtcctcgcatggctgatattcttctctctcccctatttgttacatcctaccaacgaaaagtacgaccgggaccgcatggatgaaaaacaggcgtgggccatgtatctgtatttcacgtacctgatattggtggtgttcttttacctgaatgcctgggtgtttataccgaagctggtttataaaaagaagatcgtcgattatatcctttacatcgtaggggtatttatttttatgtgcaccatgcggtatggttttgaaaagatattcctgaaaccacataacatagatattaaacccgccatcctgttcactttcttcacttttttcttcgtactatcggccagtactgccttccagatgattgtagataaaatgaagctggaaagacaaagcagtgcacgggaaaatgaattgctgaaaacggaattgtcgctgctccgttcgcaggtaagtccgcattttatgtttaatgtgctcaacaacatggtatctctggcgcgtaaaaagtcggatgtgctggaaccttctctcatcaagctttcgtcgctgatgcgttatatgctgtacgaagcggatgaggacaaagttccgctgcaaaaggaaacagaatacctgcaaagttatatcgacctgcagcagcaacgtttcgggaaaaatgtaactatccaggtatcgctggaaacgggcaacacctgttatgaaatagagccgatgctgctgattccctttgtggaaaacgcttttaaacatggtaccggcatgatcaccgatgctacgatagatatcaggctatatacgcgggatgacaagttatttttctctgtgcagaaccggttcaataaagattcttccgaaataaaagataaaaccagtggtataggtcttaccaatgtaaaaaggcgtttgaatttgttatatggagataattatgttttgcatatagataaaaaagatgactggtttatagtatccttgcaattaaatctccactgatgatgaaatgtatcgccatagacgatgaaccgttagcgctggacctgctggaagacaatatcagcatggttccgtacctgcagctcaccggcaaatgcaacaatgcatttgaggcgatggagattttgcggcatcagccggtggacctcatcttcctggacatccagatgccgggacttacggggttacagttcctggaatcgctgcccaataaaccactggtgatactgattaccgcttatgaaaaatatgccttgcaaggcttcaacctcgcggtaacggattatcttgtaaaaccggtgtccctggagcgttttatcaaagcctgtaataaagcacaggagcttttcctgctcaaaacaggtggaaaaacagcccgggaagaagctgatttcttttttgtaaacgtagactacagcctgctgaaagtagtatattccgatatccggtggatagaaggactaaaagactatgtaaaaatccacctgaacagcaaccccaaaccggttattacacgcatgagtatcaaaggattagaggagcagttacccggctccaggtttgtgcgtgtgcacaagtcgtatatcgtttccattgccgccatcactgctatccggaaaaacagtgtattcctcgacacgctggaattcccggtgggcgacacctatcgtgatgcagtatatgctattgccggaaaggccggtcagtgatccgacagttcgtagcagttttttccccactcatctcatttaatttattttatccatctggcgggtatacttttgcatgatctgaatttatataaaatgcaaaagatttatttgtttatcaccctgtttttgctttcaatgagtgctgtagctcagcctcccgcaggcgccaaaatgccgatgggtatgggaatgagcggccatgtatatggcaaaattattgaccccgatggtaaagccgttccttatgcttccgtaattatcctgcagaaccgtatggatagcgccacaaaaaaaatgaaggaaaaactgctgaaaggcgtgctgaccaaaggcaatggtgagttcagcctggaggatctgcccggcaggggcccgctgaaactgcggatcactgccaccgggtacaaaactgtggaacaagcggtgacctttcctccttttgaaaaggatctcggcaatattaagctggcggtaagcaccacccagctgcaaggcgttactgtagccggcaccaagccgctgatgcagatggatatcgataaaaaggtatttaacgtggagaaaaacatcgtcagcgccggtggtaccgcgctggatgtaatgaaaaacgtgccttctgtaaatgtggatatcgacggtaatgtaaccttgcgtaacagcgccccgcagctgtatatcgacgggcgcccgaccaccctcaccctggaacagattccggcggatgcgattgaaaacgtagaagtgatcaccaatccttctgccaaatacgatgcgtccgggggtagtgccggtatcctgaacattgtgctgaaaaagaaccgcaaaacgggttacaatggtaacctgcgtgccggtgttgataaacgcggcgctgtaaacggtggagcggactttaacctgcgccaggataaggtaaatatttccgccagcgtaatgggcaaccagatgaaaggccgtaccaatggtaccaccgagcgtaacaactttgcagatgaaccggccaccaacatcaaccaatataacgccaacaaaacagatggcggtttcgtttttggtaaacttggactcgattggtttgttaccaaccgtaccaccttgtctgtggccgggatcaaggtgcatggctccatgaatccttctgaaaggatcgatattaataccgacaccctgaataaagccggcgatataaggtccttcagtcagcgtaactccagttcccataacaagttcaacgctaacggcgtggtattgggcatgaaacacctgttccctaaagaaggggaagaactgaccgccgacttcaattattttggcggaaagagcgataataactccgactaccggaccgaccgttatgccggcagcaacatcagcggcagcgatatacaacagatcctgggtaatggcgccatgagctttatgaccatccaaacggattatgtaaagcccttcaatggtaaattaaagctggaaaccgggttgagagcctctgtccgtaaaattaagagcaacttcaacaactatatgctggacccggaaacaaaggaatatgtactgatacctgccgcctccaataattataaaaacagtgataatgtatacgccgcttatgtaagcgtatccaacaccattggtaattttggttataaagtaggtgtacgtgcagaaagttccaactacacgggtgatctgctcaacaacggacagcatttctccaacaactacccggtaagcctgttcccatccctgtttttaagccagaagctgaaacacgaccaggaactgcaggtgagctacacccgtcgtattaaccggcctaacttcttccagctgattccgttcaccgactctaccgataagctgaacatcacaaaaggtaacccggggctggtgccggagttcactacttcactggaaatgtcgtacctgaaaacgctgaagggaaacaataccatattggcatctctctactacaggcataccaacaacctgatcacccgttacctcacaaaggaaaccgatccggtaaatggccaggaactgctggtgaacacttatatcaatgcgaattccagctattctgccggtgcggaagtgactgccatgtataatttcaccaaatggtggagcgctaccgcgaatgtgaatctctacaattcgaagatcaatacagataatgtaacgcaatcgcaggatgcgctctggagctggtttggtaagctcaacagcacctttaagctgccggcaaattttgaagtgcagctcacaggcacttaccagtcgaaaaccaatctgccggtgaatgacaacaagaacgtgcaggccggtccgcctatgcagcagtcgcagaatgcttcacagggctacatcgcctctttttatggtgtagatgccgccatcaaaaagagcttcctgaaaaacaatgcggcttcggtgacctttagcataaatgatatcttcaggacacgctggtctgaccaatattcacaaagcgattatttcacacagtattacagccgcctgcgcgacccgcagatgatgcgcctgacatttgcttaccggtttggtaaaattgacgccagcttgtttaagagaaagaacatgggtgcaggcatgcagggaatgcaggaagtgattcagtaagaagttgctttaaagtttaaagcaccggaatgcgagggcattccggtgcttttttttatggattccggccgttctcccccggatatagcaaatacacggcatcactttgccacacttccttcgtatccacattcatggcggatattttgcctttgaaggccgcgccggtgtcgatgttatgcacattgcaggcgatcatggggagttcctcaccgtaattaagactaggggtatgaccgatatagatttctttgaactgcagcagtcgttttggataaaacatagagttcttcggaatgctgcggtccattgccagggcgagttcccacaggcttcggtcccaatagagcatgggttcaaacctttcatgggcggggccgtgggtggaagtgaaccctgcgtgtatatacaacctgttttggtcatcgatgtaatacatgcgcatgcggttcagaaattccttgtggccttccagcgctgcgggcgataatttattgaagctgtctaccgtagctttgccgccgttgcgttgccatgaggcttcgggcattatgccattcagccaggattcgcaccaggcgtcgtggtttccttttataaaaatacaggtgtgttgtgatgccagttccatgagccaggtgatggtttcggcagactcagaccatccatctacataatcacctaaaaaaatcagtgtatcggttgttttcggcgcgatacgctctaccagctgtttgagggctttcagcgcaccgtgtatatcacctattacgtaggttgcgggcatgttttgttttatttgtacataatgtctgttcgcagcacatatttcacaccggcggtaagcaatgcaccttcatgccgcagcgggtgatgaaatatcagggcggtacctgtttccgggcggataatttcgccggaagcaaaaatggtttccccgccggtatatgcttcgttcagatagatcataaaagtatactggctggcttcaaacctgttccgctcaaagctgccgtccttgtgcattttgaagcgttgtcccgggctgtatttatagaaccggaacaactcattcacaccggaggccgttctgttttcttttccttccggagcaaaatttttcagccgttcccagataaaggtagcataagccaggtctttatacaagacccgttcattatttcgtacaccttttatcatccgttgtacaccgccgcctacgtctacggtggcttcctcgtagcccattgcttcacttttttctatgagctgggcgcattcttccgtgctgaggaaatttttgacggtaaaaatttcggaggtgtaagtgattttttccataacatcaggtttcagtgggaatattgatctggaaactatttttcttcagttgtttattgaacttgtacagttcaggatgcctgttcttcaacccttcgcgtttcaggccggtgttgatcacgtaggcggcgtccaatattttgcggcggaagttgcgccggtcgatggttgtttgcaggatacactcatacagttcatgcaactccgtaatggtaaacagttcatccagcaattcaaatcctacggggtaatactggatctttgaccggagcctttgcagcgcctgtttaaaaatatgtttatggtcgaagcccagggcaggcattttcctgacattgaaccattttacatcattggccatactaccagccaccacatcgaatttagcggggttaatgagtgcgtaatatcccacagctattacgcggccacgcggatccctgccgggtgcgtcaaaggaataaagctgttcgagaaatacttccttcatgcccagcttcgtttgcaggatgcgggaacaggtgtccaggaaggtctcttccatttgcaggaagccgcccggtaaggtccagcagtctttgaacggctcctccttacggttcagcagcaataccgacaaggtattgttgtggtaaccaaataccaccaggtctaccgccagggaggggttcttatactcgtggaaagacttcatactctgtttgcgtcattttaacgtgaagtaaagattttttagggagataacctaaaaatgaggggattttatctgtaaacaaaaaggcggcgccgaagcaccgccttttttatttggacccgggataggattattccagtcatctcataacctacaactgttacactgttaaagtaacaagatgcaaatatacaccccggtatctatataaagtagaccgctatcccgaaggttaccagtatttatggatgatgggccaaagtcaggatatcttttacttccagcactggtttcttatagccaaaacgggtaacattgatcattgcctgccctacttctgccagcgtggacacccactgtggaaaaacccgccggaagaacggataagcccaggtcatatacttgtagtatttctgggtatacctcagtccatcggtaggcagcatgaaccccggcctgaacatatacgccgccttgaacggctgcttcagcaggtcgttctcggttttgccctttacccgcgcccacatgctgcgccctttccccgagctgtcggtgcccgcaccggaaacatagcaaaaggtcatatctgaattgagcgcggccagtgttttagccacttccatggtaagatcataggtgacccgcttataccggtcctccttcattcccacagaagaaacacccaggcagaagtagcaagcattatatccatgcagctttgtagcgataggcagcatgtcataaaaattttcatgaatgatttcctttagcttgggatgctgcacgccgcagggcctgcggttaatcaccaacacctcctttacatccggatgaagtaaacattcgtgcagcaccccttctcctaccatcccggtacttcctgtaataatggctcttatctccataggaatattttaatttcagatatccctgaatttaaacctttcatttaacttaataaaatatctatgccgggatactgtcattgacttctctttcccagaaacgatgctgtgcaatggcgtttataaagtcatcactacttttgttcagtaacagaccaggttcattattttctgtttgcagataggttttcttcagcacttctacgccttcaccacttaccgcaatcgccttgcaatgtttataggcttcgttgataaaatgcagcgctgccggctctttggctaacacggatgcactggccttgcctcctggtacatataccgcatcaaacaatacagatgccgccataagaaagctctgatcggcttcgaggtctgcgccgccatctacctttatgatacccagctttggcgcaatcaactgcacctgcgcttctgcggcctccagatctgctttcatctgagcgatgtctttgccggaaacgccgtctgctaccaggaaagccacctgcctcgacttcaccgtatttttcacggtattggccatgctcaacgccggagaagtatctacctgctgttttacggttctcggctcgtaactttccacatccgcatccgcaggccgtatgtggttaacaggatactccggtttctccgggactggtaatcccaggccttcagccacctgcgcggcaagtgaccggtcgacctgtgtcaagaccccgaccatccgctcgcgtatatccgtacgggttactttgccaagttcaaaacgcagggcgttgatcaaatgccttttctctgcttccgactggctgttataaaataaagcagcctggctgaaatgatcaaagaaactttcgctgcggccacggatctttttagcatctattctttcttcataagaagtaaaaccgccgtctttcatttttgcctggaaaggacatccattgctgatcgtattaggttcataagcggtttcacctcggttgatggtttgccgcatgtgaccatcgcgctgattattatgcacaggcgctatcgggcggttgatggggatttcgtggaaattgggactgcccagtctcgacaactgcgtatccgtataggaaaataaccttccctgcaacagcggatcattggtgaagtctatccccggcacgaggtgcccggggtgaaaggccacctgctctgtttccgcaaaaaaattatccgggttacggttcaataccattttaccgacacgcatcaccggtactacttcttcaggaattattttggtaggatccagcaggtcgaagggaaatttatgttcatcctcctccgccactatctgcacgcctaattcccattcgggataagctccggattcaatggcattccacagatcgcggcgatgaaagtccgggtccttaccggagatcttctgcgcttcatcccatgccacggaatgaacgcccagcaaaggcttccagtggaatttcacaaaactgccctcacctgccgcattgataaaacggaaagtatgtacgccaaatccttctatcatacgcaagctacggggaatagctcgatcgctcatcacccacatgatcatatgcatgctttccggtgcgagagatataaaatcccagaaggtatcatgcgcggaagcagcctggggcatttcgttgtgtggttccggtttaacggcgtgcacaaaatccgggaacttcatcgcatcctggataaaaaacaccggcatgttattacctacaagatcataattcccttcatctgtataaaattttaccgcaaagccgcgcacatcgcgggctaagtcagtagagccgcgtgagcccgctactgtggaaaagcggacaaataccggtgtttgtttcgacggatcctgcaggaaaccggcctttgtatacttcgccatagactcatacacctggaaatagccgtgagcggcctctccccgtgcatgcacaattctttccggaatgcgttcgtggtcaaagtgtgtaattttctcccttaaaataaaatcttccagtaacgacgcaccacgttcgcccgctttcagcgagttctggttatcattaatgcgcactccctggttagttgtcaggaattggtccaccccttcttctgtatgcggggtaagactatccactttcctgtttgacgttccgataataggattttttttctttgccatggttttggtgattttaatgatgaggcaggacccaatcattcacacaaaccatacctattcaaaacgcattttcatctcccttaatcgtattcctgatcgttaaaaatataatacggagatcgagatatacggaccagttttccatataccagatatcatgttcaatccttttgcgcagatgcgattcttccgtaatttctccacgcaggccgcaaacctgcgcccatccggtaataccgggtttcagaaaatgacggatcatgtattgctggattacccgggaaaattcttcggtatgacgaagcatatgtggccggggacctacaatagacatatcacccataaaaacattgaggaactgcggcatttcatccaggtttgttttacgcaggatacgaccgatccgcgtaaaccggctatcatgccgcgtagcttgcttcgcgttcgcttcgttattcacatacatactccgcagtttcaaacatggaaaattcaggttattacggcctgtacgatattgaataaagaacaccggtccacgcgattccagcttgattagcagcgccagcaaagggatcagccaggtaagaataaaaacaattacaagactgctgaagatgatatcaaacacccgtttacggatgcggttggcaatatcatccaacggttcagaacgcaatgaaataatgggaatgttattaaagtaatccacaaagatctgcctgtttacaaacaacttgaaatcgggcacaaagcggaaatgaatcaggtttaattctgcttcccttgccaaagtatacaggtaaggaaatttttcgggagataatgtggaatatatttcacggatattgttagactgtgcataaggcacgcaagcttccaggttgcctatcaccgggtagtaagacaactcatgcacgttgctgtattcttcaaaataaccttcaaacttgagattgctgttatctcctatcaactgatccgccagttgtttggaaagatcattatacccgaggattaccactttcttttccacgccgctgcgatgcaggatatgccgggttaccttgtaaaaaagccaccggcccagcaataccatgcacaggaagctggagcaatagctcaggataaacaaccgggaatataactgcttggtcagaaacaaggacaacaacaacagcaacaggtacaacaatatgctctgtatggttttgcgggcgattcggtcaaacgacaactgctgactgaggaaataaataccggtagtgtataaagcaaccagccaggagagatttgataccacgaggaaaatatccacattaatatcctgcatgcggtcgtaccgctgcaaccaggagctggttaaaaaaaacaatacattcagccagataaaatccagcacaatcaactggatactgcaaattttgagataccggttcagcataaaatagaatatggttgatcaataaaagaaagcgctacgccacctgttctttaaagcgcgtcatcacacccgaaatggaaaggtggctggctgcaaattcacgggcattccttgcaatgtcggcagtattttcccatacggccctgcctattcctgtttgaagggcttcctggttttccgcctctacgaggatgcccatctgatgccggcttaccagctcatgcaggccggtaccctcattggccgtaatcagtgcaatgccgcccactgcaagtatggtcgttagtttggatggcatcacgagatcgctggcatgtgatttttgtatgaccaggtgtacgtctgccatgttcaaaaagttattaaactgtgcaagcggttgcaatggaaaaaagatcgtgttctttaactgcagttgcgatgctacctgttccagcttggctttatatgggccggaaccacagatcaggaatttcatttcttcccggtgctgccaggacgcagcagcatgcagcagggcttccagcccttgtttttcaccgatggcgccggagtacaatataattttatcagtgggcaaaaaaccgaacgactgctttaatatagccttatccgttagcggatgaaattgtgttacatccacccagtttggaaaataaaatacttccctgcccgccttgtcacttattttacggatcatcccgtctgctatgctgcttacatgatccgcctgccggagaatcatcttttccagtttcagcagcgtgttaatcagccgcggggagcggatcatctgtaaatcgcgcgcggcctctatttgcagatcctgcacatgatacacgaagctggcgcctcgtagttttttatagagaacagccagcaaccccaggtgaaacggcggcgccactgtaattactatatcatatttctttttccataccagctgcatcacttttacgaatgcagcggctgcaaaagaaaaatcctgcaacattcttttcttgccggaaggctctgcaggcacatattgcgggcaacggtacaccgttaattttccctttccctgcggatgtacttcttttttaaaccagttcttggagcgttcatagggcgattgcacctgccattgcggataataaggataagtagttattaccgtgcagtcgtacccgttatctgccagccaactgatcatttctccgttgtactttcctattcccgttggctcgggtgaaaaattgccgcctatcagtaatattcgtttacccatatacgttatatttaaatattatttccgccaactccacaatacccctaacataaatcccacgttatcggagagctgtccctggtccactgctatggatgctttcagggcaagtcctttcgacgacacctggtactggaactcctgtagtgtataccattgccgtttcattggtttgaaaagggcggtattggtgtaggtaccataattctgtgtgtaggtaattaatgttctgccggtaatttttttcgggagatgataaagtgcgccgatatgcactcccattacacgattgttaataatattccctccttttgctctcagcgaatccttgggatcattccaattgaatggcttcatgctggggaagtaatactgtccgcgatcccggtcgatgaacaacggcgtgccgatcacgcgctcatgataatcccagccggtaaggtatacgccgttgttgtagtagctttcgcgctggtgcaacgggaagaaatcattcatctgtttcgtataaagaaactctgctgtaatcttctccagccagctgccggcttgcttattggtatacacaatgcccaggagccggtcgatgttccggatatcaatgccctgcccggattcaaaaggagtttgattatacaggcgcagcgacaactggtcgttttcccactcaatccccccttctataataccgcggtgatcgccgggacggttaggctgtatatcggtggtgccaacggttccatcatccttcgtttttacaagcagcacatccataaacccctgccagtcagcggtgatctttggcagatctttccggttaccaccccataccgcataatgctgtatgccgccaaataactttagttttcttttccctatgcggaggtagaaatttttctcatgcagccaggcgttcttgatgtactgatcgtttcccatccagccatggctgatgagccctttgaactgcagccagccattcgtataaggaatatcggtatactgcgttaccgcgatccctattttcgggatggggagcgcattgccgctgattcccatagagccgctgctgaggtccttgtctgtttccccgacgatttcctcataccgtccagccctgatttcccagtgcttgtaaccggctttcacatatccctgctctataaatgtttgatgaaactggtcgttattgtatacatccagcccatacctgacgtaataatcctccctccatacatgcccgttgctgaagcctacatgggtagacacatctcctttacgatcgctgatagtgccaaaatgattcgccatgagccagagcggctggtagtctttcgaagcaacagttcctactgcaccggcatgcacctccagcgaatccgtaaagtgaacctgcgccactgccgtggcagggcccattattaacgcgatatgtaagcaccatttcttcatatagccgctgtatttagcagggttactgtatgtcccttcatttcccgtttgcgaactgccactgcaggattcccggaataaatcagccagggttccatctcttttgatgccacactattcaccgtaagtaccgcatggctgccacaggtaacacctgcacacaccaccgccatagcgcctatccaggccccattttcaatatgaataggaccaagccggtaaggaaaatccggttgcttatagtcgtggttgccggtaagcaacaaggcgccctgtgagagacaaacatgatctcccagcgttaccgcagccaggttgtcgatccacaccgattcccctatccagcaatgatcgccgatggtcagcaaccatggatacttgatacgaacttttgtttttatgacaagtcccttcccaacacgggcgccaaacagcttcaacagcttacttttgaacccataaggccaggggaaagcactgttgaaaatatagtagttacagaagtaccataacagcactttccacttagggccggcataataactgcctgtattaaatgcagcaagattagtggtcatgtgatatcagatatgaatgttataatcctgttttagcaacgccataatatcttcccggctttcgtttccatcgagcttttgctgaaattcctgcacattaacgtctacgagcaaacgataccagtacccctgcatgaaatggaacagaaagcctttgtagccgtcaaggaaaccgtaacgcagtatatagcggaacaggaaatacagcgaggcccgcattcccggcgacatagaagcgtacaccttctctttcaggaatcgcttgcgtttggcctgcgttccactctcccgcagcagcctttcatcggtttgccagaagccatagcggatattcagcaggtctaccatttcgcggatggcgtagttgttatgcttgtttacccaccagtgaatggagttcaggttatcgtctacaatatgttctttaaacagcatcgtagcgccgtcggacaatacaatatgttcatccatccagcgctgttcgatgctgcctaccccattgcgccatatccgcaacagggtatgcgggtagaaaccgccgaagcggatccatttacctttgaataacaccttgcggcgtatatatatgcctgttataccgtccggcactttatccatccgttgccggatttcttttaccagtccgggttccaggtattcatctgcatccatgcgcatgatccagggtgtttcaatgccgcaatggtccaatgcccactgaaactggttggcataattcacccatttacgctgaaaaacctttgcgccatatctttccgctatcgctacagtatcatctgttgaaaaagcatctattacgtacagctcatccgttatttgccggagattctccaggcagcgtgccaggtgcaacgattcattaaatgtgagtataactaccgcgatcttcatctagctacatttttcatacagttctacataagacgatgccagcgtggcatcattgaaatcattacggatctgtaaaggggcagaccgtgtaatcctttgccgttgccccttttcctggtaagcagcagtgagctgcgctgtaatcatctccacgctatcgattccggtaatccagcccaggtcatgctgctgcacataggttgccagtcccacctgatcgctgatcagcaccggggtaccggcatacagcgattcaatcactacaatggcaaagttttcattacgggaggtcagcgcaaaaaggtcggtggcagcgaggaaatgaaatttatcctcactgcctttccaacctacccattcgacgctattatccatatcgagcgacgcaattaaatcctttaatactgctatatactgcgcatcaccactgccggcaatctgcagccggtagggaaatgttaccttcgctaatgcacggatcagcagatccaatcccttcttgggatctacccgggaaagaaagctgatggtaaatacctcgttctctttccgcacaaaactcccctccggtaaatccacgaggttaaacacctgtccgccctcccagtgagtattcacctgccggcattccttccactccagttccgacgatacatgcaggtaagtattctttagcaaacgtttacccatcaccgtgtgcagcagtttcttcttccggttgttccgcgccgtcagcacatagtcgcaaaacatgccatgcggagacaacagtggttttagctttctccatttacagataaaggaagcgcccattaccaggaaattccaccaggagtggatatgtactttatcaaactgttttgcattagaccaaactgctttccacaatgccggcgacacatgcgtgtgatcaccggtgattcttttgaaataggttaccttcaccccatccatgatcaccgtggtattagccgctatatccagttccctggcgccgttggccgtggtagtatatacttccacctggtgccccattaacaccagttgctctgccagccgcgctatcactacaataggacctccgtacacgtaggccggtttgtaggacggaacaataaaaagtatcttcataaacaagggttatttattcattgaatccagcgagtgaaaagcattatccaccatagccgtcatggttagattttctcccacaaattgtttggcatgttgccccagcctggtgatctcttcatctgacaactgatccagcacatacaaacactcgtccatgctatcgaagatcagcccgttgtagccatcgcggacataactatattccacgcactgcagtacttcctcgctgcgcttaaaagtgcataccggcttgccataagccattgcttccaccgccgacagtcccacccatcccggctgaaaatacaggtcggcgataccaaacagctcctgttttataatcggatcatacaccgccccaaagtcatgtacatgtggataactactgaagtcgggcttgtatttacctgccccaatgatgataaatccatactgctccggatcagtttcctgcatcagcttctccagcaaatcaatacgacggccggtttcattaaagcgggcgcaatagatcagtatccgttttgagcggatattatacttttcacggagcgctgctttatcgggcgcctcccgttgcataatcttttccacttcagaaatcgtattgttcaaagccactgcctttaaccccggcatttcctgttgccagagcgccatctcttttggtgtgtaaaaccaggtagcatcggccagttgtatcatccatttcaacaggcggctgggtcgttgttcttcctgcacatatctcttcaccgaaataccatgtccccaaaggataactttttgtttcagcaagggtttcagcaacaggatcatccaggtagacagatgcgcgaaattgagcatcaacaccagtaccttatagtctttattaaaaaaacgtaacgggttatataacacaaacgggcctatgctccaggcaggcaattgcttcactgcagtattgccggcagacaggttttgctgtttgatagcatctgcctgatcataacaatacagatcgaaaggcgcctgctcattgagccggttaaaaaaatgttcgcggtaatgcggcaccagtggctgcagaatggcaatcataccagtacatttttatgtgcatgaataatactgctcacatcataaccatagatcatgcggcggccttcgtggatggagtcgaacgccaccacgttaccatcacgcttccagcgtgggtgtaaatcgcagtggagaccgctgcgtgtaaaggccatctgttccagcgaaaacgcttttaacaccccttcttccacgccggccagtaaagggtgcgcctgcttcagatcaggtttatcgtcaatcatacggtaagtacccaacgtcactttcttttgtgtgctgtactggaaaaggaacagcgtccggattccctgttgattgggataagtatcacaaatcatccagtcgcggtcagccgggcaaaacatcggatgcccgtcttctgtaataatatcttttgccagcatagccggcgccccgttatccacatcctccagtaacaaccagttgaaaggcgctaccgcttttgcacctttctcttttgtatacaataatttcttcagcactttctttcccccggaaatcaatccggaaggcatcatcttatacaacagggaaccacgcagtttttcgatgttactgcctgttctgccccagatagcgatgtgtgaatcatctttccagtcgaaatgactgagaaagcctgtagccaggcatttcaggtcgctgccatccacaccgatcgtcatgagccgcgtggtttcacctccgtcttttaacttatagcggtgcaggaaggccagccgttgctgcgagggattcagcagcaggtgcgtgatataatgatgttgtcccaaagcgggattgattttataattagcggcagcagcaatagacagcaataatgtttgctcaccggtatatacattgtgttttacaataccggagttatcaggtacgtgaacgtgcgcatacttatcagcaataccggtgtatccatatcctcctacacgatacagccttgcgtagtcgataccaaaggcaacgccttcatctgtgatcacatgggcgggctgatgcaacacactcacacatttgccggcatttgtatcatatatccgggaaccccatacatcatcaacccggtcattcacgataaaagtatctgtatcgccgatccattgctggcgggcgccctgtggataattataagcgtaggtgtctcccatccggcggaattgctgtgctgcatcgaaatagccaatgccgcagggaatgcgcggatccgggggaacagtaatgtcgggtgtttgtaatgcaagcaatttatcacctgcagcattccaagctaccaggtcatgaaaaccaaaaaagaaatgtcctgttcctgctgataaaataaattcctgctgcatatattaatgtgttgtgatgaaagatgatttatccatgcacttttcttttctcaacaaaaaagtctgatcatgaatcttattatcaatacgtctgataacatcttcttcagataaataaaaaccgttcacaccctgcagtgttttcaacagatctgtttttacaatatccctggccataaattctgcgctgatgcgattgccggagagggttttaattttctggtgaagaaatgatttgcgataaagttttaccggtgtagcattgatattatatagttgaatagcagcctgccagtccatccatttaaactcagccacaccactgccctccgtatgtggcgtggataatataaagcggtgccagggcacgcgtagcgcatcggcgaggatggcgccgtgcatggcttccgcaatcacatactccgatgcggcgatttcctgcaacgtatgttctacgccttgctccgaccgtggtgagatataattataacccagtttattacagagtgcttcccaatcgaaaaacggcactgatttaaaataaggaatcacgctcaccttgtgctttttcttcatcttcaggaatttatcaaactccggcagctggcggatagcgtaggcagcatcagcgatgtacgggaactggttattaaacgcgtaggccgacaatgggccccgcaggaaacggatatcccagctgctgttaagactgaaggtttgatgagaaggccttacgcctgtgccgaaaacaatcttgcacttgtccggtatatccctgaatagcggagagccgtcgaacaggatggaaccaatgcccaggaatgcttccggatcattgatatttccttcgccaaataacttgggccagagccacccgttcaggtcatcaccaaaattgcctttgggatctttataataaacataatccacgttgtagtcatttacaggttagcaatacgtaatacttttactgcatcgttactgttgatccatgccgtaaagtcaactgcccgtcgttcccagctgtgggcttcgctattcaccgttgccggcgccagcttgccattagccagtttgctgatcaataccgccagtgatgccggcgcattgttgttgaaataatatccctggtgcccgaatatttccaatggctcgccaatagcacaggtaaacaccggcttgtcaaatggcaggtacatgtaaatcttactgggacaacgcgcccagtcctgcacagtatcattcagcggggaaataaatgcatcggccgcggtgaaccaggaactgagatcttcttcgggtgcgtagcccaggaattcaacctgcgcatccagctgcttttccttgacaaaagcttttgcttccgccatgtgccggccctgtcccaataacattaataccacatcacttctttccttgcttaccatttccattgcctgcaacatggtaaagaggccatagttgcgggtaagcgtgcccatatagatcagtatcgttttgcctttataagcatcctgcaattcatccaggcggatccgcggcgacgctatcacatcattattgaatgcataaggcgagtacaacaccggaagttgtttacggaacagctgcgccgcccttttcgtatatacgttacagagatacttgctggcgcacagcaatccatcggcatacaacaccgaccaatactccagcgccagcatagccagcttacggatgcctttattgtcggggataccggaaggcagctccgaatgttcgataagtattttgggttttacgttgagcttacctttggaaatacggttacggaaactgaaagaacagaataacacatagtctggtgcaatctggtttaccagctctgttttaaccctgacttcttctcctgcggagccaggctgatagtaatataccttcactgcctcactacactccatggctatacgtttccggttctcttcactgtcctgcgcaatgatagacacttcccagcctagcgacagcagcggtccggccatgcctatcgcccgtttcatggtggcaatgaatttaatatcccctagtgtaatgaagcatattttcatagctgatgtttttttaccgtttatattttcccttcgggagatagcatatcgatcgtttcatttatttgtacgggtacttcctccgtggcagattcttccataaaatcatagtaggcgcgcaacagtactgcaccaatggcaggtatgttaaaccttagttgctggatgggggaaaaaagaaaagtccatattaccccaatcgtcatcagtaccagtaccgggtacaatgctgtatccgcagcgttgcgaatgaggtaaaatcccattctcagcaggaatatgaatatcagcagtaccgcaataaatccacccagcccgcagtttacccaggcccccaacaggatcgagtgactggggatcaggtggtctgttgaggtagccagttgttcattcatttcttcattctggtacagcaacaggatccggtaatattgcaggttgtcgtcttttgcccaggaaccatgaccgaacagcggtgcatcggcaatggctgccattgcagcaaaggtttcgcccctgcctgtcatcagtaatgacaacggattataaggattatcgagccggtcgatttgctcggaagcatgatctcctcctatttcatgattcatcactgcatttacataacatacataggcaaactggaacaggatagcgcctgcaatcccaaacaccagcaaccggtcgcgggtgagatacataccactgttaaagcagtagatgataatggcgcccaggaaaaagaccatgcctgttgagcgcgagtcgcgggcaaaacataacaggctgtagcctaatagcagcgccagcactgccttccattgtcctctgcgatataaaaggaaagaacagatataaacagcgtacgacaggataggtaccatcttaaatttgaagtacgacatatccgtatcggcattatcatctgtccagataatatttttgataagggtcatgcaaaggaagaagaagatggcctggtcatcttccaaagttttaaacaggaaaataaaagagaggatagacataatgatggccgcccagccccgcatgaaattctctgaagagctatgtacaataaacagatcagtaatagcctggaacacaaagagcgctaccaatgcaaagatgatcttgcggaacatggggtatgctttaaagtcccgcaggtcaaatacaaagggggtagacagcagcaccatgatctcattgagcttcaactggcctaccagtgctacattcacgccactcaacaaagtgtacatggctattttgatccggttaaacataggcaggcattttatcgcgaaccgcgtagtgaacaatttgctgtagccgttcccggtttacgtccaggctgtattcctgtaaaaaatcttcccgtaaccgggcgcccttatccgtttccggatcaaaagccagcagggattgcttaaacgcttcaggttcatcagacacaataaagtgatgactcttcacgccttccactcccttccgggtactgataatcggtgtactgagtgccattgcttccaggcatttcaggcgtgtaccgctgccatgcactaacggaatgatcactgcgctggccacggagatataccacttcacatcatccacctttccaaaggctacaatattgcgatattcttctttgccggtaatttgtttcaacgcttctttagaacccctgcctacgagccacaggtcgtactttccggccagatcatcatcccacacgttttcgataaaccatttgaggccggcaaaattcatatatacgccgaagttagccgtcatcaccagcacacgctgctgcttcttcccggtgaagtgataatcctttgcgtccaggaagttgggaaccgtaaaaactttctgtttaggcaggaagcgtgtgtgataggcattatcatcttcactaactaccagtaccgcagcagctttgttaaagtacatgcgctcatgtagtttttccatactgaacagctgccacttgcgcagcttatccacaatattttttgagggcagctgccaggtaatcatgggctgtgcgttgtgcgtgcccaggataacgggaatctgtttctgcctgaaataagaaatataatgacctacatagccatagtccaggatagctgctgccagcggataatcgcggcacacctcttcaaaaatgctcataacggtggcagagcgctggaagtattgcttacccgtaatgcgggtcagcagatcgaaaggttttgtttcataagtataaaaagtaacgttagggagatggtatttttgcaggtccaccttctccacattctgtaccacggcaatcacctcataaccgagctgcgacaaagctttgatcaggtagtaactcctgatgcgttctcccccgttttgcgggaagggagatatgtctgtgaagaaaagaatgttcatatcttaattcgcttttaataccactagccgtgcctgtagttttgtgaaaatcctgttgagtaattgttccactttcgcagtttcatcggtggttagcccgatgagccggatgaggaatacgatgctgatgatacttattgttgtggtaacgcccagccgcataaatccttcccccatgaatagttgcgggatgcaggccagtccggctgccagcaatgccggcactattgatttgatgatcacctgccgggtaaacactgccggcgataagcccgtaatagttttcgccgccatcatgcggtaaatgccgcttacaacttctatggcgatggcactgatcaataccgtagcggccggatatcctgctttcagcagcaaccaggcaatgggtaaattgaacagtaccattgtgctgactaccacctggtactttcttattttccccaccgactgtaccgctacctgtatgcccgacgacagctggttaatcaatgtagcgatgataatcaggcggcacatcatgacggtaaaatcaggtacttgtttcagccagcattgtaatacaaatggcatttctatcatcatggggatggcgaaaaggctcagcaggaaaaaggaaaacttgctggcaatcatggccagccgcagcatcctcggacggtcgccgctgccttcacttttaatgatctgcggatttaatgcccgcagcatggtaacagaaaagtagctgagctgtgcattcacctggttagcgatgccataagccgcattaacgatggtgccaaagaaaacattcagcagaagagcgatgccctggttgcgtgctacaaaactgccggcgccaaacatattccaccctgcgtaggcaaacatttctttcaaaaggcttttgtcgaaatactgccggatgcggatgcggctttcttcatacttcaccgcgcaatacacctgcttaaacaccagcagtaatacggtgagcaatgccataaggccgccatacacaatgagccggtcgtatgaagtgtattgcaggctgagtgctatcagcagtttgcctacggattccactattcccattatagctaccatcaccatattttcctgtgcaatcaatgtagcatcgtaaggcacagagatgatcgtaaagaacgcgctgaccaccatgaactgaaaaataagtttggcagccatggtgcgggatgcaggataattgagcacatgatcaaaaagatagctgcctatcacttcaaacagcagcaccaatgccaggcccagtacaaaatgcagcaatacgctggagttaaacaccactttcagtttgtgtgcgtctttggtgccaaggtgaaaagacatataccgctgcgtgctgatggtcattgccatgttcaggaaagacaacatggcaatgaccccgctgatcaggttaaacaatccgtagtctgccgcgcccagcaggttgagtaccagccgggtggcatataaggaaataaaaacggtgatcagcatccgtccgtaaagcgcgcctgtatttaatatcaccctgttcgctacctgcatgttgatttaattatccgattaagtgttccagttgtgtcacttctttctttgcaaacaatgccacgtcgctggccatcatttcctttaccagtgcagccaggtcgtaggctggttcccatccgagtactgttttggatttggtagggtcgcctatcagcagctctacttccgtagggcggaaataacgcggatcaatagcgactacctgctttcctaacggcaacgcatatacctcgtttgtgcaggcagctacggtacccacttcctcagcaccggtgccggtgaaggcgatttcgatacccagttctgcaaaggacatgcgtacaaactctctcacggtagtggtaataccggtagcaattacgtagtcatcaggtgtttcctgttgaaggatgcgccacatggcttctacataatcttttgcgtggccccagtcgcgttgtgcatccaggttaccgaggtacagtttatcctgcagtccgagtgcgatcgcagcagcgcccctggtgatcttccgggttacgaaagtttctccgcgcagcgggctttcgtggttaaacaggataccgttgcaggcatacattccataagcctcgcggtagtttaccgtaatccagtaggcgtataacttcgccacagcatatgggctgcgcgggtagaaaggcgttgtttcacgttgtggtacttcctgtaccagtccgtacaactcggaggtgctggcctggtagatgcgtgttttcttttccattttcaggatgcgcagtgcttccagcaggcgcagcgtgcctataccatctgcgttggcagtatattccggggtatcaaaacttacccgtacatggctcatggcagccaggttataaatttcatccggttgggtttcctgtataatgcgtatgaggttggtgctgtcggtcatatcgccgtaatgcaaacggaagcgcacattttcactgtgcatatcctggtagaggtgatcaattctttcggtgttgatcagcgaagcgcggcgttttacaccatgcaccatatatccctttcccagcagcagttctgccagataagcgccatcctggccggtaatacctgttatcagggctactttcatacgatcgttattttttagtgataaaaagaaataagttattgcataagggcatttaccggggtagcagctgtattgccgataccatagtaagtgaacccatgttttaccagttgtacgtcatcatagatgttcctgccatcgaacagcagcggcgtttgcagcaggctgcgcaggcgtggccagtcgggcatccggaaggcattccattccgttaccagcaatacggcgtctgcatttgcagcggcggcatacatatcatccgcaaaggtgacgctgtcgcccagcaggtgaagcgcctcttccatggcaacgggatcgtatacacgaacctgtgcgccggcttccagcaggctgttgatcagcaccagcgaaggcgcttcgcgcatatcgtcggtgttgggtttgaaagacagtccccatacggcgaacgtgcgacctttgatgtcgccgtcgaagtgacggagcactttatcggataatattttcttctgatcttcattcacggcttccactgcttccaggatacgaagctgatagccatattcgcggccggtttggatcagggcctttacatctttggggaaacaggaaccaccgtagccaatgccgggatacaggaagtgtttcccgatgcggggatcgctgccgatgcctttacgcacctggttgatgtccgcacccacgagcgtgcatacgttggcgatatcattcatataggaaatcctggtggccagcatggcattggctgcgtacttggtcatctccgcagaggcgatatccataaaaagcagcgggtgtccgtttaacacaaatgggcggtataattgttccagcacttcgcgggcatgggtagtactcacgccggcgacaatacgatccggtttcaggaaatcatttacggcggcgccctctttcaggaactccgggttggaagccacatcataatcgatgatcagctggcgggccgacaggctctcctttactgcgcggttcacgcgggcggcggtgccaacaggcacggtacttttggttaccagcagcaggtaatgctccatgtattgtcctacctcatgcgctacctgtaatacatacttcaggtctgcactgccatcttctccaggtggtgtgcctacggcaataaataccacttcagctccgggcaatgcgctggccagcgaggtagtgaaagaaagacggccgcttgcctgattacgcatcaccatttcaggcaaaccaggttcataaatgggtaatacccctttctgaagccgtgctatctttgctgcgtccacatccacgcaggtaacactggttcccacttcagccaggcaggcgccggtaaccagtccaacatatcctgttcctacaatgactactttcataccactggttttaaggttgtaatttgaactgatcctgttgcagaaaatccctgtaagccattaccagtccttctttcaggctgatgctgtgtttccatcccaggcgatgcaatttggatacatccatcagcttgcgcggcgtgccatcgggtttggtagcgtcaaaaatgatttccccttcataacaaactacttcccggatgtactctgccagttgcttaatggtgagatcttctcctatcccgatgttcaccggttctttatcattgtaatgctgcatgagatatacacaggcatctgccaggtcatctgcaaataaaaactcccgtttaggcatgcccgtgccccatactgttacggatggtttctgatttactttcgcttcatgaaaccggcggatcagcgccggtaaaacatgtgcattttccgggtgatagttatcgccaatgccgaacaggttagtaggcattacgctggtaaagttgcagccatactgatcgcggtaagcctcgcataatttgatgccggcaatttttgcaattgcgtagggctcattggtttgttccagcgtgcctgtcagcagaaagctttctttgattggctgcggcgccatgcgcgggtagatgcaggaactccccaggaactgcaacttggtaacgttatgcttccatgccgaatgaataacgttggcggcaatcatgaggttatcgtacaggaactctgcgcggtaagtattattagcatgtataccacctactttggcggctgccaggaatacatatgccggcttttcctttgcaaagaattcatccactgcggcggcattgcgtaaatccaggctgccggaggtgcgggtaataatgtgctggtaacctaaagtttccagtctcctttttatagcacttcctaccattccgcggtggccggctacatatataagatcgtttgcctccatacgtgttgattgattgtgtttatgtttagagcagctccgggcggttttcccttacccattgatgcagttgtttaatatcctgtccacttcctttctgcatgatcagcagtgcgctttctgtattaaccaccaccatattttccacgcccaccaatgcgaccaatttatcttttccgattaccatacttttatgcggatcgctttgaataaaaaccgcctggtgattcctgtactggtagtgttgcgacaatgcgtctgccaatgcttcgtagctgcctacatcgctccagtccattttactgggcactacttttacgatgtcacttttttccagcacggcatagtcgatgctatctgaaggaatggcttccatactttctttcgacaacacaccggtttgtttccattcttccgcggcgatggcagcggcttcatagatagcaggtgcatgtttttgcagctcctgcagcatgatgcgtgctttacagcagaaaatgccgctgttccagaggaagccgccggcggccagcatggcttctgctacggcgcggtcgggtttttccacaaagcggagcacatcatgaccggagtagctgatgtagccaaatccggtgtccgggcgtgtaggcaccaggccgatggtaacaatatgatttcccgcggccagcaggccggccgtttcaatggccatggcatagcggtcgggcgtaccaatcaggtgatcggccggagtgatgagtagtatggtttccggctccgctgtaaaggcagccagggcaatggcagcagcagtattacggcctaccggttcggccaggcataccggggcagctgcgcctgcctgcatcagttgctcctgaacaatttcggactgttgttcattaacaatcgccattactttattacaggcaaaacggtttcgccggaaagcgagttgtaaaagactatagccgtcgaacagggtgagtaactgcttgggcgtttgttggttggacaaaggccataaccgggtgccggagccaccgcaaaggagaatatgctgcatcataggatgattggtttatggtcagtaatgatgtccgttcaccgttttatggccggtgaccaccgttatttccctggatggcactgttgctacgagcatgcagcccaggctattcagttccactttcacgcggttacggctgatctgtaagatcctggcggtggaaggagaacggttttcttcttcctctgcccggataggaaatttttctacagatacatcttcataatcacggagaaaatggcggatgagcgctatttcgtggtctggtatcacggccggttgccccagccagtatacgaagttgaccacgttgtctgtttcctttaccacccaactcctgctttcaggaatgtgtacgaatacgtaggatggaaaaagaggttcctggatgatcttacgggcacgtaccaatggtttagcggggacgtagtgttccacctttttacgggtgaaaaggtctgccacttttttttcgcatttgggccgggtatataccgcataccagaccggaggctgttcattaaacatagtagccggtttttaggtgatcggatagttttgtgtagaatttataaaggcaggaacgggcatgacttcgccctttgttatttaattcgactatagcgggctgcatttactttacggtgcgcctgaataatccgggtttctttgttatttccgtgtaaccgtatccgttaatatcaccatatccggatccgtatccgtatcctgccacaccttgccgtttgataccgttaaacacaatgttcagttttcctaattctttattctgatacaactcttcaatcagtttaagataatttttcggagtacgctggtgacgcaccacatacaacgtagcatcgcaatagggcgctatcaggcgggcgtctgttaccagtccgacaggggcagaatcaatgatgatataatcgaaacgttctttcagttcactcagcaacctttccagttcaccattcagaataagttcactcgggtttggcggcataataccggcagacagtaaatacaggtactcgttgtctccaacaggttgcaatatctgctgcagtgatgcttttccaacgaggtagttcgtaatacccggatccgcgcgcatgctcagcatcttgctgaccattggctttctcaggtcaaactccagcagggctactttctttttggcaagcgacaaactcatggccaggttaacggatataaagctctttccctcgccagatatggaagaggttatcaacaatgttttgcgatcgccgtttaaacctatataagacaaagacgttctcaatgccctgaattgttctgcaacggctgttctgctgttattggacatcacgatcgcatctttgctgtcgtggtacataatttctgctgcaatcggcgccgtcgttattttttcaatatctgcccggaacatcacctcacggttcatcatatctttcagcgatacaaatcctgctaccagagcaagtgccgccagtacagagataccgtacaccattggtttctgcggactgaaagcataggctgctgcttcccccgcatctaccacgcggctgtcggatacggcggccgcgtatgccagtgcggtttcttctcttttctccagcaggaaggtgtaaatattatttttgatcacctgctgccggcttacttccagcaatgctttttcttttccgggtacactgcggatgatacccatgttgcggctgttctccgcctgaaggcgtgttaaaccagcctgcagattggcgcgcaagctcccgatgttctccatgatagcaggtttcaggcgatctacctgccgtgtgaggcttgccagcagcgggctgttttcgccggtggttttgcggagtctctccagttgtaattctgtttcagacaacttgctcaccagctccagcagcaccggatcagaaagtcctaatgtaccgggtacaatgttacctcccggattctggctggtaacatatctttcaatggcatccagtacggagatctgcatattggcttcactgatcttccggtcattttcctgcacgcctgccaggaatattttactttgttcgctgatatccacaataccctgggaggttttgaagtgttccacttctgtttctgcctggcccagttctgtgctcacgatgcgcaggcgttcttccacgaagcgcatggtgtttgcggaagtcctgttcttatcttccacggcagcctggctatatacccggatgagttcattcacaatatcttccccacgttccggcgcttcgtctgtatattcaagatccactacactgccggctttcgcggcaggcataattttcatggtaccgaggatgatctgcatccatgttttttcgttcatgatatgcagtacataaccagcggtggtatctgtatgccgggcttttgcctggatgagcatttttccccaacgggtttgtaccgtatcattcagcggatattttttaccgtcgatggctatacgcttttgcacaggatcataagtaaaaggccagttgccggtagaagccatctggatagactccggttccaggaaggtaaatttcaccgggctatctttataaagtacaacgtctcttatttttcctttttctattacttctccataaagattcaggttccttaccacttcttttgtgagcgtgcgtgatttcaggatttctatttcattttccatcacggttttgctgccacccatcaggtcgagcgactgcagcatatcgctggcgccgagaccattggtagcttcctgtaccaggagcacgccggatattttatacagcggagtggcataacggagataaaggaaagcagctatcagtgcggctactacggctcctgcaaagaaaggccagtatggcagatagcgggagcggatgatagtcagcaaactctgaggcgcttccgtgtgctgggttttatgtccgttaactttttgcataacctaattatttataactaaccggtccaggataataacaagtagtgaaagactgctgagaataattggcaggatttgccgcgaacgatcagccgtcgccacttttgacttattgggttctacatataggatatcattgggttgcagaaaatagtagggtgagttcagaatgctcttgtcgttcagatcgatgcgtcgtataatccgctgcccgtctatctcccggatcaacagaatattattccgtttaccgaacaccgttatatctcccgccattcccaatgcttcaaggaccgatatcttttcgttggttacgtttactacggttggtttacttacctctcccagtatggttacacggtagttgaggaaccgtatgctcactaccggatctaccaggagctttcgttcaatgagctgatcatgcaggtatacggtgagtgcttttttggtgaggcctgttacttttacgggacccagtacggggtactgtataaatccctgttcatctaccaggaagcctcccagcatggcaccggctcctgcattggcgcctcctgcgccggaagcggaggtcatgttggatacattataaatgatcacatcctccggattaagactgcttacgttgatctgtaatatgtcgttcttttggatacgggggtcgaaactgctatctgacggcattagcaccgtatcccttacatcattgaaataaacagcatttttggttgacacgcacgaagtaaacaaacaactcaagcatagcaatcccaatcctatccaggttaagcaggctttcaatatcatcgatatggcatttaacatcatcacttacactgaccgttcctctcaatacaatattacttcagaacggggtgggattcaattactcactacagtataaattgagacgattagtttggagtccttacttattaaagtaacttaccgttcacagccactgacatattaccaaaaacgaaaatttgattattttatctgaagaagggcaaaaaacagggcgatgaataaattatttgataaaatttttgagattaactcagatttggttgaaacatttaatttaaaatatacttttttcagatgttggtttacagtgaacacggttacaaacaacttggctgccatttccttatatgagtagccttccttgagcaaggctaccagttcatactccctgcgggtaagtttgtctttgatactttccagcggatctttattgatatgagtaatgagcagatgggcagcacggggagataaagaagcgccgctttgcacggtgtccatcaccgactgatagatatcactaaggcggctggatttaatcacatatccactcgcaccatttttaatggcctcaataatatattgctgctcctcatgaccggataatacaatcacctttgtatcgggatacacccgctttacttcgcggagcccttcaatgccggatatacctggcaaggtgatatccaacaggattacttttacatccgggtaagtaaccggcaagtccataaattcctctatcgatttgcaggcaaacatgaccttacactcctggaagtcctccaggaactcacggtaattacttagcagaaaatggttgtcttcaatgattccaatgttgatcatggctaaacgggggtatggtgctcgaaatgatatggtttattaaaataatctgatagtaaatatagtcggaaaaatgatagttatctagtataattttttatgaatatgttaaaggcttatatacagatgaaagaaaaataagtccgctcaagtaattatattataataaattctatgtaaataaattctcactacatgttaaataaatgcaaccaaatgctacttttttaataatatgaataagtttcgtatattgtgtacagaaccatttacgctcctaacccggtatccttcgaaatagaaaacctttttaagaatcaaccaaaaaaagaagtatgctgaaccatatcaaaaggcatgcagttggccaaaaatcaatactggaaatgcgatcggatttcattgccatggctacccatgaatttaaaacaccgatcagtgccatctcgtcttccatagaattgctggaaaccaaaatgcagagagatgaattgatgttgccgttttacgaacgcaatttatcccgcattaaggaagaaatagacattttgagcagcatggtagacgacatcctcaccaccggcagcatggtagccggcaaccctgtaacacaaccggaagaaacggagctacctatttttgccagtatgatccggcaacagtatttcagcaaccgcgccgaccagcgccaactccgcatcaaagtatccgggcgcccgcggaatatctacatcgacaggagccacctggccgggatattcactaatctcatcagcaatgcgtttaaatactcttccggcgatccgctactcggcctgcatttcaggaaaaatcacctctgcattaaagtaaaagacaatggcatcggtataccggaggcggatatacgttttttattcacgccttttttccgggcaacaaacgctcacggtaaagagggcaccggcctgggcctggccattgtaaaatcctatgttgccgccaacaacgggcatatcagcgttaccagcggcaaaaatggttctgttttctcggttacctttaactactaacgaaccaacatcactgttcccttcaataaatgctgctcactgcggctgtctgtaaacgtacatatatatacataggcctgcacacccgccggcgtgcctttaaaattcccgtcccaccccacctcgggtgcattactcataaataccaaggccccccaccggtcatatacccgtaaccggtagtcatgaatcacatcatatactttcggacggaacaaatcatttagaccgtcgttattaggactgaaagcaccgggcatcaccaccaggcagtttttccagggagattccaccttagcggttacaccggcgctgtagtcatgtgcatccataatttccgctacatggctacccgctgcaagcccgggaaacacgctatcggtttgccattgcccgttgtccagccggtaacggtaaggcggcgcaccaccggttacatgcagcataatcctgccgtcggctacttccccgcaactgcagggctttacactagcctgcacagcaggcggtattaatgggtcaatagctgaaagattgtccatcagcagcgctattccatacatacttttattacaggccgctgttggataagcccagcaggaaatatacgtatagttgccatgcggtctgaatatggcatgatacctttgccagttttcatgggtaaaattaccggatgtccataacagctcggcggtatctcccggggcattacccccgaagatcgccaggttgccataacaggcgggatacaaataataaagtgtaaacgccagatccaaactcaatacataagtgctgtcctgtttcaacgaggcaggcaacttttgggcaatgccttccaggaatcctttaccactatgcacccctacataactcttacctgctgaaggagccagcaggatttcaaaaacaccgggctgtgtgtccggcgtaccattagccaccagccagccagaaggaaccaaacctttcccggtacggccttccagcgaagggttacttaagggtatctgctgtgcctccgcaggcacacacaacgccaaaaacagccagcagcatagtattccgtatataactgtgagatctgaaaacatgccgctcatttaccggattaaaattaccggttatataaatgatgacatatactcataccagtagtttgtcgtcttacttttcttttgttttgtttgcccgaaaaaatatctttgcccacaaaataccccggcacgcgattgtgccatagcttaatccgaaaaaaacttatcatgaaaagatccgtactgtacttagccctgggaaccgcccttctcaccacgtttacgtcatgtaatgaaactggtaaaaaagacagcaacgctgcgtacgaagataaatctgcatcttccgcaaatgatgtaattgagtacaccaacctgattgtagacctttctaacaagaactccgactacgtagtacggctggttaataatgccgaccgtgtaaccgaattactgtctggcaaaggtaatcccgccttcctcagcagtatcatcaaacctattatgattaatatgatcagtcatggtaaggtgaaagtggaagaaccggtagatgccttaaataaggcagaccagcagttttttaaagaaaaggtaaccagctttaaaggctcgttcgacaagttgaaaactacttacacgcaactggatgattacctgaaagcacaggactacaaagacgacaaaggcgcaaaaggcctggcactggcagattctatccgcagcagcgcccaggtattttttgagcagaaagctatcctgatgaaaagagtgaacgaagtagcagatgccagtgaggccatcatcctgaaagacagccccataaaagattacgtattggccatgaaagccgatatgcagtcggtacgtgattacattaccctgctgggagaaggcggcgccgatttcgcgaagatcagtgacaaagcacaggcagcttacgacgccctggaaaaaaaccaggcggcacatgcgggcatggatatggccaatgccgcgaaagaaaacaaagattcatattataagagcttctatgacagctttcatcagttcctgctgacagccaaaaggatcatgcgtgacgccaaagaaaaaggcgaaatgaccgacagccaactcgaaaccctcgataacgcgctggataccatgatcggcagatacaacagcttcacaaaataaaataacaatgggtagatatccatcgcggatatctacccatttatctaccagtaactatttcttaaatacttcttccagcttcttctctaattcttctccgcgtaaattctgcgctattatttttccgctgccgtctatgataaagttggcaggaatgcctgaaatgccaaactccaatacaggattacttttccaacccttcagatcagatacatgcgtccaggtgagtccatcttttcctacagctttcagccatgcttttttatcggtatccagtgatacaccgaggatatcaaaaccctgatcatggaagcgctgatatgcttttactacgttaggattttctgcacggcagggaccacaccagctggcccagaaatctaccagtacaacttttcctttgtagtcggtcaatttcaccagtttgccggtgctatcaggcagcgacattgccggccgggcgcccacgctcattttagcatgtttatccatcgaggctttgatagccagtccgtagtccgttttccttgcgggatctgcgagtagctgataggcggccgccgctttttccgggtaggaataattgatatacctgtccaggatcacaaatgcggctaccgcggaaccgggtgaacgctttacaaaagcggtaatggagctatccagttctttatccagatcggcaaaaccggctgctaccacctttcgctccacgctgtctttgtttttttctgctgcatctgcacgctgatataatttaccggctttctggcgtatcgcttcccatgtttccgcccacccggcatataaaggctgatttcccgagcctgctatttttgcggctcccatggaatccttatgagcggtaatggtaatagtgctattttccaggaagaatgatatcccgttatatttatcagcggcagtccatatcgaatacagttgcggtgagcctacttttcctttaaacgtaaactttccattcttcagcatggtggaatccggcttatggtctggcaacatgaaagtattcaggtataccttaccgctatccccgccgtggataacgccattaatcgtatagcccttaccgttttgtgcctgtgccgacagcataccaacagtggctgccaacaggacgattgatttcttcatattaatagtgggttttgatggttatgctgctttataggtcatacttacaattttgccgaaaccggtgaacacctttacatcctggaaatcgcccaaaggactgatcttatagcggtacaattttcctgctgtaccgttccaggtacctaccattacgtcgtcgcccgtacactggaagtaagttacctgctctcctgctgcaatagtcttaatggtccttgctttaccagaggggatatcatacaggtagatgttaccgttaacgagaaaatagatctgttgcagttttttggagctggtcattttagtgaaggccgccaattcaggagcatcgcctgtgatcagtttttttgcgacggcggggtccgagcggttgccatctatctggtacaaataataattaccattatccttgaagatagcgttgttcaggaaaggcgcatttccctggtccatagcaagaagatccttcccgatgttacgcatatcaaagtaactgcccggctcgggtgcgctgaaagccaccagggaagggatcagggaagcgcctgacaggtacacaaagcctttggtttttgtatcaaaaaagaaagcggtatagggtgttttttcaccagtatagggttgcggaccgactcctgtataagaagaaaaataatagtcatcgcccttacctcccggaaaaggaagggtattgagatattttacatctcccggaaaacctccggcaacacgtacctgcagatgaccgtcgttaatcaggatattcatgccggtattgatttgcccgaacttctgcggatggaacacggccggtgtttcccagaaccagctggtgtagtctgttagcttcgtcatttctgtatactccagttctatggcgttgtcagcgccaaacatccataccgatttagcaccgtaatagttcgtggtagctacctgcagcggttcattcagtacatagtccttattcagctctgtgaaaatatgatggaagaaggtatctgttttcaggatgatggtcatatctgttttgccagccacatcttccatcacgagccatccttcgctgaagcggttgattaccttcaggttgaagaacttaaagtaagaaacgccggaagctttcacggttactttataaatgagcctgtaaatgccaggtttcacacggatagcctggtgaaggtaacgggtgctgtcgaggatatataccggataagcatcttcagaatcattctgatggatactccattcatataccaggccattatcgcctgcaggcacggcctctttaatatcgggcttcacagttaatgtgtcaaactgcagcacggcgtcaactgccgtagtatcggagatactgagcacgttaatagggataatagctttattgctgttgtctttcaggcaaccggacagcgtgagcatcaccagcattgaaacacacaaccaattatatactgacaatttcatattgcaacttttaggataaagaaataagagtgcaggttaaatagcagggaaagtgacccggttgccattttcatctatcagcggcccgtttgtattttcgtaacggatcagttctacccgcatcttttgcaggatagacatgatctccgaaaattgtgcgcctgttcccattgtgatagcggtggtacctaaccgtgataccatgaactgatgcttggtaagtgaatatgcgccatagaagaagtcgctccaatcagcgggtttcagcaacatatccgttatccttatctggtaattaaggctattagcgaatcctgcggcaaagtcatcggaggaggctatacgaaaataaacagagaacactttattcttcatgtccggggtgcggaacaggtataccggaaactttatggcatattcgcctgcctttataacggcagggcctatatcaaaatgtgttccttttacagcggtggagctgtctgttattacgaggttgaacttcctgtcggtagcagtagccagcccggtgatccgcatattaaggtacacggtatctttcaatacggtatccggttttaccacaaatgtataattgatactgtcgggtagtacaaaatccctggaaaagtagatcgcaggcaattctttgtacatcagccgctcttccttgccacatgcacttaccagcaggtataatatggctgttgctatcagcctgttaatattcttcatgtttgatgatttaaagagatgcagagatgattactttccaaactcgatttcctggtttggcaatggcagtacgtactgcgtattattgatggtgccattaagggcgccctcaattttagccaggtttaaccgtttataataatagaagagttgtcccacgcagataaagtccctgcgatactctttaaatatttcattctgtaaagtagttgcgtccagtcctgcaggcagttctataatattcctggcagcgcggactttgttcagccatttaagcccttcagcaggagccggttcactttctgcggcgatgtaatacatctctgagagagaaagcaccggtattctcttctttagtgattccctgttttcatctacctgccagagcttactggggaagataataccattgcttacgccccacaagctgttacttacaaagcggatgtcggtactgccgcctgctgccgtctcaaacaccgcctttctgcgttcttcagtgatggtaaatttcttgtacatcttatcaccggtagccatcataaagtagctgctcacgggatctttcagcttggatacataaatggagaaaatgtgttccggtgtaaaggtcctgttgagatcaacggcattggtagttaattcaccggaagtaataaagcggaaattattgctggcaattacttcttttgcataggcgagtgcctgtactttatcgttgttatagagatacagtcttgccagtaatgcttttaccgcccaatagttcatccggttgttgcgaaaggcgaggaagtcgtcgttgccaccggggttgctcatttgcggatatactttcagtaatgcttctgcttctttcagatctttctcacataaggtaatcacctcgcttacttttaagcgcgcctgtggtgttaccgtaaaggaagtcatataaggaatggcggtagcagtagcatctgatttaggagaaggtgcatataaacgcagcagatcgaagtgtataaaagcccgcagtgccagcgcttcgcctttgataatattatagttatccgctgtaaagattgattttttgttgtcgatatttttcaggatataatttgtttgcgcgatggtggcatacatattactccagatactattgatgatgcctgttataccggcattggtatactggtaggtggccgcataaaaaaagtcgtgatctattttcgtggtgttgtcgtatccctgcgataagacttccaggaaactgaaagtcaggtagccaccgtatagttgcccgtcggccgctttctgatagctgccatacagtgcatctttgaaaccctgttcagtagaaaactgttctgattccttgatttctgtcttgggtcttacatccagccatttcttgcaggaggtaagtgtgagtgaggtgatggaagctaccaggaaaagtatattgcgtagatgtttcatgttcagatcctcttaaaattaaaaagtggtttgtaactgtaaagtgaagctgcggctgaaaggataatccaggcctctttcccgcttaatgctggaccaccagaacagctggttggtgaagagggtgagcttggtatcgtgcaggcgtaaccgtgcgttctgcgcgtcacttaagcggtaatacagcgaggcgctttcgaggctcagccagtcgtctttctgtacaaagcgggaagtggcgtaggtgatggtgttaatggtgtacccgttattatccacaattcccttataaaaagttatgtcacctggctttttccagcgctcttcaaatacacggcggtccacattaaatctcatgtcagcgctttctaccctgtcaaccagtgtttggttataggtatagccaccaaaccggtaccggaagtagaggttcacaccgatgcctcttttttcaaaattggttccgaaggttccttccagtgtagagcgggcgtctcctactattacctggtccagcggatcatacacagtagtagtggtaccgttgcgggtacgaaaaatttctctcccggtagaagggtcgatgcccagcgaaggcactgcccagatagcggtggtactacggccttcagcaaagcgggccagcggtgtggtgctgagtgaatcagtatttcttttgtttagttgttcgagggtattggagattttctcaattttattctgcacatgaaatccgttggcaaaaacggaccagctgtcgcggttccgcgaattagagaaaatggtgtagcgtaaatttacttcataccctttgcttactacgtcgcccatgttatccatatacatggaaaagccggtagatggggcggtggtgatagacacaacagaaccttttgtcttctcttcaaaatagttggcggtaatatccagtcgtctgaaaaaagtaccgtcaataccaaagttgcttttggcggtctgctgccaggcaagattggggttaccaaagccaagcagggaggtgccgaggtggtataaataatcctggtcggtatagtacctgctggtggtaagaccgaggtagctggcaaaattggaagagccggtatatccgtatgaatagcggagtttcagccggttgatagcggtactgttttccaggaatttttctttatgaatattccatccgccgcctacgctccagaaagaggcaaaccgtttattggcgccaaactgggaagatccatccaaccggtatgaaacatccagcaggtaacggttatcgtatgcgtaactcacattggcgaagtatcccagcaaacgggtaagcccttctgtgccgaatggccgtgcacctgttttgtatccgtttcccagtgtcacctggtccagtttatcatttgggaacccgttgatggtgtaggattctgaagtcagtttttcctggcgcagggtggtacccagtgaaccaaagaacatgtgtgatccgaacgatttgtttaagtcgatggtgaaagccccatcgattgtattccttaaaccgtaacctttcgtgtaagatcctttttcataatatcgttccacagggatactgtcgaaggcagtgtgttgcgccgggaggaactgatctccgccattggtggtgcgctgataggcaaagcggccggtaaagcgcagccattcttttgcctgccattgcgcaaaaaagttgttagtgatattttgctgtgtatactgatctactgtgtgcagggatacattataaaccgggttcagttgtgaagccagccgggtgtcatcaaagaagcggatatcttccaggtagtatttgggatttccgtttgcatcgtaaggcgaccagtaaggatttaatttagtataagtataaaatgagccatagggtgagttaactgccttgttgaaattgagggtaagatcatttctgaataaaaagtttttatatcgataggacaaatacgtgttaccggagatattctgccggctggagcctttcatgactccctctgtagtgttgtaggtaccattgagaccgtacatcaccgattccgatccaccttccaggtagaggttatgggtactgccaatgccgttgcgcaggggtacattgagccaatcggtattgatacctttggctacttccgccaggcggtagttatactggaaatctttttcttcctgccaaacggggatgggatagccgttataaagacctgcttctttttccagctggagtttctctttggagtttaccaggtcatagcctttgaggtcgggcagttctgccaccacactaccggtataggttacacgtaaactgccttcacggggtcttacggtttcaataacaattacgccgttagctgcacgggaaccataaatagaggtagctgccgcatctttcaggatagtgacctttgcgatgcggttcatgtcaaaatcgtttacccgttgtagtgatacttcaaagccatccataataaagagtggtgtattggggctggtggtaaagtcgtatacgttgttttgattagtgccattcagattaccgaggctgttgccgcctcttaccactacactgggcactgcgttggggttggagccggcagcgatattttccggcatctggaaagagggatcgagtgcgcgcagtgcgcttaatacgctgttacccgataccttgttcagctcttcttttgtataggaagatgctgcaccggtgaagttttccgccggcctggaaaacagccctgttaccactactgcgttcagtgacttggaactggtactgagtttaaccgtgaggttagcggatctgcgtacttccacttcctttgtttcatagccaacataactgataagcagggtggctttaccggctgatacatccaccggtattttaaaggcgcctacttcgttggaggtggtgccgttcagtactttagttcctttctcaataacagtggcgcccacaatgtggtcgccgcttttttcatcgaggatacggccggtaataactgcctgttgttggaatagttctgctgcttcattgtccgaaatgccgggattggcaataggttttacatacaataccacgctgctgtcgacctcccggtaggcgagattagtattctccagtactgcattcagcgtagcgcttacggaacggctggcagtggggagcgtgatatgtttgtacttcgctactgctgtagggggataagcaaaaagaaatccgctggcctgctcaattttcttaatagcgctgtggagcgtttcatctctgaggccgagtgtaattgttttctttcccaattcctggccccacaccggtgaggctatcagtagctgaacggacaatgccagcagaaaagaatacaagaaaattatcttcataataaaacctgttttgccctttttcctaatgtatggttggttgattcgcatagggacatagcgatccctcacggagattagatccataattctgatggttgatttagataattacaattaaaaaaattagcagctacacgcggtgcacaacgcgctttaccggatgaagatcttcaccgatattatattccgtttgttgattgactaccgttttataagcgtttatctattgattggcacatccttcaccgttcagtactactttatcgttgggataaatggtatacccggcatttgccacactgcaaataatggtcagcactttctccaaaggctggttatgaaaaaatgttcctgcaatacggcaattttttaatgcctcattggcaaataatattttcacatggtacttatctcctatcataacagctgcttcctccatacttacatcgtccagcaccaggaattcatctttccattttaccacttccatacttttcacctgcgcccttactactgtactggtaagcatatttactgatagctgctgatctgctaccagtacgccatagctgcttttctcatcatttacctttaccttacccctggtaacggtaatcactacacgctgctgatcggttgatgcttttacattaaaagcggtcccaagtacctgcgtgctgagcttaccggttttcacgataaagggtttatccggcacttctttaatatcaaaatatccttctccccataaccgcacttctcttttattccctttgaagtcgcgattgtattccaggcggctgttatccgcgagtaacactgtacttccatcgggcaggcgtacaaacttcgtttgtacttccactatttcttccgcggcaggtgtagctgcggataggttaatggctaccagcggctgtttttcgcctgcatgccaccaccaccagccggcgacaggcagcaccagcaagccagttacaatggcagccagcgccagcctccgcatgccgcggcgacggttccgtttaagcgggataatgctggcaatgtgtgattcggccgacatgatattgccgatcatctcatgatagcgctcaaatgaaacgtctggttccatgatgccactatcccattccgcatctatccggttctttatttcttcatcaaagttgcctttgttgatcaatcccctcaattcattccactctgcctcgctggctttcccggcaaggtatttatccattaatccattgaatccagggtcgttcgtcataacgattacaataactttacaggaacttacaggtagtttttcaaaacttatataataacagacacctgacaaattccgatggtggagggtgaataaatatattttttattgttatttaacaagagtgatcatcaggaggatactgatgctgccgttcaggtaacggcggatcgactgtaacgccctggccatatgggatttcacggtaacggcggagatatgcatgcggctggcgatggcttcatggcttagtccttcttctttggcaaggcggtatacttcccgttgctggggcggcaactgtccgagggcggtctggataatttcccggtattggtgttcctggatccggtggtcagtatcgtttaccattacctcccggcggccaagctcttcccgggcggcggcctcattggcccgtttgcggaaacggttcaggaccaggttcctggtcacaactttcagataggcatccagattttttacttccggcagggtttcacgcttcagccaacacttcaggaacacatcctgcaccacttcttcagcggctgcctgcgaccggagaaaccggaacgccacagaatacaccttcgtacggtagcggctaaacagctccgtaaaagcatactcactgccctgtgataacagttccagcattgtgttctcatcgtaattactcggggaaggcatatccacgtaatatatgattgcccgacaaaatagttcaaaatattttagcaaaacaaaaaaaccgcagccaggaatgactgcggtacttttcttatccactcgtttatcgttgtaaactcaacgctgtattatgcgaaaactgttgtaatgtagccgttacagccctttccagttcggcgccggccagctctttgcggaaagctttttcctccagtgcggatatcaccttgtatagcggttcatcatttactttcttctgcaggttaatttcgctgctctctccatagatcttatcccagcttttacggactaccgcccagaaagccttatgctgctcccaccattccttagcctgctgacatttactttcactggtgcggttataggtatttaatcccttttctcccacaatcaccttatccatgccgtttgcgcggatcaccttctggttatcctgctcatgcacagagccggtagcggtgatttcatgatgatttacccggtgcaatacgttatagtccttacgggttgtgtattccctgcggggtaacggcgcatctgaggcggcttcccagtagtggcggccgtctgcatgtacccaggtagcggaaccttcatagcgcggttcatcgtccacgccatatactttctgtgaccactgaccttttacctgtgcggcgggcagcgtgaccttcttccactggttatcctgcgtataggtcagcaactgttggttttcatactgccagtcctctgtccagtgtttaatcacgttgctatctgcaatcagcagatgttgcaatacaatgcggtgcggatcttctgaggccaccgttacatattcaatggcgtcaataatcttatgatatcctttaggcttatagctgctatctgccgggaatgtttctgtgtattcaaaggtcacgtcctggcagccacacatacttttgatcgctgctttatcctgcgataatttatcgccgcccttttgctgggcggttgctgccagcgttatgaatgcgctgatggctaaaatggaaatatgtttcataaaaataataatgagtggttagttgaattggcgtgtgccatttggctgataagcaaaccggaaattataataacggcttactgaattctggtccggtgcagccggcgcatccttataatagctggtcacttccagtttggcataattaccattcgcggttttcagtacaattacagcgcctgttaccggtgaaattacgtgtgtggtcatgttgtaagcataccagccggtgatggctttctttgcagtagcatcggtagtatagcctgtttccggcgctgttgccaattgactgaatacaccggtaatcacctgggcttcggctttaccaggtccgctggtgccgccattgatgataatggtagtggctttgaaaccaatgtcccatttggtggtggcggaatcgctgttcggaattactttattatctgcgaggctgtataaagtaaagctgcctttatttgctgcatctgcatcaatgtttgttaccgttttggtttccactgcaaccaccggcggtgtaacggcatcatcatccttgctgcaggatcccagtgtaaaaagcgacagtgacagcataccagctgtgagtatttgtttcatatagtatttggttaatggtttacgtgatgataaaaattccaggtggcgccaatggaatagatcctgcctggcatggtactgatatgctgtgcatccgtgtagttaaacacgttttccagcgtggcctgcatacgcagctgccgtttgaacaggtatttagctgccgcaagatttaccgtagcataaccgggcacaaactcactgtccttatccggtgtgttattcccgttctcgtcggtgaagccgtatttacttcggtacagcattcgtgcatttgcatcgatacccaaacggtacaggctatacgctattttcaggttggctgaatgatgtgagcggttaaataatccgaagtattcgcggcgggtaagtgcgcgtgtttccccggtggtttcatctttcgtatatacttccccgtttttcacctttttgaaaagatcattatcttttgagcgaaggtattggtagccggcggacagctgcaaatgcctgcctacagcttgtcccagctccgcttctgcgccggcagtagtaatgctgttgatgtttacatagctatatactgccagatcgtttgtttttacggcaatagcgcgggtgtctatcaggttttttacactgttataaaagacatttactttggtggtggtacgggaaaatggtttcccttccactcccaggttataggaccaggagctttcggcatccaggtttttcaattgttccggatcgatgttcacctgtttgatctgcccctgttgctccatttctttcaggatatccgctgccagtttggtacctaccacggtgtaaccaactgctgcgttattaaaatgcaggtatagccgcctgaaatcaggcgcacggtagccgcggccgatggtgcccagcaggcgccagttgggcgttagctgatacgacaccgataacttcggactgaactgagacgggtattggttatgcgtatcaaagcggccgccgagtaatacattccatgcatttgccggtttccagttttcctgtataaatacatacccggtattaaaggccatccgttcctcatagcgggtggcttcgagcgattcatgcacatatcccacacccgcggtgagctgatgtttcggatgcagctgccagtcggcctgatattccggtttcagatattgctgggtaaaaaatgatgcatcatacaaacttttgtcctcccggtaatgcatatcttcattggtggaataccgcgaataatacacccgccacgtttgtttgaaacgctgtaccggcgtatgaatcagctgtaacgatccgttcatatccttctcctttccgatatcatccaccattcctttggcatccgggaaataactgttatacttttgttcatagtagcgcccggagaggatggtgctccatttgccggaccagttgtgctgccagcgcgactgtgccgtatatgctttaaatggcgatacagtaggcgcagtgctttggttaccaagcgtgtatccgtcactgttataagcatttacactggcggagaaagagcctttcttataaggaatacgtgtactgccatcaagggtataggtattattggaaccataccgcgcgctgatactgcttattccctccttgctgttgttgctggtaatgatgttaataacgccggccagtgcatcgctcccatagagtgaagaaacaggccctttaatgatttcaattctttctatattactcaccacaatcctcgacaggtcgaacgtgccggcagttctgcctatgagcggttctccatccagcagtatcagtgtgtactctgcttccagtccctgcatctgcacacctgctccatgattggaggtgatgaacaggccggtttgttctgccagtacctgttgcagcaataccgctcccatggcctgtatctgttgtttatggattatagtaaccggtaccggcactttgcttaacagttgttcattcctggtagcggtaaccactacttcctgtaacactttactgccggaagtagtgtcggtttgggcaaaaagggtccctacccgcatgatgcaggtgagcaggaataaatatttatacatcttaaggtttatctgaaattgtgaagcaaaagtacgggcataaacaacagcacctttacgagtttgggaaagttatttacgagatccggaaatttgctgttaacttagttagtccggaaaactaaccgttaccggaacaattttaaatcatcacctgttcattaatatatgaaaacacaatacttcccggcggccgacagaggcgttaaagacataggctggctgaaaagtaatttcttcttcagcttcagcgatttttatcatcccatgcgcagcgctttcggtacgctgatcgcgttcaacgatgactacgtagaagccggcaaaggctttggtacacatccgcatgtgaacatggaaatcatttccgttttactgaaaggaaagatgaaccataaagattccatgggatacagtaccgagatagaagcacctgcggtgcagatcatgagtgccggcagcgggttaaggcatgaagagtataatataggtacggaagaagttaacttcttacagatctggattcttcccaaacaacaaaacatttcaccgaggtatcagcaacggagtttcccgcaggaaaaaagaaagaacaaactggtgacgatcgtatccggtgaagaagggatggaacactgctggatcaatcagaatgcgaagctgtcgctcggatactatgagcaacctgccagtgttacctatgccttcaaccccttgaataagtgcctgtttatcttttctattgacggcagcctcagggtacaggaccaggtattacagccgcgtgatgcgatagggatatgggaaaccggtgaggtgacattgcagtgcggcgaaaaaacaacattcctggttatcgaaacgcctgtcaatcagaagtaaatctcttcttaatacatattaaatacagacatattattacttttctaaaataataacatccaatttattcatacaggtaatttattccaccgggaatcattaaatttatattgcaccgcttcaaaggctcaattacctgtatgattaatacctcccaaaataattacataggtttcgaggtactctttaaccatgccaccatcagcatactggttgccgacaatcagcagcggatcgtgatggccaatcccttcctgcttaaccagtttggctatacgaaagaagaagtgacaggtcagctggtgagcctgctgcttatcagcgatcataaagaacagtatgcggtaaggaaaaacggcagccagttcccggcagagatcagccaggctaaccactccaccccggaaggaatactaaccattatttacatcaccgacaccaccgatcgccggaatgcggagatgaccctgcgggaactttcgcagcaacgcaaagaagcggctgtgaaagacggctcgctccagcgcatgaacagcttccttaacagcttatggaccagtaccggcgccatgatcatcgtaatcaataacgatggtttcatccggtggttcaaccctgcagcagagaggattctaggctataaagccagtgaagtggtggatgtatataccccgatgctgctgcacgatccggaggaagtagccctgcgggcagaagaattttcacagcagctgaaccagccggtggctcccggtatggaaacgctcaccattaaagccaggctaaacctctataatgaatatgaatggcagtacatccggaaagatggtagcacgctgccggtttccctgacggtatccgccatacgggatgcggccgatattaccgggtatatcggtattgccatcgacctctcccgcattaaacaggcggaatctgagctgagaacttccctggaaaaagaacgggagcttaatgaacttaaatcaaggtttgtatccctcgcttcccatgaattcaggacacccctcagcgccatcctttcttccatctacctggtgtccaaatatgaagcagatgatgacgtagccaaacggagcaaacacattcaacgtattatttccgcggtaaatatgctgacggatatactaaacgacttcctctcggtaggaaaaatagaagaaggaaagatccaggtacgccacagcaccttcgacgccggtaaacacatcagcaacatcctgggcgaaatggacggactcaaaaaaaccaaacagaatatttactatgcgcaccacggcgccgcccatgcctgcatggaccctacactattaaaacacattgttatgaatcttgtatccaatgccatcaagttttctccggagggagccattatttccatccggtcacaatgtagcgacaacagcttccagctatccgtaaaagacaagggaataggtatttcagaagaagacaggcagcatctttttgagcggtttttccgtagccagcatgtgtccaatattcagggtacagggcttgggctgcacattgtagccaaatatgcggaattgatgaatggtacagtttcctgtaacagcgctccggaaaaaggcacagagttccttgttacggttcccttcccccaaaactgaggctcatggaaaaaatactgctgattgaagataatgctgccatctgtgaaaatgtagcggaaatccttgaactggccaattaccaggtgctcactgccaccaatggcaaagaaggcgtggccatggcgttggaacacctgcccgaccttattgtatgcgacatcatgatgcccgtgctggatggctatggcgttttacacatgctgcataaaaacaaggccctccagaaaacgccttttatcttcctgacagccaaagcagaaagaacagatatacggaaaggaatggagctgggtgcagatgattatattaccaagccctttgaaggcacagagttgctcagcgcgatagaaagccggctgaaaagatgcgctgagatcaaacaggacacggttaccggcttgcacgggctccaggtactgctgtcggccagtaccggcaaagatcagctcaccctactcaaagaaaaccgcaataccaatcactataagaagaaacaacgcatttacgctgccggcaaccgcccggatcatttatattacctgctccagggaaaagtaaaaacgtataaacggaacgatgaaggaaaagaactgatcataggtttatataacgaaggggattttcttggatataatgccctgctcgaaggcggcaactaccaggaatatgcggaagcgatggaagacacactggtagcagtgatcccgcaaaaagattttgaacagctgatcagcagtaacccggaagtgctggggaaatttatccagctgttatcaaaagaaatggcggaaaaagaacagcaactgatcgggctggcgtataactcgcttcgtaagaaagtagcggaagcattgctgatgctcgacaaaaaatacaataccgccggcagtaaacattttacgatcgatatcagccgggaaaaccttgccgcagtagcgggagtcgcaaaagaatcattgatacgcacgttgggcgatttcagggatgaacagctgattgccctgaaagaggggcagatcgcatttttatctctcaaaaaactggcggcgctggtaaactgatgcctatactttttctgccgctataaaaatgaggaatgccacctttaaacgctcgtactcctgcatcattccctccatatcatttttcagcaccgcataaagatgcggcgaaggcacgccagccggctgcttattcagccagtcgagctgctcccctatttcatgccgtaacaggatcaacgactcttcccggtccagcatcgtgagctgaaattcttctgcctcctcaataaacgaccgccgcgtagtttctttcaacgcagccgccagccggttaatcagcgaagcattatcttctcttaaagctttcagggttctgatccagttgttacatgcctcccggtaggccgcaatatctgtttcagtgctaggatcatacggcatattgatagttgctaattataataggtttgctgcatgtgcagatttttatctacaccccatttctttaatagctgacatagatgttgctgatgatgattcatttgccggatacctgacattaactccataatatgacggagatattgttcgcccggtaaatagttttcctttcttgccacatcttccaatacagacaacatcgttttgctttgcaaaacaaattccttcactaccttataaagtttattgatgtgttcctgtgcgggctccccttccggttcccgctttttagaccttccggccggctgcaattcctgcttcatattacgcaggattacattgtggtaaatagatacctcccggtagaaatgaatgatgagatcactgaaatccaggtaaagccccggtaaactaccagctgatgcctgtacctgtgtataaaattcttccagtttcagcatcacctttgcggtttcaggcgccgctttatctgcgatacagcgttgtatttcttctgcgtaccggtcgttgttacccggcatccccagttgcatatccagcaatgttttcacaccggcatgacgtccgtattgtctgaaaatatgattcccatatttacgtaaatgcctgatgggaaaaaaaagaaaaccttcacaaaatttccgctgacgggatgtaggagttaatccgctgaacatgatttgcatttttttaacagtaggtaaaagtaccaccgctgatagaacggtgataccttctcaacagcacatcttcgctttttgtttacgccaaggaatccaggtggatgtccaaatgctgccgtaaaactaaaccggaattcgttgctgaacaatgacgggcattactccttctgttgacagtcatcatttttttagatgaccgggatcattagcggactgatgaggctggtaatttatacagcggaaaacgaggaatttccttactacgcggccttgctgggtaacaacaataggaggcagcgaccgcacggagctaaagaacggcgccagttcttctgttacaaattcccgttcatccacatcatcatttacgtcggtcagtgaattgataaacagggcattttttccttttaatgcgtttatattggttccgataaaatcgaactgcagtgcattctcaccaataatattacgggagtataccatgcgccccaggtaaagattgagcatcgcactggttttataatcatcggcagaaaaaataaaatcatcggggtattctttcgacaatgccttcacaccatcgcccagccccttccagccgatcatggtatcatctgaatgaatgggtacaggataaaaaatgatttccactgccagcgccaggtggatcaccaatgaacagatccattgccagcgtacatacttaaaggtgatccaggtgcttatccatatagtgcccgttatataagcaggcatcatccagtttatctttacccagtaaatgggagaaatgaccaggaaaataccaaaaacaggaataaaaaaacataagaggaaaagctgacgggcagagatgcgcgtaatatgccatctgtatttacggaccagtttatacacataatacagcaaagcaaagaataatacaggtagcagaatagccgcctggtgaccaataacaccgaaaaagtccagcggacggaactccacgccctctacccggtcggacgactggaaccggaaagaggcaaagtcgttatccacattccagatcaccacgggcaaaatggtgatgcagaaaaacacgacgctggccaggaaccagggggaccacaaataccgccggtgttctttcgacagtaataaataaagcaccgctcccgccggcaggaaaacagctgtgtacttgctgtcgaatgccagccccatggcaatccctgcccatatccaataggctttacgctgctcaaataccgccctgtacactgctatcagcgataaagtccagaacaatagcaacggcacatcgggtgtggataccagtgataagatagtgaccatcagcgtagcgcccagcagcaacaggctattccaggcacgcttcagtggcaggaagcacctcgataaattgtaaaaggccagcagcgtaccaatggtaaccagggtatctgccagcttgatcacaaatatatgccggccgaataagtctgtaaaagcacgcaggatccaggcaatagccggaggatgatcgaaatatgacagggcgaagtgttgtccgtagaaataataataggcgtcctggggcatggcacccataatacctataaacgaaaatcttagcagcacaatcattccgatggcgatagccatgcatttatgcgctgtgatataagcaatgaaacgattactccccggtagatcctgcatatgataggctgacagttgtaattataacagatgatgtggtcagatgccctccttccacaatctctgtgccgcttggtgatttcatacctgctgcttaactataattaacattactgtaccccttcgttcagcttcaacaagggattattccgccttcagactatttaccggattagcccttgctgcccgtagcgactgcagtcccacagtagcaaaagcaatgagtaatgcgccggctgctgctatcgcaaacaggtaccagctgatgcctgcccggtaggcaaaatccctcagccagcgttccagtagataccaggctacaggtgtggcaatcaatacagaaaagatcaccagtttgaggaaatcttttgacaacaacgctacaatcccacccacactggctcccaatactttccggatgcctatttcccgggtacgttgctccgtcatgtataccgtcagcgccagcaagcccattacagaaatgaaaacggagatgaaagtgaacacatgaatgatatattgtacccgcgtgtagctgctgaaaacctgttgaaaattatcatccaggaatgaatagcgcagcggaaatcccggctctatcgtttcccatagggcactgatatctgccagcgttttatccaggttggccgtattcaccttcacgaggagcgctcctccggactgataagtgcaatgtgcattggaaatactgtacagggtggggcgtacataactgtcaaacccctgcacctggaaatctttcactacccccactatctggtagggcacactgtcgcaggaggcatagcggatctgtgtacccacaggatcaaccacgccaagcgatttggccgccgattcgttgatgatggccgtgttgtcctggtcctccgggtgtgcatccgaaaacatcctgccagccaggaccgcaataccgagtgtggcaaaaaaatcggtacttacccgcacggaagagagtgccctactgctgcctgcataattgaaagtgctgaaagaagtatctatatcgccgccgggaaccgccgtggttttggataccagttgcaccccgggaatacgtagcagctttgctcttgtttgctcaaaattcttttcacgggttggctgcatcgcttctatctgcactacctgctcaggattaaaaccaatatcccggtgtttcataaaattcatctggtgcgccatcaccaacacactcaccataaaaaatacagatacggcaaactgcaccacgatcagcgaatggctgaaacgcttgccggtattgcccatgctgaaattacccttcatcacatgtacaacgctcctgcgcgcaaataccattgccgggtacaagcccgaaataagtataatagccaacaaagcagctccgccctggaggatcattttataggaatacagctgaccggagaaagacaacgacaacccaaacgtttggttaaacaaaggcagcatgataatacacaggcacattgccagtaacaggctgataccgcattgaatggttacttccatcataaactgcccgagtatctgggagcggctggaacccatcacttttcgtactcccacttcccgtgagcgcttcaacgtttttaccagcgacaggttgctggaattcagcgcgccgctcagcaatagtaaacctgccagcaggaacagaatcatggttgttttaaaagggctgcttcccaaacgtgggaaattatgaatatccggtacggcttccgtaaacagcgaaggcgcatgtcccgctttaatataggctgcgtaagattcattacctgttttcaggcgatgctcataaaaaatacggttcactttatcttccaatattcccggtgttaatggctctcttaaacggatatacgaaatataggaaatattaccccagccactattagcagccatatatgggtctctcaatataatggaagcgtttatatgcgaaggcgtggccggttccgcaataaccccggatacagtgaaagccatccggttatacaccattatcactttccccatgggatcttctttaccaaacaatttttcgctgaccgcttttgtaatcaatgcagaagcaggtgcattgaaagccgtagctgcatttcctgccagtagccgcaaaggaaatacctgcaaaaatccgctgtcagccatcaccacgttttgctgatatattttgcgatcatctacactgatcagtatttcatgtttacccgagggtattatacgggtgtatgcctccacttccttcatatgttcctgcagcaaaggcgccaggggagccggcacaggattgttggcgaaattactttccgtttgccgtgacacacggtatacctgtttcagcgaaggatcccagcgatcataactgagttcatagttaagatatagtaagataatgagaaaacttgccaggcttattgccaaaccaccgatgttaacaaatgaggtgaatttgcttttcatcaggcttctgaaagcgatcttacaatagttgcgaaacattgcggtgagatttgaaacatacttataaaaaaggtgccggaatccggcacctttggttatcagttccttataattaagcacccgatagacaatgttcactttcgtatggaatatgttcattttcgaacgccggcaaatacgctatggctgcatcgtccattgtttttcccactggaagaaatcaggcgcggcggccggcttcccttctaactgcgcagtgagataagtaatatacattttccagcgggggagataaaaattccgcatcaaaccaccccattccttgttggcataatcatgcagatctgtttccgggttgtccggcccccaataagtaatctgtgttttggcattctttaccagcagggctttttcagcgggtgtttgtcccatactctgcgctgcggttatccaggtatccagcctgaaatgacggctgccactcagcaacaggtcttgctgctttatgagcgcgaggaaagcgttggatgtttgtttaaatgctgccaggtcttttttccggtaggcagccaccataccggcaaatacctcttcgccctggttggcggttacctggcgctggaaatcaatggcgtcaatttcataggtagcgttatccttcattttgggcgctgccttcatgaactccgctaccgcttcggcaaattgccgggtatcatagttccgcttgcgcgtaccccaggatgacacgggcttgtcttccagcgtgggccttgcacagaataccgactcattggggccttcctggtattgcggaaagctgctgtaagcggtagcaatcaatccctgccacgcagcctgcaactgcgcgttatcgctgccataacggtaacgtacatatgattttatccattcctctatgtctgttttctccgaatgccaggccagttccaacatcaggtcatagatcaccgggttgttgtggattccttccggcataatacctactcctttgaaccgggcagcatacggactgtgcgccgcgcgccatgtttcatctgcaaagcgctgcagcttaccatagagcccggacttttccccgaagttggtaacactgcaccagataaagggcgtgccttcatatcctttgcgggtttcccagttggccgtattttctccaaaaagttcctgcaccagcactttcgatttatcaagtcctgccagcagtgcgcccgagggattggcctgccatccctgcaacacccaggtgctacccgggaaatgctgtaacatggtttgctgaatagtacgggcggcggcggttacatctacccctttactgatccctccttcatgaaagggatcaccggcaaagaagcggatattgctgccgtagagctctttcatctcttcataataaataccggctattttggtaaaggcactatctccgggcgccaggaaatccgggcgttggaagccacccgcccatttgccttgttccactaccctgatcttcattttctccttcaggcttacagggatcattccataaaagccctgcatcacaggggcaataccgagtccctgcatacgggtaagcacctgcttctccaatgttgtttgctgatcgatcatttgctgggtaaccggcccgccccatccttcgaggttgcccatgagccaccacgcagtgaatcccggacctgccacaaacttacgggcctcgtcgctgctgtatcctagccgctccagcgtatgctgccacaccgcttccgtacccatggtagcgagcattacgtttacgccattaagcgccatccagtccagttcatgctcccagtctttccagctgtagaagctcatcgtatagctgatggtgcaataattgagcgcataacggtaatcgtaggaggtattgatgtgtactttgtcctttatggagggcagcggggataccggcgccaggttatcgcccatgtgcgacatggaacggtgacaataatacttcaggtaccagttgaggcctgctgcagcggcgctggggctggaagccgtgatccttacttctttgccgggggtggtgatttcaaatacatctttgccgttttccgcggggatacttttcaataccagcttatcagccagccacggtactcggcgttgtgccagttgtttcacagcgggataatcctgcgcaaaaacagacgcagacaagcatagcagcagcgctgccagcagtttcttatttttcattggttcactgttagatcaatcaatctttaaagatggtaaaaaattatgaattccagatccttaattcataattcgtaaatttaacagacctcttttcaccaaaacaaccctgcatggctggacagatcaatttaccggagcatatcaaaggtttagatgaagcagccgttaccgcttcaagacaacaatatggcagtaatattcctccggaacctgttaccagtccgctgaaagccgtattaaaagaaatcatggaagaacccatgctggtattgctgatagcagtaacggctatttactttgtgatgggtgaacttggcgaagcctattttatgctggcggccattgcgctggtatcaggcatttcattttaccaggatagccgcagccgcaaagcgctggaggcgctggagaaaatgaatgagcccctcagcaaggttatccgcaacggagaattgaaaagtttacccaccagcgaaattgtaaagggagatatgatgctggtatctgaaggtaatacgatcaatgccgatggtatgattgtacacagcaatgacttttccgtcaacgaatccgcgctcaccggcgaggcttacgccgtattcaagcaaagcgacagtgaagataacaaagtgtacagcggcacggtagtggcatccggactggccatctgtgaagtacaggaagtaggcgcgcaaacaaaaatcggccagctgggggaagccatccttaatatcaaagaagaaacaacaccactgcaattacaaatccggcagtttgtaaaatggatggccgtggccggggccatcgttttcctggcggtatggttgtttaattatatccgcagtggcagtcttaccgacagcttgctgaaaggattaaccctggccatgtcggttttaccggaagaaataccggtagcattcaccacctttatggcactgggttccaggcgactcatgcagatgggaatcattgtaaaaaagatccgtacggtagaagcgctgggcagtgctaccgttatctgcaccgataaaacaggtaccattactgaaaacaaaatgagtttgcaggcggtatataacggcaccgactatacgctatatgaaacaggccattttccgtcagtgctgatcagcaccgcgatgtgggccagtgagccggtaccttttgaccccatggagaaaacactgcaccggctatacgaagaaatgacgccgctggatgagcgtaccaattacaccatggtacatgaatacccgctggaaggcaagccgcctatgatgacgcatatttttgagaatgctgccggcaaacgcctcgtggcagcgaaaggagcgccggaagcaatattgcaggtttccaatctcccggaaaaagaaaaacaaatgatcctcgaccaggtaaacatactggcggcaaaaggctaccgggtattgggagtagccacttctgattttaccggcaacaattaccccgccactcaacaggagctgccgtttttttttaccggtttgctggctttctacgatcctcccaaaagcaatatcagtgaggtgttccgccagttttaccaggccggtattaaggtgaagatcattaccggtgataacgccgttaccacccgcgccattgcaaggcaagcgggcttgcagcaggcagatgaagccgtgaatggtgataccctgatgcagatgaatgaaaaaaagatgcagcaaacattgcagtccgtcaacattttcacccgcatgttccccgaagcaaaactggcggctatcaatgccttaaaggcagataatgaagtggtggccatgaccggcgacggtgtaaacgacggccctgcgctgaaggccgctcacattggtattgccatgggcaaaaaaggaacagaaattgccaaacaggccgcagcgctcatcctggtgaatgatgacctcagtaacatggtggatgccattgcaatgggacggagaatttataccaatataaaaaaggcggtacagtatatcatctctattcatattcctatcatactcacggtatcgcttccgctgttcctcggctggatttatcccaatatatttacacctgtgcatgtcatcttcctggaagtaattatgggccccacctgttctattgtatatgagaatgaaccgatagaggaaaacgcaatgttgcaaccaccccggcccattacccaaacttttctctctttccgggaaatgaatatcagcatcctgcagggcctgatcattaccgcaggcgtgttaacagcctaccagtggagcgtggcgcaggatgcgggagaactgctcacccgcagcatggtgtttaccacactggtgctcgcaaatatttttcttaccttagttaaccgttcgttctattattcttttatacacagcatgcgcaaccggaacaaactgatggttgccgtaattggtatcaccctgctgctgctggcagcaatgctatatattccgccggtggcaaggttcttcagtattaccggtctttcaccgtatgaactgctgctgtgcaccgctatcagcgcagcatcggtactatggtttgaaatatggaaactggggaagagaaaatttcagcgcaatttaaactgatgatatgatgaaggtatttacaacaaggattattccggaagaaggattatcactcctgcaacgtgcaggctttaccgttacacagtggtcggaagaaaaggagatgacagctgcgcaaagagtgcagtattgcaaaaacagtgacgccttgcttttcgctggtggtgaaaaactggaccgggcatttttagaacaatgccggcacctgaaagtgatcagtcttttatccgtagggtacgacaacgtagatctgaaagccgctacagagctaggcttacagatcaccaacacacctggcgtattaagtaatgccaccgccgacaccgcttttttactgatgctctccgtggctcgtaaagcgttttatcaacataaaagaattttaaaaggcgaatggggattttctactcctaccgccaacctcggtaccgacatagaagggaaaacactgggcatatggggcctgggcaatataggcacggtaatggctaaacgctgcaaggctgcttttggcatgaaaataatttactgtaaccggcaccgcaatgaagccgccgaaaaagaactggatgccacctttgtaacttttgatgagctgttgcaacaaagcgatgttatcagcatacatacctctcttacaccggaaacaaaagagaaatttaaccgggaagccttccgcaaaatgaagtccactgccattttcattaatgcggcgcgtggaggcatccacaatgaaacagacctcattgccgctttacgcgaaggagaaatatggggcgccggactggatgttaccaatcccgaacccatgcaaccggataatccactgctggaaatgcctactgtagcagtactgccgcacatcggctccgccacactggaaacccggaacgccatgtccaggatcgctgcacagaatgtaattgctgcgttaaccggccagccggtgccgaacccggtgaatcatatttatgacctgtaaacaaataccgcggttgattgttgggctggtacaattcagtaactttagttaaagcacagcagcatgaaaaaggtcgctatcattggcggattacgtgtccctttcgtaagatcctttaaagagtataaccatatcagcaaccaggaaatgttgaccacggtactgagtgcattggtggacaaataccagctttccgggaaacggctgggagaagtggcgctgggcgcattactgaaccgctccacagattggaacttcgccagggaatgtgtactgggcacttccctggacccgcatacgcccgcctatggcgtactaagagcctgtggcaccagcctggataccactatacagctgggactccgtattggctgcggacaaatagataccgccatcagcggcggcagcgataccaacagtgatatcccattgctgtttcaacaacagctcgcatggaagctggctgacctgcgcgctgccaaaaccttttcccaacggttaaaaatactcgcctccatccgcttcaaggatttgaaaccattatacccttccatcgtagaaccgagaacgggattatcgatgggccaacatactgaaaagatggtgaaagaatggggaattacacgggaagaacaggacgcgctggcataccaaagccatatgaatgccgcaaaggcgtatgaggaaggcttcttcaatgacctcattattccttacaagggtgtaaaaagagacactattgtgcgggcagataccacgccggagaaactggctgcactgaagccggctttcgacttcagcggcaaaggttccttaacagcaggtaacagcactttatacaccgatggcgcggctgctttgctgatggcctccgaagagtttgcccagcagcagaactggccggtactggcgcacctcgtggatgcagaaactgctgccgtggactatgtgaacggtgaaggcctgctaatggcgcccacctatgctgtggcacgcatgctgaaacgcaatcacctgaagctccaggattttgatgtttatgaaatccatgaagccttcagcgggcaggtattgtgcacgctgaaggcatgggaagatgccgcttattgcaaaaaactcggatgggatacgccgctcggaagcatcgatcgaaacaaattaaataccaaaggcggcagcgtagctattggccatccctttgcagccaccggcgcccgcatagttgcccaaaccgctaagatattgcaacaacggggcagtggccgggcattgatttctatctgcaccgccggcggcatgggcgtaacggctatcctggaaagataagcatcaattcctccttacttttttaacgatgccaggtaggtaaccaggtccaccagttcctgctgcggcatggccgtagcaaggccggtaggcatcagggagtgttcatatgctttccgcgatacgatggtgctcttctgcagttttacaccctggccacccgccgtacgcacatccacttcgtcttttgtttcccctgcaacatagcccaacacctgtgagccatctttcagtttaaagaaatagccttcaaagccaaagctgatgccggcatccggttcaatgatggcgtcgtagatagcgcttttggtaagcttgctgccaatttctgttaaagcaggaccaaagttcacaccggagtttccatccaggtgacaggtagcacaataattattaaatactttttttcctccggagatgttgcccggcaaggctaccagcttatctacaggcagcagcacgtggtgtacggctgcaggctcataataggctacagctttggccttgatgtcttgccgccatgcgttggtgagtactgccctggccaccgtatccaggtcggcaggaagtgatttgccttctaccatattccacagatctgcaaatccgtcccatccatgaccgagattgcgggtcgcctgctgccgtaacgttaaagggtatatgttgttacgcatcagtgaagcaagtaacgcacggttggtgcgatcctgcgctttgccaatggcgtttatcaatataacgccggatactgaatcctttttcgaaatggctttgattaccagcggctggccgccgcattgcaggagggttttcatggcgtatccctgaatgtcgtcgcgttttgattccagcaccatctgcaaaagcgcttcattctgatcacggacatgatactttaacacgaggtcgatgaactccatatgtcctttaaatgcactcaggctgttgcggagcaggacttcaatatcccgtgttttgggcactgctttcgcatccagttgtataaatgccagtgcattgatataggcttgttgcgggtgctggcctttcagtaatcccagcagcaccggcgtgctttctgcggcgggatagaaatcgaatgcgcggaaataacgtttgttttgcaggggatctgtacccggttccaggatcagcgccgctaacaacggtagtgctgccggtgttctggcgcgccagataatatcgtggtctgctgcgggattttttgtattcggtggcaatttccgccactcgttgaagcaggcgtcccagttgccatctgccgcgatgcccagtgcttccaggtaccacctgtctttcccgttgtattgtgcagcgagcagtgcccagttggccggcatgtctttttcgcggctatgatgcatggccagcaataactggcggcgcacagcggcagaagtatctgccaccagcagattgccataggatacgccggtttctttggcagcgcggatggcggtaatgcggatatcttcatctttatctttcagcgccgtttgcacatacccgttgccgttaggcagcctgctgagcagccacagggcgcgggcgcggtagcgggagttatcactggcatacagttgctgcaactccttttctgcggctgcacccatgccggacagtttcgtccaggcaagataacgggtactgagattaggattcttcaatgcagtaatggcatcggccgcggtgttgagcaccggtggctttactttatactggctaccgggcggggctatacgaaatacccgtcccctgttcaggtcgcctacctggtgaccaccaacacctggatcataccaatcggctacaaacagggaaccatccggtgccacacatacatctgatggccggaaccactgatcggaaccgctttccaggatattttcaatggtggccgtatagccggcaccgtatttttttacaggataggatctcaccacattatggccgggctctccgtggatcatctggttacggaaaggagcgggcaacaggtcgccttcatagatcaccataccggtaggtgaacctgaaccggtttgcagcaggttaggcactacaccgggatcattgagatgccagtgccggtaaggaatagaatcttccatattcatacggcgggatgaccagccagcgccggtcatctcatccgtataaccatagttgccgtattcaagaatataattgatgcgaacacccctgttaccatcgtcatcgttatcactctgccacatgttaccaaaagcatccaccgccacttcgtagttgttgcggaaattatgcgccattacttccaggttgctaccatcttcattacagcggaaaatcattccctgccggtaaggctttcccttgttggcgataaggttaccctctgcatcacggataacgtttccatttttatcaagtatgctgtcgccggcattaccgaaattaaaatacagttttccatcaggaccaaaagtaaatgagtggatggcatgatcatgctgtatgccgccaataccgcggaaaagcaattccttcttatccgctttatcatctccgttggtatctgtaaaaataaaaacgttcgggctgcaagacacaatcactttatttcccagcacgcaaatacctaatgctgcattaatgcaggtatcctggtaaaacactttggcagtgtctgccttaccatcgccgttaagatcttccaggatcataatacggtcaccggcagccttgtagggatgaccgggatttaattcattgcggtaattataggcctcggtgatccatacccgccccttttcatcaatatccatgttggtgggattcatgatgttgggttcactggcaaacagggttgtttccaggccggaaagtgttttcagtccgtgtacggcattttcaggcaagcgttgctgcgcttccgttagtacaggcgggatagccgcaggtttattggattggcatgcgctgatagcaacggataccataaataacaatcggtgaatgtatttcatatacgtggaaataattaaatgtcaatataacacgtattaaaagtaataaaataattcacatttttttcataaaaaaacccgtcccgggaaaccgggacgggtggtccattgtcatccatttcaccgaataaataattcgttgcaggtatagtgcagataccatgccggaaatgaataaacagatgaggattaaaaacttagtgcagtattttttccagttctttttccaatgcttcccccctcagattagtagcaataatgcgcccctgcggatcgagcaggaaattctgcggaatggaatgaatcatatacaatttcgcgatatcacttttccaccatttcagatcgctcacatgatgccatacaagaccatccttttcaatagcagcagtccattttgcttcatcaccagttctgtcgagtgaaacgcccaggatatcaaagttcttatctttaaatttattgtatgcttttaccacgttaggattttcagcgcggcaggggccacaccagctcgcccagaaatcaagcaatacatatttacctctcaggtcagataacttcagcgttttaccatcaggagtagcagcagaaaaatcaggagctacctggttctttcccagtaatgcagaagctttcagcagttcggctgctttttgcccgaggcttgactgccgcaatgccgctggaaatttattaaacagttgctgcgtaccttccacgtcttccacgcggccacccatgttttcataaagggtcgccaggctcacataataatcggtgtgtgcgagcataaacttttcctgcaatgcatctttctctgttgccagttttctgaaagccatgctcagcgcataataaccggtagtatctctctcggcctgcatcatcattttctgcccgatagcacggagggaatccataccttttgtaacaggcgccagcgccgcctccatttcctgctgttgtttggtaatggcggaacctttgatcactgcaccggacaatgcgttggtctcaccaagcgttttgagtgtgaaggtcatcttgtcgttcggcgtaatgtacagggcctggttgccacgcagtggtttatctgccgctttggtcgctacgcttagcatcgccgccaaagtatcggttacttcatactgcagtttgaaagcgcctttttctatcagggcagaatccagctttttgtagccgttaccggatacattgaagaggtagatgtactccttgtcaaaagccgcgggtattttaccggtaatgacagacttcttttgtgcaaatgcacctgaaacggctactgttgccaggcagccgagaatcatttttttcatacgatgaatgattggttggttttgcccgaaagtataaaaatgcggcagccccttcaaatgcttaatgacaggcggtcgatgaaccatgtttaccggcgtgactcagggaatgagtaccagcctgctgccgccgggaacttcccgcgtccaggcagcggatatttcactgaggggcatctctatagtagtaatctgcagtttcccttcggcggcattcttcataatttcgggaagtattttaaagatagcttctatagatacgctgccaataccacttcccaggatctccaaccgcgaactgcgcaatgcgccggaagggagcgaaataggatctcctgccatagcacccacctgtatgaggcgtgtacgcggtgtttccttcgccatacctttagtcattaatgccgtgataagcgccatcaccggctcgccccacaggtaatccaataccacatcataaggttgggtggcaaaagcttttaccaggttttcgggagattgatccaacgcgatgcactcatccgctccaagcccgcgcaatttttccagtacggctttattgcgaccggcggcaattactttgcctgctccaagcaattttgccacctgtactgccagttgaccggatgtgccggtagcgcctagcaccaataccgtttccccctgttgcaactgagcccggtaggttaatgccatccacgacgacatagcgggattaaaaatagcggcggcagtggcatcagtgaggttatccggcaccgggatatgccagcccggggtggtaatgcttaattctgcgaaagtgccataaggcttacgtacggcgccgaaatatacccgggagccgtctgccagcagccctataccatccacaccgggaataaagggctgatcgccacccgcagaataatgctttcccgctgcaatagactttactacatgatgtatggccgcggcctttacctgtatgatttgttctttttctccggcggcaggatcggcgaaatatccatattgaggagcctgaccgggtgttacaattgctgcattcatcttctttgcgtttttatgttacaaaggtgcacgacgaaaaaacaggatcactttacatttgttaagaaattaccgctggagtttattcctgatccggctaagggatacaggggtaatgccaagataggaagctatgtattgcaggggaaccctttgcaggatgtgcggttgctcacgtatcagcgcctcatagcgctcctgtggcgtgtcacggatctgggatatgaacattttagcgtaacgcagcaaacgctggaaagtaatttcttccatcttcgacctgaaacccggcatactatcaattaccaggtccatgttttctttcgagatcttatagagccgggcggcagtaatagtttctattgtacacatacttggctggccggtacgaaaactttcaatagaagacaccccttctccctcaaagaaaaactggaaggtggtatctttccctttattgttaaaccacacgcgcaccgctccttctatgatgaaataagcataccgggatattttgccttcctccagcagaacagacttggcaggtacgcggatatcttcatagaggtgctggtaccgcgaccaatcaatgtattcagatccattcataagtgttgcagctgaaaatatccgagataaatgggatctgctgccacaccatttgccgggctgacctccagtgtatacctttctttgagatgcgccggtaaaatatcttttacggtatgcacatcatccacatctacgccatacttatcatccacatgtgaagtggcttctccaaatgaagtatgcttgtaaaaggccgtttgtttggatgcccgtattgatgcaccgatgtctttctgcacgctgaggatcttgtaatgaaattcttccatttcatcaggcttgtaaccgcccaggttcaggaaaaataattgcatctcctggttcaggggctcctttttctccactaccctgatccggtggttatccaccatattcacttcccggtacccatcaatgtgaagtttatctttggcctccggccagaaggccttcatatcaggaatcaggtcacgcaggtgatgaccgattccaaaaaaaacatcgtgttgttcggtatgacgcccttccagcgaacatcccaacaccaccatgaacaattttaactctgccatttttttactgtttgcagtaagaaaggtacagcatttttagttcctgttcatggcttcccggagctgtttttctttatctgcgctccagtatttgcaatcaaggctcataaaaacggaagaataggccagtgtgctgtttgttttcagcaccaccactttaaacagtcccgctgttttatccatcttagaaaaaacggaatcatgcagtaaggtttgtacggactgtcctttaaaaatctgttgcaacgtatcgcggtaagcagcggcgcccggtacatataacaactctttatccatgtaaaggattggctgaacatgtgtactgcgatccagcccttgaaccgtataacgtgccacttccggcatcgctgcaccggtattgatatacaccattccgggcgacgactgcagcgggaacgcctcatcggcaataataatccagttacggtgacccagcagcggcaacaggctatccagctgcagttgccacgatggctttgccacagcagctactggtccgttttccatcttacaggaaaacagcaatataaccgctatggctaaacgaaaatatgatttcataaattatacgatagtaagatgaaaatgctggcctgccttcaacagcagtggtgcggacagttgaatagttacagcgccgttttcttctttgaaagtggcgggtattttcttatctcccagcaatacctgcttcgcgccggtatgctgcaagcacagtgtatttatttgcagttgaccatacttcagctgcagtgtatgcctgcgcccttgttgtgtataagttccccagccttcggcggtgacaaaaggcgctttgaaatgctccttgtttatagccggtgcaaaggcgataaaacctttaggaccatgatagcggaatccgctggcagtaataaaagtaccatagctggccattgcccgcgcatagtgatcactgcattcaatttcgttaaacggattacgctttgctgcatggtaccggtcgtgtacggcgcgggtaagtgtaagcgcttcatctgtcatcccttccgccatcatatgcgcggctacctggtgttcaaagccgctcatgcattcattaaagtaaccgagctgccaggcattctttacgccgaatggaaattcttcattgcggggattcgtattcaggatcatacctccttcgcctgcgagggcatagggccggcctccgggatgagcggcgatataaggtcccacgtctgccttaaaattatatttatacagcgcctttaaagccgacaatgttttttcacggtcaattacccggtccatgcctacctggaaagcccagctctggccatatacctggtcgatatgacaggtattgtaagagccgatcaccgacctcccctttaccttatccggctgatgaataaaatattcgccgttgaataactgcgtttccatgttccgtttccctttctccgtatagtcgttgcaaatagcagcgaaggtggtgtcatttacctctgcggccatgagtgcggcggctttaacagcggcgatacacaggcctactatccaggcaatttccccgtcccaaacagcatccagtgtattctccatcggtgtgtcttccatgccgtcgttattacggtcctggcggatcaggaacagggtggccttctttatattcggccagttttgttgcaggaaagaatgatccctgctcatctggtgctcgcggtaaatacgcaatatggtgcctgcttgtccgtcgatagccgggcgcttttctgcttctccacggaacaggatgccgccatcaggcatctggccgatgccgaggtctacccgttgccgcgtgtcgcgctccagcgccgggaagatacgtccaacggcctgcgcatactgccatacgtgcgtgcaggtaccttcgcaggcgcctacgccttcccaggcataaaaacgtccggaacggaaacggtgtgccgtggtggttgccaatgttgatatgttgagaaaagtacgttccataaaccaccatggcaatgatgcatcgtaccaggtatctttccacaagcggctttcaccggccaggcgcgcataattttcctgcatgtatttcattactgccgatgcatcggtaaatttattggcataataacgtccctcaccctggatatctttaaaatgcagattggccgcataccaggagatcgcaaaatcagtacgtatactcttgcccggtagtatggtatgcctggtggcaacggtgccggtcagcttctccccaaatccttttactgcctgctttgaagacatcagggaaaaatgtgcggccgttaattcaccagggggcatcgccgggtttaccattactttactacctgctgcagcaatacaaaaatttccatagtcgtactgtttttgaaaatcgtcatcattgccgcttttagtacgtactgtttcataaatgccctgccagttctttcctttcacagtagtatttacgcgttcatggtcatccccggcagaataaatagccgtcttattttccagccatccgagaacggttgcagtaacaggtacggtatccttattctctattttataagatagaatggttacaggcaacccggaatcatcttcattcaaaggaataaaaggtgagaatgcttccagcgttacaacaaccggcagcgcgggatctgtataacggatagtggccatcgggtaagtggcttcaaaactgatttcaggccagctttcttcatcgaaccggcggataatggtttgtttgccccaggtaagctgcaacgcaaatccctggtcgagcggccggatatttttcgatggctcaatatagcaggcgccatccctggagcgtacttttttgccaccatccaacacattggcgctatagttaaccactttgggttctattccttcctggtttttattaaaaatgtcccagagccacaggcggccatcaccgccgaggtacaccgtgccacacataatacctcccaccggcataccgatgtattgcagttcatttttgcttttaagataagtggtagcgttgccacgttcatacagggaagcgatccaggcggcatccggttgccgggtgaacaataagcggccacttcctgccatagcgctgcctaacaccggcaggcgcaccgttaatgcgccagccattgttaaaccaatatttcttagaaatttcctgcgttcaatacccataaaaaagtgttttatttccaggcagctgtttgtaccaggtttttatttttatcgagggccgattgtggaattggccatgtgtaatgctttagtggattaaaggttctgtcctgcgctttgaaagcaggttgcgtccagtcgccaacaggcgctttttcatcctggttaataccataagcaggcttattcaataccagttccgcagttttccagcgtaaaatatcaaaataccttttatgttctgccacaaattcgtggcgacgctcgttacggattttttcacgcatagcatcctggttgcccagtagtgcatctacgcctggtaagccggcgcggccccttactttattcatggcggtaacgatcgcaggattagccggatcatattcgttcagcgcttccgccaggatcaacagggtttcggcataccggtagatcgggaaattcatataggccctttccgggtccggattaccgggttctgcaaatttcaggtacataaacccggttaatccgccaccttcgttattcattttctccggcttattataggcaggatgcggctgataggcggaatagctgccatcaggccgcaggcagggcacaccaggcaacaggaaagttttcttcaagcgtgcatcacggttatcccaggggctgcttttattgtataacgtagacgactgtatgcttttcccatctgtacattcataggagtctaccaggtcacgtgtcgggcaaaaactcgcccagccttcaccggtaatagaacatcctgtaggcagggccaacaccggcaacatattggtgatttcattctggatatactgataggccaggatcacttctttattggcgttgttggattcgtgcgtgaacaggtaagcataatctttttcaaggtcataagcgccggtgttcactacattttgcgcggaggttgccgcttccttccataacgtaacatcattggtaccggtatgaaattttttatagctggccatgtacaggtatacatttgcccgcagcatcatggcagcggccttattgatcctgccggtattggcgccggaataggcatcaggcaacatggatatggcggtatcaacgttagtgatcacgtaatccaatacttcttgtttcggactcctggcaatattcgattcctcaatcgtcaaaggtttttcttttatcagcggaatatcgccatagagctgcgccatacggaagtagcgcagggccagtataaaacgggcctcccccaggtattgttttttctttgcttcgtcgatagtcataccgcttagcttatcgatgcaggtgagtgcacggttgatatagtcgtatttccattcttctgcaatgtagccatctgctgccgattgactaccctggcagatataccccattccgccttcgccccatgcattggtcattacagaattatcgctgtggcagtcgcgccagaaatcacggctatcaggcagggtggcatataaggcgttcacgccttgctctgcatctgcagcggttttccagaagtcatccacagtgggctccgacaatggcgaccggtctaaatatttggaacagctttgcaggaatcctgctattgtgatcaatatatatatgctaatctttttcataattatcagaattttaagttcacaccaaaagcccatgttcttgataatgggtagtatcccccttccggatcaaatccgtcgtaaccgctgatagtagcgatattctgaccggatacaaatacccgcaggtagttcatcttccactgttgcaggatccgtttgggtaacgtatagcctatctgtatattctgcagtttcaggtaatcggctttgcgcagccagtagctggaatatttggtatcattagatgtatactggatagaaagacgcggatagctggcctgtggattgtccggcgtccatgcgtccaggtgcatgggccttgcattttgcgaaaggaaaaatgcccagccttcgtaactgctgatataacgaaaagtattcagggtgccgtacatgctggcagaaaaatcaaagttcttccatccggcatttaggttgagggcaaaacgaagtggcacctttgtattcaatactatgcggtcacctccatcaatttttccatcgttattctgatctttatatttaatatttcccgggaaaatattgggaccctgatcgggactttttgcaatttcatctgcattctgaaaaaggccaatggcttgtaacccgtatggcaaacggtattgggcgccctgagaagtatagtaggtgttggcgtccggcgtttcaatccatggtccggtacccgccatgttggataccttattctttgcatagctggcattggcggtaatgccccagttgaaaccgccttggctgtctttgtaatataccaatgcctcgagaccgcggctctgcattcccagcaggttggtataaggcgcctgtagtccaaactccattgacacgggcgcctggtagaggattttatcgcggttattaacaaaatagtcgattgtaaaccctaccttattatcgaggaaacctgcatccagtccaatgttacctaatttggcttcttcccaggaaagatccttatttacagctacgctggtataagcgccgggaacgatagcattattaaatccatagatattcggctcaaaatccaggatagctgccgtagcatagtagccaaccttttctgcatctcccaaaataccccacgacgcccttacttttaattcggataaccagctgaagtgatctgctataaaatgttcacgatgaatattccagcctgcagagaaggaagggaatataccccagcggtggcccggtgcaaaccgggaagatccatcgccacgcatatttgcttccagcaggtatttaccgtcatagtcgtagttgacccgtccaaataccgactggatcgctacttcactggcgttgccaccattttgtttattaagggtgcctatatccagcacattcacctgggcgaaaggaagtccatcccgggaggcataaaaattagtaaggttatataactcctgtgaatagcccaggagtcctttgaagtgatgcagtcccaggtgaagggtgtaatccgtggtcagctggagtgtgttccggaaattggaattagtggtattctgcaggctgttcacctggttttttactgctgccacgttgccattatcatcatacaggttgtaggtattcagccggctggttacccagttatcataactgtatttcgcataacttcctttgatgttccagttggtgagcggggtgtaagtgatatcgaagatgcccatcagctctttcactttattcttatttacaccgccctcattaacgcctgcaatggggttgcctgccatggaggaaccggtgccgtattgtcctgttgccgaggtgacaggagatataggagatacccgggctgcctgggtttgccagatggtggttccgccctgcggttccgtgatctgcgtttccgtgtactgaatgttggcggacactgataaatggcgggaaagcttaatagtcatatccggccggataatgtaacggcggtagtcgttattcggtaacgtaccatcctggtaatcgtaagagccggacaagcggtaggtgatattatccttctgcccggaaacagcagcatagttgttgttgataaccgtattgcgcttataaatctctttataccatttgttatccggcagcttacctgccttcagatcgtcctgtcctttctgaccgtatatgggcgttttcccgtcatttgccaacgcttcgtcccataatttcatataatcagcggcgcctacaaagtcgagacggaactgcggctgttgcacgccaatgctggaggaaatatctactaccggctgacttccggcctgtccttttttcgtggtaatgagaataacgccattcgcagcgcgtgagccgtaaatagatgcactggcggcatctttcaatactgatacgctggcgatatcgttgggattgagggtattgatgttacccgggataccatctatcagcgtgagcacaccggagctgttaccgatggtggaagttccccggatattaattgctgcaccggagcccacggcgccggagcttttgctcacatttaatcccggaacggtgcctgcgagtaattcctgtgcattggtaacgggccgggatttaaaggcctgcgctacatttacggtgcctactgcgccggtgagattagcttttttctgggtaccatatccaactacgattacctggtcgagattactggtagatgtaagcaatactacatctaatgtagtacggttatttaccggtatttcctgtgaggtgaagccgatcagtgaaaaagtaagtaccgcatcgccgggaacactaacagtatagttacctttttcatccgtaagcgcgcctttgccggtgcttttgtgcagcaccgttacgcccggcagcggaacgcctgttccatccgttatccggccggatacggtgatgagcgcctgctcaggcgctcccggttccaggagcaccagccctgacgaccggatttcatatttgaaaccggtgcccgccagcgctgcgtccaatatttctttcagggaggcgttcctggcgctgatggtcacatttttactctccggcaacgtattatcgttatagaacaaacgataatccgactgggccataatcaagcgcagtacttctttcagcggaacatttttcacttccacattcagtttcttttgcgagaagacaacagacgcctgcacctgtaagagtgcaaccatgattaatacagttgtaattttcataattcgcaagcacttgcggaaaaaaagccggcacacccgcttttgtttcctgtagtcatttttcataagtttgtattggattgttgaggcaatagacacccctttccttaccaagcaaggatgtctgtttctgataacatattcgggggggatggcgcaatcatcttccccttttttatgatcctgttctgattaatacaacggcataacttcgctgattttggtttgaaactatttagtgctgatttttaaaactctgctggcctggttgtaatgccacgaaaactgcccggaagagcggcttaatacggtcattacttcattcatctgttcaccttttatactaccggaaaattccagtgcttttaattgtgactgttcaaatacaacggtgatattgtaccacctttccaaccgggttgccaggctggaaaatttctctttgtcaaaggaaagggtattgtctttccacgctatttctgtaacggcttgttgttggttgtgccagagcgaatcccatctggcggtgaagatggcagttccttccctccggataagtgtaattttttgtcccggtttcaccaacgctttgtgcagggcgtcttcctgccggtattccagttgtacacttccgctgataagggatgtttcaatgttgggttcatccctgtaggcgcgtacgttaaaaacagttcccaacacccgtatagtggcatctttcacctgtatttcaaaagggatatccgcctgacgggctacatcgaaacaggcttctccttccagttgaaggaaacgccggtgtacgccatactcatcgttataaaccaatttactgccggcgttgagccataccagtgtgccgtcaggcagcgtaacctggctgcgggtaccacgattggcaactatttcatgtatcccgttttttttatgaggatgggcaaagaaaaaatatcctatggtgatcagcaaagtcagtaccatggctgccagggtcaggtatctgcgccggggaaaaggtacgttggatggcgcctccgccagttccggaatatgggtttccagcaatgccagcagccgttgttcttctgttacggatataccgggagtttcctgctgccatatctgttccagtgcagcagcggttcgctgctcctcctcctgctgcgcagataaagccgccaactccgacaattcttccggagtagcttcaccgttaagcttacgtgctgttaatatccaatatcgctgaataggcattaaaatatggttcgtcctgttaataagacaagccacaccgttaaatcacctaaaaggaataaaattattttacaagatgggcatttactgctgtatgaatgcgttgcagtgcaatagccagctggctatcgatagtgcgaacagaaatgctcaggatggcagcgatttccttgtatttcagcttttcttcttttgccagccggaaaatcagccggcatttgggaggcaggttgtcgatagcagcctgcattgcctgggtcatttccagtgtaatcagctgctgttcggggtttagtggttgttccagcggctccagtaatacctccatctcttcaaacgcataaaaagtgatcctgtcgcggcgctgcagataattcatacaggcattgcgtacgctggtaaacaggtataccctgagctgtgttatcttcagaagattactgcgattactccataaccctgcaaatatgtctgctactatatcttcggcagccagcggatcttttatgaaagaattggcaaatttggagagtcccggcatcagatgcaggtataatgccttaaaggcattactgtcattgttcaatgctatattttcctgccaggtgctgatcataacgagtgtcaagcaatatatataaccttcgggaaggattataccggatgttaacagagcgtcaggaaatgtgaagaaatcatcaggcggggatcgccttcggcgattacgcggaggttgtctttctcaggattacactgattatgttgattaccatgattagattttgttgctgattttgattttgatttttgtaaataatatggaagataacagcggatatattcgctactatcttccctaatccttataaatccagtgaacaaaatctaatcatggtaatcaacataatcagtgtaatcctgagtaagacaaaatccgcgctaccatacaaacgtagccacttctcccccgcgaagggatgcagccgccactttgccttttgctttgatctggaagtcctgcgccgccgcatcagtgtttaccacaatcagtacggttttgccgccaggcgttaaaaaggcgacgttatcaagcggaccggcaatattggaagcgattcttatggaaccggcaggaacaaatttagatgcatggcctattacgtagtaggaggagttgcgtgaaatagcctgtccatcaatggtaatgccaccgaggcattgggagcatccaccctgatcggtatgcggattccaatgcgcatcagcggcgaggttccattgcaatacattgcggctccagttacgggtggcgcctacaatcagtttgctgacattatttttcaactcgccggaaaaactgccttttccatcagaccattgctctgtgaagtaaaggtgcttttccgggaactcatcatgtactttactcagtgcatcaatagtgccgccatacaggtgaaatgcagagccatccacgtaaggataagcggctttgtctctcagaatagtgagcgggtattccggtttatcacagttgtgatcatacaggataatttttgttttgacgccggcctttttaaaagcggggcccaggttatctttgataaagatggcctggtcttccgccagcatcagcatgctcggattatttttaggatgtaaaggttcattctggatggtgatggcatcgatggtgatgccagcggctttcatcgcctttacatattttacaaaatattgggcataagcgccgtaatattgcggtttcaggctgcctccaataaacgagttgtttgttttcatccaggctggcggcgtccagggagagcctaagattttaatacccggatttagtgcggtaatttttttcagcacagggatcaggtcttttttctcttcgttgatattgaaatgcttcagttccggatctgtttgtccttcgggcatatcgtcataggtaaatacagaggcgctcaggtcggaagcgccgatgctgagacgcaggtagctgatgccaatgccatttccctttgtgaggaacagttctttcagcaatgcatcctgttgcgcagcaggcagctggttgatcagcgtggcgctgccaccggtgagggtaaatccgaagccgtctatcgactggaatttctttgcggcatctacctcaatggtggcgatacctttatcctgcgcggtaaatgccaacttagctgtttgttgctgcagcgcgatggatttgtcgggagatgttaaccagtaactgatctctttattttttttctgctgactttttactggctgtatacttcctgtcagcaaggcgaggcaacataggagttgtccggttctcttcatcatagcaaaacaaattattaatcggtaaaagtattcaggaaattccggattttcttatttggagcaattgtttcgttagaaaatatcaacctgaatttcattgctcaggcgtacggtctatacttccagtataaatgccagcgcccttttttctgaccagtaaaaatcttctccaaacttcacaaagcctacatggcctccctggtgcggagtttccaggaaaaggtagggactatcggccgctatctcataagggtaacactcctttcccaggaacggatcatctttcgcgttgatcaccaataccggtatcctgatagaggacagcaacggccgggaactgcattgttcccaataggtaagggcgtctttaaacccatgcatgggcgccgtatagcggtcgtcgaactgccggaaagaacggatgtccgcataccggtcgaggctgatgcttcccgggaactgcaactctttcaaccgcagcttttcccccaggtcgcggatgaaccgctgcatatagatgatattgtgtcttttctctaactccgcagagccgcttttcaggtcacacggcacagaaatagccacggccgactttatagcactgtccagcgatgcgcccctttctcccagatactttaatgttacattccctcccagggaaaagcctacaaggtggatggccttatattttttcagcgataccaggtattggatcacggtatgcaggtcctccgtttcaccgctatggtaaaaacgcagatttttattcggttcgccactacaccccctgaaattcatggataccgtgtcaaaccctgcaccattgaagatatgcaccattcccagcacatacttgcgggtggcgttaccttccagtccatgcaggatcactacaatacgctcattccccttttcactaaaatccaggtccaggaaatcggcatcgggcgtagcaatcctctccctcctgtaagccgccggccggatgctgcggaataaagagggataaatggtaagcatatggcgattctgcaataaaaaaggcgcctggtaatctgagttatgtaatacgggcatcctgcaaatttacggattcaaacaccttaatccgtattttcgcggcatgtcacttcccgtttttggtatagagaaaatatttaatctcccttacaaaaaggaagattttaaaatagtatatcatgcaccgatcaatatgacggtgataccggaagcgcataaacatgactttttcatgctgctggtgattagccagggtagcggtgttcataccatcgacttcaacgactacaaagtgagcgcccgcagcgtttttttcctggcgccgggccaggcgcaccactggcagctatcgaagaacaccagcggctaccaggtgatgttttctgcggagttcatgttacagaaagggcccctgtggccttttttcacaccatcgtccaaacctgtattaaagctggacaacgcacagtacgaccagcttttccgggaactgcagctgatggagcaggaaaccgccgccattattacgcaacaccggctgcagattgtgctgctgttgctgcagcgctggtacgccgccatccacccggaagaagtggctgccgcggggaatcacctggtcaaccgcttcctgctgctgctggagaaacattatgcgcaatatcatgaagtggcctactatgctgccaaactgcatgttacagccagttacctgaaccaggtatgtaagaaggaaaccggcaaaaccgccggcgcctacatccgggaacggctgctgctcgaatccaaacgcatgctcacactcaccgatatggatataaaagaaatcgcctttacgctgggctttaatgatacttcttacttctcccggttcttcagaaaatatacgctacttacccccatggattttcggcgccagttataaaatgtacccgtgatattataaccagtaccattttccacctccatacggggatacctttgcagctatagcataacattcgtatgaaaaaaatactgttctcttcgctgatactgctttgcgggatatccgcattcagccagcaaaaaaaagccgacctgctgatcaggtctgtacgcatcattgatgtaaaaaccggtaaaatcactgccaaccaggccatcgcggtgcgcaacgacagtattattgctgtgatgaataacaaacaggccacgcaataccaggccacgcaaatggtagatgggcagggtaaatatgccatgcccggcttatgggatatgcatatgcactttggtggcggcgacacactggccgaagaaaataaaaacttcctgccgctatatctcgcccacggtattactaccatccgcgattgtgccgcagatatcagcacagacgttttaaaatggcgcgatgccatcaacaacggccagttacagggccctaccattttcacctccggtccaaagctggaaggttacaaatccgtttggctcggcgacctggaaataggcacctccgcagaactacaacaggcgctggattccctgcaaaaactgaaagtcgactttgtaaaaattaccgagaataccattaagccggagatctacctcgaagcattaaaagaagccaggaagagagggatgtttatttccggacacgtaccttatgtactcaccatgcaacaggtaacagacgcaggactcagctccgtagaacacctgacctatgcctggaaagccggcgtaaaagatgatgcggcttttgcgcgtgccatcgccaatggtgaaatcaaaggaaaagatatcaataaatatatcctcaacaactttgataccgccgctgctatgaacacctaccgtcacatggcagaaaaaggcaccttcataacgccaacgcttacactgggaaatgtaatggcgtactttgaccaggataaccacgcacacgatccctacctgcaatatattggcaaaggtattcaacgcacttatgaaatgcgcgtgaagcgcgtaatagcagatgatagcgctgccattgcctggcgcaagatgatctatgaaaaatcatcttccatcctcccgctgctgcagaaagccggcgttaccattatggccggcaccgatgccggctacctgaactcatttgattatccgggcatcggtcttcaccaggaactggcactaatggtaaagttcggattaactccgttacaggcactacaggcctccgtgatcaactcacccgcttacctgcataaaaccaattatggcgctatcgctcccggcaaaaaagcagacatcctgctgctggatgccaacccgttagctgatatccacaacacacagaaaatccacgccctcgtagtaaaaggcaaattcctcaacagatccgcactcgacggcctgctggagcaggtaaaagccaacgtcgcgcgtacgaagtagagcgcggattttgtcttggctcaggattacgctgattatactgattagtttgatttttacttttggattttataaaggattaagggagatagaagcggatatactcgctcttatctcccttaattataaatctaaaaatccaaaagtaaaaatcaaactaatcagtataatcagcgtaatcctgagccaagacaatttaaaagcgccgaaggcgccctactctatcgccgagaacagccgcccccaacgaatacggttatgatgaatgctcatccagatgatccaggctttgcccactacatggtcttcgggaacatagccccagaagcgcgaatccatcgactcgcggcggttatcccccatcatccagtaataatccattttgaaggtataggtattggtttcctggttgttgatataaatttttccgtttactacgcgcagcgtgttatgttcataggtatctataatgcggctgtaaaagggcagtgtaagcgtgtccagcgttacggtggaacctttccgcgggatatataaagggccaaagcaatcttcattccactcgtagtgttttgtatcaaagggaaacaccctggaatccgcgaaggcgtcatatacataacgctttacggtagcgcccatcgacttcagggtatctatattggcggtggtgaggttgtaaataaacatacctgaatcgcgggtagcccgttggatatggtctgttcccagcacatcccgcatagagtcgctgagttctttcttatccggcatggtaacataatacctcgcttcaaaatgttcaggtgaagcggtaggtatatgattgatatacacgatgccatcgatgatctgcagcgtatcaccgggaatggcaatgcatcgcttgatccagttttctcttttgtcgaccggccgggttatagcaggaggataatttttatgaacgtattccgcaccaagcgaccgcatattcgtgtagtaatcctcatcatcgccggtaatggttttcagtacagtatccccgcagggataattaaatactaccacgtcgtttcgttgaatactgctgaaacccggcaaccgtgtataaggccattgaacagccgtggaaaagggtggggtgtttctggtaaacgggagcgtgtgatgggtaaaaggccaggccagtggtgtgatggggatacgcggaccgtaactgattttgctgacaaaaataaaatcgttgatcagcaacgttttttccatagaagcgctggggataacaaaagcttcaaagataaaggtacggataagggtagcggcaaccacagcaaaaagagcagcttctatccattctctcaccttcgatttcttccgggtaccttcctccggctgctttacatcgctgaaagaaaaattcattttacacgtggttttggataagtaactactaacaatttaattaattatacccacatcttttcaaaatttacaggaacaaaaaaggctgctgcaatgatgcagcaagcaaggcgtacaaagctttacagcagtatcatacagctgaaaacaagggttgctgcagcgaggtatctgtgttattgaagccagtacatcctgttgtactattctacccgtttccgcaaaaaagtattacctcccgttatcctttttaaaaaatttcaacaagataaaatcgttttattaaattgctctgcgtaaccacttcagtagttgcacatttacccacgttccaaacataattaccatgcatacgtcgagacgttctttcatacaacaaaccgggctgatagccgcaggtatgatgttacccggtgcgctggccgccatgaacggcaacaaagcgctgccaaagaaaataggtttacagctgtataccctccgcgaccagctggccaaagaccccaaaggcacgctggccaaagtagcaggcatcggctacaaagaagtggaaacgttttacggctaccagggagcgggcgacaaagctgagttctggggactgaaacccgccgaactaaatgccgtgctgaaacaacaccagctcagtacgcccagtggccattaccagcttaacgactacctctccaaaggcaatggcaacgcagatgcactgcagccacaaattgacctggccgccgcgctcggacaacaatattttatcgttcctgtactgcccctctccctctgggataaaaagctgggcgcagatgattataagttcatggccgaacaattgaataaagccggcgaacaatgcaaaaaagctaacctgaaaatcggttatcataaccattattgggagttcaaaccactggcagacaaccccggcaccggttatgagattatgctgaaagaaacagatcctgcactcgttgcctttgaactggatcttttctgggtcgtaaaatccgggcacgatcccattacgctgtttaaagaagcaccaggcagatttgtcgcctggcacgtgaaagacatggacaaaggcaatactgccagtcttaccgctgcaggcacagaaaacaaaacctcgatggaactgctctccggcgttacctttgcagaagtaggaaccggcagcatcgacttctccaaaatatttgcccaggcaaaacttgccggtgtaaaacacctctttgtagaacaggacaaaatcaccatcgaaccattcgacagcgtaacgcagagttataaatatgtgaagaacgttttgttgaaatagcgaaggttgtcttactcaggattaaacggattttattgatttaaggatttgatcctgttggattttaaaagatttggggagatataagcggatatgcccgcggattttctcttactcaggattaaacggattttattgattttgttgattttactttttttgattttataaaggatttggggagatataggcaaaattcgcttatatctccccaaatcttttaaaatccaacaggatcaaatccttaaatcaataaaatctgtttaatcctgagtaagaccacatccgcgaagacaaaattcgcgtagttttgcaccaaagcaagtaacctatggcgatgcatgaaattgaaacattggtggaactgtctgttctttgcctggataaaagccaggaagaaggacttgatcgcaggagcctcttttttaatctgtacaaattacaacagcaatacgacaccggctttacccatttccgggtaatggatgtattaatcaaacatcatttcgtttatacctttcccgttaccgcgcatccgttctatgccacgcatgcggcctggtttgatgcactggctgccagtcagaaattcagctttatttatgaagagcctactgctgaatgggatcaggaaaccaatcctgtagcgggttacgccaatttcgattttgccacccaatcctatattttatattgcgatgcgggatcttctctctggaccgctatggtagcccatggcgtccttaccggcgacgatgccgcagcgccggaaaagatagataccttcccgctggcgcatgaagtggcggaagcagccggcgaacaaaaagataaagatgtgctgggcctctggtaccagctccttccttacatggtaatggaggcagaacaggaaggtgaacccattcactacaaggcactggaagccatactggaactagtagtagccaacgacgccattcctgatgaaggattgccgccggcagatgaactgcccgtaggcggtgagctggggaaattctgtaagtggtggtacgcgcccgcagcagataaaatgcccgccaccgcgccggaagatgtggaagaagaaatagacctcgaagccgtagcatttacagaacaggtcgataaaagtgctgcctggtacgaacaacaggtggtacagatcctccaggacgccaatgctgccatcacgcacatggaagacagcggccccaatgaagccacacagcgaagcgtgtatgagcgcctgcaacaaggattggtgtacgccaataaaggactggagctatcacccggtcagccgccactgctcatgaacaaaggctccatactgatgctgctggaacaatacgatcaggcgctcgccgtttacaacgaagcactcgccattgcacccgaaaatccatatgtgcacctgaaccgtgcggtactcttttaccatatggaacagatccccgaagccattgcctcttttgaacaactgctgcaactggaaccgggcaatgaattcgcacaacagtggctttcacatctgaaaagtgacgggtaataactgcggttataaactatttacgcggagcggttgttaaataagaactcccgaaaaataaccgcaaatggaaaagacgctccgtacgtttgaaaaatacacctgttatacactcctgggtataggcatgttttatatcacgttccagattgtagaactgttatggcttacagctaccggccttataaaacgattccaggatgttgggtttacatatgcacctgaatacagccggagcatgaccctcctgttcttcaatatactgctggccctggagatactggaaacggtaaaggtgtttgaaaaaagccatgaagtaaaaatcaggattatcctgatggtatgtatgattgctgtaagccggaagatcctgatgctcgatatttttgaagggaatcctatgtcggagatagcgctggcagcgctcatcgtcgggctctccggtggatattacctgatcaataaaaagctatctgtcagatctgaagaacaaaactagcgggccccggcctgttgcaacagctgtacgatctctttatagcctcttttttgtgcatgttgcaaagccgttacaccgtctttgtccgctatattcacatgggcgccggcggcaatcagcatcttcaccacctgctgatgcgcggcgccaccctggcctagtatcactgcctccaggagggcagtccagcccaggcggttgatatgatctaccgggaaatttttatctgccagcaaaatggctatcacttcaaggtgtgcgcgttcgcaggcagggatcaacgcagagccgccatagcggttatacactttataatccgcaccaggcaggtatagttttaccagatcggtatagccttccgcaccggcatacaggaaaggggagttctgcaggtgatcctgcgtatttacattagcgccggcagcgagcagtaattttgcggcagcagtatgatgatgataagtcgccaccattaacggcgtacgcccttccgcatcttttgcttccacctgttcgcccctggcaaccgccgttttgatagcatcggtatcattggccgcagccgctttaaaaatgatcatatcacgcatagtcatctccttttctttttgtgcacaggccggatgcataacccagagcaggcccagtaataaggttagtcgcattgtcgaggattgttacacgaaaataaatcaatgctgtgttgataactggtgctattcatgcataaaacaggactaattaaaactactgttcttcttccgcccgttaaaaagatatatccgttcatctattttaaagccaaaatccggatttatttgctaacttattagtgattaaatccggtagaaaatgccacaggaaaacgaccaacaaaaccatccgcataaaaaggaaaaacatgaggcccgccgcgacttcctgaaacaatcctccgcgatgatggcactggccctcacaccgccgctggtaatgaaagcagcgcagcacgatgaagccattgccggcatctttgagaagatgccggttagcatggaaataaacggaaaaaaagtacaggttactgtagagccgcgtgttacattgctggacctgctccgggaacaactggatctgaccggtaccaaaaaaggctgcgatcacggtcagtgcggcgcctgtacggtgcatgtaaacggccaccgtatcaattcctgtctcacgctcgccgttatgcaggaaggcaaaaagattactactattgaaggcctcgccaacggggaacaactccacccggtacaggaagcctttattaagcacgatggcttccagtgcggctattgcacgcccgggcaaatcatgtcggcggtagcctgtatccgcgaaggccatgccggttccccggaagagataagagaatttatgagtgggaatatttgccgctgcggcgcatacgacaatatcgttcatgccatcatggatgtaaaacagggagggaaaacagtatgaaccaattctcctatgtacgccccgccagtctgaaagcagccatagatgcggtggcaaaagataacacggcccgcttcattgccggtggtaccaacctgctggacctgatgaaaagcggtgtaatgatcccggaaaaactggtagacattaaccgtttgccgttaaaagatatccagctaaatggtaataccctgcatataggcgcactggcacttaacagtgaactggccgcacatgagctggttaccacgcatcatccgttgctgtcgcaggcattactggcaggtgcgtcacagcaactccgtaatatggctaccgtaggcggcaatatgatgcaacgtacccgctgcacttatttttatgatactaccatgccttgtaataaacgcagccccaacagcggctgtggcgccattggtggtatcaaccgtatgcacgccatctttggtgccagcgaaagctgtattgccgtacaccccagcgatatgtgcgtggccctcgccgcactggatgctaccgtactggtaagcggcccaaaaggtaaccgccgtattcctttcacagattttcaccgcctgccgggtaataccccgcagctggacaataacctggtaaagggagaactgatcacagcggtggaaattcctgctaacgcctacacgaaaaatgtatactacctgaaagttcgtgaccgcgcctcttacgcatttgccctggtatcagtagctgcagcgctggatatcagcaataatgtaatcaggagcgcccggctggcaatgggtggcgtagcgcataagccctggcggctatatgaggcagagaaagcactggccggtaaagcgcccacggaagaaaatttccgcgatgccgccaacatcgccctgcaatctgccaaagcataccagcataaccggtttaaaaccggtttatctgtcaacagtatccaaaccgccttacttaaagctgccagcgtatgaaaaagcaacaaacaggacagtcgatggaccgtgtagatggccgcctgaaagtaaccggcggggcaaaatattttgccgaccatcacttgccggatctgctgtatgccgcgctggtatgcagccctatcagcaacggcaccattaagagcatcaatactaccaaagctctcaaggcccccggtgtgcaggatgtggtgtctcacctcaacgcgccgccggtgccgggatacaagaattccgatcccaacgcgaaagacggtctcaaaatattcaaagacaaccgcatctactccaacgggcaacccgtagccatagtgatggccaatacaatggaacgcgccgtatatgccgcctccctggtggaagtacaatacaaccaggaaacgcattataccgatatgaatgccaatatgggcaaagcctttcagaacaaccggatgaaagactatacacgcggggaagcagacgcctggaaaaaagcgccggtaaccattgatgccacctacagtcttccgctggaagtgcataatcccatggaactggctggtattattgcccactgggatacgccggattcactggtagtgtatgccaaaacccagggagtaaaaaatgtacaggacaccatcaaaagattattccaattacccgaacagaatatcaccgtgcattcacagtttgtgggcggcggttttggtatggcactccgcgtttggccacttgaaatagccactatactggccgcaaaaaaagtgcgcaaaccggtgaagctggtgataacgcgtgatcagatgtttacactggtaggttaccgccctgccgccgtacagcaattaagcctgggcgccacagcggatggtaaactcaccggtatcacccatgaagcggtggcagttacctctccttacgaggattttaccgaaggcattgtagccatgagtaaattcatgtacgcctgcccaaacgtaaatacccgctataaactggtaccgcttaatatcagcacgcctatctggatgcgcggccccggcgaagctaccggcgcatttgcgctggaatcggcgatcgatgaactgtcatataaactcaatatggatccgctggagctcagaatactgaaccacgcggataccgatcctgaaaagaacctgcctttctccagtaaatatctccgggaagcttatcagctgggagctgaaaaaattggctggtcgaaccgcaaagccgctccccgcagcatgcaggaagacggtatgctggttggctatggcatgagcagcggtacctttggtgcattccgcggtaaggctacggtgtcggctacactgaaagcagatggtgcgcttattctccagagcgccgctgccgatattggtccgggtactgctaccgcaatggtacagatagcagcagatgtaaccggcattgcccctgcgaaaataaagttcatgctcggtgaatctgcctatccgttcgcaccacagcagggcggttcttctaccgtatctactttaggcagcgcggtaacagatgcctgtaaggcgctgcagcaaaagctggcggaccttgccatcaaccatgtgccggcgtttaaaaatgctgcccccgaaacaattacttttgaagatggacaactgcagagagccgggcaatctgaaaaaatttcttacgaaacgatcttacaacaacaacagctgccggaagtaaatgtagtcgccacttcgcaaagcggggaagaaagaaaaaaatattccatgtattctttctccgttcactttaccaaagtacatgtacacccggctaccggcgtggttcgtataaaacatattgtaagtgtggcagatgcaggtactattgtaaacgctaaaacagcccgcagccagatgattggcggcgtggtaggcggcataggcatggcgctcaccgaagaagcggtcatggatcaccgtttcggacgttttgtaaacaataactatgcagactaccacgttcctgtaaatgcagatacaccacccaccgatgtatatttcattaacaagaaagatccttacattaatccgatggggtcaaagggcatgggagaaatagcgctgataggctttgctgccgcagtttccaatgcagtgtaccacgctaccggcaagcggatacgtgacctgcctatcactcccgataaagtgcttgatgagaaagtataccagttggaaacgagaaataaaatgaattcatgaaagaactggaagatatcgtaaaatcatattatgctgcctgcagccagggcatgaaaaccgcgctggccaccgtggtacacgtagaaggctctgcttaccggcaacccggcgcaaggatgctggttacagaaaccggtgtgctcaccggcgccatcagcggcggctgcctcgaaggagacgccctccggaaagcgcaactggtaatgatgcagcaacaacccatgctggtaacctatgataccaacgatgaagatgatgccaaactgggcgtaggactcggatgcaacggtatcattcatatattgctggaaccggtgaacgcggaagatcccaccaatcccgtggccatgttgcaggaaataatatcccatcgcgcatcggcagtattggtgaccctgttcaccctgcgccagcgcaaagcgccacaacccggtacctgcctggtactcaccgccaatggccagatgcagcactgcataacagacggcgacctgcaaaacgccgtcaccgcagatgcacatcacgcattgcaaacgcatacgtcttttacaaaaacatacctctctaccggcaacgactatacggcacatatagcttacatcccgccagcgccacaactattgatcgccggcgccggcaacgacgttatcccgctggtaaaaatagctgcgctgctcggatggcacaccatcgttgtggatggccgccccggttacgctaccactatgcgttttccggaagccacacagctgatcaccgccaagcctgcacaagtgctctcccaggtacaaacagatcactataccgtggcagtgctgatgacgcataactacaactatgatctcgccctgctggcgcaactgctttcgctgcaactgccttacaccggtgtgctgggtcccgccaaaaagctgcagcgcatgttcgacgaactggctgaaaacggcatctgcgtttccgcggaacaacgggcacgtatatacggaccagcaggactggacctgggtgcagaaacagcggaagaaatagccttgtctgttatcagtgaaataaagtctgtactctctgccgctgccgctacatcactccgggaaaaaagcactgctatccattcccgcgaacaacagattatccttcaacaacaactataatggaaacaactggtatcatcatcctggccgccggagcctcaaaacgactgggaacacccaaacaacaacttcccttccagaacaaaagcctgttgcaaaatgtagtgcatgctgcccgccagtgtgatatgcccacggtggtggtgcttggcgcctttgccacccagatcagggaacagctggtgtcagaaaaagtacacaccgtggtaaaccccaactggcccgccggcatgggcggctctatccatacggggttgcagcacctgctacgtatagcccctcacgtaagtaatgctttgctgctgctgtgcgaccagcctttcattaccactgcgctgctggaagaaatgtttgcactgaaagatgctaccggcaaacccatggtagcttgcacctatggcgacgctaccggcacaccggcgctttttggcaaatcattctttccacaactgctggctctcaatggccaggaaggcgccaaaaaaatattgctccaacacagggagcaggtagctaccgtcgattttccacagggagcagtagatatagataccaatggcgactatgaacaactgcttaccagtacaaaataaaccgctgtttcagggtacaactccagtatgaatacacccttctatctgttacccaaccgaagaaacctttatggtactgtattacaggtgcctgaccgggtatcgctttctcctttctgaaaaaatattttttggtaaataaaatgacatgcttatatttgtccacaagattggtagactaataaaaacttaccgccatgaacacagatcagtattacctaaagctgcgccagataagcgcatcaaccaaccaccccgcaatagcggcgtcttattgttgttgttaattcccactcccccctgcggccaccccaccaattgccgcgacaccattttctatttcaacaactgatttaacactgttaacaaaaaattcgtcatgaaaacgaccaaccaacccgtattctcccttgccggaggagtcactgcagcgcatcttgcctggttccgcacctatggcatcatacagttcaaaaactttctcgacaaaagtgcattggcaaccgtgcatgaagaagtggaacgtgtacaggaattactgatcaggaataacatccagaaagtaaacggtattccgctcaaatttggcacagacgtggacggcagcccgctgatccagcgcatcgccttcgcatcgcactacagcaacgtgctgcgggagctattaaaagataaaagactgcaaacactcacagctttgctgggcccctactccggcaggatcggtgaaaacgaaaaagacggactggtggtaaaccattacgtcaacactacggagagccagtttaaacaactgggttggcacaccgacagtccgcgcgatctgttcctgggctcacgcatcctgccaatgctcaatgtaggcattcatctcgacgattgcccgctggacaatggcggcctgagagtattacccggcacacatgaacagggaatactgaagttattattcagaaagaaatacttcatcgataataaccctgatcaaaaagaagtaggccttgaaattgaagcgggtgacctcacggttcacgacgggcgcctctggcaccgcgtacagcagtcgccctacaccggcgaaaaaagccgccggagagtgatgtatattcctatcatcaccggcgcctatcagcctaaaacagccagcagtcctactccgttttatcacaaactggcacatctcaaacaacatctgtatggtggcaaaccacaatgggcacatataaaagcccggtccgaaagcctcgcagaagtaaacacgccatctctttaaaaatatattccgatgtcatacgcattaataaccggcgcagcaaaaggaataggaaaagccattgctgcacaactcgcggaaagaaattatcacctgttgctggtagatatagatgaaaaaagcctggcagcaacagcggaaacactcgcggcgcaatatcacgtgaacgtacatacgttacaccaggatctgtccgccccggatgctttatcaaatgttacaggctggagcagcacctggcatcattcgctgaccgtagtagtgaataacgccggctatggcatcaacggacagtttgagcaactcacgctgcaggaacagttcaacatcattgatgtaaatatcagggcacaggtaggcttatcgtacgcctatataccggtactgcggcaattttctaaagcatacctgctcaatcttgccagcactaccgcctatcaaacggtgccttatctcaacatttacgcgtctacaaaagccttcgcgctttcctttacacgcgggctccggtatgaactcaggcattcccccatatcggtgagtgccctgagtcccgggagcaccgacacggactttgtgaaccgggcacgcatgggtgactacacccgcaacattgccaaccgcttcaatatgacgccggaaaaagtcgccaaaattgcgatagacggcctcttcaaaggcaaagcggagatcattcccggcttcaccaataaattgaacgcatggctgccaaaattcttcccgaaattatttgtagagaaaatcgccgcaggcatctatgaaccaaaagagaaggaagccggcacagtagcactcaccgcataatacaacccctgcttatatcagaaagcggcatcaggcctggtgccgctttctgatgtatatgggaacaacatttgcagcgctcttattaaaaagataatggcaactgcaggcattcatatcggcacatccggctggagctataagcattggcgcgaaatattctatccaacaggattaaaacccgttgactatcttccctggtatgcaaaacaatttaaggtaacagaaataaataccagcttctatcatctcccaaaacctgcaacggtagccgcctggatagagaaagtgccggcgcgtttccgcttctgcccaaagatcagcagatatatcactcacgtgaaaagattactggatccggaagaatcactgcccaggttctttgatatcttcgatcctttcatcaaacacctcggacccgtactcatccagttgccggcaacggctgcttttgatgcagaaagagctgatcatttctttaaagtgctgactgaaaactatcccgattatcatttcgcactggaagcgcgacacgaaagctggctttctgaggaagcaatgacgttattgcggcaatacaaaattgcctgggtaattgcactatccgggcgccgctggccgtttgcagaagccataacagcaaaacatatctacgtccgcttccacggacccgacggcaaatacgataaactatatcctgaaaaaacgatggatacctatgccggcaaattcaaagaatggcaacaggacaaacatacagtctgggcattctttaacaacgacgggcacggctacgctttgcaaaatgcggaacaggtgatggcactactcaaatagttcctgctcatccgtataataagttttccggccgccgccggtatccttcttaataggagcaccaccgggactctccgttaatttagcgttatgtaccagcataaaatcgcggacctcgccattaataatatcagggttacttttcaggattttcttttcggctccttcgagtatttttttaactgatttcaacaatgctttgatctttgccgccggtattttattggcaacagaaaaaggagagatctttgcatcccataaaatatcatctgcataggcgtttccaatgcccagtacattgtgctgatccagcaagtattttttgatggttattttcttctttgccagctgggcggtcaggtaactttcattgaagtctttcgacatcgcatccggtgccgttttttcttccggatcgagggtgatattggcagccgcctggaaatccgtcaaagccagcccggtgccatcggcaaacaataattctacaatagtatgcttctgctcattcttcttttcaaataaatacaatttcccgtgcagcattaaatgcatccccagcacatgcccgtttttaaatacaaaatgcaactcctttcctacccgctgtatatgttccagtacctgcccttccagggccgcctgcaggtctgcctctttggtatgtaatttcttcgcgttctttaccgtaatggacttcagttttttatgaagtagcgccttttccaggttatgccggaaggcttgcagatcaggtaactcaggcataatgaatatttttaagataagttaacgaatatggaggaaataataaagggccggcagcaataaccggcccatttttatggcagttttttccttttacgaaacaacaaactaaagataaggatcatagcagatcagcttttgctgatattgtccatcatttaaccaatattaaccacttatacataattttcatgtatgtgaacggcctgttaaaatatccgctcagcggcctcagacgcggatttcaggactttttaaacctaaaaatcggtatatttgcagtctatgccttttctctaaaccaataaaacacggagtgtgaacatgaaattgaagaaagtgattaaaccgttgatttttattattaccatttgtcttttcgtattcctatttacaaattttacaaaccttactactgccggaacatccaccgcggttattaaaccagctaccgctgtaaaaacggactcggttcaacgggaaagtttatacgacatgatgcgactggataccaccggtctttccagggaggcgtttgacaatgccctggtaggatacgagcatctgcaggaaaacggaaggatcaaaaatccggatgtgttgtctattatcgacttctccctgcccagtaccaaaaagcgtttgtttgtgatagacttgaagaataagctgttactttttaatacgctcgtttctcatggccggaactccggtaaggatattgccaatgctttttccaacaagatgaacagctttaaaagcagtcttggtttttatgttaccggcgatacctataacggcgaacatggttattctctccgtttggagggagaagaagccggcatcaacgataatgccctcagcaggggtattgtgatgcatagcgcaaattatgtgaacgataacctcggtaaattacagggttatattgggcgcagcctgggatgtcccgccatccccgaaaatgtgcaccgtaaagtgatcagcagcatcaggaatggtacctgcctgtttctttacagcccggataaatattattctgcacatacccgcattcttgtaaaagacagcaccgcgtcttaaattcatttaaacagcttttccttaaaaacggcgtcatgcccatatacatcggaggcaaaatataatttgcctccttctgtccatgccgtgaaataggtaataatcaccggcaccggatctttcaccgccacaaacttttcctttccgctgttcattgcactgtcaattttttcgttggtccattggggtgagtcctccaaaacaaactgcgccatttttaccggatctttcagtcgaatacaaccatgactatatgcccggttatcacggtcaaaaagacttttctcaggcgtatcatgaaagtaaatattataactgttcggaaacaggaacttcacgcggccaagggcattacgttgcccggggcgctgacggatcaccggcaacccgttcgcctgccctgttacttccatatctttcgaggccaggtagcccctgttgcgctgaatggctggcagaatttcctttcgcacaatgctgcggggtatattccagtaagggctgaataccacctggttcagcattcctgaaaacatagtcgtactgtgtccttcttttcccaccacaatatccatatcgaacaaacgtttatccccctccgttacatgtagcatgaaagccggtatattcaccaggatcagcttcccctgcggcttaacaggcatccatttcatgcgttccatattcagcagcagcgcctgcatccgctcttccgcagaaacgttcagtgcattgatcactgtatcattcaatacaccgttttgcgtatatccattgctgttacggaacgtattgatggcagtttccagttcatcattaaatacatcggtgctgtcattttgcttcagctccccggttatctgcaaccgtttttttacggctataatttcgggagatgattgccctttttttaatcccttcttaatcacgggcaatggttgccagccaccattttttacatattcccggtaggctttgagcggttccttcatgggggcaactgccggaaacattttatcattggttttaagcatggagtcagccagttccatcacggtgtagcgctgcgctggtatcatatgttcaagctgaccaatactgccgccggtttccctgaaataattgatgagccgccaggtaagctgcaattccgttttaatgaattctttgtctgtggcgctcaccaccaggctgtcttcatccataagggcgttcagccgcttatcaagcgcccggttgctggtactatcgttactgtaattgtacaggctccggaaggcggcggcttgttctacaggccctttactgtcgaaccaggcaaactcgaaattacgtgcattataaaagctgcgtaaccggtcagcaatggtatcgttcagtttttctgcagtgatgaatgcggctatcgccgaactgtccaggaacaggtcgttataggcattttcaggggtaatcccggcgttgcggggactaatgtgttcagcagacgtggctggcgcagacggggagttacagccattgagtatgtatgcaaacaatgtaatcagtagtagccttttcatactggtctactatcaaattagaagccggttgccagatgccatgctacagcggcaaaaggaagagcggacgtagccgtgacggaacaaactgtgcatatagcgcaacaaaaagccctcccggggataccaggagggctttctcacgaaaatatctgtgttaattttttagtcccaggtattgctgtactgacttataattcttccagtccactccactggcgctacgggcagcaacgccgccgggcaccagcacataacggaactgctggatcactttttcgccggggtaattgcccgagctgagatcatgactggccaggataacgattcctccttcggaggcgcggaaacttacaaacaggtaggggtccacgtaaggcaaaggcacgatataaggtgcatcggccgaatcaatgttgaaataaacatttatgacgcctttggatagtatctccttggtcagtttgggaatttctatggcgccaataaagccatcgccggttggcacgccattttcatcccggatactatcaaaagcaacgttgagccagtccgagtagatcacattggccacaccggtatcacctttggggccaccggggccggcaggaccggcggggccccctggaccagcaggaccaggatttccggcagggccctgggctccgtctttggagcaggcagcaaaagccagaattacagcaaataagcacatcaggggcaggtgacgggaagaaaatttcataaaggaagattttggatgatttaatataattaatgatatgtggagatgcaaggcaacgggatctttaacacgttagtcaatatacaaaaaaacaaacaacaaaaatgcgataatttagttcaggtagccctccataacttcctgcccctggctaaaacaaaatcgctctttgttggtttaaatacaatagaccctttttatcatctgaaccatttctttaataacctatagttaaaatatgaccgtgcaccgcaaactctgtgtaataatacctgtacataagtccgtgttgtccgaggaggaaacgttatcgctacacgcttgctacaggcatttaaaagcattcgactgttttcttgttttcccggaaggcttgcccgtcgaccgctttctcgcaattcatcccgggctcatcccaaaaccggtagctccgtcatggctttcttctctggcaaactataaccggatgaaattatctgttccgttttaccagcaatttgctgactacgaatttatgatgacctacgaactggatgcttatatcttcagttccaaagtacacgagcatcatggattcgatttcgattttataggagcgcctgtttttgagggatacctgaatgcaacaccggatgcaccattccatggtgcgcttaattccggtttttctatccggaatatacagtcatgtcttagcgtgctgaaattacttagaagatataggctaagatggaagttctaccattttatttatgccaactgcgccgctttacggaaaagaataaaacaggatcaggacgctatcttttttaatatccatcttaaaaaatattataccgggaaaaattttaatgaagatatgatctggacgcaggtagttccactcctggatccctcattcaaaacagctccgccggaaaccgccgctgcattcagttttgaagtaaatccagaacggctgtatgaattaaataacggcaggttaccactcggatgccatgcctggttcagatttcctttctggaaagaacatataaagaagataactgtgcactgatcagttacccttgtttaccatgcatcattttattaaatttactatacatctatttatcaggtatggccaattatcatgtgcaatcacctgtcctattattatccttcaaccgacctgatactgccttaaaaatatttgaacgggtaagagaagcccggcccgctaagttgtatatcgctgcagacggaccacgagccggtgtagaaaaagatacacagctatgccgggaaacaagaatgatttatgaccaggtagattgggactgcagcgtgcacaaactattcagtgaagaaaataaaggttgcaaggttgctgtagcggaagctgtgacctggttttttcaacaggaagaggaaggtattatcctggaagatgattgcctgcccaccaacgacttcttctacttttgcgatcagctgcttccccggtaccggcacgatacccgtatggtaaatatcaccggtaccaatttgcagatgggaaaaaagtggggaaacggcagctattatttctcacaatacagccacatctggggatgggcaagctggcggcgggcatgggaagcatacgacatcgacctggaacactataacgaaaaagacgccgttgctgtactggaaaatatctttagtgatcagttcctgatcgatggatggatcgaaatctttcaaaaattaaaaagaaaagaaatagattcctgggactaccagtttaacctgattaactttttccggaatggactatgtattacaccaaatgtaaatctgatcagcaacttagggttcaggccggatgccacccacacttataatgtcccggaagatcacgccaatttaccggcggaacaactggaaaaacctttggtgcatcctttgcattttacgccggaaaaacgcgccgattattattttttaagcaaagactttaggctcgaagagaaatggcaaaaagtaaaaaaagagcaactgctgagaagacggtttaaacggtgggtaagaagtctttttaaataaatcatcctcaaacgtccagcagtatgtttaaaaaaatgatagaaaaatctgccctgaaaaagatccacccctattacgaaatagatggatggctaaccgaacgggaagcgctggggctgttccttaccgcccgcaaattgcgtcgcgatgcagtagtggtggaaattggcagttggcagggcaaaagcacttactgcatttcaagaggactccggtcaggaaaaatctatgcgattgatccatttaatgcagacgcagggttcgaccagggaagccggaaggaatatgcagaaaaaggcgccactaccgatcttttgatccgctttacggaaaatatggaacgcctgtctgttcatgataaaatcatcgtgaagaaaggctactcatatgaaatgcacaacgattttcaaaagatcgacttcctctttatcgatggcgaccactccatcgcaggatgcagatcggattttgaattatacgcctctaaagtggtaagaggcggctacatcgctttccacgattactacccggaccgggatgaactgggacctacttatgtaatccagaacctggcaggcgaccattttaatttttccaggcaatatgactcgttatggattggaaaaaaacgatagattattcgctggtcatatgcacctttaacccggacgaacgcatcctgcaacgttgcctggaagcagtataccgcctggacactaccggcatttccaccgaagttattttagtggataataacagcgatctcccactccaccagcaatcatatgtaaaggagtttgaagaaaagatccccggcatgcacctcctcctggtacgggaacagggcgtaaattatgcacggatggcggccatagaaaaagccgctggcaactttatcgtatactttgattacgacaatgaaccggaaagggattacctccgggaactaaaaaaactaaacgaacaattccctaacgtggcagcctggggccctggtaaggtgaaggtggatttcattgacggcgtagatgctgccattatgcattttgccagcatggcctttcagcaacgggaagaacaaacggtaagaaccgcacgcgaaacttcatggcaatcctgttatccttttggtaccggtctttgcaccaccgcttccctgttaaaagaatttgtgcagctggcccgccagggacgctttactgcctcgggaagaaaagggaataaactcagcagcggagaagatacccaaatggtactacactgcatcagcaaaggatacgaggcaggcgtatcccccgccctgaaacttacgcatatcataccccgcagccgggccaacagccaataccttcaacgcttgctgtatggcacatttatctgttatgaaacctgcctgttacaggtattcccggaacaaaaaagatcgctcgaacaaaaaataatgccgcgatggaaattctcccggaaatccctgaagaaattcatcagggcccggtggagtaaagatccgcacaaaatgtttgacctcgtggaattcattgccaccaatgcgggcacctataccgcactggataaaccaataccgttgccggtaaaccagatagtaaggatactaaaagtggagtagcttaaaaataattatcaatatgaagtggaagattccggaaagtaatatgaaaggcgtttcagttattatttgctgctataacagcgcttcccggctgccgcaaacattagcgcatctgaatgaacaggtagttccggaaggtttttcctgggagattatattagttaacaacgcctcaacagataacaccgttgaatacaccagcacggtgtggaaggaaaataaaccggcgaacgccacctgccgggtagtggaggagcttacacgcgggcaaatgtatgcccggaaaagaggcgccagggaagctaattatgaatgcctcatattttgtgatgatgataacctgctggataaaaactacgtttatctttcatggcaggtgatgttgaaagataaaaagataggagctgcaggcggacaaaatgttccggtaacaaattcggcagcttatcccgactggtttgaagaatacaaagataaatatgccattggcattcccgcggaagaatcgggcgatgtaacacatcgcgggtttttgctcggcgccgggctgattacccgccgggcgctgttcctgcaggtatttgacgacaggtacccttccctcctgaacggcaggaatggggaaaaactcaccaccggcgacgatttcgaatactgcaaacgcctgctcctgtgggggtttactttatattatgataaagatctgaagctgaaacattttataccggcagaaagattaacaatagattacagggaccgcctgatggacggcatccgcgaagccacaaaagtgctgagcgtgtacgacagggcgcttttcctgcacaacaaaaacaaacataaaaacaggtggcgcttactcgcgataactcccttccggatactgctggcaagaataggtttatctaaaagggatctgacaacagaaagacaggtactcttttacctgtcgccatttgcacgcgaacaggacgaagtaaccagctcaattaaaaaattcttaaataataaatgatggcaagagaaagaagaaagcagtttaaggtattctctttttataatcataaagtaaatccccgcgtaccccggtaccaaaaagcggtgtttggtaaattcggagtaccggtacatcatattattgatgaacaattcagtcatggcgattttctgaatcatatatgcagaaccgttactgataccgactacctgattttttttgatattgattgcgtgcccacgcgtaaagagtggctatctgatcttttggaagatcttcgcgaaccccgtaccattgccggcgccgcgcaaacggctaatcacctgcgcgatgcaaaaaacctgtacgtttcgccattcttcttcggtatttccacggcttatctgaaagagctgggatacccggatatgaatatgacagaagatatggatgcagggcaaaacctgacagaagaaattatccggcagggcggccatgtaaaatactggtggcccacccatatcgaagacgagcaatggtatctgcatcatccggaacataataaattcggatacggcactacttacaacgatcgcatttatcatgcgttcctgtcgcgccacgatttatcgcaacgctttataaagaagtgtaaatcaatattaccgttatttaccaaactccgtttgaagctcacggataaaaaacaatctcctcccataggacaataaaaaaaggcgtctcctgttaaagagacgccttcaggtaaatattattatactcttcccattaccgggtcgctcacgctttctttcccggtttccaccctgccggcataacgctgtgcaaacccatcactgccggtggtctttacagagaaatcgtaccagccgtggcttttagccagatctattactaaggtggcggttgttcgtgcggctactgttttcttcagcacgcctttgttataccccaggtcgctgatggtaaaggtagccggctgcgtgccgcggtttaccagtttcaattctacgttcccggtcagcttcttactgttggtaagggtccgttgatagctgcactggatttccacctgcgggtcgccggcatcgccggtaaactcacggtaaaacccgttggggccgtatactctcaggtgataatgcgcgtcttcaaaagacgatagcggccaggtatctttcagttggtctcctgccttcacagcgtacgaccaggtgcgtaccggttccattgtttgcgtggtttcctgcaggtatttgccgggcgcatatacattgaagggagcgccggcagcccggtcgccaaataccttgctggccgcttcaaaactgatctcaaacgattgcttatccgctcccagttttccgcctacgtataattcataaggcaatgcgttggcaacacgggtacctttctcctgctgtggcatccattctgctgtggcgggattggcgttgatcttcgcaatttcctccgcagtgagcagcttaaattcatccggcagcttcttgaacttcgcattgtagatcgtttcaatgaactcgttcctttcaggaaatggcactgatattttttccccattaaaaggacggaatacggaagtaagatcactgcacaccgtacggcgccaggcagaaatgttcgtttctttaactggcttaccggttttatgctccaggaaatgctccattaactgcaggatggaagtatggtcgcatacctgtgaatttacatagccaccacggctccagggcgatgcaattaccaatggtacgcggtatcccagcccgatagggctttccctgatttcatctgcgctgagatatttctttgcttcttcttccgcacgtgttacatattcaataccggtatcaattcctgcagacactttgccggtaccgggtttatgcggtgcggtaaacggaggtacgtggtcgaaatagccatcattctcatcataacataaaatgaagatggtctttttccatacctcttcctggcgggtaaggatatccagtacctcagatacgtaccaggcgccataccatggcgatccagggtgatcggagaattcgcccggtgccaccagccaggaaatagttggcagcttgccctcatttacatctgttctgaactggtggaggatatctccttttggcacctgcacagttctttccgtgtctccgtctttgtaggtgagagtttccagctcatggtaatcaggatcaccaatattggtggtaaatgcttttttatgaagattttgcgcgcgctgcggcaattttgcaaaattagccgctgtaaacttttctgcatcagactttgctctttccagttccgctttacgctgatccagttgcttttgcagcttggtggcttcctccccggaagtgccagccagtttggatgccagtgtttttatttcagcgggcagttctttgattttgcgttgcaggtactggatatgccccgctgcgaaacgaacattataggcagcgaaccactctataggattatcggtaaagttggccagcatgccgtccttttccccttccaggcccgcggcgctgatttcattctggtaaattttccaggaaacgccgttgtcttccaggcgttcggggaagctggtccaatgcgcttcccggccatagtccacatcttcgttccatacgttagctttggaatcagccttctgctcatcgcgcagggtacccgtccacaaataaagcctgttgggcgtggtaccggttaatgaggagcagaaattctggtcacatacggtaaacgcatctgccagggaataataaaacgggatatcttcccggttataataacccagtgtgaggggcatcggggcccagtctttattgcctgatttttttaccagcagccacttatcgtatttgccgttgttacgggcatctacctggttaccccatgaatgcggcaggctgctcatccacgtagcctttgtttccttcaggttaagccggaaaggggcatacgtttcattgttggcattgctctgcaaccacaccaggtttttattgggcagctggatagcacgtggatcattgtagccccgtactccgcggagcgttccataacagtggtcaaaggagcggttctcctgcatcagcactacaatgtgttctgcatccaggaacgtggtacccggcttgggatcaatggccattgcccgctggatagacgccggcagggcactgaaaacgccggcagctccggatagcaacgccgccttcttaataaaatctcttctgttatccattattcgttgaatttttcatgtacactgtaaagggattacgaaagatggaaaatagtaaaaatcctgtgctatacgcaacttactatgaagaatggctgttattttattattatggttccggtttaacggaaataaaaaaggcgcccgtttccacggaagcctttatatatgttgagaaatggtaaagccggtttactgcgcagaaggtatcaatacaattttcactctcactttggtagccggtttttgtgagttaacaccgtttacacctttgatatctacttctactgcctgatcatcgtgaataatgaaataagactgattgttatacacctgcggcaataattcaaatgactgtggtaccactgttgggttgctggcatcatatctggccatagaaacgatcacaccatccaactggtttacattatttaattccgatacaggaatggagtaaaagtaaacgccggtagcagcatcaaatccccagtcgttcgggtttatttcaaacaaaatcgtttggttagggatgactacttcattggttgtttttgtgcaaccgggcaatataaaacccagtaacagcagcggcaggtaaaaccatgttttcatattgagttgcttttaatttattttaccaaatacaatgccataaacatataattccgcgctaatccgtatttttatggtatgttactgcgatacccaaaggcctttgaacatataccggccgtccggcaacaacatgccgggaagtcactggtggcgtggttcaggcaatctaatgaacccggtgaagaacaggggtttcttacagaaaactccctcgtgttcattctacggggcaccaagcatatgcacttcccggaaggtgatattattgcacatgccggcgatctggtgctgctgaaaagaggcgtgtatctgatgaccgattttattacggatggcaccgattaccagtcgcttttactgtgcgtagatgataccttgctccgttcctttatcagtgaagatggcatatccgctcctaccacacaagcgggatccccggtagtcatctcctgtaaaaataacctgctgcaggtgcggaacagcatcctggattacctggagcatcccaacacccataccacccggttgctggaactgaaaatacaggaagtactgctgctgttgctttgcggcgaacaccggcaatctgtccgggcattcctttcccatcttttcgacaacagtgcggaaaatatttccctgatcatccgcaataacctttttcaaccttttaccctggaagaatatgcgaaaatgtgcgggctaagtcttagcagctttaaaagggaatttgcccgcctgtacgatgctcctccaaaaaaatggatcaatgaagaacggctgaaacatgcccgtgaactcctcctgcattcccgcaacaatgtcaatgaaatcgcctacgagtgcggctttgaaaatgtatcttactttataaaacaataccggcagctatacggcactacacccaaaaatgcacaacgggctaaaaatgctattttctgaacgattcctgctactgctccatctccgtcggatatacctttgataaaaatattatcaactatgaaacgtatatccgtattggctttcatcctgatggccggtcatacttttgcacaacaaaaactcaatagttccgcatttatgcacgcgccggaaagcgtagcaacagacaacgacaattattatattgcagacattggcgaaggcggcaaccccaccaaaaaagatggtaacgggatcattttccgtatggacaaaaaaggcaacggcaccgtcttcgcaaaaggactggatgcacctaaaggcgcttttatcctgcatcacacgctctttgtagcagatatcgataaagtaaagggatacgacctgagcaccggtaaacagttatacaatatcagcttagcacccgccaccgctttcgtgaatgatatcaccgccatcaacgacactaccctggtggtttctgcaactgatgtaaataaactcttcctggtgtatcccggtaaaaatccgcgcgttgaggaactggtatacaccacgcccataaaaggtaccaatggtgtgacatatgacgcccgcagtaaaaagctgtatgtgtgcggctttggcggcaataataaaccagatggacaaattggttatatagatatgacagcaacggagaaagtattcaaacccctcaccagccggccgggttattatgatggcattgcacttacaacacataatacacagctgatcgtatccgactgggtagcttttgagaagaaaggaatactgctaaaactggacctggccagtggccgtatcaccacgctgaatgaggaactgattgccggcccggctgattttacactggatgccaccggtgcggcgattgtacctgctatgctggagggaaacgtgttacggtacaatatctcaaaataaaaatatttcagtggaggaagtgcgcttcctccactgaaaataatgcttacaatcttacctgtacaccggcggttccgccaatatatccaccatgaaatttgtcgttgttcctatgctcggaccatacataatggttgctcaactccgctcccacaccatgttccgtttgcacgaaattaagcgtaggcccggcaaatacttctaccctgctgccgaatcggtaggcgggaaatatgcccagtgtttgacggtgataatatccttttttgaaatcggaaagcaccagcgtggtggcttctgcattgatcctgaaatgtgacaacaatggaagatgcgcaccaatacccgcctgcagggcgtacagcggattgggattatctttaaagttatatcccactccgagaataccgtacaatattcttccgcctgatttgaaagaggcaatggtggtggcagtttcatcgatgcttacacttacctgcttttccccgcctttcacgatgttgatcacaccaatcgggcattcgctgctatccgcgatgttaataaaacctatctgcacgcctttcacctttttggcaatattcaggaaaccagttatctgtgtatgcacattctctgctttattcataaagccggctatctgtacgttggcatctttctttacaatatttgcaaatcctgctacctgcgcctgtgaattattagcgcccatattcataaaacctgctatctgcgtaccttttacatcctggcgcacgaggttggcgaaacctgccatctggaaaccttgcaaactgccggacaggttcaggaaacttgccaccataacgccgttggcgctggttttcacctggttcataaaacctgctaccgtaactgcgtgaaacgttttaccaatgtgattggaaaacccggctacctgtacaccggtagcgctgtctttgatgatattggaaatacccgcgattgccgcgcctgtttcagctttggacacgccggcaataatatgtaatgaaaaatgattggtataggctgctgcattttttccattgctgctcaacgggtatacaaaaccaatatgcgcaggactggtaagcggcgtttgcgcgtaagccgctgtgacaaagaataaaacggaaacaaaaaaacaaatgatccggctgctgaagtaaaatgttctcatggtgtgttagttatttcgtactgtataacgacacgttgaagaacttatacccctatgcggaaaatgaaatttaaaaaagactgataccagcctgccatcccagccaggaagtaactgagttgcctatattaaaagagggatagtgcgcaccaaaatcgaccgacttataaccgggcatgggtcttattttatcgtcaaaatagatcgccatcgcgggccccgcaaataagctgatgcgtttggatagtttcacctggagagaaggctgtaaacggaaaatctgcgtattacgctcccagctgcccaggaaaatattctgcgcggtaatttctgtggataacgacaacgttttattgaacgggataattttaccgataccatatcccagcgaccatgccttattgttttcgccaaaatccccgccacccagcaggatgctgtatagctcactgcgaccggctttccaggcgatattaaaaggcagcacatctgtactgaataacaccacttttttgtaccctttacgcacaatattgatgatgccgatactataccccgttaccgtatctgcaatatttaccagcccaatctgcacaccatccatttgccgcgcatagttaaaaatagcggcaatctgcacgcctttcatcaccccacggttaatattgccgccacctgtaatctgcgcaccataaacgtctttcgcgttataattggccaggccgctcagttgcagcccgtcgagatttttaccgttataagtaattccaccggctacctgccagcctcgtgtattacctcgtatcacacccgcgatcccttgtatagatgctccgttcatatttccgtatacctggccaataccgccggtgatttgcacaccttccatgttaccttccgtgatattgctgataccagccacctgtacgcccttcatggagtccagtacattattgtgaaagcctgccagttgcacgcctttggtttttcctccaactacattcaccatgccggcgatttgcacatgctgcatatcgtttttcacaatattgaaaacagtacctatttccacgccatctaccccggcagcatagccaccaagcatgttcatggaaaacttattcactacctgtccgctcattttgccatgggtccccaaacccggcgtgagagatacctggtaaggcttgtcagccaggaagccaccaatattcaagctggtcagcttctgacgggaagataaaaacatgttaccgaaccaggttttttccacgtgcgagtgcccggttatatccaccactttcagctgataagtagcaggagcaatacttacagtaatttcctggtcgtagccagtagtaagcaaaagagaagtatctgcatagaggtccttactaacactaatggctgcggtaggatatttatcctttaaccgcagcctgaagaaaccgtcgttgtttgttagcgtagaaatgagttgctgtcgttcatacacactcgcattgggtagccgttgtcctgttttccggtccgtgacgaccccgctgatcaggtagtatacttgtcccgatgattttttcagcaggatgatatagttccccgattctttatataaataatcaccgttgaataaaatatcgagtacctgttttaccgttttatttttttcggagatgcttaccaggctatcctgtgggaggatggtactgagatacgagaaataaaagttgccctgcttgctgatggtggtaagcacttccgaaagtggccgctgctttgcatcgatgctaaccgttttgttcagtagctgctgggccgccagtggaagtgaaaaacaacaaacaaataataatgtcagcaattgcttaggtagtaacatacagtacgaaggctattatttcagtgtgatttgtgatccctgtttctccacggtgatctcgtaagtaagcccgattacttttaaagtgctatccagcgaactgttggtaaaggtagagttaatctgcagattgcgtttatcgttatttgcaataacaatgtttacgccgtatgcttcattcagaatctccaccagtttccataaaggagtgttattgcatacaaatgtttgggtgcggtagtagttatacaattcatctgtattactttgtttgctgggagcggtctcctggtctgttaccaccgctttttcatgttgttttaactgtacactgttattgttttttgttacttccacggcgccgctttccacaattacttctgttttaccgtgtatacttttaacattgaaagaagtacctaataccgtcactgttacatcattcacctttatcacgaatggttttccggggtcctgtgccacgttaaaaaaagcttcgccttccagttttaccgagcgttgtttcctgttgccggcataggtaatagtagattgtttattcagtgttacctgggagccatccggcaaaacgtcctgtttgatttgttccccggagctcacgatcagcggggtattccggttctgcgagataaaccaggcgccggcagcgcctatcatgacgatgaatatggcggcaatgcggagtataggtcgccaggcaatgccggtatccagttttacgatgcgggtggtattgtcgttggtacctactcgttgctggaagcgtgaccatgcatcactttcattcaccgtgcttaccgctgccagtttacggctctcctcccatatcaggcggaagtgttcaaaatagcgctggtgctccgtatcctctgccagccatgcgtttacggctgctttttcggatggtgtggtaatgtccagcaggtgttttaccagcaggtcgtcgtttatatgtgtagatgtctttttcacggatgcacttttacaggtggagcaaaattaataacaagggcagaaaatctaccaggttgagtcgtaataagcgcaacgctttgcccatctgattttccacagtttttatagagatatccaggcgatctgctatttcctggtatttcagttcttcgaagcggctgagctgaaaaacggtgcgacatttttcaggtagtgccatcaaagctgcgtccagcttctcttccagctcccgcagcattactttgccggatgcgttaccggtatcatggtcattgctcatctggtatttggtatgtgcctggtgggtagccttcactttctggtgccgcagataattaatgcactcgtgatacactgcccggtataggtaccccgaaacagattgctttatttttatatcacctgatttttcccacagcttacaaaagacattctgtaccatctcttccgccatcacttcgtcttttaataaggtacatgcataagcatgcaagcctttaaaatgagttttaaaaacctgttcaaatgttaatgagttttctattaccggtgctgcagtgttacccggatttataaattccatgcctagggtttgatatctaacgtcaaatataattccttctgccaattgaactgatttattatacgacacctttccaagcacttacccctacgcggagtttgtctttctcaggatttaactgattatgcggattaccttgattttattttttgattttataatgattatacaatatataaactaatgttttataacatgttattaagtaatctgaaaatcatgcaaaaacaaaatcaaggtaatccgcataatcagttaaatcctgagcaagacaaccttcgcacgtcactttaacattactttatattcgtgttaaagaatatttcacaactggacgattattattgtggaaattatcccgatgaaatttatctgtacactttgtctcttactgttaggaagtactgttctgtttgcccagtccaaaacgggctacatcaattttcaacaaatgattggtatgatgcctgaaagtaagctggcaggagattcattaaatatcttacaggaaaagctgaatgccgacgggcagcagctggtggccgagtacacgaagaaggtgactgattttgacagtacccagcatacgttaagtctggctatgaaggaagtgaaggtatctgaaatcaaagcgctgcaggctaatatccagaaatataaagagatgtctgaacaggccatgaataccagggagcagcaattactgacacctattcttgataaagcaaaaaagattttaaaggcggtagctaacgaaaagggctatacgctggtgattgataactccagagacgcggtgttggtatccgcagaagccgatgacctgatgtcagcagtcaaggtgaagatgggaatcaggtagaagggcatttgaatatttagttatttagttatttgactggtctcaatgcctgatgaatcttccgccattctgatactgataatgtggatggcccgcaaataattaaataactaaatgtcaaatgtaaaataaagagctatatgtgtaagccatgtgccagcagcgttttccactgaggattgctgcgtacgaattcagccacttttttgctggaaggcaccatacggatattctgtgcagaaatttcctccataacttttcccagcatcattggcaatacaccctgcttttccaataccggaggcacttctgcacccgtcaggaaaatacggcttccgtttctttcgtaaataactttagccatctgtccggcgatatgcgcctcaaactgcctggcctctttgttgtcaataattttaaaatccttcatgatcataattattttttacatgatgtttctagcggtagcatactaaagggaagtatcttatgcaaagggaagttgaaataagatagtacgaatggtattaaaataccctgaaaaagctgattccgtctgcaaatatactaataatatagcagaaaaccgtgaaacaataatatgtaaaaataattaatacctaaagtagttggcaggtaagcctttaacaggtagccttacgtgaaacacactgccactaaggggaaattcagccatctgtccggccgtcatgtgctcccgggcggttgtaatcaataattcgttcatattcggaccgccaaaagcacaggacgacacattcggcgccggcacccccacttttcccagcaactcaccggtttcaggattccagcaatatacaccgtaaccgccccaatgggctatccacaacatcccttcactgtctgttgccatgccatccggccagcccatttccggcggaatatgcaaggccactcttgtaaaggcaatcgcaccagtggaaacatcataactaaattcctgtaccgtacgggtatgcgtatcgttgtaatacattttatttccttgccacaccaacccattggaaatggttacaccgcccagttttaatacaggcgctgctgatccgctgatgcaatacaggttacccgttccttcttctgccggcatctgcatggtgccaatccacagcctgcccgcagggtcacatttaccatcattacagcgcacctggctgcgttcctccagcacagcgatacgtttacccaatccctgctccggagaaaaaaaggcaatgccatctttcaaacccaccaccagctcattcctgccggcaaccggcaccagcgtggttacatagtcgccaacataaaactgctgctggtagccgtttacgtcctgtatataaattgtaaacccaaggatatccacccagcaccagctattcctttccggccaccagcaagcgccttcgcctagttcacaagttaatgcagataatatggaggcctggaatgttttcatgttcgcgctgttgatttaaataaaagcagtattgctattcatttccatataccacaatatatagttttgtgcgctgatattgtatattgcaggagttaacgagtgttaattccaactaccttaactccatctatgaacattaaagtatttgaaaaactccgcgcagcagaactgataaatgatgcggagcttacagcagttaaaactgcggaagatcagcagctattctccctccactgggaaatcaaaacactactgtacctgggcgtactgctgttgagcggtggcctgggcatcctgatctataaaaatatcgacactattggtcaccaggtaatattgatgatcattggtgtaatctgcgccggttgctttagttactgcatccggaaaaaagcgcctttttcatggagtaaagtaaattcgcccaatgcttttttcgattatgcgttactgttaggttgcctcacgtttgtcacctttgtgggttatctccagtttcaatacaccgcatttggtactgcctatggactggccacttttataccactggccgtgctcaccgtgagcgcctattatttcgatcacctgggagtgctgtcgatggcgatcaccaacctcgccgcctggatgggcattgcagtaacgcccttccagctattatccgccaacgactttggcagtgtacagcttatttatacgggcgtgatactgggcggactcctgttagggctggcattcctgtctgcctggaaaaatctgaaaaaacactttgcatttacctaccagaacttcggggcgcacatcattttcattgcctgtattgccggcatgtgcgtgtttgacgccagctggctcgcctggcttgcattcatggcagttattggtttctttctttttaaagaagcattcaaagagcggtcgttctactttgtgctgatcaccgttttatatggctatatcgcagtgagtattgccgtggtgcgtttacttatattaacaaacgatatcggcggcctgtatctcgggttattgtacttcattggttctgccatcggggtcattgtattattgatcagcctcaacaaaaaaattaaacatgctagcgtataattcccaaacactcgacaaccttgaaataaaagaagcagcagaaaaagcgcttcggaaaaactgtatcaccgtgcctgcttatcaggctattgaagcggcacacccggtaaatttttatacacccaatcctgtgattaaaatcggtttgtttattcttacggtggtgatcatttctttttcgcttggcttgttatcgctgatggcaatggatatgctgcgtaacgaagacgggtttgccggtctttgtattttcgccggattggtatgttacggtatcctggaaatgtttatccgtgagaagaagttattccgcgcgggagttgatgatgccctgttatggggcgctgtaatgcttatttgcagcagcatggttatcgtagaccggatctctgcttctactatctgtttcgtggttggctttgttaccgtgctggctgtcttacgctttgcagatatgctgatggcaggtgtggcttatttggcttttttaggatttatattcaccgtggcgatcaaactggggcctgttgccaaaaccattgtgccgttccttatcatgttcgtctctataacagcgtacgtggcggcgaagaaaatatccgcctatcatagcagcaggcattataaacattgcctgacggtggtatccgtattatctttactcacgctgtacctggcgggcaactatttcgtggtaagggagctgagtaatgcgatgtttgatctgcagctgcaggacggagaaagtattccgggtgctatcttcttctggatttataccgctgttatcccggtagtatatctttacctgggcatccgtaaaaaagatgccgtgctgctgcgcacgggtatgatattgctggcggctattgtatttaccatccgttattatcatagcgtgcttccgctggaaactgcgatggtgctcggcggccttgtactcacggtaggcgcctgggcgctgatccgttacctgaaagagccgaagcatggcttcacctatgcagaaccggaagatccttccctggcagataaactaagactggagtcgctgatcattgcgcaaacttatgcacctggtgcgcaacctgctggtaatgatgtacagtttggcggtggtaccggtggtggtggcggagcaagcggaggatattaaaagtggaacagtctttcgcctccgggcataaaaaaagcctgactgaaatgatcagtcaggctttagagcgaaagaccgggctcgaaccggccaccccgaccttggcaaggtcgtgctctaccaaatgagctactttcgcagatgtattaagaactttataaaaactggagcgaaagaccgggctcgaaccggccaccccgaccttggcaaggtcgtgctctaccaaatgagctactttcgcaggtattaaaaactttgttattttaagaactctcccattgaactgcattctttcgtttgcttgccccgtggcgttttcgttgggattgcaaagataggaaacggactgaaaacacaaaattttttttgaaactttctcgaatatttttcacgccgctgtatacggcaacttgctggaacacaacagggaaaagcatttcagcagaaagataagtaatactttttatttacattgtgcttggtactgcagatgcacggatcactacaggcttctttttcgacttcttccgcttaccccaccatacataaaaacccgttaccggtaacgatgcacagatcaggctgataatgaacgccaggatctttccgggcagccctgcaatagcgcctacatggatatcgtagttcatatctattaaccgctctccggcatttttatgcgagtcgttccttcttccaagcaatgcaccgctgtattggtcgaaggtaaggttatcggagccgtaataagtttcgtctcttttatttccgctgatgatgttcaccccggtttcaccggctgccgggtaaatgaacaggcgctttgcatctttcagtatgggcagagccttgctgtaagcgatatccagcggatcctggctcagttgtgcagttgttttggcagattgatattcttttatatcaggcggggtagtgctgcgggaagccactacatatacggttgtctggaaccacgtaaacgcccataccatgccggtaaaagctatcaccaatgcaataatcatggcataaaaacccagtacattatgcaggtcgtagttcactcttttgaagcctgctttccattttattttaaaactcttatcacggttggctttgttccacttctttggccaccacatgatcaacccggtaatcatcagcactacaaaaataagggtgctccagcctacaatggtttgtccgtacttatcgttcagcaacaggctccagtggatcccttttataatggaaaagaaattgtacttatagtcgattttcccggtcacctttcccgtataagggttcaccaacaccgattcatagtgctccaatgtgccaaaataggtcaaggcagtatcgttgcccttataggacataaactcccaggccatatccggcctggtgtaggtggtgatcgtcattgccggtttatcggaccccagaacggcctgggccgtctttttcagctcgcttaccgggcggaagggtgtattttgcggggttacatataatattttacgataataataatcgtttatttctttctgaaaaacaaacaaacagccggtgatgctcacaataagcacaataatgcctgctcccagccccagccagagatgcaacttatccacaactaccctgaacagcgacttgtgctgcttcttctttaacttgtccgtccgtttaaacatactaacaccctccggtagatatcattccggagatacaaaagtcgattcaaatggtcagaaaaacggatcggatcgggaattttatttacgcaaaacggaaaggcataaaaaagcctccaccggaaaaccggtggaggctggataattatgttgaagccgcagcttacttatatttcggattgtacagcgaactttcctgcacctttacttcaggcttgcccttgtatctgtgtgcgtaaagcccgtagctaactcccacgataaaggctaccatacaaaacaattgtacgtagaaaagccagcgggaacgggaaaccttgtctatagtgatatcgtacttattttctattgtattctgttccataatcagtttatttccggtgcaaacctacataatattttgaaattttcgaattttcataccgggttattttgtaagataagcaacttttcccggagcctgccgctgcctaaatcaattcagaaaaatgtttgtgtcccagaaaataatagcgccagatcataataccatgaaacacgccactcattttcatcagcttcatttccggcaggttatctttcttcacatagttcctgcgccagcgataataatccctataggcccggtaaatagccgccatatcctttggctttcccgctaccaggcttttaacgcctgccagtatatccaggaaaaaacgttgtaccagtactatccagcggtcttcgctatgcaggtttttccacagcatcatgaggttgttcctgaagttcaggtacagcttgcggggattgccctggggcaggctccctcctcctacgtgaaacaccctggaatcggggcagtaacaaatgcggtaccccgctctttgcagccgccagcaaaggtctacttcttccatatgtgcaaaaaaatcgcggtcgaagcctcctacctggtgataacaggccgaacggataaacaatgccgcccccgttgcccagaaaatatccttcacatcatcatactgcccgttgtctttctccgtagtgtacaggatgcgtccccggcaaaacgtatagcccaggatatccatccagccaccggctgctcctgcgtattcaaattcatcgggatctttgtaagcccgcattttaggctgacaggcagcaatcttcgtatcctgctgcatcagtgccactaccggctctatccagcccggttctacctccacatcctggttgagcagcacataaatatcggcctgcacatgctgcaaagcatcattgtacccgccggcaaacccatcattccggggattctgaataatccggatctgcgggtaatgttccgccacaaaagccacgctgtcgtccgtagaggcattatcggccagcaccagctgcaggttgccgtaggtagaacggcaaactgatggcaggaacttttccagaaaagatctcccattccaatttaaaataacaactgctactgatggcaatacggacaacggcaattacgtttatgcgtgaacaattatttttgagatgcaaatatgcaacaaaggattctaatatttgcgaatcattacagattcaggtaagtcgaataaggcttaaattagaagtatgtttaaacagtatatcggttggaagtttgtactggcctccatagcagtgcttatcataggcactactatctggtttgtaagtaatttatcccggaacattcaggaagaagaaagaaaaaaagttgctacctgggtggaagccaaccgcgaactcctgcgggcaagttccgaagccaaccttaacctggcagtagacatcgttaccaacaacactaccatcccgctgatattgaccgatgaaaccggtaagatcctggacagccgtaacctcgactccatgcggatcatgcaggaccccaacttcctgagcaacgaactgcaggcgtttaaaaagcaacacccgccgtttatcatggaagtagattccaaacagaaactgtataactacatctactacggcgattcgctgatactccggcagatccgctattacccgtacattcagctgattgtggtaacccttttcattgccattgtgctctttgccctgtccagtaccaaccgcgccacccaaaaccaggtgtgggtaggactggccaaggaaacggcccatcagctgggtacccccctttcctctatggaagcctggctggaaatcctgcgcgacaatgaagccaatgccactatcgtaacagaactttccaaagatgtggaccggctgaaactcatcaccgaccgtttctctaaaataggcagcgtaccgaaactggaagagaaagacattgtggcgcagatagaaaacatgaccaattacatccgcaaacgggcgccccagaaggtgatactcaccgttcacagcgcagaagatgagctgcccgctatgttttcacccccgcttttcgactgggtggtggaaaatttattaaaaaatgcgctcgatgcaatggaaggaaaaggaaagatagatatcaccatagaaaaccaccctacttttatcaccatcgatgtggccgatacaggtaaaggcattcctaaactgagcttcgagaaagtgtttaaacccggattcagcaccaaaaaacggggatggggcctgggactgtcgctggccaaacggatcattgaagaatatcaccgcggccggctgtatgtgaagtcgtccgaaataaataaaggcaccactttccggatcttattgcggaaataatgagccttttcagtaaaatatgaataaataaatttgcttattttaaaaaagccattatttttgcaccccattctaccagatgcgaaggtggcgaaattggtagacgcgctactttgaggtggtagtgcctgaaagggcttgggagttcgaatctcctccttcgcacacgaaagggtaatgttttaaagcattacccttttttatttttgttgcctgaaacctaagcccacaccggaacatcgtattttcttgaaagctctgctccttactcacttcatggcaattccaatagattttaactaaaatactttatggtagagcatttgcattttgaaaaccggatattattccggcgatgtgtttttcaccgtatccccggaaatatacagttcactccctgatgtctttgattgagccccccttgatgatcaaacccagtattttttctcctgttgagacagggaacaggagcgggcgtaattaaaacaatcaggatacttcccactttttttttattccgcatgggtatcatctcccgttcagtatacttctattattatgaacttaccgattcacgttatagaaaaatacctgcgtggggaagccaacgaggaggaaacccggctggtaaacgattggttctattcggcagacgcagcagaggctcccgcagatgaagcactggcagcattaagaatgcagataggaaaaaggatacatgaccgcctggataaaagtatagacctcactataaggcaacggaagaaacagcgcgcaggagtgcttaaaatcgcagcagcagcggctgttatactgggcatcggaacatacttcctggtccagaggggggtgttctccaacaaaccgctgcttgccgctaaaacaacagtaaaaaagggagatgccggaaataacaaagcaacgctgatcctggcaaacgggaggcaaattgagctggatagtactgcagatggacctatcgacaacaaaagcggaatacagatcattaaatccgaagatgggaaggtagcctatgtgccaacacgtgaacacgtgcagttgtcatcggtggcttataacactattattacccctaaaagcggacaatactgtgttaccttgtccgatggaacaaaagcctggcttaatgcggcgtcgtcactcaggtacccggtagcatttaatgcagacagcagggaagtggaattgtcgggagaaggatattttgaagtagccaccgtgctttcagaagagggcaggaaaattccgtttattgtatccgttcgtaacaccgggctgcccaaggccatgaagataaaagtgctcggcacaaagtttaacgtgatggcttacgatgatgaagcatccattgaaacaacattactggagggaaaagtggaaaccgcttattccacaggtactgcctcactattgccgggtttacagtcgacactggaaaaaaccaacctgaaatttaaagtttctaaagccgatatagagcgggcggttgcctggaaaaacggggaattccggtttacccggatggatattaaaggcatcatgcggcaaattgcacgctggtatgatgtttcaatagagtacaggggcaatatggataatattaacctgtccggcgttttttccaggaaaagtgacgtaaaacagatgctggatattttggaggctactggtacagtgcattatcaactggaaggaaataaagttattgtatcaaccaaataagaatctaatgccaatgaatagtacataaaattccgcgtacatgcagatccaaaaataaatccggaagtgcggtcacacttccggacgataacatttgggtccaaacagcctgtaacaatatcgctttacaaccatttatcacccaaacattataaagataatgaatcttatttccatttggggcagatttaaacgtctgcggcccttccatgcctcgttctttctagccatgaagttaattgcttgttttattcttgttgccactttccaggtgaacgccaccactatggcccaaacagtaacgataaagggcgcgaacatgtcgctgccggccatctttgaaaagatcaaaacacaaaccggttatgcttttgtataccaggacgacctgcttaaaaaagcggtaccagttactattaacgaggtgaataaaccgctggaagaaatactggtgcagatcttcaaaagccagccatttagttatgagttaaaatacaaaacaattgtgatcaggggaaagcctgctcttcaggctgtacccaggcagggccggtatattgaagcaacgggaaccgcttataataacatcggggaaccgctggtgggggctactgtagtgatcaaaggaacacaaacctccaccatcaccaacaatgccggcaagtttactataaaggtgcccgatacgggggccacgttggtgatcagctatgccacttacatttcccaggagatcaatgtgctcagtactacccgttttcctattgatgtggtactgcaattgaatgcaaaaagtattgaagaagtggtagtagtaggatacggtacgcaaaaacggaaataccttaccggctctattgcttctattggacccagggagctaaggcaaagccccgtagccaatattagcaacgcgctggccggcaggttacctggcctcatcacggtgcaaaacagcggagagcctggagctgacggatccaacctcttcatcaggggattaagtaccaccggtaacaatagccccattatcctggtcgacggtattcagcgctccttcagtgatatcgatccaaacgaagtgtcagacatcagtatcctgaaagatgcaggttctactgccatttatggtatcaacggcgccaacggcgtaatactggttactaccaaaagaggtactacttccaagccacgtataaatgtgacgctgcaaaacggatggcaaagccctaccaggttaccggagtatgccgactcttacgacgggcttaccatgtaccgcgaagggctaatcaatgacgggctgccggtggccatacagtacacggattccgtattgcaatactaccgcaacaggagcaagcccgcttaccagtatatctaccccaatgtaaattggatggatgccatgctgaagccctactccctcatgcaacagggaaatatcaacgttacaggaggtaatgaatttgccaaatactttgtatccatggggtatttaagacaaaacgggttataccggtatgaagaccagatcgaaggatacaacatgcaggccattaccaacaagtataatttccgctccaatattgatctgcagatctcgaaagatctcagcatggaactgggattgggcgctattgtgcgcgacaggaactacccgggcgccaatgcaagcgatatttttaacgccattaaatcagcgcctgcctggtggtacccggttaccaacccggatggcagccccgctgcatttaataccgtgccggcctctccatatgtgcagttaacccaatcgggctaccaacggaactttgaaacgaatcttcagtcgaccgcaggctttaaatgggatatgcattatttcctgaaaggactcagctcaagagtaagactctcattcgacaacaccagctatcgtaacgtgaaacggggcctttccaggcgcactttcctctacaagttactgccaggcgtagtagccgatacggtgaccgacctcgcaaaaagcggcacctaccaggtgattgaaaacggggatggcaccctgggctatgacgtaaatgccaacggcaccaggcgcaccacgttggaaacatacctgaactatgataatactttcggcaggcataccatacaggccatggtgctttatacccaatcttccttttttgacggcgttggcggcggagtgagtaatgctattcccgggcttccgtataaaaaccagggcgttgtaggaagggtgatgtataactatgatgaccgctacacagtgcaattttccggcgcttacaatggtgcggaaaactttccgtccggtaaacgcttcgggtttttccctgctgtttctgcaggctgggatatagccaaagaatcatttgtccgctccgctccggggttatcatttgtagaccaggtaaagataagaggctcttacgggatcaccggaacttatgctttaccatccggaaggttctcttacctaagccagtggaaccctgatgatgcaggctaccagtttggcgtaaaccgtgatggtaccggttatggcggtgcttatgagcaacggattcccaaccccaaccttacctgggaaaagggttataaaaccgatgtaggactggatgtgggattatggaaaggaggattgaatatgaccgtagaatatttcagggagaaacgtaaagacattcttattaactccgaactggtgccggccaccgtgggacttctgaatcaacccgctttgaatgccgccattgtgaataaacagggaatcgacctgtctgttgagcaccggcacgaattcaggaaacagggctatgccgttcgtgttaactattcgtacgcaacaaacaggatagcctattatgcgcaaccggactataaaggcagggaatggcaggccagggctggcagcgaagtgggatccatatatggatataccgccatcggtttctttaagaataatgatgatatagcgaaaagcccttcacaatccgtgtttggaaccgtgcagcccggcgatatcaagtacaaggatattaatggagatggtattattaactctctcgatgccggtttcctgccgggtaaacgtaatcagcccacttctattttaggcgtaagcttttcttaccactacgccggttttgatgtaagtgtattattccagggtggttatggcggctccctgctggtgaacgggtctggtatctttcctttctcaagatttgcaggtgtgctggaagatgtgaaagacaaccactgggtagcctccaatcctgacggcgattataaatatccacgcctctcttcgcaggacaataccaacaaccagcaaaattccacgttctggatttactccagcaattacctgcgcttaaaaacagtagagataggctataatattccccgttactggcttaataaaataggattcagtaatgcgaggatttttgtaaatggtattaatctcattacctgggataaattgaaaatttttgatccggagatagccagcgacggtaccggcacttatccgcaacagcgggtcatcaatacaggattgaccttctcattttagtaaatcaatgcgatcaggcacctgttatctgaataattaaaatcaacaacaaatgacacgtaaaatattattccacggactcctgcttctctgggtaacagctatatcctgtaagaagtatctggatgttgttcccaaggaaattgttacagaaaaagatatttacgataatataaatacggcggaacgggcctgggccaatatgtacacgtcgttaaatacaagtaccacgaacatctactataatacagtgttgggcgcctgtacggatgaatgcaaaaatcactgggaaaatgtgccggagttgaaatttaacgctggcgcctgggggcctacggataattcgctggataattggggatggtcttaccagtttataagaagagccaatattttcctgaaaaatatagataacaccccgattccacaagaccgggcagattactacagcatccgcataccccagtataaggcagaggtacgttttctcagggccaaattatattttgagctgctcagatcctatggtgcagtgccgctgctgggagacgatgttacggatgtaagcgaaggtattcctgatgtactgaataccaggaagccggtagatgaggtggtaaactatatagtaacagaactggaccagttagcgccggtgttgcccatcgattataccgataacccaggggaaaccgggcgcataacccgtggcgccgcgatgtcattaaaagctattacgctcgcatatgctgccagccccttgtttaacgggaataccatgtacgccggcataaaaaatacagacggcgcacaactctttccacaaacttatgacaaggaaaaatggaaaaaggcagccgatgcagcaaaggcagtattggatatgaatgtatatgcgttgaacaatcccaatccatcgaacccgatagataactatgcacgcctgttctactcccgtgagtataaggaaaccattttaccctatttgataggctccaccagggatttggaccagacgatgcagccgaatgggcaggatgcacaatcggccggcggaaatggtaaattcagcgtattccaggaaatggtagatgcctacgaaatgaacaacgggctgccaattaccgacgtccattcgggttatactaaagatggtttctgggatggccctctctgggacgggaaagcataccggcaggcaaaaaatatttccaacatgtacaaaaacagggacccgcgtttctatgccagcatcaattttcaatatgccttctgggattccgccaaccacaggcgcccgttaaaatatgcctactttggcaacaatggcggggcttctgatggatggccaaaatcaggcaccaattgcgagagcgggtataactggagaaaatggtgtgaccctggtgtaaacctgaggggagggggaaatggcaacaggaatttcccggtgatacgactggccgaaatttatcttatttatgccgaagcaatgaatgaatacctggatgctcccagccaggatatgtacgacgccatcaataaagtaagagcccgcgtatcgatgccggcattaccggtgagcggcacaaatgataatacaaaagcgggaatgcgaaaacgaatccagaatgagtggcgcgtggagtttgcctttgaaggaaaacgtttttgggatgtgcgccgctggctgatcgctgaaaatgtagataatagggatgtgcatggtatgaatgcccggccctcctcaggcgaactacaggctaccggatttgatccgggtagcgaagaagcaggcctcgccgtgttttacaagctcaccaccatacagcgacgcgtgtttacaaagcggcactatcttatgccaattcctcaaacagaaatagataagggaggtggtaaactggtacaaaattttggctggtaaaaacaaataaaaagcgccggtacctttgcaaagataccggcgctttttattatcctaaaaacgaaaaaagcatatgcctgagccggaactttaaacgttccagagctttatggatctggttatccactgtttttttgctgatgttcagtgtttgggcaatctcccttgagctcattccttcttcccggctgtattgaaagatgagcttgcatttttccggtaactggtctatttccttatatacaagttccagtatcctcctgttatgtacggcatcactgatttcgggtactaattcaggatggttgtccatagcagcatccatggtatatttccgggcgtaagccttcttcctgatctgggtgagcacctggtatttgactgccgttaccaggtagttttcgaactggcctatttccaccttcttcctgttgttccacaaacttaagaatacatcatgtaccacgtcttctgctgccactgcatctttcaggtgcttattggcaacaatgaataatttttcccaataccgtttgtataagtcgttaaatgaatctctatcaccgttggctaaaaaagtaggtgattcttcagacgtggacataaatgtaataacctatttaatcacgaatagatatactgatctggattttaaagagctcttcgctatagcacaaatatagtatattccgggagcattatggctccatcatgcgttttttggtaatgcggatttgggggagataaataaaatccggtatacttacttgtccattcccgttgttgcatgtgaaacgccggtagataggtggtgctcccatacgcctgggtaagtaaccattttttacctcttatttttggggcaacaaaccggcccgctacttaaaaagcacttgcgcaaagttgaacaggttattccgccataccggccaggtgtggccgcctggatattcgctataggtatgctttatattcaggtcatccaattttgccagcatcaattgacaattcttgtaggcgatatcttcctttcctcccattgcaatccacaacgttttcaaattattgttaatcgtggcggtattggctttcataaaatcgtactgcgcatccgcaataccagcctgccgcgactgtatccagcctgaactgaatacacccagggaagaaaacagatccgtgtttttaatacctgtatagagcgtatggatgccgcccatcgacaatccggctaatgcccttttctttgccgtcgcttccacacgataatttttttctaccaggggaataattacctccttcagttccgattcaaatgtcttcaaggcggattcgtcgaaagcagtgccacctacattggcatcaggcatcaccaccagcataggttcggctttctttgcggcaatcaggttatccaggatcagatccgttttaccctgcgtagcccacccggtttggtcttcgccaccaccatgcaaaatatagagcacgggatattttccgtttgtatttgcatcataaccagggggaacgtagatatacaactgccgccatgaaccggtaacctttgagaaatattttttgatacggatatctccatgcggcacatctcttaacgcataatagttaccgccggcaaacggtatttcaataccgcttgccattcttcccatgccgtaaaaggtttcactggcggggtccgcaacggctacttcatctatcagcagcgaatagtaatgaaatccttcgccgatggaatctgttgttacggtccatacaccaccggtgtctttcaccatgtcatatttgcggcccaggtcaacctggactctccgggcttccggcgctttgacgcggaaaacaacgcgatggtctgccattacctgtggatactttgcattgcgcacattggttgctgcaggggcgcctaccaccgggtactttgggaaggtggtagtatccaccggtttaaagatcagctgcgaaaacataaacagcccgttcttccacactttaaagtcatgtactcccggttcaatgtaatagatatgcggcacatcgttttttttcaggtaatcatgtgtacgcttgctgaaagaaattaatccgtcgctggcgccgcaggagatccagagtagttttattttctgcctggcactggcaggatccggtaccagttgctccggtactttcgtgtttggagcagacgaaaaaccgccgatccatgcaaatgtatcgaggttacccagtccgaaattcagtgactgccctcctcccatcgacaacccggcgatggcccggtgatccctgtcggtataaacaggatacttcttttgtatatagggaataagatcgttcaataaatctttttcaaaagtggcaaacgcctgcaccttatcgggagccattatattacccgtagcccggtcgtctttcatggcccttccgttaggcataacaacgatcataggctcaattttcccttcggcatacaggttatcgagtattacctggggcgtgccgccgttcagccattctttttcgtcgccgccaatgccatgcaacaggtataacacagggtatttatgcttcctcgaaaatcccggcggcaggtatatcagcgctttgcgcggattgcctacggttacggagctatagctgatggtatcgatccggccatgcggtatagctgcatgcagggtatcaaaaccaggcggtgcatgctcaataatgccttgcgtaaaagcagtgagggtaaacaatagcagaatgacaagattaaatactttctttttcatgttgaatgatttttcctgttacaaatgcgcgtagtgggttaaagcacctgttaataaaacaaaaatacagggacccgcttttaaccgatggcttatttgttgaaattgatagtataattgtcttatggacaataatttccatcataggaaacaattaaagggttagtgcggcgtacatcttaagcgggcggcgtctcataggatctgaagcacgctgcccgtcaactggtatttgatatccgtagttttcgacaggttatccataaattccggcagcccttcttttttggtaagcaccccactcaccgtgatgttttccgcacccggcgcagtgaattgtaccttcacatcaaacaggcgcctgatcaccactgcaatttctttcaggctggtattcctgaagtaatattttccttccatccaggcaagcgtattccttgcattgaattcatccaccctgaaaccattgccttgttgaggattgtaaatggcttcatatcccggcgacaactgtaccctttgattaccggttttacttttcagggaaaccttacccgaagaaagcgaaagtcgggggctgttgctgctgtaggtgttgatattaaaagcagtaccaagtacgttaacagaaaactgcccggtatgtacaataaaaggccggttaatatctttgcggacagaaaaataggcttcaccgcttacaaacacttcacgtgtgcggccattgaacgataccgggaacctgatttcagacatcgcatttaaccatatttctgtactgtccggcaacgtaagtttatagtctttccctgccggcacctgcaacaggttcatcgcagtaggtgcgtcggtacctgcggcctcgtattgcaggcttttggacgacacccgcatctgcgcagagccgatattgagcaacgatgactgtgtggtatcggaaagcacaatggtttgtccgttggccatctgcaggataacactgttggccggcgcggcgctttttatagcagcaaccggttgctgcggctgttccctgggaaaaagaaagtacaaagcacttacaagcagcaacaatatgccggcagcagcccaatacaatacctgcatattgcgggtattatttttcttaaacaggtgttttctttcttcccacaactgcgattcatccatttgatcgaggtattgttttgcagcaggctcattgagttgctgttgcaaacaactgaacgcatctttcaatgccggatcggctgccatgagctgctgcagcgcatggtcatcttccccggaaatactcccggtcagcttttccagcattaattgatcaatatgttgtttatcagaggtcattgatagtaaacttaagaagataggtgaacgcttgcagtacatttcattccgacactggtggatgcagtttggtgcgcagtgttttaacggccattttaagatgggttttcagtgaattgatgctgatgcccatattgtcggccacttcatgatacttcttttgttgcatgtacaccagggtaaatgcccgctgacgttgggccggaagctcgctcagcaattcatgcaactgccggtgaagctgctcctgcgcgctccaccggtcttccatatccctttctttaagcatattcgactcgtgctgataagaccggtcaaccgtttccgcatacttctcaatcttcttcaatgccctttgcttcaccttatgataatcattcacctggttacggactgcggtgagcaggtaatttttgagacagcccttgatattccggtacaatttcttttcccacataccgcttaacaccagctgcacaagatcatccgccgccaccggatcgctggtgccgacataggctttcgcccacattaaccggtaatatttcttgaaaataaactcaaaagcatcaccggtatttccagtttgtaataacgccagtatgacttcatctcccggatattcaggcataaaaatactttttaggctggttgatcagataacgcggacaatattcatttgggacatagaaattaaatataagtcgtttgtctgataaaatgttagtttgacaattattaatttttttaagcaagcgggataaaggttttttcattcacccgtttttaaaatgtgtcgtcttagtatagtgcaccacaaaaagcaggcacccatcgttaccacgttacagtcattgtcaaccaaacaaggaaaatgaaaagaagtatcccgttattgaatactggccggcgtttttttgccgggtccagggtgtgtatcaccatttttttgctcttttttttacacttaaatgcacgaagtcagcaaattcctgcctccacggtaactatcaaaggaagtaatatgacgctggaaggcattttccaggtgattgaaaaacaaacagaccttacctttttttacagcgacgacctgctgaaaaacgaggtaatcagcggccctattgactatacgaatgccaaagtggccaccgtgctgaacgaaatactgagaggccgcagtttgttgtatgaagtgaagaaaaacgtggtgctgattaaacggggacccaaacccgctgccgacgatgccagtccggccgaaaaaaagaatcccggcgctgcgcaggaccgccaggtagcaggcctggtacttgccgaagatacgcggacgcctttgcccatggcgacagtgatgctgaaaggaaccaccaccggcgctaaaacagaccaggacggccgttttaaactaaaaatcaccggtgataacagaatattggtggtgcaatacgtaggctacgtaccgagagaggtacccgttaaaaatatcgtgggcgattacgagatattactctcgccgaaagacaacaccattaaagatgtggtggtagtagcttacggcacccagaagaaatccagtatggtcagttccattaccgccattgacccaaaagaactgaaaggacctaccgggaacctcaccacgatgctcgccggcagaattccgggcgtcatttcctaccagcgcagtggcgaacccggagccgacaatgcacagttctttgtaagaggcgtgggtacctttggtgcaggaaaagtggacccgcttattttaattgacaacatagaatcctcctccagggatcttgcccggctgcaaccagatgatatcgccggcttttctgtgttgaaagacgcgacggcttcctcgctgtacggagccaggggcgccaacggcgtgatactggttactacgaaaacagggaacctgggaaaaatgcgtttcaatttccgcatggaaaattccacttctgccaacacacaaaattttaaactgtccgataatattacctatatgaagctcgccaacgaggcggtgctaaccaggaacccgttgggcgtattgccatactcacaaaataagatcgatcataccgctgcaggagacgacccgctattatatcctaacaacaactggattcaacagctgatcaaggaccgcaccaccaaccagcgctttaacatcaatgccagcgggggatcagacaaggcaaagtactacctggccatgacctataatattgataacggtatcctcaaggaaaacgcactgaataatttcaacaataacatcaaactccgatcctattccatcttatcaaacgttactttaaatctcaccaaaacaacagaagcactggtgagcctgaaagggcagttcgatgactataacggtcctatcggcggcggcgccgctacctttaataatgccatctggagcaacccggtggcatttccggcagtatacccatcggacctcatgccctatgccaaacaccccctgtttggaaatgccctggtaccgggtggcggcgggttatatgtaaacccttatgcccaatcgctttccggattccaggccaccaataccagcacactgacagcccagctcagtttgcgccaggacctcgcagccattacccccggcctttccgcaaggatgatggcatataccggccggtacgcaaattttgccgtttcccgccagtatagcccctattattaccaggcagggtcactggacggaaaatttaccggcttaaacctgatcaacgatggtagcgtgggaagcgttggaacaactcccaccgagtacctcacctatacaccaggcgataaaaatgtaaacaccactacctacgccgaagcagccgtaaactattccaggatcttcgataaggtacacaacgtaggaggtatggtgattggtaccatccgcaattacctgaccggcaatgcctccaccctgcagctttctttgccggcccgcaaccagggcatatccggcaggttcacctatggctacgacaaccgttatctctttgaatttaacttcggatacaacggctctgaaagatttgccgccaaccaccggtttggatttttcccttctgtgggaggaggctggatcgtatctaacgaaaaattctttcagccgctggcgaataccgttaaccagctgaagttccggttcacgtacggactggtgggtaacgaccagataggcagcgccaccgaccgtttcttttatctctcggatgttaatttaaacggcgcttcaacaggatacttcggtaccaacttcacctacaaccggcctaccgtagccatcaaccgttacgagaaccgcgatgtcacctgggagttgtcgaaacaaaccaatatcgggatggatctcaccctgttcaaagatttcactattacagtagatgcttatgaacaaaaccgttccaatatcctcatggtaagaggcacggtgcccagttccatgggattacaggcaaatatttcatccaatgcaggaaaggcatacagcaggggaatagacctggcagccgattaccgtaaaacatttaataattccctctggatacaggcacgcggtacctttacctatgctaaaagtaagttgctggtaaatgaagaaccacagtacgcagaaaataaccggaacctgtcgaaagtaggcaactcgcttggccagatctatggcctgattgcagaaaaactgtttattgaccaggcggaagtaaataactctcccctgcaatatggcagtattatgggcggggacattaaataccgggatattaacggagatggaaaaattaccgatgccgactatgtaccgatcggctatcctaccacgccggaaattatatacggtttcggtttctctgttggatacaaaaattttgatctgagcactttcttccagggttccgccaggtcgtctttcatcattaacgccgccaataccactccgttctatctgaacggcggctaccagaatggtttgctgcaagttattgccgacagccactggtcggaagataaccgcaactcctatgctttctggccgcggttaagtaataccgtctccgaaaataatacgcaaccatctacctggtggttaagggatggctcctttttacgcatgaaatcagcagagatcgggtataaccttaccggtcagcttttgaagaaactacacctgagcagtggacgcgtttatgccaatggcctgaatttattcagcatcagcgcctttaagctatgggacccggagatgggcgcatcaggattgggataccctgttcaaaaggtatataacgttggggtagttgcaggtttctaacattcaaataaagcatttaatcatatgaacgataataagtttaatagcaacagcctggtaagcacacccgcttacagtaacaccgggcatcgtattgccgcttccatcatctgcctgctcattatgatcatttccggaatggcctgtaaaaaacctttcctggatgtagtgccggataatgtagccaccatcgataatgcttttacttccaaaacggaagcagaaaaatatttgttctcctgttatgcatacattcctgtaaactacgatcctacttacaacgtagggctttcggccagtgatgaggtgtttgtgctggatccaaccaatgctatcaggtcgaccaatatattaaggctggattatggggaccagaatacatcaaatcctatcgccaactacatgaccggcgacagggatggagtgagctgctacaaggctatcagggattgtaatattttcctggagaatgtaagcgatgtaagtaaagtagtagatctcgacatcgacaccaggaacaggtgggtggcggaagtcaccttcctgaaagcctactatcattttcttatgttcagggcttatggtcctataccgctgatagacaaaaatttacccatcagcgcttctcttgagcagatgtttgttaaacgccagccggtagattcggtagtagattatatcgccggtttgctcgacgccgcagcagtgaacctgccggtaagtatcgccaatgtctcttcagaattagggcgtgttacaaagcccgccgcattaagcttaaaggccaaattgttagtaactgccgccagcccgttattcaacggcaactccgactacgggtcttttaaaaataaagacggggcacaactttttaatactgttttcaacgccgcaaaatggcaacgcgcggcagacgcctgtaaagaagcagtagacctctgcactgcacaaggcatccgcttgtatactttccccacgcaaacgataccgctgagcgacaccactatgacgcagatgagcgtccgcaattccatgagcgaaccctggaacagcgaactggtatggggttctaccagcggtgttacctggggttgcaccttcctgcaacgctgtggtatagggcagtttgattttgtaaatgcagtggcttcaaaaacggcagggcatcctttactgggacccaccatcaagatggctaaaatgttttacacgcgaaacggcgttccgattgatgaagataaaacgcttgacttttcaaatatcgctgcactgcgggtaggttcacatgccgaaagatttaacatcaaggaaggtgaaactactgcccgtttaaatttcgaccgggaaccaagatattatgccgacctgggatttgacagaggcatctggtacatggccaacagcccgtcgaaaagcgatgagaataccttctggctgatggcccgtggcagtgaactgagccagtcatcgccggtgcccatagcaggattttatatgaagaaagtagtgaactggcatatggactggaacacagttacctacccgtcttacccgtatcccgaaatacgcctggcagatctgtacctgctctacgcggaagcgctgaatgaagcacaggggcctaccgcagatgtatatgattatgttaacaggataagggccagggccggcttgcaaaccgtgcaaagctcatgggccagttacagccggaacccttccaaatacactaccaaagaaggaatgcgctccatcatccaacgggaaagagctattgaactttgttttgaaggacatcgttactgggatctgctacgctggaaaactgctgcacaggaactcagcggcaatatcaccggctgggtagtaagcggtcaaacggcagaactgtattaccgcgaaatttcttttctctccaggcatttcgtagccccccgcgattacctgtggccgataaaagaaagcgacctgctggcgaatcccaacctggtgcaaaatcctaactggtaacctgcacaccgtgcggatgtattaacattaaatcattaagaagtgaaaacaataaaaccaggtacaatcttatatacagcctttttcctgatgctgatatcaggttgtaaaagagatgagctcaacaaagccattattaccaataccaatcctcccggcgtggtaactggaataacagtagcgaacacaaatggtaagtcagtgatcacgtattccctgccgcccgatgcagatctttcctatgtaaaagccgtgtatgaaacttctcccggtcatccggcagaggtgaaagcttcgcactatgaaaataacctgacggtggatggtttcggcgatacgctggcgcacactattaaactgtattgcgtaaactccagcgaggtatcctccccggccgtaactgttacggtgaatcccctgacacctgctattaacctggcttacagatccctggatatagaggccacgttcggcggattcaatcttacctgtaataatccaacgctggaaaacttagcgatcattcccctggtggatacgtccggtaccgggaaatgggtacaaacatcgggaatggacaatgtatacagcaatgacccggtgatcaaaagcgcagtgagggaacaacctgccgttaaaagaaattacgcctttgtggtaagagaccggtggatgaatttttcagataccttgtttgtatcactcaccccattttttgaacaactgttaccaaaatcagattggagcaactacgtattgccaaaagatgcagagatcctggataacggtggcagaacagatgtacggtacatcttcgatggcgacttacacccgggatggccacgttgcctgtttaccgtggaacaggccggcagtccgcaaacagtaacgctggaccttggcaaggcgcacatcttcagccgtatgcaggtaaatccctacaaagaggttggcgacaactactatgtaagaggcaatgtgaaagactttgaaatatgggcttccaacgcccccagcctgagcggcgacctggatgaaagctggaccaaactaactacctgtcatgttataaaaccatccggatctccttatgccactgaaaccgcatcggaccaaacactggcttacaacggctggcagtttgattttcctgcaggacaaaccccttaccgctacatcaggataaggagcttgtcgaactggcagggatcttactttatcaatatcgcggagttcacattgtggggtaactagttatgatcaatcaacgaaatttaaaacaaatgaaacagcatcaacttacagcttcctgtatcattctggcactggtgttaattataagcgcctgctctaaaatggacgattacagggataaatatatgaccggcggagccatcacctatcccggaaaaatggactccgtagtggcgttttccggtaaaagcagggtgatgattaccggtctttttacctcagatcccaagattgccggttacaaagtattctggaacagccgccaggattctattgaagtagccgttaaaagaaccgccggtgtggacaccgcaaaggtaattatccccaatttgccggaaggactgatgaacttcgagatccggacttacgatgccgccggtcacgtttctatcccggtaaatactgccgccaacgtatacggacagctatacgaaagcgcgctcattaaccggggtatcgccaatgcggaaatgcagcccgacggctccgccctgatcagctgggcagatgtgaatgcagatgccggcgtggtgaacatgcggataaagtatgaagataacgccggtaacctgcacgataccgtgattgtgtccggcagtaccgccttcaccacttcgttgcccgcttttaaatcaggcaatgcaatcagttaccaaacggcatacctgcccaatacaacggcgtttgacaccttttatgtcgccttccaggaccatagcgtaaaagccgatgtaaccgtccaataccttcagaataccggtccttttgcaagggccacctacgacggcggcagatggggcaccctggctgcgccctggatcaccagcgccaacgtaatgaaccactccggttttggtggctacgcagcagatgccggcggttgcctggtaatggaatccggatggagcggaactgctaatatcatcaatggtaaaatttatcaaacggttactttacctgccggcaattatattttcctggtgaactactacacagaagcgcttgacccggtatacgtggtagccgccgccggcaatacgctgccggacatcagtgacctctccactacagcaggatacaccgcatttaccaccaccaggttcgtgaacggaaccgcacagtgccagtttaccctcgcccagccacaaaccgtttcgttaggctttctggccactatgacttccggcaaccaatactggcgcgtgccttcggttaaactgataaaaaactgatcctttttacctatgcctaaaagcctgttccggtaacggacaggcttttttttaagacttactacagcggcaatccacggcagggtttgtcttgacctgattcgtccgtaaaaattacctgataaggatagttatataaagatttttgtaaattaggtttatatacctattatttgtagcacatgaaaagagtaattcactcatactttacttcataaccccaggacataacttattgatgcccggcctgttttaaaacaagtgtacaaaacaatacaaaataataacctctgaaattaacaccatgaaaagatttctatttgcattagcagcattattccccttagcggctttctcccagaacgcaccaacagtaatagaacccggaacaaaacaaatggctgcgcaggccctggtggaaaaaggatatactactccttccggatggactgttaaaccgggcgatgaacttaagataggaaagggatccatgcccaataaaacattttcgttcatttatcagtcgcccgcaggatttgcaacagaaacttccggagacaattatagcaataagcgatatgcgggtacaaatatggccggtaaatcaacaaaggtaaaatcattgattgcttatggaaataagaaaacagggtacaccattgttgcaagggttggctttggagagctggttaactattggatcgaaatagataatgccgttgacggcggagaactcattccacctgctgcatatgccaaaaaagagcagggtggtacttcaacaggaggctctattgccgatgaattaaaaaagctaaaagaacttttagattcgggcgcccttacccaggaagaatataacgcgcaaaagaaaaagctactggcacaataacaacattggctaaatgtatataaaaaagcctgttccttaccggaacaggcttttttcgctattggcaatctccgctacaggcaccctccaaaataggataagccataaataagccatagaagggttcacatatcggcaattgcgaatatatccggaacacatccttaacaattccctaacccacacttaacttccgtctaacaatcatttcccatcttgccgctgttacccccgccaggaaatgctatccaattgaaaaacccgactacgttgtttgttttagccattattgatgcagaaggaaggaagagcaagcgccttcctttttttattccggccaccaaacccctatctttacgtaattttttactgagatactatgggaacatcaattacctgtcccagttgcaagcaccagtttgtcatggaggatgcttttgcagcggatatagaaaaagaaatgcggggaaaaatggaagatgaatggcgccgccgcctgaaatctctccaggaggaaaaagatacacttctttctgaaaggaataagatggcactcgaacgccggcagatagaaacgttaaagcagcagcaggaagaagaagtgacccgccgcgtacttgcagaaaaaaaacagctccaggaggccatggagcaggaactgcgtaaatccatcaccgccgatttcggcagccagctggcagcactaaaggaagccaaccaggaacaggaggaaaagctccgggaagcccgcaaacaggagctggaattcctccgcaaggagcaggacctgaaaaccaaagaacaggagctggaaattgatctgcagaaaaaattactggaagcccggtcggaactggccgaccagatacgaaaagaagaatctgaacgtaactccctgagagatacagaacaccagatgcgcctccgtgagctggaaaagcaactggaagaccaacgcaaactggcggaagaaatgaaacgccgggcagaacaaggctccacgcaactgcagggggaggcacaggaactggtactggaagaaatgctgcgtcttcatttcccgtttgatgaaataacatcggtgggcaaaggcatccgcggagcagattgtatacagctgatccgcaatcaatacggacaggaatgcgggcgcatcatctatgaaagcaaacgcacgaaagaatttatcaaagactgggtagaaaaactgaaagcagacatgcgcagccagggagtggatgtggccatccttgttacccaaaccatgccgaaagacatggaacggtttggcgaaaaagaaggcatctggatctgcaccttcgcagaagtgaaagcgctggcttatgtgctgagagatggtatcatcaaaatttcgggtaagctccgctcacaggaaaacaaaggggataaaatgcatatgctctacgaataccttaccggtggcgaatttgcagaacaatggaaggctatccgggaagggtttatgtctatgaaattatccatccaacgcgagcgcgatgccatggaaaaactctggaaagcacgcgaaaaacaactcgaaaaagtattgctcaacgcagcgcatatcaaaggctctattgaaggcattgccggcagcgactcggtagacctgcagctacttgaagatgcagccgatgaacttcctgaataaatactaacctatgcaacacaaaaagatcaacacaattatatttgaccttggagctgtattgatcgactggaatccccgtcatttgtaccgtaaaattttttcttcagaagaagaaatggaaaccttcctccgcgatgtatgcagctccgactggaacgaaacacaggacgaaggcagaaccctcgcagaaggcactgagctgttggtgaaaacctttccgcaccatgaagaaaacatccgcgcctattacggcagatggagtgaaatgctcggcggggaaattgaaggcacaaaaaatatattgcatcaactgaaagaaagcggacaatacaaattatacgcgctcaccaactggtcggatgaaactttccccattgcctgggccatgtatccgtccctccactggttcgacggtatcgtagtgtctggcaaagaaaaaatgcgcaaacccgaccacgccttcttccagctgctgctggaccgctataacgcagatgcatatacgtcattgtttatcgatgataatttacgtaatgtaaaagctgcgcgtgagtttggtatagataccatcctgttcgaaaatcccgaacagttaaaaacagcattagaaaacagatctatattaatttaatccactacattacttattgtatttgttaacccctcgtccactttaagatttcattaacactccacagataaactttctgtaacaatcaaccatctaatccgttcaagaagcatacacggaaaccggaatgtcaggataccaatctgcttggttcatgaccgttagcctgtatattttatttttttaaattaatacgctaggacatgaaaagaactttgtttttattcagtgccgctgccgcattggtagcgatggtttcattcagtagctgccgtaaagatcccctgaaagatatgactaatgaagagtcgaggatctacatcactaaccacgacagcaccgctaatttcacctcttattccacttttagcatagtagattcagtggccgtgctgacacgtagcagcgactcagctaaaaaagagctgactgactacgacaaaaaactgattgcctccgtaagcactgctatgcagcaacggggctacacccttgtgagcaaagccgccaaacctgatctggctgtcaacctcacacgtatcgacaactcctataccaacatctcctggaacccgggatggtggggcggcggcggctactgggatcctggttactggggatatccgggtggcggctggtactggccttcctattacacggtttaccaggtgaacgaaagacaggtagccatcgatgtgtttgacctcaaaaaccccaagaacaataagctgacagctgtatggaattcattatggcgaggctcaggcgtatggagtatcggtaacatcgattcaatggtgcaggcatcttttgcccaatcaccttacctgagtaaaaccgctaattaatgttgattgacaacttttaaactgacaggaaatgaaaaagataagaaactggatattgatttttgccggatgttttgctgcccaggcagtatccgcacaggttcgtccccctttatccgtagatgtgaattattccattgcacaaccccttggctcattaaaggactattccgataaaaccagcttccgtggctggagtgcagggctccaatatcaattgaacaaccagtggtccgtaggattacgttccgggttccaggacttttacgaacggcttccgcgtgcagtatatcccgataaacaaggcgatgtatctgctgttcagtcacgcacattgcaggtaatcccgatccaggcaacggtgagctatgcgttcacaaaacctgctgcagccgttattccatatgctaccgtaggtgtaggtaccgctaatatgaattatgaaaaatactggggtgaatttgtagagaaagataacagctggcaattcctcgtgagcccggaaataggcatcaatgtgccttttggcaaggcttcaccgttgatgttcaatgccaatgtacggtataactacgcgccttataagtatggcgatatcaccaattacaataccgttcagggaaatattggattgaagttctcattgaactaaatccttttgagtccatattctaggaagaaagtgtgcgtgtgagtcccgttcgtgaaccagcgaacgggacattttttttcagaactccatatacgccttaaagcctttactaaaggcttccttaatggcgccatctgtgcctttataaatataaatagcttccagtccatactccggatgctgtgcaatataggcgagccccttttccacacccatcaggataagcgggttatcaaaagcatcggcagtaaaacaatcttttgcaattaccgttacgctgataatattattatgcagcgctatccctgttcccggatggattgtatgcgcaaaacgtgtacgcccctggtcaaaaaagcggcggtaatttccgctggtagcgatgcctttaccaggaagccgtaccagcccctgtaccggctcataggtagtatcgccgggcgatggcctttctatccctatactccatactttatgctgatggttatgcccttttgcacacaactcccctcctacatccaccaggtaattatcgattccctgttgcgataaaaaatgtccgatcacatctaccgtatatccctgggcaataccattgcaatcgatctgcacgcctttctttgcggcatacagctggttgccttttacacggagataacggtaaccaatatacgacatagcggccttgatactgtccggtggcggcacgcctttaaaagaaggtttggtaacgccaaatccccagaggtataccagcggctttaccgtaatatcaaagaggccattggtggctttactcgtaaacaaggctttctggataaccgctttcatgtgctcatccatcgtgatatggccggtttcattaaaccggttgatggctgatccgggtttatacagggacaacgactgatcgattactccaaataaagaatcaatgcgtttatccattgacgtagtatcggccgataaatatttcacgagataataagtgccctgtgctttcccttcgcaggtgatcagcttcagggcaggcgcctgctgcgcccgggtgttggcagaccacaggagaatggccaggaaaaaaaatcgtttcatgtacagctgttggcagtgagtataagcggctaaacgcttataccgctatttaaatgcgtctaacccggtaacatccataccggtaatgagtaaatgtatttcgtgtgttccttcgtaagtcattacgctttccaggttcatcatatgccgcattaccgggaattcgccggtaatacccattccaccgaggatactgcgggcgttgcgggcaatattggcagccacttcacaggaattgcgcttggccattgaaatctgggcagccgtggctttcccctcattttttaatacgccgagccgccagttgagcaactgcgctttagtgatttcagtgatcatctccgccagttttttctgcgtaagctgaaatccaccaataggacgatcaaactggatccgttctttcgcgtatctgagggccgtatcgtagcaatccatcgccgcgccgatcactccccaggcaataccataacgcgcagaagaaaggcaggttaacgggccttttagcccgcgggcttccggcagaatattttctttaggtacttttacattatcaaacaccagttcccctgtagcgctggcccgcaaactccacttcccttttgtttccggcgtggtaaatccttccatccctctttccacaatgataccgcggatcacaccaccttcatcctttgcccacactacggcgatatctgcaaatggcgcattggagatccacatttttgcgccgttcaggatcacatgatctcctgcttcccggaagttggtaagcattcctgcagggttggaaccgtggtcgggctcagtaaggccaaaacagcccatcatttctcccgtagccagttttggcaggtatttctttttctgtgcttcgctgccaaaagtatagatagggaacatcaccagcgaaccctgtaccgaagcagtagaccgtatgccgctgtcgccccgctccagttcctgcatcatcagtccataagcaatatgatccattccgccacctccgtattccaccgggatggtagggccgaagcaacccagttctccgagtcctgctaaaatctgtgatggaaaagcagcgcgctggcagtagtcttcaataatgggggatacttctttctttacccattggcgtacggcgtcgcggatcaaaaggtgttcttctttcagcaaatcatcaatggcaaaataatcaggcgactgaaacagatcttgttgcattaactacgggtttaatacccaatataagaaattacctgttaggaaccacgtccacggggagatttcagccatggaacctatatttttttcctgcaaaatacctgcacaacaatcacgttttttcatgacaagtttgtacctttccatcaaattcgacaactatggcaagcaaagttatacctgcgcttttgctattgggatttttagtcattgtgatgttatcatttcaccccacaccattacaatctgttgcactaagcaaagtgctccccccaaaagtcaaatcaggcgcaccacctgaattaaaaaggtattggatggttctgctaaagaaaggtcccgtccggaaccaggatactgcccttgcggcaaaaatccaacaggctcacatggacaatatcaataaaatggcaactgccggcaaattgctggtagcgggtccttttgaaaatgatgaagaactgcgtggtattttaattatggattgtaaagacagcctggaggtagtgtcgctggtgaacaaggatgctgctgtaatagcgggccggctgaatttcgaggtaaagccgtggtggaccgtaaagaactgtattttcaagtaaaagatcagggagatgccggtacctggcgcctgctgcaaaccgcagctgccaggtaccggtattaaaaagttatttacacggtagctacaatcttgttgagatacccggccatttccacctggtattgttttgctatgcgacgggcgtctgtagcaaaatcgtctccattacctgcataaatgatagcgcgactggcgtttaccagcagtccgcaatccttattcatggcttgtgtggaaatttcctcgaggcttccgccctgagcgcccacacctggtaccaagaagaaatggtcaggtaccagtttacggatatatcccagctgtgaagactgggtagccccgatcacgaacataaggttgtccggagtgccccattccatgccggctttcagcactttttcaaaaaggaactcatctccgatctgttgcatctggaaatcctggctgccttcattggaggttaatcccagcaggatcgcccatttttcagagaactggagaaaaggcgttacactgtctttacccatgtaaggcgcaacagtcactgaatcgaacttataggtttcgaaaaatgttttggcgtactgggtggaagtattgccgatatcaccacgtttggcgtctgcaatagtaaatatcccgtccgggatatactcaatggtccgttgtaaactttcccagccgcgcatgcccatactttcgtaaaaggccgtattaattttatacgccacacaaagatctttggtagcgtcaataatcgccttgttaaaggcaaacaccggatctgcatgagaaagcaggtgttttggaatcttttgaatgtccgtatccagtcctacacacaggtaagactgcttttccttaatcagattcaccaattcctgtcgattcatagtcggttaatttggggcgcaaagttaagaaaaacttaagcattgacgcttctttaaacatattatgattacctgtaattgaaaaacaacgctatttattcactgtggtagttgtggtttaccgacaatgttggatatttttttaacgcggaagattaaaataaagatattcctttttgggattacgaccatcaacaaaaataaaatgtttccgtctatttttgggttgaccggcgggcttccatttctgcagccacacgtaatgaattttcatcgcccaatgcccgcagatgagcgattacgctgaaataatccgcatcttttttattctggctgagcttataattggcatttacctcgcggatgctcatttcaaatcccacaatagcttttacattgttgctgagtgttttatcatcaatatcgctgatatgcaccgggcaggcagatgccgcctcgtagtgatccaccagcgcgcccagcgcctgtactacttctgcttcttcctggatacggatggtaccgtgaatatgcacggccatgtaattccaggtaggtatcttttccttttcataccacgaggaagaaatatacgcatgatgtcctgaaaacaccgccagcgtttcatttttctcaaaccattcccactggggattgatccgtgcgatatgtccgtgtaaaacaaattctcccggtgttttttccaccagggtcatgggaatatgcgtagcatgcggggttccggcattatctgtattgatcagcaatccaaaaccattctccctgataaaattggcaatagcatcccagttggtttcccgggtgagttttggtgtatacatacggagttgttagagaaaaaaattacggatcacagatattcctatctgtaatccgtaacggatgattcttttatacaataatttctacaatcctggtgggagcaacattggcgttgcgcatagcgatgctgcgtgcagctgcaccggcaacatccaggaaagccttgcgggttattttatcgtcgccggccatagcgggcacaccggcatcaccgccttcgcggatgctttgtaccagcggaatctggccaaggaacggaatatccatttcttctgccagttgttttccaccttcttttccaaaaatgtaatatttattttccggcagttcagcaggggtgaaataggccatattttccactaatccgagaattggcacattaatctgctgtcccatgaacatggaaatgccttttttggcatctgccagggctacatcctgcggcgtggttacaatcacagcgccggtaacaggcaccgtttgtaccagggtgaggtgaatatcaccggtgccgggcggcatatcgataatgaggtaatccagttcatcccagtatacatccgtaataaattgcttcaaagcactgctggccataggtccgcgccataccaccgcctgtctttcatctatcagcaaaccgatggacatcaccttgataccaaacttttcaatcggctggatcatgcctttgccatctacattcaccatcaggggcctttcgccgcgtaatccgaacataatgggaacggaaggaccataaatatccgcatccatcagccctactttggcgccatcacggcccaaagccagcgccaggttggctgccacagtggatttacccactcctccctttccggaggccaccacaatgatattttttacattagacaggacaccctgcccgtttgctcttttggtatttacattggccgtcatgacaacttccacttccgcatccttgcttaccagcatgtgaatagcgttcacacaggcattgcggatgaggtccttcaacggacaggccggcgtggtaagaatgaccgtaaatttcactttattgccatcaatctctatatcttttaccatgttcagcgtaacgagatccttgcccagatccggctcttctacgttgctcagggcctttaaaacctgctctttcgtgatcataaattgttgttaattttgaatccagacagcaaagttaacccaattgggatttaatttacaatttctctgagcaggtgatcaactgcatggaaacacgtaattaaatttttatatcttagggccggcatgcatcagaaaagatcctacatactgtcactcataattgttttcgttttatctcctttccttttgaaagctcagatcgcggaattcagagacagcgttatacaaatttcgggtattaccatgacggcagacagcctgcgggccatccccgcggtgagcatcctggtaaaggggcaaaacaggggaactatctccaacagatccggtatattctctatcgttgtattcaaaggcgataccctgtcgttcagtgcagtgggtttcaagcataaaaattaccgcatacctccggatatcaaaggcaatagcttttccctgatacagctgatggtggaagataccacctatctccctgtaactattatcaaaccttatctttccagggaagaatttgaaagggcctttgccaatatggacattcccgatgatgcctatgaggtagcacgaaaaaataccagtaatgccaggcttcgcgccatggcccgttatacacctatggacggcacggaaggcaccagtcaatacctcaaaaaacaggcacagagcctttattatgccggtcagccacctccgcaaaatatctttaatccactggcatgggcccagtttatccaggcctggaaacagggcgactttaaaaggaaagacgatagttatggcagttactaactgtaacgcgtaataccttaaattagcgccttattcaattccgacaaatcactacaccatgcaaaaaattgcggttatcggcgctggtactatgggaaatggtattgcgcatgtatttgcccaacacggctacgccgtaaacctgatagatgtttcggcccccgcactggataaggcgctgcaaaccattaccaaaaacctggaccgccaggtggcaaaaggcactattaccgaagccgtaaaaacggataccctccgtaatatttccctgcaaaccgacctggcaaccggcgtaaaagaagtatccctggtagtggaagccgccacagaaaatattgcacttaaactgaaaatcttccaggacctcgacctccatgctcctgctgacgccattctcgctaccaacacctcttctatctctattacaaaaattgcggcagttaccaaacgcccggcaaaagtaataggcatgcacttcatgaatcccgtaccggtgatgaaactggtagaaatcatcaatggctatgcaactgataaagaagtaaccaacacgatcgtggcactttccgaaaaactggaaaaagttccctgcgtagtaaatgattatcccggctttatcgccaaccgcatcctgatgcccatgatcaacgaagctatctgctccctctttgaaggtgtagccggtgtagcggaaattgatacggtcatgaaactgggcatggcgcatccgatgggaccactgcagctggccgacttcatcgggctggatgtttgcctctctatcctgcaggtgctgcatgacggctttggcaatcctaaatatgcaccctgcccgctgctggtgaacatggtgacagcgggttatcttggtgttaaaagcggtgaaggattttataaatatacgcccggtagtaaagaccttgttgtaagcgggcggttttaataagaaggcctttagcgattgactttgtcaattgctaaaggccttgtataatgagattatataaaaggtcgaaatttgtcagctatcatactacatgctacagagaataaatgtaacataactcccaaatgctgtctttagtagccttcagtccaaatttatcaaagaatgctttcatctcaccttccagatttgaaaactctttttcaatcactgcttcacatttcgttttgctcttcagcacttttacatcattgtttgttacggctaaaatcttcctgaaaaaaggtaacaggtaagcggtatatacctcatgtcttctgttattgacagacggatctgccaactctttttttgaggtagccaataatgacgttaaagctccttcttcaatcaggcggatgatcttcttttcacaattccggaaaaaattctcatcaaggacttgggtgtagccaatatccaccttaatgtgagccgaaaggctactaagcccatcatcaggcctgtcaataggtccaacccataaagtggtttgcagggaaccatcctccttatacaccctggcgatgacataacaatagaaaatatcttcgatatgtttactcaatgccaccaaatgggaataccataatttcttcggctgtttaaaatcaaattgcttaatcagatcttcaaattcattgactacgctaaaaaactcagacatactatatctcttattttagtggtgaccagggtatgttttaccatgtgtacgcgttatgccggcatcatccattttcttcagtaaagccttcatttctgtcgctacacctggatcatgatcaaaatgccagtgcggatctgctcttccggcaactttgttagcaatatctttatctatctgtttatccatcctggctaaagattcttttgatctcgggcctttggagaagttatcagatttgaactcaatatctttgccgtcgtaatatttatcgtagttacgaccgcttatagaccgtcccttattacctgttccaaatatctcatcggcacgtttatcatgccattgtttggcccagttgagccagcccctgcctgatcccgctcctgcaccaccagccaatccatacacgtctacccagctattcggatcatgcacatagctgtaaaatttcatacctcccagcaatccaattggatcctgggaaatatacatgccgcttccggagtcgtagtaccggaacctgttataacttaaccctgtttcggcgtcttcatattgtccctgataaagataattacaaaatgttttatcaccatgcaggcgtctcacttttccgtagcaatcaagttcgcgctcccaaactttatttcctgatgtatcaaatgcgtgcaccggcgtaccaaggtgatctgcaacaatactgtaagatcctgctgcggtgagcttcgcgcagggtaccagggaactttcttcaaatacccaggttaccaggttgtctaccggctcctgttcaatctgcaacgccccatcggctactgcttccaggtgtggtggataatcacccgtatactgccattcatgcaatggcacattgccatcccataaccagcgggttacctcctgcttccgtttatttaccttcgcaatacgccttcccagcggatcataactgaatacaatttctcctcctgccggtgtgatcactttccacagccatccgtttgctttccactcatatacccagccggtacggcttcccttcaacactattttgtttgctctggcccatgcctgcttatcttccgctacctggtggttgtgacggaattccttgcagataagatttccttctccatcatagtaatagaagtaatccgggcattccagtaagcgtccgcctttgccatacacgcgatcagttcgtgcaggtgttctgaaaagatgccccagcttatcgggtatgcgataaacggtatcgactgcgttactgtttgactgaccgtaggaagcacttaccaggttatcaaattcatcgtaggaaaactgcgcctgcgcaccactcagttcattcaccatccgccgcagctttgtattttttccccattcataacgaatacggctctgttctgccttatgaaccccgatagattgcctcaccacctttccctgcttatcacgctgtgtttgcacggttactccaccggataacatccgcaatacttccaatccactttcattatgtttccactgcgcctgccaggaattatcggttccatcagttgcctgcattccatctacatatcctgcggcatggtgttccaggtgaatagccgcgcccaacgtacttcctacaaaaaccggttctccccattcattatattcgcgggttactgcgtaagcgccttgtatttcaccgatagtgtgcccatacgcatcgcgttgaatggtaactacgccgtcttcattgaaggcgcctgtcagctgcccgtctttgttatatccatatgccgttacgctgccgtcactgtactcctcccgcaccagtaaaccggtaccatcatattcgcaggcagtccagcgattgtctggccggaatatctttttcacacggcctgcggcatcccgctcgtagtggtaatgcacaccatcgaagccccattcattaatgatattcccgtttgcatccggctcctgccggtacagctctccaccttcattggcaatactgcgtaactgcaactccttgtcataattaaaccggacatttacgccatgctgacttcttcccgttaacacgcccagtggtccataagtaaaacttacttcccgatggccgtctcctgcctttatcatgttgtcagcggcgtcgtagctaaacagatgaatactgccatcggcttcttccacgcgaataacattaccggcaacatcatactcatatgcgtaccagtaacccgtttcagtggtttcttttatcaactgccccaattcatcatacttccagtggcgttgtgcattttcaggtgacgtaattttgctgaggttatgttgctcatcatattccagctcaaaggtgcggccatttttataggttacatgggtaagataagggcctgtatacctgtatttcgttaccactccctccatgttctttttcctcactatcagcccttcgtcgttgaacatccattccattcgtttgccaccgggcgttttaagccctgttaagcgctgctcttcatcaaaataaaacaaggtggattccccgttaccattggtttctttcactttatttccaaaggcgtcgtattcgtatttctcagtgttgccggcaggatctaccactacttccagttcatcatacctgttgtaatgctgcagggtaacaccgccattgccatcaatgaatttataaataagctgacgttcgtcgtaatagtaagttgtcgtgtgcccgagaccgttagtaacaatggttttccctttttcatatcgtgcatggtattccaatacgccttcatctccccacgtatgcacacagcgtgcatcatctcccttaccttcatattcccagtaaaaattcattccgctctggttcgttagccgcaccaataagtgtcctttataaaaaaagtatttgttgacatcccgcgcattggtagtgctgctaagattaccgccttcatcaaaggaataacgtaccaggtgaataacttctgctcctttgtgggtgtaaatatcttcaatgcggccatggtcatcggtggttacctgtaacagccggttgctgctatccacgatccgttgcagatagccttgcccgttataccggaactggatatggaacccggcggggttgcggatttcagataacatacaactgccatcgggcccgggccgggcgttgaagcgatattgaagttgttctttatcttccaggtaatagccgctgctgtcacggcgccaccataactgctctcccctgttgaaatagctgctgtttggcggtattgccggcatcacggtttcgcggccgtctgccaggcggatgctgaagtaaccgttacgcaggtcatacaggctgagattgtagctatggtgccagttgtaccctaaaggcccccgcacttctgcgtcgctgtaatacgtgcgttcccataccagtgggataggtccgggcaattcaaaatctatattgttggaaaccaccctgccggttacggcatccactggttccccaaatcttttacatttaaagtcctgcagcataccagccagtttgggaaaccggctttccattttattgacggttttctgcaaagccgcgcctgctgctttggacattcctttcaggcccagcttaaacatcagctgaaacaggtcgatggtcggcggaccgcctaccaataccggttttccggaggatgtcatgatcagcaacatggacgtgggcgccatcagcgccatagccgtactttttttattcagccttggcggcgaaggaagtcctaccaggttacacgacaatgccggatggaactgcgtagaaaaagggccgccatctgccagcacagtagaactacccatccacatttcagaagccgctttgggcttcacgatcgggaagggcaaatgtgcaatgatggcgggtaaatgcaggataggtgtacctgcattggctacccattggttatgaacttttacggaagggctgagcgcatgcaccagcatttgtgcggtggctgccagcgagaatggttccggtgcgggttctttcccttcctccaccggtggtggtggcggcggtagtggcactacactggcaatagcagccataatagcgcctatgatatcgaacaccataccgatgtgcggcaccggcaataacggcgaaggaggaaatacggaatcgtgaaagtcgatgcctatgccgaggtcaaaatattttgcagcgggcattcccgggaaagcaggtaagatactggccattcctttctggatatggtccagtgagtttttcttttctgcaaataatgccccaaagcctttgttttctacagccatgatatgattactttactccctcttgggataggatcttagttaaactcaaacaaggttgatttacgtcttacagtggctttatccataccgtctgcctgtaacaatgtatgccagtcgtcgcccaataattccagtaagttgctttccagtattgccagatcttccggcccgcggatcttttcacagaggtgtactgccattgctgcggcatgcaggaaagtggattgccttcttacttcccgttccaggtagctgccgccggtcattgacaacaacaggttttcaaaagccgtattcatttgccccagttcataatgcaggtgaccgcaaagccggtatccttccatgatcataaaagcatcgcctttattcacggcttccagcgccagcgcttcatagagtgcaatggcctgttttcgtttcttcttgccggccaatatagcggcgcggatcatcacacaggatttccaggtgggataccctgcgggatcattcctgtccatcagctgcctcgacaaccggatggctttatcagcgtagcctgcgctcttatcggattcacgcgccatgaaataagcctgtgcggctatcatcataccagctacttcatgaggctcgccccccatttttttgctcagtgaaagcagcaccgatatttcctggtccagcgtgggtgaatcgggttgtgtggtacaatccatcactttacggatctgtttacggaaacgtgcatctacactgatggtgtcggaattgccaccgcctttatccatttcatggttaatagcggccaccatttgcagtgatggctgtaatatctttacctggtgggcaaatgttctcggtatggttatacgggaattagccgctatatctatcgtaacaagccggataccgtccggcagtccttttttcagtacatcggcataccaggcgcccgcatcgggctgctcgggtcttaagggagggaaataaatacagcacccggtttcttccagtccgcgcacacagcccataaaacgtcgcagttctttccagatgctttgtactgttggtgcgaggtggcggtcgggctgataatctgttttcagcagcccgtcttttttcagtgcactgtaaacatcatattcttcgcggggtacgggttcaaaccattccaggaattcattccacagcgactgttcatatgcctcgtgatcttcctggtaaggggaatcgaatctgaaaaatatctctttaaaaacaccaatggcggtacgttcggtttccaggaatttatcgataatttccacatccgcatactgtatcagccagatagccagtttccattggtgatcacggtcggcggcagcccatgtttcccttactttataaaactcctgcccgatagttggtgaggttgtcataagtgagctttaaggatcaggaatttattttcaccagcccgccggaaactactacgtcgccatgcccggtcacggtaacatcttttgtaccatttaccgaaacggaggcgccggtaacgttggcatttttgcttccggacgccagcaggtctttcgataacaaggtgagtgactctcctcctttcacgatcgcgtctttactgtttacggttaccgtttcggtgccttccaggtagattcctttcttggctgtgatagagccctgctcggaggctgcgatgctgaatttctctgaggttatttcaacttctttggaagatatggacatttttgttttggagaagagagacattttatctgtgccatcaatgaagatggtgttaccggctttatctgaaacggtaacgctgccatcggcatcattcagcaaaatggagatgccggtgcgggtacggatggctttcatgtcgttgttggcagtaccaaatcccgacttaccttccccgttataagtggttcccagcacgaagggaagttcggggttccctccttcaaaatccactaccacttcttcccctttttccggtaccatgtacatgcctttgctgccaccggcgtgcgggccaaccaccctcatccagggggtcatgccttgttgctgccatttgaaacgggcccttacccttcccaggtctttcggatcatgattgtccactacgatggcgctctgcgcctcacagaaaggcatattttccaggttcaccggcggagcggccgcatctgcagggataccttcaaactcgttgtaatagtcgccgttgccggttacgtgatgggtgaggccccagatcatgaatttcccatgatcatcttttgcatatacgttctcctggatagagatatgatctcctacgcggagcgcagtatgcctgctgctgcctttcagttgcaccatagcggccatacgtccttttttctgccgggttaccagcgtatccagttctgctttggcattgctggtaaaggcgtgggtcattttataggtggatgtattgctgtataatttttcgcttagtccctgtacatgcgaggtatagtcattgactttcccggcgggctgtgccaccgtggtattttccactactttattgttccggtagtcaaatccgttcaactgctgattgttgggttgcaccttcatttcgaggtcgaagctcatgaggtcaaccaggtgaaccaacgatacttcgcggggttggtatttcccaaaaaccaattgttgcccgttataaaaaaaccattccccgaaccgctcggagagccggtggaggaaatcaaatgatgtttctttgtattgcactatatacttcagcggcgatgtggtattggggtctaccatcgggcgtgccacatatgggccgcaggctttcagcgttgtgtttacaatagcgcccaggtcctggttttcaaaggtctgtacatgcaggtcgttactcagcagaatagtggggctgtatccgcggatcacgcaaaagccgtgggtgccgtcactttctttgcccgagctcacagacatcacaataccattgaaaataagcggttcatacgtttgtaattgttcaaaggcctgtatggtaatgctcacttcttttcccagaaatgctttggtagccgacactataccggggcccagttcctgcagccagtcgtagcctatttttagctcaaaatgatgatgtccctgtaactgttgttccaggcgcagggaatgaaattgtttaaactgtttgtcagcaatagatacggttgttatggtatgtaacatatacaggggggcttttaaattaatatggtcctatatctgatctgaaaaagctggatgggtgctgctgtataagcaactctcatctcaaaaaatacctgaaaaacgggttaaggaaatcctagttaacaaaattaaatttaaggaaatttatattacaaccccctcattttatggaaatggggaaaatattttcggggtcatttttgggggaagatgatcctgaagtacggattcctatctacatgttgtaacatccgcctgcttaccaggatcatccattcttcttattaatttttttgtggttgcacctgcaacccgtaaatatcttttaagcgcagcagacaaagttcttcgcctgatttcggaacgcctatcaccatttcgcagaacaactgaagttcctgtgagataacggtgcagttattttgctttaccaccatcatcacgtcgttcatgatggtatagtcgaagctgaggtggtattttgcttctatgtttttctggatcacggggatcagttgcagcaccatagcggcgctcatcttataagcgttgataagccccggtacaccgagcaggctgccgccgaaataacgcactactacaatgagcacatccgtaatctgtttactgtctatttgccccaggatgggcttgcctgctgagccggaaggctctccatcgtcgctggcgcggaactggagccccgcggtgccaaggcggtaagcataacagtgatgggtggcctttgggtgttcttttttcacctctgcaaggcattcttttacttcctccggcgatttaacaggaaatgcgtatgcgagaaatttgctgcccctgtctttgaactctgcgactgctgttttatcaattgtaaaataaacctccatcaaaataatttaatacgcgcttaaagctgcgcgggatgataaaaatcgatacgatcgcccgctacctgcagggtatgtgtgagcaatgcgttggtgagtaccggcgctaccagtccttccggtagtgtacccgtaccggttataacacgcgcctcatcccacaaaccggccgcaatgaattgctgcagcaccgcctggccgccttccaccaggatgctctggatctgccgcctgtgtaattgctgcatcagttgcggcaacagggcagtattgaaatccagtggcagggtttcggtaagaccgtgggtttccgccgatgcggcagtgataaagatggtaggaatgctgccatcccacacatgatgggaccgcggcactttcagatcccggtcaatgatcaggcgtaccgggtctttaccggtccacagccggttgttgagccgggggttatcatttatggcagtgcgggtacctgccaggatgcccatttcttcgctacgccatttatgcaccaggcggtcgctgtattgattggatatccgcacgggcgccccgcctgcgccggcgatcaggccattgctggtttgcgcccacttcagtacaatataaggccgttgttgttcatgaaaagtaaaaaagcggcggttgatttgccggcaggctgcttccagcacgcctgtttgcacctgtacaccggctttctccagtttttcaataccctttccggctactgctgaaaaggtatccacgcagccaatcaccacctgccggatgccctgtgatacgataagatctgcgcagggcggcgttttaccgtgatgcgcgcagggttccagacttacatacatggtagccagcggaatgagcgaacgttcttccggggccacgctgttcacacagttcacttccgcgtgggcctgcccgtactgccggtgatagccctccccgatgatacgcccctggtgtaccagcacggcgcccaccattggattaggcgctacctgaccggctcccatagcagccagttcaaggcaacgctgcatataaaattcattgaacgtgctattcataatcaccgcgcgaagtaatatttttgcaaaagtatcgtttttaacgaatggaaaatgccgctcccccaggtttgcacttttcctgtcacatgccttaaactgattatattgactatacaaacggcctttacctatattacaggcgccatcagtgaactatatgatgagcgggaagccgccaacatcgcacatatcataatggaatatctaacgggtatgagtaaactggacaggattgtccacaaaacaaaaatcctttcccccgatcagaagcaacgtctccaggcagccatagaagcgctgcaacgccatgaaccggtacaatatatcactggcaccagctggttttacggcatggaactcatagttaataaaaatgtacttattccccgccccgaaacagaagaactggtagaatggatggtgcaggacgcggcacaccgccaccggcttcacttgctggacgtaggcaccggcagcggatgtattccgctggcactgaaaaaatcactgccggatgcgcaggtatctgccattgatgtaagtgaaggcgcgctggaagtggcgcgcagcaatgcagcacgccaacggctggaagtggagttcctgcaccttgatgcgttgaaccctgaacagatggccggtttaccggagtttgacatgattgtgagcaatcccccgtatatcacgcagagtgagcaaacctccatgcaacagttggtttggggcttcgagccatcactggccctgtttgttcccgataatgatgccctgctgttttatcgacatatctccgaaatggcacattccaggctggttcccggcggcgccctctattttgaaatcaacgaggcgctgggaaaagaagtagtggcactgatggaaagtatcgggtttaccgcagtaacgctgaaacaggatatgttcgggaaagacaggatggtaaaaggaaagaaggcataaaataaaaaagacctggtggtatcgcaccaccaggtctgctatacattaaaggcattattacttatgagcggtggccagtactactttggctcccatctccctggccacttccatcacgctcactacatcttccaccggtacagatttttccgcattgataacaatggtgggatcaatcttttcattgccgatagaaggcgccagcgcctgtttcaggtgatcaaaggttactttattggtgcctacaaaaaactcgcgtttatcgttaatactcactactaccgtttgtttcgacttggtattgctctttgcttttggcagcagcagtttgatcacattcggattagccagggtggaaacaataaggaagaacaacaacagaatgaacaggatgtcattcagtgctgagttgtgcatttccacctgtctcttatttcgtctgcgtaaattcatgagggtggttttagcgggttggttcctgcaaaatatcgatgaattcagcagaagcgccttccatcttgtttactaccttgtctatctgggcgttcaggtaactgtagccgataaaggccacgataccgataattaaaccggaagcggaagtaatcatttttacatagataccgccggcaatggtgcccagtgtgatatcagaggtgatggagatattaaaaaaggtttggatcatccctgcaatcgtaccgaggaagccgaacataggggcaatgcctgcaatgatagacaggatcaccaggttcttttccatccggtaaatttccagcttacccacattctccatggatttttcaatattctcaataggcttgcctatgcgctgaatccctttctcgatcatacgggcgattggtccgtaggtattttttgccagcgatctggcagattgcatgttacccgtggtgatctgatcacggatcatgggcataaagttatcaggcaaccggccggctttactgatggtgatggccctttccacgaatacatataccgctatcagcgaaagtattcccagggggatcatcagcacaccgcctttcatcagcatatctatcagatggatttccggcgccggggctccggcagcaccagctgccagggctgctgaatcagccggaagagacgataaagaatcctgtaataatgtaataaaacctaacaacatgaactatattttaacgggtgcataagtagaacactactataaacggttaaagtaataaaatatttgcgaatgtgcgcggcaatattttacgccttctcttcccaaacctgtgccagatacacaattgtttgcacggctttctgcatatcctgtatgctcacgtattcatgtttgctgtgaagcgccatttcaccggtaaaaatattggggcacggcaggcccataaacgacaggcgggaaccgtcggtaccaccgcggatgctcattctcaggggctgtacacctgcacggcgaatggcttctgccgcattggccgttacctcggggtgatttaccagcacctctttcatattgcggtattgttctgttactttcagcgtggcctttgcgccatggtgctttgccagcaccttatccatgatccggcgcaggaaagtttcatgtgcttcaaggtggtcagtttcaaaatcacgtataataaaatcgatctccgttttttccacagtgccctgtatgcgaaccgggtgaataaagccctcccggtcgtcggtggtttcaggggaaagaccgtctttcggtaacgcatctacgatttcaccggctattttgatcgcgcttaccagtttatcttttgcagcacccgggtgggcgctgatgccatacactgtgatcctggcgccgtcagccgaaaagttttcatcttccagggaacccagttcaccgccgtccatggtataaccaaaatctgcggccagcttcttcatatccactttttccacaccgcggcccacttcctcatccggagtaaacaggatgcggatagcgccatgcttcacttccggatgcgtcatcaggaagttggcggcatccatgatttcggccacgccggccttatcgtctgctcccaggagcgtggtgccactggctgtaataatatcgtcgccttttttgctggccaggtaaggatgttcttttgcactgatcaccactgtttcatcgtcgggcaacacaatatcgccgccattatactggcgatgcacaattggcttcacgccggtgccgctgctgtctgaagaagtatccacatgtgaacaaaagcagatcaccggcacttttttgtcggtgttggccggaatggtggcgtatacataaccatgttcgtccagtgctgcatcggtaatacccatttcctgtaattcctttaccagcaaccgggaaagatccttctgtttttccgtggtaggaaaagtgttgctcatcgggtccgactgtgtatctatctgtgcgtaacgcatgaagcgtttatctactgtatatgagtaatttgtaaacatattgcaaacgtaaggaaaatcatcttcacactcctgccgtagattattctgttttaccatctctcacaatatcatcaacagtaaattattcttcaaaatgctacttttttaagacaaaaaaccaaaattaaccggaatgatcgaacaaacacctaataataataggtttgtatagaataaaatacatcctatatatgctaaccaacattccaggctatccgagaataggtagccagcgtgagctgaaaaaagcctgcgaaaattactgggccggaaaaatttcactggagcgtcttgagctaacgtcaaggcagctacgaaaagaaaactggagcgggttacagcaagccggtattgacctgatcccttccaacgatttctcctggtacgaccaggtactggatatgtgcatgaccctgggcgtaattccttcgcgctttaaagctttgcagcaaacatttgccaacccgggctgcccggagctgtatttcgcgatggcaaggggttaccagaaaaataacttcgatatcaccgccctggaaatgaccaaatggtttgataccaactaccattacctggtccctgaatttgaatccgctcagcaatatacccttcaccagcccaagtgtgtggaagaattcaaagaggcgcttagtcatggtatcaccaccaaacctgtactcatcgggcctgttacctttctcttatgtggaaaaattaagggagatgaccttacgcacgcgcagctgctggaaaaactgctgcccgtttatattgaattgctaagatctcttcaacaggccggcgctacatggatccagctggatgagcctttcctggtgaccgacctggaccccgccaccagagacctttaccaggccgcatataccgctatcagccaggcattacctgcgctcaaagtactgctcaccacctattttgggacgctggaagacaataccaccctggctttgcagctgccggtgcaggcggtgcatatcgacctggtaagggctccggagcagctggacaccgtactggcggccctgcctgcagataaaatgttgtcactcggtgtagtggacggacgcaatatctggaaaaatgattatgccgcttccattgcgctgattgaaaaagcaatagggcaaatcggcgaagaacgggtactgctgggtacttcctgctccctcctgcatgtcccctataacctggaagatgaaaccgcattagaccccggaataaaacagtggatggcttttgccaaacagaaagtagccgaggtaatagcgctgaaacacattatagccggcgatacttccctgcttgtggataatgaagcggtgatgaacagccgcaaaacttcctcccggatacaccggccggaagtgaaagccaggctggaaagtattaccacagcggatacacagcggcacagcatcttcccgcaccgccagaaattacagcaatcggtattacaacttcccctgtttcccaccactacgatcggctctttcccgcaaaccacggaaataaggcaactccgcgctgatcttaaaaaagggatcatcacaccggaaacttacaacgccgatatccgccatgccattacggaaaccatttaccgccaggaaagcctcggactggatgtgctggtgcatggcgagtttgagcggaatgatatggtggaatattttggcgagcagctggacggatttgtatttacccaaaatggttgggtacagagttacggtacacggtgtgtaaaaccaccggttatttttggagacgtacaacggccggaacccatgaccattgcctggagccgttttgcgcagtcgctgaccaataagccggtaaaaggcatgttgaccggccccgtcaccattctgcaatggtcgtttgtaagaaatgaccaaccccgtatgcaaaccgcgatgcaaattgcactcgctatccgtgatgaagtgaaagacctggaagatgccggtattacgatcatacaggtagatgaacctgccctgcgcgagggcctgccgctgcgtaaagcacagcgcgccgcctatctggaacaggctgtgaaagctttccgcctggccgtaagcacggtggatgattccacgcagatccacacgcatatgtgctatgcggaattcaatgatattattgagcacatcgccgcaatggatgcagatgtgattaccatcgaaacatcgcgctcacagatggagctgcttgaagcatttgcaggatttaaatatccaaatgaaaccggtccgggtgtatacgatatccactcgccaagagtaccggcggtggcggagatggaggcattactgcacaaggcggccgcgttactgccgctgcgcaatatatgggtaaaccccgactgcggattgaaaacgcggaagtggccggaaacggaattggcgttgcgtaatatggtaactgctgcaaagaatgtgcggcaggcggtgagcaactagcgccgggggcgttgggtaaatgcagcgaaaaatcatctgcgctgcatttactgaatgctgtgtaaaatccgtaattttagggatggcatgtcatgaaaccgtaacctgtccgcggtgcgaacgcacctttgaatgccgcgtaggcactattctgcgctgtcagtgccaggatgtggtgttgagtgaagaagagcgatatttcatccagcaaaaatacagtggttgtctttgtgccgactgtttacgtgatatgaaaacaatttaccagcaaccggaaacatcgtcctgaaactgtttcccttaatgggtttccgccgttgttccatctccctgaaaatcaggcagcagcataaaaaaatttacggatgcaagggtagtgttatccaccggttcctgcatccgtaaatcaaaaaaataactgaatattatgcgatttcaaccagttcgaggtcaaataccaggtcttcgccagccagcgcgtggttagcatccaaggtaataaattcgtcgccgatagcggctacttttacctggaaaacctgtccctgaggattgctcatctgcaattccatacctacttcaggattcagatcagccgggatattttcttttggaaaatccatgatcatttcatcacttttgggaccatatgcctgatcaacagggatatgaatggttttcttgtcgccaactttcatgtccagcacaccattctcaaaacctttgataaccataccggcacctaccttgaattcgagcggagctctaccttcggatgaatcaaaagtagttccgttcgttaaacggccatggtaatgcaccttcactgtatccccgtttttaacagtttgcataaaaattaattgtttagtgttaataattacgcgcaagatacaaaaagcagccataatccgagctttttgatacagtcaataaagctttgcattatcttaacggtatgaaccgtattctccttctttgcatcttcctggcaggatgtatttatgaaacctccgcgcaatatgcggaccatgtattgccaggcgccacgcaaacagcgcgttaccttccactgctgaaaaacaagcgggtagcgatgatggtgaatcaaaccgccaccatcgataaaacgcacctggtagattccctgttgaaactgaatgtaaaaatccagaagatctttagtcctgagcacggcttccgcggcaatgccggtcatggcgaaaaagtggccaacagtatcgattccgctaccggcattcccattgtatcgctctacgggcaacaccgtaaagctaccgcagccgatctgaaagatgtggatatcctgttgttcgatatccaggatgtgggtacccgctttttcacctacatttcgtccctgcaggaactaatggagtccgcagcggaaaataaaaaaacactcgtcatactggaccgccctaatcccaacggcgactatgtagacggtcccatcctcgataccgcctaccgttcctttattggcatgcaacccattcctattgtgcatggcatgacggttggcgaatacgcccggatgctgaacggcgaacgcatgcttcgcaacggcgtgcagtgcgatatcaaagttattccctgcgaaaactacagccataaaacattttaccgggtacctatcaaaccttcacccaacctgcccaatatggccgctatcaacctgtattcctccctctgcttttttgaaggcacggcacttagcctgggacgtggtaccgacaagcctttccaggtgtatggctcaccggattttcctaaaaagggttactcatttacgccccgcgccagcgctatcaatccaacgcctgtgctgaaagaccagctgtgctacggcttcgacctgagcaatgcgcctgaagccacgccgcatgccggccgtaaaattgaattgaaatggctgctggaggcctatcgcatgttccctgataaatctaaatttttcattcctttcttcagcaaacttgccggtaacaacatactacagcaacagatcgtgaaagggctgtctgaagcagagatccgcaaaagctgggaacccggactggcgaagtttaaggttataagaacaaaatacctgttgtattaaaaagcagaagggatagctttccgctatcccttcgctaaaatccgcgaaaggtcgttatttttgcatcctatgagtaaagatcttcgcattgtttttatgggtacccctgattttgcagtggcctccctcgatatattagtacagaacggatttaacgtagtgggtgtgatcacagcgcccgataaacccgccggtcgtggtttacagctgcaggaaagcgcagtgaaacaatacgcagtaagtaaaggacttactgttttacaaccggagaaactgaaaaatcccgattttattgcagccttaaaagacctgaaagctgacctgcaggtagtagtggccttccgcatgttgcctgaaatagtatggaatatgccgccggaaggcactatcaatgtacacgcctcgctgctgcccaactaccgcggcgccgcgcctatcaactgggctatcattaacggcgaaaaagagtccggcgttaccactttcaaactacagcatgaaatagataccggcgacatcctgtttagcgacaaagtagccatccgtgaagatgaaaccgccggtgaactgcatgatgccctcatgcaaacaggcgcccgcttactgctgagaactgtacaagccattgctgccggcgatatcaaggaaacaccgcaggccaatattcccgcggcagcaataaaacatgcgccaaaaattttcaaggaaacctgccagatcaactggcaggagccattaaataacatctacaacctggtacgcggccttagtccctaccccgctgcctggactaccttccagggcaaaacgctgaagatatacaaagcccataaggaacttactacacccgcaaaagcaccgggcgacttcgacaccgatcaaaaaacctatataaaaatagcagcgccggacggttatctctacctggatgaaatccagctggaaggcaagaagaaaatggatgtggagtcgttcctccggggttatcgcttctaatcgcgcggattttgtcttggctcaggattacgctgattatactgattactcggatttttacttttggatttttttggatttttagattaataattaagggagataagagcgaatatatccgcttctatctcccttaatcctttataaaatccaaaagtaaaaatccgagtaatcagtataatcagcgtaatcctgagaaagacaaaatccgcgatcattaatcctcgtagctcagttcgcagtagaacttcgtttcgttgctgccgagtgcctgcatggcgctgtcgctcaacttgatgatgaggcctgcattggctttcatctgtggtattacgtccagtactttggcgtataccgctttgccgttgagagggttggttactttgatgatggtgccgcgtggtgcagtgttgtgcagcgcatagtatttgcctaccgcattgctcttaaaccaggtaccagggcccttttcggaagtagttttcttgccgttattggtttgctgctcatacaattgttcaaaatcagtgctgctgctaacaggtgcagttttaaccggggcaggcgcaggagtttctgttacttctgctacggggcgtgtttcaggttctttcttagctgtttctttttctaccggaggtgggggtggtggtggtgcttgtgtaaccactggttcaggcgccggtgtggctttctcctttactttttcagggcggggagttgcttctgcggcagctccgccggctttcataaagcccacaactatgtagctgttttttttgagtccatctccggaaaaattattccattgacggatattatccagcggcactttattgtagtttacgcttacacggtataaagtttctttttcggatactttatgatatacgggtttgccggatgcatccgccttttgtgagaaattggcggtagtgagcgggatgtgaagcttgtggccaagctgtaatccctgttccatattcactttattggccgcagcaatttccttcggtggtaatccgtaagcgcggctaaggctataaaaattttctccttttttaacaacatgggatatatagagagcgggggaagtaccttgtacttccagcgtgtcctgcgcctgcgccgccgctgcactaaaaccaaacaagacgattgatagaatcgattttatcatactaactctgtttatgatggatatgctgactactgctctctttcattttacggaaacatctgttccgcaaagcatattaatccggtatcacagcagcagcagatcctgaatttttatctgctatttcgggcaacgaatatatgcgttaaaattgacaaaattatttaataaaccaaacggagaaaatccctttttgttgtggccaccggtataaacggcgccccgttggcactgtatttcaaagttggtatcattcccggataaatagcgcccggctgttttttacaccccggtaatttctttcaggatgcgcaattctttggggtagtaattgttcatgcggttgggtaaaattttcgcccagccgaggttcatgtcctcatatcttaccagtgcccagccacgcacccttgtattcactcccggatcctcctttctcaggtattgtaatgcctggcgcaaatccagggataccaccggcagttcatcggataccaatgtactggctgccagctgatgatccggaattaattccttcgcactgggatgccccgcttttacacccgccttgcgaatatacaattgttgccgcaacaatggtatttctgttgccaccaaaggtggcaaaataaatacttcttcctggtgcatgaaatactggtagttgtcgggtatatctatccagggggtaatcacttcctgctggcgggcagttaatgctgttgatttatgctgcttcggtttacgcggagtttcgctgctgcgcttacggaaggcagctataaaaaacccttctcccttcagtttgtccgggtaaaaccggtaaccggtacaatttcgtttgtgcgttaccgttgtaacaatactccattccgggttcagggtaaccgggatattttccagttcaaaatgatccgccagccaatccaggatcgcttcatcttcttctgcagaaaaagaacaggtggaataaatgacaacgccgccttcttttacacttggcagcatatctgccataatcctttgctgccgctggctgcacagcgttacattttccggcgaccattcctccaccagttccggatcgcgacggaataaaccggagccggagcaaggcgcatccactactgccaggtcgaaataaccaggcaatcgtgaaaagtcacgcggatcattattactcaccactacattcgcagcgccccattttgtgagattgtctgacagcagcgcagcgcgtggcttaattacctcattggctaccaacaggctatcctggctgatcagggattgcagtaaagtggattttccgcccggagcagcgcaaagatccaacaccttcagtggttgcgaaagatccactgttgcccgcaccatttgttccaggaacatagaagatgcctcctgcacataataagcgcccgcatgaaaataaggatcaaaagtaaaggaaggccgctccggtaaataatatccctccctgctccaggggaccggggtggcgccggtgacagacaaggattgcagtacggctgccgcccgttccggcgtttttattttattgggattcaatcgcagtgaagtaatcttttcggcggcggcatgcacctgctcaaatgtttcccggttataacccggaagtcccgctaacgaatctaatagcgctgctggtaattgactggacaaaggaaatttttttccgcaaatttagcaaaaatgcggagatatgagcgtaggttgtctttctcgctgattacgctgattttactgattaactggatttgatcacgttggattttaaaggatttggggagatggaagcggattttgtctttctcaggattacgctgattttactgatttagggatttgatcactttagattttaaaggatttgggtagatataagcggacatattcgcttttatctacccaaatcttcttaaatcctttataaaatccaaaaagtaaaatcaaacaaatcagtaaaatcagcgtaatcctgagaaagacaaaattcgcgcgttagacctccttgatagcggaaagtagctcctgcaacaccttcttggcgtcgccgaaaagcatggaggttttgggttggaaaaagaggtcgttttcgatacccgcatagccaggtttcatactgcgtttattgactattaccactttggcgttttcaacttccaggataggcatgccgtaaatagggctggcgggatcgcttttggctgccgggtttaccacatcattggcgcctaagatcaatactgcatctgttgtggggaattcggcgttggcatcttccatttccaacaacttttcatagggcacatctgcttcggccagcagcacattcatatgcccgggcatacggcctgctaccgggtggatcgcatattttacttccacacctttctcttccagctgcttctccaactcgtgacaggcatgctgggcctgtgccaccgccaaaccataacccggtacaatgatcactttattggcatatgccagtactacggcggcatcattcaaactaatttctttatagttgccctgctcctttccggaggcagcagcgccggtcgcaccaccgccgaaagagcctatcagcacgtttttcagggagcggttcatcgccttacacatgaggatggtgaggatagttccggctgaacctaccaggataccaccggtgagcattactggattactgtacaggaatccgccgcaagctgcggctacgcctgtaaatgaattcaacagggaaatcaccaccggcatatccgccccgccaatcggcagcacgaataataccccatagaacaacgccagcaggaaaataacataaaatacaacgatgcctgttccaggcgacaaaccaaagacacacaccagccaaacagacagccctactatcagcgccaatatgcccatgttgaggaagtgctgtccattgaaggaaaaatccttcacctttccggtgagctttccccaggcaacaatgctgcctgcacaggataccgcgccaatgatcaggctcagcaaaatgatgatcaccattcctttggatgcagacgactccagtaactgaagtgccagatgatcgtcagaaacaggtgcatataaattctttatcagcttgatcaggtggtcaaattccacgatagaaataagcgccgcacatgcaccgcccatcccgttgaacatgcttaccatttctggcatcgccgtcatcttcactttctttgcggacaacacgcctattacaccaccgatgaccagcccggtgaatatccagccataattatgcaggggggcatcatttacccggtagagaaagatagtgccgaggatagccagcgacattcctgcggcagccaccagattgccttttcgggcagtatccggtttacttaacattttcagtccgaggataaaagtaacagagccgatcaggtaaataattgataaaatgctggatcccataagtattatacttttagccgttagctatttctttttgcctttgaacatttccagcatacggtcggtgactacaaaaccacctaccacattgatcgtacccaggatcaccgccaggaagccgatgatcagcgcgggataattatccgcttcggccttccccatcacaatgatggccccgataattacaacgccgtgaatagcgttggcgccgctcattaatggtgtatgcaatacagacggcaccctcgaaatcacttctattcctaaaaaaacagacaggataacgatgtagataagatcgatatgctggtgaagaaaagttaaaatatattccatatcagacgggtatttttacgatctcgactactaagctggctgcatcaggtttttcacacggtcattcacaatttcaccgttgtgcgtaatacaggcgcctttcacaatatcatcttcaaagttcaggtgcaacgctccctcttttgttaatatcagtttcaggaaattgaatagattctttgcatatagcttgctggcatccgccggcatagtggcaggcaggttggaattcccgatgatggtaactcctttgtactgcacggtttcattgttctttgtaacgccggtgttaccacccgtagcggcggcaagatctacgatcacagaacctgcacgcatgcgatccagcatttcactgcttaccagcacaggtgcggctttacccggaatctgcgcagtggtgatcacaatatctgctttcgcaatgctctccgcaatacgttgttgttgctgctgcttataggtttcgctttgttctaccgcatagccgccggcggaggaagcatctgccgctccttccacttccacaaatttggcacccaggctcatcacttcttcttttaccgcaggcctggtgtcaaatacttccactacagcgcctaaacggcgggcagtggcaatagcctgcaaaccagctaccccggcgcctaatatcaatactttagcgggagcaatactgcctgctgcagtcatgaacatgggaaagtaacgggaatagctatacgcagccagcaataccgccttataaccggctatattggcctgggaactaagcacatccattacctgcgcacgggtggtgcgggggatggtatccaggctgaatgcggtgatgttacgggaagcccagtgctccacttcgtttacacggtacagcggttgcagaatacccgcgataattttcccggaagggatctggtctgttatttcttttgacggaggctgcagcgtaaagatgatatctgccccggtgagaatgtccgcagctgtttttatttccgcacccgcctgcatataggcgtcgtcgttataaaaagcattgtcgccggctccctgctccacccacacggttaccgacatttgctgcagttgctttactacttcagggacaagagacaccctggtttcgccgtttttttcttttaaaattcctgcaatcatctggtggaaatttataatggaatttaaagaaaaaacggcaacaacgaactatttttctgtttaatttttcttcagcgaagcggccaaagcagccgcatgttgcagtaaagccgggatggctacgccttgcaggtagtttcctgcaatatgaatacctggatattttttttcaaagtctgttacggcattccgcaacttaacatgaccaacattcaactgcgggatagccttattccaggtgctgaaccgctgcatcaccggcggagccgacaggtgcagtaaagtctgtacttccgaaaccacctgctgttgcaaggcttccggagccatctggtcaaacaggcgctcctgcctcgctcctcccaggaataccgtaaacaggatttttcctgcaggcgccttatccgggaagatagcagagttgcagatagcaccgaggaaatgcatattttctgcattcggcaccaggaaaccaaagccttccagcggctgtggcagcgcagcagcgtcgaagcccaggtgcagcacgcccatgcggggataatgaatgttgtttaataaggcggcggtggccgcatcaagttgggtgatggtttctgcggtgctgtatgcgggagtggtcagtacaacttttgaagcagcataactttccgaaacaccgttctccacagcactcacaatgtacccgccattggcagccgtgatgccggttacgttgcaattaaagcgtacaggggtagtgagcaactgttgtaaacggtttgtgagcagctggttgccgcctttaaagctgataattttccggccacccatagcgcctttatctttcatcagtcctttcgttacgctgccgtattcccgctcccaccgcgggagggcaggtaatacttccgctacgctcatcagatcgggattaccggcataaatgcctgataataccggatcaaaaacatattcagcaatctctttattaaatcttcttgttacaaaatcactgacggtttcttctccagatacggttgccggtttacggaagcgctctgtaaacagccgccacttgctgctccggctgagatacggggaagccatgatcttaaaagggtggggagaaactgcatgcagttgttttcttcttaccaggaagcggttcttgctggcggcagcagcggtcaggatttccttgtccagccccagttctgtaaagtattgcagcaattcaggagaggctgcaatggtattggcgcctgcatccagctcaaaaccatcttcccgtatagatttgattacgcccccgctatgatcggaaacctccagtacctggtagggcacctgcagtttctgcaattcatatgcaatgctcagcccggacaggccggcgccgacaatcaatacgggttgatcggacatatgttaaatttaaacggcttcggttgcgattatctgcgtgcaatatttaaccactgcttttacccacaacgggtgaatattcaaacacggaatcatggtgaaggattcaccgccgctgttcaggaaagaatgcttcccttctactgcaatctcctccagcgtttccaggcaatctgatacaaaagcaggacacacgatcaacagtctttttttgccttcagcgggcaatgtttccagcaaacctgcggtgtagggcttcagccactcttcacggcccagcctcgactggaaagagatgccccatttttcccgcggcagtcccagcttttccgctaccagctcagtagtcactgtaatctggtgacggtagcagtagtcatgtgcgggcgattttacatgacagcagtcgtttaccttcatacaatgagcgccggtaggatcagctttgcgcatatgcctttccggtaacccatgataactgaataatacgtaatcatagtcctgctgaagatatgggcgcatgctttctgtaagtgcatggatatagtccggttcatcataaaacggcggcactaccgatagcttgaatttgtattttttctttttgtagatttcctgtgcgtattccactgctgtttcataagaagacatggcataatgcggatacaacggcaacagcactacttctttcaggtcaggattttgtttgagcaggttgtcgtaagctacctgcggatgcggattaccatagcgcatagctatttccaccggaatctccatgtcgttctgcaccgccatctgcagctgctttgttaaagccaccaatggtgatccttcttcccaccagatagattcataagcccgggcagattgctccgcacgcttaggcacaatgataccttcaattaagatcttgcggaacaaccacggatagtcaattacacgcttgtccatcaggaactcattcagataacgcttaacatccggcacggcggtagaatcaggcgatccgaggttcattaatactattccaacatcagatttagataccatttcttttaaattggtgcaaaagtaagcaaaaagccgaaagcgaaaagcattatagtcgccacgcagcctgcacgattagtgtcattcttttgtaaaggcaaaacctgataaaaatcattttttcgtcgtaatgattaccagtagtagaaatgacacactaatgacagctaaccccttttgtttgggacgtatgaaagtacttttgcaaccggaagcttatacaaaatcatgcaggtcagtcattcaaaagaaatagcaaattttcatatcgttggcatcaactataagaaaacagacgctgctatcaggggattatacgccatcaatccggctcagtatcaacaactcctggagcatgccagggtagtgcaattagacgatctttttgtgctctctacatgcaacagaacggaagtatacggatttgcagcgaacccggggcagttgttggatttgctttgcagggaatcaaacggcgacagaagccagttggaagaattagcttataccaaatcgggagaagaagctatcaggcatttgtaccaggtaggtacaggcctcgactcccagatcctcggcgactacgaaatcataggtcagatacgtaacgccactaaatttgccaaagcgcatcacagcctcggcagcttcctggaaaggcttgttaacagcgttttacaggtttccaaactcatcaaaactgaaacaggactcagcaaaggcacggtatcagtggcttttgccaccgtaaggatgctggaacgcatttgtcctgatataaaagataaaaagattgtattgctgggtgtaggcaaaattggccgcaatacctgcaagaacatgatcgaatacctcggcgtaaaagaagtaacccttattaaccgcaccctgcaggtggccgccgaattcgccggtcagcacgggctgaaatacgctcctatcgaagatatggtcagcgaaatgcagcgggcagatgtgatccttgttgcttccaatgccccgcatccgacggtattggccaaacaccttggcaacacttctcccaaactcatcgtcgacttatccattcctttcaatgtagaagctgcagtaggtgaactcccgcatatcaccctggtgaatgtggatgaactctccaaagtacaggacgaaaccctgcaaaacaggctgggagaagtaccaaaggcgatctccatcatcgatgaacatatggaggaattcctttactggtataaaatgcgcaaacacgcggtagtgttgaaagccgtaaaagataaactgcaggaaatacatacccgcgaaatacagcaacagaaaaacggaggacactacaacatggaggatatcgaactcgtatcttcccgtatcatacaaaaaatgattaatctcatggctggtaaagtacgcaaggaaacagacaaaagtgaccagtacatcgccatgatcaacgatatttttgagaccggagttaaccaggaataaacaaatggataaagttatcaggataggcacaagagaaagtcagctggccttgtggcaggcaaaccaggtaaatgatctgctcaccgcacaaggttaccgtacagaactggtacctatcaaaagcgaaggagatatagacctggtaacacccctgtatgaaataggcgtacagggtatcttcactaaaagcctcgatctggcattgctcaataaccgtatagacattgccgttcactccttcaaagacgttcccacacaactgccgaaacaaattgtgcatgccgctatcctgcaacgcggaccggtaaaagatttgctggtatacaaaaacgatacaaatttcctttcacaacccggttatatagcgaacatcgctaccagcagtgtacgccgtaaagcccagtggctgcggaaatatccacaacaccagctgcataacctgcggggtaatgtaaatacccgcctgaagaaactggcggaggaaaactgggacggcgccattttcgcggtagccggactggaaagaattaacgtccgtcctgccaattccattgatctcgactggatgttaccggcgcctgcacaaggtgcagtggtgacagtttgcagggaagatgatcagttttgcctggatgcctgtgcagcttttaaccacgcagaaaccgcactcactacacatattgaacgcgaatttttacgcacgctgatgggcggatgcaccacccctatcagcgcttacgcatatatacaaaacaatcacatacatttcaacggcgaactgtgtagcctcgatggcgcccggttcttctctgtttcacgcgaagtgccactggaacaagccaaacacctcggacaggaagctgcggaagatattatggcccagggcggcgctgaaattgtagcacagatcagaaatgcaaaatgataaataccgcatattaagcaccaggcatttaacagacagctctgtggctgttgctggtgaaagtggtattcacatagatgtacaggattttatacagataaagccgcttaaaaatgaaatgctgctgggcgaagagcgtttgctgcaggtgttccggccggaaacagtacatgtgttcaccagtgccaatgcagcaagaatactggataaatactatctccaccaggatgatacgttttatgtgatcagcgagccaaatatctgctgtatctccggcagcacgaggaaagcagtggaaaacgtgttcactgattgcaacatcttagcggaatcgccctatggcagcgaacttgccaggataattatacaacttgatataacttccgttaacttcttctgcggcagtatccggagaaacgaattaccggataccttacaggaagccggtattgaagtaaaagagttcgtgatctacgagaatattcctgcgccggccgtaatagcggaccattacgacggcatattatttttcagtcccagtgcggtaaaaagttacctgtcggccaaccggctaaacagtaaaaccgtttgcttcgctatcggcagaacaactgccaccgaactgcgggaacataccgataacaaaattattatcagcaccgatatcagcgaagaaagcatggtgcaaactgctatattttattttaacaacattaactgctacgaatgagcgcattgaagaacgacttattgctgaaggcccttaaaggcgaaactgtttcccgcacaccggtatggatgatgcgtcaggctggtcgctatttaccggattatatcaaactgcgtgataaatatacgttctttgaacgctgcgaaaacccggagctggcaacggaaataacggtgatgccggtagaccaggtaggcgttgatgctgctattatcttttccgatatcctggtagttccccaggcaatgggcatggaagtacagctggtggaaaaagtaggaccactcctgcccgctcccattaaaaccgcgcaggacctgcagcgtttatgcgttcccgatgtacaggaaagattgcactatgtatttgatgccctgaagctaactaaaaaaacactggatggcagggtgccgctgatcggctttggtggcgctccctggaccttactctgctacatggtgcaaggcaaagggtccaaaacgtttgatgaagcaaaagcattctgttatcagcaaccggctgtagcacaccagctgttgcagatgatcaccgataccaccatcgcttacctgaaagcacaggtgtccgcaggcgccgataccgtacaggtatttgactcctggggtggattactcagcccgcaggacttcgaagtattctctttacaatatatccgccagatagtagccgcgatgaaggatgtttgtccgactatcgtatttgcaaaaggcgcctggtttgccctggaagatatggccgctaccggcgcgcatggactgggcatcgactggtgtattaaaccggaactggcccgccagtttgccggcagcaacatcaccctgcagggaaattttgacccggctaaattgctggcgcccatccctgaaattgaaaaggccgtaaaggaaatgctgaaaggctttggcagacagcgttacattgccaacctggggcatggtatcttaccaaatgttccggttgatcatgccaaagcatttgtggaaacagttaaagcacacggataattaaccatgagcatcaaaaataacttcatatcattcatacatggcctgcaggataaaatctgtgccgcgctggaaaaaacagacggcaaagctactttcctggaagaccgctgggagcgtcccggcggcggcggtggcaaaacacgggtgattgccaacgggaatgtatttgaaaaaggcggcgtaaatacttcggtcgtgcatggcgaattgccggaagcaatggcacaacagttcggcgttaccaacagccagtttatggcatgtggtatttcgctggtgcttcacccggtgaacccttttgtacccaccgtgcatgcgaacttccgctattttgaattgtatgaccaggatggaacactgaaagacagctggtttggtggtggtgcggatcttacgccctattaccttgaggaagaagacggtattcatttccaccgtacctttaaagatgtctgtgatccttttggaaaggaattgtatccggcatataaaaaacactgcgacgaatattttatcaataaacaccgtaacaacgaagcgcgtggaataggcggtatcttttatgattacctccgtcccaacgcggaaagaaccgcagaagaactcctgaatttctcaaaagcaaatggaaatgccttcctcgaagcatatcttccgctggtagagaaaacaaaaaacctgccttataccgatgcacataaaaactggcaggcgtataggcgcggacgttatgtagagtttaatcttgttcatgacaggggaactttgtttgggttgaaaacaaacggccgtacagaatccatcctgatgagcttaccaccggtagcccgctgggagtacgactttcatcctgcacccggcagcccggaagcgcagctggaagaatacctgaagcccagggaatggataaaataacaagcaggcagacgacgatataaaaacaataaaatttttataaagatgatcagaagaaacagaatattaagagtatctcccgctattcgtgcaatggtggcggaaacaattttaacacccagcgattttatagcaccgttatttgttaccgaaggagaaaatgtgaaggacgcgatcagctctatgccaggttatttcaggtactccctggaccttactattaaagaagccagggaactctggagcctgggtattaaaagtgtactgctgtttgtaaaggcgcccgacagcgtaaaagataataaaggcaccgaagcagtaaaccccaacgggttgatgcagcgcgccatccgtggcattaaaaacgccatccccgaaatggtggtgatgactgacgttgccctggatccctattcttcctacggccacgatggtattgtggaaggaacagaaattgtaaatgatcctactgtagaagtactggcacgcatgagcctgagccatgcacaggcaggcgccgactttgtagcgcccagcgatatgatggacggccgcatcctggctatccgcaacatcctcgaagaaaatggcttcgataaaacaggcatcatggcttacagcgctaaatacgcttcctgcttttacggtcctttccgtgatgcactcgactctgctcctggcttcggcgataagaaaacctaccagatggattatgctaattcccgcgaagcaatccgggaaacactgatggatattgaagaaggcgccgacatagtaatggtaaaacctgctatggcttacctcgacattatgcgcattattaaagatcgtgtaaccgtaccagttagtgcttatcatgtaagcggcgaatacgccatgatcaaagcagctgcagaaagaggctggctggatgaaaacaaggccatcatggaatctatgaccagtatgaaacgcgcaggcgcggatctgatcgctacctactttgcaaaggatgcggtaaaactgctgaatgcataattccctatcttgcgtaaaataataaaccacgaaacagatgtacagtaaaagtgaaatgttattcgggaaagcaaagcaggtaattcccggcggtgttaactctcccgtacgtgcatttaaaagtgtaggcggcacgcccgtatttatggaacgcgccaagggcgcctatatgtacgatgtagatggcaaccgttatatcgactacatcaattcctggggcccaatgatccttggccacgcatatgagccggtagtaaaggctatacaggaatatgccacctactccacatctttcggcgcgcctacagaactggaaacaaagatcgcagaactgattacaggcatggtgcctaatatcgatatgatacgcatggtaaactccggtacggaagcctgcatgacagccatcaggctggcaaggggttataccggccgtaataagtttatcaagtttgaaggttgctaccacggtcacgcagatgcgttcctggtaagcgccggcagtggcgtagccaccctgggcattcaatccgtgccaggcgttaccactgcagtagcagaagacacgcttactgccccgtataataatttacctgcagtagaacaactgattgccgataacatcaaccagattgccgctgttatcattgaaccggtagccggcaacatgggctgtatccttccgcagccgggcttcctggaagggctccgccagctttgcgatgccaacaatatcctgctcatctttgatgaagtaatgacaggcttccgtttggcccgtggcggtgcacaggaattactgggcatcagggccgacctcgtaacttttggtaagatcattggcgccggtatgccggtaggtgcagtggccggtccgaaagaaatcatggaacatcttgcccccgccggaaaagtataccaggcaggcacattaagcggtaatccgattgcaatgattgccggttatactttattgcaaacgctgaacgataatcctgttatttaccagcaactggaagataaagccagctacctggtgaatggattaaaagaagcatttggcgctgccggcattgtgcatagcatcaaccagatgggatcaatgctgagtgcacatttcacggagtatccaattgtggatttcaccgccgcctctgccgccaacaacgaattattcaaacgtttcttccatgccatgctggagcgtggtatatatttgccgccttccgctttcgaaagctggtttatgagtaatgcactcactaccgaagacctggatgaaactattgctgccgctaaatctgccatgcaggcaataaaatagttaacaattcaatcctgtgcagagtggaaagggctgtctctataaaacgagacggccctttatttttaaaacaaccttaccatctatcaaaaaataatccctttacaataaactaatcttcaaataaactaaaaactattaattttgcggtttaatgaatgatcgtacgtacatattaaaacgttggaccctcgtctgcttcctgctgtgcttacagctggcaacagccgtcctgccttcgtttgcggcacatcgtcattatttcctgttgcctgatcttcacaaacaacaggtagagcaggaccggttattaagtcttgttaataaaatcccggtacacctcgaagcggatgatgatagtgctgaaatatggcacgtcaccaagcatcgccgtaaaacacggtggtacctttctgctgcggctccacaggtaagtactgccacccgcattgtatatcttgatgcagacaatactgcatacagtcttattcctgaaaataaaaccggtgagtatggcagccagaaatccttccggcccgcctactattcctttctcttccggttcacgcccttttgaatagcaacacagtttctattgtaatcatttttaatttttcttagggagatgcctgtcttttctgctaccatagcggatggcctcctgatgtgttgtattcacctattccggttatgccgggatcaatatcttattgctatgcgtcaatatacagggattttaacatcgctgatcgctcttttcatggctggttgcgccaccaaaggagaaagcaccaacaaagaggatctgaaagttttgccggttaccacactggtaacaaaagatacagtactgcaccgttcttatgtaacagatattcaggcagtacaaaatgtggaaatacgcgctcgtgtcaacggctttcttgataaaatatttattgacgaaggacaggaagtaaaaaaaggacaactgcttttcgggatcaatgacgcggaataccgggctgaactggccaaagcaaaggccgttctcagcagcgtggttgcagaaagcaaggccgccgcactggaactggaccgcgtaaaattactggtggagaaaaaagtagtagcgccctccgaactggaagtggccagtgcaaagctcgccgcagcccaggcaaaaatagaagaagcccgctctgccgccgccaatgcggaaatgcggctgtcttataccagcatccgcgcaccttttgatggtatcatcgaccgtatccctttaaagaaaggaagcctcatcagtgaaggctccctgcttactacggtatcggatacacgcgaaatttatgcttacttcaacgtatcggaaacagaatacctccagtataataaagcgctggccaaaggcgacaacagctaccgccaggtggcgctggtactggctgatggcaccgattatcaccataccggtaaaatagaaaccatagaaggtgaatttgaagaaaacaccggctccattgccttccgcgcccggttccccaatccttccaagctgctgaaacatggcgccagcggtaaagttcgtcttaccactgaaatagacagcgccgtgatcatcccgcaaaaagcagtattcgaaatgcaggacaaaaactatgtgttcgtggtagatggcagtaacaaagtgaaaatgagaaactttactccacaggcccgctttgcacatttttatattgttcagtccggacttcagcccggagaacgtattgtgtgcgaaggtgtgcgcaacatccgcgatggtatccggatttcaccacgcggcgttgccatggatagtttactcagtttataatcacacagcttttgagctgaaatcacggaacaatgtttgaaacttttataaaaagaccagtgctatcactggtcatatcgcttattatcacactggtaggcctgcttgcgctattcaccttgccgatcacccagttccccgatattgtaccgccttcggtaacggtaacggctaaatataccggcgccaacgccgaagtatccgccaaagcagtgtctacaccgctggaaagagccatcaacggggtaccgggtatgacgtatatgtcgtctgtatccagtaacgacgggatcaccgtgatacaggtattcttccaagtaggtaccgatcccgaccaggccgctgttaacgtgcaaaaccgcgtggccactattattgatgaactaccggaagaagtaatcaaggccggcgtcaccacggaaaaagaagtgaacagcatgctgttgtacctcaacgtaatgagcgaggacactaccctggatgaacagtttatctacaactttgccgacatcaacgtactacaggaattaaaacgtatcgacggtgtaggccgtgcggaaatcatgggcgccaaggaatacgccatgcgcgtatggctgaaacccgatcgcatgctggcttacaacgtatctgcggatgaagtgatccaggcgatccgcaaacagaatattgaagcagcgcccggtaaaaccggcgaaagctccgataaaaacgcgatgatgctgcaatatgtattacgctataccggtaaattttttgagccggagcagtaccagcaaattgtgctgcgggcaggccaggatggttccgtgctgcatctcaaagatgtagccgatgtggaatttggctcgcttacctacagcatggtttccaaaacagatggcaagccttctgcttccatcatgctcaaacagcgccccggctccaatgcgcgcgaagtaattaacaatgtgaaggcaaaaatggaagaaatgaagaattcctcctttcctccgggcatgaccttcaacttcaactacgatgtatcccgcttcctcgacgcctctatccacgaagtggtgagaactttatttgaagcattcctgctggtatttatcgtggtatttattttcctgcaggacttccgctccaccctcatcccggcgcttgcagtaccggtagcgctgattggtacgctggcgtttatgcagatgatgggcttctccattaacctgctcacgctgtttgcattggtgctggctatcggtatcgtggtagacaatgccattgtggtggtggaagccgttcacgtgaaaatgagcgaggaacatctgcctccgatggaagccacgctggccgctatgaaagagatcagcggagcgctggtggcgattaccctcgttatgtccgctgtgtttataccggtagcatttttgtctggtccggtgggcgtattctaccggcagttctccctcacactggccatttccattgtgatttcaggtatcaacgcagtaacgttaacgcctgcactctgtgccctcatgctcagagatacgcatggcaaaccccgcaaaaagagcctgctgcagcgcttctttaacggtttcaacaaaggctataatgctaccgaaaataaatatgcgaagcttatcagcttcatcgccggcaggagattgatcacgctggcctgcctggtgtttttcttcaccgctacctggggtattagcgccatcctgccttccgggtttattcctacggaagaccagggcatgatctatgtaaacgtgaccactcccccgggcgcaaccgtggaacgtaccgaagccatactggaccaggtgcaggccattgccgctgaactgggagaagtggaatctgtatccacacttgcgggatacagcctggtaaacgaagtagccggcgcctcttatggtatgggcatggtgaacctgaaaccctgggacgaccgcaaagcatctgttcaggatatcattgaaatattacaaaagaaaacagccggtattgcagatgccagcatagaatttttccctccgcctaccgttccgggattcggtaactccagcgggtttgaactgcggctgctcgatcgcagcggcaccggcgatctccggcaaacggcgcaggtcaccaaccagttcatcgacgcgctgaaaaaacgcccggaaataggcagcgccttcaccagttttgatgcggaattccctcagtacctgatccacgtagaccaggcgatggcagcgaaaaaaggcgtgagtattgaaaatgccatgagcaaccttcaaacactaatgggcagtttctatgcatccaacttcatccgcttcgggcaaatgtataaggtaatggtgcaggcggatccttcctaccgcaccaaacccgatgacctgctgcgcctctatgtaaaaaatgaccgcggcgaaatggtatcttactccgacttcgtaaaactggaacgtgtatacggaccggaacaactgacacgctataacatgtacactgccgctatgatcaatggcgacgccaaaccaggattcagcagcagccaggccattgccgccgtacaggaagtagccgccaaagagctgcccagggggtatagctacgaatggagtggtatgacgagagagcagatcctttccggtaaccaggccttctacattttcatcatcgtgctggtgtttgtatacctcttgctcgccgcccaatacgaaagtttcctgctgccgctgccggtattgctgtcattaccggccggtattttcggtgcgttcctttccctgaagttactgggcctggaaaacaatatctacgcacaggtagcattggtaatgctgatagggttacttggtaaaaacgccatcctcatcgtggaatttgcgatcctgaaaaacaaacacggggctaccatcctggccgcggctaaagaaggcgccgtatccaggctgcgtcccattctcatgacgtctttcgctttcattgccgggttaatacccttgtgtattgcctccggtgcaggcgctatgggtaaccgttccattggtaccgccgcagccggtggcatgctcatcggaaccattttcggtgtactgatcatacccggattatatgtgctgtttgcttccatgatcaggaaaaaaaccgttgaactaaaagattacaccaatgaataaacgaatatatcaatacaccttatatgcggcgatggccactgcaacagtggcctgcagcacacaaaaagaactggcgctgccggaacgtataagcgttcccgttgtatcaggcaataacagtgataccatttcgctgcacaattttgcacaggtgttcaatgatccgaacttgcgaagccttattgataccgcattgcgtaacaactacgacctgctctccgccgcacagcgtgtagctacggcacaggccaacctgatgatggctaaaaatgcctggctgccatcgctgaaccttgccttgtcggccggtgtggataagtatgcggattatacgctcaatggcgttggtaatttcgataccaacctgtcgcccaatatcagtaaagaccaacgcattcccagtcccacacctgaatattttgccggcctgagaagcagctgggaaatagatctctgggggaaactgaaaagtcagcgccaggccacttatgcacgctttctcagcagtgaacagggacgccgcctgctcaccacgcaaatagtggcaggcgttaccgggctgtattacgagctcactgcgatggacaacgagctggctattatacaacgcaatatcaaattgcaggaaacggcggtagctaccgtgcatattcaaaaagccggcggacgcgccaccgagctggcagtgcaacaattcaccgcccagttgctgagtacacaggcattggaatatggcgtaaaacaggaaatcgcttccctggaaaaccagctcaacgccctgctggggaggctgccacagccaattgtacgcagcacggtaaaagacgcgcaggcgttgccggaagcgattaaaaaagggatatccgccagcctgttattgcaacgcccggatatacagcgtgcagagctggagctggctgctacaaaagcagatgtaaaagctgcgcgtgctgccttcttacccggacttaccatcacaccgtatgcgggctttaacgctttcaaagcaggactgttgttccagtcacccgcgtctatcgcatggggcgctgtaggcaatttaaccgcccccatcttcaataaaaaacagatacaggcacaatacaatatcagtaccgccaatgcctggacggcattctacgaataccagcaggcaattgtaaatggctaccaggaagtagcttccgccttaaataaagtggaaaaccagcaggaagcctatgcgctgaaaagcaaggaagtactggtattgcaggaggctgtgtctaccgctaacattctttttaccaccggatacgccaattacctggaagtgattactgcacagaagagtgtactggaagcggagctggcgctggttactacgcgccggaatgtgtaccagggaatggtatcgttgtatcgtgcgctcggaggcaactaattctttcttttaaacacagcggatcgctttacgaggcgatccgctgtatattttattttttacggtgctgaaacaaccacggcattacgcctggttccacaaacatattatcccagctattgtgacccacgccggggtattctgtatatttttcttctgcaccaagcgttttcagtttggcgtcatacgccctggaggcttctaccggtactactttatcatcgccgccatgaaagatccacaccggcacttttttagcaaacctgtccgccgcctctacgttgccggcgccacagataggaaatgcagctgcaaatatatcggggcgtttggtgatttcgtagaaggtgcccattccacccagcgataaacctccgatgtatacccgtttggtatccacttttccgccggccagtaagctatccaccaactggttgagtaaagccgtgggcggtgtaggatcgccatccaacggaaaatctgcctggattaccttaccggtgctgtcgcgcacaaatttcatgggcgcccaggtttgattggcagggcattgcgggaaaacaacgaatgccgggtaattggcgcggatggtatcacgcaggaacatggcgccgccatgcagcagctgcgcgttattatcactgcctctttcaccggccccatgcaggaaaacgatcagcggatattttttgtgacggttatagttggctggcagcagcaggcggtagcggagggtatcacccttacggataaacgattccctgctgtactgggaaagactatcctgtgcagcggctaccaggctaccggtgagcgcgcaggccaggaagaataatttaaggtaacgcataacggggtatttttgttcccaatatactacggcaaagtcagtatttcagcgtgaaatgctgcttgactttaaaatctttccggaaaaataccagcccgataaaaaagaggtcgatggtcatggttacctgcggatgttcctgtatcgtatgccaggcggcttccatatcaggcgtccagtggatatcgtcgaagataaaaacagagtattcatctgcaaactgcaggcactgctcaaaataggccagcgtgggttccttgcggtggttgccatcgatatacacccaatcaggcaactgcatttgtttcaatacatccggtaacacggtatcaaaatttccggttacctgcgtgatgtttttgatatgaagcgcttcgaaattcttggcggccctggctgctatattcgggcatccctcaatggtataaatacgcgcgtgcggtgcggcctttgccatatacgctgtagaaagccccatagaagtacccagttcaagaatacgggccggctggaggtattgtatcaaccggtagaagaattgcccgaatttaggctgttttgccgcgtagcgggtaatatcccttacacggcgttcattaccggccgatatcagcgaccccgcgcccaggtcggttacctggagcgtttcattactttgcagcaactgtttgcgcaactgttctatttcccggaaagccggctgccgttttttatccagcaacacatcctcaatcagtgaaaatacaaagggagaatgtacgtcgtgacgattgcctgaagtaaaataatacttcaggtactttccggctaaattatactgttgcgctaaacccactgctaaattattttttaatagatctttccttttacgatgccccacatatgcaaacgatgctgcagtgatactctcaaaacacccaacccgtaaatggcgctgcgtttgaaattgatactggaggcctcgtcgaagtatttggtaggacaggtaatttctgcaatatcgtatcctttcataaatatctgcgaaaccatttcattatcaaatacaaaatcgtcgttatcagccatgtagttgatgttacgcaatacttccgatgaaaaagtccggtagccggtgtgatattcactcagcttctgaccaatcaggatgttttgtgtcaatgttaagaaacgattaaatatgtatttgtacatcggcatgccccctttcagggcgccttttcccagaatcctggacccgaaaaccaccgggtacacctcattggcaataatactgcacatcgcagtaatgagctttggcgtatactgataatcgggatgcagcatcaccacaatatcagctcccaggtccagtgctttgttgtagcatgacttctgattaccgccataacccttgttgttgtcgtggcgtatcaggtgctgaatccccagccgcttgccgacttcaagggtatcgtctctgctggcatcatctaccagcactacatcatcaactatgtcaaaagggatttcccggaatgttttttccagcgtaagtgctgcgttgtaggccggtaatacaaccactatctttttgttattaagcatgaaagtggatcaaatttggcagcaaaggtaactcacctgctgataattcaaaatatatccggaaaatgcattccggacaccacctatcatgatttaattttaactgttattaattatttatctttgcctgatgatgtttttggcatcatattttcttaaatttttgttaacaaaaagcaaaaacaatatgttaaaacacctaccaacggaaatgaggcacgataaacgcttgaccagcaagcccgatgagtcattaccgttagtacacctggctcaaaaattcctgacgaccagatggattaaagtgctaccagcccctcttgttttactttttactttccagacagcttacgcacaggacccggaactgaaaagcaccacgtctcctgtcattaaaactcaggataccaccatccgcaaactgctggaagatgtacaacggatcaccgacaatgacaaacaaaactctaccgctatacaggccctgttacagggaaaggaaatagataatatcacgaagtacgagctgataaaaaataatatcatcaatgccagtgaaacgtattatctgctgaataagaaaattatcgatctgaagtcgcgtactacgaccaataacctcgatgttttcatcacctccctgaataacccggaaagtaaagcgctgggcttttctttgagcgaccgcattgtagagctggtagaaaagatcatcctgaaaaataaaggagataaaggagagaagaattctaaaattgtagagtctaccaaatccatcatcaacagtcctattttccagagctttacctccctcactcctccgctggcgattgccaactcagtaatgaactttctgcacagtgtgagtgtgaataacaaacagattaaccagaagtcattacaggatttcgaaaaagagctgaacaaatatgtagtgtattacaccgcattgaatgatgccaaccagaaatttgaatatggcctgaacttcaataaagatcagctaagccttttacaggataacctgtttgatcatctttcgtttaccgccacttcccttaaatttcctgctccgcagaaagggaatcagggtttgagccaaacgatgaatgaatacttttttgattttaagaaagaaaaggtagttgattacttcgctaaactggaagagaaatataccaaaggcaaacggatcgattatgaatccctactgcgcgaaaactcttccctgaaagaagtaaacaaccagctggaagacctggttttgcaaaccaagcgattcgaaaatctttacaacgaatatttcacgctgctggattcttactataccaaagtaaacaactcgctgaaaatagcccaggataatggattggcagataaaagcatcatcgatgccaaacaggcggaattcaggaacctgaaaacagaagcagtaggagaaatccaggcgtctatcaatatcagggaactgtatagcaatacagaaaaaatcaagtaccgttacaggatattctagttaaacatattactataaaagcaacaggcggtagtgaaggatttcactatcgcctgttgcttttataggttttaacgtcttcctatagattttatttatacctttgctgcacaatcttagaggaaatgacgacagttcaattggagtacattgttgcggtagatacctacagaagttttgtactggcagcagagaagtgctttgtaacccagccaacgctgagcatgcagattcagaagctggaagatgagttaggcattaaattgtttgatcgcagcaaattaccggtagtccctactgaaataggtatatccgtggttgcccaggccaggatcatcattaaggaaaatgcacgcatccgtgaaattatagcagaccagaaaaaggaagtacaaggcaatctgaaagtaggcatcattcctacactggcgccttacctgcttccccgtatcctcaccgggttcatgaaaaaatatccgaaggtgcgcctggaaatatgggaatatcctacagagcaaattatgcagcaactgaaacaggaactgctggattgtggtttgctggccactcccctgcataacccgcacctggaagaacatcctttattttatgagtcctttgtggtgtacactgctaaaagcaatcctttatacgagaaaaaaatcgtaaaaacagacgagctggatatcaaagatgtgtggctgctcaatgaagggcattgtatgcgtaaccaggtgttgaatatctgtaaggataaatttaccatgggcgataacaagaacctggaatacaataccggcagtgtggaaacgctgaaaagaatggtagatctcaacgaaggctatacaattttaccggagctgtcattacaggatctctcctcccggcaactgaacatggtccgctatttcaaggcgccggaaccggtaagggaaatcagcctggtaacccatcgtcactttattaaacaggcgctgatagaagcctttaaaaaagaaatcctggcacatgtgccggagaagatgaaggtgcagaaaaataagaaggtaattgagattctaacggaataagggaagatataaggaaaacgggctggtaatactacattaccagcccgttgctttttaaagaccttatgctttcgccggtgtataatacttcattgcttccggcatcagctgttgtaatttttgtacgcgggtagcgtcgctggggtgtgtgctcaggagttcaggtggtttctgacctttactcatactggccatgcgttgccagaaaggaattgattcctgcggattgtaaccggccatcgccatgaatattactcccaggtgatcggcttccagctcattaccacgggagaaggcgagtgtacctaagttgccgcctacgccaaatgcctggttaaaaaggtttaccgcggtagggttcttgttcagcgctacagcgccggctacctggataccctgcattaccagtccctggctcatacgttcgttaccatgacgtgcaatggcatgtgctatttcatgtcccattacacaggccagggcagtttcattctgggttacgggcagcaaacctgtatacaccactactttaccgccgggcatacaccaggcatttacttctttgttatctaccaggttaaattcccatttatagctggatatttcaccccccatattattttggttcatgtacctggtaacagccgacgcaatgcgctgccccactcttttcaccatctcagcgtctttactggcagtttgcgccactactttgttttcagacaaaaatgattggtattgttgcacagccattgattgcatcgtgctttcaggaacgaggttcagctgactacggccggtgatgggtacacgagaacaggccgccaatgcgaggcttgcagtaaagaataaaacatactttttcatgggagcatcaatttaaatatgcgaaaacgcaaaaagcaaaaagcaaaaagcatgcacatttttatggctgtcgctttttgcttcctgctttaatatataactgtaactagttcttgtcttttctgttcttgaataacggcactttactttctacacctttcaacagccgcgtgatattcttctgatgggttaacaccaccattaaagctacagcaatagcaaatatgcgataaaagatttcaggttcattgaagatatagaggatcaggatcgggaaagcgatactggcaataatagaactgagagaaacgtatctcgttaaaaaaaggatcattaaaaatacacccacacagcataaagctaccaacggctgtatggcaagcaccagcccgaacagggtagcaattcctttaccacccttgaagtttgcccagatagggaatatatgacctaccactgcagcgagccccagaccgatctggaggttcaccaattgagtaagatgttcaggatcaagataataaggagccagataagctaaacgtactgctaacacacctttcagcatgtctactaccattacaaaagtacccgctttaggccccagcacccggaatgtattggtggcgccggcattgccgctgccatactcccggatatccataccaaaaacgcctttactcacccaaacagctgtaggaacagatcctatcagataagcacaaaaaagcaataaaatttctatcatcactacaagttaggaatgctaagataacaaattctgtgttaaaatagagagaatattagaaaagattataacacaaaagttggattatcaacgctatttatatgtaagttttaatctattttgagtccggtacagaaaattggagcgccagccagttgtctttttcgatccgtttctccatgataaatccttttgaaaccgcggccgctgcaatgttttcttcatccgtaggtaagatgccgctcaatagtaatttgccccccggcactaacaaatgccccatatctcccataaatttcagtaaaatgttatagttgatatttgccagcaatatatcatattttccggtaattgcctcaaggttgtccgcctgccatacttttaccttgttcatcccgttggcagcaatgttctccaacgtattatttacggaccattcgtcgtagtcaattgcatccgctgtatcagcccccatcatctccgccaggatggcgaggataccggttccggtgccaaaatcaaaaacctttttgcccttaaaatccagcggctccatgagctttatcatagaggccgtggtagcatgatgccccgtaccaaaagccatcttaggcgtaataataatttcatatgcaggctgcggatcaaatggcggatgaaactccgcccggataccacaaaaattatctacctgcaccggttggaaattgctttcccacagggcattccagttcaccggtaaaatcgtttcttttgtataggttaccccgtaggcttccaattgctgctgcaatgcggcctcgtcaaagtcggtggcaggaatataagcaatcagcgtatccggctgctcctcaaacccttcatatttcagctcagataattgggcaatcagcaggtctgtttgtgcggcgccggcccgcatggtaatagcaatgtaagacataggccgcaaatatagccattagctgctagctttcagcgttttgacaccccatccgcagctaaaatcatcactcaatattaaaaattgttatatttgattaataaatcatatcatatatcctatgaaagcactgttcctcctgctcaccggcgtggcgttgtccctgtcgggaatggcccaggtaattaaagtacggcctcctgaacctatcacagattccatcatttaccagactgaaaatgtaacattgatctttgaccggaagcatctcacggaatatatgacgggtatggattccaccctgcgcaacagtaaatacagtaacaaggtatttaacagcgtgcagtttgcacacctgaatgccatagatatgggcaaccatttccgcaaggcttattgctacctggaagacactgccaacaaggacttcagctacagtaccggtaaaatgaatatgttgtgggcagaagatggcggtattatgctcccctacgtggaagaaattatgccggacctgctggctggcggggaagtacgggtgatagacaggagtaccaaagcgctgcaacctgcttataagatgattgccgaaccggtggatggcaataattaccgggtgtttcgcctgaacagcggccgcgaaattttcagggaaagcactttccgtgtagagcaactgaccaggagataaaccaccttgtcataaaaataagaaagcagccaccagggtgactgctttcttttgtatttaattccagttatctgctagctataacagcgcctattcggcatcaaaggtaggctcctgaggtttatcaggaccggcgttgtaatttccgccaccacggttaccgtcgcggttgaaatcacgtctctcgccgccaccgcgtctgtcatcaccgccacgtctgtcgtcacggggaccacgtctgtcgccacgatcaccgccgcggtctccacgatctccacgatcacggaagtcgcctctgtcgccacgctcttcacgttctggtctttccacgtaaccttccggtttaggcatgagcactttgcggctcagcttaaacttaccggttttaggatcggtaccagtcagttttacttttactttttcgccttctgtcagcacaccttccattgtttccaggcgtttccaggaaacttcggagatgtggagcaagccttgtttaccaggcatgaactccacgaaagcaccgtaaggcatgatggattttacaacggattcatatacttcacctacttcaggtattgcaatgattcctttcacccatgcaactgctttatcgagactttctttctgcgcggagaagatacttacttcgccggtttcaccaacttcttcgatgttgatggtagtaccggtttcgcgttggatctcctgtataattttaccaccgggtccgataacagcgccgataaattcacggtcgatgatgatcttctccatgcgtggtgcatgtggttttggttcaggacgtgcagccggcattacttcgtacatggcttccacgatatgcaggcggcctttcctggcctgagccagtgcagagcgcattacatccatgcttaaaccatctactttgatatccatctgtatacccacaataccatcgcgggtaccggttactttaaagtccatgtcacccaggtgatcttcatcaccgaggatgtcggttaatactgcccatttaccatcggaagcgcgggagataagacccattgccacacctgaaacgtgtttaggcaggggcacaccagcgtccatcagtgccagcgaaccagcacatacggtagccatggaagaggaaccatttgattcgaggatatcagaaaccacccttacagtgtaagcgtagtcgctgcctggcatcatttgcttcagggagcgcatggccaggttaccatgtcctacttcacgacggccgggaccgcgcatcattttcacttcacctgtagagaatggagggaaattgtagtgcaggatgaatttggaataattggaaacggctgcgctttcgatcagcagttcatcttccggagtacccagtgtaacggtagtcagcgactgtgtttcaccacgggtaaacagggcggaaccgtgaggagaaggcaggatatctgcttccattgccagcggacgaacctgatccagtgcacggccatccagacgaacggattcatccaggatcatgttgcggatcacttctttttccaggtcatgcagatattcttttaccagcggctggtcttcttccggtaattcacccaggtgttctttcagttcagtgccaatggcagcaaacgcatcgctgcgatcgtgcttggctgaagctgacttggctacctggtaaattttatcttttgcaaaagcttcaattttcgctttcagttcttcgttctgatgaggttgtgcgtattcacgtttgccggttacacctttcaggtcacgcagttcttcctgtgctttaacctgcactttgatcgcagcgtgtgctgcttcaatagcaaggatcaggtcttcttcctggcactctttactttcaccttccaccatcatgatgttcttatcggtagcaccgatgatgaagtccatgtcggctttagccagttcagtacggttagggttgatcacgaatttaccatcgatgcgcgctacgcggcattcagaaataatttcctggatgggaacgtcggatacagccaatgcagcagatgcagcaagacaggccagtgcatcgggcattacttcgggatcagatgaaatcagggacaccagtacctgtacttcacataaataattatcggggaacaggggacgcagagcgcggtcaatcaaacgggaaataagtacctcggaatcagacaaccggccttcacgcttgaaaaaagaaccagggatacggccggcggatgcaaacttttcctggtaatcaactgtaagggggaagaaagactggcctggtttgggttctttatttgctaccacagtggccagcaatattgaattccctaaacgcaccgtaacggcaccgtcagcctgacgggccaacttgccggtttcgatggtcaccatacgaccgtctcctatatcgaatttcactgaaataggtgtcagattcataataaagtgaggattaaaaataaaattattcttttttgatcgctaaagaataacaaaaggtatacatacaaaaaaactattcccaaccatataagttgggaatagcgctataattaagtcatggttatttcctgatacctaacttctcaatgagggcacggtagcctgtgaggttggttttagataaataggaaagcaaacgctttctctggccaaccatcttcatcaaaccacggtgggtagaaaaatcttttttgttttgtttcaggtgaccggaaatgctgttgatacgctcagtcagcagtgcgatttgtgcttccacagagcctgtatttttttcgcttccaccaaattccttaaaaatattggctttcttttcaacagttaagtaagacatctttaaaaataataagtaataataatgttttttgtcgctatttttccggtgcaaaggtaatttaaaaaataggaattaccaattaacgggaaattaataataaatgaaggataatgtacatccgtaatattttctttctcaacaactcctaagaagaaaaattcacagctgcattatccgttacatgcccgttttctgtacgcagtactctcgacgggaatttctgtaatactatgtaatcgtgtgtggccatcactatggcggttccttcacggcaaatacggaacaacagctgcataataccatcggaagtttccggatccaggttaccagtgggctcatccgccaggatcagttttggcgaattcagcatagcacgggcaatatccacacgctgctgctctcctcccgataactcgtacggcatcttaaagcctttggtacccaatcccaccttttccagtacatcgttgatcttattctccatttccttaggatcctgccaaccggtagcccggagcgcaaatttcaggttatcatgcacgttgcggtcggttaataactgaaaatcctggaataccacacccagattccggcgaagatacggcacttttttccaatccatcttcttaagatcaaaaccaactacctgtcccgtgccatcatttaaaggtaaatctccatacaatgtctttaacaaactggatttcccggtaccggttttaccaatgagatacacaaattcacccttgttcaccgtgatattcacatcagctaatatcaatgaatggccctggtatatactggcgtttgttaattgtatgataggttgttcaggcgtcatgtcctttctgttttttacggtctgtgcggacaaaaataactaattaaaaaataactcgttgtgataatatgtcaaatatccatctctctgaaactaaaaaaatagttgtcaaactaaactattagttataacttggttttacaaacgagcaatatgaaacaactcaccaaagcagaagaacagatcatgcaggcactctgggaaaccggcccggccttcgtgaaagatatcatagaagtaatgcccgaacccaaaccgcattacaatacggtgtccacccttgtgaaaatactgattgaaaaagggtttgtcgactttaaagcttacggtaaatcacaccagtattttgcccttgtaaccaaagatgcttacagccacaaaacagtcaacaatatcgtgaaaggctatttcgacggctccttcagcaacatggtttctttttttgtgaaagaaaaagaactgagcatcgctgaactggagaaactggtacaaaaaattaaagcagcccaaaaatcttaaccatgacagttctgctcacctatctctccaaagtgatcatctgttcagccgttttatacggctactactatatcgccctgcgtaataaccgtttccaccaatggaaccggtactacctggtgctcatcaccctggtttccctgctcacccccctcctgaaaattccgctgccaggccaggccgccgaatcttccacggtgctgtcttatacaacacgcattgtgaacatccgcgaaaccgtgataccggccaaccccgggatcagttccggcatggtgctcaacatcctgtacatcgtggtgatagcgttgctgctgacacgaacactgatcagtcttttcaggattaagaacctcatccgccgcagccaggtgcaggaaattcctccctaccggtttgtaaagaacaaggacatcaaagcgcctttttctttcttccgctatattttctgggatcaacaaacatcattgaattcgcccgaagggcaacagatatttaaacatgaactggtacacctgcaggagaaacacagtacggataaactattcatggaactggttaccgcggtatgctggatcaaccccttctttcacctgattaaaagggaactggcactggtacatgaattcctggccgacaaaaaagcagccggggaagaaatagccggctacgcgcaaaccatcctccagatggcctttcaaagcaaacaattcagtattacaaacgacttttttcatccgccaataaaaagaagaatccttatgctgacacaattccacactcccagattcagttacctgcgacgcatcatggtattgccgctggctaccttcattttttgctcccttgcatttgtggccgataagcgtccgtccgccattccggcgcttaccaccactgccgctgctattccttcggccaccatcgcagtggataccacaccggttaaaaaggtaaccaccaggaaagacaacgtttatacttcggtagaccagcctcccactttccagggcggagaagaagcgcttgcaaaatatctttccaaaaacacccggtatcctaaagctgcacaggaaaaaaacatttcaggtacggtgtacgtaaattatgtggtagacgaggaaggtaatattacagatgttcgtacggtgggaaaaaacccgggctttggtcttgctgaagaagcgatgcgtgtagtaaaaggaatgccgcaatggatacccggcaggcatcagggccgggctgtttccgtacagtttaacctgcctatccgctttatgctggatgctggcaaacagacaccgaaaaccggtgatcataccgtcaatttcccgccacctaacgataaagaagtattcacctttgtggaacatccaccgaaattccccggcggcgaaaatgcccttggattatatcttagtaaaaatatccgttaccccaaacaggcacagaaagcgaatgtaagcggtaccacctttgtgcagtttattgtggatgcagatggcagcatccatgatgtgagaacaataggcgcaaagaaaggttacggcctggaagatgaagcgataagggtagtgaaagccatgccgaaatgggaaccaggtgtgcaaaatgaacgccaggtggcggtgcagtttaatcttcctatcaggtttagtctgcaaaactaacacaactataaatgatcaataagggcaggccacggttttacactgtggcctgcccttattctattcatcatcctcagcttggaattacttctggggtacttcgccaatgcctcatacctgggtataccatggatcatccatggactctccatgcacttctgatggactcctcatgcactatcaatgcactctccatacactccctatacactatgacctaatattcaaaggttccagccggcgctttcacggttactttcttctcttctgcggcttctaccctgcctatgatctgtgcatcgatattaaaacttttggaaatgctgataatatcagctgctattgcttccggcacatacagttccattctgtgtcccatgttaaacacctggtacatttccttccagggagtaccggactgctcctggataagactgaacaacggaggcaccgggaacaggttgtctttgatcacgtgcagtttctcaatgaagtgcagcactttggtttgagcaccgccgctgcaatgtaccatcccgtgtatctgcggccggaattgctccagcactttcttgatcacaggggcataggtacgggtgggcgataataccagtttacctgcatccaccgcgccaaagccaggaatatttattttatctgtcagcgattttttaccgctgaacaccagttcataaggaatattgggatcaaagctttcagggtatttttccgcaatagctttgctgaaaacatcatgacgcgcgctggtgaggccattgctgcccataccgccattgtattccgtttcgtaagtggcttgtccgtaggatgccagccctaccaccacatcgcctgcctggatccggtcgttggagatcacgtcttcacgtttcatgcggcaggtaacagtagaatccacgatgatggtgcgtacgaggtcgcctacatcagcggtttctccaccggtagagtaaatgctgataccgtggttccgcagttctgccaggatttcttctgtgccattgatgatggcagcaattacttcacccggcagcaattgtttgttgcggccaatggtggaagaaagaaggatattgtctgtagcgcccacgcaaagcaggtcgtccatgttcatgataatcgcgtcctgggcgatgcctttccagacacccagatcaccggtttctttccaataaatataagccagggaagatttggtgccggcgccgtctgcatgcataatattgcaataagcttcgtcgcctcctaaaatatcaggtacaattttgcagaatgcctttgggaaaaggcccttgtcaatgtttttaatggcattatgcacatcttccttgcctgctgaaacaccgcgtttggcgtaaatattattatccaccgggaaataaataaatatgtaaataaaaagtaaactaaataaagatgctcttcaggctgcaaaagtaacagattccatgcagaatgcccgccgaatgtgttagatttgcacggcgattttgatagttattgatttatatgcaggttcacagggacttagaccatttaccggaattccgtaatgctgttatcacgataggcactttcgacggagtacatgcaggccaccgcttcattattgagcaattggagcaggctgccaacacctgcggcggcgaaaccgtgatcattacctttgatccgcatccacgggaggtattacaacccaaaccgaataatatccggctgctgactaccctgcctgaaaaaattgccttgctggagcgtgccggcattcatcacctggtagtagtgccttttacgaaagaattttctgagatgcccgcccgcagttacctggaagacttcctggtagcgcgcttcaggccgcacaccattattataggctacgaccaccggtttggccacaaccgggaaggcggactggaactgctcgaagcagagcagcagcagtatggctttaccctgatcgaaattccgcagcaggtagtacatgatcttacggtgagttctaccaaaatccgtaaaagcctgcaggaaggcgatatccggctggccaatgaattgctggattacacctattttttaaccggcaccgtagtgcatggcgataaaatgggccggcagctgggttatcccaccgctaatctgcacctcaccgacgaaagaaagctgattccggctgaaggtatttacgccgtaaacgcccaactcagcggccgcagcgaattattacctgccgtgatgagcatcggcttccgccctacttttaatggcaccgatctccgtctggaagtacacatctttgattttcatgaagatatttacgggcaggaattaacggttcattttgtagcatacatccgctccaacctgaaatttgacaatatagatgcgctgatagtacaaatggataaggattctgcgcaggcaaaggagatactggcgaagatttagaattcttctcccaggagttccgttttttgctcgtcctttttagggggcttcattaaacgaaccccacgccatagaaaaaaggcagacgcgattacataaaaacacatgatcatagccgtattggtgctcatgctaagatccaacccgatcgctccacgatgaagagtgatgatgttcatcagcacaattaaagcgcagcaactacttaaaacgaaacacagcaggccaaacagcaatctgaatatcttctttaccccaatagccataaaaaaacagcataattaattaattcatcaccttatacatcagttctttcatcagttccccgtcttccacgccactatcgttaatgcctatactccgcaggttatattggtgcagcagcaaaatagctttctcggttccttcgggtccgtattgacgggcagcgttcatatagtcctttacaaaaaacggatgtacacccagcgccgtggccacctccttttcgcccccttttacgctgaaaatgaggtttactttagcgaagaaattatagagtgcgggcaatgtcatctggatgggcgctgctttgggattggcggcaaagtaagcgatgatccggaatactttagccgtattcttctgtcccagggcgttttgtagttcaaatacattgtactctttactgatgcccacatacttttcaatatccgcttcgtcgatctttttctgggcgggaaggtttaccagcaacttatctatttcattggagatacgggaaaggtcgttcccgatatgatctaccagaaggatagccgctttttgtgagatggccagtccgcggctgctcacatagctttcaacccacgtgggcagctggttatcatataattttttggtagacaggagtacgcctttttcctttatgagcttggccattttactcctgccatctattttgccctgtttatgcgccactacaaacaccgtagaagtaagcgggttatcgatataggtttccagtttcagcagatcgcgcatggcctgcgcctctttgagcagtaccacctgtctttcagcgaacatcgggtacctgcggcaggcgttgatcacctggctccagtcagtatcctttccataaaggaccgtgaggttaaagcctctttctgattcaggtaacagctcatgttctgcatagctggtcacctggtcaataaaaaagtcctcatctccttccagccagtacaatgatttgaatttttgctgcttccaatccctgatgatatcctggtactccattactagaatgctttttgtctatttttttacgataataatatcttcctgtgtcaatgccggtaaacgtttgaacttcagcagcagctgtgctaccgccagtacatccttctggcaataggcggcaatacgttccagatctttttcctcccagtataccttgcctaccatgctgccgtctatatcgtctttgggcgtatcaatacccataacggccgttagaagtttcagggaaatataatgtttaaagtccccgaagcgccacagatgcagggtatcgagcatgggaatttcccagggtttaaatccgtgcagctgtaaaggctgtggcaaagataattgatggataacagacctcctgcaaataaaaggaatatcaaattctttgatgttatgcccggcaaactggaaccggggatatttcgcatagaatttattgattaattctaaaaatcctgacagcacaactgcttcatcatcattacaaaatgatttcagccttagctggtacctgttattttcaagactaaagaagccggccgaaatgcacacaattttcccaaattcggcgtagatgccagccctgtcagcgtatgctgaatcttcatttccggaaactggcgcagtttttgcaattttgtcacgccagagctgttgcatgtcttcggataagtgctctatagcaggagccgcgggtgttgtttctatgtccaacagtaataattgatctaacgcaatatttggaagcacgattgaaaaacagttttatagctatttataaaataggaatattataagtacttttgaataacaatttttaaccatataacaataaacataaaactcacaactatgacggagaacacttttaattcacctgcaccgggatcacccggaccagaaaaaccacgtagccgcaacggtctaatttacggtattttaattgcagcattagccggtacctggatatatatgttgtatgataaaaataaatccaacgagcaaattgttcaaaaaagcacccagatagattcgatctcttcgtcacgtgacgcactgcagcaggaatacaatgcggccaatgcccgcctggatgatctggtttcacagaacacccggatggatagcctggttaaaacaaaagataaggaaatacaggatatgaaagccaggatctctactatcctgaacaacaaaaatgctacacaggcgcaactggcggaagcccgtcgtttgattgagcaactgaaatccaatattgaaggttattcagaaactattgaacgcctggaaggtgaaaaaatagtattggctggtgaaagagattatgcacgtaaagagcgcgactctgtgtctgtggtaaaggacagtctgaataaaaaagtggacctgggttccgtactccatgcttccaacattaaactgttaccgatccgtgtaaagaataacggtaaagaagtagaaaccagcaaagcaaaacgcgctgatatgatgcgggttacttttgacctggacgacaaccgtattgcaccaaccggtgataaagaaatttttgtggccattactgctccggatggagcgccactggctgtagaagcgcttggttccggccgttttacactggaagatggtactgaaaaattatatactgccaagaaaacagttgcttatactactggtcagaaacaaactgtaagcatggactggaaacagaactccgatttcaaggtaggcgattatgcagttgaaatctatcacaacggtttcaaaataggacaaggtaaagtaacactgaaaaaaggcggcttgttttagtaacaatcagcattcaggataaagtcgatggccggagcaaagattattctttcactccggccattcgcttttgtggcggttttatagcggattcatggtatttttttcgcttatctcatttgttaatgattagttattgacaaaaagatatatataaaaataaaattaaattaacgttctttgctgcacaattaaagatagccggaggccactgcactcccctgaccaatgcttaagaagaagaatgtgacaggcatatgatgccggtttagcccgtgattcattctttaacatcgtcttatgtgcgccttttgttattattggataagatcagaagcccaattaaaaccgaagcatggaagacatgaataaaatagtgtacgttgtagatgatgatgaaatatttcattttatcatcaaaaaaatgttggggcaccaaagcaatcacctgatagttacctcttttctctgtgcagaagaggccctggagcagctttccagtaccccgcaaactaccttaccctctcttatcattcttgatatgaatatgcagcgaatgaatggctgggattttattgaggcctacagaggattgaaaacttctctgaaaaataccatcccgattataatgtgttcttcctctgtggatgtacgcgacatgcaaaaagtgcagcatacgccggagctgatggcgtacattaccaagccgctcgataaaaataaattaaaggtaatagaggagtatctgtaagatataaaacaccattaaaaaaagaagcgaatgatcggcagaccattcgcttcaattattttcagttatcttacttttacgctaaaaccgcgctgccgtacatttcttcgcgcagtgctttcacacgctcatctgccaggtactcatcaaaggtcatcagcctgtcgataatgcctttaggcgtcagctcaataatacggttggctactgattgcatgaaggtatggtcatgggtggtgaacaacaccacgcctttgtagttgatcatactttcgttgaaagactggatagattccagatccaggtggttggtaggctcatcaagtatcagcacattgggatcctgcagcatcatgcggctgatcatgcaacgtactttttcaccaccactcagcaccgaagttttcttcatgatctcatctccgccgaataacatcttacccaggaatccacgcaggaaaggctcatccacatctgttacatgtggtggtacgtattgacgcagccaatccatcaggttcaggtctttattggtaaagaacgcggagttgtcgtttggcaggtaggcactggtaacagtggtaccccattcaaacttgccaccatcggcttttgcttcattgttgatcacttcaaagaaagtagtgagggccaggtgatctttagacaggaatgcgatcttatctcccttgttaacggagaaagtaacatctgtaaagagtttacggccatccaccagtttttccagtttctctatgttcaggatctggttacctacttcgcgctgttgcttgaagatgatacccggatacttacggttagaaggctggatatcttccaccaccagtttttcgagggctttcttacgggaagtggcctgcttgcttttggaggcgttggcgctaaaccgggcgataaagtccatgaggtctttacgcttatcttccattttcttattcttatctgccatctggcgggccatcagctgggatgattcgtaccagaaggtgtagttaccactgaagatctggatctttgcacggtccacatctgccacatgcgtacatacggcatccaggaagtgacgatcgtgggataccacgatcacgatattttcgtaatcggccaggaagttttccagccagccgatggtttccacgtcaaggtcattcgtaggctcatccagcagcaggatatcaggattaccgaacagcgcctgtgcaagcagtacccgcactttaaggctaccggcaatgtctttcatgagcactccatgcatttcttccttcacacccagatcgctcagcagtactcctgcatcgctttctgcggtataaccacccatttcgccatattcagcttccagttcgcctgcgcgcataccgtcttcttcggtaaaatcttccttggcgtaaatagtgtccctttcgtgcgctatttcccaaagcttcttattacccatcaatacggcattcagtacggtaacctcatcaaacccaaagtggttctgcgtgagcacgctcatgcgctcaccgggggtgatttccacagtacctttattcggttctatttcaccggacaatatcttcagaaaagtagacttacctgctccattggccccaatcacaccataacagttcccttttgtgaaattgaggtttacttcgtcaaacaatactctcttaccaaaagagagcgttacgtttttaacactgatcatgctggctatgtaaattttgaagctgcgaaggtacagattttatgcggggtttccaagaaggcgtcctcccaggcatatcaataaaaagtactcgttaatccattcatcatgaaagggttgtctgcatatatctttctatgcgtatctttagcgcataaaaatggaaccgcatgacagcatataacgagatatttgagaacaataaacgttggatagcttccaaaacggccacagacaaggagtttttcgaaaaaatggccgactcccagaaaccagactatctgtatattggttgcagcgacagccgcgttcccaccaacgagatcatggggcttgaagcaggtgaagtttttgtacaccgcaatatagccaaccttgttcccaataccgacctcaacgtaatgggcgtcatcaattatgcggtagtacacctggaggtaaaacacatcatcgtatgcgggcattataactgcggcggcgtaaaggcagccatgcaagcgaaagatctcggcatcctgaacccatggttacgcaacatccgtgatgtttaccggctgcacatggacgaactcaacgctatcgccgacgaacatgcacgctacaaccgcctcgttgaactcaatacgcaggaacaatgtattaacgtaatcaaaaccgctgcggtacagaagtcgtacgtaggaaaaggattccctaccgtacacggctgggtgtatgacctgaaaaacggcttgctgaaagacctccaaattgatttcgaaggcgtactgcacgaaattcaaaagatctatgacttaacaggttccggcctgatgcaaaaagataccgaataatcatgggtccgatcggcatattcgactccggctacggcggattaaccgtactcagggaaatagtagcggaactcccgcagtacgattacatctacctgggcgacaacgcccgcgcaccttacggcaaccgtggctttgataccattcacgcttatacgctggaatgtgtacaaaaactgtttgcaatgggctgtccgctggtcatcctggcctgtaacaccgcctctgccaaagcgctgcgcaccatccagcaaaaagatctgcccaatatagctcccgacaaccgggtactgggcgtgatccgtcctacttcagaaatggtgggtaccatcacgcaaaccggtgaagtaggcatactggctaccaatggtacggtgtcatctgagtcttacccgctggaaatccataagtttttcccgcatgtaaaaacacatcagctggcctgccccatgtgggtaccgctgattgaaaataacgaacatgaaagcgaaggagcagactactttgtaaaggaatacctggataagatattattgggctcaccaggtatcgataccctggtactcggttgcacccactatcccctgctgatgaaaaagatcaaacagtttttacccggcggtattactgttttgtcgcagggtaaaattgtggcgcacagcctgaaagactacctgaaacgtcatcctgaaatggaaagcaggctgagtaagcaacagcagcgtagtttttatacaacagatgatcccggaatttttgataagatggcggagatcttttatgggcaaacagtaacatctgcaaagatgctcaccaaataaaaaagcctgccggcatcatgtaccggcaggctttaattttttatctccttccttacttcccttcaagcttcagcaggaatgaatactccaacgccacttcctccagcgctttaaaccttccggaggcgccaccgtggccagcttccatattggtatgcaacagcagtaaatgatgatctgttttcatttcccttaatttcgccacccattttgccggctcccagtattgtacctgtgaatcgtgcagcccggtagttaccagcatattcggatacgccttatgctccacgttatcgtaaggagaataggatttcatgtaatcgtacgagtctttattttttggattgccccactcatcaaactcaccggtggtaagcggaatactttcatccagcatggtggtaaccacgtccacaaaaggtacctgtgccacgatgccattgaacaaggtaggctccatattagctacagcacccatcagcaggccacctgcactgcctcccatcgcataaagatgcgcggtatccgtgtaatgttgctgtatcaggaagttggcgcaggcaatgaaatcggtgaaggtgtttttctttttaaacatcttgccatcttcgtaccattgccgtcccatttcctggccaccgcggatatgcgcgatcgcaaaagcaaaaccacgatcgagtaaacttaaccgggtagaactgaaagtggcatccatgctgttgccataggaaccatagccatacagcaataacggccccttgccatttttttcaaacgttttcttatatacaatggacaccggaattttagtaccgtctgtggcggtggcaaacaaccgctctgttgcataatctttcggatcatagccgcccagtacttcctgctgacgcttcagttcattggcgcccgtttccatattgtaatcatacaccgagttgggtgtgatcatggatgtatagttataccgcagttccttgctgtccatttccgggttgctgctcacggaagcagtatacgctgcttctgaaaatggcagatacttttccgtgtgtgttttatcattgatgatccggatatgggttaaaccgccctttctttcttccaataccgtaaactctttaaacagctccactccttccagcaatacatcgctgcggttagggatcagttctttccagttttcacgggaagttttatccagcgcggtttccatcaggcggaagttgagcgcgttccagttggtggtgatgtagaatttatcatcacggtgatccacatggtacagcatatctttttcacgcggttggaaaatgcggaatgcttcgttaggtttagccgcatccagtatcctgctttcagatgataaggtgctttcgctgttgatgataatatacttgccggattttgttttagatacatctacatcaaacgtttcatctgcttcgtgatatacttctttgtcggctgcgatacccagtgaatgccgcatgatacgatcggcccggagggtaacggtatctttgcgggagtagaacagggttttgttatcactggcccaggtgctgccggcggtggtttcatgaatttcgtctgtgagcagttcgtttgtttccaggtttttgatccggatggtataacgtctgcggctgaccgtatctatcccgtaggcgagtaattttgcatcggggcttacactcaggccggccacgtggcaataggcatgacctgcagccagttcattcacgttcagcattacctcttcaggtgcttccaggctgccttttttacggcaatgcaccgggtactcctttccttcttcataacgggtatagtagtaataaccgtttttaagatagggcacactcatgtctgtttccttgatccgggatttcatctcggtaaagagtttttcgcggagctttttttcgggcgacaggatcgtgtcgaggtaagcgttttctgcgttcagccaggccagtactttcggattttcccggtcattcatccagtagtaattatcgatccgtttgtcgccgtggatgctgagttctttagctatcttttctgctaccggaggttttatatcagcctggtcgttcatagtatttttcttttgattacaagacaaaagcaccgttcccaaaagcaaccaacaattaccctggaagtttttaaacataggagatagatttaaatagtaaggttttaactcaaaagcattacaaattacgaattctccctacactattttcatatttaccgggtcccagttgatcagttttttgctgaagtaactttcatttgtaaccagggctggtcctgcggcgcgcagaccgaatacggcatcttccacaacgggtttaccggagcgcatggattcaaagaaattggtgaaatgttccagccggtcgtcgtatcctttagggggagcgtaggagttggatgtttcgatggcattgcgtttatctgccgggtatttggcattatattctttcacatattgcgcctgttgtgctttggtgaaagtgttataagtgtcccagccaccgtagcctggcgcttcgggcagcttgtgttttttgattttaaagtcgttccagcccagttccaatacaccttcggtgccaataaaacgggtgtattccccaccgccgctgccgtcggcgaaattcacgcggagtgtcatctggaacgcgggatgttctttagtttcgggatagtcaaaaatggccactaccacatccggcacatcgcggccatctttccattgtaccaggttgccactggcataaatagatgtggggccaagcgatccggtaataaaatgcaggccggaaatcaggtgtacaaacaggtcgccggggatgccggttccataggcgcggtaattacgccagcggaaaaagcgcaccgggtcgaagggcaccttggaggtatctttcaggaaggtatcaaaatccacggtagcaggggatgcatccggcgggatggaatattgccaggcgccgagtgcgctgtggcggtccatccgggcttccactacgttcagccgtccaatttcacccgcctggtaacgtttacgcgcctccgcaagcgctacgctgctaacgcgctggctacccacctggaaaacggctttggtgcgttgttgtgcggcaattactttatggccttcttctatctgctgtaccatcggcttttcgcaatacacagctttaccggcttccattgcagcgatggcaatcgtatcgtgccagtgatcgggtgtagctacaataatggcatctatatcttttcgtttgagtaattcgcggtagtcgcgggtagtatatacctgcgggccaaacacttccttcactttgtcgaggtgaccggtgtacaggtcggcagcgcccacaaattccactcccggcactttgatagcagtttccacatctccgaatcccataatacccattcctacacatgcgatacggattttgtcgctgggagcgatccttttttcgggctgcaggatttctacatgttccttttcatttgcgagggccgccagctggcctattccgagcagtgcggcagtgctgccgatgtgtttgataaactttctgcgtgattgttctgacatatgttctctgttttacattgcgtggaaaaaacacatgatagtaaaaaaatttagaaagataaagttcgatggatgagcggggggagcggaggttgtctttctcaggattacgctgatttgggggattttatttttttggattttgtaaatgattaaaaaagtttggggagatgatagcggttttggatttttttggaagatttttagtttttaggagagataaaaagaaaggagataagaatgaacaagccattcttatctccttaatatattaaaagaaaaaatcaaggtaatcagcttaatcagcgtaatcctgagtaagacaaactccgcgcgcgcttatttctcagaagaaaatcctgctccaataaactccctgttgaggcgggcgatattggtgagggaaatttccttcgggcattctgcttcgcaggcgccggtgttggtacagctaccaaagccttccttatccatttgcgctaccatgttgagggcgcgggttgttctttcaggctgaccctgtggcagcaatgccagctgggatactttggctgatacgaacagcatggcggaagagttcttacaggcggctacgcaggcgccacaaccgatacaggcagcagctgcgaaagccaggtcggctttatttttatctaccggtaaacagttcgcatcctgtgcgttacctgtgtttacggaaatataaccacctgcttcgatgatgcggtcgaaagctgatctgtctaccgtcagatctttaattaccgggaatgcgcctgctctccagggttcaaccgtaatggtatcgccatctttgaaagcgcgcatgtgcagctggcaggtagtagtaccatcccacggaccgtgtgcgcggccgttgatatgcatggagcacataccgcagataccttcgcggcaatcgtggtcaaatgctattggttctttgccttcattgatcagctcttcattcactacgtcaaacatttccaggaaagacatttcagaagaaatgttttttgcctgtaaagtttcaaatctaccctgatcgtttttgtttttctgcctccacacttttaatgtgaggttcatgttataatgttccatataccttggacaattatttgatttataatcctggctaaccgttaaacggtttaccaataaccattatttgtagctacgctgtgttggtttacattcaacgaattccagcggttctttgtgcagttcatactggccatcgcctttgtattcccatgcagatacgtagctgaagttttcgtcatcacgtttggcttctccttcctctgtttgtgattcttcgcggaagtggccaccacatgattcgcggcggttcagtgcatcgatacacattaattcgcccagttccaggaagtcggccacgcgaccggctttttccagttcggggttgaactcattggcttcaccgggaacacgcacatctctccagaactcagcacgcagcgctttgatttcttcgatcgcttctttcaggccctgttcattacgcgccataccacatttgtcccacatgattttaccaagtttcttgtggaagaaatcgactgatttggtgcctttgatgttgatgagcttattaacggtttcccttactttattttctgcttccacgaaagcgggatggtcggtagggattgcctttgtgcggatttcatctgcgaggtagttacctactgtgtaaggaatcacgaagtaaccgtcggccaggccctgcatcagtgcagatgcacccaggcggttagcgccgtgatcggagaagttagcttctcccagggaatataatcccggaacggtggtacccagttcataatccacccagaggccacccattgtgtagtgtactgcaggatagatacgcataggcagttcgtaaggattttcaccggtgattttggcgtacatgtcgaacaggttaccatatttctcggctactacttctttacccagtttaatcacttcttctttggaaacattggagagctggcgtttacccacttcaatattaccataacgttcgatggctgcggcaaagtcgaggtatactgcctgtttggaagtacctacgccataaccggcatcgcatctttcttttgctgcacgggaggccacgtcgcggggaacgaggttaccgaatgcaggatatcttctttccaggtagtaatccctttcatcttcaggaatgtcgctggctttgcgggtatcgttttgttttttaggcacccagatacgaccatcattacgcagtgattctgacatgagggtcagtttcgactggtgatcgccggaaaccgggatacaggtagggtggatctgtgtgaagcaggggttagcgaagtaagcgccgtttttagttgctttccaggcggcggttacgttagagcccatggcgttggtagacaggtagaacacgttgccataaccaccgctgcagatcagtacggcatgaccgaaatggcgttccagttcgccggtgatcaggtcgcgtgcaatgataccgcgtgctttaccatcgattttcacgatgtcgagcatttcgtggcggttgtacattttcacgttgccgagtgctacctggcgttccagtgcggagtaggcgccgaggagcagctgctgaccggtttgaccggcggcataaaaagtacgctgtacctgtgtaccaccgaaagagcggttacttaacaggccaccgtattcacgtgcaaagggaacaccctgtgccacgcactgatctataatattaccgctcacttctgccaaacggtgtacgttagcttcgcgggcgcggtagtcaccaccttttactgtgtcgtagaacaagcggaaaacagagtcaccgtcattctgataatttttggccgcattgataccaccctgggcagcaatactgtgtgcgcggcgcggactatcctgaaagcagaatgcttttactttatatcccaactctcctaatgaagccgctgctgaagcgccggccaaaccagtaccaatgataatcacttccaggttgcgcttattggcagggttcaccagtttacagtgtcctttatagtcttcccatttggaatttaatggtccggcaggaatttttgcgtcaaacatatatccttactttacagaattatttgaaatagattacaacggggatgatagcaaaaccgataggaattgcgataccaaacaaccatatgccaatgaagctgagtaagccgttgtattttttatgatttaaaccaaaggtctgacaggcgcttttaaagccgtggatcaggtggaaagacaaaccgatcatcccgatcacgtacaatgcaaccagccagccattcttaaaggtttcataagataaagcgtacaggtctttcaacggttcaatgctgccttcataagtacggatgggcatttccgcgtagtggaattgtccccagaaattaaccaggtggataacaatgaagattaaaaggatacttcccataatggccatctgacgactgaaccaggaagatgtctgattacccgggttgatggtatatttcaccggacgggctgctctgttgctgaacgtgagctggagcgcaatgatggcgtgcagcagtatcacaattttcagcccccaggcaataaactgaatcaggctgttgtgtcccataaacgcagcatatgcgttaaaggccttgccttcgtcgttgtacaacagctggaaattacctgccaggtgtacaataacaaaactgcaaagaaacaagccggtagcacctaccaataacttcttaccgatagaggtattaaaaaactgtgaccacttcataagtaaaattctaagcttcctagtataaaaagatgtttgaaatgtcgggcaaatttaacgcaggaaaaataaaaaccaaatgatatttatcaggtttttatacgcatatattattattcatatgcactatgtattcataatcatacaaacacgcataatatctttcattttgtaatgaaaattaatattattccagccgttttaacatgatattatccaccatattgaacaggtgtaatggttgatatgtccgccatttatcatcatcgagcaggtgaacatagtagtgcaggcgggctctttcaaactcttcacgggtttgtaccggcatgttcaggcttacgatccagccgccttcatcgcggatatcttcccaccattcttcataataacaatcatcggaggaatggaagttcatcacattttccgtgatgagaatatattttgtgatgccctgggcgatgagggtatcgatgatgttacgcttcatggtcatgatgtcgttatcaatggcatcattccattctcccagtaattctatgatagcgaagttaaactggtaatcgatgaagaggattttcatgtacaggttgcgtgagccaaattcatcccactgtggatgtatataatagttatacaccgaattggaatattcaaactcactgtattcccttccataaaagggagagtactcatcttcttcggcggtgtacaaatgccgccagttataatatggctctatgttgtgcatacctggtttatgggtgcaaaggtttttaaatcatttcccggtgaagtcgtccaccgcttttttcacgctgccggcctttaacagcagttgttgcgcctgttcataatcggtgagcgataattgttccatgagcattttcacgccccggtctaccagtttttcgttgctgagctgcatgttcaccattttattatcttctactctcccgagctggatcattacggctgtagacagcatgttcagcaccagtttctgcgcagtgccgcttttcaggcgtgtgctgcccgttacaaactccggtcctaccactacctccacggggaagtcggccgccgcagataccggcgtatccgggttacagctgatgctgcctgtaacgataccgtgcttgcggcattcattgagcgcgcctattacataaggcgtggtaccgctggcagcgatgcccactaccacatctttaccggtgatattgtatgcctgcagatcttcccagccctgcgtgcggctgtcttccgcaaactccacggctttgcgtatggccgtatcgccgccggcaatcaatcctactaccaggccttgcggcacgccaaaagtaggcggacattcagaggcatctaccacgcccaaacggccgctggtaccagcgcccatataaaagaggcgaccacctgccagcattttatcggctacggctgttaccagtttctctatttgcgggatggctttttccacggctaacggaacggtctgatcctctttgttcatattggtcagcagttcctgcacgctcatcttttcaaggtgacgatagtgtgaggcctgttccgttacttttacaaatgacatattgaatgcttaaaaatgattaacgatgatattccagcaagccttccatgggcgtgcgcagcactttgcccataggcaattcatacagttcacacaattcgctgatgatgtcgcggaagtgccaggcaacgccaccggtaaaatgcagtgccgtagtccagctttcccggtatttataaatatgattaaagaagaagtcgttcagcccgtcctccaggatgttctggatcatataatgctcgcggttttccgacaggaactctgtaaaccctgccaggtaacggttggctaacggcttccggtatacgctttccaggatctcatctttattggtatggtacttatattcgaagcgggcgtgcaggtcgtcatcaaaactatgatagaggtaatactgaagcaccttacgcccgaggtaggcgccactgccttcatcgcccaggataaagcccaggcccggattatttttcaccacttctttaccatcatagtaacaggaattggagccggtgcctaaaatgctaaccactcctccctgcgtgccgcaaagtgcgcgggccgcgcccatgaggtcgtgctgcacatcaaatgcggccgccggccatactgcctttattgcatcggataccagttgcaggttcttgggctgcgacaggcctgtcccataaaagtatacgtccgttaccggttggccggcaggtaactggggaaccagttccgtttcgaagatggccttgatctgttccgcagattgaaaatacgggctcacaccctgcgttttcaataccagcggttccgccgcgcccagcaagccccattccgtcttcgtagatccgctgtctgctattaactttattccagcacccatatccggttatttatgaaatttaagaatcctaaaagtttgcacccgatttatgctatttttgtcacaatttaaacaaaaggggttcataaaaacaaatggcccctttaagtttaggtgatgatgatacatgtatgcagcagattgctttccgccaggtgcttttgctacatggatataaagattggtcatataaattagcgggataataatctgattatgtctaacaggaagttgaatgtttttttacctcttctctttgcagttgtattagccctgggaatgttcctcggacataaaatgcctggatcgaacaacggaggggcgactgtattttttaccaaacccaacaggggcccgttacaggaagtaatggacctgatcaaagcgaaatatgtagattcactcaatacagacgatttacagcaggaagcgatagaaggattattaacccacctggaccctcactccatatatatacctccttccgaactgcagcgggtgaatgaagatatggaaggtaactttgaagggatcggggtagaattcaatatcacggcagatacagtgaacgtggtgagtgtgctgagcggcggaccgtctgaaactgcaggtgtgcaaaccggcgataagatcctgaaagtgaacgacagcctcgtagccggcaacagcattactcctgaaaagatccgcaaactgctgagaggccccgcaggttctactgtgaataccattgtgttgagacaggataaaaagattaccattcccatcaaaagaggcgttattcctttgtatagtgtagacgccagctacatggcagctccgggtgtaggttatatcaagatcagtaaattctccgctaccacctacgatgagtttatgaaagctatccgtcagctggaaaaacaaggcatggagaaactggtcattgacctcaggcagaaccccggcggctacctggatgcagccacccgcatagccgatgaacttatcgacgaccagaagctgattgtatacacgaagggcaaagatttcccgcgtacggattataaaacgaaacggccgggcctttttgaaagaggcgccctcgcggtacttactgatgaaggctctgcatccgccagcgaaattcttgcaggcgccatacaggactgggaccgtggcaccgttattggccgccgcacctttggtaaaggcctggtacaggaacaatatgacctggacaacggaggcgcactccgtcttaccgtagcccgctactacattccttccggcagaagtattcagaaaccctatggaaaaggacatgatgattatgatgatgacatcattgaacgttaccaccatggcgaaatggtaaacaaagacagtatcaaaataatagatactgtgctttataaaacagcagcaggccgcccggtttacggcggtggcggtattacaccggatattttcattccgtttgatacctcccgctttacacctactttaacagccatttatacccgtaatacgttcagtaactttgcgtatcaatattataccacgcaccgggaaaccttcaagtcctataagaatgcagaagctttcaccaaaaatttccagaccacgccagaactgatcagcgactttaaagcgtacgcccaaaaagacagcgtacctggcctggatcatcttactgcccgtgacgaaacagaaatccgtacaaggctcaaagccatgctggcccgccaactgtacagaacagagggtttctacgaagccattaacgccgaagaccctatggtaaagaaagccctcgaagtagtgggcaaggaaaaaggcgcctctgactaatcgccttcggcgatgcggagtttgtctttctcaggattacgctgattatactgattctctggatttttattccttggatttttttagatttttatttagatttttttataaataattaagggagatagaagtgaatactcacttttatctcccttaatcttttaaaaatcaaatatgatcaaatcttagtaatcagtataatcagcgtaatcctgagaaagacaaactccgcatcgccgaaggcgatcttctactggttcttacgctgcatcttaggcaatgactgaacaatcaggtcgttcattacgttcacggcttcatcgagatagatgtctttggttctgatcctgatccagtccttgttacgggctatcttggaagagtcgctgccaaatttctccatgtcggatttgatgtttacgatattgagttcttttactttatcgtttactgcatcatatttcttgagtgcagcggtgtttgttttttgttctgttttgtaagtctgcaggttcagggaataggtttcctgtttttccagcttctttaaagtgttcaggttttcattgagcagtttaaaggctgggctggtggccattcttttttcgctgttctttttcagtgattctgcatttaccgggttataccatgcggtgaagcttgcgcggggaatttcatcccatgccagtgcgtcagagtctttgcgttcagctatttcgtagtatggatccggcagtacaatatcggaagccacacctttcagctgggtagagccgccatcggcacggtagaatttctgctgggtaagtttcagggcgccgaggctgccaccgtcttttacagggtagaaatcatccaggttgaagagacgctgtacggtacctttaccgaatgtttgggtgctgccgataataacggcacgtttgtaatcctgcatggctgcggccataatttcggaggcggaggcgctgtattcattcaccatgatggctagtggtccttcgtattgtacattcttatcgcggtcgcgcagcactacagcgtcgccaccacgggaacgtacctgtaccacggggccttccggaataaacaggccggccatttgcactacatcctggagggagccaccgccgttgaagcggagatcgaggatgataccttctacgttttctgctttcagtttagctacttctttggcaacgtcttccgcgctgcgggcgccgttacggtcgttgaagtcggcgtagaattccggcaggtagatatagcctattttatgttgtccgttgatgatcgctgatttggcgaatgtttcttcggtaacaatttcatcacggatgatggttatttctttggtggtaccatctacgcttctcacggtcagtttaacgggggtaccttttttaccacggatcagtttcaccgcatcttctacggggtaacctgtaatatccactggttcggtatttccctgtgctactttctggattacatcgttggctttcagttgtccctgtttccagcttggacttccggtaacgatgctgattacgcggattttgtcgccttcttctttcagctgtgcaccgataccaaagaatttaccggccatctgttcttcgaacgcgcgtttttcatccggcgggaagtagtcggtatgcggatccatggtagtggtgatcgcatttacgtagagattaaagcgatcattatcgttctgcctgtttttcagacgttcaaaatagcggtcgtacagttgttttacctttacgcgggcttctgcttccagttccacatcggttttggttttaatactgtcctttcctttatctttttccctcatttcctggaggtccgtcagtttttccagcgtacgatatttcagtactttgcgccaggcttctttacgggcattttcgtctgcagggaaatccactttatccggatccagtgttaccttttcatctacggtgaaatcaaaaggtttggacaggatttcaggatagatcgctgctgcttcagccacccgttgtttgatcagggtgttgatgctgcggaaacagtcgatcggtgcgcctttcagttcatcatcaatatgaacggcgagcggcatgagcttatccacatctgttttcaggaaaaatttcttttccgtatccaggctacgcaggtatttattaaaaacttcggtggagaatttatcatctattgctttaggttgataatgcccttctttcagcatctgccctaccaggttcatgatcacctcgtaacgaccgggaggatcgtcattatgtccgagcttattaaaagccaacacgcctgcggagatgctaagcagcacaaccggtataatcactttcagtctcatatgtatctcaattgaacttaaacgttgtcaaatcaaatataaaataaaatcacccgtcggtcgtgcaatttatttccttttaacaaaaaattgggccaaacgggcaccaggcgagatacatggctgaaaagcgttgcttttcccgctcgctacagtacctgtaagggtgttgttgccggtccttttatacggttccatgacgggagtataccctaagtatacggggagtatcctgggagtatcctcctatgaagggtggacctagtgtaaacgattaaggtggctggaatgttgaaataattattcttttaccagcttatacacggctcctttaaagccactgctgccggaagtgctggcaagcatataaagttcgccctgttcatcctctccccagctgaggatctggaggttatcggcagggcggccggtgagttccaggggagcgctgtcccatttttgcccgttgggcctgagtacaaaggttttcccgttataatcgccgaaaacatataatcctttcagtgccgggatggcgcttccgcgatatacatagccgccggtgatacttatccccacatcgtggctgtattcgtggataggtgcaatcaatgccgacttatcagcaccggcaggcacattataatcgtggttgccttccaggatgcgccagccgtagttaccgcccttggtgatgatgtctacttcttcatacttattctgtccaacgtcgcccgcaaagagcatcctggtggttttatcgaaagaaaagcgccagggattccgaaggccgtaggcccatatttcaggccgggtgtcgggccggttaacgaaaggattatccggcgggatggaatagggtgttccattgacatttattcttaatattttacccagtaaagtattgaggttctgaccattaccgatagtaccgtgtttgtcgccgccaccaccgccatcgccgagtcctatatacaggtagccatcgggaccaaactgcagctggccgccgttatgattggattccggttcatccacttccagcacgatccttttggaagccgggttggccaggttgggatttgctgctgtagtggtaaactctaccaggcggctggtgtggtcgaagccggactttttggtgggcgagctgtaatacacataaaatttatggttcgatttaaaatcgggatgaaaggccattcccagcaggccgcgttcatcatacccgggatttacggagatcatatcgctgcttacatccaggaaaggggtgggaaggagtttattttgctgcacgatccatactttcccttctttctgacagaaaaataacctgccggtaccatcccctggcacggccatatttaccggagatatgaactggtctgttaccagctgcagcttcgctttccggggcgcattagccggaggctccgggccatcatcgttggaattgttgccggcacaggcaaactgtatgaatatcgccggcaataaagcccggaaaatgagggtatgtatttccatagaactgcggtattaatgcagaataaatataaaccagaaatgggaaaagaagaagtgattgtggtgggcggtgaaagcggattgtccgatattctgctgtcgccgtttgtgatttttgtaccttcgcaaaaaactcatcaggttggacactacggcaccgaaaaagaacgacccatacgcttcgctacgctttccggaattcaattattacctggtaatccgctttgcgcttgtatttgcgctggctatgcagtttgccattatagaatggaaagtatatgaaatttcaaaagatcccttctcactgggattgataggtttggcagaagtaattccagccgtgttgctggcgccgtttgccggtcatatggtggacaaacgggagaagcggggcatgctgctcaattgtgtgattgcttatttgtttatcagctcgggattattcctcttaacctgggaccgtgccgtagccggtgtttcaaagcactgggtgctgaacctcatttacctgctggttttcctgggcggcattgtgcgggcctataccagtccttccaactttaccctgatgtcgttgctggtaccgcgtgagttgtatgccaatgcctctacctggagcagttccgcctggcagataggcggtgtactggggcctgcgctgggcgggcttttcattcactggttcggcgtgcactggtcgatgttgatggtggtattcgttttcctggctcctttatacagcttgctgaagataaagcccaagccggtttattataaaccgaagggtgagagttttgtgaccggtcttactgaagggatgcggtttgtatggaaaaccaaagtagttttaaatgcgatggcacttgatatgtttgcagtattatttggcggcgcggtagcgatgttaccggcatttgccacggatgtgctgcatgtgggttccctgggatatgggttgctgcgttctgctcctgcggtgggcgcattagtaaccatgtttatacttgcgcaccggccattggtgaacaaaccgggtattaagctgctggcggcggtattcggctttggtttaaccattatattgtttggtctttccacgagcttttacctgtcgatgtttgcgctgctgatcagcggtgcgctggatggtatcagcgtgatcatacggcaaacgattttgcagttaaaaacgccggacgacatgcgtggccgggtggcatcggtaagttcgatgtttgtaggttcttccaatgagctgggggcgttcgaaagcggctttatggccagggcaatgggactggtgccgtcggtggtatttggagggtgtgttacattgggtgtggtgatcaccacttatattatttcaccggctatgcgtaagctggatctgaagccgtagtggggcggtcagcgctgtgaagcaccaaccgcttccggcacttatctttataaatccatcttttcctttaacttttccagtacataataaacggccgggcaaacggtgctgttttcgtaagtgatcttcgggcgtttaaagaagtcgtaactatctgtgtagggatagttggcgcaatcgccgggacgtacatcatagatgccgcagtagttgtcggcgcccaggaaagggcacggtgtgaacttcaccacatagtcctcatccttatccagccgcaggtaggtttcaatgaaatcgccttccttcatgcccaggtgtttggagatgcgcctgatatcgggtcctttgaagcgggggctgatggttttgcagcagttaccgcactggaggcagtcaattttactgaatgcttcctcatgcaggtccggtaaaagtttctctactccttttccacggcgggtttgcagttttgcgagaaactgtttattcgctttttgcttgtcctgggccttctgttcccagtcttctaatattttgctcatttggtgcaaagataggtaattagtctgtggacaaaattatgacatatacgcccatccctgaagtatcatttatcactgttttcccccgccagtattgattgtttggccgttgcttaaaatctgcatagctttgcgcattctatttcaaattacctgcttacatcatgaatctttttgatattcaacaaaatgaattcgtgcaccgtcacatagggccgaatgaaagagagaccaaccagatgctggaaaccatcggggcctccaacctggaccagctgatcagcaaaaccgttccgggcgccatccgtatgcaacagccactggctattcctgcagcgatgggtgaaagcgattatctccgtcatctgaaggacatatcgctgaaaaacaaagtttaccgcaattacattggccagggttattttgatacgattacgccgagtgttatcctgcgtaatgtatttgagaatccaggatggtatacccagtatactccctaccaggcagaaatttcccagggccgcctggaaagcctgctgaactaccagacgatggtatgtgacctgacagggctgccaattgccaacgcttccctgctggatgaagccactgcagcggcagaagccatgacgatgttcttcaatgcgctgaacaaggatcatgaccatgtaaccaggcctaaattttttgtagataacaacgtatacccgcaaacgctggatgtaatttatacccgtgctaccccgcttcagattgaagtggtagtaggcgattacaaaactgcttccttcgacgaattatactttggtgcgttgatccagtatcccgacaacgtgggtgctgcggccgactaccgtagtttcattgaccaggtacatgccgtgggtgcatttgtaggtgtggcaacagacctgctggcactaaccctgcttacttctcccggcgacatgggcgctgatgcggcctttggttctgcacagcgctttggtgttccattaggctttggtggtccgcacgctgctttctttgcggtaaaagacgactttaaacgttctatcccgggtcgtatcattggcgtgagcattgatgccaacggcggccgtgcgctgcgtatggcactgcaaacccgtgaacagcacatcaaacgtgaaaaagcaacttccaatatctgtactgcacaagctttgctggccaatatggccgctatgtatgccgtatatcatggaccggagggactgaaaaatattgccacccgcatttcgctgctggccaatacactggccggtaagctgaagacgaaagggctgaaactggcgtcagacagcttcttcgacactattgtagtggaaggcgcggccgctgatgttaaagatgctgcagaagcattgggcattaacttccgttatttcgccaatggcaatgtaggtatctctctcgacgaaaccactaccattgctgatgtaaatgatatcctgcacgtatttggcgcaggtactacagatgcagcaaccgtttccaacggtaccaccggtgttcctgctgatctgcaacgtacctctccctacctgcaatacccggtatttaacagctatcacagcgaatcactgatgatgcgttacctgaagatgctggaaaacaaggatctttccctgaacacttccatgatctccctgggttcctgcacgatgaagctgaatgcagctaccgagatgattcctctgagctgggcacactggagcaaaatgcatccgtttgcccctaaaaaccaggtaggcggctatttacagatggcggacgaactgggagaatacctcagcaaaattaccggctttgacgcatgcagcctgcaacccaacagtggtgcacagggcgaatacgccggcctgctggtgatccgcgaataccagaagagcagaggtgaaggccaccgtaatgtaatgctgatcccgatcagcgcacacggcaccaaccctgcatctgcagtaatggcgggctacaaggtagtcattgtaaaagcgctggaaaacggctacatcgatgtggacgatctgaaagcaaaagcagcggcaaacagtaaagacctcgccggtatcatgatcacttatccatctacctatggcgtatatgaagaaagtgtgaaagatatctgcgcaactatacatgaacacggcggacaggtgtatatggatggcgccaatatgaatgcccaggtaggtttaaccgcacccggactgattggcgcagacgtttgtcacctgaacctgcacaaaactttcgctatccctcacggtggcggcggtcccggcatgggccctatctgcgtagccaaacacctggcgccattcctgccaggacacgttacgctgaacgacggcaaaccatccaacgcagtatctgcagcgccgtttggttctgccagcatcctgctgatctcttacgcttacatccgcatgcttggatttaaaggcgttaaactggcgtctgaatttgcgatcctgaatgccaattacatgaaagcacgactggaaaaagcatacgacatcctgtataccggtgttaacggcacctgtgcgcatgaattcattgtagatctccgtccgtttaaagcagctgccggtattgaagcggaagatgtggccaaacgcctgatggattacggtttccacgctcctaccatgagcttcccggttccgggtacgatcatgattgagcctaccgaaagtgaggataaaggtgagctggatcgtttctgcgatgcaatgctggctatccgtgaagagatccgtgcggtagaacagggtcagagcgataaacaaaacaacgtactgaaaaatgcaccgcatacccaacaggtgatcactgctgatgaatggacccgtccatacagccgccagcaggcagcattcccactggaatatgttaaggcaaataaattctggccttctgtaagccgtatcaacaatacattcggcgacaggaacctgatctgtacctgcgaacctgcaagtgcctatgaggaagcagcagtataagctgttggtttaatattaaaagagaaggggatagacatggcgtctgtccccttctcttttttatgcagatatataacagttattgtaagacaggctccagtacttccaggcgcccgtcgataggctgtgtaatatccaggccaagtattcttgctactaacgggtacacatgtacgttttcaaaagtggcaatacgggtatggggtttaaaggccgggccccaggccatgaatatagcgttcatgttggtgaggttattatcataaccatgatgaccgggatgtgcttcttttgccggtgtaaatatatagttggcttctgccagcaggacaatatcaccaatacggttgtaaatatcttcctggccatagtgccatctttccggtgtttcctttttcaggtaagcggtataatgattttcgtgttgtttgagataatcgtaagcggttttgatttcctcatcggttttaccgtatagcattaccttttcgttccctggcatacttttcaggggttgcagagcgggtacatctggcagggtgatggtgtgagtggtgtctgcctgcatcatgccgtgatcggataccacgataaaatttaccggcaggttcagctgtgctacagctgtcaccattttaccgatggcggcatccacgaattgtacggcgctgcgtaggctgtcggcgtccggtccccaggaatgccccatgtgatccacttcggggaagtagaaggtaatgaagtgcggccgttggtcttccggcaggcggagccagtttactactgtttggatgcgctgatcgatacctgttttttcctgatacttaaaatagtaagtaggacgtatattttgaatggcgctttctgatccaacccagaaatagctggcgctgagcatttcctgtttctctgccagcacccataatggcacgccattgtaccaggtaccatcctccacggcatcgcggttgcctactttataaacggcatcccgtttacggtcgtaaaaaagattatccaccaggccgtgatgagccgggtaaagcccggtggccagggaataatgattgggaaaagtaagtgatggaaatgccggctgcatggcggtagcgcgaacgcccgctcctgaaaggcgcagcaggttttgtgcgttgtatttttcggcgtaatcataccggaagccatcaatagaaatcatgatcacatagggcctcgattgctgtgttgcgctgttcttccttccttccaccaccagttgggcagtatcctgggcatagccggcaaagctgatcgataacaggatggcggctaataaaaaaatccttttcactatttacgatgtttatgattgcatagtaataattggggaagaataacagatgatgggttataatgcggggcaaattagaaaactatttccattcaaaacgggatcagcaattatatatccgttaaaaaaggacagttgtgagttaccacaactattaaaatctccataaacatgtaataatattttaacacatattttctcaaaacagctatatatcagcaaaatgataatcactaaataaaaaattatatatataattttaattaattaattgtttatctatatattagcctactgaaaaaccatctaacaactatgtctgattacacctttattacaactgaggaacattttttattacaggatgcgctgaagaggaacaagcaacagttaacaaaattcacccttatcggttttgggctattattgattgctgcagtgataccgcaaatttatttgtacacccacaacaacctgggtgatgcggatgattcgctcctgtcgttcaaaaacctttggttctgggtatggctgttatgctttgtgatagcgttgatatttgcgttgataaaagtaacggatatacgctactgggctattaaaaaggatttgtcggccttgcagaaaggcactttacaggcgccgatggaagcggtatacctggaaaacaatgatacgcaaaccaatattatgatcctgctggagaataaaaagaaacgcctgttttactggatgcgtggggcattggaagggtacagggccgggcaggaagtggaaatcacctatgcccgttattcccgcgtaattatcagtatcaacaagaaataatttaccaccgttttgaaatgccggccctgtgcgtgagcttaacagctgacgtgcagggctgtattatttgcaaaatgtaacatttagccggtaaaagcgtttgtatcataaaccctgtacccgtgggggatgcgcttgataatttgatgttgtttttctccgggaaactatctataaaacagtatttttaaccaggttgttaatgcgtttacttttgctacatccaataaaaatcctactgtattgtactgcgctgttgctattcatcatagcgcccgcctgccaatgcaaaaaggataatagtgttactcccccaccccggccggaaccaccaaaagacatttacctcgttacctccatccgtgtgaataacgtaccgaaagacagcctcgtttataacgatcaccaccaggttacagaaagatgggactataatacatcatacaggatctggcaaaattatgtggcctaccagtacaaccaggaaggttatgtatcaatggccagatattacaccgaaaatgataataccatcaaaagtcttagccagaaggactctgtagcgtggacaacagacaggtttattgtttacaccaccttttacagggaactcggtaatgaaatttccggatacgatacgcttggttatttacatataaacaatcaaaaactgctcaccctcgaaggtactaaagatacctttcttactggtgtaggggtggcggtgttattcaaacaatatcaatataacgggaaagatgtcacacagttccttgattggaactggtaccatgtatataacgggcaacccattttactcatgaacaaatttgacctggcgtatcttccatttgagaaccccttgtttccacaggtatcaaaaaatccgctgttgttccgcgccattggtggtgataaatttccttatccttccaacgaatattacccttacctcttgagtgaacacctggcaggtgcttttacgtatgaagcagatgatataccttcgaagatatgcccggtaacctataaaatgtatgataccacgcattatccacaaacgcaaagcattgcaggcatcaataaaacaattgattacacttataaagtgattaaagcagagtaagaacccgattatacccatgaaatacattactcaactggcctttgtgcttgcgatacttagtactgccggatgcagaaaaaaagatcggcctaaagaagcgaccggaccggcgcccttagaagttacccgcctgttgacgttcatttataaagataatgttctttatgagcggctggactataacaacaaacaactgaccacctggcatcattttgaccccaccactgaagtaaataatatccgtctggaatttaaaaccgataccaacggaaagctaataggaacactcctttaccaaaaagacggaaccggttttaagctgatagaaaaaaatgaggtacaatcactcgaaaaagaatttaagataacaggaaacctgtatcggctatcctccggaaccccggacacgataccggatgccatgcgatttgcatttgatgacaacggcagaatgattgaactcacggatacattgacaacggagaagaaaaccgattatctgagtcaactcatagtcatcactacctgtaattattctggcgatcagctcaacaacctgacacgcaaagcttacaattattatgtttcccccacactgcctggcggagaaaaaatcaatctgtaccacacaggtatatttcagtatgaatacgatgatacacccaactttttctatgcccttggcaaacgatatccttatctgcggtttataatgacgccggagcatcctttatttgccggccgcaccaatgtaaaaaaaataacgtatcctggtggccagactgaaattatccatctctttcaggatacccatgatgaccacgacaaccatatcatatacactacagaggtgactctaaacaatggtgttaccaatagtaccacccattggcagtatcattatatccttctcccataatttccggaaattttcctgacttttgtaaccagatataattgttactcatgaaccttgcacaatttcaggaatattgcctttcattacccggcgttacagaagagtttccttttggagatgaaaccctggtatataaagtttgcggaaaagtatttgcactcagcggcctttcaaattttgaatccattaatctcaagtgcgacccggaagaagccgttgaactacgggagcgctatgaaggcgtgatccccggctatcacatgaataagaaacactggaatactgtggatgtacattccggtatccccaataaattgctgctggaatggatccggaactcgtacaacttagtagtggcgagtttgccaaagaaagaaagagagaaactgggccaataaccgttccccatatacctggcaatcatcccccgtttttttattacattagcccgaaatctaaatctaaaataaactgtttatgagaaaatggctgctgctggcctgtgccgcgctgtttgtaattccggtggcatgtaaggccgttaaccaggattcactctggatgtatgagcactacacaaaaaaggaagtatacatcaccatgagggacggtattaaattgtttacctctatttacctgccaaaagatcaatcggagaagcatcccatcctgatgacccgcaccccctattcctgcgcgccttatggcgaaaatgtcttccgtccgttgtataaaaatcattacaaggaatacctgaaagaaggctacatcatggtcatacaggatgtaagaggcacctggatgagtgaaggtaaatttgtaaatgtaagacctttcaatcccgctaaaaaagggaagaaggatattgatgaagccagtgatacttatgatacgatcgattggctcgtaaaaaacctcggtggcaacaatggtaatgttgggatattcggtatttcctatcctggcttctactcaacaatgggcgcgctgagtggtcacccggccctgaaagccgtgagtccgcaggcgcctgttacggattggtttttgggagatgattttcatcacaacggtgctttctttattgcagatgccttttctttttataccgtgtttgaccatccgcatcccaaacccactacggaaggaccaaaaggtatcgactactatacgcacgacaattacaaatactacctggaaaccggcgcgttgcccaacttcgccaaaatcatcggcgacagcgtaaccttctggcatgaaatgtatgcacatcctacttatgacagctggtggaaagcccgcaacgtgcgcaacttcctgcaaaatgtaaaacctgccatgctgattgttgggggcgtgtttgatgcggaagattgcttcggcgcgtggaatacctataaagcaattgaaaccaaaagtccggctaccaacaaccgtattgtaatgggtccgtggtaccacggacaatgggcatccaatgatggtacccacctcggtaatgtgcgctttggcagtaacaccgccgaatactatgcgcaaaacgttgaaattccttttttcaactattacctcaaaggcaaaggcgctgcacctgatatcgcagaagccactattttcttcaccggcgaaaacaaatggaaacaactccctaaatggcctccggctaacatggaagatgcaccggtttatttgcaggaagatggcaagctctcttttaccaagcccgctgctgctaatagtttcagcgaatatgtaagcgatccggccaaacctgttccatatacagaagatgtgcattttggacgtaccattaactacatgaccgacgaccagcgctttgccgcccgcagaccagatgtggctgtatttgaaagtgaagtactggataaagatattaccctggccggcccggtagtggcagacctgattgccagcaccagcactacagatgccgatttcattgtaaaagtgattgacgtattccccgacgatttcaaatatgaagaagacgcgcctaccgaacatcgccgggtgccttctgccacttacccgatgggcggctaccagatgctggtacgtggagagatcatgcgtggtaaattccgcaatagctttgaaaagccggaagcatttgttcccaatcaacctgctgaagtgaaattcacgatgccggatgtagcccataccttccagaaaggacaccgcattatgatccaggtacaaagcagctggtttccgctgacagaccggaacccgcagcagttcatggatatttacaaggccacagataaagattttaaaaaggctactatccgcatctatcacgatgcacagcatccatccaatgtggtgctgccggtagtgaaataatcaattgccgggatgatgccgatggcatcatcccggtattattaccaccgtacttttccaccccctccccattcgatccagtcggaagctgctccgtttacggttttaagtccgagttgtaaaaagccgtatttagcaatgttataacggatagccagccgcataaaataatcgcctttttcattatctcttttccacacgtaagtacccacctctgcccttacctggaaacgcttaatatttaatacataggccaggtgtgtgcccatcagcattttatcgctggggcgaacttcgccgtagcgctgctggtaggtccaacccaaggaaccgtcgtagaaaccatccatgccaatgccaacgctgcttttatgactgaagcggtaatcataacccaatatcagggaggcggtgccataaaaggcttccagcttttcatcgctggaggcctgcactacaccaaaagcgccgtataaactgatttcatgataacgttgcagcggtggcaccggcgttgtaatgaatgtagggcggcgtgcggcttcgtatgtggggtcaatctgttgctttacgatactgcggatggtattataatgataacgcacgccaatattcaatcccgccatattgagccccaggttgggcgtatgggtgcgcccgtttgaaaaatgggtaagatcaatgccataaagaaaatcgaatgaattcgacactttcagcactccggtgatgctgaaattaacataggcatccagcttagacccgatggcgtcgttgagcgggttggtagtggagtcgtaagggttcaggtcgtatgtgataccgagcgacagacccgcttcaaagtgatttcttttccggcggtggaagggcgcataaaaaaaaccgtacaccccgctggggttgccgagaatggtagggttaccgatatcgccggtgtagaatccaatgccataactgggatagttgaatacccgctgccactctttttccccggtcgactgccaccccattctcagttccagcgacttataaccgtcgttcagcgcgtttttcagctcatcgctggtataaagatgcgtgcccccgtggagtttcagttcaataaacttatgtcttcccaggtttggattcaacctggcttttttccacaaatccgtggtatcctgtgccggcaggcatctcccgtaaaataacagtaaaacaaacagggtaaatttccacataataaaaacagatgaaaacaaggtaacgtaatcgaatgttcatctctgcaaaaggcttgcctgtgaaatattatattgattaacttgcagcatctttaaaaagccttattttaactaacatttctgtctattatttatgatgtacaaaaaatacctgttcataggagccctgggatgcttatccgtacaaggtttcagtcaggctaaacctgcacctaagaagccagtggccaaaacagccgttaagtcgccggtattgaaaaacaaactggattccgtgagctacggaattggggtgagtgttgcggaaaacctcaaagcccagggactggaaaatgtgaatcctgccctcctgtccaaagcggtacaggatgtgttgaagaataaaccattaacactgtcaaaagatcaatgtgatatgagcataagtaattatctgcagcagctgaaagcagacaaagctgccaaaaaccgcgaagcaggacttaaattcctggcggagaataaagtaaaaccaggcgtggtaacactgcctgatggtttgcagtaccagatcctgaaagaaggcaatggccctaaacctacagccgccgataaagtaaaaacgcattatcacggtaccttaatcgatggtacggtgttcgatagctccgtagacaggggacaacctatctccttccctgtgggcggcgtgatcaaaggctggacagaagcgctccagttaatgcctgtgggctccaaatggcgtcttttcatcccttccgagctggcgtacggcgaccgtggtgcgggtccgaaaatcggccctggagcggcgttaatattcgatgtggagctgctggcgatagagcagtaatgcagcgggtgggcgccttcatagcgccttcggcgcttttaaattgtcttggagcaggattacgctgattatgctgattgagatgattttcccaccttttgttgtttgatattttgaggggatatgaaagcggatatttgattttattgattttttttacctttttgtaataaaatattttggtgagataaaagcggatatttgattttattataaccaccagattaacaaaattcggggagatagcagcaaatgtttttgctgttatctccccgagatatttagtcaaaaaatcaataaaatcaaatacccactttcatctcccctcaaaatatcaaacaacaaaaggtgggaaaatcatctcaatcagcataatcagcgtaatcctgctccaagacaatttaaaagcgccgaaggcgctactccgctctaaacacccgcgggcggcgctgttccagcaggaagaagtcggccagtaccatagcggtcaccgcttccagtaccactggtacgcgcagcgcgatgcaaaggtcgtgacgccccttcacgctgaaagtttccacttctccgctttttatgttgagggtttgttgttctttcggtgtgctggaggtaggtttcacagcgatgcggaataccagcgggttgccattggtgataccgcccactacgccgccggcgtgattggaggctgttttaccggttgtatcgacgatgggatcgttatgttccagtcctttcattttagcggcggcaaagccggcgccaaactcaatgcctttgatagcaggaatcgcgaaaacggcatgcgccagtgcggattccagcgaatcgaagaagggttcgcccaatccaatggggaggccatttactacgcactctacgataccacctaccgaatcttttgctgcaatagctgcttccagcccggcttccggatcggggttgccccctacttccgtgatagtagcgtttacctggatttcttcgcccaggatctttttagcgattacaccggcggctaccaggttgagggtgagcctgccgctgaaatgtccgccgccgcgatagtcttcaaagccgccgaacttttcggtagctacaaagtcggcatgccccggacgtgggaattcccgcagcttttcgtaatcagtactgcgggtattgttattttcaaaaagaatagtcaccggtgcaccggtggtgaaatcgttaaaaacacctgacttgataaagggcaggtcttcctctttgcggggcgtagtgcccctggagccgcctttacggcgttccaggtctgccaggaaatcttcctgctttaacgggataccggcaggtataccatctatatttacgccaacgctggcgccatgtgattctccaaaaacatttaccctgaataatctgccaaaactgttcacacgctgatgatttaaagtgaaattatacggttactgccactttaccacccagcaattccaggtggtcataaaattccgggtaggatttattgattgcttctgcattgtcgatgatcaccgggccatctgctgtgagggcagctactgcgcaggccattgcaatacggtggtcgttatgtgaatgtacgtgtgcgcctttaatgccggtgccgccatgtaccagcatgatatcgccttcgaggtcaatgctgatacccatcttgccaaattctgcctgtagtgttaagccacggtcactttctttatgggctaaacggctaacgccttttattttcgtagtaccgttacagttagccgccagcgctaccagcggagggaacagatcggggcagtcggtggcatctatttcaaatgcgttcaatccgcctttttctatgtttacggtgaatacgccggacattaaatgtgccccggctttctccaatgcttccaggatggctttatccgactgggcagaggaggtgttgagatgctgtacttccgctttaccggctactgctgcagcaaccagcaggaatgcggcgccgctccagtcgccttccaccgtatagtcgcaggcgttatatgcctgtttctttccgaaatgaaaggtttcaaaattcttttcttccacctgaacgccaaaatgcgccatcagttggagggtcaacgcaatgtatggtttgcttttcaaatctgttacggtgatcgttacattttctgcggcagcaccgtaggccatgagcaggccggtgaggaactgagagctgagagaaccatcaatcgtaatatctttcggatgtaacgggccctcgatatgcagcggcaatttaccgccctgcgtggaacactttacatccagttgtggtaatacttcttcaaagaaatccatcgggcgggtagttaaactaccgtggccttctatggtgatgggcagtgacgacaacgctgcgatgggtgtaaacatacggatacccaaaccggattcgccgcagttgatttcatcataaaacggtgctacaccgttgctggtgatttcgaaatagtcgtattcccgtttgattttagcacccaggttttcggctacttccagtgctgccaggcaatcattgctcaggccgggattacggataatactcttcccttttgccagcaaagctgctgccacagcgcgttgcatggcgcttttggaaggattggccgtaactgtgcctttaatgatggctggtgatacagtaacttgcatatgtatatttcgtctgcctttaattgattagaaaaaaatttacaattcctgcagtaacaacttcagttctgcaatgggaacgggcatggtggttgctttcccgatctgttccagcaacacaaaatgtattacatctttctcccgttttttatccagtttaaagatgtcgaacaccgcgtctttatctgaattaaaagctacgggcagctggtaatcgctgatcagttttatcaggcggatggtttgatctgccggcaggttcatcagcttttccgagaagcgggcagctgctaccattcctatcgctacggctttaccatgcgctatatgttcgagtttttccacggcatgcccgagggtatgaccaaagttgagccatctgcgggggccgatttccagctcatcttccagtactactttcgtttttgctgctaccgatttttccaccaggtattgcagtacttccacatcacgggccagtgctttctccctgttattttcgagataatcaaacagcgtggcatccatgatacaagcgtatttgataatttcagcaaaaccgttgtgccattcttctgccggcatggtgaggggcagggtgtaatcgaagaggataaactccggctgacggataatgcccagcaggtttttctgtttaccatgactaaccccgttctttccgccaatggaggcatctacctgcgctaataaggtggtaggtacaaagccaaagggaatgccgcgcatgtatatgctggcggcaaatcctgccacatcggtgagcattccgccaccaattcctaccagcgttgttttgcggtcggcttcgtaagcaataagaccatcgatgatcttatctaccgtagccatattctttaattcttccccggagggcaccacaattttgttccagttgtgcagatgatgaccgtgatagtattctacattttcatcaattaccagtatagccctgtgacggtttacatgattgcccaactccatcaggcttgctcctaaaaaataggtcgtttcctgttgttgaaactggtgggtttgtatgagcatggagcgattagctttagctgtcagaaaaactactgccggctgttgtgattgtccaacagccggcggctgatggatctacttatcttcgttcattactttgttctggcggttgatggattccaggtgaactgcatcgaaatacttcacgatgaagtctttggtcagacccagcttctcacccttagacacagcgcggtccaggatttcattccagcggtttgtttgcaggatggtgatgttattttctttcttgtacacaccgatcttttctgcaattttcatacggttgccgagcaacagcataatttcatcatctacctggttgatctgcgcgcgcagtttttccagtgcggagttgaaatcttttttatcggaatgttctcttctccaggtgataccatccagcaggtctgctaatttttcaggcgtgatctgttgtttagcatcgctccatgcgttatccggatctacgtgtgtttccagcatcagaccatcgtagtcgaggtcgattgcttcctgggaaacttcctgcaggatatcgcggcggccggagatatgcgaaggatcgcagatcattggcagttcaggcatacggcgtttcagctcaatagccaggtgccacatgggtgcattacggtattgggtgttgccatagctggagaagccacggtgaattaaaccaactttattgatacctgctttctggattctttccacggcgccaatccacagttccaggtcaggattgataggattcttaattaaaacggtagtgtccacacctctcagtgcatcggctacttcctgtacagagaaagggtttacggtagtacgtgcgcctacccacagaatatccacaccgaaatgcagcgcgtcttccacttgtttggcagtagctacttccaccgccagtggcaggccggtgatttcacgggctttctgcagccatgccaatccctttgtaccgatgccttcgaaagaaccggggcgggtacggggtttccagataccagcgcgtaaaacgtccactttacctgttttctgcagggccagtgcggtggctaatacctgctcttcggtttctgcactgcagggtccggaaatgatcaacggctttttatcggaagacggatcggagaattttgttttagataatatctgttccattgtctgtaccatagtattgaagttaagtagattatcagaatttagttatttcaggatcttcctgattttattggatttttgaatcaatttgtaaaaggtgtcgtagtcttcgttttccagcaatgttttcatttgctgtaactggctgatgtgctcttccagtacatcaagtacattgttccggttgtgtttgaagataggtacccacatatcaggggagcttttcgccaaccgcacggtggattcaaaaccaccgctcgccagttcgaagatgcgtcctgactccttctcttttttcagcacggttaaggccagtgcaaaagaagtgatgtgggaaatgtgggatacataagcggtgtgcagatcatgttcttccgcattcatatatacggtgcgcatctgcagccggtctaccatgttttccactacttcaagtgcgtcttcatcgctgtttttcacatcgcagagcaccatcgttttgttaacgaagagattgcgtacagcagcatcggggccggaatactcggtgccggccatcgggtgagccgctacaaagcgtcctctgttgggatgaccggcaacgagttgcagtattttttctttggtagaacctacatccataatcacctggccggggcgcgctttatccatgatggcaggcagggcttgcagcactgcatccaccgggatggccagtattaccaggccggagcgattcatggcatcctccaggctcgcgccttcatcaatgatgttcagttccagtgcccgttgcaggtgctcctggttctgatccaccccgatgatccgctccgccacgcctttttccttcagcgtgatggcgagcgagccgccgattaaacccgttcctattattgttgcaatcattttacgttggttttgatacgttctatcgcttcctggaaaaccttttcatcctggcataaactcaccctgatatagccgttaccgttacttccgaatattcctcccggagtaatgaatacacgtgccttctgcagtatttcatcagtgagcgtatatccgttctcgttagtggatggtatcttcgcccaaacgaacatgcccacctggtttttatcgtaggtgcaatgcagcagatccagtaactggaatactttttccctgcgtgcacggtaaattttatttaagtcgtcgtaccagtcttttcccagctgcagtgcttttacagcggccatctgcataggctggaacataccggaatccatattgcttttgaagcgcagcacctgtgcaatccattctgccttgcccaccagcataccgatacgccatccggccatattggatgatttgctgagggagttcagctccagcaccacatcttttgcaccttcaaactgcagcaggctttcgggttgttcattcaggatgaagctgtacggattatcatgacagatgaggatattatgttgtttggcgaaagcgatgagctttgcggcaaattccctgtttacttttgcgccggtaggcatatgcgggtagtttacccacatcagtttcacgcggctcaggtctttttgtgccagggcatccaggtctggcagccagctgttttcttctgtcaggtcataatcaacaacagtagcgccactcaggttcactgcggagcggtaggtagggtaacccgggttagggatcagggcctcatcaccttcctgcaggtaagtcatgcagatatgcataatcccttctttggaacctattagcggcaatacttccgtatcggggttcagggttacgttgtaatagcgttgataccagtctgccatcgctttacgcagggcgggaatgcctttgtatccctggtagttgtgcgtattcggcaaagcggcattttcgttcaatgcagccaccactgaaggatgaggaggcagatcggggcttccgataccgaggttgatcacctttgtgccggtttggttcatttcctcaatttccctgagctttttggagaagtagtattcttctgtgccttgtaatcttttagcaacctgtatctgcataaaactgattaatgtgtttttccttttttataaatacccagcactttcaggtgttctgtgagtggctctattttcgataatgctttttcgaagtgagcggcgttatcaaattccatgtcggcgtggaagtaataattccattcttttgccggaatcggaaaggattgcagcttcgacaggttgatgccggccactgcaatctgggtaagtactttagccaaactgcccctgtcgtggcttgtttgaaagtatacagatgctttgttggcatcttccggcgtagcgatgggcgtacgggatacagccagaaagcgggtatagttatttttattggtgtggatattaggcgctatgatatccagttcaaagatttcggcggccagcttacctgcaatagcagccgtacttttcagtttcttctgtcttacgtgcttggcactgagggcggtatcttctgtttccaccagtttgatatgcgggtatttttccaggaaatccatacactgcaaaagggccatcgggtgagaatgcacctccctgatatcttccattgtttgcccgggcaacaccatgaggtgctgattgatctggagataaatttcaccggtgatatgcagaccggagtttttaatgagactgtagtttggtaagatgctaccggcaattgagttttcgatggccatcatacctgcatccacatcggtttgttgttttgcttttttaaccagttctgcaaaggaggcacagcattctatttcagtttgtttaccgaaatacccctgggcagcaacctggtgaaaagacccttcaaacccctgtatggcaattttcatgtgtatgtgattgattttattcagttatagttgctacagcaactagctatttaaaacagaaagggtcccgatccgggaccctttgcgctgtacttttatatgtaagtatgttattgcaaacgagtcccctgcttcttcgcataaaagaagtaagagaagtaataaaaaaagtatttgcctgaaactggctgtaacatgtacttatttgtttgttggcatccactgccggtcatggtattaaaaaaggccttccggttccggaaggcctttttgtagttcttttatcttttacaaacgacctccctatttctggtaccagaaataataaaagctaaaaaagccgaaagaggtttgctgcgtcatattattatttgttactcgttttgagtgtaggacaaaaatacggcacgattttaattatccaagggctaatatcaaaaaatatgctttttttaataataaaggtcctttattgaataactttcaaagaaacatatttccgtaaccaaaaacagggcataaaaaaaccgttcaggctaagccggaacggttaattataaattctaaagtcagattagtgatgagcagcagctgaatcaacagttttagcagtagaatcaacagttgcttttgcagcgtcagctacagagtcaacagctgaagtagctacctgagcagctgaatcgatagaagcaccagcagcgctagcagtagagtcagtaccattttcagtttttgcaccaccgcaagcaactgcgaacagaccgaaagacagagctaagaaaccaattttgattacgttcttcatgttacaattatttaagttgtttttgaatgatttaacctttataccgggatcacctaaaaggtaacccaaacttttaaaaatattttttttcgctactttgggttaccaaatgcctaataactgtattaagagtgaagcaaaatcaagacataacaagagaccgggaattattgctgggactggcaaaaggcgaggataagtcattggaaatcatctattctgagaattttccggtggtattacgaatgatccttcagcataatggctccgaagatgacgcaaaagatgtgttccaggaggccattatagtattatatgaaaaggtacaaaccagtgattttactttaagcagcaggctaaaaacctttctttattcggtttgccgccatctgtggcttaaaaaagttcaacgtacctacggattatatgctttaacgcccgaactggaagaagtgattccggctacggaagagctggaagagcacgatgcaaaggatcaggaattcaggatcatggaaggcgcgatgagcaatattggtcaaccctgccaaaccatcctggaagattattatctgcataaaaaatctatgcaggaaatagcagaaaagttcggatacaccaatgctgaaaacgccaagaaccagaagtataagtgcctgatgcggttgaagaagttattttttgatcaatacaaaacaccactataagcagaaagcagccatgaaagaagacatgatcttattacgtgaaattgagcgttacctggaaggggaaatgagcgaacaggagaaaactgctttcgaaactttacgtcataccaatcccttgattaacaaacaggtagaagaacatcaactgttccttcagcacctgggcaattacggcaaacgccagcagttacaggcaaagctcaaccagatacatcaacaactggatatgccaagcctccgcaaacaggcacaggaagaaaaccagactgcaagaagattaaccatccgccgcagaaccattacgaacctggctgccgctgcctgtatagcactggttacttctttatccaccattgcgatcatacagaatgtatctaaaagtaaatcaactgcacaatacgaagatgtaagaagggtactgaataatattcagcgttcccagaatgcactcatcaacgatatgaacagcaagagccgggctccgttaaaccccggcacttatggaggtactggtttcgcggtatccggtaatggctatatcgttaccaactatcatgtagtagccggcgccgactccgtatatgttcagaataataaaggagaggcttttaaagccatcagcatatttgaagatatttccagtgatctggcaatactgaaaattgcagattctacttttaaaagtcagcccctgccttatgctttgaaaccacagagcgtaaaactgggcgaagaagtattcaccatgggattcccccgcgatgaaattgtttatggcaaaggttatatcagcgccaaaacaggttttaacggggataccactgcctaccaggtatctatcccggtgaacccgggcaacagcggtgctcccctgctggatagcaaaggagatgtagtaggaatagtaaccggcaaacaaactacttccgatggtattgcctttgcggtaaaatctgcccacctcaaacacctgctggatgagatgccaaaagacaaacaaaccaggaaggattggaatcataagagccgcctggaaggaatgaaccgggtagatcagattaggaagctggaggactttgtatatatggtgaaggtgtataattgaaccaacacctattaacataaaaaagcgcgggatataacgattgttatatcccgcgcttttttatgttccagcctggttatttcttcaaccaggatttgtatttatcagtaatccagtacaacagatcgttgttattaatggtacgcatggtattataatcaggataattatccctcataaacaactggagtgagtcgcctttaagccctgttacccggcttaccaataccggtgtaaagcgggagtctataaacttctccttttccatcttctcataattctctttaaactgccgtttttgtttttcttttttggagaaacgggtaatcggactaaacacaataccagcaccttcaggcgtactaccgccagccaatggcttgtttggattatccaggatatagccgtactggttacgtctttccattgaatctatctggtaaggactgtactgggaggtgatttccactcctttcaggaacttaccggcagattccatcaccacgttaatggtttgagtaccggaagtttgggtaacaatgatcgtatccggcttgtaccctacgaaagtaaccaggagccggtcgttgcgggaggctgatatcctgtaataccctccctggtcagaaagcgaccgcttcccggagttgagattgctgacggtggcgtagggcagcaccagcttgttgctgtctgaaatcatcccggtaacagttacctgggcctgtacctttggagcaaatgccatactgaatatacagcctagtgctatgatgcgcatgaaaaccttcatataaaatataataatttttacagccgaatcccttccattctttacaaacagatcagtatagacattgttcatctaccctaatgaagtacaaattaaagaaaatgccacggtgttttaaaaacaaatccttccaccccgggggcggaaggatcgctgtatttaaaatttcaggttgtaccaatcaggcagacttcagtaaatcgatcacttcgtcccggcttttacccaatttctgctgcagttttccgatcaatttatcttcttgtccttcttcgtacaacaggtcatcgtcggtcaggtctgcatacttttgtttcagggtaccttttatttcgttccactttcctttgatctgtaacttgtccataatctttcaatttatatggtgatataatcgggttgcttatgaacatgaagagccaaagaatatgccatcacccttattttataaagatacctggatgcgggtactgaaaaccctgctttcgccggcagccagctgaaccagtccgagtccgttgttaaaggcgtccggcgcgccgctgaggttttctacagcgatgctggtacggtgcggtggaatatatatctgcaggatgggatagctattttcgggatagaaggcaatgttgatatttttcttcggatcgtggatcgtggccagcggttgtggctttgtgagatccagtacaaaagaattatccagctccacgtctttcaacacctttccttcaacaaattcggtatatggcaaaacgtttcctgtaggcagcagtttttcattgaactccactatttctttggaagcgaaggtaagtaccagctcatctaccggtgtacctgtgctgaagtatggatgccagccatccatcacgggaatggcaacgccactcttattcacgagcgtggtattcagctgcaggtcgttgccggcccgcagggtaaaggtagcgatgcagtcgtatgcaaaggggtaccctgcatcatcggtttgtttaaaatgatgggtaagggttaccgatgcctgctggtcatctgcctgttgcgctgttacggtaaagggcgcatcatataataagccgtggatggcatttccgggtgccaatgttttctggatagtgtagggtttgccttcccaggtatattgtgcatccttcatgcggcatgcatagggactaagttttacgcttttgaagctggtgcggagatttgcttccaggtcggcgatatctttgtaactatctatcagattcagtggtcctgttgtatgctttactttgaaagcgtgcagcagtgcgccgaaagaaggaattatttccacctgtgtacctgcttcgagatcctggagcgcaatgatgtcaaatcctgcctcttgaaaagaatggatgccaaatttcattgttcattattttggaagaaaaataaaacattttgggattttactttgggattatttggtaacagccatttgttgctaccggtaatccaaagaaaaatcccaatagtatattagatgcttgcgttgatcaggttttccagccattcctgtttgccgctggtttgtttaggctctccatttgccactgcaaaattgcggaggtcttccaatgtaagtttacccgcttcaaattcctgtcctttaccgctgtcgaaagacgcgtaccggtcctggcggaattttttatacggtgtggcggtcaatactttttctgcaacaatagcagctcttgcgaaagtatcgatgccacctatgtgtgcgtggaagatgtcttccaggtcggtggagttacgacgggtttttgcgtcgaagtttacgccgccgccggcaaatccgccagcttcgagaataaccagcatgctttcaatgaggtcgttgaggttggtgggaaactgatcggtatcccagccattttgcgcatccccgcggttagcatcgatgctgcccagcatccccgcatctactgccacctgcagttcgtgctggaaggtatggccagccagtgttgcgtggtttacttcgaggttcagtttgaaatctttatcgagaccaaactggcgcaggaagccgatcactgtggcggcatcataatcgtattggtgcttggtaggctcgcagggtttaggctcaataaagaaggtgcctttaaaaccctgtgccctcgcgtaatcgcgggccatgcccaggaaacggcccagatgttcctgttcgcgtttcatattggtgttgagcagggtcatatatccttcacgaccgccccagaatacatagttttcgccgcccagtgcgatggtggcatccagtgaatttttcacctgggtacctgcataggccaatacggcgaaatcaggattggtagcagcgccgttcatatagcgcgggttactgaatacattggcagtgccccataacagttttacaccgctggcttgttgtttctgtttagcataggcaacgatctgctgcatacggctttcatattctgcgatgttggcgccttcgtctaccaggtctatgtcatgaaagcagtagtaaggaagccccattttggtaatgaactcaaaagctgcgtccatcttgtctttagcactctgattcgcatccggggaagcgagccaggggaattgtttggtaccaggaccaaaaggatcaccacctgttccgcagaaggtatgccagtaggacacggcaaaacggaacagttctttcatagatttacccgcgatgaggcggttttcatcataccatttatacgccagcgggttatctgactgtggtccttcaaactgtattttaccaatccctttgaaatactcgttgtttcctaatgtaatactcataactaatatggttttttaaaatgccagatctacttatatgtttccgttaatgcatcagggtacgaagaccgttcagccagttgccataaacatcccggtattgtgattgcagggcgggatccggttctattactgcgaggcattccatgccacggaaagcatctgccatgctaacataaccggcgcctattgctgcgccgcgggctgcgccctgtgctccatctgtattatatagttctatcacaacattggcggtattggaaaaagcttcccggaataaggggctgaggaacatgttggcatgtccggctcttacgcgatggatgctgaggtccatttcagccatgatatccatgccatagttgagaccaaacacgatgccttcctgtacggcacgcataatgtgcgcgcggctgtggcggttgaactcaaggttgcggagggtagcgccgaggctcctgttttccaggatacgttccgcaccattgccaaaaggaaatacctgcaggccgttggcgcctatcggcgcctgttgcgccagggtattcatttcgggatacgtgatatcacctaccaggtttttgagccagctgttggcaatgccggtaccattgaggcacatgagcaccccatttctcgtatgggcgtggtcgttattcacatgcacaaacgtgttgacgcgactttgctggtcgaagctgtttttatcgtgcacggcatatacaacgcctgaggttcctgccgtggtggcggcttcaccgggttgcagcacattgagagaaaaagcattgttaggctgatcgccggcgcggtaggtaaccggtgtgccgggcgccagtttcagtgtagcagctgcagccgctgtaagctggccctggatgccgaacgtaggtacgatggcagatagcagttgttcgtctatgttataatatttcagtaatgatttggaaactgcattttcctcaaaatcccagaaggtaccttctgataagcccgagatggtggtgcaggcttcgccggttaatttcatggcaatgaaatcgccgggcaacattactttatgaatgcgttcataaatatgcggttcattttcctggatccagcgaagcttcgaggcggtaaaattaccgggtgagttcagcaggtgctccagacagtactgttcgccaagtgctttaaaggcagtattgccggtatttacagcgcggctgtcgcaccagataatggccgggcgcagcacctgctgttgtttatccacacacaccaatccgtgcatctggtaggcaatacctattcctttgatctgtgcaggatccactgtaaagcggttcagcagcagttccgtagcgtgaacaatttccttccaccagctctcggggtcttgttctgcccagtcggcgtgtggtacatcaatggccatctctttttcggggcaggtggcggtggccacgcaggcgccggtgtcagcgttaagcaatgctgctttgatagatgatgacccaatatcgtatcctataaagtacataacgtgagaaattaacaatctgaaaaaggaccggatattttacgacaggaaaatgtcctaaaatatccggataccaaaataataaaatgttcttattaccagaatacagtgtacaaggcgataaggataccaacaatcagtaaggcgcccaccgtaaagcccaggttgggtttaaacatgctggcatcgatagccagtcctttcggattgttcacactgcgtttatccgacaacgtgataatgatcatacctactacgcacactacaaacaccagtcccatacgatcgatgaaagccatttcgtataacccgctgtccgggttcagtgcggcaaagccaagctgatgcaaaggttccaggttcacccatgccggcataaacttcaggaagaaggaaaggagtaaaccaccaatcatcgcaaacatggctgcgctggaggttgtccgtttccagaaaaacccgagggcaaacatggcgaatacgcccggagaaacaaagccggtatattcctggataaactggaaaccaccttttttatctatgccaaggaagttggagatcacgattgcgatgatcatggtgataattaccacagcacggcccacgcctacgatcttcttttcatcggcatctttgttatatatcttcttataaatatccagggaataaatggtggaaatactgttggctttacctgccagggaagccaccaccgcagctgttaaagcagcaaacgcgagtccttttaaaccggaaggcaggagattgagcaataccgggtaagcgttatccgggttcagggaacctcctttcatcatggattgtgcaaagtcgccgtgattctgggcatacagtacataagccgcaataccaggtaatactacgatcaccggcatcaggagtttcaggaagcctgcaaacagtaatccctgacgggcagttttcagatccgcacccaatgcacgctgcgtaatatactgattacatccccagtaattcaggtttacgatccacatcccccctatcagcacgctcaggccgggcagatcgaggtacttgggattttctttatgaaggatcatatggaaatgatcgctggcatgttgcgtcatcagggagaagcctcttaatacgcctttttcgccgaagtgctcagacaccagctgtaatgccaggtaggtagtggctaatccgccgaggataaggaaaaacacctgtatcacatcggtgtagccgatcaccttcatccctcccagtgtaatgaggatggcgaagaaggccagcgccaccatacacacatagaagttaataccggagatcgtggacaccgcgagggcgccaaggtacaggatagaagtaaggtttaccaccacatacaataacagccagaaaacggccatgatggtacttaccgtttgattatacctgcgttccaggaactggggcatggtatagatcttatttttcaggtaaatcggcaggaaaaatactgccaccacgatgagcgtagcagccgccatccattcgtaagtggatatggccagccccatactgaatccgtttccggacatcccgataaactgctccgcagaaatattggaagcaatgagcgatgcgccgatagcccaccaggtaagggaaccttctgccaggaaaaagtctttggaatccgttgtggtcttcttctttttctgatagatatagtaaccataaccagccactattaaaaaatataccaggaataccaggtaatcaaagatgtgtaaggattttgtttgcataacgttcaaacgtggttataaaaaatttagcggatcaatatacataataaatgtaaaaaatacgcttacaattgttttttttgcgtgaaataaaaaaacgcgagggctgccgcggtttaccgggtgttaaaactatacatttaaattgctcatcatagtgcatttatgtaaaaagaaacaattgataccctttactttcacaaaaggtacctgtgaacggaataaaatatcttccaggttgatttcctttcctttatgggggtggggaattgtcaactgaatgcctggtagcgtggaaataaaaaataaatatagagcacagaaaaccgggaagcaagtttttccgctccgtcgggaaaaaacattttaatcaatgggcaggtcggggcaaatcccgcgggcgccttcaggactccagtgccattacagcgatgttatccccgattacagaaccgatggccactcccattcctcccatgcgtacgcccatgatcacattattcgtatgtgcttttacgataggttgttttgttttaccaaaagccatgatacccgtccacttgtcggctatggttacctctctgccgggcagtattacggtgcgcagcaatacttccagttcgtgctggatccggtcgttgaaccggaagtcggtggaagtttccccggcgaagtcgagctggcggccaccgccaagcagtacccttccttccagttccctgaaataataatatccttcttccatgtggaaaacgcctttaaagggcaggtcttttaccggtgtggtgatcagcacctgtcccctgccgggcactacttcttcctccgggagcagccggcgggtaaaggcattggtgcagatgagcaccttacgggctgaaaaggcaatatcttcttccagggtatgatgcggcacgataacgttcacacctgtatgaaaatcgtctattgttttcacggtgcaaccggttttaatttccactccttttaatacagctgtatcgatcagcgcccgcatcattttgccggtatgcagttcaccctcaaaattattgcggataagtgcttttacatatgctgaggcaaaaccgaaagcaggaagacggtcgtttgccagcgtgaatgcgggttctccgttgaagagctcacccaggatgtgatttacttccgggagctggtgcagggcccattcttcgcgggggccaatcagttcatggctgccattttcctggtagccgatggtggtatcgccgaggcggctgcgcagcaggcgtaagccttgcagccgcagccggaccaggtccctcaccgcatctgtgggcattgtttgcagatcggtcagtatttcggtgaggcttccgatgcaggcgaagccggcatttttggtactggcgccggtgggcaaaatgtcccgttccagcaccagtacccggcagccgggcgctctttctttcaggctgatggcagccgacagaccaacgataccgctgccgataatgatatagtcgtattgcaacaagctttccttctcccagaaacttaacatacttgatatttatacagtgcctacagatccgccgtctacccggaataccgcgcctgtgatgaaggaggcgtgatcagaagccaggaacgccactatgctgccggtttcttccggggtgccggggcggcccaacacctggtagggacggttttctttcaggaattctttggcagcttcggcgatagaaatatttttttcttttgagatgccttccagcatttcatctaccagtggtgttttgataaatgccggcgaaacggtgtttaccaggatattatcttttccgtaattctgcgacagcgtttttgaatagttattcaatgcggcctttgtagcattgtaatggcccatgttggggtccggctgttccgcattttcggaggagatgttgatgatcctgccgccaccctgctttttcatgtgaggaattaccagctgggtgagcgctaccaagccgaagaaattgacttcaaatacctgccgccactgcggcatgctgatggtgtccaacggaccgaatgcgtctataccgccggcgttatttacgaggatatcgatgtgaccgagctgctgcaccgtggtagtgaccaattgctgcaggtccgcttcttttgtcatatctgctaccaccgccagcacgtccagtccctgcaggcggaacatagcggctgtatcttccagttcatcggcattacgggcggtgatcactacagtagcgccttcctgcaacaaagacgccgcgatccctttgcctatacctttactgccaccggtaacgatggctacctttccttttaaattaagctccatgatcttatattttagaccaaaaataaaaaccgggtatctgtttattactgtataagttattgaaaaaacagtaaaagcagctgtttaaccccgcaggattccggatagtacaaattatgtagcttcgggggactaaaattatacaccatgattgcgacaaaagcttatgctgtgcaggatgctgcatcaccgttgggtccctggaattttgaacgcagagagccgggaccgcatgatgtgcagattgaaatcctttattgcggggtatgtcattccgatattcaccaggtgcggaatgagtggggcaattcaatttacccgatggttcccggccatgaaatagtggggcggatcaccaaagtgggtgatcatgtcaccaaattcaaggtgggcgatctggcggggataggttgctttgtggattcgtgccgggtgtgcgatccctgcaaatccggagaggaacaatattgcatcaccggtggcgccagtacctataatggttacgaaatggacagaaaaacgcatacctatggcggatattccacccatattgtaacagatgaaaaatatacgttgaaggtttctgataagctgccgcttgagggagtagcgccgctgttatgcgctggcatcaccacttattccccgcttcgccactggaaagtaggcaaaggtcataaagtagcggtagtgggtttgggcggtctgggccacatggcggtaaagcttgcggcgtctatgggggctgaggtaacgatgctgagcacctctccctccaaggaagcggatgcccgccggctgggcgcccatcatttcgcgctgatgacagataaagcgcaggtaaagcagctctacagtcaattcgattttatcatcaatactatttccgccccccacgattacacgacttacctgaacctcctgaacctggatggtgtgatgatttgcctgggagtgccaccggaaccgtccgtggtaccggccttcaacctgatcatgggacgcaggagcattgccggatcattgatcggcggcatccgcgaaacgcaggaaatgctggactactgtgcggagcataatattaccagtgatgtggaagtaattaatattaaggatatcaataccgcttatgagcggatgctgaagggtgatgtgaagtaccggtttgtaattgatattgccagtttgaaataagtgtagccggagtggccactttatttatacccgttccggtaaaccggaacgggtatttttttgttatgcagttgttaagcagaaattgtcctttgattttgttggtatattagtcactatccctaaatttcccgttatgtcgagtactacctcaaagaaccacaacaggtaccggcacctgcatttagctataattagcacggttgttatagccattgccggcgttttactgtacttttttgttaagcggcacacgcctgatttaccggatatcgccgccaacctgcaccaggcagtaatgccggaagaagataccagtgtaggaaaatgcgcgcagtatcccatcactgcattagagcttcaaaagctatatctggcgaatgatccggtagccgtggaaaagtatacaaatgaaacggtgtatataaacggtgtttacattggtactggtattaacccgatgggtactgcctacatgatccttaaaagtggcgacaggtcccattccattaagtgttttctacagaacaaagaagatattaatttaacgaaggggagccgcgttttactgaagggttattgccgggggcagatatgggatctcaaaattgaggagtgtgaattactggatcttccggttgtaacatcgcaaaaaaaatagcgcgcccttttacgggcgcgcctcatctctatacaagatatccgaacaggctgtcgtctttattgagttcggtgatctggaaattatatttctgacaattggcaatcagtttatcatagtcctcgcggtttcgcagttccacccctaccagcgcgggacctatctccttattatgtttctggatatattcaaaccgggtgatgtcatcatccgggccgagtatatcgttcacaaattgtttcagggctcccgggcgttgtgcaaaacgtacaataaaatagtgtttcaatccttcatacaggagtgaacgttcctttatttcctgcatgcggtcgatgtcgttgttactgccgctgatcacacatactacttttttccctttgatttccgcggcatggtcgtccagtgctgcgatggacaaggcgcccgcgggttctaccacaattgcatcttcgttatataaccggaggatggtggagcacacttttccttccggcacgaggtgcattttatccagcacatctttgcagatttcgtagttgagggtacctactcttttaacagcagcgccatctacaaagcgctctatttcatcgagggtaacgggaccgccgttttccagtgcgcggagcatagagggtgcgccttccggttccaccccgatgatacgggtattagggctatatgttttgaaataagtgccgaggcccgcagcaagaccgccgccgccaacgggtacaaaaagaaaatcgatagcggactggtcttccaggatttcaacggctacggttccttgtccttcaattattttcgggttgtcgaatggtgggataaaggtcatactattggcttttgtgaaagcctgggcttccacagagcaatcgtcgaaggtatcccctacgaggcggatttgtatatgatcgccgccaaacatatttacctggttaactttttgttttggtgtgatcaccggcataaacaccacgcctttaatattcatggctttacatgcataagcaaagccctgggcgtggttaccggcgctggcgcaggtaacgcctttggccaatagttcagcaggcaggctgctgatcaggttataggcgccgcgcagtttataagagcgtacaatctgcatatcctctcttttcagatatacgtcgcagttataacgccgggaaagattggcgctatacatcagcggagtgcgggtaacgattggtttcagtttcacagccgcgtccaggatattcagggaattgacactactcattacttcagacataaaatgtaattaatacaaatggcaaagcattttcgggattatcgaaatcatggaacctgtattcagtatcagaaagatgtattcttccgtactaaatacgagcgccaataatttcaataattcgaaaatgctttgccatttgtaatgtataatatttgctattacgcgttgttagggcgcagcttacgtacggccgcaccagcctgccacatttcgctttcacggagttctttcagttcttcgttcagtttctcacggtaatccggagtgctgttggaagcgatagaacgggcagcttctttacctgcagcaacgctggcatacagttcatcaaatacaggctgggtagcagttttgaacttcttccaccagtcgagcgcaccgcgctgagcagtagtagagcagttggcatacatccagtccataccattttctgctaccagtggcatcagtgactgtgtgagttcttctactgtttcattgaaagcttcagaaggtgagtgaccattcttacgcagtgtttcgtattgagcagcgaagataccctggatacaacccatgagagagccgcgttcgccggtaagatcggagaaaacttcttttttgaaatctgtttcaaacaggtaaccggaaccaacaccgatacccagtgctactacgcgttctttagcgcggccggtagcgtcctggaaaatggcgtagctggagttcagaccctgaccagccaggaacaggcggcgcagtgaagtaccggaaccttttggagctaccaggattacgtctacatcagcaggaggaatgataccggtttgttctttataggtgataccgaaaccgtgggagaagtacagtgctttaccaggagtcaggtgttgctttaaagtaggccacagggtgatctgtccggcatcagacagcaggaactgaagaatagtacctttctgagctgcttcttcgatatcgaataaagtttcaccaggaacccagccatcagcaactgctttgtcccaggttttggaatttttacgttgacctacaataacattaaagccattgtctttcaggttcagtgcctggccaggaccttgtacgccataaccaataactgcaatcacttcgttcttcagcacttcccttgctttttccatagggaattcttctctggttactacttgttcgagtacccctccaaaattgatggttgccatgtgttgtttttttagcttttagctactagctgttagctgttagctgaggtgtgatttgaatgaataatgattaagatgtcagctgccggcggctggccggcagccagttatttgctgaaagcacacggctaaatgccgggagcttcctgtgtgtgtaattctttcaggtgctcgtggaaacggcggctccattttacaatggctacccttccgctcttagtgtactctatcaagccatatggctccagtttcttgataaagtcggtcagctcctgctggtgacctgttttctcgatcacaaaataatccgcggtgatcgtcaggatacgcgcattgttttcacgtatcagtctttcaatatcacctgtatgtaacgaccgggtagaaattttgtacagcgccagctcctggtataccacttcatcttcttcatgcacaaaagcgcggtgaatttcaatcagtctttctatctgtccaactactttatccagcttctcacgtgtagacatcaccgttattacaaacttatacacaccgggaatttctgtttcagcggtggttaagctggtgatattgatacccctgcgggtaaatattatggtgatacggttggttatacctatacggtcttccgtatataccgttactgtatactctttttgcatatacctgttgtgaattacaaatgatcaatgtgaatcctccgggatgctgctactccagcctgatgctggaaacaggagcacctgcgggcaccatagggaatacgttatcttctttttccactaccacttccagcagataagcacccttgtgcgccagcatttcatcaatagcggcggatatatcttcccttgctgttacttttttgccggggatataaaatcctttagcaacctgtacaaagtcgggattgaccatttcagtggaggaatagcgcctgtcgaaaaacagctgctgccattgtcttaccattcccaggaagttgttattcaggatcactattttcacaccaatctgtgactggtgaatagtggccagttcctgtaaggtcatctggaaacaaccatcgccgataatagcaactacttctttttcgggcgtaccggttttagcgcccattgctgccggcagcgaaaagcccatcgtacccattccacctgaggtgacattggtattgggatttttgaagcggtaatagcgggaggctaccatctggtgctgaccgacatctgttaccagcactgcttcgcctttggttttttctgagatcaggcggattacttctgccattttcagctcaccttcctgtggatacagttcagcatgctgtactttatcatattcttttttatcagcggcgcggaattcttccagccaggcggcatgctcagcagggtttacctgtttgatcaatgctgccagggctggctttgcatctgcgtgaacggctacatcagctttgatgatcttattgatctctgctgcatcgatttcgatgtgtataactttggcgttgggaacataagtgcctacgtcgcccgttacacggtcatcgaagcgcattcccactgcgatcaccacatcggcttcgccggtgagcatgttaggaccatagttaccatgcattcccagcatacctacatacagcgggtgatctaccggtacggcagacaggcccagtaaagtagatccgataggaatggcggctttttccgctagcgcgatcagttctttttcggcacctgataacagtacgccatggccacagaggatgaatggcttctttgcaccgttgatcaacgctgctgctgctgttaccgcatcctggtttaattcaggaataggacggtaactgcggatatattcacatttcttgtactcgtattcaaattccccgaactgtgcgtttttggtgatatccaccagtacagggccgggacggccgctgcgggcaatgtaaaatgctttggccattgcgcccggaatatcttccggacgggtcacctgtatattccacttggtaataggcatggtaatgccgatcacatctgtttcctgaaatgcatcggttcctaacagggcggcagctacctggccggttacgcataccattggggtactgtccatataagcgtcggccaaacctgtaaccaggttggtggcgcccggaccggaagtagcaaaagctacacctaccttaccggaactgcgtgcataaccttgtgcagcatgagtggcaccctgttcgtgccggacgagtatgtgatggacctgatcctggaaatcgtaaagggcatcataaataggcatgatcgccccgccgggatatccgaaaatggtgtccaccccttcttcgatcagggagcggatcactgcttcggaacctgtaatcacaggctttgcagctaactgtttatctgctatctcaggcttcatcggtaacacatccttctgttgcattttttacaagttttgcgtacttaaataagattccattggtcactctcaatgcgggttgtatccacgctgcccggcgtgcggccagctcttcgtcactgatttccacattgataaagttcttcgttgcgtctatttcgatgatatcgttgtcttgtacaagtgcgatatttcccccttcaaaagcttccggggtgatatgcccaaccacaaatccgtgggtaccaccggagaagcggccatcggtaatgagggctacgcttttgcctaatcccacgcccatgatggcgctggtaggtttcagcatttccggcatacctggtgcgcctttcgggcctacctggcggatcaccaccacatctccttcttttactttaccggaggtgatacctgcgatcagttcaaattcgccgtcgaatacacgggcggggcctctgaagcgttcgccttccttaccagtgattttcgctacggagccttctgtagcgaggttaccgtagaggatctggatgtgggcggttggtttcagtggtttttccagcggcacaatgatatcctgtgtgctgaagtctatgtctgccacgtcttccaggttttcggcgattgtcttaccggtaacggtcaggcaatggccgtggatatacccttttttcaggaggtatttcattaccaaaggaacgccgccgatgttgtggaggtcttccatgaggtatttaccacttggtttcaggtcggcgatcagcggtgttttgtcgctgatgcgctgaaaatcttccagcctgatggaaatgcctactgacttcgcgatggcgataaagtgcagtacggcgttggtgctgccacccagggccatgatgatggtgagagcattttcaaatgcctctttggtcatgatgtccttaggtttaatatctctttcaaggagcaggcggatgtatttaccggcagcaatacattcatcttttttgtcctggctcaatgcggggttggatgagctgtacgggaggctcataccgagtgcttcgatagcggaagacatggtattagcggtgtacataccgccacaggcgcctgcgccggggcaggaattctgtacaatgcctttgaaatcgccttcatccagtttaccggccattttctgacctaatgcttcaaatgctgagatgatgttgagatcctggcctttatattttccgggtgcgatagtaccgccataaaccatgatagaagggcggttgaggcgacccatcgccatcagggagccgggcatgttcttatcgcagcctggtacggtgatcagggcgtcgtaatactgtgctcctgcaacggtttcaatggaatctgcaatcagatcacggctaacgagggaataacgcatccccggtgtaccattgctcataccatcactgacgccaatggtatggaaaatgagtccgaccagatcatttgcccagacgccttttttgacatctttagccagatcattcaggtgcatattgcaggtgttgccatcgtagcccatgctaacgatacccacctgtgcttttttcagatcttcttctgttaaaccaattccatacaattgtgcctgcgcagctggttgcgtagggtcttgcgtgatcgtcttgctgtatttatttaattccattgctttttgttattaccccgattacaggtgtttataggtaccctattttaaaaactctccacaaattacccggtggcgtcgtcaaattcaaaccaacttattccaatttaccggtcttcaaatctgccttttaagctttaaaaccctttactgtaaaggattataagtttttcgatttacaaccttcaaaggattttaactgtcagctgttagcatttagcgaatgctaacagctaacagccaacggttatgccagttgagcttcgcgttggaatgctttttccagcactttagctttgtaggcctgttggagtatttttccgagcgactgcgcccagggcttgctgaaagactgaccgtccagggagtcgataccgatgatttctgctgcagtaccgcagaagaaggctgcttcggcttcttttaattccgggatggtaaataatttttgttccagtgggatattcagttcctggcaaagttcgataacagtggcgcgggtgatgcctgggaggatgttaccggcgggaggagtgtatattttgccgtctttttcaaagaagatgttagcaccggggccttctgcaacgtaaccattcatatccagcagcagcgcttcatcgtaacctttttcttttgcttcctgcgaggccagtattgagtttacataaaggccggccgacttggattctattttaaaggctttgggatttggtcgttcgtaggaggaagtcattacgcgcaacagcttttctcccaggtaagctccccattcccatgcgcagatcaggatgtgcgactctgcggcggctttcagcgtcatattcggcggacagaacaccagcggcctgatataagcttcttccatgttattcatctccagtactttataacaagcggcgatcagctcttcgttatcaaatttgtaggggatgtggatcagttcgcaggagcgcttcaggcggtcgaagtgttcttttgctttaaagatcttcacttcgccgtttgcggttttgtaggcgcggatgccttcaaaaacagcataaccgtagtggagcgactggccatacaggtcagttgtagcagcatttgctttggtgtactcaccgttgatgtaaagaaaagtgttgtcgttgtaatagctatacataaaattgaaattataccaggaatatacagtccaaaaaaaagcctccctctttgcggaggaaggcgttatattttgtgattatatgcacgtttacctatcctccatactggtggctaataatgacaacgacgataatcacgaccttcgtgatagcccagttgagctgaggcacgatgtgattaagttttatattgtctttatttacccacatggaggtgcttattttctttagcgtttctacaaaagtattcgtgaaaaaaataaaaaacaacaatacaggcaatatttagtaaaaaattaatcacattaagggtttttgaaaatatttaaaaaaacaaggcaatagttgcttgttttctaaacaaatcataggatcgttataaattaatctactggttttgtgtacaaaagacgcggattttgtcttttccgctgattacgctgattatactgattacctggatttttactttttggatttataaaggattaagggagatagcagcggatgtatccgctttatctcccttaattattattttaaggaaatctaaaaaatctaaaaaaaatccaaaagtaaaaatccgggtaatcagtataatcagcgtaatcctgagccaagacaaaatccgctcaaaaaaaatcccggtgcttcctgcaccgggataaaatgatttcatttcatttactgttcacgttctaaaaaatgatttcatttactgttcacttgttacattgacgtgcaggcatttatcgatgatatcctgcagtactgtttctttttccatgagccgctgcagtaaaaccagttgattttttgcgcggtcgtaattgtgtgtcgggtacttgatgggataatatacgtcaccgttcagataatcggtgaggaagcgtatcccctgcatgtagatcataaacttcccggcaaagaacagttgttctttttctacttttgtcaaagtaccgccaatctctgcgaggtacccctgcataagggcttcgtagtattcttcgcggataacgatctggctgaaatccctttcttcttcagacacggggcaaacataagtgcgtaccatgtcgcctaggtctgagatgatttttccgggcatcagggtatccaggtcacatacacaaataccttcataagtatccttgttgagcaatacattattgattttggtatcgtgatgcatcagatggtccctgaattcaggatttgttttcagttgttcatacgttactgcgatgtcagaatagcggaggaaatcttcaatcatctcttctgctgcaactttccggtcttcctttgccgttcggatagcctcctggaaggcgctgtaccgaagggtcaggttgtgaaagtttggaatcgaagctttaaacggcttcaggtcaattcccgaaaggtaactggcaaggcggccaaattgtctggctgcttcatacgcctgctttgggttgtcggcctggtctaccgttacggaatccgcaataaaagggatcaatctccagtattcgttgtcaattacaaagagctcttccccattaaccgtggggatcggcgtaataaacagatagccgggatgatgaactgccagataatccgctgccattctctggttggcggcgatcactcctggttccttaaatacgtttacgttgatcttttgtaaaacgtatctactgccgtcctgctttttttctaacaaaaaagtgttgttgatgtgtcctgatccaaattttcggacatttaatccttcaggctcaagtccgaaagcctgaaggatcctgctgttgggttttatttccataaattgtctggatattctccattcttaaccagcgccgacaagctggcctgcactcccggtgcatcttctttgtaagtaacgccaaaccattttgcgctggttggaattacttttacctggccaataccacggcgggtaaattcgtcggctacaatcgtaataaagaattcagatttaggattgctgctgtttttctccagaaattcgctgaaaaggccctggctcaattcaaatacgctcgggtggaatccccagaagttcatggataccggcgtgttggcaggtaacggatgtttgctgccatctgcttcttcataaacgatctggtcgttttcagcatatatcttggtcctttcgttgatagccgccaggttgccgtctgcgcttacttcgcatacgccgcgggaaacagaaccgtgctcactgatagttttgcccagttcatagccaactacgctgtatacgttgggcttacagtcgttattcaggaaagcagccattttaacgaaagcatctgtaccataaaagtcatctgcattgatcactgcaaatggctcattgatagcatttttggcgcaaagaaccgcatgggcagtaccccatggcttggttctgtcggccggaaccgtatgatctcctaaaaatgcatccatttcctggtatacaaaatcaacagccacgcggcctttgagctttggttcaaagatttccctgaactcagccgcaaaattctcgcggatgatgaacactatttttccaaaaccggcgctgatagcgtcgtaaatagagtagtcaacgatagtttcaccgctggggccaaattgctggatttgctttaaactgccgtatcggctggccataccggccgccaaaatcaataaagtcggttgcatttttctgatattagttttataagtgtcaactatttacctaaaaatatcggcgctaaatttaatcattaaaactattttcacactttctttttgtagtaacgcccttttttaaagattaattaaactgaacaatgaagagattattagtgctgggagccgttgccatgcagcttcttactactgccaatgcgcaacagaaaacaaatccggatgacattaaagaaaaaatgcagtggttctccgatgccaaactgggcattttcattcactggggcatctattctgtcaaaggaatcgatgaatcctggtcattccacaacaaaaaaatatcctaccccgattatatgcagcagctgaaaggctttactgcaaacaattacaacccgcaggtatgggccgacctgatcaaagaatccggcgcccgctatgcagtgatgaccaccaaacaccacgatggcgtagcgctgtgggacagcaaatacagtaaactggatgttgccaacagtacaccggcgaaaagagacgtgctcacccctctctacgcggctttgcggcgcgatagtatcaaatgcggtgcctatttctccctgatcgactggagccacaacgattatccgcagttcctgaaagacagcaaccgctatgatatcaaagcccagcccgaaagatggcaacgcttcctgaaattttacgaaggacaaatggccgagataatgacgaagttcaacccggacctgtggtggttcgacggcgactgggaacactccgccgaagaatgggaagcccccaaaatgcgacagatgctcacctcccataaccctaacaccattatcaacggacgcctgcagggatacggcgactatgaaacgccggaacagaacttccccgtgtcacgcccgaaataccactggtgggagctatgcatgaccatcaacaacaactggggatggcagccacaggacaacaactggaaaacgccttttgaaattatcaccatcttcgtggatgccgtaagcaatggcggcaacctcctgctcgatatcggccccaaagccgatggcagcatcccggaagaagaagttcacatgctgaaagaactcggcgcctggaacaaacgcaatggcgaagcagtgttcaataccatcggtggtattccgcagggacacttctacggccccaccaccctctcaaaagattccagcaccctctacctgttcctgccggctaaaaccagtggccaggtaatggtgaaaggactttccaataaaattgaaagcatcaccgtactgggcaacaacagccagctgacccacaaagtagtcggcaaaatttcctggagtcctgtacccggactggttttcataaacgtaccggaaaatgtacaggataaatatatcactgtgctgaaagtgaagctggataaggccgtgaagctgtacagaggccagggtggtttcctgaccaacgattaataaacgattttaattttatatttggggagatgaatgctgcaatatgccttcatctccccgatctttttactgccttatcacttaatcgctacatgctttcttacgataacatcacccttgaatcctttcaaacttcctggctgccggagcatatccacgctgccatgctgcgtttggataaaattcacccggaagtatccgggaataagtggtttaagctgaaacacaacatcgaagcggctaagactaataacagcaacggcatccttacctatggcggcgcttactccaatcatattgcagccaccgccctggcctgtaaggaagcagccttgccctgtgcaggaattatccgtggagaagagcataagggccagttgaatcatatgcttcaaaccgcagcagacaatggcatgaagctggtttttattagccgggaagattatcgccatcacaaagcaggtaacaccttatatcccggctatcatgttgttccggagggcggtcacaatgccctgggcgcccggggctgtgaagagatcctttctatcttccccacaacaaattatacacatatcctttgtgccgcaggcacaggcaccacactcgcgggcctgatcaacagtgctgcaccgcatcagcaggtaattggcattcccgtattaaagggcgcgcagtaccttgaaaaagaaattactgacctgctgcatcccggtaataacaaccgctggcggctattatacgaacaccacggtggcggctatgccaaaaaatcgcctgcacttatagattttatcaatactgtctatcaagaaacaggtattcccacagattttatttacaccggcaaactggtaatggcctttcgtgatctggtccagcagggctgctttccggcgaacagcaatgtattgctggtacacaccggaggcctccagggcaatctttccctccctcccggcgttctatccttttaaaaactgttcattatatttgaacggtagtgtatttttgccaactttaagagctcacggaataatcagtatgaagcagattgtgcgtataacatttgttattggaatttttttattgaccggatttgcaggaaaggctcaggcacaggagtttgtgccacctgtgctgcctaattttaccgcttctattaaaaccggtaggatacaactggactggatctccggcttcacacaggtaaaggaaataggtattcagcgctcgctcgacagcgtactgaacttcaataccattggttacgccagctaccctactcaaacaaggaacgcctatcttgataataaaccgttaccgggcagtaactattaccgtctctttattttattcaccaacggacgtttcatgtacagcaaaacggtactggctctgtccgacagcactatccgcgccgatcagaaattgcagtatgccgacatcatggatgcttcaaggggcctgagaggcaaggaacaggaaaacagggagccggaaagagcatcctggcacccctccaactatatttacactactgccgatggcaatatcaacataaagctgccggatgcaccgcaaaagaagtactccattaagttttatgaatccaacggtactttccttttcgatatcgaccaggtaaaaggcccttccctcattttagagaaagctatttttatgcatgcaggatggttcaacttcgaaatatttgaggagggaaaattaaaggagaaatggaacctgttcattccgctcaactacaaaatgtaactataccatttcagcgttgaacacttcgccgaaatgtttactcagcttagctttcacttcttccaggcttaccggcttacccacttctttatcgagtgaggctacctgtttgtcggcaataccacatgcaatgatgttgttgaagtagtccatcagggtattcacattcagggcaaagccgtgcatggttacccaacggctgcaacgaacccccatagcgcatattttacgggctttcgctttatcgtgcggatccagccatacgccggtttccccggaagaacggtcgccggttacgccatattccgccagcgtgcggataatcacctcttcaaggcaacgcaggtatttaccaatatctgtaaagaaattttcgagatccaggataggataacccaccacctggccgggaccatgaaatgtaatatctccgccacggttggtaggcacaaagcctatcccctgctcctgcagctcctgttgggagatcaggaggttttccatatgaccgcttttaccaatggtatacacgggaggatgttcgcaaaacaacaggtagttggtagtggcctttggcaactgatcggctaccctggttttcaactgcacattttccttcagcaactgctcctggtagtcccaggcagcctggtagtctattacgccgaggtctcttactacaatcttctgctttactttatccatgatcatattggtctttttcagctgcgcaaaggtacgccaattcgctgtgatacggaacatttgcccacagggctgctaaactgccaactaagctttacctttgcaaaaaattatattaatggctgaagaattgctggaactggaagatgagctggaaaacggggatggcagtgaggaactatatgaaaagattaatatggtggtcgacaaaggtcaggaccctatccgtattgataaattccttactaaccgcatagaaggcgccacccgcaataagatccaacaggccctggatggtgaactggtgttggtgaacgacaaacccgttaaggccaattacaagatcaggccactggacaggatcgtcgtgttttccaaccggaacccggagaataccgacatcattccacaagagctaccgctgaatattgtatttgaagacgacgatattatgatcatcgacaaacccgccggcctggtagtacatcccggctgcggcaaccgcgatggtacactggtgaatggcctgtcgtggtacctgggcgataaaacccaggctaccgagccggaaatcccgcgcttcgggctggtacaccgcatcgataaaaataccagcggattgctggtcatcgccaaatccgacaaagcgatgaatgacctggccaaacaattcttcgatcacaccgtgcatcgccgctatattgcgctggtatggggcgactttgaagaagacgaaggcaccgtggtggcccacgtaggccgccatcaacgcttacgtaagattatggatgcatatccggatggcgaatatggcaaggaagccatcacccactaccgcgtactggaacggtttaattatgtaaccatggtggaatgccgtcttgaaaccggccgcacccaccagatccgtgtacacatgcagcatatcggccactcgctgtttaacgatgaaacctacggcggtaaccgcattgtgaaaggaaccgtatacacgaaatacaaacagtttgtggaaaactgcttcagtattatgccacgccacgccctgcacgcacaacagctgggcttcatacatccccgcacccgcgagcagatgtactttgaaagcaacctgccttccgactttacctccgtactggaaaagtggaaaagatatattgcagccagaccgctgaaagacgacgaagtataactcataactggttttagcggagaactgtctccgctaaaatcatcttctcctaaaattcatatttattattataaatattctacatgtttaggttatcttagcagcaattacccatgtcattacatgagagaccacatatctgttttctgtcgattcttattccttataccggttttgctggtatgctgcctgtttggcaacaaggccggcgcccagaacaccccctttgctgtatcctctacctgtgtaaacgatacttcttttttcctgatcatcaatcccgcgggcattgactctgtgaagtggttttttaacgatcccccttcgggagataaagactcttccaggagcatgcaggcgtatcatatttataacagcgttggcacttataccgataccctcatcgcctggcgcaatggccttccggataccaccattcaatctgttaccattgttacgcctgtgatcttcgatctcggcgatcaggacattaccctgtgtgaaggcggcaccatgacattgcaggcgcccatcattcccggcgctacttacctgtggcaggacagttccaccggcagcagcattcttgtagatacttccgctacctataaagtaaaaataaatggctgcccgagtcccgactccgtcaatattttctatacacccatcccggaaatagagcttggcaaagacctcgtgctatgcaccggcgaacatattgcgctggatgctaccgcgcaaaactgtacgtatctctggagtaccgggaatacagagcccacgcaggatgtttacacctcaggcacttatcacgtagacgtatatccgaaaggttgccctaccgtgtcggacgatatcaccattacgttcaccggcgccccttatcccttttcactgggtccggataccctgctgtgccccggagaatcgatccgcgtagctcctgccattcccgaggccacccggtgggaatggagtaccggcgccaccacgccggcggtgactattagcaataccactaacctgtgggcgctggtagaaattaacaacacctgcagtgtggtagataccatcttcattaattataaccgtttaaaaaaactggacctgggcaacgacaccagcatctgcaaagggaacttcctggtgcttaccgccgatttcggaaacgggcaatatctctggcaggacagctccgatcaggccacgtattatgtgaccaagcccggcttctattatgtgcatgcacaaataggccgctgcgaatcgatggatagtatctctgtaaaatttgaagacaccctgcgggtaaaccttggtccggatacactgctttgcagaaatgaagtgtaccagctgcgcgctaccggcgccggcgggggtacctataaatggcaggacagtaccagcacacccatgtataccgttacgcggccagggttttatgcgatggtggctaccaatagttgcgggcaatccgttgactcggtagaagtaaaataccacgattgcgaatgccagctgtattttcctactgccttttcccccaacggagatggaagaaatgattatttccggccggtataccggtgtcccatatacgattatacactcagcatctataaccgctggggagaacggatcttctttaccacagatccgcaggttggctggaacgggcgtgtaaacggtactttagcggatattgccacctatgtatggatagtggattataaagaagtgatcaccaggtttgctgtgcataaaaccggtaccattactttggtgaattagctatcactgcgcccctgtgaaattcaggaacctggctgcgaacacggctgtttcccttttcttgaagggtacgttccaggtgccgttataggtaaccagggcggggatcaggaggccattgtatttggtcatctgtacatccatcttcacattaaaatcaaacaacatcgttttgtaagaaagagcatatttacggccaacgatctcaaaattatctttgttaaaccaggtgatcagctcatctatcaccacatctgccctgtcgatgcggctcaggccgggctttgttttggcggtaaacacatagcaggaggtcccgtccacatagtttgcagcagtgatggaaaagtcataataccgcattacttcactgttgaagatggctactttgggccctacgatgggtacgccacggataggtttcccggggttaaagatcagctgtttcaactgcgccttgtgccgggcaaggctgccgctggagcgatcgggatcctcacctgattcatctgtacatacggtgcctttggtaaagaagaggttagcgtataattcagcggtataataattataatttcctttgcgggtatagaaatcgccggttactttttcgttagaaacctgcatggtgcggcacttccctttcatttcctggtgggtttgattataaagggaggcctgtacctgcgcatttttgccaagtacctggatatcgttgatggcgtcaaaacctacgatatgcaggtttttgaatgcgcggtaaaaggtggtgtcatcttccacccttttaataaagctgttaacgtcgaagcctatacgctttgcggctacaataacttcatccaggttaaccgtcattcctttatagcgggctgtgtcctgagcgttgagttgtaaacattgtaacaggctgagggcaatggttccggctatatttttccaaaaatgtgacatagctgcaatttagtaaaaaagagcaaagtgggtgccaggcaaatactaaaaacagaaagccgttgtaagtagcacttacaacagctttctgtttttctttaaaaggagatagagaagaactatctctttttatcaaccggggatttttccggccacatacatttgttccatagtaggctgcagcgcaccaccttttttctccagggtaacagcaaacatttgtgctttgccggttactttcattttctggaggaggctggctgtatcacccatttcgaacacgcccatatcaaccggtttgccatctacgatagcccagagttgatactgtttgtcggcagttggttctggcagtttgttaactttcagatacacttcctgactttgcgggttccagaatacagtagctaatgcttcagggaacgctttggtacctggcatcggcactttcagaactttaggatcctggataatttccatagattcctgcatttgttctaagcgggttttgtaaagattgctctttgacaaaatggagttctgggatacgagcaaagattggtatttatctttgtactccttgaattccttgtaccggttaaagaacacataatttaaaacaagacttcccaccagcagcacggcggcggcggtggcaagccatttccaggataggcttttagtttcttgcatggacactacttttggttgttgcaggtcttgatcgggtacaggttcaccctcctgcaaattgggttcattattgatttgtgtgaataaacgtgttttaatatccgtctccggatttttgccctgcaacctgatatattcttccatactgcggcgataggcttccacctcttcggccacagccgggtattgggccatagcggcttccagctcccgaatttcttcatcgctggccatacctgctatgtatagctcaataattccggacgatatgaaatgttgtgggtccactattgcaaaaaatatttacttgtttaaaatggttcttaattgattaatggcattgcgcatcctcgttttcacggtacccaaaggaatgtccatcacccgggcaatttcttcctgggtacaacctttataatatgctaaatctatcagggtacgctgttctttggtaagcttttccaggatccgggaaaacccaaggtagtcggtagatggctgcacagcaatgaggctgtcgactacatgtacgtcatccggcatattccggattttctgctccatcttatgggatttggaccggagaatatctatcgcggtgttccgcgcaatattcagcatccaggtaaaaagcctgccttttgtttcatcgtagcggtcgagatgacgccagatcttcatgaatacgtcctgcaatacatccccggcggagctatcgtcgttcagcacctttacaatcaccccgtataatgccggcgaatactggtcatacaggtaactgaatattttctggtcacgggcttttaaaccctgcaccagctcagcttctgtatatatagcagcgtattgcaaaacagattggatatagttttagatagttagttacggatagatttcacaacacgacagaacggaacatgatcatcatgccttcagctttcacggatattttttttataacagttgtgcttctttgaaatggttaatcggggtgccggtaaaggcaagatactcatttatcatgataaacaaacccggcgttattttgccagttttgccgacatgcatacctggtccatactgggatcctggctgccgcctttcttttcaagcgtaatggcaaagccttgtgcagcagccaccgctttcatctgttgtaacagttgtgatgcatcggccccggtgaggaatacacctgcatccaccagtttcttattcacaatggcccacagctggaattgcttaccggccggaggtataggcattaattgtgcctgcaggtatacggcctgtgtttttgcattccatcctacggctaccaggttgcctgcatacttgccgccaccggggatctttgtccatttaaaatcggggttattcagcggatctgcttctgctaccacgttggcgggcgtttccttcaaactggtcagtgcctgttgttccttatctgcttccagcttttctttggtggctatgagcgactggtagcggcttttatagtcggtggatttacggaagaaaaagaagttcatgaaaacactgcccagcaacaaagctacaatggcggctgtgagatacttccatagcttgtcatttgattttttttccaccggcagctgttttaccggtgtttcccgggagggttgctgcacttgttttttatttttcccgttcaggggagcggagatgggcgcacgcagttcatccggcagcaggttgtttccttcctgcgtgttttcctgacggatcatttccatcagccgttccttaatgccgtagggaggggctatcgcgtacagctgcacaaaacgctccttgtcatgctgcaatgaatccactgcagctttaacgtcggggtattgagatacggccgtttctacctcaccttgttctgtttccggtaacataccgaatacatagctttcaaggattccggatgatatgtatcgttgtacatccactatttcttataattacaattgttttaacagtgttctcaattgtataatagcattacgcatgcgggttttcaccgtgcccaatggtatttcaagggacttggctatctcttcctgggtatgtcccttgaagtaagccatgtcaataataatacgttgatctttttgaagcttttcaatcactttggttaaaccaagatggtccacagataaatgcaccgccagttgtggttcatacatcagtgccacgctgtttacatcctgtacgcgctgttccagtttgtgattttttgagcggagactatcaattgctgtgttgcgggtgatattcaacatccaggtgaataacctgccttttgaggcatcataacggtcaatattccgccagatctttacaaatacttcctgcagcacatctccggcggctgtttcttctcccactactttcagggctacaccatataaagcgggtgaatagtgatcatacaaataagtgaatatcttttcatccctggctataaggccctgaatcaattcaacttcagtgtatgttaaggtagctcccaagtttgaggatatggatgttatactttatgataccaaaataacaggttttctttacattacaaaattatttcctatttagggaaagtcatcctgtaatctactcttattttacctttggtaatatcttccagcttacttttcaacattctgcgctttaatggcttcaggtgatcgatgaataaaaccccgtcgatgtggtcatattcatggaggattacccgggcagtcacgccggtgaatgttcttacatgcggggtaaaattctcatccacatagctcagggtaacggtttccgcacggtttacatcttcacgcacctttggaatgctcaaacatccttcattatatgcccactcttttccgccggtttccacgatatgtgcattgataaatacaccttttaccccttcatctccgggataatcgttcttttcgtcttcttccaggttatgaataatctgctcactatctaccacaaacagccggatcgccttatttacctgtggagcagcaatgcccacaccgttagaaccatacatggtttcccacatattggcaatcaattccttcaggtttggatattcaggagtgatgtcttctgctacttttctcaataccgggtgcccgtaagctacaattggcaaaatcatgttcaaatacttggtttaatccgcaaagatagacaatttcggagttcagcggaggttgtctttctcaggattacgctgattttggtgattttttatatgttattatattttattacggagatattcctgtaatataatagtggcacttatttcgtctaccagggctttattccggcggtccattttcttcagaccgctgtcgatcatcgtctggaaggccattttagaggtaaaacgctcatctacctttacaacagggatatcggggaaattctttttaatgatgcggatacactctaccaccagtgcagtggcatcggtagcgttaccatccagtcctttgggttctcctattacaatcgtttccacctgttcggcggcgaagtactttttcagaaagggaataaggtcgtgcgtggcaacggtggtaagcccggtggcaatcatctgtaaagggtctgttacggccagtcccgttctcttttttccgtaatctattgccatcaggcgggccatatactagcttttaacagggttagggctaatgaaaaacgagcatatctgtgatcgcaaaaacagcgaacaccacgctcgcaatcccgttggtagtcataaacatgatattgatcctgctgagatcattgggttttaccagtaaatgctgggaaacgagcatcaccacaaaaacagccgctcctatccagtagatccagtgaaaatgcccggttaagccgatagtcactaccagcgcggccgctatcacatgaagtaattcagaaaaccgcagggcgccggaaagtcccagccaggccggaatggaattcagctgctgtgatttatcaaaatcctcgtcctgcagggagtaaataatatcaaatccggatacccagcataataccaggaaagataccagtaccggtaacagtgcaaaactaccggttactgccaggtaagcgcctataggcgccagcgacaatcccacgcccagcaccaggtggcaaaacgcggtaaaacgcttggtatagctatatcccagcaccaccagcaaagctaccggcgacaggtaaaagcataccgggttgataaaccaggtagcgataataaacaataccacattggctataataaagaacagggcatttttgggagatatgataccggccgggatttccctttttgccgtacgtggattgagcttgtcgatatccacatccagccaccggttgaatgccattgcagcgctgcgcgcaaacaccatgcacagcactaccagtaaaaaagtaacccagttgaagccgccgcctcctttggtggtagccataaaaaagccggtgagggcaaaaggcatggcaaagatggtatgactgaactttaccagcgataaatacttgttgaccgtagaaatcatataattaatcctttaagccttcttcaattttacaaagatatcccaaaccacaataccagtgctcacggaaatattcagggaatgcttcatgcccagctggggaatttcgatacaaccatctaccagcttcattacttccccgtccaccccactcacttcattcccaaaaaccagtgccagcggctgatctgccggaggcgtaaaactattcagcatataactgttcaccgcctgctcaatggccatcacccggtacccggctgctttcagttcctgtaccgcgctcacggtggtgtcaaaatactgccactccaccgtttcggtagcgcccaaagccgttttattgatatcgcggtgcggtggcaccggcgtatagccacaaagaatgatcccctgtaccaggaatgcatccgcggtacggaacactgatcccacgttgtgcatgctgcgtatattatccaataccagtacaataggcgttttatcggcagccttgaactcttccaccgttttacggcccagttcatccatgcttaattttctcatcacctgcaaagataataggatgggatgagttttatatatttgcgccatggcaaaaagtaaaacggaagaaacaccgctcatgcagcaacataaggccatcaaggacagataccctgatgccgtactgttgttccgtgttggcgatttttatgaaacgtttaatgaggatgcagttatagccgcccgcgtactgggcattgtgttaaccaaaagggccaatgggtccgcctcttatgttgacctggcaggatttccccaccactcgttagatacttatctccataagctggtaaaagccggtcaccgggtggccgtgtgcgaccagctggaagatcccaaaacagtaaaaggcattgttaaacgtggcgtcaccgaaatggtcacacctggcgtagccatcaacgataagctgctcgaaaacgccagcaacaacttcctggcggcggttcattttggtgcagacaccaccggtgtgtctttcctcgatatttccaccggcgagttttttattgcagaaggcagcacggaatatgtggataagctcctccagagcttccgtccggcggaagtactgttcgccaaacaacaacagaaaaatttcaaagccactttcggcacccgtttctacacctatacgatggatgagtggatatttaccaccacctatgcggaagaaatactgctgaaacatttccagacccattccctgaaaggatacggcgtggaaggcctgcccgctgctattattgctgccggcgccacccttcactacctgaaagataccgagcatcccaacctccagcatattacacgcatgcagcgcatcagccaggacgattttctctggatggaccgcttcaccgtgcgcaacctggagctgctcaacagcagcgtggaaaacggccataccctcctgaaagtactggacaataccgttacccccatgggggcacgcctgctcaaacgctggatggtattccctctccgcgatatcaaagccatcaacgaacggctggataccgtggaatactttatcaaagaaaccgatctctccaaatccctggtacaccacctgaaacaaaccggcgacctggaaagactggtatccaagataccgctgaagaaaataaatccgcgggaagtactacagctggcccgctccctgcaacaggtacaggccgtgcaggcactcctggaaaacagcagcagcgactacctccgccggctaaacgaaaaactggatccctgcgtccccttactggaccgcattcttaatgaaattatggaaaacccgccggtactggtcaacaaaggcggctgcatcaaagaaggcgtaaacgcagagctggatgacctccgcaatatcgcgaacaaagggaaggactacctgctgcaaattcaacagaaagaatccgaagctaccggcatcccttccctgaaaatagctttcaataatgtattcggctattacctggaagtaaccaacacccataaaaacaaagtgcccgaccgctggatgcgcaagcaaacactggccaacgccgaacgctatattacgcccgaactgaaagagtatgaagaaaagattgtaggggcggaagataagatccaggtgctggaaagcagattgttcgacgacctggtacaaagcctgcaggcgtttattaagccggtacaggaagatgcgcaggtgtttgcgcggatcgactgcctcctgtgttttgcacataatgccatgcagtacaagtaccgtcgcccgaatatcacggaaggatttgacctggtcatcaaagaaggccgtcacccggtgatcgaaagaggactccctgccggtgaaagctatgtttccaacgatctgcagctggacaaagcatcccagcagatcattattcttaccggacccaacatgtccggtaaatcggccctgctgcggcaaacagcgctcatcaccctgatgtcgcacatgggcagctttgtacctgccaccagtgctgatattggtcttaccgataaaatatttacccgtgtaggcgcttccgataacctgagcggcggtgaatctaccttcatggtggaaatgaacgaaaccgccagcatcatcaacagcattaccccgcgcagccttgtgatactggatgaaatagggcgcggtaccagcacgtacgacgggatctccattgcctggagcatcgtggaatacctccacgatatgacggcgcactgccctaaaacgctgtttgccacgcactatcatgagttgaatgaactggaaaacaaacatgcgcgggtaaagaacttccatatcactaatatggaatcggggaacaaaattattttcctgcgtaaactggcgccgggcggaagtcgccacagctttggtattcacgtggcgcgcatggcgggcatgccgcctgagctgatcaacagggccaatgaagtgctggcaaatctcgaagaaaaacatattgatgcgccattgcagaaaaacataaaacagatcagcacaccctctcagaaactacagctgaatatatttgacgcccacagtgatgtgttccagcagatccgtgagaaactggatactgtggatattaaccggttaacaccggtggaagcattgctgaagctgagcgagattaagaatatgatcgggtaggtttctgatcgtctttataataaaaaacgtcccggaatatccgggacgtttttttattataatcattgttcactggtccttaacgaacgtcccagaaaattttgatgttggctttgtcctttgacgctacctgagcatagttatcaggattgtaaatctgctctgtagatggatacagcaaacgctgtggtggcgtcgtggaaccggaagatgtaccggtagcaaaaggtaatacaggataacctgtacgtcttacttctgtccatgactcgcctgcctgcaggatgaagaagttcacccatttttgtgtccagatctttgccagtttttgctgggaagtaccggtgtaggcaatggctggcctggcaatgaaactgctgataacagtgccggacggtgtaggcagtataggccacacaccagagctgaatacagcagattggttaatactgtaataaaaatttactgattgagcaataccgttttcataatctgtttgcggtgtaccaatgctccatctttcacctgcttctgctttcaggaagcttacttcagatgccgtaaatattacgccaggcacattgtagttattaaagaaagtagcggtatcgtaggtagcataccctaagttttcataatcagtagcagtaccatttgccgggaaaccatgcataccgtgctttgcacccgcatcccaataaacatctgtacgtggatcaccattgatcgccatcacagtatccagcagaaaagcaggtgcaaacggactacccgtcagagcgctttgcaggtcgctttttaaagtaggcgaactcattttgatcaatacgttctgagaattgtcactcaccagcggatatttggacgggttggtcagcatagctgttaccgctgttttggcattagcttctttcacataagaagtatgcatcaacaggcgcaggcgcagggagttagcataacgcctccaggcggtaagatcaccattcagcacgaaatcagctctctgaaaagcggctaacgtttcaacagagatagaagccgtttcaaaataactgttcaggttgtccagtccggcaatcagtgtatcatacacagcagctgcattatcaaaaggtgcaggtatcaccacacggtccgtgttgagagaaccagccttgctgaaaggaatatctccccagagatctatcatttgtgcagcctgatcgtacaacaccactttggcacagttcaggaaaatcagttgatctgcctgctgggccggcgtcaggttactataagtagtttccatttcccggtagttagccatgatacccggaccaacatagttcaggtcattatcgtcgcttttgctacctgcgtaaaaatcgatccaacggttctctgtataagccggagtaggaatatacatttttatggatggcgacagtgccgttgtttgcgaaaatgctgcagtggtaggcagtataaaggtcgcgtaatcccagtaagacgggcgcatacgcttgttcatgtacataccgctgagcagtttgctcattgagccggtagtagttaactccgggttcgggtaggcgtctgcaatttgtttcttgcaagagctgaaagtagctaccagcaagatgagcagtgaagtatttattaaaaggcgtttcattttaatctgttaagttcgtttacaaatcagtattctgctagaaacgggcacgcaggctggctcccaaacttcttgttggaccaacggtaccaccatcaattccctggctaaaccattgagaacctactgctacttccggatctaaaccttttggtaaagtcttccatacatagaagaggtttctgccaaccaatgagaactgcaaaccctggaagtgtaatttttcaacaatgcttttaggcatgttataagtaagggttacttcacgaagcttaatataactgtttttcattacagcattctcatacaggccattggtttgccaatcatactgattcatgtaatattgcgcagcagtaattaccttttcattcttcttaccatcagcagttacacctggtaaaatcacaccatcgtgatgtgcaccattcgggttagccaccaggttaccactggcatagtcaattgcatcgtaagcaataccaccatgagcagcatccctgtattgcagggtactgttaaacatacctgcaccgatctgatagtagtaaggaatagatacgagatcgccacctaaacggtaatccagcgtaaaatccagcgtaaagtttttatagcggagcgagttggagaaaccacccactactttaggcatgatgttaccggctaattcccatgcgttggtattagcggtataaataccatctgcatttaccaggtagttaccgttcgcgtctttatcacgtgggtgtacataaatgttacccaatggatcacctacgttggattgcagcaacaggtaaccaccgtcataactctgcatggttaaggttgtcataccatctctcagcgcggtcagcttgttcttgttgatggcaaaattaaagcgggtagtccagctgaaatttttggtagtgatgggagaagcattgatagctgcttcaaaaccggagttgctgaggtcccctgcattcatgatctgagaggtagcaccaccggatgctggtgtactcatagtcaggatttgatccatgactttgttattatagtaactgaagtctacaccaatcttatttttcaggaaccttgcctcgaagccaacctcagtttcccttttcttttcggatctcaactcttcattaccaaaggcgctgggattggtttgctgatagggaatgttatttttactgagggtaaccgtgtaaggattgtaggcaacattagcctggtacatgtttggatgattacccaccagaccgtaagaagccctgaatttcgcataatccatgaaagaaggcaactttactacttctgacaacaggaaaccagcattcacggaaggatagaagtacttgttattttttaccggcaaagtggaggtagactcataacgaccggttccttccaggaacaaaaatcctttataagccaggttcaccataccaaagccggctacatcaatctgttctgcgcgaactcctgttgcatacaacggatcagcagagttggccaaactgaaccagttttcatccatcaaaccacctttcgtctgggtaaactgattcttatatttctgtttgcggcccgtaacaccaccggtgaaagacatatcaaagtccttcgctactttagggttatagatcaacatcgcatctccataaaaggagttattattacgggtattcagcgcatactgaccggtatagccataaacagccggtttggtgttgtattgctgatcggaagttgtaacattggtgaagtcaccacctacacggcctctgaaacgcagactattcagaaggcttacattcagcgtagcgctgttgataaagcgattctgtgtttcatcatacctgttacgcaggttattccacagatagtccatcaggttggtagccctgaagcggtatgccattttctcatcctgatcgtactggttattgtccgcagctacatatttgtaaccgttactggtctgatatttattgaagaacgtactcatgtcatcgaagcggctgaagaagccatcgaatgacccaaatatgttactcatcacattcgcgcggttgtgaacaaaggtgttgttataagtagatatcagatctacgctgaccttgtcacttaattttaatgtaccgttgaagttaaagttgtttttatagagattacttcctggcataatactcttataatctacacgattgtaagaaaaccggaaactacctttatcgcttgcgttggaaatagccacgttggctgcagagttataaccattctggaagaagtccttgtagttatctttctgcgctacatacttgcgggtagtgccatcccagtatttcacgtcgcggccgtcgaattttggtccaaattgatcgtacgctctgtaataaggatgcatagcaccatcagcgtctgtaatccagccatctggtgtagcacctacggagatgttggttgcggggtcataaccgggaccatattcattctggtaatccggtgtagctgcgagtttctcctggttgtaaacataattaacgtctacattcaggccgcggcctttcgctcctttcttggtggtaattaccaccaccccgttagtggcttcagaaccgtacaaagcagatgcactggcgcctttgaggatcgtcagtgtttcaatgtcttccgggttgatatccagtgcaccattcccctcaatccttgagttgctggtaccaaaagtgttggtggtaggatcattaaagtttctcagcggtacaccatccactacgtacagcggttgtgtgctcaggcttacagaagaaactcctcttacctgtacggaaacaccactggcagcgccaccgggagcagacacgattttcacaccggctgctttaccatacaaggcagaagcaaagttggtacttccgctttcggtaatttctttggaacttacggtgctaacagagtaacccagtgccttggcttctctcttaatacccatagcggtaaccactacttcattcagattcttgttgtcttcttttaatacaatgtttacggcagactgtccatgaacagctacttcctggttgataaatccaatgtaggaaaaaacgagtgtagcgccgtctgctacctggattttaaaatttccatcggggccggttgtagctccgttggaggcgtttttctcttttacggtaacacccggtaaaggtgttccttttgcgtccttaacggttcccgcaacagctttcttatcctgcgcccacgcagtgatacagcagcataagaaaagcaacgtggtgagaagaagtgatcttcgcatagctttcttttggtttagtgaattataacaagtgaatcagacacataagcaaaaaagacacgaaagtcccgctaccattaacttgcctgcattgcacaggagtcctgatggtaatcacgtggtttccgttcttaaataatcaaatggaattactccattggcattaattgttattctgacatcataccagtagtaaaacgttttagcaataccacataaaaaaaacctgtacccaccttcacatttctttttcactacaagtttggctgatccctctgaataatggtttcaaacttagggataattatgagaagtgcaaagaagatttaacaatttttttatttatcgttaacagctcgttaagaaagagaaaataatattccatgtgatcaaaatagcattaggaggtgatcgccttcggcgatgcggaaattgtcttagctcaggattacactgattatactgattagctggatttttactttttggattttttaaagactaagggagataagaacggagatacttaatttatccgtttgcaatctcagtcataagcgaccccgattggggagataatccatagataagccgtatctaagctgtatctatataggtacggcttatctatggcttaccctcgttttatctcccgatataatatgaatatacggagtcacaccttctgattacagttggttacataacgattaagggagataacagcagtatctccgctcttatctcccttaatctttaaaaaatccaaaaagtaaaaatccagctaatcagtataatcagcgtaatcctgagccaagacaatttccgcatcgccgaaggcgatcacctccgcgaagacgcgcggataatcaattccggctccagcactacctgttgttgtggagaagcaggtgcccctgccggatgatttaattctttcatcaacacttccacaatacttttcccgatggcagcaataggttgtgaaacacaggtaatggaaggactatgcaaacgaaacaggtcgtggtcatcaaagcccaccagtccgatctcttttcctatttcccatcccattgagcggatggtttcaatacccgcaatgcccaggtagttggtggcaaaaaatacggcgtctacgccctttgcagcagtgaggaatttctttatttcattattgaaactttcgcggtccaggtcgaatggcaggcgtttcacgaacgatttattaaaaggaattttatggtctttgagtgccgccgtgaagccatccagcctgtctttcatctgcgtttgatcagatgcgatggtaacaatcgcaattttcttatagccttgctccaccaggtgcgcagtagcatcataggcgcccttatagttgttgagcaccacatagtgacagttcacatgcgggaaatagcgatccaccagcaccagcggcttcgcagccgattgaagcagttctatttctttgtcgaggtttttggtgggcgtaataatataaccatctacctgccggtacttcagcacttccagtagtccctttgccttttccgtattatcttccgtactgccgtaaagtactttataaccgtgcttgtcggcctcgtcttccactactttagccagcgtggcgaagaagttgttcgcaatgtcctccacaataagaccaatcgttttggttttgccggttcgcagtccgcgggcaagctggttgggtttatattttagccgggttgcaattttctggattttcttacttacctgttcactgattcttttctcctttgctttaccgttgagtacaaaagataccgttgtgggagatactccggcctgttttgcaatatctttaatagagatccctttcatagaaaaaatgctacatcgatttagccggacgtaatttacaaaatgaagttggaaattacattgttgtactaattattccaagtacccccgccaaaactattgccctaccccggttgattttctatcacataaaaaggttattttcgggaaaatgatatttttttaaccaatttttaataatttggcatcattcataggacgatatcaatactactcacctgcctgcatagggttcccctgagccaggataatggcgatggtaataaagtataggacggtcacagtaatatagtagcttaaattaatacatgaatgaaacccatccttattaaagttggggcttttgccgataatcagatcacgatcatagaaagaagtgatccttatttcaatacaccattccacttccacccggagtgcgagctggtatatgttacggaaagccatgggaagagaattgtaggggatagcatcgaaagctttgaagaaggcgatatggtgtttctcggtccgcatattccgcatgtatggtataatgaagaagaatactataagggagatgaaaatctgaaagcccgctctgtggttatctattttcccaaagacatattcggggagaaattttacggattgccggaaaccaaagcactcagtgaactatttcaccgggcacaaagagggatgaaaatcaccggcgccacccatgaactgctgaaacccgaaatcctggcgcttccgcggaaggagggactggaccgcatcatttcccttctccatatcttaaaaacactttcggaaacccgcgactgctactacctggccagcaccggttactctcacgcctacaacgtaaaggataatcataagatcgatgaagtgttcaagtacgtcatgaataacttctccaaggaaatatccctgcaggatgtggccagcatcaccaacctctcaccccaatccttctgccgcttctttaaaaaccgtacaaaaaaatcctttgtacagttcctcaatgaagtacgtatcggtcacgcctgtaaacggttaaccgaggaagactggtccatcgcggaaatcgcctactcctgcggctttaaaaacctttccaatttcaatcgcttcttcaaggaaattgtaggcaaaactcccaaggaatataaaaatgaactgcgcctgaaggaagcatgataaaaaatgtaattattttatcatttggttctttagttattttaaaaagtaagcgccaaatgtcagaatatcaaaattttcttcttacattcatttcagtaattatcaaccaaaacgcttaattactactgtaattcgatgtacagcagttattccgacaaccagctaatttcgctgctgaaaagcgacgacagcgctgccttcaatgccatctacgaccgctacagtaaaatgctgtatttattcatacacagcaaactggatgcctcagagatcagcaaagatgtgctgcaggaactctttatttccctatgggagaagagacattcactgatcctcaaagaatcattgaaagcttacctgtaccaggtagcccgtcacaaaatcatcgatatttaccggaaaaacgccacttaccgcaaatacctgcagcaactcatcgaacatttcgatgcccagccgcattccatcacggaaacagtagacaataaagcacggacacaggaactgtttgaggcgatcaaccacctgcccgaccgcatgaaagaaattttcatgctcagccggtttgaaaacctcaccgtagaacagatctccactcatcttggcctttcccaacagacggtaaaaaaccagattaccaaagcattgaagatactaaggaccagttatgccaggaccgacctgatcgtactcctgatatatatttatttgtttatttagcccgcaggcccatagccaggtaaaaaataattaaatgtacatggtaccttttccacgttattacgacttatcaacacataaaacggcaacaggtggacacagaacagattaaaatattgctggagcgatataaccaggggaattgctcaccggaggaagctgctattgtagatcagtggtttgaaaatattaaccggcataagtccacttacatagcagataaagaactggaccacgagctcgacagcatccgtttacaactcaatgaacatatcacacccacgccaaaggtgcggcatatccatacccgttactggtacgccgcaactgcggctatcatattactggcagcggggcttttctggtttaaccaacaaacgccccgtaccgggccaggtgccggcaacttccagcctccggttattgcgcggcaatccaaccggatcatcaggaacggatttgtggaaatcaccacgcccaaaggcaataaagaaagtattaccctcgaagacggcagctccctggaactgaacgccggtagtaaagtacgctaccccgaacatttcgacagcaacagccgcaccattttcctggaagaaggagaagccttttttaatgtagccgccgacccggccaggaaatttgtggtgaataccggcgaactggccaccaccgcactcggtaccgcctttaatatacgcgcatatgccagcgaacataaagtaaccgtagcacttgtgagcggcaaggtaaaagtagaccaactgaataaaaacagccaatccgcttcatcactcattttgctgccaagtgaacagatcagctacgaccctatttcacttagcctcgtaaaatctgttttcaataaacccgaagacatcaccggctggaaacagggataccttgtattcaaagatgctccctataatgaaatagtaacaggtatagaaaatcgttatgacgttaccgttatcaacgaaagcgacaaaaaagaatggaactacaacggctctttcaaaaacgaaagcctgaaagacgtcatggatattatttgcctggccaaatccctttcttataccattaaaaacgataccgttcacctgcaaaacaaaaactagtccatatgagggtaaagccatgccccatgatgtggtttgtatccatggggttgatgctgacactactgttggcggggagcttgaacacaacgactagtgccatcacgcaaacacccgacccgcccacaggtatagttgtcaccatacaggtaaaaaacaaaaacctggaagaagtaatggccgaaatttcggtaaaaacaggactaaactttcattacgacaaagctgatcttaacctgaagaaaaagattacgttaaactgtacgaaaacacccattgatgaagtacttgcgttattatcagttcaggccggattaaagtttacccttatcaacaacaaaatcattgtaggcgcagaaagtgaagccaaaccctcacccactgcagacctgctgaatcatgtatccctggagagagagatcagtggaacagtacgcgataacaaaggcacgccgctcccgggagtcaccattcagatcaaatattccaataaaggaacccaatctaacgccgatgctggtttttcactaaaagccagcaccggcgacgtgctggtgtttagttccgttggctttatcacccgggaagttaccctgagcgccgacccacacctcgatgtacgcctgcaggaaaatgtaaaggcactcaatgagctggtggttaccgcactaggcatccagaaaaaaagcagggaactgccctactctacccaacagctggatggagatgacctgcaactggtgaaagatgcgaacgttatcaacagcctgaacggaaaaacagccggcgccaccatcacccgcagcgcctccggtgttggcggctccgtgagagtagtactgcgcggcaacaaatccacccgcgaaaaccagcccctttatatcgtggatggcgtaccttatgccaactacacacccgcgcaaccttcagatgtatggggccagtcgcacaacatcatcggcgccggcggccgcgatggcggcgatggcatctccaacatcaaccccgacgatattgaaagcatcagcatcctgaagggcgcttctgctgccgccctctatggcagccaggctgccaacggcgtgatcctcatcaccaccaaaaaaggaaaacccggcagaagcaaaatcgaggtttcttccgattatacccgggaaatgcccgcaatcctgcccccgctgcaatatcgctacgcacaaaccgatacgcccggcgtagataaagtaggcacgccacaacccggatcactcggcagctggggcagacctgtgaacgcacccgatcatgtaaaaaacttttataacaccggctccacctttaccaacaccatcgccttcagcggcggcacagaaaccgcacagagttacttctcctacgccaacaccaccaataaaggaattcttcccaccaacaaattcgaccgccatacggtgaacctgcgcgaaaccctgaagctgctgaacgacaaactggtaatggacgccaatgtatcctttaccgcacaaaacacgactaaccggttgtcatccggattgtactacagtcccatttccgggctctataccttcccccgcgggcaggacttcgactattacaaaaacaattttgaatactacgaccagggccgcgacctgtacatgcagaactggtggaacatccgcaatgataaaaaatggattggccaggacgaccagcaaaaccccatgtgggcgctgtaccgcgacctgcgcctggattcccgctaccgcggcctcgctaccatatcgcttacctggcaattgaacgattggctgtcgctgaaagggcgcggcaactttgacaaatcgctcgatcaatacgaactggaagcatacgccggtacacaaatcgtactcgccggttccaacggccggtataccctcgaacgggaatttaatacccaactgtacggggatatcatgctgaatgccagccgcaaaatgaacaagtggctgcacctggccggtaatatcggtgcaagcatcaccgacaccaaagcacacgaacgcacttttaacggctccaatcccaatgccgatccgggactcacgtaccctaataaattttcggtatccaatatcctgagtacctcgctcgatgcacaacacagcatagatcagaaacaattgcaggccgtattcggcaatgtgcaggcaggcatcaacaactaccttttcctggatgtcaccggtcgtaacgactggtccagcacctttgcctatacctctaccctgcataaaggatacttttactattccgccgggctgtctgccgtatggagtgagatgtttaaaatgcccgccttcattgatttcctgcgttcccgtatttcctacgccaaggttggtaatgatatcgccgcttacgcatcccggccggcggcatttacgttacaaaccattgccggcgtaacacgggtagtattgaatcaacgtaccctgtatcccggtctcagcctggaaccggaagacaaccgttcttttgaaataggactggaaacacatttgctgaaaaacaggatcaccgccgatgtaaccttctataaaaataataactacaagcagtacatggaagtgccggcgccattgggtaacaggtataacacctactacctcaacatggggaatatacaaaaccagggctgggaagctacgctcaccttaatgcctatacgtaataaggcagtatcgtggaccagcaccatcaactttgccgcgaataaaaataaaatcgtttctctttccaattccaggatcattggagcggatacgagcagcatgtttgtgctcaccgatttcggggtaaatatgtttggctccttcattatggaaggcggctcctggggcgatatctactccaataaagaattgttgcagaacgataagggcgcttatgtaattgatgctgccggcaaattgcaaacgcgcaacgcatttaaaaaagtaggcaatcccaatcctgatttcacattgggatggaacaacagcatcgactataaaaatttcaacctgagcttcctcatcgacggccgcttcggcggcaaggtgatgagtgtaacacaggcggtattggactggtatggcgtaagtgaagagagcgccaaagcccgcgataaaggcggcgtggaaataaatgcggtgaacagcaatggaacgccttacagcggaaaactggatgcgcaaagctactataccaccattggcggcagggccggcatcggtgaaatgtatatgtacgacgccaccaacatccgcttacgggaactgagcctgagctaccgcataccgctgaagtggaaatggatacggaatatgcggatgggcatcgtaggcaggaaccttttcttttttgagctgcatgcaccatttgatccggaagtatcgatgggaacaggcaacggactgcagggcgtagatgtttttggcttaccgcccacgcgaagtatggggatcaacctgagattaggcatttaaaatactcaccaatgaaaagctggaaaatcgccacattatccgccgttatggcaattctgctggcaagtgcatgtacgaagaattttgatgagattaacagaaaccctttcgactttacagaagaggagctgaaagccgattaccggctgatgggggaacccttatcccaggcgcaactgaacctgcttatttataacgacccgcctaccgcgcagttacaacagaatctgaatgcagatgttttctccggctatatgatggcccccactccttttgagggcaatatcaataacaccaactatggcctgttgtactactggaataataaaccatggcaggtaacttacagcaacgtaatgaagacctgcgattttgcacagtcgaaagcgaaaggccattatgccgatttttatgcctgggcgcagatcatcaaagtggaagccatgcaccgcatcagcgatatttacggtcccgtgatctacacaaaatatggtatactgaatgaagaaatgggcattgattatgattcacagcaggaagcgtactatgctttttttaaagacctggatgaagcggtggacacattaaccggttttataaacagtggcttcccccaacgctttgcagccttcgacctggtatacaaaggcgattacacccaatgggtaaaatttgccaacacccttcgcttacggctggccatccgtatttccgggattgatccgaagaaagcaaaggaagaaggagaagcagcgctgcggcatccgctgggattgctcacaacacctgcagataactttgcagtgaatatttcaccggttacgcatccgctgaatattatgtgttatacctgggctgatctgagaatgagcgctcccatggaatcaatcctcacgggatataaagatccgcgattggcacattattttgtgcctaccgacgatggcgtaaatatttaccatggcatccgcaacggtattaagattgctgccaaggaagaatacagcggcttttcacaactggtaaagtttgatagcaggatattatttatgacagccgcggaagcctggttcctgaaagctgaggcggcgctgtatggctggcagggcgccggtaatgcagctacgagttatgccaccggcatcaacacttcttttaatcaatacggcattactaacgctgatgcatatatgaataacaatatggataaaccccatccatatacggatcctcaaaatagcgacaataacataccggaaggcgatccgcatttaagtacggttaccatcaagtggaatgaaagcgctacgcttcaacagaaactggaacggattatcacgcagaaatggattgccatgttccccgaaggacaggaagcatggagtgaattccgccgcaccggttaccctaaattattccccgtagtaattaacaacagcggcggcaccatttctaccgaaaaatttatccgccgcctgcccatgccgcagatagaactcgttaccaatcctaaagcagtagcccgcgcagtagccacgttaaaaggaccagacaccggcggaacaccactctggtgggatctccggtaatatctcaaaaaaaaaataaaaataatttaaaacaggatagtactaaatatatctccacacgactcctttccggaagcgccacatttgaacgctttatgctacgcagcctgtaaaaaacagacgttattaaaaacaacatttcatgtaaggaaaacacataacaacaaactgctttgctcaacccggtcaacacattgccattagcgatgaggccttgcacgcccctataggccggtaaatgcatgtaacacgaagaaaaacagccgctaaaggatggtacgcgccatgctaacggacatctcatttccaaacaatgcacgcaataaaaaaatggtcagtttaattcaacaatacaaatcccatttattaaccaaaaaaaaggcaagtatgaaaaaaaacctacgccttatgaaagtgtgcgctatgaccggtctggccctcacttccatattagcagacagtgcatatgtgaaggcagccagctatgtatggtcgcccgcatcttcattccgtagcactttccaggaaaaagaaatcagcggcaccgtaaaggacagcaaaggcaatcctcttcctggtgttactgtacaaattaaaggcgcctccaaaggcacccaaacaagcgcagaaggtaaatatcacatcaatgccaaaaccggtgatgtacttgttttcagctatgttggttttgccattaaagaaagtaccgttggcaacagcgctaccctcaatgcaaccctggaagacaatgtaagaggactgaatgaactggtagttaccgcgctgggcatccagcgtaaagcaaaggatctcacctactctacccagcaggtaaaaggagaagatctcacgaatgtaaaagaaacaaacgttatcaatagtttatccggtaaggtatccggattgcagatcaaccgcagcgcttccggtgtgggcggctctgccagggtgattttacgcggacaaaaatctatccgtgaaaaccagccgctgtacgtgatcgatggagtacccatcgcgaacttcaccagcgcacagccaggtgatctctggggacaagcatcaggcgcttcctccggtggacgcgatggtggcgacatcctgagcaccatcaacccggacgatattgaaagcatcaacgtactgaaaggcgcttctgcatctgcactgtacggcagccaggcgggtaatggtgtgatcatcattactaccaaaaaagggaaagccggtcaggcaaaagtgaacttctcttctaacttcactatcgacagacctgcatatctgcccgaatcacaaaactcctatcttcaaaccggcgccggcactattgatagctggggtaaagcaggcagcagtaaggaaattgtaaaagacttcttcaaaacaggcaccacctggatcaactccgtaaacgtagccggcggtacagaaaaggcacaaacctatttctcctactccaataccacgaatacaggaataatgcctactgcaaagtatggtcagcatacgctcaacttcagggaaacaggtactttcctcaacgataaactgaacattgacgcgaatgtacagatgaccacacaaaatgcacataaccgccctacttccggtttatactataacccgcttaccggtttatacatcttcccaagaggactggacttcgaaagttataaaaacaattacgaatacttttctgcccaacgtaacgtgaacatgcagaactggtggaatatcaattatgataagggccaggcgggagaagactttcagcagaatccatactggatcctcaacaggaacgtcactgaaaacaggaaagataacctgattgcttcgctgagcttacgttatgctatcaacgactggttaaatgtacaggtacgcggtaacgccaacaaagcatgggataaatatgaactgaaagcaaatgccggtacacaaactaccattgcagacgccaacggccgttatacctacgattacctgaccagcacacaatactacggagatctgttagtatcgggtaacaggaaactgtccgataaactcgggttcaatttcactgccggtaccagcatcaacgaccttaaacaagaccgtacctttatagattccaaagacggcgacctggcctttgccaacgtattccacattggtaacctgaacctgagccctgccgcaaaattaacgcccacaggcgccagaaggcagatccagtcggtatttgcaacagcgggtgtgaacctgagcgaaaaagtattcctggacctgaccgcccgtaacgactggtcatccaccatggcttataccccttccatgaagaaaggttacctgtattattcagctggtttaaatactattctgagtgatgtatttaagatgccttccgcgatcacgtattcaaagatccgcgcatcttatgcgaaggtgggtaacgacgtggaccagtttgtaacacgccctaccaaccagatcatttccggaacgctgatatcaaacattgccggtccttttggcggcgtggcattgaaaccagagatcaccacttccgttgaaatcggcacagagtggagattcttcgacaatcgcctgaacctggatgtgacctggtataattcacacaccaaagaccagtacttcgacttccccgtatccgttggttacctgtatcctaatgcttacctgaatgcaggtgatgtacagaataccggtatagaagccacgctgggtttccaggtagttaaacagaagaacgtgggttggaataccgccttcaacttcacccgtaacaggaataaacttatcaaactggcgccgcagttaaacggtgattataccctcacaccaagaggcgataacgttaatacatatgcgctagtactgcatgaaggaagctcctatggcgacatttacggcaggaaagcagtgcgcagtgaaagcggtgcactcgtaatagatgacgaaaccggtaagccaaaagcaaaagacggcaaactggaatacctcggtaatcccacaccagacttcctcctgggatggagcaatactatcaactggaaaaagttcaatgtaaacatcctggtagatggccgctttggtggtaaagtaatgagtattacccaggccatgatggaccagtatggcgtatcaaaagcaagcgcagatgcccgtaataacggtggtgtggatgtacctgctgtttatgccagtggtaaggcatacaccggaaaagttcctgcagatctctactaccagggcattggcggtcgcgcaggcatcactgaattctacatgtatgatgctaccaacatccgtttaagagaattatccatcagctataatttcgcattgaaaccaggattcttcaaagacatgaagcttggactggtaggacgtaacctgttcttcatcactaaaaaagcgccttacgatcctgaattgagcatgagtaccggcaatggtgtacaaggtgtggatgtatttggtttaccatctacccgcagctttggattgaacctgaaatgtgcattttaacctgattaagaacaacaaaaacaagagctatgaattataaaatattcaaaatagctggtctggcgatggcagccacactatgcttcagcagctgtaccaaaaactttgaagacatcaacaaaaatccatacggctccactgatgaggagttagcggctgatttcgccctggtacctgccctactgcaacaggcacaacgcagtatttacctgtatcagccggcgcctaccttccagttgcaacaaaatctcctgagcgatatttacagtggttatatgatgtctcctactccgtttggcggcaacatcaacaacatcacatacagcttcgtggatggctggatcaacactactttcagcaccggctataccaatgtaatgaacccctgctataaagtagccggttttacaaaaggtaaagtacccgatagctacgccatgtcgctgatcgtgaaggtggaagccatgcaccgtacctccgatatctttggccccatcatctacagcaaatacaatacacccagcggtgatggttctgttgagtacgacagtcagaaggatgtttattataccttctttgaagaactgaaaacagcgatcgatattctaacgccgctggccgataaaccgtctacagagctgtttaaaaaatcagatctcgtatacggtggtaattacaaacaatggttacagtttgccaataccctccgcttaagactcgcactgcgtatcgtaaacgtagatgctgcaaaagccaagctggaaggtgaagccgcactcgccaatgccggcggactgctgcaaacttacaaagataacttcacggtggatatcggaagcaccacgcatccgctgaacaccatctgcggctcctggggcgatattttaatgggcgcacccattggtacttatctcggtggttacaacgatccacgcctgcccctgtacttcaagaaagcagtggaccctgctgtaaaagacaggtacatcggtatccgcaatggtattaacattgacggtaaagcacgttacgccgactattcgaaactggtagacctgcctggtaaactgcaactggtaacagctgccgaagcctggttcctgaaagcagaagccgccatccgcggatgggcaggcgccggtaatgcacaaaccaactacgaaacaggtatccagacatcctttaatcaatattcattaggcagcgccagcacttactacaacaatgccacttccctgcctgctgaatacattgatcccaaggccatgactgccggacaaaatgatattaagaagggttcacagtacctgagcactgttaccatcaaatgggaagaaggcgttacactcgacaggaagctggaacgaatcattacccagaaatggatcgctaactttcctgaaggacaggaagcatggagtgagttccgccgcaccggttatcctaaactgttccctgttgttgtgaataacagcggtggaaaagtaagtacaactgatttcgttcgcagggcgccattcccaagtaacgagtactctaccaacggtgctgctgttgcgaaagccgtgagtaccctgagcgaaccaaaagacgtaggtggtacccatctgtggtgggatccgaaaaaataattaccagacattcttattttgaatcgcgtgcataaaaaaggccggtcctgttgaggaccggcagcgaattttgtcttggctcaggattacgctgattttactgattacctgtatttttacttttggatttataaaggattaagggagatagaagcgggtatattcgcttttatctcccttaattattattaaaaaaatcaaagaaatcaaaaaaaatcccaaagtaaaaatccagctaatcagtaaaatcagcgtaatcctgagccaagacaaaatccgctcttttacctttgaaagaactcgtggaaaaacaacagctggtatttcactgcgttagcccagtatttccagttgtgttctcccgggcgctccgtataatcgtggtcgatacccgccagtaataattttttatgaagatcccggtttacatcgatgaagaagtctttcactccgcaatcgatgatgatggacaatgcgccggatttgaggctatctacctgcttgaggaccgtatagtcgtaccagttagcgccatctgttccgggttcacccaggcgttttttcagatcccagttttttgggaaggggcggaaatccacgccgccgctcatgctgccggcggctccaaatacatcctggtggcggatggcaagaaacatagcaccatggccgcccatgcttaaaccggcgatggccctgtgagcgggttcgggtaaggtttggtaatgctggtcaatgtattgtggaatttccttcgacacataggtttcaaaacgcatggagctgtctacggggctgtcgaaataccagctggttaccgcgccatcggggcatacgatcatgcactgataggtgtctgccagttctttgataatgggtacgttggttacccagttagcgaagttgccaccggcgccgtgcagcaggtataccaccgggtagcgctgcgtaccatttttataggtattgggggtgatgaccacgcatttgtaggcgcgctgcattttgctgctgtgaatagaaacggtatctacatccgcggccctggctgtttgcgccaggcatatcaataataaaaatcgggctattactttcataactcgggcttttaaaagaatctaaaaaaatatagcggctaccataccaggatgatagccgccacaaaatataaaatagcttgtttattttgtatttgctttcttcatggggttatcgccggttgaagcgccacgaatgccgcccgatgatttaaacaactcaaacctggagggtgcggcctcccgcggccagctgttgttgctttcatcgatatcggctgtttcacgtattgggtcgagcttcacggctactacctctttatcttttgcaaacacctttgtaacggtgttttcatctttgcgccagatgtaggcagagatccggtcggtttctttggtgccatctgcaaacgtccactcaatgatgagcggcatcaccagccctcccttattagagaatgtcagctgataaaagttcttcttactgtcgtacaaggctttttcttctttgctcaggccgttatagaactgcgtgtaagccgctttatcttcctggcttacctcgaagcggttccatttgctgtagaagtcctgcaggctggtatcctggtccaccgtgtattttacgccggccgccttatttctctgcctcgctacgtgatccatgtttttatcgtaagctgcctgcgctgttttagctgtttcttccgggtttttaccatccatgcgataccatttgaggctgtcgatagagatatctaccggttccgttccgaagaaccatccgcgccagaaccaatccaggtctactgcagaggcatcttccatggtacggaagaaatcggccggtgtgggatgtttgaaggcccagcggcgtgcgtattcacgaaatgcaaaatcaaacaggtcgcggcccatgatggtttcgcggagaatattcaatcctgtagccggttttgcataggcattaggtccaaactgcacgatgttctcggagtttgtcatgatgggctccagctgatctttcggcatcttcatataatccacgatcttatgagcgggcccgcgggaagaagggaagttgctgtcccactcctgttccgccataaactggcagaaggtattgaggccttcatccatccaggtccactgcctttcatcggagttcacgatcatgggaaagaagttgtgccccacttcatgcgtgatcacgccaatcatcccgttctttgttgactcactgtaggtaccgtctttatcggcgcggccatagttaaaacagatcattggatattccatgccgttggccgcttctacggaaatagccaccgggtaaggatacggaatagtatgtttggagtaggactgaagggtatgcgccactactttcgaagaataacggcggtagagcgggtaggcttccggtccgtagtacgacatggccattactttgttgccttccacgttggtcgccagggcgtcccatacgatgcgacgggaagatacccaggcgaagtcgcgcacattctgcgcttcatatacccaggtgtttgttttgcccgcgtggccctgcatggctttctttgcgtcgtcgaggctcaccacttcaacaggctctttgctgttctgcgcctgttgccagcgctggtattgggccggtgtgagtacttctttatagttctggcattcaccggtggcgcccactacgtgatctgcaggaacggtcatgcgtacacgaaagttaccaaaggtgagggcaaattctcccctgccggtaaactgcttgttctgccagccctggaagtcggaatatactgccagtcgcggataccactgggaaatagtgtacaggtaatttttatcttcctggaaatattcataccctccgcggcccccgatggtcatgcgatcggaaatattataccaccaggatactttaaaccggtacttctcaccgggcatcaatggctttggcaggtcgatgcggagcatggtctggttgatggtataaggtagtgctttgccatcagcatccgtgagctttacaatctttacgcccaggtctttcccggaaggcagaatgctgttcaacgtagccagcgtcattttatcagacatacggctttcattgaactgctggttatcgcttttgctgtcgtgttcattctcgtcgagctgtagccacaggtaggtgagcggatcgggagaattgttaaagtaggtgatggtttctgcgccggtgagtttctgctgctcatcatccagttgcgcctcgatgtcgtaatccgctctttgctgccagtatttagggccgggagcgccggaagccgagcggtacatgttgggtgtttgcagcattgttcccagctgctcaaaacggttgccatggttggatcccgggttactttgcgcctgcagcaacaaaacgctgcaacacaatacccccgcgaggtaaagttgttttctcataaacagtattatataaacagtgctcttacgctttgaatgatcattaaaaatgcgacgccaaaggtggcagaagaaaggaacatgttccaatcccggcgttttacgcctccaaaattcacgatcgcagaggaaatgagcagtatgcacatcacaatgatgatctgcccgaattccagtcctaaattgaatcccagcagtggctttacaatatctgcctggcttcccagcaaacttttcagataattggaaaatcccagtccgtgaattaaaccaaaaaataaggcgtaaaaatagttcagctgcagcttttgcggctcatcgtctttccggataatgttagaaacagctgttacacaaatagtgaccggtatcaggaactcaataagcgccgcaggtatacggataatatgtaacacactcaaagccagcgtaatagaatgaccgatggtaaatgcggtcaccaataccagtactttcctccagtcacgcagcaggtaaatggcactcaacgctattacaaaaagaatatggtcatacgcatcccagtttataatatgttgccaccccagctgaaaatacaactcatccattgttcccttttctataattttggtaattataaaaagtaaaagttaattttttttaaaatcttagtccagtgggtttattattatgtaaatggtggatgactttgtggctcacagccctgcaccccttctatgcaagcgtgacagagatttcgcacgacgccggtaaaaaggaactgcaggtaagctgccgcatttttacagatgacctggaaaatacccttaaagctcagtataaaattcctctggatatcacccaccctgccaacaggaaacaggtggaaggttatatttccgcctatctttcccagcatctcatgatcacactcgacggtaaaactgttcccctgcacttcattggctataaaatagaagaagatgcagtgtggagcttcctggaagcggaaaatgtgcccgcaccaaaacaggtacaggtaaagaataacctgttgtatgaacgccatgttacgcaaacaaacatggtgcatgtgctggtgggcggagagcggaaaagtgtgaagctggataacccgaaagaggtggcggtgatggggttttaggccataaaaacagatttcgaaaatttcaataaactaaattaaatttcatttattgaaatttaattcttaccttcgagaggtaaactcttgttatggtgatcgtttcgagacgacttatatgtttttgatataggtggaaataaattcagactaatagcaaggattttctctcgtgtccgaaccgtatatataagatttataggtactcacaaagaatatgataaagtaaaacctgattcgctttaataacaggcccacctgcacatggggtgatgtgtgcacgcagtaaaaacgataatatgaaaaagttacccaacccttccttttctactgaaaaagagtatgctgccgcaatgcaacgtattcacctattaatgaaaaaaggtgaatccaatttaagtgctaatgaattaaaagaacttcaacaactttccatcgctgctgagcattatgaagatacacgttatccaatccctaagccaactacattggctggcatgatagcattaaaaatgtttgaaatgaaactcaaacaaaaagagatggcaagtatgttggatataggagaagccaaattttcacagatattaaatggcaaacgagatccggatgtggattttctgaagaaaatttatcacaagctcaaaattgatgcagagtttattatgcagcatgtttaactcctgttatccaaaaacttcaccggcttccggctgttctccggaaactgcatccgcataatatcctgctgactggtataccgtacctgtggaattacgcgcagctttgcctgcagataagattttattttgcggtccatttcctctgattcttcccgcggccacaggtgcagtagtatttcatccgtaccaagttcattggaatacacttccaccacaaattctttcacatcttccatatcattgagcaaatcaaacagcgcaggtggatacaacgtagtacccttatatttgatcatctgttttttacggcctattacgggagataaccggagcgtatgtctgccgcaggaacaggcttcataatgatactggcagatgtcgccggttttataacgcagcaggggcatgccttccacgcccagggtggtaatagttacttcgccttcttcacccggggcaacaggctgattgttttcatccagcaactcaacatagagcagttcgggatggtgatgaccgccctgcccggctttacattcagtaaaagcagtttgcatttcagtggatgcgtaggtggaatagagctggatattccattgctccgtaatcttcttgcccagtacattcagcgaaaaatccgtattacggatattctccccaatgcaaacagctttctttacagacgtctgattgatatctatatgatgctcttgggcataagcaatcagctttacaataaaagaaggaacacctacaatagtggtaggctgtatccgctgaatgttttcccactgcatgcttggtacaccaggccccacacgcagcacgcccgctcccagtttacggatgccattgtaataagccatacctgccataaactggcggtccagcgtaagcatgagctgatagatgtcgctatcggtgccatctgcacaacagaaagaaatatattcattataacttaaacgctgcaggtccttttccgttaaggcaataatcaccgggcgtcctaaagtgcctgatgtagtggtgtattcggctattttacttttatctacacaaagaaattcccagttgtgttcctggagatcttcctttgttacgggcgggatctgtgaaaatgcttccagcgattgaacctggtctgcaacgatgccgtgttttttaaaccatgctttatagaatggtgaaaattcacgcaggtaacctagcaggcgcattacttccttttcctggtaggccctgatggctgctttcgactgtagttcaatatccggtatatacatctgctataaatttatccttctaaaatcaccattgcaacagcggcacttttttcatgggataaggatacccatattttcctgatgcctgatgatgcatatctgtcagcaccatttcctattaaaaataattccggtttcccaacttcattattacggatctctatttcatcgaagttaacaccgccgtttccccagccggtacccaacgctttgagcagggcttctttcgcagcaaaacgagcggcatagctttctgccggcatcgcctggttttcacaatagctgatttcaaaaggggtaaataccaggttccggaatccatctcccttcgccagcttggccgcgatacgcggtacttctacgatatctgttccgatgccaatgatcatagtggttagctttttagtttagcattgcacagtgccagttgtttgcggatgtgatcttcctctcctttggtagcaattacttttgttaacgctgtttcgtaataacctttcgcctttgcatatgctttctgctgatactcataatcgccggccagcacataagtatgatagtaggccgggttggaagcgatcaatgcttgtatatccactgcctttccttctttcagctggtctctcagcctgcggtaggtttcaaaggcaagataatcttttgacagcaggaaactatcagccgcaatgctctgcgcgctgtcatatacttcatggtcggtagtaagaccatgcatgctgaaaattttattcagatcgtaagccacaaactgtcccagctggtaaggagctgtagatacccataccatccccttcttaggttcaaatacgattgagtgatgtgcaatcagctggttaatagctttctcattccccatcccgatatcggcattgtgtaaaccaccgcggtcgcgcaggatatccaccgttttctgaacagtattgggtcctttctctttcatcagctctgtcaacctttcgtagcggtattcagaggcgctttcctttatctgcaatttgttagaggccaggctgcccagtgaatcgccctggaagtgattggtacaggtaataaaatttttaccggagctgtacatatccatgccctcaggcgttttttcaatgagcaccgctttattatcttccgcagaacctacgaggaaggattctgaaacaaacatcttacgcttccgcgcaatctcccatgcttcctggatgttcttcgcatattgcagtatttcccgcgctaccagcgataccggcgtagcagcagctgtaggtacgctggttttggctgcattgatcgttacggtaagtcccttgtcgttcatgccggaaaccacgccggtaaagccgccccaggtgacaaacataaagttgtgtcccttttcaggacggtagaataccaccatcttctcttctgcaaaggcatcacccatgtaaaaatcgaaattgcggccgatgatcaggttactgtcggccgattgatcattccaggtgccgaacgacgtacaacccaccagcatcatgccttgcagggcatgtccaatgtcgtgcgctgcatgatagttcatcagccgggcatagttggtcccgatataatcgtagttgggtgaagctgaaaaagactctccgtaaatttcttccttaaactcttccggcacatgatctgccaggtcgcggttaaaccagccgataaaatatttcaggaaatgcaggtaaaaagtggacggcaccattttactgaactgtgccacaaatacgtcttcctggcgccggatcaactccccggagagcttaccgttgatcacgcctctttcaaaaggagcgccttccacatacatctcgtataaaccactgttgcttttacggaaccagttgttacccagtgtgtaggcggtgctgtccagttgggtacgttgcagctgcaatgcacgctggtcggctattaccggcggcggcattttacttaccgataccaggtaaatggccagcccgataaaaagcaatacaaaaaagccgatgatgtatagtagtatgcgcccaaatcgtctccagccgctgcgtttcttatttttcacttcaagtatatattgactgattaatttcatttaccaaaaaatccattcccagcaactctgccgaggtgatcacactactgatagttacccctaaaattccatgcaagttcaggttttgaccggtaagatacaaattggatagtttggtgcgggccgaaaccattgtccgtagcggatctgcactatcttttgttatgccgtacatactgccgtcgctggtaccgatgtaatcacgataagataacggcgtagccacataggaagtataaatacaattacggaagccgggaaactgcttttccacgcaatcgatcagcaggttggcttttctttctttaaaagcttcatagtccgcgcccctgctgccggtttgcaacactgtattaaaagtatgctgccattgctttacttcgtcgtaccgcatgtaggtcatgatggataaactatcggcccaggtttcatgccgcgagctggccgacacatacatcgcataggtttgcggccaatcttcttctttatagtcaattcctgcccaggcgttgcccgtggcatggtagtaatgattgtagttaaggtatttaaaggtacctggtttcaatgccacgttcaatacaaaagcccctatagagttctctaacccctgcatacggctgcggtaagcgccgcgcaatacatcgctgtgggtaatcgccatggtttgcgccggatgcaggttggaaatataatgcgtggcctgtaccgttctcccatcctgcaatacaatatgatttaccttatcaccttcgccgtggatagcggtaaccgccatattgcggattacctctccgccgttctcccggatctgttggcacaatagctttcctatttgggagccgccatccacacacttccaggagcttttcatataactgtttaacaccaacgcgtgtacgtaaaatggtgtcttctccgctacaccagcatacaaaagattgttaccagccaatacctgctgcagcttttcattgctggtaatactgcgcaaatactcagcggtattcagctgtaacaccgaccgcttctcttcataatcgccggtacggagattatacagcgggaacttactgcagacttccgtgattttattgcaataagcacgcaatgcgttttcttccccagggaaatcttccagcaacgtgcggataaaattttcttctccctgcgctatccggtatactttatcatcaccggcaaaactgatatggtcaaaaccatccatatccatacgtttcagccggagcttatcataaatgccgaggtatttaaatactttgtagagattttcaccgggcgccagtccgccaatatagtgcacccccgagtcaaaaataaccttatcgcgtgaccatgtttgcaggcatccacccgtttgcctatttttttcgtatatgcatacacgatacccatgccggctgaggatagctccacataccagtccgccaaggccgctgcctataatgatcacatcatagtggtgcataatcctcccggggaagtttttttatcacaaatattacgttagaggtataccgcgtattgtctatttcctccgccaccgcgccgtatttgtgaacaagactacggacatgtgcagctgagaaaaacgacaatggctggtctttcgttttattaaacccaattacttttgtagacataaactccgtgaacttcgtccgctcgtgccttttggccatatcgctgtcgccatcacggattacaatcacgccatccggcgtaaggcgcgctatacactgctgcagcagcatttcctgctcaccggcaggcaggtagtgcaatacatcactcagtataaaggcgtcgtatgctgcaaaaggagtagccgaaatatctccatgaataaattgcagctgttccggcttattataacagtaagcggcagtggcaatcttatcttcgtcatagtcaatacctgtgatggttctgcccggtgcggtccaggtaagcatgtaatccatgaatccatatccgcagccaatatccagtatacgtccttctttgggcagcaactcatggaacagctggtaattgttttccatcgccgttttcacgcgcatataccattccagcaccggccctttgtagatgtaattatacttcagctgctcccggaaatactttggcacttccgtttctgcgcgcaatagctcgtattgttgtttaaaataccggctgatagatttcgtacgtgcgctgtagttatctccccacgacttatcctcctgcctgatacgcggcaggtattttaccgataccgttccatctttcaacaggaaatctcctttactcatcgtataggcggtaccgtgaatcaccattggtaaaatatccaatcccagttgctctgcaatataaaaggcgcctttatgaaaacgcttaatagccggatcgggagaacgggtgccttccgggtacaccacaatggaatagcccgccttcactctgtctctcagcctgtcaatagctccttctgcgccatccgctacggggtagtaatccgccaggcgaaccactgacccaaataccggcgaccgccatacccattgattggtaagcaatatcaccttcgggtgcagcatagtggataccaatatatcgaggaaagactgatgattactgataatcaccgccggtttctccagttgttcattggaaggattgatgatgcgcttcttcacattgcgcataatatacaatacgctgtgcgtataagcagaaagtatacggtgatacaacaccttgcccttttctttattgaacggattccagcggatcagtaccgtaccaatggcggtaaggataaaactgcccatggcaaaataagtaaaggaaaacacagacagcgtccatcctttgaaagtccatggtgcaaagcccttccgtacacggccggtgatcagccagttaaacaggaaagggatcattacctgcgaaatcagtactacagtgctaataccgataatagaaatcagcgcaatagatttaagcgaaggatgttgtgcaaagatcagcacacccagcccaagaatagtggtgatggccgacaggaagatggatgatttaaaagaagaaagggttttctttccggtcctgtactcctgcaacagcccatccatcataaagatgctgtaatcgtctcccaaaccaaaaataaaagtagaaaggataatatttacaatattgaacttaatcccgaaaagccccatgatacctaatatccatacccagctgatggccatcgggataaaggtgatgagcgccagttcaatgcggccatacgataacaacaacgcaaaaaataccagcagggaagtcatccacgcaatgctgttaaattcatctttcactacttccaccaggcggttagcggcgtattgtttgtccagcactgtcgtattcgggatattttccaacgcatcgtatactgcctgtttgtgcgccggatctactttcagcaatgttactacggaggtagtgccgttcttctctatgataaagtctcccatgttgccgctgcgcagtaccttcaaagcatccggatcaagtggtttgaaatcattgtttatcagctgatcgaacggatcaaaagctgccttgctaaagcccagcacacttccctcactacggagatattccagcaattgttgtttcctgtctgccgtccagtatttgttccagcggtcaatgcgcgcctgttgttctttattggataacagtaacgcctgtacgccggcgtacttttttacgacacccttctgctgcaaccgttcaatgaccggcaacagcttttcgccgctttcaagcgccccttccaggtcccggccatccgatactacatataccgactgcgctacataggaattcacactgttgagctgtgcttctgctgcttttaattgcggcgtcatgtaattcatacgcatcatatcgctttcaaaggatacgttgcgcgcggtatagaaaaatacgatggtcagcaggaaaatagcgcctaccaggtatttatttttctccggccggtatgccgataatttgtcgagccagttatcatgatgcgcggctacctgcaccggttgttgccccatcacaatccagtggggcaggaaaatcagcgaaaacaatgcagcgcccaccaggctgagtgcggcaaacagccccacatctttcagcatgggggaatgcacgaactgcaaacacaggaacccgccgatagtagtgaagctaccgagcgtcataggggtagccaggtcgctgattacttcacggatatcctgcgaatggcggtagtgattaaatacatgcagcgaataattcaccgcaataccgagtactacagcgcccgcacccatggccattacagagatatgccctttaataacgtatatccatgccagtgaaaacagtccgccgaaaataaccggcagcatgaccagcaccggcgctcttttctttttaaaaaacagggcgatcagtactatcaatagtactacggtaatgccttgtgttaaaaaagtatcctgtcttagctgcgtggcattgcccacagatacagcggttcccccgaagtaagaagcggcgataccggggtattgccgatcaagactatcttttattttatccagtcctttcaggaactgtgcattgatttttgtggcgcccggcggatttgccggggtgataaggatcatcaggtgtttatgatctctggtgatgatgtagttgtcgtacagttcaaactggtcatcatactgcaggtgttgcagtttctttacgcctatccaggagatgcctacgggatcggcctggatcatcttttttaacaccagtcctgttggtgatatcagcgtattataatcatattgtaacgattgctgcagttgcccgggtaacaacaaactatcaatcttcgcgtaatcatttttttccaggaagatgggcaggtgttgttgtatcacctgcatcaatcccattatcatggcgtcgtctgtttgcgactggatctgcctgatatagggcgatagctgcgcgcccgccctggcagacagttctgcggcataagccgttaggctgtcgggccgggcttcctgtatagtatctttttgggagatggtaacaatcagcttgtctgcaaatctggaatcctggaacacctgttgcagtttatccagtttcttatcctgcggtaaaattttggtaatatcttcttccagctttatttgtgcagcaaaatatccaaccagcaaaaaactggcgatggtgcaacaccacagccacgctttacgccgctcaaaaaaattatagatcgctacaaaaagattacccatttcttcgttcttttctaaaaattgtcagtattgcccaactcactatccaggccagcaatccacccaatactgccagtgtaatactgccaaatacatattgtaacaggttatccctgatggtgtcgaagttaataccattggaaaataccaggtctttggcagtttgccccatccatatccggccggccaggaagctggcaaagatcacaaacggcgttagcggcggcgtgctaatatgcgcaaaaagcagtaccaacgccttattcaacctgaattttatagacaacaggatagataccagcagctggaatccccagataggtatgatccccataaaaataccaaagccaatggaagccgctttcctgatattggattcgtcagacttcagcacttcttctttccacatctttttccagttttctttttttaaaagaaaacggatcaggtcgcggggcttgatatataaaaaggtaacgaacaccagtatggtattcaatacagtaatacgcgaaacgtcccttaccggtctgaaatgtgatacccgctcttccggtggcgggtaatatacacgcacaggtgtccagtccaccttgatacctttccacgcactacgcaccaacacctctatctcaaattcgtatttggtgcagaagtaatgcattctccccatgcgctgcaggggatacaggcggtagccggattgtgtatcagggccttttaatccggtagttacgtgaaaccagaagttagatactttattggcagaagtacttttgcccggcatattctcctggtgcaggttccgggcgcctatgatcagcgccccgggatgttcttcaatctgctgcaacatggtgggcaggtcggtcgcaaaatgctgcccgtcggcatccatggtgattacatagtcgtagccctgctccagcgcataggaaaatccgcggcgaagcgccactcctttaccacggttggggctatacgaaactatttgcagggaagggaacttttccagcaccgcagctgtttcatctgtagcgccgtcgtttaccacaatcacatgactggtataggtaagcgcatcagacaatacagcgcccagggtaccagcgttgttatacgtaggaatgagcaccgcggcgcggtgacgttcaaaatgttcgttatgtgtaggctgactggtcacttaattgaatataccctggaacttcataaatattttatcgtcgcgcttcagcgtagcattcactttccaccctccttcatcttctttgtaggtaagtgaaacatccaccagtggctgtttcaccgggtctatcatatgcaggaatttcatctggctggcctttttcagcatcacctttttatccagcgcgctttccagcatttccgtaatggtctgcatcatgcatacaccaggcactacaggctgttccgggaaatgaccctggaatataggatgtgccgcattcaattcgatggtggcagtcacctgccctggttcccgggattgcgctgtaatggtataaaaatttcctgctaacattgaacttatgtgattatataattaaggtgacgttttacttttctactttctgcaatgaaatattgaatttgaaatgctcatgacgaatattgatcgtatccggcacgccattgttataatgctgcatccatacggtgacaaccggtttgcggcgcgacgacttttctatccgtaccagttcactacaagccgtgtccgtgatataatagttattacctttttcggtaggtaccactgtataacggtaacggttatccgaagccgtatgtgccgccagcagatcgggccgcagcagtactaatgcaaagtcctgctgcaaggttctcaccaccgccttcttgtccattttggccatcaggtagtgtttggtaaaatttccctgcttgtcaaattcaaaatcaaagaacttaaatcccatctcattggcaaataccacgcggatactgctatccggcatctgcttaaaaaacaggagtccgctcaggtgatgcttcaggatatccacctgtgtgctgtacagcgtggaggtgaactgcgggctgaactgcctgatacaagtcacatcgccgtttacaggctgtaaccctttgtacaccgaccggcaacctgccatcagcaacacgatgcccaacaagctacttagcagaaaataccgcatccgggatatttgtgttcaattgtttatgtaaaaaactaatggtggtatcatcacctgatgattctgccattgtaatctttgatacagaatagtcctgtttatctaccagcaacacaatcgtttggaaatatgttttcatcaccttgtttaccggcgtaagctccaggcggtaatactgcgcattttcagcggctttggtagaaaaatcggcgttatccagtacagttcctcttacacaatccaccgtaattttattgatctgctcaaacagcttattattctttcccgatactttattctctttctgtgcatctttgatacggatatctttcccgttaatcaccagcagataataagaaggctggaggtattccattcttactttattatctttcttaaaccagaatttccctttagacacaattttatcagacaacatgctcaggttcttttcctgtacaaaatcgcactgaatactttgtgtgctctgagccgcttttgcaaactgctgtttcagcggcgccatatccgctaccggtttaaacccggactgcgcctgcatttgcaggcttaccacacatccaattaataataacagccatttacacatatgctcgaacatttaacattttatcaattctctccaggcggtatcccttttcacggatgccccggatcagctgaggcagtatatcggcggttattttacaggtatcatgcaacaaaataactgctcccggtttcagctgctgcatgatccggtgcaacaaagccgtttcatcttttgctactgtatccagtgagcgtatgttccagcctaccggcagataattccctgcctttactgcccttgccaggttaggattggttacgccgtaaggcggccggaacaaccgtggatgcaagcctgtagcatttaccgtaagcgcatccatttcctgcatatccttcagcatgttaccagacaacttcatatcaaaccagaagtgatgtgaataagtatgattgcctattacatgtccctcttcgtatatccgtttcagtaagtactcattccccctgatatttttcccgatacaaaaaaaagcggcaggtacctgttcccgatgcaggatatccagtatctgcggcgtatatgcctcctgtggcccatcatcaaaagacagtgccactaccttttccgtagtactggcctcacagaacgcctttaaaaaaaaacccgattcaatattcatcgccccgtaaacagttaccgggagaaaaataagcaccggcaaactataccaccagaaagaaataccatacgccattactttatccaggaataaaagtaccaggagcgtgataacagcaatgatatttacaatcctgttgtttagcatgcagtgagtaataccagtgaatgatgtgttccctggtgatgattatagattaatactttttttatcttctccggcgtcctgccaaaaaacactgctgcttccggcacttcctgctgcgctataatggcattcgccatccaaacgccaaatgccgctgctgtagggtattccccgcagaggtgtttaaagctggcttccgcatgatcaggaaataaggcatcggctacttcttcataaatttcatcctggtcaatatctccattcctgccggtaacgatcagatcgatatctgcaggcgtgcaattattatcttccaggaatttcatgatgtgcccgatcacttctccttcccagagcggcttgtataaggtgcttacaccggataattcggctacagcgccgggttgtttggcaatacccaatgtaaaaaaggcggcgccttctccggcaatagtgcccctggaaggactattcagcagttccatcgtttttaccggcgtctttttatagagtccgaaacgcgacagcaactggtgactgtgattcgtaatttcatccacgccaccggcgagaatatgttgtgccgaaccttctttcaatatcatgatagcgtccagcagggcgttttcaaaagaaaagccgcgatgaacgaaggtgttgttatatccgttgcaacccagtagcagcgcaatctggccggctacggtgttgtgggtgctttgtataaatgcagtaggcgtcagcatttcctccagctggttcaccattttagtgaggaatacgccggtgtcgtccaggcagccataagcagtaccggtaatgatagcatccggggcggtaacaccggctgcttccaggcttaaattcgctgcccctactcccattttcaccacgcggctcatcctgcggatctgtttcacatcaatccactgtttgtagtccgggtccactgcggccaggcgtacctgctcatattcccttggagcggccagcaaagggcctccctgtgcagtttcctgcggagaaatacaaccggtgccatttatatagatctgcataatttatagctgttaactggcccttgaaaatacgaggctggaacaattgccgccaaaaccgaatgagttggacattacatgttgcagatcatgacctgcagaaaaggcggtaacgggtgcaaacggtaactccttcatctggtgttcgaaacgtgcattcgggtaaataattccttcctttactgcgagcgccgaaaatacagcttctatgccgccgctggcgcccagcgtatgacctgtaaaggatttggtagaactcattgccgggaaatacggtgcaaagagccggtttatagcgattccttccgatacatcgttgttctgtgtaccagtaccgtgtaaattaatataaccaatttgttgtggctgcaatccgctcatatccagcgcacctttcatggccaggtagttaccggtgccatccggcgaagaagccgtttggtgaaaggcatcgttggcgttggcgaagccgctgaagcggcaccagggctgcaaacgggcagccaggctgtcggacaccagtaccacataacccgcgccttcgccgaggttaagccccgtacgggtatcatcgaaaggccggcagggctgctgatccaggatcatgagggtattgaacccgttgagggtaaagcgggtcagcgcatctgtaccaccggcaattactacatccacaatgttgttgcggatcagccgggagccatacatcagtgcgttggcgccggaagaacaggcggtgctgatggtagaaatatgatgacgcaccccaaggctgtcggccaccagttctgtgatgctcccgcactcgtggtgaagcaggttctgcaaccggccaccacggggatcagacaggtactccgcgaaaaaatcctcggttttatccatcccacccacggtattacctgaaacaaaccctacccggtattgggaaatatctcccaaaccgctggattgccatgcctcacgggcggcaatcatgctcagcagggccgtacggctgatattttccggcatccgtgctatatcggcaagggtggcgttatcggcctttacttccgctaccggaaaagtactgcggtgaacagaagacaggtgctgcatggcttccataccgggcttcatgtcccggaatgattgtatacaggcaggtacgtccagcccgataccgcagatcacaccaccacctgctatccacaccttttcactcatgcctttacggtttgattttcggtaatatacaccgccatcgtgcgcaccgagtggaagatcttcggtccttcttcaggattggcaatgcggatattgtagtgctgttgcagcaatacaatcaattccagcgcatcgatagaatcgagcccaagcccctcctttgtaaacaacggctgatcgttgccaatgctgtccggtgctacttcctgcaagttcaattgttctatgatctgcgctttcagatccgccatcaacttttccactgtagtttgattaaagttattaactgtttttttgttgatacaacgctgacaaagccgcctccgttaacgggatggcattgtttcgctgtttattttccacgaggaataatattgcctcgtatgcttgttccattacttccacccacccgcaaatacaggcctgcaaaggtgtttctgccagcagctgtgccggataggtactcattaaagccgtatcaaaaatatctgatacaaaaaaagtattctctcctttaaaaccatgccggatagaaatctctcccatcacgatattgggcagggtatacacaaacagcgccggactggcaaagtcctttacagtagcgtaataccgcaaatccgtatccagactgctgctccggttggacaataccatgcccgtttgctccggtgacaacgaatggatgccggtatctttcagcaatacttccgctgccagccagcccagcttgctgagggcatccattttatggaatttaggatattgaccggaaaaacggtcatatcccgcccgcagaaattcaggtaattccagcgcggaatccgcttcccacaacaaagagccatttaaataaaccctgttttgccgtatgacgcaactccccgtaatatatgtcgatccgctattcaatctcagggctgctttttaatttttctgttaattcaatagttcttgccagacgttttaaggcagtatcatgatttttcacaaagggattgttcatatcccacacataaccagccagtacagaacaaatttgtccttttatcagcggatcagcatcttttttaaagaaaatagtatccagggtaccttcgtaccaggccattacataagagcggaacgtattcacgccctgcatagtaggctccatatactctttctcccagtcaaccgcctcacctttcagtttccggatcaccagttttgccgccgtttgtgaagaaacacaggccaaagttacaccagatgagaaaatcgggtccagaaattctgtcacgttgcctgtcagcacaaatccatccccgtaaaatttatccgtggtggcagaccacgactgtaaaacacgtggttcaaataccagctctacatcgcggaaacgttccctggtatagggttccgcctccagcagggcgcggtatttgtcctcatcagtgccggggtactgttcaaaaaactcaggatctcctacaaaacccagggaggtaaccccggtagagaaaggaatgatccagatccatacgccttttttatgcaccaccgcggtaatgcggtttggctggtcggccatggaacggcgcacatccaccgtatgggcaaacaatgccttacggggttgcaggttggagtttttctccaggttgaataatttgggaattacccggccgtagccactgccgtctacaataaaacgggcggctatctgcgattgctggccatctttatcttccacggttgtaatggaatcggatccattaaaacgtatatccgttacggttgtttcataagctaccggcactcccatactttctacggtgtcggcaagcgttttgtcaaaatcggcacgcgttacctgccaggtccaggtccagcccggcgtaaattgctcttcgaaagtaaaatcgcagagcgcatctccttttacaaactttgccccatacttctgctgaaaaccttttgctttgatggcatcaataaatcctgcttcttccagggcttccatgctgcgtggcaacaggctttcgccgattacaaaacgggggaatttctgcttctccaccacttttaccttgtaccctgcctgatgaataatagacgccgctactgttcccgccggacctgcccctattaccagtacatcaacttgctcagttttcataagtgacgattttgggagttataaattttatgcgattggattggttattttttttgacatttcaacaaagtataattcatgcccatctggtcattttcctcgataatcgttaaccccgcatcatcaatacactggaagaaatcatctgtgtgatacatctggctgttaccattagccatagcggtaaagtacagggaagtctgctgcaggcaaaaagcggcggatttaaattgctggcggttccagaaaggttccaggatatatactgttcctccgtcgttgagcgcttcgcggcaacgtttcaggatggaaacaatttctgcttcagaaaaacaatcgaggaactggctcatccagatggcatcaaagcccttcggaaagggtacttcctcgtggaggatgttggcaatatgaaaatgcacgcggttttccacgccggcatctttcattttctgctgtgccagtcctgcctgacccggcaaatcaaagatggttacttccacttccggatctttggccgtgcaggccagggcccacttaccggtgttaccaccgatatcgagcaaacgtttcggtttcttttcaaaaacaatatccagcgcctgcggagtggcaaggtctgaatagtaatggtcgaagtcgaaccagcttttacctacttcaggtggcagcagcgacaggccgggataaatagtatcccagggaccgagttcgcgcaggccggcgggctttccttctctcaggctttcctgcaggtgattcatgcctttgtagcagatatcctgtgaaaagtccatattgatgcgggtaagctgatcatgtaaaataaagtaaccggttttggtgagggtataccgtttatcgttcacgatcaccagctccatacctaaacctgcttccagcaacactcttacggcataacgcgacattttggtttgctccattatttcctcaatggtaataccggcagagcggctgttgctcactgccgttaaaatgcccatatcacgtaatgcccgggtagcctgaaaagcaacgggggcaaatgccagacgcaatgccgcttcttttgcttcgagtgctgtttttgtttctttattaaacacgacaataactttgtttagctgttaagattaaaaaccatcgctgcattgcatccaccgaaacctgatactgttttcaggaagtggcgggatgttttttgcagcagggtattatgaacattcaccggcatacttacaccgggtatttcaaatccttttgttggcaataccacaccggctttcatggcctgcatgctgatgattgcttcaatgagcccggcggcgcccagcgtatgaccgtagtagcccttcaggctgttcactggtactgctgccaggcctgcgtggtgcagcgccttcgcctccatttcatcgttgtacagcgtggcagtgccatgcgccgatacaaaaccgatgtcggcagcggttagtccgctgccatttaccgcgagctgcattactgccgccagttcttcgccggtacgggaaggaccggaaatatgattggcgtcgttgctgatagcgcctgcacccaatgaaaagagcgcattccctttctccctgctgaggattacggtggccgcgccttctccgagtgtaacacctgttctgttggcatcgaatggtttacagggaacggcgcttaccgcctggaacgactgaaaccccgataacacaaagcgggtgagcacatctgcgccggccaccacaatatggtcataacgccccgattcaatgagccgtttgccggttaaaatggctaccagtccggaaatacaggcactgctaatcaccagcggttcattagcggcgttaaaatgggccgctattttctttgcggtggtgtacagctgcatgttggccagcggcggtacggcgccttcgggttgctgctccagtaattcaatatttccttttgtagtggaaacaatgaagccggtacgtgtatccgtaagcgtaacagcagtttgctgcagggccgattgtatggaggcaaccagcagccgctcaaaccgcgtatatccttttacgttagtgtttgccgtaaaggcatccagttgcgcaggcgttgtgatggcgctataaaacggagcagcggcataggcagcattgttgtgctgcgctatgccactgttgccagataacacctggtcaaaattttcccgggtagtactgccaagaggccccacaatattatctgctactacatacacctgttgcatagtaccctttggttataccagtccgtgcttctttttccattcactgaaaaaaggaggagcaatcaattgcagggaagaagtttccttgtccaggaatacctgtacggaagaaccctttgctactatttcccctgtggcgggattggtaaggatgtattcaaattttatttttgctgccaggtcgtccacataccttgtttctactattaccctgtcgccgtagcgcaaagagcgtttgtaatcacattgtacatttactaccggcacggtgaatccttcttcaaaaatatccaggtatctgagcccgtatttttctccgaaagcttccctgccatcttcaaaataccgcacataatgcccgtgccatactattcccagcggatctgcttcattaaatcgtatcagtatgttggtgcattcagtgagtatcataatttatcctttcttctttggtttctttgttgcgggtgttgtaccggcagctttagtttccttctttgctgctggcgcctgcactaccggctttggttcttccggatctctggcgtcagcatatttggttttcagtttgctgtaatcatcattgatctcttccaacgcgcttttaatggtagccagccagtagttgcgccatgcgaagctccatttctggcctttacccacataacgttctgtgagcagtacatttttccggtccatatctactatggccagccacatagacgcacttttgctggttttgctcataccttccattaccagcattacgccaattccgtgttttccggaaaaatcatacgatttcactactttggtgatgtcttccggtttaagacgttcaaagtcggaagattcgtcggatttcagcgcatctttattgatggcttcattgcgtttgttcaccaaaccaatactggtattgtatttatcgcggtgaaatgcgcctggtacatcgtacttcttttgttcgttcacaattacctggttcagggcagtaaactcgtggtctacgatcgcatctgttttggcagcggcgtcacctatcagtttagcctgtgtaaaatccacgcccagccaggtaaagctcgaatctttgttgtccaggaagttcttcagtgtctgagcatttgctgtcatagccatcatgctcaacatcagcaacggaagtgcaattaattttctgcagttcatgtgtgattaaatttggggattgatgaatattttcatttcacattgtgccatcaggcggccgtcaaacattactttgccggttaccatagtggcgttaaacacttcaccgccgatttcggtggtcgtttctatcatttgtcctgccggcggcagctccagtatttccaggtctttcaccgcgccaataaatcccaggggaacgggtgtattttgttgtttggcgatatagccgatgcgggcagcggcggtttgtgcaatattctccatcaggccgggcgccgtaagcaccccattctccacaaaaatattatcaggtgcgatatgaagaccggtgcgggtgatagggccatctactgccagaataccactgatcattacaatgggggtacgctggggaatataggcggtgatatcgtctgaatgaataaacatctgcacaagttattattaaatatgaaacacgaaataaatagaattatacgaaattatgaacagtaaaaacacgcattattcccaaaaatcgtaataattgaaccattgcaccgggtaacggtatactttttcttccacatgatgcacaaaatcctgcagggcggtttctactccctggttacgccggccgtggtactgacggggctcggtcgcaaaaaaatgatagtgggcagacgattccttaaaggcgaataccacggaaaccggcacccggaaggtggcggctaacaggaaaggacccagcgggaaacgggcgtcctgtcctaaaaaagggactgttacagttttattaccgggcagaaacctgtcggcatgcatacacaccagttctttattactcaatgcttcattgatagcataaatgtgcgacaggtcgtctttgatcacgataacattcatattccggtcgcccgtaataccagacaggtaatctttgatccgctggtgttcgccatcgaacatcacgatattaatacgggtttgcaggcgcttaaacaaatgacctgccacttcccagttacccacatgtgcgctcagcaggataccgcctttgccaccggcaatcatttcacgcaaatgatgttctccctcaaactcaaaggtgaatttattggacatatctgccattaccaccaccttatcgatcagtgtttgaccaaatacgtaataattccggtataaactgagcaatgcgcgcgccctgctataaccaatttttttacggagataatgatagacaggttttgaggaactccaggaaaatgcaaaaaaatagaaggctacaaatctcagcaacatatacgcaggcaccacccctccatgcttcaacaggaaaacaaaacaactatatccgaacttactccctttagattttccttgccaggagggcattataccagttctttttgttgtacacgagtggctacataattgtagaaatcctggaaagtaacaatagcctggaattcttcgggatttactttaaatccgaagttatcttctattactaccaccatatcgatataatccaaactatccagatccagtgtggatttcatgtttgcttccggcgtgatggccgcggggtttgcttcaaactcctctaccagaaacttattcgtaacagttattatctctctaatgtccataaagtgtgaaatcagatataggtcggtttaaaaattgtgtttacgtagtctattggtcagctaatcctattccgagcgcccaaagttaaggatatttattttccattccacccccttactaccagggacgaatttgttcctccaaagccaaaagaattcgacaaaaatatattaaaatttttattaattgtactggttacaatatttagcctcgcggcatcctcatcggggttatccaggttgatattgggggcaataaagccgtgctgcatcatcagcatggaatacacaatttcactggcgcccgccatccagcattcatggccggtcatggacttagtagagcttacgtacgggcgcgaaccgccaaatacttcatgaatcgccttggcttcgctggcatcgccggcggcggtagatgtagcgtgcgcgttgatatattctatatctcccggctgtaaccctgcatcctgcagggctatctgcagggatcttacaggtccgtctacagtaggattggaaatatgcgcgccattggaggaaaaaccatatcccagcacttcacctaaaatagtggcgcccctgcgctgcgcagattcaaggctttccaggatcacggtggcagcaccaccactgggtaccagtccatcccggtcgcggtcaaatggccgggaagccctggtaggatcgctttccctcaccgaaaaagcggcaatggcatcaaaattacccatggcatacacattcacttcctgggccccgccgcagatcacagcgtcctgcataccgttgcggataaacatatacccaagcccgatggcatgtgaaccactcgcgcaagctgcacttacagtgaaattcacgcccctgagcttaaaaatagtagccaggttcatatttaccgtggagttcatggtctggaaaacagatcctgaacccaccagcatcgtatcttttttagcccgcattatgtcattggcttctaccaccggttttgcggagctgtcgttaccatataaaagtcctataggtgtggagtcgatatattcaggtgtcatgcctgcctgtgcaagggcttcccgggtggccatataggcaaattccgcctgttcaggcatcataagcctggcccggcgatccagcaatcctttgagttcaggtctttctatatacccggttaaaccggaacggtaaccaaatgtctttctttcaggatccagtacaataccggatttgccctgatacaatgaatctttcacttcctgcatgtcctttccgatgcaggaataaattcccatcccagtgatcactactctgttcatagctcttagcttttagcggttagcctatagcccagtaatattgacgttattaagtgtgcagccccccattgatgttcaaaatttctccggtaatataacctgccgacctggaagccaggaaggccactgcatctgccacctcttcggctgtgccaaaacggttcatgggaacctgcgctgccagctccttttcattcagttcagccgtcatatctgttttaataaaacccggcgcaacggcgttcaccgttacccctcttttggctacttcctgtgccagcgcctttgtagcgcctattacccctgctttggcggcagaataattggtttgtccgggtaaacctttaataccggacagcgataccatattgatgatacgcccgtaacgtttcagcaacatgccattcagcacctgcttggttacgttaaaaaatccattcaaactgatattgagtacattactccattgcgcctcattcatccagaacatcagggaatcttcccggatacctgcattattcaccagcacttctatctgttgatctttattattttccacccagcctcccaatacctgttgcacttccgcggcatcgcctacgttaaatggtatcagttcaccggtactgccttttgccttcactgcttccagcgtttccagcgctgctgcctcatttcccttgtagttgatcagcacatgataacctgcttcggccatcttaatacatactgcccttcctattccccttgaccctcctgttactaatgcacatttcatgaattacaaattacgaatgacgaatgacggctaaccacaattatctgatcagaactggatcggcatattctttaccaggtaagctttaatttgctgaagatctttatagcgcgggctgtcctcaataaatttagggaaaattgctctcacttcctggtatactttgtgtgaaaatcccgccaaacggtcctggcaattcagataatccaccgcctgtaacactgtcattacctgtatagccaatacctggaaagtattttctattactttgctggtcataacagccgcattggttcccatactcacaatatcctggttatcgttgttgttcggaatactgtgtacgtacatcgggaacgacaatgtctggttttccgccacggtggaggttgccgtaaattgcaccccctgcattccaaaattaaagccaagtttgccgaggttcataaacggcggaaacttgtgattcagcttatcattcagcaggtagttgagttgtctttctgccagcatcgacaatttggtgatggctatcttgattttatccatttccagggagacataatcgccgtggaaatttccgccgtggaaaacgttttccaggtgatgatccactacaggattatcactcacggaattcagctcctgtaccaccagcttctctgcctgtgcaagggtatcgtaaacaggccccaggatctgcggtacgcagcgcagggaataatactcctgtactttatctttaaaaatttcttcttccagttctttatagagatgatcagggcgatggcgcaccattttgctgccagtaaggatctcccgcatttttgcggcaatctgctgctggccttcatgctttttcacggcattcagttcggccgacaggtgatcgtcgaatgcttctactatttcattgatcatggcagataataccaccgaccatcccagcagcttcttcgcttcaatgaggtttaccagcccgatacccgtcatggcggaagtgccatttataatggccagtccctccctcacgtggatgcctataggtttcaggttcagtttagcaaaaacatctgccgtaggctgatatttatcttcataccaaacctctccttccccgatcagtaccagcgccaggtgggccagttgtaccaggtcgccgctggcacctacgcctccatgctcaaacacacagggatatacgtttttgttgatcaggtcttttaaaagatgtaccacttccgggtgaataccggaatgcgcctgcataaagctgctcaaacgggcgatcatcagggctttggtatgcaacggcgacatgcagttgccggcgccggagctatggctgcggatcaggttatactgcaactggaaagtatcttcatcactgatgcggtattgggccatcggaccaaaaccagtgttgataccgtagatcagtttctttgccgaaaatttctcgaggaatagaaaactagcttccacctgctgcaaagccgctgcttccaatgtcagctcttccccgcccaaaaggaccctgtacacttcttccagagacagtgccttacttcctattgcaaccattttatcttaaattaaattatttgtatatgtaaaaaagtgctcaaaattagcataaagctagatttatccaaataaataacaatcccattcaacgaattacgggtaattacgcatgcggtttttacttatcagggaagggagcaagcctattcttcttcgtttgttgttggcggtgtaaccagtactttgtcgatacgatgcgcatccatgtccactatttcaaaggtaaaatctctccaggagaacttctctcccgtttgaggaatgtgttccaggtgatgcaggataaaccctgccagcgtatcaaaatcctgctcaaattcggtcatccagtcttctttatcaaattcttccaggaaatcataaaacgggatctgggcatctaccagccaggtcccatcttcccggagcaccatttcatagtcgtcgctttcagctgtttccggcatatcgcccactatggcttccaggatatcattcaatgtaatcattcccaggaaggtaccatattcatctacgataaaagcggcgtgcaggtgcgtttccttaaatttctccaacacctggtaagcggtattattttccggcacaaacaacggcttacggataatttctgtaagcggggtcgactggcccgctaccgaatacaggtctttgatggtaattaatcccttaatactgtctatctgcccgtcgcacaccggatataccgaatgcaggctgtcgaggatcgtttgccggtaggtggccggttcatcattgatatccagccaggtaatatcattacggtaagtcatgagcgacgtgatattacggtcgcccaggtggaaaaccctttctatgatctcctgttctgtttcttcaatggcgccggaactggtaccctcattaataatggctttgatctcttcttccgtaacatggggttcaccggatttgagatttaacaattttatcagtgccgcagaagaagcggttaataaccagataaaaggaaaagtaagccaggaaagcacctgcatgggcttcgccataaacttggcgatcgcttccggtttggccagcccgatacgtttcggaaccagttctcccaataccatagaaaaataagtgatcaccactacaatgagaatagtggccaccacactgctgtaaggctgtatggccggaaaggtattgagccaggccatcacatcagttttgatgttctcgcctgaataaatacccgttaagatgccgatcagcgtaataccgatttgcacggtagaaagaaaggtgtccggattgttggcaagctttaaagctgcctttgctttttcatcccctttattggcctggttctccaatcggatcttccgggccgagaccaacgctatctccgacatcgagaacaggccgttcaataaaataaggatgaggataatgacgacttccatatataaagcctaaaaataaaaaattattcaaatatcagggttagaaatgccagaagcaagcctacggctattgccagcactttcttcctgctgagttcatgatgttttgtaccactttcgtaaaagatagtagtggaaatgtgcagaaatgcacccaccaccagcgctaccacgtataaaaagtaatgttgtatcacttcaaagcggcttcccagccaacccgccagtactgcggccagcggcgttaccagcgcaaaaatgatcaggatccgccagagatccgcccttttcttatgggcatgcatcatcacggtaataagcgttaatgcctccgggattttatgagcagcaacgcccgccatcagtgaaggcagcgcagaatgatcattatatttaaagcccagcggcaacccttccatgaacgcatggatggaaagccccagcaaaagcggggtaaccgcaatatgatgatgatgctcctgcggcatatgggtatgaccgtgttccattccatgcgaaagctgctgcaggaatacctgcaggaaaaatcccaacacaatataaacacccgcctggtgacccagcgcctcgtacacttctggcagcaggtgcataatgatcacgccgaaaagaaaagcccccgtaaaagcgagcaggtaaatggaaaagttggcattgacgcgttttactgtcatgggaatcatcccaccagcaatggttgcagccagtattagtatcagatagttccagttcatgatgcgagttcagactccagtcttatgcggcgttgaaaaaaactgccgctcagcagtccgattaaaatacccagtaccgcacctcctgccacatcgagcggatagtgcacccctacgtatacctgagcataggcaatagcagccgcccatgcaaagaataaccaggcgtaccggtgaaatgcctgttttaaagttatgaaacaaaatgtagccagtgcaaaatgattggcggcatgattagaagtaaagcttccgctcataggacaatacaccaccaatacccgggcgtagtgcgacaccagcggatcacggcagggccgcacccttccgatcgcgcttttcaggtacaagctgctctgatctgccacgccaaagcacagcaggaaaaataatatccagaaaaggcctttccagccatagttaatagttacaaacagccccaggaacaggtacagcggcgcccaaacaaaaggctcccttaaaaaaggcagcaccacatccaggaacccgttataccattgaccattaatatgaaagaagagccggagatccccgcggagtatcgattcaagcatggctatgattttgtggcgatgatgatcagtcgtggcgaacgttgttcatcatagctgttaaagtgatagtcgccgaatatttctgttattttgagtccctgtttggcaaacatgacctcaaactcctgcctggtgaaggcattcacgctttctgtgtaagtagcgcggcgcattttttccttatccaggatactgatttgcttcataaatttatgcgccttcagttcccggcggatatcaaataccacattgtccttttcctttacttcatcattcaccaggtgggcagctacataattactgttcaggtagtccagcaccagtttaccacccggcttcaacgcatttttgagtgtacgcaatgcgttgtcattatcgcgctgcgattcaaagtaaccaaagctggtaaagaaattaaacaccacatcgaagtagtttacccagaaaggtaagcgcatgtcatgctgaaaaaagctcaggtgattattttccagctttcttgccacattaatactttcgatagaaagatcgatcccggttacataataacctttatctgccaggtatttggcgtgccgtccccttccacaggctacatccagcatttccgcatccggcgccggttgcagataggtgagtaacttatcaataaatgccgcggcttccctgtcatcccggttgttgtacaacaggtgataataaggagaattaaaccaatctttaaaccatagtttatctacttccatattttgtgcagctataggcagaaactaacagctattttttattattaaacatcaaatatcgggtgctttcgtaaaagccacgtgttaaattatcgaggcttttcgccgtatccggttgctgggcacggatattcttcaacgggtcgcccttcagatcatacagagcggcagcatccgtaaccaggttgatttcgtacaggtaacgatcgcccaatgtagcgtaaaaaggcatctgattacgcaggtaggtcatgaacacatatttatcgtttacccgggtgctgtcaaacaggtctacgcccaatgtataatttttatatggcattcccaccagttttgccacggtaggatacacatccagtaagcttcccggcgtattaacctgttgcggcgccaggtgcttcggactgtacataaatgcggttacatgcacgccgccggtggataactcatactccggcaacggcataaaactatatggattgagcacacagttatgatcaccgaaaaatacaaaaatggtgttatcaagatagccatctttgcgcgccatatcaataaggtgccccacgttataatcttcatacctcaacgcattgaactgatccaccgacacaaagcccgattgtttaaactttttcatatcgaggtctttctccgtcagcttcttaaaatcgccggagccgctggtggtggtatacggcgggtggttatctgccagctggaggaacgctacaaaaggcttcttcttatcattatcttctttaaaaataccactggcctccgtgatgaggtcgtaatcggaaataccccacacatcggctttcccggatttgtacatgccctcttcgtagatgcggataccttccacgttattggtaaataccgcgcggatattggcccagttggtatttccgccaagcaggtacagtttgtcgtatcctttgaactggtccatcacaatacgctgatccagcattttaggatgacggctcgctgtttttaccgcggtaatgtccggtaaaccggtgtgcacaccaaatactgttttggcggtgctgatagccggcacataaaaattcttaaacaggataccgctgtctgccaggcgctgcatatgaggcgtggcctgcatcggatttccgtacatactggttaccgctgcaccagtggattccagcatcaccaataccacattgagcctgggcttgctgctatcgccggcaacggtacgaacataattgaggttattaacatccgtggaatccactttcaggtaggaagccaggtaagggtaatattttttggtggcttccaggttgtaagtatctccttttacggagaagttggaagcgaaatacaggatgggattgagtcccaggctggttacgccgttatcgcgggtaaacatggcctggctccagcgcagcgggaaataagcgatattcccatagatgccggcggcaaacagcagcaccattcctataacgtagccggtaaagggccagttacgcaggtaagtaaccggctgggcggcaaatcttttccaggtagccttctgcaaacggtatacaaggaacatgaacactataatgcccagggcgccccgcactacggggtaactttgccataccatcctggcattgtcggcccgctccccctttgccaggaacctcagtacagaagggtcgagacgttgtccgaggtagtcgtaatgaccgaggtcaagaatataaagaagggtaagtaacaggtaaataaggaaaaaatagataaaactggtattacgtatagccctggaggtaaaaaatttattccgggtaatcagcgttaataacaagatggggatcatgaggtaaagtgccagccggagatcaaatcttagtcccaggttccaggctttgagtatcgctgcatgctctgtaatggttgttttaaagaaaaacaggtaaaatatagccctgaacatcaccattaacaggaagaggtaaagcgtttgaacaaacacataacgaatataccggggtatattcttccacgagtattgcatgtaacgtatagctgttttttgaaaagcgtagctgcaaatatagtgaaaagtgatggcggaaaattgaaaaacaggaatgacagcagcgtattcgtggtcatcttttcataattaggatttctggaatggatttttttatatttgccttcctttaaaattgaatcttgtggcactgatcaaatcgatatccggcatacgcggaaccataggcggtaagcccggcgagggactttctccattagatgtggtgaaatttaccgctgcctacggcacctggctgagccggcaaacagacaaccgtaaggtggtaataggccgtgatggccgtatttccggcgaaatggtaaaaaacctggtagtatccaccctcaacgggctggggattgatgtgatagacctcggtttatccaccacccctaccgtggaactggcggttacaatggaaaatgccgcaggcggtattattctcactgccagccataaccccagagaatggaacgccctgaagctgctgaacagcaaaggcgagttcatttccggtgaagatggtgcacagttgctggaaatagccgaacaggaagactttaatttcgcagatgtaaataagctcggctcctacaccgtcgacgattcctatctgcagaaacatatcgacctgatcgtgaactacccattggtggatgtgcctgccattaaagcacgtaacttcaaaattgtggtggatgcggtaaattctaccggcgctatctttgttccacctttgctgaaagcattgggtgtggaggaagtagaagtgctgtttgcggaagtaaacggcaaattcagccacaatccggaaccgctggcagaaaacctgaccgctctttccaatgaggtaaataaatccaatgccgacctcggtattgccgttgatccggatgtagaccgcttgtgctttgtttgtgaagatggaagcatgttcggcgaagaatacacgctggtagcagtagccgattacgtgttaagcaaaagaaaaggtaacaccgtttccaatatgtcttccacacaggcgttgaaagacgtcaccctcaagcatggtggagaatacaccccgtctgcagtaggtgaagtgaatgtggtaaagaaaatgaaagacaccaacgcggtgatcggcggagaaggcaatggcggcatcattgtgcctgacctgcactatggccgtgatgccctgatcggtatcgggcttttcctgagccacctggcgcacagcaaaaaaagcatcaaagccttacgcaacagctatcccgactatttcatctccaaaaataaaatagagctggataaaggcgtggatgtaaaaactatcttcgaaaaaatcaaggttaagtataaaaaccagcctttaaataccgaagacggattgaaaatagagttcgacaaagactgggtacacttgcgcacttccaatacagaacccatcatccgtatatacgccgaaagccagaatgaaactacggcagacaatatcgccaaaaggatcatgcaggacattaaagaatttatgcactagatcgccttcggcgatgcggattttgtctttctcgctgattacgctgattttactgattacctggatttttacttttggattttttttgattttttagattttcttaaaataataattaagggagataagagcgaatatccgcttctatctcccttaatcctttataaatccaaaagtaaaaatccaggtaatcagtaaaatcagcgtaatcctgagccaagacaaaatccgcttacatcaattctttcagtcgctccactaccttgtccacttcttctttggtgttatttttacagaaggagaagcgcaccgcaatttgattaggattgctgttgatggcgcgaataacgtgagatcccgcattggcgccggatgtacacgcactgccgccggaagcgcagatgccgttgatatccatattaaacaggatcatctctgttttctcagatttgggaaaagccacattcaatacagtatacaggctacggccatacaggtcgccgttgaaagctacttcaggaatatgcttttgcagttgttctgccatgtacatgcgcaggccattgatatgtgcgctgtgttcttcatggtgtatggtggccagttccagggctttggcaaaaccgatgatgccatacaggttttcggtgccggcgcgcatgttacgttcctggctgcctccctggatgaaaggtgttatcttaacattttcattgatgtacaggattccaactcccttggggccgtggaacttatgcccggcgccggtgatgaagtgtacaggcgtattacgcaggtcaaaggggtagtgacctacggtttgcacggtgtctgaatgaaaaatggcgtcaaactctttgcagaggttgcccacggcatgaatatccagcaggttaccgatttcgttattggcgtgcatgagggataccaggcaacgctcctgagcattctgcagcagttcacgcaggtggtccatatcaatatggccggtaggcagcacattcacaaaggagagggctatgccgtcgtggtgatgcaggtattctacggtgtgcagcgtagcatggtgctcgattggcgaagaaatgatgtgcttgcagccaagatcctttactgccgcgttgatggccgtattgctgctttcggtgccgccggaggtaaagaaaatttctcccggatgtgcattgagtgttttggcgactgatttacgcgcgttttcgatacccagtcttgattcccgtccgtaagaatagatagaggaaggattaccgaacttttccgtcataaatggcagcattgcttccaataccgctggatccagcgatgtggtagctgcattgtcgaagtatattctttccaatgtttggtggtttttgataaaagaataataattaatggtggttggtggtcttaaaaggaagcgaagttccgaaaattttgggatttttgattttggttttttatgaacggaaatttaaaaggaaacagcccgcccaagctgttggagcgcgttgtttccttttaacccacatctcccgaagggaaaatatattatgaatttctgttaatcacgtcatagaaccggtcgcggtacccatctgaaatggggatcgactggttggcgatcatcacggtattcttctccacgcagttgattttattcagggaaacgaggtatgaccggtgtacccggatgaatttatcggccggcaaacgggtttcaaatgatttcaggctgcgcagcgtgagtaccggcaggttttgtgtataaatcttcgtatagtctttcagtgcttcaatgaaaagaatgtcttccagattgatcttgatgatcttgtattctgtttttatgaagatgtagtcatttacccatgcggcgtccatcgggatggcattattgccggcgcttacatttttctgctgggtggcagaccatgtttcgctggctttggcggccgccttcaggaagcgttcaaaaggaacgggtttcagcaggtaatctaccacatccaggttaaagccatccagggcgtactctccgtaggcagtggtaaacaccaccattggcgggtatttgagggacttcaggaactggatacccgtaatatcaggcattttgatatcaaggaataccaggtctaccggttcatcctggatgaagcgtaacgcggtggccgcgttttcgaatttacctgccagggtcagaaaaggaaccttacggatgtagtcttccatgatttccagcgccagcggctcgtcatccactgcaatacactttatcattttttcaacgcaattttaagatcaacaataaattggttctcggtttccgtgatatcaatctcatgttcatgctcatagagcaatgccaatcgttttaatacgttgtccaggccaacgccccccctttcggctacccgttctttaaagtgactgttcttaaccgttaatctgatcatattttcagttgtagcaatatctatgtctataaaggaatcttccgtgtaactgatcccgtgtttaaacgcattttccacaaagggcaccagcagcataggctctatctctacgccatctgcatttccgtttaactggtaggtgatctctatgtcctttggtaaccgcaaacgttgtatttcaatgtaatcatggaggtatttcagttcgtgcgacagcaataccctggcttcattggactcatagatcatatagcgcataatggttgacagcttcaggatggcgtgttctgtttgcgccgattgtttatgcgccagcgagtaaatagtatttagacagttaaaaaggaagtgaggattaatctgcgactttaaaaattttaattccgcatttaatttctccactttcagctcttcccgttgtttttcacttttaaaccattcgagggcaatctttataaatccgctcataaacaacatgagcaaggcaaaaaatccggatctccgcagcacttccggaaaaaacaggtactccaggatagttggcgcatccggctccattggcggcattccgggcggcaagggagtagcggctacactggtaacggcaacaccggcggtatcgttaggcgtgtctctcgtcacagttgcctgctcaacagggatcgcctctgcacccgccattctttccctgatcatcatacgacgacgttgaaacggcggaaagtcgtcggatgttacttctgaattgttaaattttttatccaggcgaatagccatcatcggatgcgccctgtgcgcataattccggaagaaataaaaatttaagaccgcctgttgcgccgtaataaaaacgatcagcaaaacgatcgtgctgagataaatagcaatctttttcccgttaaaaaaacgggggatcaacacataaatattgagatagaatataccgattaaaaacaggttgtcaataagttccttaataaagaaacctgtatgcagaatctggatgcgataaatgaaaaatggaaaaaacagaaagcacgcccagccaaggatgtgcagtgaaatgaggaagggacgacttttgataatccgtttaaaatttagcatcacattatttgatgcgataaacttacaccagatagggttaggcttgtgttaaaatttgttaatccgatataagggtttgttaaatttaataaagaaattaaaaacagcttaaaaacgcggaaattgtcttggctcaggattatgcggaggttgtctttctcaggattacactgattatactgattagtttgatttttacttttgggattttataaaggattcggggagatagaagcggatagattcgcacatatctccccaaatcctttaaaatccaaagtgatcaaatccctgaatcagtataatcagcgtaatcctgagaaagacaacctccgcgtaatcctgagccaagacaaaatccgcgcgcgttattgcgcttccgggataccgatggctattaattcctgccgggataccgatggtattttgttctgtgtcagcttcgctgccacggcctgtccaacgcgcagggcgtgctcctttgaactgaaaacacggttgcccggaacgcctggaatgatatcctggtagatgtaggtatgtccgtctacgtttaccttatatccccatccgttgtgtatttcaaagggcaccaccgctaccggaagcatatcgctgccagcgtcgtgtggtcgccggtaagatctccccaccacaaaagccagtatgatcacggctataccggttacgataatgatattacgcttagtcatttttattgtactctgcactaggattaaattcccataagtcatccagcgacaggctggagctggcgcccaaacctacaaagccacggtcttttataccaaagcctactgcacccgaccgggcagcaccttcaaaagcagttttctgcacccaacggtcggtacccggagtgtattcccacactgcggcggaatagccacccttaataccggaaacgatgtagcctttgccctgcatagaaaacgcggcggcagaactgcctgcaaagttatagtcatcatcaaagctatcgtcgcttacattggaaatctggttcagcgtcgtccacgtagttccgtcgaatgaatagaagtcggttacattagcagcattggcggtacccatacaaacataggctttgttgccgatcacaaacgccgaagcatctgttctcttgccgctgttcatgctttctacctgcgtccatgcattggtacccggatcatattgccagttatcctttaaccagttgccatcataaccggtagtaataaagcctttatcgttcagtgcaaaagccaccgcgccataacgggcagtacccttaaaaggagctttcgctgtccagctgttggcagctggatcgtattcgtaaaaatcattcagtttatttaatccgtcgtaaccggtacctacataccctttaccggccatagccatgccaacggctccgttacgggccacaccggtaaacggcgctacctgtgtccactggttctgatccacgttatatacccagaaatcctgtaacctttcagttccatcatagccggtacctacataagctctattatcaattacaaaggaagctgccgagctcctggcaacgccttcatactgagagcgcttaacccagttccctaccagcgtagtagtatctgaacctttcgaacaggctgccagggaagccatcaataataaactataaccttttaaatatcgcattagcatgttctttttactagcgccaaaattatccgcaggagcattccggcaaacaggaaatagctgttcccctgtttttagcggacggataccgttatttcatctaccagtgggtttctttcgcctgaaatgcctgttgctgcgctattggcggcataaaggatatatttcgttattcatcgatgaattttggccgttggcatattaaaggaactgaaagtatcgatcctgtctaaaattgcgcaccatgaacaataccatgtatcacttatttttcaggcgtacggcagggagtttacgcaggtatctcccggcgcttttactggtggctgctgtttcttcctgccaaaaaacaggctttacctataataatgttgtagataataatcagaatacagattacatcctgaccgacacacttaccgtaaatgtgaaaaccgtgcagcaggattctgtacccacctcgggagtagaagtgctgttggccggtaaaaataccgatccgctttttggcaccgccaccatacaatcctttttccagatagcacaacctgccgccgtggaaattccggcgaatggctccgcatacgattcaatggtgttgatgatgcgccccaacggttacatcgccggcgattccaccataccacaggaactccaggtataccgggtaacatctaccatacaaaccgcaaaaaatttctattacctgtacaacaacagcagcttctcaacagaaagtaccccaataggcagcttcaacggccttatacggcccggtaccgacaccatcgttaccgtacatatgtccgatcagctgggcagtcagctatttaccatgctggttaacaaaagtccggatatcaccgccaataatactttcctcgaattttttaaaggtctgaatgtacggggtggcccgaatagcaaagccgttagcggctttcgtgctacagaaaattatctcgtaatgcggttatactatcatgtcaacgaaattattaccaccgttaaatatgttgattttaaaatgcaggcatctaacctgcaattcaaccaggtagtagcagatcagaccggcacgccactggcgccgcttacaggcaacgttaaagaactttcctccgccagcaccggcaacagggtgttcacccggcctatcacgggatcggctacacgaatagatatcccttatatcaagaacctcgtgtacatggggcagttctttaaaataatgaaagtatatatgacgctaaaaccggtcctcggcagctacacagataaccgccttccaccgagaatggcactgtgcgaggtgaataaactgaatgatgtaacagatacccttacttatggtcaactgacagtagataaactgtatgataaaaataccaattacaccttcgacatcaccaactatgtaacaaaagaacaaactgtcagcgatgtcgactcccgcggccttttgcttacaccaagtgctaccgacagcagaacaacgctggacaggctggttaccggtgatcagaagaatacgcaaaaccagcttaaaatacagttatactacctgttgtataaataaaggacactcatgcgaataaaaatatatagcggattaatcttactcctgttgtgcacggctaccgtaaaagcgcaacgtggccttaattccatttattctgcctacggcataggcgacctggaatcgagggattacagccgcaatttcggactgggaagcaccggcatcggccgcaggcactccggttatctcaacgaactcaatcccgcttcctatagcgcactgcctccgcaaaactttatgtttgatgtgtcgctgaaagcacaacagataaattatagtggcaataatatttcacaaagcgccggggatattaactttaaacggcttgcacttggattcaaagcagccaaatggtggggcatcggcgcaggtatcacacctttcagcacgattgattacaaactggaaaaccagcaatttgtaaccggtaccggcagccccgtaaccgccactactaccggcaccggcgggttcaacagggcctatatctccaacggattccagatcagcaaaaacttctccgccggcgtatccaccgctttcttatttggcccgctgaatactacacaatacattggttctgactccttacaaacacagcacaataaatatgggttcaaacctaactttacagccggcgcacaatatgcaggaaaaataggtaaagactggcaactgggactgggcgccacttatcgcttcgaaacaacaatgaaactccaggaaaaactgaatatcgttaaccaggacggcacgtcgttgtatcagaaagaccaggacccttctttctttaccctgcccgcagaatacggcgctggtctgagccttaccaacggtaccattacctgggtggcagactaccgccattcactgtggaactcactgaatgaaaaaggcgctacctaccgctaccaggacggagaacggtattctaccggtgtagaatatacgattaaacggcattactataaccaaagctttgaaggagccgtgttacaggccggatttgcttataataaaaccccgctggtaataggcagcacgcaaatcaccgatatctcgggcacactaggcgtatcactccccaataaaaacgggcagctcagatactacgtcggcctggaagccgggcaacgcggaaaagaaggcacggcactggtcaaggaaacttatgtcaacgccgtattcaacttcagcttgcgcgatatctggttcttcaaacgcctggcacaatagcgcggatgttgtcttggctcaggattacgctgattatactgattagtttgatttttacttttggattttttttggatttttagattaataattaagggagataaaagcgaatatccgcttctatctcccttaatcctttataaaatcaaaaaagtaaatcaaactaatcagtataatcagcgtaatcctgagccaagacaaatttcgcatcgccgaaggcgatctccgctatgatcccgccgacagcagctcgcggaaccagtagccggagtctttaatcatgcgctgttgtgtatcaaaatttacgtacaccaggccaaagcgtgcacggtagccttcggcccactcgaagttgtcggtgagggtccaggcgaaataaccgtctaccggaatcccttctttctttgctttcagtacggcagcaagatattcctggaagtagctgatgcgggctgtatccgcgatacggccatcggcgccggggatatccgggaaagcggctccgccttcagtaacgatcagttttttcactcctttgtaaccggcaaactgccgtagaatttcgtataacccattgccgttaatctcccatcccagtcctgttagcggtacattcctgtacctggccttcacctcagagatccttaccaccggcatgaaagtgttgtactttactaccagcggaaaataattctgcacaccaataaaatcaaaatcaaaggccagccggtcccagtcgcgccacagggcgtagcggcgttcaatacgtttaagcaacggaaaatctgctaccgggtatcccatccccagcgagggttccaggaacaagcggttaaacagtgcatctgcgcggcgcgcggccagcaggtcggcatcgctgttgctgttgggaataatctgtgagcacgacaatgccgtgccgatattggcgccggcaacttcttcccggagtacccgtccgccttccgcctgcgccatcaccgcatggtgcaccgccggcaaaaaccaggaaaggccaaatttgccaggtgcatgcacacccagcatataaccaagggcggtaaacccgaaaggctcattcatcacaatccagttcttcactttattcccgaattcacgggcacatacccgtacaaattcttcaaaagcaaaaacaacaccccggtggctccagccacctttatgctccagcgcctggggcaaatcccagtgatacagcgttacataaggctccagccccaactccaggcacgcgtctattacccggtggtaaaagtcgatcccagcaggatttaccgcaccggtgcctttaggcatgatgcgtgaccacgacaatgaaaaacggaaaacggaaaagcccagcagctttgccagcaggatatcctgcgtgtagcggttataaaaatcggtagcggtttgtgcgtggcttttatctttgatcttgcccttacggccggtgaaagtatcccaaatagaaggccctttgccatcggtatcgaaggcaccttcattctgaaatgcggaaatagtaaccccccagagaaaatcgtccccgaaatcctttcgggtaaagggtacggcagttgtttgcatatgcaatacctgtaaccggggccaagtgcttcccgaaacagcatgcagtttacaacagttttcggggaaatttaattatataattgttaacgggtaattacggtgtgaaagtccgccgtgaaaatttcgcaaaagctgttttaatatcctatttttggaagcctactaaattgatagacaaatatatgtttaagataaacctattgcttggccttgcattcctgagcgcctgcgcgggcaatccgggaaagcaggatgcagctgccggcggaaaggactcactgaataaaatggtactgataccggcgggaacttttacgatgggagccgacgattcaaccggtatggccgatgaatatcccaaacacacggtggatatcgccgggttctggatggatgaacatgaagtaaccaacgccgaatttgcacagtttgtgaccgcaacaggatatgtaactactgccgaaaagcccatcagcaaagaagaattgctggccagcctgccgcccggaacaccggaacccgacagcgcggcattggcaggaatgatggcgccgggagccctggtattcacgcctcctgatcatgctgttccttttaatgatatttcccaatggtggtcgtttgtaccgggcgccacctggcagcatcccgaagggccggccagtaatatcgataagcgggaaaatgagccggtaacgcaggtgtcgtggctggatgcacaggcttatgccaaatgggccgggaaacgccttcctacggaagccgaatgggaatacgcggcacgtggcggtctctcaggcaaaatatatccctggggaaccgaagccttaaccagcggccaacctaaagccaacacctggaacggtaacttcccctaccataataccaaaacagatggttactacgggcttgcgccagtgaaatcgtatagccctaatggttaccagttatatgacatgtccggcaatgtgtgggaatggtgtgaagactggtacgacgccaattattatatccagggagaaaaaggggtgaagaatccggccggaccggcagcaggatttgatccggacgatccgggccaggccaagcgcgtcatccggggaggctcctttatgtgcagtgatgaatattgccggggataccgggtatctgcacgtatgaaaagcacgcctgaatcgggcctggctaatcttggcttccgttgcgtgcgttcacttgtccagaaatgacggcaattcacggtagtcgccgttataacgtttgccgtttacataaaaagtgggcgtaccattcacgccgctgcgaacaccgctttcaaagtcggcttccaccctgctcagtagtttgggggattccatgtcttccctgaattgtctcagatccaatccgagactggtggccagctgcaatagcaacccttcagtcaaatcagactgacgggcgtagatcgcatcatgcatttcccagaattggttttgccggctggcggcctccgctgcgagcgcagcatccatcgcatattcatgggcttcggacaaaggaaagttacggaacacaaaacggagccgggtatccagttgttcccgcaactgttttataataaaaaaagcttcgccgcagaaagtgcattgaaaatctccgtattctaccagttcaatagctgcatcaggtttgcctagcacatgatccatagcatttaccggcgggatgagggtgggcatatcttatttatttttgaggttttccaatgcttcgaggataccatctgcaccggggttttcatttaccggcgataaatagctccactggataatgccgttggcgtctattacaaacaaggcacgtttactcaccccaaacttttcttcatatacaccgtaagcaatggaaacggcgcctttcggctcaaaatcggaaagcaggtcgaagtggatctggcgggcgctggcaaatgcctgatgacaccaggcgccatctacagaaatacccagcaacaccgcattgtacttttcgaaatagggcagtatttcgttatacagcgccatctgatcgctgcatacaggactccagtcggccgggtaaaaagccaggataacatttttcccgcgaaggtcttttaaatgcaccttcttttcaggagtggcatccagcgtgaaatcgggagcagtttcgcctttttgtaacataagcaatgagttcttaaccctatataaacagctattgcggaataatgttgtgcagaaacaaaaatgccacggtggcggaccgtggctttttgtgacagattattgccgctactattttattttaaccgtatccgactccatggttatcacaccagatacaatcagttcatccggattgtctttggtgctgatcatcactatcccgtttggctgtggcgtacctttgtaaagggtagccttaccgcctttgtacacattaacagatttgatattggaaggaggtattgcccccacttcttctttagtcatttttttaccatccaccaataacagtgcaccttccgaggcactaaaggaattacctgttactacaacgcccgatgctttaatgggtgtcatagtcgctgcagatttcttcagcgtaacacgtataaccccattttttcccctgtcgccatacaaagcagttgcacttttgtcttttaatacctcaatggcttcaatcctgttagggtcaataccttcaattgattccgcaactttaccatcaattatatagagcggtgcattggcggggtctattccccgaagagtcatactaccgttcagtttgacttccggcgctggtacttcttttacttttgccggtggtgtcggtttagccacctttattttaggtggcgccggcggaggtggaggaagtggtggcgccggcggagatggcggtacagtgtccttgacgataacaagggctaaaggattaacggaaggcgccttggtgtaattgagcgacaaaacggttccacctaccagcagtcctaataccaggtaacgcgccatttgataacgtgatgactttttgctgttcatcatgatgatcctgttttttagatgtgagaaattgaaattgtttgcgatggccgtcgcatatgggatcccacttactttaattaaattgtattgataggcggttttatccacaccctgcttcagcaggtacctgtctgttataaactccaggttttcacggatggctgttttcatcagccatgcgccgggattgaaccagtaaaaaatgttattaagttctcctaacaccacatcaacgctgtgccactgctgtacatgcactttttcatgacgcagtatggcgggcagctcttcaggttgatggagtaccggattgatatagatattccggaaaaaagaaaaaggattcaccggttgccgcaatacctgcaccgggatatcggctatttcactgcgttgcgaggtacggtgtatcttccataaggataacaactggaaacaaaaacgtatagccattacagatacccctgtccagaaaatatacaccagtagtgtccagatcgtgaacaccggtgcaggcgcccgccagccggccagatccggaacataggtcatgacgttgcccgccagcacttcatgcctgtttacaaacgcatcaatgggaattaagggaaacagggacgaaaagacaataccggtgagcaggaacaacctgttcccggtataaaaggtaagcctgcgcaaaccaaagcggtaagcgagaaaaaataaggtgagtgcgatatttgcctttaagaggtatattaaaatagcaggtaccatggctgtaattttattatttacctttttctatcatgttgataatttcctttaactcatccgggctgatctttttctctttcgcgaaaaaagacaccagctctttgtaggagttttcgaaatagtcttttacaaagccattcataaacttctgtttataagccgcttcttccataaccggcgtatattcatatacgttacccactttccggctttccacaaatccctttttctccaggttcttaatcgtagaagccaatgtagtataaggcggcgccggagcgctgtgcgcttccaggaagtctttcacaaaacctttccctactttccagatagccagcatggccgtttcttcttgctgggtaagtttttccatacaaatgaatattttgaattacgattctttcgtaaatctacgaatgtttcgtagataaacaaatatttttttagataaatgatcttagcaggcaaaattgtttaaaaaagaaagaggtgcaagaataaaccctgcacctcttgatatgtttctcccggagaggaaattattacttcaatatttcttccagcttggaggccagttcctcaccacgcaggtttttcgctacgatctttcctttaggatcaatcagtacattctgcgggatggcacgcacgccgtaaaggtctgctgctgcattcttccagcctttcagatcggaaacatgcgtccaggtgagcttatctgcatcaacagcagccagccatttgtcttttttgtcatccagggaaacaccgaggatttcaaagcctttggacttaaatttatcgtatgcctttaccacgttagggttttctgcacggcagggaccgcaccagctggcccagaaatcaaccaatacatatttaccacggaaagacgacaggctgatgtccttaccattggcatctgcctgggcaaattcaatagcaggctgaccaaccgccgttttacgggccgcctcaagacgcttggagaattctttaccggaaggtgaattctttgcttccttacttaatttcttgaacagcggtgtaacttcagcaggttttatatcgtaaccggctacctggtttaacaggaacatcgcaataggagaattggtatttttagaaagaaaatcgttctcaatttttttctcttctgtatctaacgaatcatatgctgcttcaagtttcttaatcccttcttcgtccttattcttcgcaagttcacggtattgtttctgcaaagctgcacctttctcatttacatctttcagcagttcattcagatttttgtaatcatcgtttgctttagagcccgtaacagtagctttgctgatagaatcagtagtgctgatagtgataacgcctttatccaggaaaaccgccagcatatcacgtcccatcgacattggcttttctgaacctttttgtaccagcatcaggctggccaaaccggcttcttccaaagttccgttaaaggtaaatttgccgtctttgatctgcgcgctgtccatgaagttctcaccgcccttgcgcatcctgagataaacagtagccggattctgttgctgggaaacagttccctgtatagtataaggttttcctgcagttgcgcctttcttatcctgggcaaacatgatccccggcactaaaagggcaacacctataatcgcttttttcattggtttttgttttacgaataacaaatttgtaaaatccgccgctctttagcaacctgattttgataagcggctattttaacaactgctccagcttcgcctccagctcttccccacggagattgcgggcgataattttcccggcaggatctaccaggaagttggtgggaatagactgaacgccatactgcaccgctacttcattgccccagcctcgcaggtcggatacctgggtccaggccagtccatcctggctgatagcccgtaaccaacgatcacggttgtcatccagcgaaacgcccaaaatggtgaagtttttatccttgaacctgttataagcctttactacattaggattctcctggcggcagggaccacaccagctcgcccagaaatcaaccaatacgtacttaccacggaaagacgataattttaccggattccctttggtatcctcctgcgaaaaatcgtcggcggccacattcaacacatttgctttcagactttttacataggcggttacgctttgtccgtacgaactttcctgcaccgacttatccagtgattcaaacaattgcctgaactcctccggttccagcctgctgcgcagctcattcatcatcaaccatatactggcaatactctttggatgtgaggtaataaactgcttaccagtgttcaccacctcccggctgaatgtctccgctttcttacgaaaggcattcttccctggctcatcctcggggttaatctgctttgcttcgttattcagctcctgcgcctgtttgatcaggggctcaaatgccttctggtactcctgcatcgccagcgtattcgcatttcccttcacggaagtagcaattggataagtagccacggaagtagtaaactgaacaggctcattccctgttacaaacaacatcgggtaatttacatcccgcaggatcaacgcatacactgctggctccttgccactttttacacggaagctgaactgctcattctttatcaccaccgaatcatccggattattatcctggtcgtcaaaaagataaatggttttgccgttgcctcccctcacaacacccgacacctgctgggcattcacacctgcgaaaaccaacaccgcagcggctaacagtaaaatctgtttcattacaaattattttaattagttagtggggtgtaatatacgaagagatttttttatggcgaggggtgccggcttcgccagcactaaattgtcttattgcatgatttagttgattatactgattaccatgatttgattttgtttatgagcaagcttataagttaattatcaacctctaataaataaaaataaaatcatggtaatcagtataatcaactaaatcatgcaataagacaatctaaaagccggcgaagccggcagctacttgtggcgctgttttaacaccgatataacatctgccagctggaaaccctttgcctgaagaaggatcaggtaatggaacaacaggtcagcggattcattgaggaacagctcatcgttattgtccttagcttcaatcaccacttctaccgcttcctctcctactttctgtgcaattttgttgatgcccttttcaaaaagactggcagtgtaagatttatcggaaggattatttttccggtcggtaatgatgttctccagggtagaaagaaagtcgttgcttacattcttttcatcccagcaggtatcagcgccggtatggcataccgggcctacaggactggctttgatgagaatcgtatcctggtcgcaatctactttaaggtcttttacgatcaggaaattgccactctcttctccttttgtccacaaacggttttttgagcggctgaaaaaagtcaccttgccatccaaaacggttttctccagcgactcccggttcatataaccaagcatcagcaccttattggtgatggcgtcctgtataatggctggtacgaggccatcgggcgacttttgaaaatctatctgcattgtttacttatttcaggtatcacttaaaatcttacgttcactcccttgttataaagaaaagttttgagcgcaggaatttctatttctttataatggaagatgctggctgcgagtgcggcatctgcctgtgcgttttcaaaaacatcggtaaaatgttccattgtaccagcgccgccggaagcgataacaggtacattcaggtgctgtgccagctgcccggtaatatccagggcaaagcctttcttggtgccatcgttgttcatggaagtgagcagtatctcaccagcaccacggcctaccgcttcttttgcccagtcaaatgcctttatatccgttttcacacggccaccattcaggtacacataccagtcgccctcctcaaagcgggtgtcaatagccagtactatacactgactcccaaattcacgggccagcctgtccaccagtgcagggtccttaaacgcagaggtattcaccgaaatcttatccgcaccggattgcagcagcacgtatacatcttccacggaagatatgcccccgcccacggtaaaaggaatattcacatgacgggcaatattcgttaccagttccgccagcgtctttcttcgttcgttcgttgccgttatatccagaaataccagctcatcagctccctgtgaagcatacaacgctcccagttcaacagggtcgccggcatcgcggatattttcaaaattgatgcctttcacggtacggccgtctttgatatccaggcatggtatgatgcgtttggtcaacatgtgctaatagtttacaggaatgtttttaatgcatccatggagatgttaccttcatagatcgctttaccgatgatagcgccactgcagccaatttcctgcaaggcagccacatcttcaatattactcacgccgccgctggccacaaagttaatatccgggaagcgttctataatctttttatacagctctacagacggtccctgtaaaagaccatccttagcgatatctgtacaaaagatattgctgacgccctgcgcgatattgctttccagaaaatcgaataccgacaactccgttgtttccagccacccacctactgcaatcttttcttcttttacatcggcgcccaggaatattttaccggctccgtattgcttcacccaactgaaaaacagttccggttgcttcaccgctacgctgcctatcgtagccaatgcagcaccgctttgaaatacaatctccagatctttatccgttttaataccgccgccaaaatctgttatcaaaccggttttaccggcaatgctctccagcactttccagtttaccactgctcctttcttggcgccgtcgaggtctaccaggtgaaggcggcgaacgccgatggcttcaaattcctttgccacttccagcggatgttcgttgtacactttctgctggttataatcgccctgggtaagccttacacatttaccatcgatgatatcaatggcaggtataacttcaaattttttagttgtcatgttttgctgatccaaaggcagttccattctcacaaaagtgattcctcccttaacaaagtaatcccctttcttcgtatagcccagcctgtcataaaatgttactgcggtatcacgggcattacaccagagcagttttattttttcttttttacagatgtccaccagatgtgccagtatcgctttgccaaagcctttcccctgtgcagccggcgctgtagccagtttgcggaactgtgcgctttcgcggcccaggaaaagggacactactgttaccagttgcccctggtcaaaaacgccgaagtgcagtccatctgcatcgtggtctacttttacggcttccagcgactcattgggatacatcacatccctgcggagttgcagcgtgtcatctgcgctgattttccggatattcatcttacaggttcaaaaagttttcaataatacgggcgcctgctatagctgatttctccgggtgaaactgcaccgcataaaaattatccttctgcaacgcagcgctatagttgatcacataattggtgatggccacggtatctgccccgagtgccgcataatagctatgcacaaagtacatataggagttctccggtacgtgttcaaacaccacgctgtgcaaaccggtgatattgttccatccgatctgcggtattttcagcaggttttccaccggcgattgaaaacgtttcacatccacatcaaatacaccgatgcatttggtatcgttttcttccgaatatttacacaacagctgcatacccaggcaaatgcccagcaccggctgtttcaggccggcaattacggcatccagttttctttctctcaggtactgcatcgccgtgctggcttctcccacaccgggaaaaatcaccttatcggccgacatgatctcttcgtgatcatccgtaacagtgccgtttacgcctaaacgctccaatgcaaactgcacagagcggatattaccggcgttgtattttatgataaccgttttcatgttattactgaattattcccgaaataaacgttttcaccgtttcgtcaatattcttactgtgctcaatggccctgataaaggcagtgccgataatagcgccattggcataagcagatgccgtatcaaaagtagctttatcttttataccaaaaccaattaaaacagggtttgtgagctgcaactgcttcagccgctcaaaataagcctgctggtctttcatatccttgtcttttcctgtggtggaagaagaagatacggcataaataaagcctttgctcagactgtctattttacggatccgtgcttcactggtttccggcgttaccaggaaaatcaggtgcaggttgtatttttcaaacactggtctgtactcattttcatattcggccattggcaggtccggcacaatgataccatccacacctacttctgcacattttgcgcaaaaggcttccacaccgtaagttaataccgggttgaaatatcccatcaggataacaggcacctgtatacggtccctgaaaccggtaagttgttcaaacagtttgtgcaggctcatgccgttctgcaacgctttagtgctgctgtcctggataacaggcccgtcggccagcggatcggagaatggcatgcccagctcaataaggtccgctccatattgctgtaatgcggtcattacaggcagggtgtcatttaactgcggaaagccagccgtacaatatatatttaaaacgttgtgccgcttaacagcaaacagttgatcaatacgattttgcataatccatttatttattcatgtgacggatataggtatccagatctttatccccgcggccggaaaggcataccaccactacatcatcagtattcaggggcaggtctttcagtttagccagggcgtgagccgattccatagcaggaataattccttccagcaggctcagttcataagccgccgccagggcttcttcatcggtagccgacaggaactgtgcgcggcccgattcatacaaatgggcgtgcataggtccgatgccgggataatcgagtcctgcggaaatggaatgtggttccacgatctgtccgtcgttggtttgcatcagcaatgttttgctggcatggataataccaatggtgcccagctgcgtagtagctgcggaaaacccgctgtgtacaccctttccgccagcttccacggctaccagttttaccttttccctgtcgaggtaatggaagtaagcgccggctgcattgctgccgccaccgatacaagccagtacataatcaggattctcgctgccggttttctccaacagctgtttttttatttcttcgctgatcaccgactggaagcgggccaccatatcaggatatggatgcggacctgcagcggtgcccaaaatataatgtgtatctaccgggttgttgatccagtcgcggatcgcttcattggtagcatctttcaaggttttactgccgctggtggccggcactacggtggctcccagcattttcatccgcgctacgttgggcgcctgtctttctatatcaatgctgcccatatacaccacgcactccatgcccatgagcgcgcatacggtagccgtggccacgccatgctgaccagcgccggtttcagcgatgatacggcgtttgcccaggcgttgcgccagcaggatctgcccgatggtattgtttactttatgtgcaccggtatgattcagatcttctcttttaagataaattttcgctttatatttttcagacaaacgtttggcaaaatataaaggggaaggccttcctacataatcccgcaacagggcttcaaagtcctgctgaaaaccgggatcgctgaggatgccgagatatttggactgtaattcctctacgttgggatacagcatctcgggaatgtacgccccgccaaatctgccataatagccattcttatccacctgatacctggagttgccagtattaatcgcaatatccatgaccgcttattttattattgatgaatgaatttgtttcacaaattgttttaccagcgcaatgtttttcacacccggactgtcctcgaatttactgttcacatctgctgcaaacaatgccggcaactgcatctcctgtatttctgttgcctggccggcactgatgcccccgctcaaaaagaagggatggtcaaacgggtaagttttcagcaaatcccagttaaactgctcgcccgttccgccataaccttttacggaagcggtatcgaagagaaagtaatcggttaccggtataaaaggcgccacttccgtttgccagttaacgttatcacctatacgaaaagctttcaccaccgggatgaaggtacggacagcagcgcaaaactccggcgtttcctcaccatgcaattgcaccaggtccagtgcataatcactcacggtgcgttggatctgttccagcggcgcgtttacaaaaacccctgcctttttgatgccggaggtttcccgtaccgatctcgcatctattttgttaccggcaaaacgcggtgacttctcgtaaaaaataaatcctgcatagtcaacgccgttatccaccagcgcctgcagatcatttatcctggtaataccgcaaactttaatacgcatcgtgttatgatttatgctgcagatcgctgagtgtttgtacaaaattttcaaaggcacgtgcgggatcttcctgcttcatgaaatgctcgcctatcaggaatccctggaatccggcggctttcagtgttacaatagcagcggggtcattgataccactttccgccactttcactttatccgccggaatcttcggcgccagttcacaggaacggttaaagtctacctggaacgtgatcaggtcgcggttattcacgcccaccaggtgggtatgtgccgttactttttccagttgcgcttcactgtgtacttccagtaatacttccagtccgaggttatgtgcaaaagcagccaggtgtgctacctgtgcggcatccaggcattctgcaatgaggagtattacatctgccccgatagcctttgcctccagtatctggtattcatctatcacaaaatctttccgcagaatcgggatctggttgaagctacgcgcctgttgcagatcgtcggaagaaccaccgaaatatttttcatcggtgagcaccgacagcccggaagcgccgtaacgggtgtatgcggtagttacctgttgaacagttacatcgccgttgatcactcctttcgaaggagagcgccgtttgaattccgcaataatgcccgttttttccggctgctgcaggaaatggcggagcgataatgtttccctcgggaaggccggcgactgctccaggtcctgcgcgctgcgctgcaatttgcgggcagctacttcgatgtgtttatgagcaacaatttctgctaaaatattcttcatgataaactatctgtactacgactgcaaagcaatcagttttttgaacgcattatgtgcattgcccgactccagggattctaccgcggcggcgaagcaatcttcatacgaattatatgttccgaggctgtacaaacccattgctgcgttggcaaaaacaacggaattctgtgcccaggtaccttcgcctttcaggatcttcataaagatctttgcggcttcttcagtagagttaccgccgtaaatatcttcctggtgaactttacgtttgcccagctgctccggggtccagtcctgttcacctttattggtaatcactttggtatctgccgtgagggatatttcatcatatccatcgaggctgtgaacaatcacaaactgcttgtccgtttgctggaacaggtagttgtataccctcgccatttccaggctgtaaacaccgatcagctgatgtttggccagcgccgggttcacaaggggaccaagcatgttaaagaacgtacggatacccagctggcggcggatgcctgccacatgtttcaatgccgggtggaacagtggtgcgtgcagaaaacagatccctgaatcctccagctctgttctcagtttggcatcgtcattcttgaatttataccctaccagctccattacattggaagcaccactgacagaagatacgccatagttgccatgcttggctacttttgcccccgcgccggctaccacaaagcacgacaaggtagaaatattaaaagtattttttgcatccccgccggtaccaacaatgtccagtacatcgtaaccgttgagattaaccggtacacagagttccagcagcgcgtcgcggaagcccagcaactcatcgatggtgatgctgcgcatcaggtataccgtcatgaaagccgccagttcgctttcgttgaacatgcctttggaaatactgatcaggatatctttggcagcttcgcggctgaaagttttatgttcaaaaaggtaattgagaatctttttcatttttggaagaattttgctgattgagtgttcgataattttaaaacgggtgtcgcgctgttattacaggcttaaccagtttcttacaatcttttctccctgcggggtaagcacactttccgggtggaactgcacaccacttacatcgtatttgttatgctgtacagccataataaaaccatcttcgtctttggcggtgatcaccagttccgcaggcagggtagactcatcaattacccaggagtgataacggccggccagtatttgtcgtggtaagccgttaaacagccgtccatcttccttaataatatttacgttggtagcaacgccatggtatacttccttcaggttggtgagagaagcgccaaatgcctgtccgatggcttgctgccccaaacacacaccaaagatggatttggtgggcgcatattctttaatcagcggcagcagtaatccagcttcttccggaataccggggccgggcgataaaataattttatcgtagttatttactttctccaatggaatttcatcattgcgtaccacggttactttaccgttgatgattttttccacgagatgaacgaggttgtatgtgaaggagtcgtagttatcgaaaacgaggatgttcatactaaattttttgtgccagcagaatggcttgttttaacgcattgagtttgttgttcacttcctccagttctgaagaagctactgattttgctaccacaccggcgccggcctggtagtacagggtattcattttactgagtatggagcggatcatgatggcatggttgaagttgccgttgaaaccaacagcgccgatacaaccgccgtagaagccacgtgcagtgggttcatactgatcaataatttccatggcacggtattttggtgcgccggacagtgtgcctgccgggaaagaagaagccagcagcgtgaacggattcagcttcggatctacctttccggttacttcgcttaccaggtgaattacgtgtgaatagaaatgcacctgtctgtaagaagctacttccacttctgtggcgtttctgctgagatcattcctggccaggtctaccagcatcacgtgttctgcgttttccttcggatcttccagcagtttattggccagcagtttatcctgttcatcatccccggtgcggcggaaagtacctgcaatgggatgaatagtagctttgccatctgtaatcacgatctgtgcttccggtgaggaacccattaatttataatcgccgtaatcgaagaagaaaagataaggagaggggttgatggagcggagggcgcggtaaacattgaattcatcgcctttgaaggattgctggaaagctctggaaagtactacctggaaaacgtctccgcggaagcagtgttgtttgccctgttctaccatctgcatatattccgcatccgtcatattgcttttctcttccccggtagtggcaaacggatacccgggggaatctttgtgccggataagcgactccagtagctcaaactcactatcgatgccgtctatctggttttcacaaagataaagttcatctttaaagtgattgatcgctattacatattgatagtagcggtaacgcatcaacgggatggtattaccggcctcttgtttctttttattgaattcaatggtttcaaagaactgtacggcatcaaaagtggtatacccgaagaggctctgcgccattggtaccgggtgtttgccggagaaagaatagttgccgagaaactgctccatttcatccagcacctgttgcttatttttcagctctttcttttctacgggcaggttgggatacttaaattcgaagtgcgacgtggaagtaacttcgatacctgcaatgggcttcacacaaataaaggaataactgttgtcactggccctgtagtcagtgctttcgaggaggatagaacccgggaatttatcgcgcagccgcagatatattcccactggcgtgaaaatgtctgccagcatctgtttggatctcgtttttacttggatggtacgcatgatgtattgggtgaagtatttgttttttttaaaatgggaagggctgaaaaagcggaaggcccgctgtgtaacagcgggccttccaaatatatttctaaacgaaacatggcactgtaacacagatcaggaattgattccgtgccaccaccaatgtttgtttgtaatgatattttgcatagcgagaacaaaaatgaaacatttttttagaaaatgcaaattttttttgtggggggcggtgccttcggcaccttttgtctttctgcaggattactggattaatcgtgattgcactgattttcccacattctgtttgattttatggtgtggagataaaagctgatttttctaatttctgttagaaaatcggtatggagataaaaaacaaaatacgcttatatcttctccaatcatttaatcttatccgcttctatctccgccaaataattaaaacaaaaggcgggaaaatcagtgcaatcacgattaatccagtaatcctgcagaaagacaaaaggcgccgaaggcgccgcccgtccgctacagtacccccttcgttgaaggcagctgcatattagccggattccgtttcaccgccattttaatagacttggcaaaggttttaaagatggcttctatcttgtgatgttcattttcgccttctgccttaatgttcaggttcgctttggcgccatctgagaaggatttgaagaaatgatagaacatctcggtaggcatctcccctattttttccctcttaaactccgcgtcccataccagccagttgcggccgccaaagtcaatacccacctgggccaggcaatcatccatcggcaggcagaaaccgtatctttcgataccgcgtttatcgcctaagcctttggcaatggcttctcccaaggcaatgcccgtatcttctatggtgtggtgctcatcaatatgcaggtcgcctttggcggtgatcttcaggtctatagcgccatggcgggcaatctggtcgagcatatgatcaaagaagcccagccctgtatgaatatccgctttaccggttccatccaggttcagttcaatattgatatctgtttcattggttttccgtacatgcgttaccgttcttaatcccagtttcaggaactcatagatccggttccagtcggtggtttcgagggcaatcacggattgcagcgcagctgcgttatcgctgatttcggcacttcccaaaccaacgccttcattgatccagatagcttttgcgcccaggttttttgccagctccacatcggtgatacgatcgccgatcacaaaagaattggccaggtcgtagctgccatcgagatatttggagagcatgcccgtgcggggtttgcgggtaggcgcattatcggcgggaaaagagcggtcaataaacacctcatcaaatttgatcccttcgttttcaaacgctttcatgatcatattctgcgcaggccagaaggtatcttccgggaaggaagcagtacctagtccgtcctggttggtaaccattgccagctcatagtccagctcagcggcgatccgcgccatattcacaaatactttgggataaaactctactttgtccaggctatcgatctggtaagttggcggcacttccctgatcagggtaccatcacggtctataaagagcactcgtttcatgcagatgcagttgtggctgttttcaggttaaaagatttcaatacttccagcagtcgcaggttttcggccggcgtgccaatggtgatacgcaggcagcccatacacagttccactttggaacggtcgcgtactacaattccctgttcaatgagataattgtagataccttttgcatcggtggttttcaccaggataaagctcgcatcgctgggataaatgtgcagtacttccggcaactggatcagtgcgccggaaagcaggtcgcgttctatcactatttcgcggatccattcatttacctggcttacattttccaatgcctggagcgccagctcattggtggcctggctgatattatagggtggtttcaccttgttgaaggtgttcacaatatcttcactggcaaaagccatcccgatgcggagtccggccaatccccatgccttcgacagtgtttgcatcaccacgaggttagggtattcggtaagttcctgtataaaagttttctgacgggagaaattgatatatgcttcatctatcaccacaataccatcaaaattattcaacagcagttctatgtccgagcggttgatagaattgccggtagggttattgggagaacagatgaagatgagctttgtgttggcatctatggcctgttgcaacgccgggatgtccagctgaaaatcttctgtcagcgttaccttgcggataatagcatcgttgatgtgcgcgcttacttcgtacatgccataggtaggcggacaaaggatcacgttatccacacccggattcacaaaagagcggtaaagcacgtctatggcttcgtcgctgccgtgaccaataaaaatattttgtggcggcacacctttgatatcagcaattttgtacttgagctgccattgcatcggatcgggatagcggttgtaattcaccggcaacggggatccgaaattattttcattcgcatccaggaagatggatgcttctcctttgaattcatctctggcagtagaataaggcaccagtttttttatgttttcccttaccagggtatcgagattaaacatattgcattaattaatctgttataagtgagccggtgtattccagctgttttaatcttacggtaacggcgtttttatgcgcctcaagtccctctgctgctgccatggcttctatggtacttccaatattccgcagcccatcgggagatatctgctgaaaagtaatcttttttacgaagctgtccagcgacacgccgctgtaagccctggcatagccgtttgtaggcagggtgtgattggtgccggaggcgtaatcacctgcgctttccggggtataatttcccatgaaaacagaacctgcatctgttactttatctgccaggttttctgcgccttcacaggccaggatgaggtgttccggcgcataggcattcagcatgtcaatggcagtatccatatctttcaccaggatcatcttgctgttttccaatgccgctgtggcaatgcctttgcggggcagttcgtccagctgggcattcaacgcattggttacattggcgagtacctgctcacttgtggtaaccaataccacctggctatcggggccgtgttccgcctgcgatagcaagtcggccgccacaaaagccggcacacagctatcatccgccagcacggccacttcagaaggaccagccggcatatctatggccacgccgcttttattcaccagctgttttgcacaggtaacatactggttacccggaccgaagatcttatatacctgcggcacgctttccgtaccataagccattgcaccaatggcctgtacgccgccgatagtaaatactttgtcaatgcctatcagttgggcagtatacaggatcgccggatgcagggaaggcgtgcaaagcacgatctccttacaacccgctatcatggctggtatgccgagcatcaggatcgtggaaaacagtggtgcggaaccaccgggaatatataagcctaccttttgtatggcgacagatttgcgccagcattgtacgccgggcatggtggctattacctgtaccttttcctgctgtgcgcggtgaaaggtagtaatgttttttgctgcctgctggatagccgctttcagcgccggttccagcgtagcttctgccgctgcgaaagcggcggatggcacctgtaaattatccagcgttactttatcgaattcagctgcaaattttctgatggcggcatcgccgccggtgcgtacttcctgcaggatatcattcactttcttttcgagcgtggaggtatccattacaggtctttgcagcagcgtattccaggaacttttatcgggaaatctggttgtttgcatcgtttactcagtttatcagatcaccattttttcgatgggtactaccaggatgccttgtgcacccgcttctttcaaactttcgataatatcccagaaatcattttcattcagtaccgaatgaacagagctccagccggcttcagccaaaggcagtactgtagggcttttcatgcccggcagcaaaccaataatttcattcagtttatcattgggcgcattgagcaggatgtacttgttattttttgctttccttactgcctggatacggaataaaagtttgtccagcaacagctgttgttccggcttcaggttgtggcaggctgccagcactgcttccgatttcagcaccgtttccacttctttcaaaccattcatgaacagggtagatccgctgctcaccaggtcgcagatagcatctgccaaaccaatacctggcgctatttccacggagccgctgatttcatggatttctgcggtaataccgttttgttgcagaaaatcttccactattacaggatagctggtagcaatacgtttattttgcaggtctttcacggaagtataatccaccgatttttccaccgccatagacaaacggcattttccaaagcccagtttctgaacaatatttacctgcttttgtttttccagcactacattttctcctacaattcctatgtctgccacaccatcttcaatgtattgcggaatatcatcatcacgcaggaaaaacacttccagcgggaagttggtggcctctgttttcagtttattaacaccgttgttgatgtcgatgccgcactccttcaaaagtttgatggaatcgtcgtgcaggcggccggatttctggattgcaattttcagtttcatccctgataaaataaaaaaaggggcttacctctgcggtaagcccctgttgatgatgtaatatggtgatatacacaaatcatccccctgcctacccttgtggtaagatatgatggtggtgatgtgtatgtttgtttgtaatcataatttcaggtgcaaaaataggaagtaaaatgaaataacaaaggttttttttggaattaacgggaaatttaaatataagcgcttatatataatcactggtataatgaacctttgccaatatctcttttcagcattccagcctgcttatttcgccagcctgctttgcagttcaggcactacattttcaaacgtacgcagcagccggtcccagttccggaatgattcatcagagcttgcagatacaccgggaggagctatttcacttaccagctttgccttgtaggtaagcgggtctgtgttccctgttttaatgataagacgggtacggacagtagctgctttaaaagattttactacccaggcagtgcacatgtatcccgtcgctttatcggtaaccgcaatcacatcaaaataaccggtaatgatgcggttgatcagcttccaggaattttcttcatcatgactggtccgtacatcgatatcctggttcgcgagattcgttaccatcgaattttcgtacgcatcgtctttctccagcttaatataatctgtagaaggcaatgtatgctttccatcattgatgtagttccgctcctgtgtaataaaacctaccttttccacacggatgtttacctgcgcgtatgctgctaccttgatttctgtagaagtgttattgaccagttttccatctacatagatccgtgcgtcgttctccgtattaataacgatctttttggatttaacttttgcagctgcatggttgggtgcaaagaaggtgaaggctgccaggcagcagaaaaggagtgctttcatttgaatgcccataagaaataaggattatctgaggtttacaatattttcaccgcgcaaaatttaacggcgcataaaattatgtgtgggacatacagggagtgtagaaaaaaaatccggatgtactgaataacaagtgattaacattaatataaacggccaataaatgataaatattgaactggatacattatcttcccttctgtcaaaaaaaatcttactgcgcctgttttagcaaccaggattcatagctcactgatctcccggcacttacttctcccctctcctgcaacggatttccatcttttgcaaacgatgtgttaacggatttcataaactaataattttagctttattttgctaataatattagtatttacaaaaacgatagttatatgcaagtgttgaaactgagtgacccgcacattaccctgccattctttaataccagtgtccctgcagggtttcctactcctgccctggattatgaagaagagcagattgatctctcccgtatcctgcagccaaatccctctacctccttcattatcagggtaaagggcgatagcatgactgatgccagcattcccgatggttgcatggcggttgtagaccgctctatccgaccctccacgggagatattgtagtggcggcactcaatggggaatataccgtaaaacggctcgtaaaagcgggtcgcagctgggtattacatcccgaaaatcctttttataaacctattgttatcacagaagacgccgacttccaggtatggggcgtggtaaccgccgtcattgtagatatgcggaaatagcgcaccgggacagatacagaaataaaagtacctttatccgattataataccacgacagataatatgtgttacgatattgcctttacctccagcatagagagcattttcaaatacctgccgcgacttaaacccggcggcaaactggatatcgacttcgaccctacctggcacaagatcgggatgtcttatccgcaatggcccgtagttaccaacaacaacggcatcaaacttgaaaaatacacctggggtcccatacctaaaatgctggacaccctggaaaaagtaaaacgccagcggcaacttttcctgaacgcccgcagcgaaaaagtacttgaaaacggcaccatgtggaatgccatccggcaccagcgctgcctcgttccagccagcggcttctttgaataccggcacattcccggatggaaaaataaagtggcctattatatcaaacccaaagaacaggaactcttttttatagccggattgtgggcaatgtctaattcctgggatgtagataaacccgcacgtattcccgcgttcaccctgctaacccgtgccgctaacccactgatggcacagatccataacggcggcgacaacgccggcagaatgcccatgatgcttactcccggactcgcagaacaatggctgcaacctgaactaactgatacggatatacgctcaattatacagtatgaactgcccgcaacacaactggaatgctggccggtaaattctgtcagaaaagcaaagcctgatgacgcagcagtaatagcccctgcagcatatgagcatttacctgccctgcagatgtaatatcgcttcccaggcaccacaaaaaaacggacgcccctttcacaaggcgtccgctcagtattgctacgtttcaatgcttacttagctaccacgcccgcaggcactttaccatcagtattatccaatgataatccaagcagttgcgctaccagcggtgccacatctgttacattcatttctttcacatgaccgcctgccactatccctgctccggaagccacaaagccggtttgtatctctttaaaatccgggaaataaccatgtgtgccccctttggctgccattaccagttccccggtggagccacccccaatggtaacgccatcagaggcggaaatggccaaagcagcatgcggatcagcgcccactgcatccagctgtttgcggccaataatccggaacatttgctgctgtgccgctggcagtgctttcagcaacgccagtactttctgctgtgtagctgcatccttcggatctttgagatgcaggaaggccgacccgccggaagaatggaactgcgctttccaatcacccgttttgatattattcagcaaaccattttgcgccagcaatacattcggggaaaagcttttgccgatattcacaaaaccatgatcgccggtaacaatgacggtcgtattttcgtatatgcctgcgcgtttgagcgcttcaataatagtacccaacgccctgtctgcccccgctaccgcctttcttaccagcaggccatcccggccctgttcatgctcataatgatctgtacaggccagatgcagcgtggtaaaagcaggcttataggtagtgatcaggtaggccgacatacgcgccacattttcatccaggatcatttcttcatcctccatcgtgaaatccttttcacccagcttacccgtggcatgttcctgtacttcctgccataacgacacaggattggtgacggtagccatcagctcccgcctgtctttttttccaataagccatacatccggtatattgtaatcgatcggtgcgcccacagataccggccagattacattagccgattttttcccggctttatgcaccgcatcaaacagcgtaggcgttttgatgctgtcgtaataaaagtaccagatgccgctggcgccattaggctcaaaaggtgtgttataataaataccatgccgcgccggtgttacaccggtgatcagcgacgtgtgattgggataggtaacggtagggaatacactgtttactccgtccgcataagcgccgctgtctttcatggcccgcaggtttaccataccccaggaagcgtctgtataaaactctggccggaagccatcaatggtaatcagcactacatgcgaggcgcgctgcgcataggaagtgaatcctatcatcagcaacaatgctataccggtaatcttcttcatacaatatattttttcaacgccggtttcaatgccagccataccagccaatataaggcttcaaaggtaaagggccaagtccgcagcgtaccagaatgtaaaaacggaagccctccgggatcagctcaacgcctctttcgcggcgtatctccggcaatacagcgtgtattacgctttcgttaacattcgggaaacgggacaaggaccgcatccctgtaaggtatactactcgtagcagtgagtatatacagcggactataattccgcaatacgtaggaaaaagaccctaacaaaaaaatggctgaactccccggaatcaacgccttaattcccctataataagccataggaaaggaaaatagcgcctctgcacatttttcctgtgcattggtataatgattgccggatagtgcatgaaccttttccggatgaactcatccggaatatttatctaccttaaccatacaactatggcacacttagaagttcaacccaggaaaagaaatccagcgtggctatggctgatcataggtcttatcatcatcgctgctatcctgttttttctgatgcgcagcggtaataaccgtcaacaggacgtaatcactaccactgatactgttagcactaccggcaacgctgcacccgcagcagatactcccggcgcacaaccgtaaaggttttcacctattctttatctaaaaaatattaccatgtctatcactgaaaccaatcgtcttgaagaattaagcggcagcagatttgaaattgtagacggacagcccgatatcaggaactggggggtggaagatctgcaaggcaataaattcggaaaagtagatgacctgctgttcaatcccgcttcacgcagggtgcgctatcttgtcatcaacctcaagggtaaccggataggactcaccgaccggaaagtactgtttcctatcggcgtagccatcctgcatgaaaaggatgataccgtattgctgccggaaataactcctttacagatcagcatccttcctttttatgaaaaaggtgtgatcgttacccccgaaacagaacgggatatccggaatgtgtttgtgtcgccggattcatataccgccgataacgacttttacaaccacgaccagtttgaccaggatagattttatggaacacgtgcgccacgggataaccgcgtatagtacttgcctaaataatcgtccgttgatgttagcctgcaaaagagaaagcctccggtcggaggctttctcttttgcaggctaacactaaatatgttttatttgtacaacaaattgctccggatgaaatatgctttggtgtgcggcctcgtgttactctctttttttgccaacggccagaaccttgtgaactaccgcgatacggcgaatcacttctccgtaggaattcccaacggatggcaggtaataaaaaacaaacagatcccttccctgaaattcatggcgcagcgggccgatagcgccctggtagcgcctgaaaacttcacagtcaatgtagtggatgaaccccgctccaacgtagatgccgttgcaaaaaaactcctgtactatatcggccgcaatccttatttcaaactactggattccggcagcattgtcagcgccggtaaacggatgatctggctggatgaaatccacctggagggaagcaggaccgataccatgttcgccagcatctttattgcgtattcaaacaacaaaacctacctgttgacctccaccactcttttgccgttttcggccggttttaagcctttattccatgaaataggcaattccttcaaaacaggcaaagcagcgggaaaagagcgccttaaaattgtgctgccggttaatgtaaaatggacaacgatcaccgataccgaagtggacaatctcgctacccgccagttcctgcctgccaatgaaacggcgcagcaatggaccctgctgatcaacaatatgaccatggaaaatgcacgggtcgataacattgatctcgctgtaaaaagcttctcggaagccgctgtgagtaaagcatcacaggcaaaggtgacattgcttggaaaagaaaatattccccagcggcgctgggcactgttcaaagtggaaacacccggcgccggaagtccggaatcgcagctgtattatgtgatacagggccccagatcctttcatgccattttcattgcccaaaaaacagaaactttgtcggccgccttcgtaagcaaatggagcgccgttttcagaaaaagtaaagtggtgaatgaataacccattaactgtgtatttatttacgcagccctccgcaacagcagcctgtaaatcaagctgtttttagtggtgcgatgtttggactttccctggaaaacttgctttatgaccacacaacctaaaacacccggaccactgctcaatgacgatcttcaaccagacgatgtttttagtcaaaaacaacaacccgtgccgcagagaggcaaccaggatgaacaatcccggcggggcgacgacaactctgatgaattactcgacgaagaagatgacgacgtggaaatagatgagctgctggaggaagaagatattacggatgaggatgtatcagaaaacagcctggaagaagatgatgcgccaaaaaggccgctggagtaaaacaatacgaacggatacgggtactacgccccgcatccgttcgttataatgtttacttgtaaatcgaaatttcaattttgccgtctttggtaacggcgccccggtacatgccttccgtgttaaaagacatggtcatgtttccttttttatccagggcaatcaaaccgccatcgccacccatatcccctacttttttgatcaccgtattacccgcctgctgtacagaaagccctttatacgccatgagggcagacaaatcataagccaccacattacggatgtaaaactcaccccagccggtacaggatatggcagcagtttcattgttcgcataggtacccgcaccaatgataggcgaatcaccaatgcggccatattttttgttggtcataccgccggtagaagttgctgccgccaggttgccctgccggtccaacgctaccgccccaaccgttccgaatttataatcccggttttttatacccagcttgcccgggttcgtataggcgtttgatttagccgcagcaatagaatcctccctgatggcactctgcaggtccctccagcgcgattccgttctgaaatacgaggggtccactatttccagtcctgcttcctttgcaaacttttctgcacccggccctaccatcatcacatgctccgacttttccatcaccgcccttgcagcgctcaccgggttgcgcacggtggtaacaccggctaccgcacccgctgccctggttttaccattcatgatggcggcatccagctcgttgcgcccttcgtgggtaaacacagcacctttgcccgcattaaaaagtgaatcgtcttccaacacccttacagtggcttctaccgcatccaggctgcttccgcccgactgcaggatcttatagcccgtttccagtgctttttgtaaagatgccttgtacgcggcttccttttcaggggtcatattctttttaagaatagtacccgcaccaccatggatcaccagcacataagatgatgccttctgttgcgcctttacaggcaaaacaaaaagtaccatcagaaaaaataaaataccaaacctgcctttcatatcaaattttattacggaaataatcagattgcttttttcttcagctgtcccttttccacccaccaccaataccaggcgccgccactggccgttgcggcatcaaagtcagctacccggaaactgccgttgccggaagcgctggcagggatttcatataccttcaatgcctgcccgccatggttccattgcagtggttgccccggttcacaaagttccggttttttaagactgtcagacataatgaaataagccttgctcacgccaaaaactttggccactcctgcttcatcaatacacaccgccgttttttcatcgggcgcaatgccttttggaaaaatgccctggtctttaatgatccggctcataaaagtaacatgcctgccttcgcggccacgtttcaggtaatgctggtcactgattacatcacgaagataaggcgcatgcaggaaatcgttgttatacacttttaccagcgaatcatatggattggccagcaccgaatcagacaccgcactgcctccctcgccgctgtaataaaacccggtcaggatagcacaacccgcgctggtgccgcccaccggcactttcttttcctgcagtaaataattgatcgcatcatttactttggtacctctccattgcagcatgtagcgcgactgatcaccaccggcaataaacaacatttctgcattacggataatattggccacggtatcattattggccagttccctgttggtaatattcagcgtttctactgagttcactttccccagggagtcgatgtcatggttatagccgccattgccggaggcggtaagcactactacatcaccgccaccgctgcgttcaatcatccattggaaagcgccgtccacattcccgccaccaccaattaacgctactcctccttttaccggcgtggttacatctgccgtatcgccaataatcccgatggaagccggccggccggcaatagtcagcggtttgggcatacgcatataacaggcatttaaacatatagccgttatggttagtacagttattattcttttcatcagtagccgggattttgtttcatgtttttattagctttcgtttctgcatcaggaataggaaatacatatcccttctgaccaggtttcagcaacacagcacccagtgcgttgatagcgtcttccgggttgcgggttacagacagtccccttcttctcaggtcgaagagacgatgcccttcaaaggccagctctttgaatcgttcggtgtataaagcggtgatcaatgcatctttattactaaaagactgcggcgtgtaaccattgatacgcgcagcgcgcaggtcgttcaggtcagcggcgccatccgccacccggttactttccgccaatgcttctgcacggatcaggtacatttctcccgttctgaaaagtttaatatctgccaggcccatgctgccggaagatccaaaatatttattcaccaggtattcagagttgccatcaccacgggtatcgtcaaactgtatataagcaggataacgcacatcgttatttttatcgaacaggttaatcagttcaaaagaaggcacatataacgctacatccctgtcgaaataagcactgccgatcaactcatcatcactacctgctacctgtttcagcttccagataacttcagattgcttggtgtctttccagatgccgggaaaatcactggcggaggccagcggcagcgcatcaatagcttctgtagcataggtgatggcatcggtccattttttggcgtataaagctactctcgcctggatagcagaaatggccggaagcgtaatcctcgtgttatcatctgcttcagctgggatcagtgttttagccagctgtaaatctctttctattccagctactacttctccaaaagtattccgggcaggaaaactgttaacggaagtatccatataaggtactcccatcgctgccggctcatatgcctctgcataactctgcaatagctggaaatgacaataagcgcgtatcgccagcgcctctccgcggtactgatctttcaaggctatctcatcacctttggcagtaacattgcccatagcgcccaatacgcggttagcgcggtcaatggcaatataatactccccgaaagaagcagtaatagtagtattgctgggatctatctgccagcggtaagtggctacaccgccgccagtaccgttctcactgggcagggtacattcatcggtaaccaatgatacgccgtagatggtgttgtaggtaagaccggcataagcgccaagcaggccgccattcagatcactgacagtccggaaggttcttcccggatctataatgctgtcggtaggagaaaggtccagttgcttattacaggcaagtgtacacaacgacaacaggagtgtaaaagtatatttgatataacggatcgtcatgagcttaatgatttaaaaattaacgttcaggccaaaagtgtaggttcgtgcgctggggtaatcaaacctgccgtcgccataattattctcaggatcaaaactcttccagctggtccaggtgtacaggttctgagcctgcgcaaatacctggatgccctgcacaaatttcaggtgggtcatgatttctttcgggaaattatagccgatgtttacattccttaaacgcaggtaagaggcatcctggatatctttggaagaaaatcccctgctggcatcaaacttaggcaggatggcattatcaccgggtttcttccaacggtcatacagcatacgtaccgattgattactgctggcaaaacttggattctcgttgtaataatcttcgttgagataccgcatggttttatctgcaaatgtaaacagcgcattcaggtaaaaacctttccagctaacggccgtattaaatccaccggtgaaaggaggaatataagtgccgaattcggctacgctcaaagccgtttcattataatcgcttgttttattacctgacctgtcatagtacaaaggatcgcctgtttgcggatccacaccggcccatttaggcgcatagtgagatccgtaaggcaagcccactcttacaatctgtgtagtaccctgcgtaaattcaccggacacgcccagatcggtgatcacatttttattataggcaaagttcacacctaccgaccaggtgagatcttttcccttcacaatatctccctggagatccatttctattcccctgttgcgcatagcgccggaattgaggaacatggtggaaaatcctgacgtaatagataacggctgttctataaagaggttattggttactttattatatacatctgttaccaggcggatgcggttattcattacacccaggtcaaaaccgatgttaaattctttggcgtactcccagtcgtagttcggattacccggctggttaggcacaatcgccgggttaccgccatactggtcggttccataagtccggaaataagcaaaggggccgagattggaaaatggattggcggaagtaccatagctggcccggaagcgcaggttatctacaaagctcacatctttcaggaaattctctttctttacttcccatccaacacccagggagtagaacccatgccagcggttgtccggtggcacggtagaagcgccatcataccggtaactcgcattcagggtatatttttcattgaaagtataccggcctacaccaatgtaagaagccagcgcacttttggtgcggcctccgcccagcaaggcgctgtagggcgaaccgggtgtaatggcggcaggagtggcgggtaacctgtcgtccaggtcataacctgtataatcaaatgcgcggtaattattcctggtaaactcaaaataaccggatacttcgaaatcatgtttgccggtaacttttgaatacgttaaccccgaagtgctcaccagcgtaacgttcctggtaacgccttctccaaaacttcctcttccgccgttatccactttatagccggaataagaatccgggttcacataacgctcggtggtagtttccctgaagtcgatgcccaacctggttttcgccaccaatcctttggccaggatgtaattcagtgaagtaccgataatgcttttcagctggttatctttactgctggtatttaataaggcttccagtgcattactgccttcccgcagatcatataccgggtacacatcatcgttataattggtaaccagtgtgccatccggtgcataaggatattcataaggcagggcatagtataccgctgccaacgggttgctgccgctactggaggcttctctttctataaaggaagactcagaataggccagtcctacgttgatattggcggttaatttacccgcattgaaatccaggttatttttaaagctgtagcgttttaattcagagcgtttggcaataccctgctgatcgtaataattcacagaactataaaaccgcacattttcattaccgccgcttacactcagctgttgttcctggaatttacctgtctgaaggaaaatttttctccagtcggtattaacacctcttaagctatcaatgatatgatctgcctcttgttgttcctgtggtgttttattgaggtagtcaggatttttattggagaactcccaacccggtcccaggttagcgccggtttccaggccaatctcttcttcaaactgcaggtgctgcagggagttcatcatctggaacttgggggtggtcatattggaaaaaccatactgcgatttatacgacaccgctattcttccggcctgtcctttttttgtagtgatcacaattacgccgttggaaccgcgtgatccgtataatgctttagcagaagcgtctttcaatacggtaacagaagcgatgtctgaagggttgatgccctggaactgccctgcttcaatgggaataccatccattacatataaaacggaggagctgccattgatggtaccaacgccccgcacggtaatcgttgcagcggtacctggttggccggagccggcagatactaccattcccggaacccgtccctgtaatatctggtcgaaggtagccatcggtacctgcgtaatcttatcagcgcctactacgccggcggctgcggtagatttatccctggtataattcgtatacccggtaaccgttacggcattcagcgttttgatgtcttctgttagtaccacattgatttcacgtctgttgccaatagttacctgctggctgagataccctaccagtgagaactggagcgtggtggcattgtccggggcgatgagcgtataagcgccatcttcattggtaagcgtaccggcggtggtgccggaggcacgaacggtaactcccggtaaaggcaggttatctattcccctcaccgttccgctgatcgtaatatctacggcagatgtactttctgcgcctgcatatactaccaccagcccgtcttctttcagggtatatgccaggttggtaccggcaaatgcctgtgaaagcactgcatccagcgtggcttcttttgctgctaccgtcacctttttgttttcaggcagtgttttatcatggaacacaaagcggtaggccgtttgatgctccagtgctttcagcaattgtttgatacttgtttcttttacctgcagggtaatggtctcctgcgcgaaacaaatagcctgcacctgaaggcaggtcaaaaaaagaagaacagttaatttcatagtaagcagcaatttgccggtgggaacaggtttccccttccattccaggaatacaagttttaacatacctttgatgttggtttagttaatgatcattcaggacattttctagcctaattccgggggaagtgttccagcacttcccccttctttatttggttgatgtataattatttatttactgatgataatctgaccgtttaccattttaaaactgaatggataagataactgcagggcatccaatgctttcaggatcgtttcactttcaaaggtgccggaataccggtaatgctttacttcttcatccgcaaaggtgaccttgatgccataccatttttccagcttgcccgctatcacttccagcggctcattttcaatttccagccggtttcttacccaggctatttccctggctttatgatttaccgggtctgcgtccagcggcattactttaaaaggattgaccggcgccggcagcccggcaacattcatcgttagcttctggtttggttgtaatatgatcttttcttcgggcttattggccagcgtaacctccaccttgcctttaaacaaagcggtttccgactgatggctgccggcataggcacttacgttaaaaacggtacctaatactttaatatcaaaagcggcagtatgtacaatgaaaggatactgcgcatgctgcgttacatcaaaaaaagcctcccctgtaagggttagcttcctgttggcctcattaaatccctccgccagttccacggtactgttcttccgtaaaataatggaagagccatccggcagcaccacggttttacggggatcgttgccggcattgataacaaccatgcttgttttgggtgaggtgatatcagtaacggtgttggtacggctgaacaggtaaatggcgccggccagtagcaggatgccccccaatgcggcagcatatttaaataatggaccggttttcctggcgggagcaggtgtattttgccccaacggctcttccagggccgaatggagcagatcatactgtaaaataccatctttcaggtgtttcaactgctccaggcggttaccctgccgggccgacaataccccaatcatataccgggcctcctgtacagcagccttcttttcaggatggcgggttatccagctctcccaaaataatatatcgctgtcattctcttccaggcaatagcgctggaaagattcatcacatgcaaagtcggcggcttcgaaatcctggaaattcatgtagataatgcctttgactatacagacggcaaaatcaatcgtttttcctaaaggttttataatttttttttcgggagatgggaaagccgggcttatttcagcattttccttaatgctttgatggcatcataaatagtattgtaagccgttttcaccgtttgtgaagtttgtgcagcaatctgttcgtacgacaatccttcaaaaaacttaagccgtatcagctctgtctgtcgcggagtgagcgctttcagcgcctgctgcagccgctgctttaattcttcgtcctgttgtacctggataataatttcttcataagataattcgcgctccgcttccttatcagtcatccggtgaatagctgcatggatcttcgactggtacgccaactgatccagtagctgtcttttcagcgcggtaaataaataggccggcacgttggttaccgggcgcagactttgatgccgggtccacagctgcaaaaataattgtgtgatacagtcctttaccagttcatcgctgccgcaggttttcaatccaaacctcagcagatgtgaataggtattattatacagtgcaaacaacgcctgcttatcgccgtttctcaggcgttcccaatgaatattattgtcttcttcataagacataaaatgcaggtcgttataatgttgatggagcagtttccttcatcaattccctgatggctgcttccagttgctgatctcttcccttaattatttcttcaggcgcattccttacacgtatatccggttccgtttgatgattttccaggtaatagccctcccggctttttacacccagtgaaggcacgctccaatggaggttaccatcgggcaatgtttccccggtcatgaaggtacaactgccaggcactggcatccctatcagcttacccatatggagatactgataatcgaacacaaaacagctgccatcgctatagttggcttcgttggcaatcaccaccgacggctttgtccagcggaagccaggctctatgctttccacctgctcgtctgttgtatttttcctgatctccgtgccgctcagcatcatgcccaggtctgaagccagatcgcctccccggttaaaacgggtatccactacaatacctttacagccggcgtacctgcccattatttcgctgtaggcattgcggtaggcggcgtcgttcatccggtataaatgtacatatcccaattgtccgttgctgaggcgtgttacttcgtccctgttacgttttacccatcttttatacagaaggtcgttttctgcttccggcgtaaccggcgtcaccactatatcccgtcgctggccaccatcatcaatacgcagccgggtatttttacctgcccggtgattaaggtattgcgaaagatctttatctgccgtaatctcctcaccatctacggccgtaataaacatgcccggcttcagattaaatgcttcctgatccagcggtccgccaggaagtatttcacttattttcacaccgtcgccactgtaagatacatcgtaacaaatacccagggaagctgtttcttccttttcttccaccacatggctgcccgttgcgccactatgacttacattcagctcacccagcatttcactcaccatttcggccagttcaaagttgttggcaatatgcggcaggaacttttcataattccggccatacgcttcccagtcggcgccgtgataaccagcggtataaaacgcttcttttgttcttcgccagatatgggaaaacatcgccttcctttctgctgccaggtctattttcatggaaccgttaatggtaatgctatgctgcgtttgccccgtagtatccaattgcaggatgcgggcatctgccagcaggaaaagttgttgttgtgcagcgtcccattgcagcgagcaatcttctgccttcaccgacaaaggcatcgtggacgttttagtggtaatatctgttatccacaactggtaagccgcaccggcttttaccaggtaatataatttgttgccgcttttactgagtaatacatctgccagcatagcggctgaaggcgtcagttttgtaatctgttctgcatctttaaagctgccgccggaaaacggtaacgcatatacgtcctgttgccggctgctgctcgtggaaaaaccccggagtccgttccggtcgcttttccagatcatcatctttccgtccgttgcccattgcggcgcctcatcaccaaagccgctttgcgtaatattttgtacactaccactaccatcggctgctaccaggcccacttcctggttgccggcgcccggctggttgtattgaagcaggagataccgggcatcaggactccagcggaaatactgatcatgatccctgcgactgaacaacgacgcaatgcggcgactttttcccgaagcgatgttatatatttttaacgttaccctgttttcgatataagctacttcttttccatctggtgaatataaaggctgatagttttcctggttgttggccagcaacacggtttcctttccatgtagcagatccatttcacaaagccgccagccatggctactttcactggcatacaacagtttggtaccatccggtgaaaagctcaggtctgcttcttccccgggagtatgcgtccattgccggataacgccgtgttccatgccggcggaaaatacatctccccggaaaataaacgcgatgtccttaccggacggtgaaaccaccccgtatttaatatgatccgctaccggcactacggttgtattttccgtaacccggctggtaagatgtatgtttacttttttgggcgcagtgcccggcgcctgtaaataaatatctccgttaaaaccgaagcacagtgtgccattgcgggatgcactcaaaaaacggacggggaattgcttaaatgttgtcagttgttctgatgcgccgggacgaccgggccacaaacggtgcacattaaaactgccactctcttcactcaaataacaaatggatttccctttgtcggtaaacaccggtgacctgtcttccccgcgaaagtctgtcaattgcttatacgtatcgttttgcgtgtcatacagccatatatccctcgccgcagcagatacctggtgctttctccagggattctcccggttcttcttatcgtgataaacaatgaatgggccgttgagctttgcaccttccgcaggaacgcccagtaactgggttacccgtccaccgtgtacggatacacgatatagctcaggctgtgcatctgaaggaaactgccggctgtttaccgcatccattctcaccccaccaaaaatcacctgctgatcatcttcactaaaatcatagggatactcctctgccgaatgaaaggtgagttgtttttcagttcctccttttgcgggtaccaggaaaatatcggcattaccataacggtcagatgcaaaagcaatactgctgctgttatggctccatacaggcatccactcttccgcagggttagccgttaactgtacagcagtaccacccctggcagcaacggtgtataaatcgcctttataagtaaatacaattgtttttccatcaggagaaagagaaggataacgcaaccagcagggagaactttgggcaaaaatatattccccccaaaacaagatgagtaaaataatgatcagtcttttcattcgcagtgcatgaatgcagtttgtaacagcccggataaagatacaaatatataattcatattttccgggtactctacatcctgctaaatgcccagcatcacccgctcttcctccgcttcggcttctgcctgcgacacatgtggcgcatcggttatttctgtgagcagcagggtataccccagcagcaacacgatcagcaatacctggtaccgcaatacaataggcgcggcaaaaacgctgaatgcaaaattcagcccgatgaaagcccagcacaacaacagcgcaatattaaatttacggctggttttccaggtaccttttttaataagatagcggatcgtttcttctataaacaacaaatgacaaatcacgatcaaagaagggaacagcgacatcagcgtgctttgccagttattatatttaccttccggcttaggcttgtccccatctttaaaaaaagtggctacctctttattcaccaggttaataacaggccggttatacccgcccagcacttccagttccggcaacagataaagctttgtattgcccagcaaataatagcgggtaaaatcccaggggtacttccggatcatataattgccgtaatcactgcataaaggcgccacgccacaccagcccgcatatacatctttaccctgatgcgccaacccataatctctcagcaatcctttctgcggcccgttcatgtcccacataaaatacgatccgtctgacaccactattttcctcggcagcttcttcagcgccgtcatgtagtgatataccgccttatgtgttttggcaaactgtggcggcacgcccgcagaatccagcggcacatactgcatcatatacatcgcgttattcatgatctgccagccgctgaaagcagaaaatattttcaccccggaatgctctgctgttttctgacgggtaaacagtacaaacgaaacgatcagcattaccggcaacaaaacagccaccactttctgccacggccggtaagcagataataaaatcgggatcagcgccaccaacgggtaaaacatggcattatagcgcaccgtaaacgcatagcccagcaacagcccgtgaaataccagtaacaacgtagttggcttatgcaggatccacagcaacaaagtaatccaggtaagtccgagcgaaaggaacagcgcatctgaaataaaataattgctcaggaaagggaacaagggattaataagcaggaaagcataaaagccatacctgaaatagctctgtggattaaaaatataacatacactgaaatagaagaaaaacgcactggtttccagcaatacaaactgcaccacggtgagcatcgtttctgagcgggaaaactggtgaaacaaccacaggaatttggaatatcctataggccagagattataattcctgttctgcagggccgtttccatataagaaccggtatctgatgtaaaatctatgtacgggaaaaaatgtttgaataccaccatcttgatcaccgcaacaataatagcagctgccaggagcaggccattacgccggctggcaaatacaaaggcgccgaaaccgggagcaggggcaacaagggaccggggagatagtaataacatagcctgttttgagggatttgacttatagctgcaagtataaaagaagccactgaattggcgcgtcagtatatgattttcagcgctttaaggatctttttttgagaaaaaaggattaaaaatttggtaattatcagaaatgtcataatttcgcggtcctgatttgctattgcctgatagtataacggtagtacgacagactctgactctgtttgtcttggttcgaatccaggtcaggcaacaacctaatcgccgcagacgcttgctagacaagtgattgcggcgttttcttttttatgcggttgtcgtttttgtggttgttttaattccaatgtctaaaataaattaccgcattactttttgtctctccttttattaactactgctatagcatcccagatgcgccaattttactatcttgattataatcttttgcgcatatgataacagaacaaccggcttctctcttaagaactattatcctgcaacctcagaaaccatatgacagctatggaggtttgatattttcagatattcgttttactggggatggctacctaagtgtgcaagggcaatggccacgcgatctttatgttacagattgtgaatttgaaagccagttaatcatagaagagattatccataagaactatacatttaaaaattgcgcttttgaaggagatgtaaaaattctgtgtaaagaaagcaagaatttcattcgcttcattgattgtattttcaagaaagacttgataataaatggaaaacagtttaattctgttataatcgaaagtaatatagaaggtgcgctttacattgaagctggaaaatttgaaaagttaataattggggccgactttaagggtaaaaagtactccgttaattcttttcatattgacttttctggctcgaaaggtgtaatgctttttcgacatttactaattgataggttaaccttatatgggacgaatagtaaagattctgaggcgtctttcttttcaataagggcatttagaattaatatattgaacctgtctaatgaagggaaaatacggttctccgatttagtatggaatgatacccttacagacgaatcttatcgttcattttactgtttccaatcgaatttggggaaaacggagttcttcaatttcaatttcaattgtttccaagaaatagaatttatacaaagtcagcttattgaatgtgttttcataaatacagtgtggccgcggcattactataagttaaacctcaaactaaaggaagataggttagcagacctgagagaagaatttagacaattgaagtttgtattgtcaaaacaaggtgatagcgttaaggagcatgaatttcatgccttagaaatgcggactcttttacttttgtcaactcgtagattgtttaagtctcaaaacagtgagattaatcgtacttacacatggaggcaaaatttacaaaattgggttgtccttcttctcagttggttaagcagtaactttggattaagttggctacgacccatatttttcatgctagtggtgaactttttccttatttacttagggatatatgggtttaggctacaagctcttgctaacatcttcagttttcactcttcagtagactacaatgccatcggcaattttttatactattgctcaccattcaggagatttgacaatatcataacaggcaaagcatccatttttgatatattaattaggatagtatcatcctacggaatatacaatttcattcgtgctaccagaaggtatgtcaaataattacactccttcttaggcttaaagaggcaaatcaggtaaaaaatcctttggcgaacatttgaaaaccttagccaattcattaagatgccggatattatatttatccctccgcttattgctttctacattggaaataaagctatcggccattcctaaatgttgtgataaatcaatctgtcttattttttccttctccctcatttctttcaccttatttattacaaacaaatctacttccgtggcgtgtggcttgctttccatagtcattttgagagtaaagcaatgcctatcgaaagaaaaaaccaaccggacatgtccggttttatcaatatttccctatatttgttaaaatgattttgaacttatggatacatcatagttttattacttttgcgggataataaaatactaagcgtgtttgctttgctctctttgctgaaaactacgacctttcaagaacaagagggaaaaaggtaaatcgcctatactatattggtgtaggcgttcttttctcttgttcggggtgtcgtagcccttcagcagtgataggaaccaacctacaccatttttatgcccgctagtttccccccgccctcacttcatttcttttaacccttcaattatccaaaaatgcaaaaagaaattataataaaaatatcatctggcaagtcaaatgcagccctagaccttcatacacttttcagcgcattgccaacagttttcagggagtatgtatgtgaagaatgcaattggagtactccaacattttacagaaagttaaggacaaaggatatggtaaatcccgaaaatccgaaaagggtaatttctgctatcagcaaagccgaaaaggataaaattatagaaataggactaaaggtgtttgaaaaggcagggatgtacataagcaaatacaatcctcaaaccagtaaacaataacaagattaaagctggttctatgactgataaagaatttctaatacaagcctgtgctgaaatagaggctaagaatcttctattaaaaagggattgccgcaaaatggatatagaaattaaaaaattgcggaaggaaatagccctacagaaaaagaacggagggcttatttgcagtggtgcggttaatacccaaatccggcttaatccataataataaggtcaataatgtgaaggaggccggacattcgcaccccggaaaggcagcagttttgctgcctttttttatcagcggttgcctttatcttttaaataataataaaccgttgtcctgctttttcttagtatgcttgctatttcccggtaactatgaccttgcctgaataactcttttgcgcgattctgcaatgtttcaggcgttgccaattctttaaatttattatccctagcgtaccgctgtatagtacgtggtgaaatattcaatagcgttcctatttcaaccgcgtttaaacctttcaaatagtattgataagccctttctacaagtaaattattaaaccttgtcttaggggctgcatttacgtttcccattaaaattcactttaaattaacctaaaatatacttaaacgtgtcgcggttgtttacaccaatatgggtagtttgttgaactgttttagatagtaccccccatacgttatttgccctaagcaatgcccctgtataggaaaaagtatcaaacaacctttaaatctatcttaaaaccaaacacctaccagatacggaacattgatacaataccgatccggtaggtataaagcatttaagagccgcaattgccctaagctgtaaacaattgcgactgtacaaaaacagggtagtacaaaactggctcgtttctttcagtcttacgcaattgatagcggataaacgcagcctctttgttaagccccttacagattataactatatcgtatagccttgcttttaagcgcaattctccattttcattatgtatctgttcccgtagttgcttttcgcactcaataaagtaacatctggctaacttccctttttcggtacgctgtagcatggatatttcctttgcagtatccattgttaaaatgtaatccgttaatgggcgaccaccaatacttttggccaaaattggccgaaagtccaaaccattatcaaatccgtaagcaaacatttccttgctccacttatggaaagcacgtttaacatctaaaaatttgtgcaattcctttgctgatactacgttctgtccagcgtggttctgaattttaattagtccattcattatttttaattttaaagtttgattgtataaattgtttagctgcttttccctttatagtttccggcttttcgcccgatgcaacaggcataatgtcaattttcgtaatccggtctaaccacgttttagttatatctagttctgaggggtgcaacgtatctgtataagtctttcccccaacctgataggtgattgatataaagttttgaatgttcatagctttaaaaattgtgcgttttaaatctctacggcggttactgtctttatttctacaggatttagctattttcccataccggctttcactacaaaacatactggttacctgttgactggatatatcccgaccacaacttttacaggtacgcctttgaacatttttcgcgctatatattttaacctgatccagtgaataaatttgtgcaggattcgcacttttttttctcctattactgttaagggataatgctaccttttcccctacatattcaaggtgtgaaaaggttgcatccacgcaggtattttgcccgcctcctaactggtgaaaaggttgcagtttttcagcttcaaaaaggccgttccaattatctagcagcaaggcatttaaaagaggtttaaggttcctctttgaatatttcgttatcaggtcgtttaatcgctgccggttacgggtcaattggtatttactcatggcagcccagcttaccggattactcagcattagaaattggtttaattccggctttgatagctgcctttggtctatggaataatcaaagaaaacgataccatgtaatacttcaataagcaggcttatcagactatacattttatcagcttccgtaagatcagccattgacgtaatccggtaaggccggagataccgcatttttttaacctttacttcaaaccgtaacatatacccgcatggctgcttactttgagcctgcttatcgtatagctttacatcatagtccgtaaggcaacaaataagccccatacgctttacctttttatctatttgggtaaatggcttattccggtagcaaacaacctgtttaaatattcttaatggcgaaaatggcaactttatatttactccaatctccaaaccatgcagggttgccgcacccggaataaccgcgaacctggctgtcaggtcttttacggtattgaccagctgaaaaaatgaataatcatttgcattatgcaaaccgtcattactgtatttatgtaacgatccgttaagcaaaagtgccgctcccggccctttaacagatggtctaatttcaaaccgcaatcctttataatccgctatttgcgcaactgatataatttcaccggttgccaaatccacatcaaccccgtaaaccagcagcggattaccacgccatgcgtcaggttgtaaatatgggtgatggctctttatccagtctatcatatcaattaaatacagggttaaaaattagtggtttgctgtttgcttgctgatagcagtttgcgtatactccaaagcaattcctaataattgcccggtgctgtatatggcattttgcggcatcctgcctttgatacacctttccagtattccaatggtcatgcggataatattatctgcaatgatcacatcaggtatgcttttagtttccaaatcagggctagggtaaccgtaaagggccattaatactgattgtaggattggaattgaggatttgccggtagtgtgaataaccgccaattcatcaaatgcagcgataatggctccttccttttgagaaaggatagataacgccttattcatggttacctcctttccgggaaatatccttagcagctgctactacctcactacggagaaaacgggttttattggcaattttgtaaggcttcaaaataccggcattcatccacgcatgaacagtaggtagggagattttaaatagctcggcaacttcatggcgggtaatgaatacttcgttgttatcagctatagccggggttaactgatccaatcgcttgttaaggtcatcaaacaaccctaaaaggactgtgccttctaaattttcaatctggattaatttggtttgcgtcataatttttaagttgattatgacgcaaatctcaaaagaagtaaagaggggtatgttcaagtttattcaacttgaacaaaaaaaatatctacctgaactatttattgggggttttatcaacaatagctgtaaagtggtttttattcaattccgatagttctttcatgaaatgttccttgtctacagcctgttttgcggtttgggcttttgcattgagtagcttgtcaatattggacaaatccgtattaaacaccttttcaaaaacttcctttaatgcttttttggtaatgggggtgcctcctttggtgatgcgtttacttagagccagcgcattaatcaactcactcatttccgttttatcactccattgtagcccaaagcctgtagattgttccgctttcatttttccgtttttaatttcttttataaagtcatccagaaatttcaagtaattcttttcagtaaagaatagcagccgctctgtatacctaaaatccgttttacactcgataagataaaatttctttgcctgatcactgtctaacttagataccgcttctcttatttcttcaaataatagcaaatctttcgtcctgtttatttcctctggaagaatgtcaaaaacagttttttggtcgccatgaggtgccatactgcgcaacatttcagctgttctcaataaagattgaatgacttcattatttttctggtgttctttggctagtttttctaaccttagtctattttcaagccaagcaaggcgttccttcaaatcctctatttcgcgagctttttcctgatcttcgtataatttttcattacccaataggtcaaacatggcttataacagtttttgctttaacaattttttttactactttctttgccgcttgcttaggtttcctagctttccacatatcccgcatgatgttggcgtgttcctgctcggatagctttatatattttaggaaaacagcctctttaatatgcccggtaatcttcatgattgtttgcgccggtatccccattttatacatattggtagcaaatgagcgccgggcagtatgattggtgattaactgccatttttcaaatacctccgtagtacgtatcccggcttttgttacctgtatttcaatcttttcagtgagttttaccagctggcacaactctttaatatactcattcagcttttgatctgacatacgcgcaggagtattgccgccatatttctttaatatctcttttactgtagcatgaataggaattatcactttcccgcctgttttggtctggaaaagttcaataaactccccttttatattgtggggctgaatattcataaaatcacttacccgcaagccggtatagcacccgatcaggaataagtcacgggcgcggataaggcgttggttatcttttaaatcaaaggcagcaatattctgcaactcgttttcaggaagatatacggcggttgtgttttcagtgataactttaaagctgcgttttatccgttcagtgtttatattagctattcccgctgtagcagcttcgctcaggatcatttttaacgtggcaatatgcccgcctatggtgttgaccttcatttgttttacctgtgtcaggtactctttcaggtcattgtaaaactctatatcaatattataaaaatcaatatggcggcggcttgccttctcaaaatctttaagcaaaccggaaaaaacgttgtatttctgaatagtccgttttgagattaacttcccatttttactgaaacgtttatcagagtttttgataaatgattcaaggaatccccaaaaatgcttttccggttggtcgttccgtctagtaaaatcgtccagcttttcttttatcagctctttggtgacggtttcccgcttttctacagctgtagcataaaccctgatagtttctgcctttagatttttaagatgtgaattaatagtatccctgttaagctcctgaataatattacgcacttcatgtgctttggtactccaatgtttaggtttaacgcttaattcggtagaatatacaaggcggtttccattccaacgggcgataaggtagataatttggggggtgtcgctatccattcgacggagattaaattttactcggatcattgattttgaggttgaggtgttggcaaaggtaaattaaaagtattttggttgttgctttggttgtcgttttttcttaactattctttacttattttaattttccttaacgtgttgattagtcgggtttttaatagaatcgttaactgtgctgtattcagacagattttatagtcctttcggggaagccgaaataaaataggtgtgcattcaggtcaggcaacaaaaaggtccgctatgacagcggaccttttttattggggaaagaggtcgtgatactatcacgtgatactatcagtttatgaaattcttcgccgggagcgctaaaatatttacttttgatagtatcacgtgatactatcaataccgctaaagatgacgcctccatatcagattacccatcggattcttcaactcattgtctctatttcagagaaaatcggggaaattaatgcctcgcatttacaaaaggcgccagcggctttaaggaaaaccaaccggattaaaaccatacaatcttctttggaaatagagggcaatacactcacggaagaacaggtaaccgccatcctaaacaacaaaaggatactggctccgcaaaaggatatcctggaagtaaaaaatgcaattgcattgtacgatgctattcatgaatttaagcctaatagtcaaacctcctttttgaaggcccataaaatactgatgcagggacttattgcaacacccggaaaaatacgaagcacggctgttggaatcgtaaagggatcaaagatctcccacattgccccgatagggcaaatggtaaagccattgttgaatgaattatttgcctatttaaaaagtaatgaagacctgctcctaattaaaagctgcgttttccattatgaaattgagttcattcatccattcatcgatggaaatggaagaatgggacgcttctggcaaacgattatcctcaaagatcattaccctgtctttgagtttctgccaattgaaacggtggtgaaaaggagacaggcagactactataaagcgcttagcattgccggcaaattgggaaactccactgtgtttattgaatttatgctggctgtaatagaagaggcgttgaacgaattatcgctgaatcaactgcttcccataaaaggaaaagacaggataacacaatttgcagcgctaataaaggacgcctctttttccagaaaagattacctggaaaactttaaaaacatatctgttgcaacagcaagccgggatttgaaagaagcagtaaaagcgggtatgctggaaaaaacaggagataagaacacggcagtctacagatttaaaaagtattgagtataaggatccgcttaaaaaaataagtattttcacatttgcggatggctattgcctgacaatataacggtagtacgacagactctgacactgtttgtcttggtttgaatcaggtcagacaacaagccggctaaaatcacaaaaacttgatcgtaggcagccctattggtgtggatggcgcgatcagtgatgatgaagctctggattcgttttgtatagtaattatcaagcagaatatttattgaaaattcttccggtttataattacattaggtgtacaggtaaccaatttaaaaaataaaaatctccatgtgatcctatgtactatgacaagaacccagtcatagcaacttattgtacatgttaactataatcaacattaatttttctaaacacaattccatgaattattgtagcaaaatcattttagtgttggccattgttgccggacaatccctgatgacatcctgccggaaagaaatagcaacaccaacccctgaagagaccgcactggtaaataacactggtaaaacatcccccgatggatcattacttgggtacccgagccagtccattgcaaatggcatttatcagttaaaggcagttcacagcggcaaagccatggatgtagatcgcttctccatggaggatggaacccctctgcaacagtttacctggaacggcggtgataaccaacactggcagtttacttacctgaacaatggctattataaaataacagcggtacacagcggtaaagccatcactactacaaatgtctttccttccgaaggtggacaaatcattcagaaagaatgggcgaatttagtatcccagtggtggatagtaaatgacctgggtaactaccaatactccatcgtacatgctctgagtggcagatcgatcggtgttgctggcggtgccaccttggacggcgctaaattagttccacaaatatggtactcttcaaacagccagaaatggtttattgcatactgatacagatacctatattattttaaactaaaagatgccggcttcaataaggagccggcatcttttcattgacgttggaccagggcaacacccgcacatcgggaaaattaatacctcgcatttacaaaaggtggccgctaacagaagatggtagtaccatcctattaattttgtcgtttaaattgtttagtttttgaatgagggaatcaaaatcctccgacttaccatatatcatctcagagcgcattgtggcatagtcagcccgataaatttctaagatttctgctggaggtctgaagtttaaagttgccggctgaagtttatcatagttcacccctttctgacgtatccagtatcgccggtgtaataatagtttttcataaaactgtggatcggtcaaaagctgatctgcaattcctttgtcatccattctgattagatcgaataaatgcctggacccgcgttccagcttaacatcttcgggtaaaatctgcctttgattaataatttgaaatttttcatgaagtaggaacatcttttccaatagcgtcttcattggatgggtagctcttattttagataactgctccgcatatctgggattaggaaaatgttgccaaagaagagattgaatgtccactgtctcaaatggttcagtcagggatcttacactaaactcaatctttacttcatttttcaaataagggtggggctcaaataaagagcgataccgtacataaattgtttgaggatctttgtcccgcattagaggatctattgcttcggcgaacaattcaatgttggcaagatctaatcctgcctgttgtagactgactgccaattctttaattatagtatccgaagtaaatgcacatccttcccttttcaatccctttacataactatgggtaggctcatccttatactttttaccaaaagcttccggggacagggctatatctatgtcttcagaaaaacgctcaattaatccaaaccctttacttaaggatgtaccacctttaaaaataaaatgtccttcattgggggttgcaaaaagtgctttaagtaccagggttacccaccagtccttttcaattgcaacaggaatcactcccgatttaacagcagcctggttgagtgaagttcgtctttgggcatctgtaagatttagccactcgatcattctaatcgcttaatagatgtataataaagtcataaacctgggcaggagctaaagccaaatcttttgtcagtgcctcacttttttcggtttgaagaatttccttaattcttttttcaaattctgctgagagatttttggttccaatttctatgagacctagtataacaaggctacttaactcaccctcaaatgccatctttttgggagtagtaggtttaaactcaatatacaaattgcccattttgatttgcctgcgctccccgtctgttaaataggtcatttttgttggcacttgggtagtaagccctaatttgtgcagcgcctgagaacccgttggcctaatacgtactttttcctttttcgctacagcttctgctaccttttcgggatctggatataattccccaaatacgcgatcttgtttgggaacataataaattccatgagaaagtcgctttaacttcccctttgctgtaagcctggataatgccattttaatggcagcacttgaaccctcccccctgaaatcagcaggaaaaatgagactcccttttttaatgtgagaaattttatgctcaatattggtttgaatacttcccatatatgcaaatataccgaaaatcttcaaaattgttacttttttaataaaaaaggtaacaaaatttcaaaactaattactattaaatcagttaaaatcaattagttgtacaaaacatataaatgctaatatagagaaaataacgaacctaaaaaggacttcaaggtcaatacgcaaatccttcaaacatttgaaactaggtagaacaataacagcttattaaaagctgttatttacagatacaatatgaatattatcaggtttgttatataataaaagtaagatccctgttaaataaatagctggtaattcctttattcgccgcaaaataagcggcgaataaaggagctattatccgcagtcatattccaaagccctcctacctctccacatcccaccatactctccccgtcaaatcatccttgccatgcagccccgactgcgcggcaatagcatcttccacatgcttggtattcacattgtgctccgaaagcgggtatccctgtctccgcggaataggcgtgttattattgtccggcgcaggcgtcaacacaggatagcctgttcttcgccattctgcccatgcttcatagccattcatatacaaatgcacccaacgctgatacgcaatctgtttaatggcagtagcgggattataagctacttccgggcgtgcgagataagcggcaacaccggtggaagagcccgtccattgattaatggaggcggtaacagcggcattgtaatccagcaatgcagcggcatcgccgccggggacccatcccagcttcgctgcttctgcacgggcaaacagcgcctgcgcataggtcaccaaataaaccgtagcatcctgtttgcggatagccgtgccctggaaagacacattgcccgctggtatattctgcgcctcgtttccctggaggccgtaaggcatgcccacataatcgccactgccggtggtgcctgcatatactttcaaacggggatcgcccagcggcttcatgtaatctaccagtggcttactgatgcaataccatctgcggccctgcacagaatacacgtaataccaatagttctggtaagctgcttctcccaggtgctgtgaaatagcgttgtcgtcgttactggtaaaaatgccatcgctcagtgctgccgcaaattcacgcttgccccaggcaggatctactttcgatagccgcagtgccatcagcgcatgcagggtgcctgccaggcgtttccatttactgatatcaccataatatagcacatcgcctgctgctgcagttttactgtcttccagctgggcggcggcttcggttaattccttaaacagatctgtataaatatctttctggctgtcgtaagcaggatctattttttcacgtcccagtaatgcttctttatacggtacatctccccagcggtctgtgatgaaccagaaaaaataagcccggagtatcctcgctactgctttctgattattagcggacccttcatcttcattaaagtgaacggttttaatgatcttgttcaggttcatcaaagcgtccgcatagaagctggaaaattcaaaggagatgttgatataacgggaagcatctgtatacactttttctgaaagatgctgcacatacaacaacccataaggagtggccatggtagtatccattctaaggatggcataggtaagcaacttcggattggaaaaagtatccggcagattcgggttgcggttaatactgtctgaaaacttggtgcaggatactaacgtaaacgcaagtacgataacaatatataatagcttcttcatgatagtctgggtttacagcgaaatgttaagattaatgccaaacgagcgggtggtggctaactgacctgtttccagccagctgatagacgaccgcccggtggaaagctcggaaggatcaagccctttcggcgcctgctggtaaatcataaaaggattacgtgcaataagcgccacattaatgctgttgaaaggcattttccggtacacttcacgactaaacgtatagcctacacggagttccctcattttaatatagctggcatcatacaaccattcttcatataccgatgtgcccagcaccgtacggtaatacgattttgcgtctacataagcagtcacctcctcccctgttacactggaaataccatttactttcacaccgccgccatctgccagcggatcacgcacattctttcctttatcattaatggctgctgtttcttctgcctgaccggatttaacactcagcatttttgtccagctgaaaaattgtccgcccgactggaaatcaatcatcgccgatacatcaaaccggccgatacggaaactattcagccagccgccggtgaaatccggtaccacgctgccaaaattgtggttctcttcaaacatcggtaaattggccgcatccagtaatattttacccgttttagcatcccgccggtaagcattccctaccagggtgccaaacgcagcgtttacgtccgcattcaggtaaacgcttacccgcgaataggtattcacatccagctgcagggtatttataccgggatacaattcctttaccaggctcctgttcctgctcacattcagcgtggaattccagttgaacacttttgtttgtacaggcatggcagtcaaactcagctccatgcctttattctggatcttaccggcattaatgattgtattctcataaccaatagcacccgacacaggtatgctcagcacctggtcaatattctgctggttataataagtaaatgcaagccctaaacggtttttcagcaccttcaggtccaaccctgtttcaaaggagttacccagcgatggcctgatccccgggttattaagcgtggtaggcaggtgcatggggaggtaggtattatcgtcacgtcctttatacggcgcttccaatatataagactcatagatctggtaagggtccaggtctgatccggccttcgctaaactgatacggacctttccataagagagcggctcccattgcagcaactcactaaataccatactaaaagaaacagatgggtaccaataagaattattacctgccggcaaagcggaagaaatatcattacgtaccgtggcatccaggtaataaatgttatcatagccaaacgaaacagctgcaaacgcactgcgcacctccttcctgcgaagataattggatacatccggccggtcgatggacgcggaaagattatagaaattaacaacagataaaccaccctgcgttcttccctggatgccgttataacgctgcgtaagcaggttaccgcccacgttagcgttaaaactcagtttatcaaatgttttattatactgcgccaatagctcgtaattcatttccttattctcaaatttcgcttcgtagtattcattgatatccctgcccccgtaagccttgcgctgatcaatgctctgcgtatacatatcccctctcacggcgccgcttactttcaggcccggtaatacatcatagcttagtcctacattaccaaagaagcggtcgcgcgtatcgtgattaagattctcgtatgcttcaaaataagggttgttccagtcgctgcccggcttcttcaggaaatcaggatcatcaatatcttcatgattccagtgataaaaagtaccgtcaggatatttatactgcttcaaccggttcatatccagcgaccgctcaaaccactgataaaagttgcgcgaaccctggtaatatccctgggccgggcgcaagcctttattgttggcgtaattgaagctggtagtcaccgttagtttcggcgtcaggttcagcgagccattgaagcccaggttatttcttttgaggtaggtattaggctcaatacccttgatatcagtatgattgaacgacaaccggaaagtggtattttcgccgccaccagacatgctgatgttgttattaaaagtggtacccgttacaaaataatccttgatattatcgggatgcggactaaacggcgtcagcttgccataatcgggatcagcaggatagaaactatacatttgtctcaccggtgttccatccattttcgggccccagctttcatctgtgccggaagccaccaactgctcttgaccgttcacggtaatagtactgaattgctggctgctgcctgcgccatagatgttctgcaacggcataaagttgccggctttttccacagaaaaagcggagttaacatccacgttcacttttctgtttcccttacggccgccttgccgggtggtgatcaggatcacgccatactgtcccctcaatccatataacgcagaagcagccggacctttcagcacattcacggactcaatgtcttcggggttaatgtcctgcgccaggtttcccagatccggaccgtttctgcccgcaaagttattattggaaatgggcgttccatctactactatcaacggctcttcctgcccgttgatggagttaattccccggagctttattttctgcgtgccgcccatactggcgccggatgcacctactacctgcacgccggctattttacccgccagggagcccagcacattctgttctttggtaagtgtaaggttgctgccttttacttcctgtacagaataacctactgctctttctttacgggagatgcccaacgcagtaaccaccacctggtccaggttccgggtgtcctgttttagtgtaacggtaatgttgcccttcccgccggtatttacttctgtggtgagatagcccaccagccggaaaaccagtgtcacatccgtattgccggcgtccagccggaaattgccatcggtgtctgtggaggtgcctttattagtgttctttatctgtacgctcacgccgggcaggctttcacctttttcccctgttaccttaccggtaacaatacctgtttgtgcaatggaggataaggaaaaggtacagtacactaataggatagtgaagaattttttcattgaatagaggttagattttggttaagatatactatacaaaatagcatattaatctcttaatgtcaatagcagggggaagctcctttttcgctttttcttcgtattttcagtagaaaaacaaatcgatatggcaaaacaatctgggttattccaattcaccggtaagttggataatgtgatcggttaccggagaaatgggagctattttgtacgcaccatgccggtcactgtaaaacaaactgccgctacgcggcaggcatcccgtaatttcgggatcgccagcaggaaagcaaaacttatccggcaggccattacgcctcaactggaaatcaaccgcgacggctccctcgtgaaccgcctcaacaaagcattgattaccgccggaaaagatcagtggaaacaaatagagggcttccggttcaacaaacacacgggaatcgataagttcttccccctgcagccggtcatacaaaacgggaggttgaaaatacccgcccaaacattaccgacgcaagacgcccttacacacctcgaaataacagtaattgccacacgaatcagcttcgtggaacggcggatcacccggcagcattccaccaccataaaagtggatatcaacacgcccttcagtggagcagaactggatgcctccatccccgggaaaggcatactattcatcgtattgcaggtaaccgcccggaaaggagccgatctcaccagggaccgccgctttatggccgcagatatccttttcaccagcacaccggcaactaagaaagaaactcccaaaaggaaacaacaaataccggatattaggaaggtattaccatacaaaccagcaaaaataccaggcgctccggcattacgcaccgccaataaacagcaacgggaatgaatcccccactgcataaaacaattaataaaaaaatatccccttaccccccggagccatcgttccatggagccgccatgcgcccctgtaacacatctcgcaaaaaaaatcaaaaatcccctatccaactaccaacaatcaaaaaaaatcataaaaatcaaatcaaaaatcaaatcaaaaacaaaaaccaatcaaaaaactaatcaacataatcagcgtaatcctggttaagacaaaatccgcttcaagtccacctcccatccgtgtacaccgcgtgtatactgtatatacaccgtatccccgaagccaccccaccgcatacacgcaatatttccccagttttccgtaatttaacgcatgcgttatatcactatctatatactcatgctcctgtcctctatcaccaccgtggcacaaaccgtagccccggtagcgctcggctccctgtcttccgacaaaatcaaagaagcctccggcatcgcctccagctccaccctgaaaggctgctactggacgcataacgacagtggcaataaaccagaagtatacctgctcaacagtaaagcggcgctgattagcaccgtgaaactcactgatgcagggaaccgcgactgggaagatatcgcggaaggtataggccccgaaaaaggcaagcactatgtatatgttggcgatatcggcgataactccggcatccggaatcatatccgcatttaccggttccaggaacccgataaactgcccgcggcacacgtggaagttacccccgatgtgctcacgctgcactaccccaacagcccccgcgatgcagagtcgctcatgattgatcccatcagcaaacaaatttatatcctcagcaaaagagaaaaagaaataagcctgtataaaaccagccagctgttctttaaagacggcgataaagctaccctcgagaaattaataaaactcccctacacctggatcacctccggcgatatctccaaagacggccatcacatcgttattaaaaccctcaccaccgtttactactggcaccgcaataccaatgaaagcgtggaacaggccatgtcaaaacctgcaaaagaactgccttatgtaaccgagaaacaaggcgaaggcattaccatcctccccgacaacagcggctatgttaccatcagcgaaggaaaacacgcgcccgtaaatttttataaatggaaattctgaaccgttaacctttattgctgccgtcgcatttcagtaacatcgtctatacttgtatagtgcgggcagccctcattatctgctgctaacccatataatatacaccctcaaaaaaaacaggtaattcccttgcccggaaatacctgtcgtaaaaccattttttctactatgccactaacaaacagcttccaccatttctttgcccggggaatgcctctccggcaggtaatttccgacaggtaattcacaacagctcacctcagaaccatttattcaataacctcattcgctcatgcaaaagaaagctatcatcattggcgctggccctgcagggctcactgctgcctatgaactactacagcgcaccagtatcctccctattgtactggaaaaaagcacagacatcggcggcatctccaaaacggtaaactataaaggtaaccgcatcgatatcggaggccaccgcttcttctccaaatcagaccgcgtaatggactggtggatgaacatgatgccgctggacaaagaagccgcggaaatattctctatcagctatcagcaaaaaacaagagaagtaaaagccgcccgcaacagcaataacaccgataccctggtagctcccgaccccgacctcatcatgctggtcagaaaacgcctctcacgcatctacttcctgcataaattctttacctaccctattcagctgtcagtagataccctccgcaaactgggcttctccaccaccatcagcatcatggtatcatacctgtgggcacagatctttcccaggaaagatgaaaaatcgctggaagacttcatggtaaaccgttttggtcttaccctttatcacctcttcttcaaagactatacagaaaaagtgtggggcgtttcctgcaaagccatttctgcagaatggggcgcacaaaggatcaaaggcatctccatcggcaaagcaatttcgcatgcggtaaaatcagctatcgaagcaggaaagccaaaagacctgaaacaaaaaaatgtagaaaccagcctgatcgagcaattcctgtaccctaaacatggtcccggccagctttgggaagaagtagcccaccaggtgatcaacaaaggaggcacggtgctcatgcagcacgatgtgaaaaagatccgtacctccggtaaccagatcacggccatcgaagcgctggaccgcaccaccggtgaagtagtgctcctggaaggcgactacttcttttccaccatgcccatcaaagaactggtagccgacctggaagcaaatgtaccgggtaatgttagggaaatcgcggcaggattgcattaccgcgactttatcaccatcggcatcctgttaaaaaacctcagcttcgcggataaaagaaccggcgaacacaaaccactggaactgaaagacacctggatctatatccaggaaaaagatgtgaaagtaggacggctgcaattattcaacaactggagcccctatatggtgaaagaccccgacactacctgggtgggaatggaatacttctgcaataaaggagatgatttctgggaactgacagacgaacaaatccggcaaacagccatcacagaactttgtaaaataggactggcccaacaggcagatgtgctggacgccaccgtactcagaatggaaaaaacataccccgcctattggggcacctatgcccgctttgaggaattgaaaagttatatagataccttcgaaaacctgttcctggttggccgcaacggtatgcacaaatataataactccgaccactctatgctcaccgccatggtagcagtagataatatttcaaacggcatcgtcaccaaatcaaatatctggtctatcaacacagaacaggaatatcatgaagagaaaaaataaaaaatccgcagactttgttcctggaaattatctccaggaacaaagtctgcggacaacatccattattaccgtttctcgttatacacgccaaactctgcaatcgcaggcgtttcagcgtaaccgtctatcagtatccttactttattaccccacacacgcggaaaacggtgaatcctcacacgccccgcattttcccctgctgacggcaatggcttccactccccgttctcattatactccagcctgtattgtttaagacgcactttatcttccgtaatcacaatcatgttaaaaccctgctgccggtcgaattccacttcaaaccagggctgcttcaccgcggggttcgactgccacgtacttctgaaactatcgtcgtttgcaaaatccatgatgttcatatcactgctccagctggaattagccgcctggtgcttggcaatattaggagaaataatgggagaggcatacgcaggtaatgccgctaccggcccgtcatttttccattgtttgcccacttgctttaatgtttccagcgcattgttgtcaatcaatccatcccggttgggcgctacgtttaaaatgaaattacaccatgctttattgaaaggaacaatgttttcatttaccagtctgtccacactcttcaccggcgtagtaggaaaatcagctttccagaaccaagcagtattgataggcaaacaggacagcgccggtaaacggttattaccggtggagatatgctggcccgcaccctgctcgtaggatttgatatcggtataaaacaaagcctccgtaggatacttggcggcattcaaatccattaccaggcatttgggctgcagccttttgatcaggccgtaaatttcctcaaaaggaacatcatcataggaaatccttgaccacggcgcgtcccagccgtcgatgatcaacgccgtaatgtcgccataattagtgagcagttcagtgagctgcgctttgatcatcttaatatgctcctttgtaatttgtcccggtctgattttatgatgtgtatccaggatggaataatacagcatcaccttcagccctttcgcacgaaaagcagtggtatactcttttaccacatcccttttcaacgggctgttcattacattataaggagttgttttggtatcccagatggcaaaaccgctgtggtgcttcgtagtcaaacaaccgtaagacatgttcgctgatttggccgcttccgcccactgattacaatccagtttctttggattaaaaatagccggcgatgcttccggatcggcccagtcatcatccataaaagtaggaatattgaaatggataaacataccaaaacgcagatctacaaactgctgctgcaatgctggcagcgacggcgtttgctgcgctcctgcccgccccgttataagtaacagtgctgctgccaaaatgctgataacctgattctttttcacaagctaatgagttaaaatatcaaaaaataaaaagtacctacttccattcgggttgttgcaccaatttgcggccctgatccagtatgccctgtggtattggccatacataaaatttatccgtagtaaaatgccggtcttccagctttgttttaggatacttatttgttttgccgccagtggcaggaatatccgttaaaccggcagatgcatctatggtgtagacaggcccgttcaatgcctgctggccgatccgccagcgcaggatgtcgaagtagcggtgtccttcaccagccagctctatccggcgctcatgacggataaaagtacgcagcgtttccttgctcatactccatccgttgagggcaaaagtggcagctacatcgggcatgccggcacggcgcctgatttcattcagcgcattggtaatatctgcagatggcccggtggcttcgttagctgcttctgcatacgtaagcaatacttctgcataacgaaggatcttccagtcgttgccaccgttatcgcgcgattccagttctgttttatcgaagatcttcttaaaggcgtagccagtgtatgttgctttatcaccgcctattttatccagcgtactgttaataggatcatacatcttggcatttgccagtgtgctgcccgggtaatagatggtggcgtttaaacgcggatcgcggttcttccacggtgcgtgcacatcataggccgggtctttggtgtaaggataataaccggcagcgctttcataatcatctaccagcgaaggcaaaggattcaggtaaagcgtacctcctgaaacggaattcacaccggcaatatcacgcaggccattggggcgtaactcttttacgtggatataactgatgatgctttcagcagaataatctccctcctgctgaaacaggttataataatcaggatacagggaatacaccttgctgtcaattactttctttgcttccgcagcagcgcctgcataatcgccggtatataagagtacacgcgctttcagtccccaggcggcgccctgtgtaaagcggcctttatcatcaccagtgtaagatggcggcaggtccggcgcagcttcatccagccatttgatggcctgggcaatcaccagggctttcttgtcctgcggcacatccgactccgcgggagtagcaaatacttttgtcaccaaaggcacatccctgaaaagcgtagccattataaaatagcggtaagccagtgatacctttacttctgcttttaatcttttcttcaacccctcgttcatatcaggtactttgtccacacgatccaggaattcgaggcaatgcctcacctggtcgtatttccattcgtcgccaagattaccggtggtggctacaaaagtgctgttgccaatcagctgtgcattgcgaagggtatttccccaggaagccgttttggaaaaagcgttgtcgctcattccttcatagcaaacaaaaaaatcggcggaaggaaggaactcatataccctggaagcaaacttcaccgcatccgattcagtggtccagtaggtgtcatcagagtattgatccagcggcgcacggtcgaggtaatttttagagcaggcagccaaaaggcagcaggcgcataatatagtgaagatgtgtagtcgtttcatgttcttgttgttttgcagtgatagcgtcatcagaatttcaggttcaaaccaaaggtgtatgtcttcatttgcgggaagtttacacccgactgccagttgtcgatttccgggtcaaagtttttcgggaaacgtttcgacttcagcgtcagcgcattttccatcatgaaataaaaacggagctggccaatcttcgcacgctgcaaaatatgcgtgggcacattatatcccagttgcaggttctttaaacgtacatattttgaatcatacagccaccagtcggaaagatcgtagttcacgctcaggtcctgacgcatcaatggatagcgggcgcctttattctccggtgtccaggagtccatcaggtcggtggtaaaggaaccgccgtagttgaacgggctcacggcatagccggtgagataggttttgtttttcagcaccccctggaataacatgctcaggtcaaactgcttccaggaaaaattggcgttcacgccaaacatcacgtgcgggtctgcatcacccagtattacacggtcttccggggtaatttttccatcgccgttggtgtcctggtatttgatatcgccggctttattctgcggcttataggtaggcgatgctttcacttcctcgtcggactgatacaggccaagcgctttatagccgtaccaggtccaccgcgactggcccaccatgacagggttttcctgcaatacatccggtgtgccgcccaggtcaaggatcttgttgcgggaatcgtagatattcaccattacgccatacttcagcttattatcgcggttctggtagccggcagatacttcccatccccagttgctcatgcgccccaggttcattacgggggcatcacggccaaaggtcgacggcacactgggcgttaataaaatcccggtggtcttctctttaaaaacatcagcggtaagggtaattttctcatctaagaatcctgcatccaccccgatgttgccggttactttttcttcccaggtaagatccgggttagcggtattgttatagtaggtagtggtttgcgccttatcgttgaaataagaagcgccggtacctatcaggctggcccaggaatagataccacgtgtatccgttcccgttgcattctggttacctactttaccgtaagagccacgcagcttcaggttgctgacaatatcagaccctttcaggaaatcttcttccgaaattctccatccggcagaaacagaagggaagaatccccagcggttattcttgaaacgggaagatccgtcgtaccggccgtttacttccagcaggtagcggtctttaaagctgtaagacaaccgtccgaacatcgactggatcgcccactcatacgcaccgccgccggtagtccactggtctttttccatactgccgccgttgatgacgtgaatatcattattcagaaaatcctggcggcccagggaataggagtcatatttcaggctttcctggctgtatcccagcagggctttaaagtcgtgctgctttacctgtaatccataattaagcgtgccaataaaggtttggttaatggtggtattataatcgtcgttcagtgaattgggcgattgctgggtggtaacgaggttctcctcatcatcatacaacttgtaggtagccctgaaaattttatgtttgatatcgcgggtgttgtaagaatactgtccttttaccgacaggtttttagcaataccgtaatccagggtcaggttggtattaaagtaattgtctttgtaattttcaaatccgccgtgattgataatcgctaccggctgggaaccaccgcggtagcttctgtcgcggccctgcggtgtatacgcccattctgtagggtttaaaatatacgcccagtgcatggcggtagtgtaaataccggcgcctgcaaagcttttaggggcattcatatacacggtattgatcccaaacttcaggttatccaatatctgagtattcacgtttaccctggaggtaaagcgctcgttcatgacgccttctaccagtccttcctgtttcaggtatccaagtgatacaaagtaatccgtattttttgttcctccggagatgccaacgttatgttgcatctggagtgcgttttctttgaagatggcactgatccagtcggtgctgggcaattcgccgctggcgtattgctggatattggcgtcggaaaaacgcacggtggcatcgggattatcgttcaactgggattcattccatttgcgcataaaggatactgcgtctaccagttttgggagataggtaggttgctgtatgcctgcgtaagcatcgtaagcgagcgaaggcttgctgttcagtttacctttgcgggtggtaacgagtattaccccgccggaagctcgcgcaccataaatagcggtggcagaagcatctttcaggatactgatgttatcgatgtcctggggatttacggtttccagctgaccggccacgccgtcaatcagcaccagcacggggttgctggataaagtgctgataccgcggatattcagtttgttgttgttggtgccgggcataccatcggtttgttgtataaacaaaccaggtacttgtccctgtaaggcgtttaccacgttaggcacgggcctttccgctactgcggcgccttttacagaggataccgcgctggtaagactggcccttttctgggagccatagcctactactacaatttcaccgagctttttggtgtcttccgtgagtacgatacggagctgggtatccttaccgctggctatctcctgggtattatatcccataaaagatactacgagtatggcattttcaggaattcccttcagtaggtattctcctttctcatcagtaacggttgccatggaagcatcttttacccggatagatacaccgggtaagggatcgtctttttcatttactaccttgccccggatatctttatacatcaggcccgcatctgcgtccagcagcatgtttgccagcatttcattgctgcggcggatgatcactttatcatctgctataaaatattccaaagaaaacggcgccaggagatccttcagcacattgcctactttctggtgctttgcccggatagtgactatgctgttgaaaatttccttattcaccgcatagctgaaagaaagattggcgctggcgcctatctcatccaaagcatcatgcaatgctcctccttccactttcagcgtaattcttttttcaagcagttgagcttcggtatgcttggccagcaatgttagtgtggtactacatacaacgactacaatacacaatgacattttcattagcatgcctattacaggtacacattttttcatacttttacgtagattaaggttgagtaaaaactagctgccatcggttaccaggccagtgtggcatactagcgttaagacttaactttcagcctcccgcaagggaggttctttttatgtaggtggcgcttctttatgcataggttggtggtttatatcataacgttcagcattccttgtccttcctgatgatgtaagtggtccctttgttttccagtgtggcattgagcgacaaacacagttgccgcaacgctttctccaaagtgccgttggtattaaattccccgaaataaaaacagttggaaatatctcccgtgatctcaatgtttacgttgtagtaatatcccaggtcggccgccacttcccgcagccccgcccggtcatatttcaggatgccttcccgcctgctcagcaagccgttggtagctacctggtcttccttcgtgattttacccgttgccttgctgaataccgcccgctgactgggagatacatgcaccgcgctatccgcgttgcctacagctaccttaccggttaatacggttaccgctacatccggctgcgcatcaaatgcctggatattaaaagaggtgcccagcacccgcgtatctacgcgcccgctgtgaataataaaaggctgcccggcatccgtagccacctcaaaaaaggcttcgccgctcaatgtaagttcccggttccctttcccgaaagcatccgagtattccagccgggaggctgggctgagccaaacaatggtactatcaggcaggagcatctttttatgctcccccgctttagtggccactaattgctgttgggaatgagcggacgtttgcaccggggggcgctggaaataccaccagccggtggctatcagcaccagcacaacggctgctgccgcggccaccttagcccaccagatgcgttttaccggcgctgtttccggctgcgaggttctgatgcgcaataatagctgctgctccatttctgcctccagcagggctttagcgccaagctgcgcttcatcccattcggtggtagccttgaagctgtgatagtaattcattaatgattgcatctcctccgtgctcgccgatccgtccatccatttatctatcaatgaaaaaaactcctgtctgttcataccgggtattttatcactagtgacaaaaaacaaggcctacccccaaagcagggcaaaaaaaattatttattaacaagcaggagaagcagcaaagcatagcccagggcggaccgcagcttacggatggcaatattgatctggttttcaacggttttcaccgaaacattcagctgtgtggcgatctctttgtgggaaagatgttggtcccggctcatccggaatatgatccggcatttctccggtaaagtgtctatcagggtattcagcagggattgcagctcttttacggcgagcttactttccggcgaagcagcttccatccgctccatcatatgatcaaacaactcctctctcaccgggttttgccggatataccggaatactttgtaacggatactggcagaaagataagctttcagggaaacggttaaccggatacgatgggatttttgccacagctctgtaaatagctcctgtaccaggtctttacaggcttctttatctttcagcacctggtaggccgacaagaacagtggttcccagtgccgcttatacaacagggtgagcgcctgttcattacccgactgcagcaacaacaacaattcttcatctgtttgcccctcaatggccggcatggctgatattaattttttatggtgaaggcggaatcccggggtaaatatagagtttaaattattatacttcgggcaaaaaagatgagtggttatttcacgccggccagggtcattttttaattatgaggactacttcaaaagcgtaaaggcgcctttttgcaggagcatctggttttcaaaaccataatacgaatactggataaaatatacatatgcacctattggctgcaatacatttttgtaacgtccatcccaacccattttggtattattcgtttcaaatatcatttcgccccagcggttataaacggccaggtgatatttggctactccatttattcttggccggaaaacatcatttatcccatcattattaggtgtaaaggcattgggaacgtataagttccttacactggatacggtaacatgcagcgtatctgatttaatgcaattcagccccgttttggttgttacaatgtaggtggtattctgtaaaggcattgcaattggattggggcaggtagcacaacttaaactttccgcaggcgtccattcataatcgggcgcatttaccgctgtaagtgaaatcgtttctcccatatttatggcgatgtcgctattaaggatctgcacacgcggatatatattattcaccaggttgatggtggtgtccatactgcatttattaacatccaggatctttaaatcataactgccggcgcctaagttttcaataggggccgttgttggcatgccctcccagtacaaactatacggaggcgtgccgcctttgatgtcagttagtacctttcctgttttccggtcgcaaaggtcatcctctgtcagtaccttcaaatctattaccccgggcgccactatctccaggtaggcactatccaggcaaaccccgttgcgggtatataccatgtatttaccgggaccaatatccgttaaaacaggttgcgactggaacggttgccccttgatagcatactcaaaaggcggtactcctttttgtacatttatggtaatagtgccgtctgttgtggcattacaggtgggcggtgtggaggaagccgttgttttgagcagtctgtcttccgctattttaaccgctaaggtgctggtagtagcacaaccgtttttatccattaccttaaaagtataactaccctgtggcaattgatcaaaaagagggtctgttcccggtgcagcgccatcaatggaaaatgtataaggggctgttcccccggtggcggccagttttattgcgccctgcttctcattacaatcaatatctgtaatagtactgctaacagccacgttatatatgtctacttgtacctggtctttcgcggtacatccgccgttacttacttccacttcataaacaccgggttggtcaactgaaattttccgggtggtttcaccggtattccatttataggaagaaaatccggcgccgccgtctaactccaccattgtgccgtcacatactaccctgtcggcacccagatctactaccggcacaggcaataccactatatttttacaaaaggcgctttctgttagggtaaattcatcctttagcagattaatggtgtaaataccgggctggttataagaaaacaccggaggctgttttgtattggcagagggaatgctggaattattacaattactgaatacaagcctggataaggtattgttataggcattggtaataaaagcatacaggttatttccttcccggaaaacagtagaaatcgaatgggggaagctgaaatttccgttggcagcgatggaagttccggttaacccgaacggcagctggctattgattccatctttgaaatcaattcttaccatactgttgtctcccctgtttactgcgagtgcgaatatattaccacaatcgtggatgagggacaggtcgcggggactattcaatatattatccggattaccgagatttacgccagtgggcgtattggaaagggaggtgcccaaatccagcctggtaatggaggaagatccttcattggtaacaaataaatgccactctccgttttctttcatagcaaaaatgccggtaggatgatccattaccccaagattaccaaaattggtagccaccggtatattactgaacgagttaccaaattcaaacctggtaaccgtattgttataataatttactgtaaatccataccagttcccactttcctgagtgatatacaaatcaaccgggtaatacagcgaacctatatttccccaatctgtctggctaatcactgcgttagccagtgagttacccagatcgagttttacgatctttgcagtgccgggatcattgccacctactattatcaaatgccagccggtagcatccttcaccacctgcaatccttcggtagtattggtcagcaatcctccaaaagttccaagatcctgtgaaaccggcgtattcaataaactggtaccaaacgatagcctcaccaggttaccaatgttattggtgtaaaaagcatagtaattagccccctctttcgcagtcaccaaaaaaacaggtaaattcattagtccaccaatgtttcccaggtttgtaacctggggtggattatataaccccccggaacagaaattccacaggaaagtattccctccaacagaagtgttagttatgttgaccggcatatttacacaaacggtatccggcgcagtgaaactggcctggctaaataattgattggatatcaggttaaaaactatgatacaaaataaatacagggatatacgcatcaaactatcgggctaaatttaactcaagctactcaaccttcccgaataaaaaaagtgcctctgtaaataatataccgccgctaaccgttcctgggctcctccggcgatttaaccatccggaccggtaagggttccattcctcctcctgacctctaaacatgcttaacaatttcttaaaatgcctctgccagccgatatggtaactttgagtacaccggatcgcttatacatgaaatggataacagggatgccatcttacaattataccaaacacattatcacacgttgtttgctgcaggctgttatcttacggatgacaaggaactgatacgtgactgtatccaccagctgttcctccattgctggcaaaaaaaagatgagctctccaaaatactgcatctgaaaaattatctcaccgttgcattacgcaaccggctgttgactgccttaaagcagcagaacaaaattattccctacgagcccggggaaatggatggtatagaatactcttatgaagaaatactgatacgtaaggcagatgaaactgcgctgcaggaaaacctgcagcgcgccctgcaaagcctcccgccacgttacagggaggtgatagagatgcgttttttccgtcaatacagttacgaagatattgcccgcatcaccggccagccggtaaaaactacctataattatgtatatgaagccctcgcaatgctccgtaagcagttgaaggcaaaaccctctctcccatattaaggaatcgttaactccatttttctttcatggaaatttctccaccttctttgtcctactaacggaacaataaacattggatcgttggaagaacaatattacgcgctgccggaagattttttatcagacatttcgttctgcaactattgcaaaggtgcgcctgaaaaggatgtgcgttactgggccaactggcttaaaacgcatccggaaatggcacacgtattccgggaagcagaacatctatacaagatgataggcatttatgatgaaggctaccaacaggctttcgagcgcttcagcaatgagatccatactactatacagcctaaacgccgctggctcaatgtacgcaatgcagtggctgcagcatgcgtgctggtgctggcatccgcatcgctttattatactctgcgtcctgcaggcagtacttttattgcacaaacaaacaggccgttatatgatacaatagatgccggcattggccaggtgcgcagcatacagctggcggatagcactacaatagtgctcaacagccattcgcggttgctggttccaactgattacaataaacatcaaagaacggtagtgcttgcagaaggcgaggcattctttaatgtaacccatcatgctaaccaccctttcactgtaaaaagcaaaggggtggaaaccagggtactgggtacttcctttaacgttcaggcatatacggaacaagcaggcatgcgtatcacgctgctcaccggctcagtatccgtgcataccggcattgcgccaaagcccatcctgctaaagcctgatgagcagctaacaattgccgctaaccgcacttatgccgtacaaaaggtatcagccgcccggtacagcaaatgggtgaacggtgaacttgatttctacggccagtcattgcaggatattaccgccatactctccacccgttatggcgctgcttttgtatttgaagatagtatatgccgcaaggaactgttcactgccacctttgataaaggcatgccgctcaaaaaggtgttggcgctattaagcaccaaccgcaacatttattttgtacaaaagggagataccgtgctcattaataggcgataacaaacattcatattcatttccaggtctgatattaccgcagctttactgcggctggccgcttattgtcccataaaaaacaaatatgcatcagagaactttacgcttttgcttaggctggctcctgctatccctgctaccttcatttgccgcgaaagctgtcgtggaacagcaggaaacactcgaagctgtactaaaccgtattgcagatcataccggttttcactttatctatgatcccgccattgtgaaacagaaggtcgtaaccattcctatcaccgttaccggtcgaacaggtatccgttcctgcctcgaccggctttctgccaacaccgccatgcagtttacaattgatggcaacaacatcatcgtatccctcaaaccccaggtggtgtatggcaggataacgggccgcatagtggatttcgaaagcagtgagcctttgatcggcgctaccgtaagggtggccaatacttccttcgccactgtaacggatgaaaaaggatactatacgatcgataaaattccgcccggtaaatacaatcttatgttcagctatgttgggtacgaaaccggcagcctgaacggtgtaaaagtagagagcaaaactaccttacaggccagttttaagctacagccgaaacgcggactgaaggaagtagtggtaaaaggtatttcacaccgtaaggtcatcaataccaccgatgcgcagctgatagatgaggtacgccaggcccgcagtgtggtatccggcatctccaatgagcagatctcccgcagcatggatcgcgatgcggctgaagtggtgcgtcgcgtagccggagtgaatatcacaaacgaccggttcattgtagtacgtggacttaaccgccgttataatgtcacctttctgaacgacaacatcgcccctgcaacagagctggacagcaaagcattttcctatgaccagattgccagcagtatgatagaccggatcttaatttataaatcacccgcaccggatcttcccggcgattttgcaggaggcgtcgtaaaaatatacaccaagaaaagccagctcacacgtcaattcgatctgcaactctctgctcaataccgccccggctccagcttcagcaatatgtctacctacgcaggtggccgttacgacgcgcttggattcgacgacggtacacgcgcattgcccgcaggcttaccggatttagtaacgttcaataccggcgccccgaaagataacgcccgctactggaaagcctttcccaataatttcaagtccttcaaggtgaaaaccgatctcgataaacggatactggcgaattactacgatgcctggaaaataggccacaagtatattaacaacctcacctccattgcttataccaacaccacgcaaaataataccataccagtgtacgacagccgtaatgccaatggctcggaaggcgtgatccgcagcggcacgcaatccgcacgtatcaccctcatccagcaaaacaccctgcccgttggcgacagcgcacacctggaattaaagcaatttgtgaatcagctgggcaacaaacaaatgatgtcgtatatcctgtcaagagaaagtgattatagcggtcagagtaaagacaaccagctgatatttcaaagcaccttcctctacaccgcacaactcagcgcctactggaacctgaagaacaaaggaaacacccatcttttcgccaatacaggttatactcttgtgcgcaggaacgatcctgatacccgcgaaatatggtaccgccggaacagccaggacagtacttaccctgaacatatcgccggcgatccctggttgataggcagtgcggcgcaaactttcggcatacgccgcatttacacccgcatcaacgaaaataccgcacaggccaatgcagaggccgagcattggttgttaccctggtggtctgcaaaagcgggattctttttcgagcagaaggaaagacgcgtgaacttacgccagttcggccttaaccagggcgccgcatataatggtgattttgaaaacggccatatcggctatcagctcactgaagaaatgctggatcattatatgtcgccggacaatttccggacagacaataccggtcatacctggtttgaagaaaccagcccatacgacagctactttgcagataaccgtaatctctcctacttcctggctacagacatccgcatcccccattccaatctttccatcttcggcggcctgcgggtggaaaataatcgtctccggattattggcgcactaacagccggccaggccaattatcctttagtggtaaaaaattcccgcacacatgcccttccctccataaaccttaactggaagcccgcagaacgtatcattgttcgggcgggatacggcaaaacccttaacaggcccgaattccgtgaagtagccccattcccttatgcagatatagaaaactacctgatgtatgtaggtaacccaacgctgcagaccgtgaatattgacaactatgatatacgactggaatggtatcccgaaagcatgctgaaaaatgaaatgtttaaccttggcttcttttataaaacactggataaacctatcgaacaaatcctgatcagggaaaactactacgcatcgttcatcaacgagataggctttatcaactctggcccaacaaaagtatatggaatagaagcagaaatgcgtaaaagtctcagctttataccgggcgccttgttccgcaatctttcctttatgataaacggggcgtggatacatagccgtgtagatatgcagccgcaaggttcagatggtaaccaggtaggccgtaaacgcccactgcaaggacaggcgccttatatcctcaactcctcgctcaattatgaagatccggccatcggcaccaaaatatccctcagctataacattaccggcccaatgatcctgctcctgggcactaacaaccaccggcccgacgaacaaattcggggtataccggatgtaatgcaacgtgggcaacacctgctggattttacctggagccagcgcctgaacaaacatatgcatctcaaagccggcgtacaaaatctgctggatcaaaaacgggaattattcctcgactttaaccgcaactataaatacgatggggtagtgaaagaccgtaataactggacaaaagacaggccataccagcttttcagcccacggccttattactcacttgccctcaattttatttactaacccggatcaatcaatacatatgaatgagataaaatacttcctgctactattactaccggtatgcttttcctgcaaaaaagcattcgatgaagagctgaactcacgggagagggaatcaggcattgttatggcagccacgaacacgcccggtatcgccatgcgcggagagccactcacattgtacgtaaagctcggtaagccggatgccgatctgaagatttttataggcaatgccgaagcaaccgtgctcacgcacggacaaacaaagctggaggtgcccatatccaaatacacagacgataaagaaacgatcgtagccgataccttcagaatgttagtccctgactcctcacagatcggcgaaaccagtatctacattatagtaaacggtatcaggagcgcacctttcaaattcaccgtaaagaaaccggatatcctgtatccaggcgacgtaaccgtaacccccttgctcatgacacccagcgccgagcgtgaacctatagacggaccggtgggcaccgccaccgttggggccgtgcacgatataggcatggataaggagggagccatttatttcattgataacggcgcctacgattttaatcccgagcatggatataacagacgtaacatgatcatcaggaagtttgcaaacaaccagatcgtaaccctcggtggcggaggtaacaacgaatttgcgacgcagttgagtgatctgaaactgaacagcatcgatgctatgaggattgctgaagatggcaccatctatcttgcagtaaccaatgcaccattaagccgtataacactcccaggcaccacagaggtaatagaattcgaatttcgttttcatcgcatactgaagatcaatccccgcaccaatgaagtgaaaacgctggtgggacgtaacgacaaatattgcatagataacggtatggtctacgaggtgatcatggacggacctgctgataaggccatgataggtgctgtaagaggtatggaactggataaagcaggtaacctctacttcctggatggcggactaacaggaggaggagccgtgctccgcaaaatatctgccgatggcatggtgaccacagaagccggcgcaatagacgacctggcggattacgtgttctataacaacgatggaacccacccggaaaccatgaaagccggcgctatcgtgaactccggcagtaatacagtggacggatttggttcaaaagccaggatctgctcccccagaggtattgtgctgggaggaaacggcaaaatatatctcgcgcaaggagcaggcagcgctgaaatgaaagaatgcgtacgggaatacaatccactcacaaaggaagtgactaccatcattggaaagcctgtcaacgcacccgataacttcctttactcaggcacctttaaagaagtagatatgcgcaccattacttcttttgatgcagacttcgacggcaatattcttatcgggtacgatgagcagatctatgtggaagaaccccgtggtatttataaaatagatgtgaataaagaaatggtgtacaaaatagccggttataaaggagcttccgatgccacaaagccacagccgggccaaacagctatcgtaggtgcggtgagccgcatcctgttcgaccagttcgggaaactatatgtgggctatacccgatacgatttttttgaccagatacatttgtccaccatctccatcaccaggtaataaatcatttaactatgcgaaatatctttttcagattattactgccggtaactttttgctggataacggcttgcaataagtcaacagaagcacccccatcacctgacattacccacctgatgatttataatggcagcacggcatttatcagtaaactaagccaggtgtttgtagataccgcctttataactgccagggcctacaacgatatcgatggttccggaatgggcatgtttaacaaagccagttacaactgggtggctccgggcaaacatcgtatcggctttactgataccagtggcaaggtaaagattgcagaaaaatacactaccctcacaaaggatacctggtatactttttacctggcagatagtttaggctattaccaggtgctgatgtctgaagaaaatatggcagatcgcccggaacacaaagcccgcatcaggttcgtgcatctctcacccgacgccggaccgctggattttttcattgatacggtaaaagtgcccgggatggatagcctgacctataaaaccatcaccccctttatagaaataactccggcagaaaatccgtctttccgggtaaaaaaaacaggtgcagcgaaagatgaaccacacctgctcagaaaggcgtttgccacgtatgcaggacgttcctataccttcatcttccgtggatacatacagcagcaaggagaagatcccaacaccaccatcaatatgtctgcaattatcaacttttaaacatttaaaaatgcgtatagtctataccgttataatacttggaatactggcatcctgccggcaggacaaagatgaggtccctgcactgccaaccccggagatcacggcaataagccgcgaaactgtgcaatcgggcgacacgctggaactctccggcaaaaaccttcaacttcccgactattccacggaagctttcatcggtgaccgccccgcacgcattatcagtcaatctgatactaaattacaattgctggtacctgaaaaagtattcaccggcaatatcgttgtgcacataggtccgcaaaccacgctgtggcctgaagtaaaagtgatcggctctccgaaaataaaggctgccaacccacgctatgcctatgccggcgatacgatcctcctcaccggcgaaaacctcggtaacgacccctcgatactgaaaatatggctcgacggcgtgcccgttaacattgtcactgtaaagcctgataccgcccgcatcatcactcctgccggaacaggcatacgtgcagtactgagctggcaaacctacaacggcccaaagtacaagcaagacgatctgaccgtagcagtaaggccggcgaacatcgttgctaacagcattcttgaatacctgcaaaaggatccgggaatggatcttaccggcgcagtgatggattacatgtcgcttacacctgctaacaaaagcctgaacgatacactgcgtcaatacctcaccggccagatcccctgcatcatgttcctgcctgataacattgcaatgaatgcaataggtatttaccagcacagcgatgcgcctaatgcgggtcttaatttcaacgccttgctgaacggcgtattgaaacaaactactgagccggagccggacaagctctatccgtcggaatatacaaactatgtgtacgaatacttcgatggctttcccgactggcatgcgtttattgtgatcagggaagtaagtggccagcggtatgtgctttccaccatcaacactgctgcagaccaatccatctccgaatatggcccgcagcggcgtatcatcaggaagcatcaatgcggcaacagtataatatacgaaatagatggacctatgacttttccgatcggcaactggtaattaaaacagcgatggcgcctttctaaggcgccttttttatgttacatgcaacgatcttactaagaacctacaagatcgtgcaaccattgtgggattaaagcttcattacgcggaaaggttttcagatcatcgataaatttttcattagacggcgtatattcaaattcaggtttattgtcataatcaaattcagtttggaacttcccggtattgtccaccgtaaaataagcggaataccaggcgccattaccaggagagagccggtacatttgttcgcgtagggattttatcttcatagtaatatcattaccattttcttcaggatcaaatgaaagcattttgccgccttcttcgcaaaaggctccgatttctatcattttgtttaatgcctttattgtaattgaaagactatcccaggtagttgaaggtatattgtcgcaagccccctgaatgatttccctgattagttggttcgtctgttccataacttgtttgtttgctgaaaaatattgatttctttagttatgcgggtactaacttaacttttcaacctgatcatgcagctcctggtcccaaatgaattccatatcaaattggccatcaggggtcaatgtaaaaattgctttgttccatttgttattgccaccttctgtagtaactttatgtagttcgtttaaccaatctgtaatatcatcatcaatgttttctaccgacatatccttttgctcattgtttgcaaaataatctccggtataaccaacaacaccattaccaacaatctcaatttccaacctggcgttagtccaattcccgctttcaataacattagagatttcctggccgatttttaaataaatttcgtctgctgtcatgataagcattttaattattgacttcttttggatattcttcatccatttagaaagttaacaatttaatcgggtatattcttgacgctggaataattattgttggagcctaaaaacaaaagagagaatggaaataattccattctctctaatttggttgcccaaccaggattcgaacctagacaaacagaaccaaaatctgtcgtactaccattatactattaggcattgttcaatggggatgcaaatgtagtttttttctctatgaaaacaagtatttatcttttcctcctgatagacaatgccgcgatacccactgccacagcgtcttccaatccgcctaccgctgcatcccttacgtgtagtttcctgccggtagccttgcgtaaatagaaaaatgcatatgctgcggctactgctgccacgccgccaatcagcgcccctttccaggctttctcaccttttgcctggtagatcgtagctcctgccaatgcaccggaaagcgccctgcccgtaataccggtagcggctatacgatttggtgtacccggtgctttatctatcaccagttccccggcggccatggtttgtaaatagcgggaagtcacgtttttttgcataaaccccaaaggcgacttacgcagcttttccgaaggttgccggctaacaaaataactggcaaaagcggggcccatcgcgccgcgcattccggtaacaatacccaggccaatagcccggcaaatagtaggtatcatagcttttttcataccgcagcagccgcaatcattgtgccatccatgccgctttgcttctgcccgctgcggcatggatggccattgaaatagtaagctatcgcgctgataagcgctgatggtctttctccagttgtgccttcaactgcgcataatccacttcctgtaccgccttgttcccgttaatggccagtactgctgccgtggcagcactctgacccaggatcataaacaccggctccatccggatagagccataggcaatatgtgacgccgacatgcataccggcaccagcaggttactgcactcttcccgctgcggaagtatggacccgtaagatacctggtaaggctccttaatatccacaccgatgtcgccttcattctgcacatacccgtcttttttcacataacgttgcgcattatgcgcatccagggtataggaacccatcccgatcgattgcggcacaggactttcgccaagtaccgattgctgcgtcatcacatgcacgcctttcattcgccttgcctcgcgcacatacagctggtgcggccagttcttgttgtcgcggaattcatcggccgacaatccccatgtttgcatgcgttgctgaatagcggccggcacacgggcatcgtgtgcaaggaaatataataagccctgctgatacacttcatgctcatggataatctccttccggcgttcatacgtagcttcaggataatcgtagttcatgccaatgttatcaaaactaaagggaccgtgattgttcacatctgttttatggttggggatgggatcaaacttattgaatacttcgttccaaccgctgtccagcacacggatgagtaattcatactgcgtggcatcatatccctccggctttggaaaaggaatgcggttggcaggcttatcggtcaggcacatacggaaacaatatgcctggatctttttatctgccgctcctttttcaccggggtcttcgccggaaacacggggcagtaatccacttttcgcatcaccgggaatgcggtacggactaatgttttgcttgaaatgatgcccatgatgtaacacaccggtttgcacgccgttccagctttcgccataagtggctactgcttcgcgtcctaccgtgtagcttacgccggcagccgccatcaggtcgccttcataggtggcatcaataaatactttaccgctataggtatgcccgctcagggtagtaattgccgttatctttcctccttccttttttacgccctgctggcgatccagccattcgtcgcggtaaatcttaatattattctcccggatataatcttcaaatacctgttctgctacatgcggttcaaagatccacatggtgcgctccgtaccatccattgccggcgtgccctggcctttattgccatactccgcctgctgttgccagttccaggcggcaagttgctggtagtgcagccagatgcggtggtaaaagtcgcgggccagccccccgatgactgatttattgccggtatcggtaaaaccaagtccgccggccgaaagaccgccgacatgtttatccggcgatactacgatcaccgttttacccatcttatgcgcctgcaccgcagccacaatcgcggccgaagtgccgccataaataattacgtctgccttatccaccggcgctcctgcccgggaaaataaataagggatcaccaggatcgttgctaacaggactatttttctcatgtcataaattttttaagatatgcgggataacttttctttcctgatactaaacgcggaatggcaacaaataaccactgtattataattcttcacgtggaatccagctcgcgtggaaagtaaacggcaaaactaaatttacaatttcacacggtaccctgcaaccggctaaattatcatgattaaaaaataaaacatcagatgtttaactaaacatcatacctttgtagggtaaatgaaaatttatggagcaaccatccaaattgtcagaccgcgtgatcaacgccatccagaaagatatctcccaggggaaatataaacccggccagaaaatacctgcagaacccgagctgatggtacaatacgccgtaggccgctctaccgttcgtgaagccattaaaacactcgccatgatgggcatcctgcgggtacagcagggcgcgggtactttcgtcaatgaaaccgtgcaggcggaatcgctggaccagcggctcaggcgggccgacttcgaagaaattaaccaggtaaggcgcatgctcgactatgaaattgtgaaactggccgcagaaaaccataccaaagaagatctccaccagctgaaatcattactggaacaacgcaaaaaggccatcctggaacaagcataccaggaatgcctggatgccgacatcgcctttcacaccgctatagcaaacgcttcaggtaataatgtgctggccgatctctttcgcagcttcactgctgtaatccgcgactttttcactaaacgcgatacgcaaagtatcagtcactttgccatcagccaccacctgcatgaacaattatacaaagccattaaaagtggcaacgccaaattatcccggcaggtaatggaagacatactggacaataattattaaatatcaacagatgaatatcctgatctttagcttaatactcctggcgggcgcctatgtggccgggcttttaggctccctcaccggcttgggcggcggcgtgatattgattccattactcacactcgtatttcatgtagatatccggtatgccatcggtgcagccctgctggcttctattgccaattcttccggcgccgccacggcgtatataaaagaaggcattaccaatatacgcctgggcatgttcctggaaatagccaccaccgcgggcgcggtgggaggtgcgctgctggcaatattcactcccgtaaatactattgccatcttgcttggggtagtgctgatattttccgccgctatgaccatccggaaaaagcatgaacatgcggagcaaacgggcagtaaattatcttatctcttaaaactaaacagcagctatccaacacccaccggggaagtgagttacaaacttaaaaatgtagccggtggcttcagcatcatgctgatagcaggtgtgttatcaggcctgctgggcatcggatcaggtgcattaaaagtactggccatggatagcaccatgcgcattcctttcaaagtaagtaccactaccagcaattttatgatcggcgttaccgccgcagccagtgcggtggtataccttcaacggggctatatcgatcccggtatggccttcccggtggtactgggcgtattgggcggagcctttaccggcgcccgtttgcttaccttcatcaacgcacgcacgctacgcatcatcttctgcgcagccatcacatttgttgcgctggaaatgatctataacggattaaatcaccagttttaatgaggatgttatgaatatatttaagaaaatgctcggcgaccgcgatatcgaattactcatcggtaaacaactgagaaccggggtaattaccgccagctgcattgcattgctgggaggcatcttttacctcgtgcaacagggcgctgccagcgtaccggactattcgcactttaagggagaagacgcggaatacacttctttccggggaatttttcacggcgtagctacgggcagcgccatcgagtttatacaactgggtgtactggtgcttttggccacacctatcctccgcatctttttttcactgatagcgtttgccgtggaaaaagacaggctatatgtgtttattactacgttagtgctggggattattttgttcagtatgttcggcggactgaaaatataatactattcttctctcaaccgttcatcggtatacgtaatggctgttctgccatggggaaccggttttcccagttcatccacacttacaaataccattttatccaccgtaagaatagttttttgtgtaatcttattccgcacctggcaggtaagtgtaagggatgttctgccaaaatgcgtggccttaatacccaattctacaatatcaccctgacgggcagaattgataaaattaatttcagacatgtacttggttacacatcggttggtgcctaactggatgatagaatatatagctgcttcttcatcaatccaacgcagcaaactgccgccaaataaagtgccgtgcgcattcagatcctccggctttacccatttccgtgtataaaaattcatgacctgtataattttatatccttctctcttatttttttggaagatgatgacgttattttatttcccccttcggaggcatttcagcctcattatgcagcttcaccggtttctcggaacgcgattttaccttcaggttcagcacctcgataaatacagagaatgccatcgcaaaataaatataccctttcggaatatgctgatcgaagctttccgctaaaagcgaaacgcctatgagcaacaggaacgacaatgccagcattttcaccgtaggatgcgtgttcacaaaacggctgatagattctgatgccagcagcatgacgcctactgataccactaccgcagcaatcatgatctcaacatgatctgccattcccaccgctgtaatcacggaatccagtgaaaacacaatatccagtaacaggatctgcacaatcacctgtccaaacctcataggtttggcgttggcgacgccgtgttcatctccttccagtttctcatggatctccgcagtacttttataaataaggaataaacctcctaccagtaaaataaggtcacgacctgaaatggccagctttccaagccactccgtattctgcacaccaatccagtcgccgatattaaaaagcggttttgtcagcgacataatccagctgatcgacagcagcaataaaatacgtacaaacatggcaagtcccagcccgaggcgacgggccttcttttgtttattttccggcagtttccccgccaggatagaaataaacacaatgttatcgatccccaacactatttccagggcggttaacgttaacaggctgacgagcgagtcaacggtaagcaggtgttccataattgacagttatatagattatgtatgtgcaaacccgaatatacttccttttttgatagtgatgaaatctgctaaacacgtgctaaaaacatttgtcgtaaattgcagggtacatacactgattagcacttctcccctcctgctcgttttctgtatcacaacacgttttctgattaaaataataatatgaaaaaagaggaatggcatatagtgcgctttgcttcgcgcggtaacaacagctttattgaatctgcaaaggctgcagtacaggattatttttccgctaacaacatctctgtgtatgccaacagggaaatgtggattaaaacgatcgtaatgctcgccttatattttgtaccctatacattgatggtggtgggcctcggcgcaggaagcgtatggctgtacctcggtttgtggctgctcagtggtctgggtgttacaggcatcggcgcatccattatgcatgacgccaatcacggctccttctctcccaaaaagagcatcaacaatatgatgggacatatcctggaaattattggcggatatgcgcctacctggaaaatacagcacaacgtgctccaccacacgtataccaatgtgtccggtctggatgaagatatagacagtattaaactgctgcgcttctcccctaatcagccacgcgcctggtatcaccgttaccagcacatgtacgcatggggcttttacatgctcatgacccttttctggatgacagcaaaagattacctgcaggtactgcgctataaaagtcatggtctgctctcaaaacaaaaagttacgttaaaacaggccatgttcaggatctccgtattcaaagtattttactacggatatatcctggtgttgccgttaatattttccggaatgccctggtattgggtgctggcaggattcttcctcatgcatttcaccgccgggttactgctggcctgtatcttccagccggcgcatgttatgagctcttccgggtatgccgctcccgatgcagacaggaaaatgaaagacagctgggccattcatgaaatggaaaacaccaccaactatgcaccgcgcagccgtgtattatcctggtgtatcggtggattaaactaccagatagaacatcacctgttttccggcatctgccacgtgcattaccggaaactggcgcctattgttaaagaacaggcggcagcctttaacataccttaccaggttcaacctacctttatacgcgccctgtgggaacattcccgcatgctcaaaaaactgggccgtcattaaatataaaatggggagcaccgccaccggtactccccattttatttatattcctattaggccagcccctgtacctgttcgcggtaagcagaaggactcatatcatgatatctcctgaaaaatttattcagatgactctgatcgttaaatcccagttcataactgatttctttcaaagaaaaaacactgtaatgcaacctgttttccagcaattgtaatttatactggttcacataatcccgcagcgtagtgccggtttgctccttaaaaaaagcccccaggtaatgtttggaaaacccaaacaactccgccagttgctctacctggatatcatccgcctggtgaatatgctcgtgaatatagttcaggatatgcgttacccgcgcaccgcttttcgggcctgcctccaacaattcatgatccgccacctgtttgatcatggtaaacaacgcctgcaacaaaaagaaaacagtatcactgctttcctgcccggcagctttccactctgccgccaccagctgtatcaatggctccatacgctgaatacctgtcttcatcattttcttttgccgtgcctgcaataacaactgatccagctcctggttccagctttgctgcagccgcatattgccggcgccatgcaggtacacattggtaaatttgataaaggtaaacaccgtaggcacggtaatctcaaaatgatgtgcatcacagggcgccagcaaaaacaaacacggcccctcatacgggatattcatccccgaaatacaatgcgtaccgctgcctttatgtataaagatgagctcaaaatgattgtggttatgcaccggatgctcccattcccgggcagtaaagtgcgacactttcaggtattcgtgttgtatgtatctcttcattctttaaaatataccaatgaaccccgcggatgtacaagtaatcctgaacccgcaacgctgatctttgtaccgttaaaaatacaacacagatatggaacagcataataataagaaagtagccctgatagcaggcgcacagggagtaataggacgcaatcttatcgattacctgcttacgcagcccaactgggatatcattggtttatcccggagaggtggtactgatacggccaaagtaaaacacatcgcagtagacttactaagcctggaaaacagtgaacagcaactgaaggcacttactacggtgacgcatatattttacgccgcctaccaggaccgcggcagctgggcagaactggtggcgcccaacatgaccatgctccgcaacgtgattgaagtggtagcccccattgccaccaacctgcaacacatcagcctgatgcagggatacaaagtatacggcgcccacctcggtccatttaaaacacccgcgcgcgaaacagatgcaggcagctttatgccgccagaattcaatatggaacaacaacgtttcctggaagcatatcaacagggcaaatcctggtcgtggtccgccatccggccctctgtagttggtggctttgcattgggcaatcccatgaacctcgccatggtgatcgccgtatacgccgctatttcaaaggaacttggactgccgctgcgcttccccgggaaaccaggcgcctacgataaactcatggaaatgaccgatgccggcctgctggcaaaagctacagtatgggcagccgaaagtcctgccggcgccaatgaagcctttaatatcaacaacggcgaccttttccgctggtctgatctctggccgcgcattgcccgttattttggcatggaaacagctgcccccctgcctatgcagctcgacgtagtaatggccgacaaagagcccttgtggaatgccatgatggaaaaatacggattgcaatacagttatgcggaagtatcttcctggaagttcggtgactttgttttttcgtgggactacgacttttttgccgacggcagcaaagctcgccgcgcaggttttggagagtttgtagatacggaagttatgttcctggaaatctttgaaaattttaaaaagatgaaagtgataccctgaactatgctttctccaatgtgaaatttacagcagccgtaaggcgtttcatggcaatagccaactggttttccaccgttttaaccgagaggtttaaaatggtggctacctctttataacgaaggtcgtattgctttaccaggatgtataccattttgcatttgggaggaagctgttcgatggtatgctccattttgcggatcatctccgcagaaatcatcagttgctccggatcgctttcaaaggcaatttccagcttatcttcttccgcaaaaactacctgccgggagctggcctgtttgcgcatatgatcaatcgctttatttttcgctaccacaaacaggtatacctgcggattttttatgtccgtcagtgattgccttttttgccagcaatacataaaaacatcgttcgttatttcttccgccacctctttattacgggtaagcgaaaaagaaaaacgtaacaacttgatgaagaaatgatgatagaaagctttgaaggccgcctgatcattgttcaccgtgatgtttttaaataattcattgattgtacactgatccatcccttttaagccactgatattggttgcaataatatataacgcagattacgctaaagttaacaaaataaattatcccgcaatttatttttaagatcctcttttggggagcctggaatgctgatatctgcccggattccggggaaagaaaaaatttgccggtggctttgggggtttttcattttcttttcgtccttctgatataatatggataaaaataaatgatcgagcgcaaccgggtaaatatattgatggccaggaaagtatcgggagaggccaccgcagccgacctgaaagaactggaaacattgctgatgcagtttccggagctgcagtacgcctttactattgtcagtgatatcagttccgttaacagtgccagggggttttccccggcggaggaagaacagctggccagcgaaggaatggaccgcatcaacctgttccttcagcaggatcaggagcagcctcccgccaaacggctgattccctggcggatgatcagtggtattgccgccggcatcgccctgctcatcaccgcgtattccctgtggccggtcatgccgcgcaaacaggctttccgcaatgaggtggtcaccaaaaccggctctaaaaccagcgtggtactccctgatggcaccagcgtaatactcaacgcctgcagccgtctccagtacgacgccacccgtttcctgaacggcgagcgtgaagtgaatctgacaggtgaagcctactttgatgtaaagcacgaccccgcgcacccgttcatcatccaatccggtaacatcaatatccgcgtactgggcaccgtatttaatgtaaaggcctatacagaggatgctaccgtggaaacaaccttactcagcggaaaagtggaagtgaacttcccggataacgatcattccggaacgaggaaaaccgtacaactgcaaccggaacaaaagttaatcatcggcataaaagaaaacaaacaaatacccgtaaacagaaaaaccaattttagcattacaccggtaaaaacaatcgctgttgccggcgcccctacaacagcggaaaagccagccaccgcctgggtgaacgaccgcttcgacttcgacaatgtcacttttgaacaattgtcgcacgacctggaacgctggttcaacgtaaccctgcgttttaaaaacgataaatataaacacgaagtatttaccggcgcattccggaaacaaagtattgaagatgtattgcaggcattacaactgatgtctggctttcattatgaggtgaacacgaaagaaaatgttatttacatatggtaaaacacaacatccaaacgtcatctatggcttgataatccactgatttttcttattgcagacagcaaataaaaaaagggaaatgcagcaacattcccccttttcaaaatgctggctgaacaatgtaaaccgatttccttacgatctggtaacggctcattatttaacctaacgaaacaaatttatgaaaaaaagctattggtggccttcccatattccccagcggaatatgaggaaactattattgcgtatgaaactaacctccgtattgctttgtgccgggttcttacaactaagcgcacacgggttttcacaggaacggatcagtgttaattataacaatattaacattggtaagctgctgactgtcatcgggcagaaaagcgactacactttcgtgtacaaaaacgccagcatccccgaccggaaaatctctatctccatgaaagacgctccggtagcggaaatcctggacaaggcgctcgcgggcacctcgctggggtataaaatcatgaaagataacctggtggtaatcctggaagcaggtgaaactgcacagaatgttcatataagaggacgggtaaccgatgaagccggcaacccgctgattggcgttaccgtgctggtaaaaggtaccacccagggcgctaaaacagataacgaaggccgcttcaccctggaagcgccggaaaatgccatcgtggaatttacctacgtaggctacgaagcccagcagatgaaagcacgcgaaggcgctacctttaacatctccctgaaagccaattccagcggccttaatgaagtagtggtagtgggttatggtaaacagaaaagggctaacctcagcggcgccgtagacgccatctccggtaaagagctggaaagccgccccatcgccaatgtgggtaacggcctgcagggattattgcccaacctgaacattaccaacgacaacggccgcgtatcttccgcaccaaaattcaacctgcgtggtttgacttctatcaacggcggcgacccattcatcctggttgataacatcccctttaccagcgacgaagtatcgcgcctcaatcccgccgacgtggaaagcgtaaccaccctgaaagacgccgcctccgccgcgatctatggcgcccgcgccgctttcggagtagtactcattaccaccaaatcgggtaaagacagccggctccagatgaatgccaacgctaactacgccgtgcgcacactgggcctggtacccaaaatcattacagacccgctcaccaccatgcaatacaagcatgatgccgccaccccgctgtatgacctctatcccgctgccgacagggcctatgcagaaaaactggccaacgacccttctctgccaagagtaatcgtaagccccaccgataaaacaaagtacgcctactacggatctaccgactggctccatgaagtataccagaaaacagcgcccgcctataatgccaacttcagcatttcccgcggagatgaaaaactgaattactacttctccggagattattacaaacaggatggaatgctccgctataatcccgatcaatatacgcgctataacatgcgcgcaaaagctacctataccatcaacgaccgcgtgaagtttggtagcaacaccatgtacaccaacaccacctattcacaacccgccaataccgttgattacttattttttcacaatgccaaccgcacaccttctttatcggtaccccgcaacccggatggaacctggacttcagacggcgcggccttactgggcaacctgcaggatggcggccgctccgcagatacctggagcgaatttatgaccaccctcaatgcagaaataaacctggtaaaagatgtgtggacgctgaaaggagatgctacctatcgccgcggaaataatgtaggtaaatcctatacactgccggttccttacagcaacggtcccgatcagccaacccaatataccaacggcaaccagtcgtctgccaacaacagtaccaatgaactgaagtataatgtgtataacatttataccgacttccataaaacatttaataaaaaacacgccgttggcgcactggcagggtttaaccaggaataccactacacgaatatatttaatgtaaacaggcagggacttatcagtactcaataccccaccccgcaactggctaccggtaatatcactgaaaagcaagccatcgaagactgggccgtaagaggtattttctaccgcctgaattatacttacgatgataaatatattgtagaagtaaatggtcgtaacgacggatcatcgcgcttccgcgccgataaccgctggggcttcttcccgtccgcttccgccgcctgggtgatctccaaagaaaaattcttcagtagtattaaaggcatcgacctactgaaactccgcggctcctatggttctctcggcgatcagcaatggaaagcttacggctacatgccactcatgtccgccggaaacatcaactccgtgttgaatggtcagctgcctatcggcgtatacgcacccacgccggttaccgccacctacacctggcagtcggtaaaaacggttaacggcggtatcgacttcagcatgctgaaagaaagattatttttcagctacgaccgctacacccgttacaccaacggcatgttcgccaaaagccaggaactgcccaacgtatacggcgccccggctccaagaaccaattctgccgacctgaaaacacgtggatgggaaatgaccctctactggcgcgatcagtttaaaatcggtaacaacgatttcggatacggcgtgaaattactggtggccgacagccgctcctttattacccgcttcaccaatcctaccggtaccctcgccaactatgacgccggctcgctggaaaaccgcaactactacaaaggacaggaaataggcgacatctggggccttgttacggaaggatttttccagaatgaagacgaactgaaatcacatgccaaccaatccaaagtaggttccgacgaccagcagtaccagttctatgtgggcgacctgaaattcaaagatctcaatggcgacggctcggtagactatggcgataacaccatcagcaacccaggcgacaggaagatcattggtaacaaccagccgcgctttccttacagcattgacctcaccgcttcctataaaggtttcgatttccgcgcactgatccagggtatcgggaaaagagactggtaccccaacccaggtaaccactacttctggggcgtatatgcacaaccgtggacaaacgtacaggtacacaacctcgatcgctggacacccgaaacacccaatggttacttcccgcgcctgaaatcatatatcgcggaagatgcttccgaactgggcgcaccacaaaccaggtacctgcagaacgctgcatatacccgtcttaaaaatgtttccatcggttatactattccaaagtccttcacagagaagtataagatcttccgcttccgtgtttatttcagtgcggaaaatatctttaccatctcccatctgaaagcgaatatcgatcccgaaggactggacggttctgtatatccctaccagaaaacatactcgttcggattaaacctgaacttttaattaattcaaacatcggaacatgaaaaataaaaggctttatttatcactcatcatactgggctgtgcagcagcttcctgtaacaaggacttcctgcaacgcaaccctcaaacggagatctcaccggaagcatactttaattcaccacaggatctgaatacctacatcaacggcttatacgatgataatctttccgcaccgtatgatgataacaattcagataacgtttccggtaacaccggcagcgaaatggacaagctggtgcacaacaccctcgatgcaactaccgtgggcggatgggacgactgggaccggctgcgtgatatcaacttcctgctggacaatgccggcaaagcaaaaggagatgcagccgatattaatcactacatcggtatcgcccgttacttccgtgcaagattttattttgaaaagatagctacctattctgatgtgccctggtacggtcacgcattaacagatgtggacccggatctgtacaaaggtcgtgatccgcgttctgcagtagctgattctgtgctcgccgacctgcagtttgccgtggataatattaaggtagatgataaagacaacggtacccgcgtaaataaatacgctgccctggtgttaatgtcccgcttgtgcctcttcgaaggaacattcagaaaataccacgaagaagtaaaacttgcgaacaccgcagacgcatttctccagaaagcagtatcagcagctcagcaggtaataagcagtaaccgctatgtgatttacaacaccggtaaaggtggagaagattaccgcgctttgttttccagcctttcattaaacggcaacaaagaaatcattcaatggagagattatccgcagagcctgggtaagggaaacaatacccataccgtactcggatggacctggtcactcagccagagccttgtttacagctacctgatgaaagacggcaagccattcacttcacaaccaggctttgataaaattggcttcacggcaactttcagggaccgtgatccccgcctggcggaaacggtggcctaccccggcttttccaccacgcaggataacaatgtgtacattgcaaaaccgaacctcggcgcatacgaccagctgaaattttatccgcgtgatccgaaacaacgccagggatgggaaaccaactacaccgctttacccgtataccgctacgcggaagtactgctgaactttgccgaagcaaaagcagaactgggtaccctctcacaggccgatcttgatgcatccgtaaacctgctgcgccgcagggtacaaatgcctgatctcaacctcgctgccgccaatggaaacgtagacccggtgctgaatgcagcctacctggtaagcggacccaataaaggcgtgctgctggaaatacgccgcgaaagaagagtggaactggcctgcgaaggactgcgcctcaaagatatcaatcgctggaaagccggggcacgcctccaggaagcgccacagggcatgtatgttcccgcactcggcggcattgatatgaccggcgacaatgtagccgatatcgccatcctgcccaatactacagatacctcatctatcgccgggttacccgctgatgtaagagcaaaattgtcgcgtttctatctcatggataaaaccggggagaataacttctacctcgaaaacggcaccaacggtcatattaaatttactgccgaccgcgccggtcgcacttttaaagatcctcagtactactatcgtccgatacccaaacaacagacgatactgaatgataaactgaaacagatattcggctggtaaaccggataaatagtgatgaaccaggattaccatgatccatgttttgcagtgatattattcccgcaacaacatggatcatggtaatcctttttaataccgccatcatgcttataaaataaacccattcatgaagcaattactcttaaccctcctcatcgcctgcagcctgcaaacgctgatggcacaaggattctccggcaaggtgtttatagacaataataccagcggacagccaaacaacacagaaaaaggactcgcaggtgttcgcgtatccgatggactgcacgtgaccatcaccgatgccaacggtaactatcaccttcccggccacgcaaaaataaggttcatatttatcaccacgccggccgggtaccggttcaccaaaacattctacatacccgtggacagcgccttgcaggcttacgactttggcgtacagcctgtaaataaagccaccgctgccaccgcgaaattcgtacggcttacagacaccgaaacctaccagttcaacaactggatcaccgatgcaaaggcatatgcacagaacgaaaacgccgacttcatgatccacacgggcgatatctgttacgaaaaaggcatggcattccacgcgcaatatattaatacccgcaccatggggttacccgtgtattactgcatcggtaatcacgacctggtaaaaggtccgtacggcgaagcactgtatgaatccctgtttggcccggtatgctattcctttgacgccggccccgcccacttcattgtaacgcccatgcgtaacggcgattatcaaccgtcctacaccctggatgatgtggtacaatggctcaaaaatgatctcgccaataccgcaccggaaaagcctgtgatcatattcaatcacgacctgctcacttatgatacgctgtttaccatccgctcaaaaaacgacagcatcaaccttaatgagcaccacctcaaagcctggatctatggtcactggcatattaattttgcccgtacccacggcaacaccggtatccgctccctttgtgcagcgccgcctcccggcggcggtatcgataattccgcttccaacttcgatgtaatcggcgtggataaaaacggactttcgtttgtacagcggcgttatacctatgtacacgatcagctggtagcggtatcgccatcagcagcgggcatcgctttcgaccaggataaaatggtgatcagtgcaaatgcttatcatacttcttcgccggtaaataaagtgctgttcagcttattcgataaaaaaggaaatctcgtaaggcaggtgccgctgcaaccccgcaccgattggaactggttcgccaccaccgctattcccggcagctggttaaacggcgtatatacggctacgttagaagctacattaggcaccggcagggtgctgttccgcagggatacttttacactggcaaaaaatatctctgtaaaaaataacggtaacacacccgactggccggaagtattacagaacatacaacgtacaggcgttaccgctatacctaccgccggtccgctgcatttaaactggaccgcaaacgtgggaggcaatatctggaaatcatctcccatctgcgcagcaggtaaaatattcacaggcactattgatgacgaaggtaatcaccatagcagcatcaccgcactggatgcacaaaccggcaaacagctgtggcaattccccaccggcaactccattaaacacagcatcagctaccacgatggcctgttgctggccaccgatgcagaaggcgttacctacgcccttgatgccgctaccgggaaattgaaatggaaacatgcgggcgatcttaaaaacctgcctgcctataattctgccggcgctatccatgaggacgtttattacaccggcgcaggcaattacctgcaagccctggatatccataccggtgaggtaaaatggaccaaccacgactggaccggcggcgaaggcacgcctgcagcaatggccatccacaacggggtgctcgttacttcctccaactggaaccacctgtttgcacacaatgccgccaccggaaaactacaatggaaacgcagcgatgaaggtatccgcttccgcagcggcacacccgctttctttgacaaccggctgtatgtacacggtatcaacaaacttcatatcctggatcctgccacggggaaaacaacagacagcattcctcttaccgaagatctgaaaaccatgacagcgccgctggtcaccaaccagtatatcattacctgcactgccgccggtggtatgctggccttcgacaaaaaaacaaaaagggaactgtggcgctttgtaccgggtgaagccctgttttactcagcgccctactcttccccttcttccgctactatcgaatccacaccgttactggccggcaaccgcctcattgcaggcgcgtctgacgggtatgtatatgtgattgaccttgctacggggaaaatgatcagtcgatttaataccggcgcgcccgtatttgccgatatggccgtgtataacggcatgctgtacgtggcagatttttcaggaaacgtgaatgcgttccggttataagaatagctatccggtacaaaagaggatatctccgttaaaagagatatcctctttttatatatcaaattattgcgttacgaatattgcctcccttttttagattttttattatagtttgcagcggaagaggaatattgaatacggaaagcaattgccaatcaaccaaacatataacgggaaggagcttcttttacagatagcagcgggagatgaacttgcctacaggcaggtatttaacagccattggaaccagatttaccaggtggccctcagcttcctcaaaacacccggagaagcgaaagatgcggtgcaaacggtattcatcaaactatgggaaaaaagacacaaactgccggaagtcgaaaatttcgatgcctggctgtttattgttgcccgcaatactattgtcaacatccttcaccagcaagcctcctttgtggatgttcatcatgtggaggatagcgttccggaaaattatcttatccccgacgctttgctggaatacaagcaaacggcctcccttatccaggatgccattgcgcagttgccaccacaacagtcgctcattttccgtttaagccgggagcagggtttaacgcacccgcaaattgcaaaggagctgaatattgcgcctgctaccgtgaaaagccatatggtacgggcgctcaacaccatccgggaatatgtccggaagcaaggaggcaacgcattgctcctcatctggctgctggaaaaattaggaaaataaaaaaagttttccctcaactgcacctatcacccttttttatggtctttatagtaaagacgcaatttttgattgtcttaaaatgtaatcgtgtatgcacgcttcaggggaattccagtcattaatggataaatacctcaccaactccatcacagcaacggagaaggaactcctgttcgccatgatcaggagcagacaacatatgcccaccctggaaaaagtggtggacgatgcacttggaacacccattgaagtaaacgaagacaccctcctcagggaagaaatcttcgcctatgtaaaagcacataaccagccggtaaaaaagataaatcactggcagcgctatgccgctgcagcagccattttactgctcattgccgcgggcgcttattattggctgcaaccatcctccaaagcgcctgcgccggcagccaactatatcagcaccgctaaacccggcgttaataaggccattctcatactggccgatggctccagcattgcactcgacagcacgggcgcgcagcaattgcaacagggcggcacttccatccgtcaacagggcagccagttgaaatacgatgtacaaagcagtgccccgggcgtaagctacaatgtattgcgcaccccgcgtggaggccagttccagctaacattaccggatggcacaaaagcctggctgaatgccgcttcatccatcaggtatcctaccgcatttaccggtaaagaaagaagaatagaaattacgggagaagtatacctggaagtaagcccttttaatacaggcgccgcggaaaacacgccttttatagtggtatccgcacatcaacaggtaacagtactcggcacgcactttaatatcaatgcatacgaggaagaaggagccaccagcaccacattaattaccgggaaagtaagggtatccgcgggcggtaacgccggcgttatactggcgccggatcaacaggcagtaacggcccataacggcactatcaacaccatcccggtacggtccgtggaaacttcaaaggtaatagcctggaaaaatggctatttcgattttgaagaagagcgcctgtccgtggttttacgcctcctgtcgagatggtataacgtggattttgaggcggatcccgccatgcttaacctgaaattcagcgcggtaatagcccgctcatctcagataagcgaagtattgtcattgttgtcggccaccggcgccgtgaagttcagggaagaaggaaatagaattagagtatactgatttttttataccaactgtcttttagagcaaaccatgcgtaccaccgcgcatcggggtaaagtttgctgtgcactgcaggcaaagcaaatgatgccatcattcaataacgcgattaaaccaaaatccacacaaatgaaacatttgtggctttatcatcatttcctgcactatggcagcaggacaaagaccaaaccattatcaaccatgaagtttaaagcaatttttctgttgatggcctgcctgcaggtagcagcaacaggcttctcccaggtaacgatctcaaaaaacagcaccacgctggcagaggtatttaaagagatccggaaacaaacaggttatgtattcatctacaataacgatatgttaccggaagataaacggtttgacctgcatgtaaaaaatgcgccggtgaaagacgtactaacgcaatgcctgaagggcttaccccttacctggtccatacgggacgccaataccatcgtgatcagtccgtacaaaccatccggcagcacagacgaccaggcgcaaaccgtaatactgcgtgggcgggtcttcgacacaaacggacaaccattacccggcgccagcgtaatcgtgaaaggaacccgccagggtacctccaccctttcagatggcactttccttatccgtgtaccggacgaaaagacggctgtcgtcatcacctttgttggcttcaaaccgctggaactgaagccctggaaggaaggaatccgtaccatacaaatggaaagaagcgccgtggaaatacaggatgtagtggtgcgtaccgggatgttcgacaggaataaactcaccttttccggtgcagtagcctccttcagcggcagggagctacgtcaggttggaaacctcaacgtagtccaaagcttaaaaacgctggacccttcctttatcgttaccactaataacatccagggttccaatcccaaccagctgcccaatatagaagtgcgcggcaaaacaagtctttcctccagcaccgtaagagaccagttttccaacgatcctaaccaaccattatttatcctgaatgggatggaaaccaccctgagccagatcgttgatctggacattaaccgggtggcttccattaccctgctgaaagacgctgcctctactgcgctgtatggctcccgcgccgctaacggggtagtcatcgtggaaacgatacaacccaaacccggagagctcaatgtgtcttataccgctgatctccgctgggaaatacccgatctccgcgattataacatgatgaatgcagcagaaaacctggagtttcaacaactggccggattgtacaaaaaagagtttggctactccggtatcaccaacgacaacctctataatcaacggctggcagccgtgcgcagcggggttaacagctactggctcaatgttccgctgagaaacagcttcaccaacgggcactcgctccgcgttagtggcggcagccaggaatttcaatacggcataggactgaactaccgcgggctgaacggcgtaatgatcgggtccgacagaactacctggggcgctaccgtggatcttgcctaccggaagaaaaaactgaacatcaccaaccagctgtatgtaaacggtaccaactccaacgaatcgccttatggctcattcaatgatttcgtaaacatcaatccctactaccggaaaaaaagagacgacggcagcctgaataccgaccggtacctggaaacatacctggtaaataccaactcctttatcccggatacggtgagagtaggcaacccgttatacaatgccacgcttaattcaaaaaacaataccaacacgctcctgctccagaacaacctgaacttcatatatgatttcacacaaagcttccggttctccggtggcttacaggtacagaaaggcaccaccaaaggcaccctttttattcctgcctccaataccatgttcgacacggtggatacttaccggaaaggccggtacaccgattcccggacagacaacatgagctaccaggccaacctgatgcttacttacagaaaagttttcaacgaggtgcatagtcttaccgggaacgcccggacggaaatgcaggaacaaagtcaaacgtattccgcgtacaccgccaccggtttccccgaaggcgtaaatcccaacccggcttttgcctatggcttcctgccagatagcaaacccatataccagaaaacaacggtaagaagggtgaacgcactgggcagtgttaactacgcatacgacaaccgctattttgtagatgcgaatttcaggatagatggctccacttcttttggcgctgaaaataaatactcgcctttctggtcggtaggtgttggctggaacatcagcagcgaacattttatgtcggagatacaatggttaaccatgctccggatcaggggaaacataggtaccacgggtaaccaggcattaggcagctatgcttccacatctgtttacgggtatgaaaataacctgaacatttatggacaaggtctttatctcacccaactcggtaacccgctgctggaatggcagaaaacacaaagcaccagcgttggtatagacgcctccctgtttgacaaccgcttcaccgctactttcaacgcttatgagaagctgtcgaaaccactgatcaccaacggttccctgcccgcatcatccggcgtggccacctatgtgctgaacgtaggaaacctccgtacccgtggcgtggaagccattgtacggtatgcacctgtctaccagccaaagaaaaatatcctgtggacactcggctacaccggaagcttatataaaagcaggtatgaaggattttccaacatcctcaaaaacctgaatgatgaagcacagaaatccaactccctgcaacgctatctcgatggttacagtcctgatgaactctgggcagtaaaatccttcggtattgatcctgcttcaggtaaagaagtattcagaaaaacaaacggtgaaaaaacactggtatatgatcctgccgacattgttcctatcggcaacggcaggccgcaggtagaaggtgtgatcagctccaatcttaatatcaaaggattcctgtttggcatcaacctccgttacagtattggcgcttatattttcaactccgccctgtacaataaagtggaaaacatcagcttcgatcagctgcagtacaaccaggataaaagagcgctggaattacgctggaagcaaccgggcgatgatgccttgttcaaaggtatcagtctcaccgatgtaacacccatgtcgtcgcgcttcatccagaaagagaattacctcaccggtgaatctatcaatgcaggttacgaattccgctccgtacaatatccgtgggtacggcgcctgaaactgcaaaccatccgggtgaacgcgtacatgaacgatatcttccgcctgtcgaatataaaatctgaaagaggaatcgattatcccttcagcaacgcggtttctttcagcttaaacatcttcttctaaatatcttttttatgcaaccgataaaacgcatcattccgctcctgctgcttaccaccatcgttctttcgctggtgtcctgcagtaaatatctggatgtacagccggaagacaagttcctggaaaaccaggtatacggcagccaggcgtccattcgcaacgtcattaacggcatttatctgaacctggccaaacccaccgtgtatggccgtgagctcaccgctaccacgctcgatgtgctggcccagtactataactgcgccgccttctcccatcccttttataccacagcaaggtatacatacacagatgccgccactatgtcgcataccaccgacatctggaacaatgcctatacggctatcctgaatatcaacctctttattcacaacctggatagcaccaacaatgtattaagcgcaacagaaaaaagcctgctgctgggagaagcatacggactgcgggcatttgtagcttttgatatgctgcgtcttttcggaccggtatatgccaccgactccgttaaagcttctattccatatcctgtcacaccggattcgaaaatagaggccctgctgcccgccaataccgttattacaaatgtgctggctgacctttctactgcggcaaccctgctggaaaaagacccggtacgcacggccggcatcacggccccggatgctaccccggataaattcttcagcctgcgcaaccgccgcatgaactattatgcagtgaaaacgctgcaggccagggtattgctctaccggcgcgataatacaggagctgccgccgcagcaacagctgtgatcaatgaagccgctccctggttcccgtggagcccctctgccctctctgctcccggcatcgtgaaccccgaccggatcttttcttctgaagttattttcggactggaaaatgcagatatgtatgctactcaaaccagctggtttgccgccaaccttaacaccaacctgctggcgccgctgccacagcggcttaccgctatttatgaagattataacaatgattaccggtaccggatcaattttgatgtggacagaacttctgtacggacagacaaaacttttttcaaatatgcagatatacaaaacaaaaacctgctttaccggaaactgcaacctttaatgaggcttacggaactgtattacatcgccatagaaggagaaacggacgacagcagggccaccacgctgttgaataccgtacgttataacaggggcctgcctcccgttaccattaacggcgataaaagaatccagctcactaaagagtatcaaaaagaattttggggagaagggcaactgttcttctactacaaacgcatcaacctcccggccatcagcagcggcgcttccgccaatgccaccattaccatgacgccggaaaaatacgtagtaccgcttccgttatccgaaaccactttcagataaaaagtctttagtctcaaatgtatcaatgcaataacatgaaattttttccaatatacttccttctcctcgccggcctgataacgggatgcactaaaagtgaactgctgcgctatacggaagaaaataacgttttcttctcctacgtccggtcaggtactaactatgatactatcatgatcaattttgccttcctgggaaatagagcagaagacagcgccgggttttatgtaaacctgctgggaaaagtcaccgctgatggcaggttgttcaatatgacggcagacaaatctaccactaccgcggtggcagataaacattatcgtttacccgttaccgatagcctgcttattcccggaaacgccaatgaaaaactggtatctgtgaaagtcttccgcccggcagacctgcgtgaaaaaacagtatcgctttttctgaagctcagtcctaacagcaactttcaaacaaacatgagcgtgatcgactttgcagcgacgaatgtagtatctgccactaacctggaaattatcatacaggatattcttccaaagccagatctctgggataacaacatcaacgcgctgggggcatactcgcgtaaaaaacttgaactgttcatcgccaaccagtcgctttcgctggcgaagttctactccggcacgctgtattccaccacacagctcaccaactacgcccggcaattccaggcctatctcaacagccagaagagtgcaggtaaaacaattacagaagaagatggaaccgaaatgaaaatgggatccgctgttcaataatattctttcatcttattcaaatacaaacatgaacacttattatctcaaaccaatactctttgcctttattcttgcactgctgctgccggcgtgcatgaaggataaaggtaattacacctatactccgatcaacgctatcactatacaaggggtagattctgtttatttactggattacggcaaccgcctgcagatcaaaccggtgctgaaattttcaaaagatgatcacgaggatacggccaactatacgtataactgggtagcggatcacctggtaggatacacgatggaccctaccatcatttctacggcaaggaatcttgataccgtgatcacgcttgactatggcctctatgcgatgtactaccgcgttactgataaaaggaccggcgtattcaccgacaactattttacattgaacgtaggcgctccttcctatgaaggatggatgatgctgtgtgatatggaaaatggtaacagccggctggatatgatttcacataaaggcaataccgataccttataccccgatattcttaaagaagtacactcttcttacaaaccaacgggcactcctgcttttatagctacccagttctcagacattggcggccctaccaacggatcactcggcatatttgtagccaccagcaaaaatgcggtgctgctcggactggactcactggattatgtaccggcttacgacatgaagaattttatgcaggcggcggaacctgtcagcgactggacaggcgccgacatctccctccggttctacggcggtttgctttatgtcaacaacaatatatatggaataggctacagctctattaccaaccccgtaaatacgcaggacggcggcaccgcgcttttcaaaccatcgcgctggatgagtcagaacacatcggggcagtcgatcctcttcaatgaagacaccaaaacctttctgcgctatcctggctcgggtactacctgcctcacacttccggctggcgacctatttaatttcagcacgggcatggatttaatatacagcgcctttgcgcctttcaacagcggggaagtatttgccgtgctgaaaaacagtaccaccggcaaacggtacctggcgcgcttcacaacagccggtaaacagaactattttgcagaaatcaccggtgatggcattgctgacgctgaaaactttgccgtgagtcctgatcttggctacctgttttataacgtaggcggcaaggtgtatgaatatgatcatgctacaaaacgcagcatcctgatgcacgactacggcaaccggaaaatttcactgatgaagttccagccttttgcttctacatatgccagcgcagctaacgctaactattatatcgggctaagcaaaaagttactggtagccacctatacccaggggcaacccgcgaactccggcacacttgatatctataacgttcctgacatcaatgcatctttacagctgtataaatcatataccggaatgggtaaaatttcctgcatcgcctaccgcgaacggtaacatctccattaaaaaagaaaccgctgcaaacaaatgtttgcagcggtttctttttgctatatccaatacgctatactgcttctgcgtgtacaatcgccgccacaggcggcgctaccaccggaaccggttcttctgttacttcatctcctaccaccggcccgttatgcgccagctcactgccttctttcttcgatttaaaaataggccataacaactgtgcataccattcctcttctttataatgtttcaatccgtaagcacttggatactgacgggtaataataccagtaccaaaaatgatgtcccagataaaaaacatattcccgaagttgcctttgtagttccctatgccatcatctgtggtatctgcatggtgcgcatgatgcgtggccggcgttgaaattaaacgctccatgatccagcctataggattgagccaccggatggtataaaacggcttatcccattttagactggaatgcgccgcagtagtaatcagcgattttataccgcctacgaaaagcgccgggtagccaagacccaggtaggtcagcgtaaccgtcaggtagatctgcgaaaagaacgccgtgtaaataatattctgcctgctcgtcatagccatacccatataaggcgcggaatgatgcgtgcggtgaaagcgccataacagcggcagctggtgatgcagccggtgataccagtactgcgtaaggtcatcggcaacagccatgatggcaataccccaccagaaaggtacccaggcaaacgcattctttgcatccggtaaaacaaatggcaataacttcaacccgaaataagcaatcatcggacgcaacacaatttttggaagtataaaacatacgatatccagtgtgcgttcattttttgtccacttgttttcgtacagtcctaccgaaaactctatcacccctactaccagcataatagcgggtaacccccacgttttaagattattaaataccgcatccaggaatgccggcgcccggaaggaaagatgctcagaagtggcgttcagccaaggtttgctgccactgatataaaacgacagaaacatgagccctatcggcaatacatatagcagtaaactaatcagggagtccttcaggatcacctgcgtctgcgtttttgctgttgttgtcatactttatcttttttatgtgatcagtgatgttgattaaataaaaagtgtatcagccagatgctaccagcaataattaccagcggtatcaggaatatcaatatgccgatggcaattttttttgttattaaaacaagatctgctaacgtcataataatgcatttaaagtgatggatgtataatttcgatatggttaagtttaccggtaaaattgtaaggcgacttatacaacggagataccgccgaaccctggtcccgccctacgtccagcccttcatcatagggtgaaatagtagcatcagctttgctgatggcccgttctgccaccttttcatcattgatatacagtgcctctgtacccgccggatctgtgagtcgcaatgccggtgtgtacgtcagttcataacggagtatagcctttcccaacggaagcgccttacccgaagtaagcgaagtgagttgcccgttgttgttatgcaccgcctgcagttttcctccctgcacaaaaaaagtaaaccctgaaaaacgcccgcccgtacttaataacacgccttcattctttgcatcactcaactccacatctgctttaataataaacgattgctctgaaagaaagggagcggaacgggaaggcacctgcgtgatacccgggtataatatagcgctggggcggctatccaatggtcccctggtaaggatagccggtgtaagacgggtggtatctcccagcagaggatacactttatacttccatgcctctgtgtcaaaaagactttgtaactctttcagcttcgccgggttgccggcggccagatcatgttgttcattaaaatctgtattcagattatacagttcccaggtgtctgtggtgaacggcgtaccccgtttgtggctcacagcagctttccagccatctttgtaaatggcgcgaccaccggctatttcgtaatattgtacatgatgcctgcctggcgccttttcattattgatcgtgtaagccaaactgatgccttcgagcgtatcctgcggataaccattgatcaccttcggtattttcaacccggcaatttccagcacggtaggcgtcacgctgtttacatgcgaatactgcgtacgtatgcctccttttttgatcagctttggatagaaaatcaccagcggattacgggtaccgccttcactgttcgcatcctgtttaagataacggaaaggtgtattcgccgcctgcgcccagcccaccgggtagttgggaccggattccgggcttcctatcttctcatataaactatcaatatcctttatcctgcggtcgtagttctcggtaaacaaactgccgtcgatatactcattaatgccatgcacatggccgctgagtcctccttccttgctggcgccgttatctccgataataagcacgatcagcgtattatccagctgcttcgtatcccgcaggtagtttaccaggcgtcctacttcataatccgtatgggaaagaaatccggcgtacacttcaaagaagcgggaaaacactttcttttcagtggcggaaagtgagtcccacggcttcacgcccgggttgcgtggtggcagggtggcatcctttggcaccaggcccagcgccttctgacgcgccagcacctgctcgcggtatacatcccagccggcatcaaatttacctttgtacttatctatccaggtcctgtctacctggtgaggcccatgtgtagctcccggagtaaagtacaggaagaaaggtttatcgggtgcagcggagtgctgcccggcgatgtaggaaatcgctttatctaccagcactgttgtaagatgtttcccctgcagatccggttctaccttcaccgtgttttcccagagcgccggtgtatactgatcggtttccccggccatgaatccaaagaaggcatcaaacccgcgccctgtaggccagcggttaaaaggccctgccggtgtaagatccgggctgggcgttacatgccatttaccaacggcataagtattatatccgtcttctcttaatatctccgctacggtacctttttcaaacggcatataaccgttatgtcccggcaggttcaccgcggcatcaatcacggtaggcacattcaccgaatgatggttgcggcctgtgagcaatgatgcacgcgtaggcgagcagatagcagtagtatgaaagttcgtatagcgcaggccgttattagccaaactatcaaaaacgggcgtttccactaatccgccaaacgcgctactggcgccccatcccacatcatccagcatcacataaataatattgggggcacctgccggggcaaccgggttaaaaggcgcaggggtaataactgattgtgcaagcgtggtacctggctttccggcatagcttttctgcgggctgtactgcgcataagcgcccgatgcagcgcccagcagcatcaacgaaatgaaggatccggaagaggttgaaaatttcatgtcttattatttagttggctgatagtttatttgtcccaccacaaagcaggtgattgataccccgatcccgccggggtgtttttattcaacgattgctcattctgcgggtaaggaatcctgcgcggtatttgtccattcggattggcaacgctggtggcgtttttagcgagcggcaacgccggataacctgttctgcggtaatccgaccacgcctccggctgcaggaacaatgcaatatatttttgggtgataatcgtattcagatcattgccggaatcgccgcttaatatagccttcgccgttatatatgcctgttgcttctccggtgtggcataagggtccgcactattgctgattacccgttgaaaagacgaacgtatcgccgcttccaatgctgttttagctaaaggatctgcggggtttatcctccaccgcgcttccgcctccaggaattttgcttctgcaaaactgctgatcaccaccggcgaagtagctgttccataatagctgccgatcactgaaaaggcgccaggcacgcccggagcgctcccgcggtaggtactgctgcccacagggtaaggagtggcaaaataagcccgtcttgggtctaccagcagcccttccggcttagtgggatcatctgttacagcgtttccgttcaacaggtttacaaaagaagcgcccagccctatccatcccggcctgttggtattctgctggtaaaagggattcgcattggtagtggatgcaccaaataccaccagcgcatctccggagttatcggcgattcccctgtagcgggcgccgtcatacaatgcgttcaaggtggcttgtgcggcagtggtgctgtttattttagtaagatgtatcgcgaaacgtgctttcaaagtatacgcaagcgatttccaccgctctatgttaccgccgtatatcacatcatctgtggccggcaatgcgcccaggttactggccgccggtaatgaaagctctgcgatagcggaatccagctgctcctgcagcgatttataaatatcctcctgcttgtcatatacggggttggtgatattgttgccatacagggattctttataggggatatctccaaaaagatctgttaaagtgccgtaagtatatacgctcaacacccgtgcaataccgctgtaatagggcaactgctgttgcgttgcggtggttcgcacaatcttcagttcatccagcacctctacataaaagccccgccaggtttggttaaagtactgggtggatgaagcgtagttatcaaaggacgcggcatcaccgttggcgccggaagcctgttggatataaatgttggcaatcaacccggcattaacgcccaggttaaagcccagcgctacttccgcgccggttaacaccgcactgacggatacctccgtagaggcgttagggttaacattggtatcttcaagcgagcaggaagcctgcagggctaacatactcactgcaataaataaacgtccgatattagatggatatattctcattttgctgattacttaatggattaaaaagaaacattcagtgccacgccataacttttcgtgttgggcgttgtccagaagtcgatacctgctgcattcgacaaaccattgcggcttcccaggtccggatcactaccggtgtaattagtagacaacaaaaagttcctggcggtcagcgtaacgcttgctgcagatatgtgggccggcttcaacagctgtgctggtacagcatacgtaagattcacatctttgagctttatccagtaaagatcatgctccacataaagcccctgtatattgaaagtgttacggtaccatgcctgcgacagcaccgccccaatggtattgggttctccttttgaagcagtaacgccatcaaaaacggtggtagtacctcttgcagccgtggaggcatccactccattaaacaccatctgcaaccgcggtgcattgaacaggtcaaagccaaagcggccatccagtaaaaatgaaaagctgaaggaaccatatctcagttcattacgcaaccccacattaaagtcaggattgggatcgccgatttttgtgaacgtagtatttaccaatggataaccgtagctggcactattgggattatcatcgatgatgggcttccctgctgcattacgttttacatcagtgccgtagaatacgccgtagggttggcctgcctgacccctcgcctccatccatatgccaccaagactcacactggaaatgttatcggcgatataatttacacggctgatgtttttgttaaacaaagcggtggctgtccatgaaaatttccggccgctgacaatacgttgctgtaagctggcttcaactcctttgttaacgatgttgcccgcattagtaagcgtgtaggcggcaccggtagagtaaggcagcgtaaccggtataatctgatctttactgctgttgtaataataaactccctccagttgtgttttatcatggaagaaatgcagatccacgcctgcttcccaggtgctgatgcgttcgggtttaagattggggttgccgatagtagcgctgtaactgagtccctgcttgccattgaatggaaaactgattccgctctgtatccatccgctgctggtggtaggcacataataagtttcaagagaataaggatctgcgtcattacctacctgcgcgtaagtggcgcgtatcttaccaaaattcaggatactgttattcaggtgaagtgcgtctgtaaaaataaaacttgtactggcggaaggataaaagaaagcatttttacctttggccagcgtggaagtccactcgttcctgccggtcagctccaggtataaccatttcctgtagtccagctttacatctgcgtatccggccaccaattttctccggatggtttgattaaatgtttgggtagatgacgcattggcgatattaaaattaccagggattgttaacccgtcgccacgggtatttacctggttcttccaggaattataatagttgtatcccgctactacggtaaggtccaggtctttgttaagcttccggtctgccaccagtaaaacatccaggttattgtctctcctggaataatttacgtcattgatggtaccagtacctacgccggaggtaccgcgactaaaagcgcctttcctcacatcggtatagttgtcgatgccataacgggcagtggcttttaaccagcttgtaatatccaggctggcttctgcaaaagtaatgaagcggttcagctcatcggtttgcggattcatattgagcgaccagtacggattatcccagccaataccgttcgcgtatgaacggctgtcgccccacggcttgctggtggtagccggcagcttataggattcgggatgctcccatggttcggagtaaccattggtgatgtcaaagtttgccggggaattgatcagcgcacgaacaacgttggtattaaaacctcccattagagccctgttaccggcgccgtctttgatgtaattgaggccaccggatactttcagccggtcgttaacggtatagtcgccgttaaaacggaaagtatgccggaagaaatctgttgtcggaataatacctgtctgtttcaggtttccataagaaaaataatacccggcatttcctgtatttccataaaagctgatgttatgatcattcgtatagccgttaacgaaaaactgcccgatattgtcatacctgttcaccggtatgccattggagagcggggagcttcgccctactatcgtgccgttcttatcaaagttgctgggctgtgagctgtaagtgagtgtatccagcaatgcgccccagttttcgtcggagccggtagtgccgggttttacatattgtccgccgatgccattggaaaaactggtttgccgcggctgcatgcggcggtttattttatcaaccgtaaatgatccgctgtagcttaccccaaaagatttatctgtgagggaactgcctctttttgtattgatcaccacggcgccgttcgaagccctgatgccatacaatgcagccgcagcgggaccttttaaaacggttatgctggcaatgtctgcactgttaatatcaatgcccctgttggatggtgtagccagggatacactgtttgacacgggaagaatatcctggatagaattatctacaggtacgccatctaaaataaataacggcgcattatttcccagcagggaactgtttcccctgatttttatggtagatgatccaccgggcgaaccaccggaattattgatctgcacaccagctacctttccgctgagtgccgctactatattaggttcacggctgtctttcaatgccgcggcctttacttctcccacactgtaaccaagtgatcgcgtggcactcctgatgcctacggccgttactaccacttcagataatgcctgctgttgttccagcttcactactttgttcaggtcgtcttttgtaatcagtacttcctgcgactgatacccaataaaagtaacgatgatggtttgcggtaatttcaacaggcttagctggtaggtgccggcagcatctgcgagcgtgcctgtggcgccgcctttgatacgcacggatgcacccggtagtgcttcctgtgttttattatcaattacttttccttttaacagcacaggggcctgtgaataaatgctggtggtaaagaataacaaggcagcactcaatagtgtctttcgtaaatatttgaacatacaaaggggaattagatgttggaagaatgggacaatacatggccatgatgaccacgccaggtgtcatttaaataatcggatgtgccaatcggaaagccctaacaacaacagcaacacacggatgtcactgtatccgcgtaaaatttccttttgcctctattgttgtacaatagctgattcattgttgaaatgtttattaaactggttgatcaggtcgcccctgtaaggcaacttcaataaagaacactaattcagatttgctttgtatggtggggacaaagactttggtggtggtaaattctattagtctactattattgtagacaaatatacaaccgggttttggaaaacgcaagcatccaacaaaaaaagttttcggaggggcggatttcctgcaccggcacggcatttcgcggctacagaaaaaactcgcgcggggaatatggctattctttacttttgattatggtacatccattaagaacgcatatagaaaccgtctgtaagctgacagacgaagagtttgaatatattttatcgcactttactcctttaaaactgaaaaaacacagattactggtgagagaaggtgattgggtgaaacacgagtattttgtgctaaaaggctgtcttcgctcctatattacaaacgctgattcgggtaaggaatttacttatcagtttgcggcagagaactggtggatatcggagcgggaagcttttttaaagcaaacaccggcaactactgctattgaatgtattgaagattgcgagcttttgggattgagctatgaaaaccggggaaaattaggccgggagatgtggaagtatgaacattacgtagcggtgaagtcaaatcttggatatgtagcgttgcaaaaaaggctgcaattaatgattatgggtagtacaaaagaaaggtttgaaaactttgtgaaacaatatcccaacttgtatagccgggtacccaaagctgtaatagcttcctacctgggtgtttcaagagaaaccataagccgtttataccgtaaataatggcagatttgtcacatttttaaagtgataaatgccctcctgcatggaaaataaataggggaattttgtagaataattttataaaaatgaaagttctacatgtattttccctcagagggatattcgtatcattgctgctgttaaacggtttgcttgctgtaagatcacaaccggcagcgcctaaattgccggcccagcccgggttttattctatgcagttaggcgatttccaggtaattgcattgtccgacggaacgattcctttaaaccttaacgggctgttgcatgaaacccggaaaggtgaggtgcaggagctgcttcatcaaaactaccttgacactactgttgaaacctccataacagtttatctggtgaggaaggacaatcagctgatattaattgatgccggatgtggcagctttctcggaccaaccctggggaaactaaagaccagccttcttgctgcgggttttcatgcggaagatatcagtgccatattgattacacatcttcatgcggatcacgttggcggacttatagacggcgataaaatcatgtttcccaacgccactatttatatcagcaagccggaagcggcgttctggttaacatcttccaataaacaaaccgccaataaaagagcgcagcctttcttcgatccggcacaggcggctcttacgccgtatcaaaaagcaggcaagataaaattgtatgatccgggtacatcaatttttccgggcatttcgtctatcaacacacccggccatactcccggtcatagttgctacgcactggaaagtaaaggacaaaagctcgttttctggggagatgttattcatgcaggcgcagttcaattcgccgatccttcggtaactattgattttgatgttgacttatccgctgcagctgaaatgcgccgggaaacttttgaagatgcagctaaaagtggctactggattgcggcgccgcatctttccttcccgggaattgggcatttgcgcagtaatgcacagcattatcaatggctccccgtcaattattccattaattaattagtttttaacagcgtaaagcaattatccagtaatgcaacaatgttgcactactggataattgtttatctttattctcaaaaagctggtttatcatggaaaatttctgggaatcgagttttattgaaaagcaggagatgtgggggtttgagccatccgaatctgccatttcagcaaaagaatttttcttaaaagaaggtatcaaagacatactgatccctggtatcgggtatggcagaaatgccaaattatttgtagacaacggcatcaaagtaacgggtattgaaatctccaaaacagccattgatctggcaaaaggccattatggagatcaaatgaaaatctatcatggttcagtaaccgaaatgccgtttgatcagcatttatatgagggcatctttagctacggactaatttatttgctggatagcgaagaacggagaaagtttatccgtgattgttataatcaattgcagccggacggacacctcttcttttcagttatttcaaaaaaatctcctaactatggaatgggtacacaaataggtaaagaccgctttgaagctacaaaaggagcccaaatatttttctatgacgaagaatccgtaaaagaagaattcgggaaatatggattgatagatttctttgaaattgatgaacccaataaaatgatgccgggcaaacctgccttccggtttatcattataaaatgtaaaaaagaacgcgcttaaaggaaagccccgtcctgaaaatacagggcggggcagtaactaactgttatggcggcatatactaccggcgtgtaagactgttcaggtaattttccaggttggtataaccattgacagcatatccgttgcgatcggccgcatcattgggattaaagccgttagccgtttcataactgtcgggcatcccgtcatggtcgctgtcggcaggcgccggcaaagacgttaacactggccaggcatttacggtttgactgtatggtgttccatgaggacaaccgccctgcacatcaatgataccaccggttctgttgcgcacatcatttactattcgctgatcgagcgtatcacggcccggcagcgaacaacctgcacgctgtaataccgattcaaaagcatctgctgctggttccgtattcaccgcataaccatgattaaacggtgtggacaccagtacctccgcaggattagtagtactcactcccgcggtgttatcagcggtgttacccggcgagccatctacataattcccattcacataccattttccaaaggtaaccgtggcactgttactgggattgcaaatgcggtactttaccccgcttcccgtattgggaccgtatttataatagttattgacgacgttatagtttccaccttccccaccgtacaccgtgttgatcccccaattgtaaagcacattattccggaagtctacattctctattcccagggtagaaggcgtataagtgctgataccggcaaagcgtggattacggttgcggcaatgcgctatcaggttgtgatgcatgctccctcttttcgcaccccatataccaccataaccatgacgctcataatcagtatcacccgtttcaaaatggtaggaataattcagcggctccgagatcatgcaccattgaatagtgaggttgtcgccacggtaaatagtcagcgcttcatcgttactccagctggcggtgacgtgatcaacaataatgttgctgggacccgtgccgccaaaagcatcatcaccaccactgccgtctaccgggttaccatttgcatccagtttctgctgattcttatcgcccaaacggaaacgcatatatcgaatgataacattgtcgccgctgatatgcacggaatgatccgccacacagatcccgtcacctggcgctgtttgccctgctatagttgtattggcttttatactgagaccggaattgagatggatggtacccgaaacacggaacaccacggtgcggtaagcggcgggcgctgttaaggcgtaacgcaggctccctatggaaccgtcatccagtaaatttgttacttcaaaaacggtggtaggcgctgtggccgtgccccgtccccctgtggtaaacatgcctgctccttccgccccggggaaggctggctgctgcgcatacaaaacaggcgtcttgaataaagacagcaatactagcaggcaacttgccagcggcttgattctgatatacaacatataactggtttgctgttttcaaattgacgaaaaaatttatctccacctgggatcacctgtactgttccggccaggatatgcattatctgcaattttgaaatcgccaataccaggcgcctgccacaactgtagcgccggtcgcgtataggtgatgatgttcgggaaatcattacctgccgacaagtgatcggacgtacgatagttattactggctccaatcacagtgccggcgcccgccctcacatctttgacggtaatagcgcctttgctgtctttcccaatcccgaaaatgcaattgcttaccgtaattccattggtcacctcattggcattataatcaacataataatttttgctgttacccagcggcgcctcactaaatgtgcaatccgatatgcgtaccgcagcggagccttgcgcgctggcaatcacaccctctactttgtaaatagtgctgttggtgatggaaatatgattgatcctgctggaagcaccgatattcaatataaaataattgcctatactgtcgatgatacaattgtcgataacaaaatcgttgacgttggtagtccccgattgaagccgcaccatgccccggaatatttctgcgcggctgttaacgaactttatctttcccacagtagcgctgttactgttgttaaatacatagcgacctccgtaattatctcccaacatataaatgtcattaaattcaagagaatcaatcaccgtcccggcttcaaaattgaaattactggtaaagaaaatcttcgcctgcgtggtattggagaggtccggagcgctcatgataacaagcgatttatttaggctgaccgtggaagatatattataggtttcccctcttttcagcaacaccgtactaccggaaggaatcagcggcaacgtatcagccaatacaccgggtcgtccggtgatggcggttaaatctacaatagtacctgaaaacggtgctttggtagtaaaatccgcatatcccctttcttcgttgccactatacaggaatataatgtaccgggtagaagcttccaggccttcggctactttgaactcgttcaccaggtcccctgcagttaacgcgacagttgataccagggctttatcagcagccttcaaaatttttatggacgttacggcagcaccttttgttgtccagcgtacccgtaccgaattatacgtgatatcgtcgatacccggcactttcaatatggatgacaaggttttaacagcgcccaggtctgaccattttgaattgagcaatgtatcagcagcaatggcctttacccgtacctggtataattggttgaacaataactttttcacgacagctgcattcgtatctaatgacaacgacaaatcggtagtccggaaggtatcccggcttaactctaatgcataagcagcagcgcccgcaattttttgccaggacgcaacaaccgtgttggaatcggcggttaactcaccggcaatcactggtctgaataacctcgatggcgcagtgtcgtccttctttttgcaggatatataaatacaggaagttattgcaagaatgacagaaatctttttcataaattgacttatttccccggaaaaaatgtgctaattaataaccatattcattcttcaacgtacccaaactgttcgatatcacagaactgtgtagaggcagaacatagcgtggcggagtgtttcccgtattatcgctatatcctctccattgccacagcgtgtaattcgcagggccgtctgtagttgtattccacaggttgcgcatccagtttattttgatattgtattcggcaggaacaacaccggatactttctgaaaacggtttaaaaaggaaagggttttgtcgctgtttcgtttcgcatacagatagtcggggagatggctgtacataccaacacctgcaattgcgtcctgccccatctggttcagcactttcctggtttcggcaatttgtttcccgtacaggttccatcttaccaggtcaaacttccgcaccatttcaccgcccagttcccaggcacgttcattcacaatagcattaaagaacgattgcttgcttccgccaacggcagtaatataaatttctactttatccccccacaacgcaggaggaaaagcgcgctggcgaactttgcgcaaggcatcctttgcatcgccggtagggccgtacagttcgttctcactttctgccagcattaacagcacatcggcataacgcatcagcggccagttaatactcgtgccttttgatgatgatggccccagcggcgtaggcaccagcatacggttccatttgtttatagtgatagaagtaggccctgtggatacctgtgccaatgtatcgttataagcaatgatggaacaggtggcagcaagccggaggtcggttgtatcaaatgagtaataataagtaggcgtaaggctcatttgaatggtggtagcgccaaatgaatgataactgattccattcgttacacctactcccacgcaccagccaacatccccaaaaccaggggcataggccacttcgtacaatatgtcactgtttaatggtttaatgtatttgttctcattcataaatacagtagcaaaatcggttaacattcttggcttcatgcttactaattttttactgtaggtattagctatcttataatattcctggtaatcagccttccgcttcatggtcatatcaggataaagccagtaaccaccacggataagcgatagccgggcaattaaacccatcgcaaactcccggttaatacgctcaatgccattatccagctgatctgcccattgcatttttgattcaatgcctatcaggtcgttgatcaaaaaagtcaggatagaatcccgtcccgtcttgggcaggtaaaagttatccccggcgcgggatggtttgatactaaaaggcacatctccccagtgatgcatcaataacatataccaataagcccgcaagacttttacttctcccagcaaattgagatacgtcgcatttgttggatcttttaccagggaaatggtggttaatccatgttcacattcattggctttattgatagcgctatacgcgttgttccaaacggtgagcaggtcgttgttggaagtagtagcttcaaaggaccacaggtcacggcgcgcgccatcgggcgaagcacttaccgaattccctacttccacgtcggtattaccggcaaaaagtgtggacacacgcgatgtaaacgcatcctggttgaacatcgcatataccatgttcactgtttttgtggcgtccggctcggagccaaaaacatattcttcagaaaatctggaagcagaatcagatgtgagatatttcttgcaggaaacaagcagcagaaataatataacggtggaaaaatataaaggacgtttcattgcttttttattaatgtcatgctaaaagtcagaaggttacatttacgcccacagtatacgagcggcttttgggaaagcccgagtagtctactcccggcaccagctgattataaccattgctccttgtagtgctaacttccggatcgtatccgctgtattttgtccatacaaatgcgttgtacaccgtggcgtatatcctgcacctcgtcatgtaagcgctggagattatttttttgggtaaagaatatcccaatgacagtgtatttaaacgcaggaaagatccatcttcaacagcccctgaatggaaataaggcgatgcagtacccattgaaaagggcgaccaggttttaggattaggattcaatgctgcaagctctttcagatctgtcaccaggttaccctgcgcatcgatatagtggaagcggttgtcgtagctggaagtgctcaacatgttaccataagtggttctgtaaagcatgttgaaagaaattttgccggtgttataaacgtcattaccgtacacccagttaaaaatagccgacaggtcaaaccccttataagtagcattcaatccaaaaccgccggtagcctttggcaatgcgctgccgataacggtacggtcactggcatcaataacgccgttgccatcaaggtcttttaacttcagcacacccggccgcaaactgatcccgcccaagtcctgctgagcggcgccttccttcacgatgtatttcctggctaccggatcgtaagaactgaaatcatcaacggtatacataccgttctccacatatccatacatcaaaccgatggtgcggccaaccatcaacctgtaatcgtcaatgcctttcagatcggtaccggcccagttagagttgaacgaccgctcgtctactccatccagtttatcaattcttgcacgattgatgcctatattaaaattggcgcttaaccggaacgctttcttattgatgatatcagtgttcagcgccagttcaataccgcggttagaggtttgtcctatgtttcgttgctgcgtggagaaacccgtcgtttgcggaatggcagattgcaccagcaggtctttagtggtgttgtggtaaaagtcgagcgttgccgatatcttattattgaaaagatcgaaatcgaaacctacgttacgggtaacggtagtttcccatttaacatccgggtttgttaactgtgagctggcataggtgtaatacggattgggtatgtcaccggcgccataaggacggttactgctcggcgcaaataaaagccgccactggtcagatgcaatattgttgttacctacaataccatagctgaccctgaacttcagatcagaaacaaactttacattgttcatgaattcctccgaagaaatacgccaagcaaacgaagccgcagggaatattccccactgttttccaggcgcaaagcgtgttgaaccatcgtagcgcgccgttacattcagaatatatttttcatcgagctggtaaatagcgcggccaaaaaatgaagcggttttgtccggagcaatttccgttgtgctgtggatatcttgtgtgcccaggcccattgtggcaaacagcttctcaggcgtaatatccatactaaaatatttcgcccggttatactcttcaaaaccttttcctcttgacagtatctcctgccctaccagcaaattcaggttgtggcgggaacctttctcccattgataattaagggtatttgtcaggcgacaatcctgcaaccgtgtttgcgtgatttctcccaatggcaggttgccgccttcgttcctggcggtaccggttaaaggtccgtagtaacggcggttctctgaaaaagtcattcctaaactatattcagaacggtaagtaatatttttggtgatcagccaggaagcgccggcattcacgttaaaaatgcggctggtacgcttgcggtaatcctgtgtggataattccaatggatttatcaggttgctcaaaaactgttcatagtcatcactgctgccgggatcaataataatcatatcggcaattccatttacaggacgcgtggtgataccatctccaatgcggaagctggcgcccccggccgaacccgcgccatttataacaggatgcgtataacgcatggatatatcgagcttcagggctttggaaatatcatgattcaatttaaagttcagataattgcgtaaatagttgttactggaaattaaacctgattctttattgtaagtgtagttcacggaaaattttgtgtggtcatttccacccgtcaggctgatattatgctgttgggagaaagcagggctgccatacagttcgtcctgccagtcggttcctttctgggatttgtagatgtccaggtcatcgtaaacaccgaagtatttggtgaaattatcaacgtcgctctggcttctcagccttgcatactcatattgcgcaagtacaaattcgtacggggaaagcacttccagtttacgtggcaactgcctcgcctgggcaaagccgttataggaaattgtagatttaccacctttggcacttttcgtggtaacaattacaacaccgttagcgcctgctgcgccatatatggcagcggtggccgcatctttcaggatatcgatactggctatgtcagatggcgcaatgtcattaatattattcaccctgaatccatccacaataaacaacggatcgttactgccggtaatagagcccccgccacgaacacgtattacaatctccgctccgggttgcccgtcaaccgtagtaacctgtacaccaggcagccgccccgtgagcgcctccgcaacattggctaccggcgctttttccagctgcgccccgctgatggaagatactgtgccggttaagttctttcgctttatactctggtacccgatcaccaccacttcattcatgttcttattctcttcctggagcataataatgatgggcgacttgccggtagcaacaatttctttcgactggtaaccaacataagaaacatacagtcttgcgtctggccgggaaacattcatactaaagtttccggcttcattgcttaacgctttattattagttcctttctccactatagtagcgccgggaagcggctccttattgctgccggttatggtgccgcttatggggatagccgtaccgccgcgggaagatgatgtccctttagcaggcagcttttctgataccacaatagttttttccacaatggaataggtgaatggcaattgtgaaaagcaaagtgctaacgcctgttcaagtgtggcgttgccaacaacaaccgtcaccttgtttgcattattgagaaggccgtcaacataaaagaaggcataacccgtttgacgggttatctcgcggaatactttctcaaccggggcgtttttttcattcaggataattccctgtgcagagatgttagcgcccgcctgcaggtaaaccatcaccagcaaggcaaaggtcagtttcataactttctggaatttatcgccggctccgggacataacggggcggcgggaaagcatctctttaacgatgcttttccaaagacaatcgatgacataatttattcctcttttggttgaagaaaatagtggtgctacattttttacctcaaaatttttctggtattcaggacttcgttcttatgatccggcagctgcagcaccggtttcattactgtttaactacaatgtttttcccgtggatttcaaaacgtactttattggttaattctaaaattttaaacaactgttcagcattggcgcttctggaaatctgtcctgaaaagcgcgcggaaatacctcccttatactcaatctggatatcataccatcttgctgcctgccgtaaaaccgtttcaatatcggccgccttgaactgaaacatgccgttcttccatgcgatcacttcttccgtatttacatcgtcctgcaacttaatatccccgttagcgataaccgaagcctcctgtccgggtttcagcctgctggcttgttttccgctggtaacttttacacttccctccaacaacgtggtacggattacagattcatctttataactattgatattgaaatgcgttcctaacacttccacatctatactgtttactttcacatgaaagggcatcgactcattcctggctacttcaaaatatccttcgccggttaactccacccttctttcctttcctgaaaaatttgaaggatatcgtaagctggaagaagcattcagccaaactttggtaccatctgccaatgtaagctggtattggcctcccctgggtgtagtgatggtattatatacaatttccgcaggcgtagtacccgttattttataagatacctgcccgttacctgatttaataatttttgcctgtccttgttgcagcaacattccttccgttaagctgtcgagcatcacctctgtaccattgcctaattttagtaccgccttgttgctgccgggcggaatcgggatgttcttgtcaggcacatttgcctgtgccacttcatttttcaatggcgtctttaatacaaaccaccagtaacctactccggcaagtgtcagcgcaaaaacagccgcagcagccattctttttaaataaagggaaaatgttggcgttctttttccatccgccttaatatgttgctgcaattgattttgtatgccttccaacactttattatcaggctccccttccagcgcgtgttccttcaattcggtatcaataatcgcttccagctggctttcatgctccggttcttttaacatctggctgaaaatcttccattcctgttcagtcatcctgcctgtcagatatttatctaataactcctgaaaaatattgttctccataaacattcaattcaattccaaaaagcagctgtattattaaagacgcatagctaaaccaaaaggggacgttggtttaaaaataaatatgtgcaggtccatcaaagaggaggtaaacaattgataaaagcatcgttatatctaaatgaccgctgatataggttctgagaaaaccaagcgcacggcaaatatatttcttcaccgcttcctttgatacctgcatgttcttcgctatttcttcatgagacaagcccaggtcgcggctctgcagatatgcggtcttttgttgctgcggcaattgctcaatcgccctcgctatcaattccgacaggtttttctgtgataaaattttatcggggagataatttttctcttcaatttcccattcatcacgactaaggggtaattctgtcttctttctcagggcgctgataatatgattacgggcgataataaacaaaaatgagtcaaaacgttctaccccggaaagcttgtttctttcctgccagatctttaaaaacacatcctgcacaatgtcctgtgcctgacaggatgattttacataactcagggcctgccaatagatgttattccacttctgtgctacaagcactgcaaaggccttttcgctgccttcagcaatttgccgcagtaaaagcctttcatccattgcatttatgttcataacgtgaattttgctattaggttacctgtggaattaaaagggaaattaaacatttgtctatttaaacaagctaaacaagccggaaacctacgggaacgattgcgtaaataaagtgggagaataaaaaatgatggagatggatgggaataacttgctttacctttcttttttataacagggacgaaggcggaaaaaatgcaggtaaaaagaaaaagccttttttaacacccctatgattacctggatcataaagaaagctaaaaaaggcctgtgatattttgttgcccaaccaggattcgaacctagacaaacagaaccaaaatctgtcgtactaccattatactattgggcaatacccttattgtttgggatggcaaaagtataactttttttatttctgcaaaaaaaacttgcaatatttttaaaatatccttcagaatcctttgctgcaaagacttataaaactatctcattcactttttccgctatctgtgctggttttatccactccatacaggcgtaatcccctctgaagcagggtttgttaccgaatacggaacagggccggcatggcaggtcatgaacctggatagcattttcaggcgactgcccataccccataaatccggcaaaagggtgggtggcgccccaaacagatactaccggcaccccaaagagggaagcgaggtgcatattggctgaatccatgctgatcatcacatccagctggctgatgatagccatttcctcctccagggaaaaacgccctgccaccacaattacctgcggatactgggctgccagctgcgtaagcaataacacctcctgctttccaccgcctaaaagaaacacctgtatcccctgttcctgcgccagcatacccaaaacggccgccatttgctctaaagggtacattttttcgcggtaagtggcaaaaggagccagtcctacccattttttatccttttttgcaccagtaaccgcggtcagcgttccgggcaacgcacggggctgaaaaacgggtttgcggcccatttcacagcgaagccccagttgccggaatactttcgcatacctttctatggtactggttaactgctgcaataccttgttgtccttccgggtcagcgccttcttttctgcgcggcctttgtcaatagccgctacgggtgtaccgctcaaccggaaaaaagtccggatgatctgggacctcagcacattgtgcaggtctgccacggcagtaacccgatgcgccttttttacttcacggaacaaacgatacagcccttttacccccttatgaatgccttttacatctgccgggaaaaaggtcagccgcgaaatacccgcgcataaagcgccccagttccggttggtcacaaaaacaatctccacatccggattttcatccagcacctgcttcatcacaggaatggtcatggctacatcgcccatagcagacaaccgggtaaccaatatcgttttaactgcgcccaagtaggaagatttatttttcgtttttgtataaaaccgggttcagggaaggatcattatacatcttcatttgcttgtataccttcatgaactttttaccggcggcaatatcggccagcagcgcctcaatggcggaactcaggtcctgttgctgctccagcaggatatccagcttgcgctggcacgctgcacgatgttctggtgtggcatccgcacgggtggcttcttcctgcatgtgataaattttcaacgccagaatagacaaacggtctattgcccaggccggactttcggtattaataccagcatccgcagcaggtgccgttttgccatatttttccaggaaataactgtcgatgtattccaccacatccgtgcgctcctggttggaacggtctatccaacgcttaatacccaatgcttctacgggatcaatcttcggatcgcggataatatcctccaggtgccactgcaccgtgtctatccagtttttcaggtaaagcaggtgctcaatgctgctcttttcatagggattggaaatggcctgatgcacatcgttgtgctcatggtaggccacgatactctggttaaatatcttattgcacaattgtgtaaacatgccgcaaatgtacaaaggctggcgacaaaaaagaagcgcatggtagagaccatacgcttattgtaaaagattgtcatgtgaatgttcgagaatgcaaatcgtgaaggctttcaatggttatcttggggttgagatgccgtcaaggttataccaccttattttccttttttaccttgtaatgatgtaatcacaccatatcggcaaataatatttttatgattgtttgtttttgaatattttttgaatgcagtaaaaatcaatcactctaatggctaaacgttttattgagggtgttctaaaatgctatagctgttaacaaattaccagatcactaattacaggggccaggatcacagacgttatatttcataaacctggagtggcctcttaccactactttttatgggaatcttctgctaatgttgacaacttcatttgtttaattctactcaaatagtaccgggttttctaaaattatcagggtttaaggtggacatctttatgtccgtgtgtcttagtgcaaattaaaaggggccactgcattttgcactgcagtggccccctttttttatacaacgtttgtggtaattacaaggttttcttgtccaaattagcttttggtggtagccggtcgcgtaatcttggtaagataaaacagcggaatacccaataaaataattcccagtccgggtaaagtatagttggtttcaaataccagcaacaaagctgccagcgataatgccactatgatatagatcattggcagtaccgggtaaccaaaagctttgtagggtctttctatctccgggcgtttctttcttaaaataaaaattccgaggatcgtcagcacataaaatatcaataccccgaaaattaccaatgccagcaagtcgttgtacctgcctgtcaaacacaacatggatgcccatgcacactggatccacaaaccataggcgggcacgctgtgcttattcagctcacctgcttttttaaagaacaatttatcttccgccatcgtgtaatagatccgcgcacccgataaaatcaacccgttattacaaccaaaggtggagatcatgatcatcactgcaataataatagcgccgctggaaccaaagatctgcgccgctgcagccaccccaacacggtcgttggcagcaaacgcaatttcattcagtggcagcacagccaggtacatcaggttacagctcacataaataatggtcacaatcagcgttcccaggaaaagggaacggccgatatttttagaaggatttttgatctctcctgcaatgaaggtcacattgttccaggcatcactggaaaacaacgagcctttcatggaaaccgcgatggcgccaaacaacgccagccctgataaagctgccgttaccaccgtaccgttctgtgatgaaaccgctgccgcatcccaggcatgctgccagttggcctgccagatctcagactttgccccaaacagtaacccgaaaataatgagtccgaataaagacaacagcttcgccaatgtaaatacggtttgtatcagcttaccgtggtgcacaccacgtgtatttataaatgttagtaagatgatagatacaatagcaactatctgcgccgcagaaatctgcacaataccggcgtccagcaaaatgttcttctcactgaaacccggtatcaggtaagcagtaaactttgcaaaggcaaccgccacagcggcaatggtgccggtttgaataacaccgaactgcgtccagccaaataaaaaggcaataaaaggattgtaggcttcccggagatatacatactggccgccggctttggggaacattcctgacaattcaccataactcatggctgcaatcagcgtaacaaagcccgccagtacccacatagcggtaatccagcctgcccctcccacgctacgggcaatttctgctgttacaataaagatcccggaacctatcatagatccggcaacaatcatagtagcatctaataggcccagggatggcttgaatgatttagtttggttgatttccatattgatatttataaaaaatcccggctcataagggaaccgggactataagatagaaaaaatttctgatggtttattcgcttatttggcaggagtggcggcgctgttattattcattcctttaataacgtccggtgttacatcgtaagccggatctttatacaggatgttgctggcggtactgcggtaagagaagatatacgcaaaacgcttgtcggcgttaaatgatttcaggaaatcgtccagtctcttctgcagttcttcattaaacttagtttcctgctcggtataactggcacgcaggttctgcgcttcctgctctaactgctgttgtttagacatcaggctgcgttgtgctgcctctccctgttcctgggtaagggtagatgctctgcgttgcaggtcttcatactcactctgcaatgcacgggccttgcctttcagctggttgtccatctgctgctgcttctgctccaataagcctcttttttccttgaaatactcaaaatgcgcttccagtgaatccagatctacataagcaattttaaaactacccgcagcaggagtaccgctgtttgccgcacttgatgcagctggtgcactgttaccagctttatttccctggcaagacatcaataaaccggctgaaaatgccgctaataatcctttattcactaattgtttacaagtgcgcatgttaataggtggatttgcttcttttagtacatttgaaaaatggaacggctaaaataaggtttttaatggattttcatattcccgtccatttttttagctaggttttaacgaatattattacttcaccttctccaacaggatctccggctcattggtggtaatataatccaccccgttttttaataaatcgtccattatttccggattatctatcgtccatgcattggtagttactttatgttgcttcgcagtggcaatgagctgcggatcattcctgaatacctgctgattgtaatccagtccccagataccatcggcctgcaactgtgcgggcgttttatccccattcaggtaagctattttagccgcgggatccagctcctttatttttttgcagatattgtagtcaaagctgatgtagaacatccacgcctgggccttcttggcctgcaccatcgctactgctttggtggccagcaaatcgcccctgccggtacgggagggcttcaactccagcacgagccgtgtacggtgttgttcctggatcacatcaataaactcctccaatgtgggaacccggtcgccgtttttcagctgaactgtttgcaaatccgccagcgtactctcttccaccttctttccccctatctccggatcatgtgaaattaccagttcattatctgacgataaccacacatcaaattctgatccttcacaacccagcttcatcgcatctttcagggaagtaaggctattctggctgcccgcctgatgcttccatgcaccgcggtgggccactaccttattgcggataaagtcatccgccaccagcaggaattcagcagtgtccgccccggctttaatgcggaccggatacttaaaatcaccttctttgcctacggcagctttctttttcagtttcaattcatggccgctgacagtaaataacccggacttgtcctccagcaaggtagccgctgataactgcccgttcctgtcatagattttaccaattaccgcgttcttttgctgaacgggaatcgtataggcatcaaggtaaggagcgctggcttgctgcgccgctgcagctgtacctatcaaggttattcctgccatcagaaatatttttttgcaattgttcatgtggtccgcgtttgtggctaaaatagcgcgcaatttattcatttccatcccctggatggaaaaacactacgttaaattactataaagctttaagatgcgactgctttaattatgctgtatcagcaacacattgaacctggcaggatccagcggataaccgttgctgataagcgtatacactttaccggcctgggtagccatgtcgaaggttttcaacactttggaggaatcaatccagcggaaattgatcttgtaatgggcgctgtcgccgtaaagcggcgcaaatgcagtttgtgcaggaaatgtcaaccccctgaagaagcggggaaacgtatcggaataaacatcaatgccaagcggtgtacggtttggcctgaatgcctgggcaaaattaatcaccctgaatttagacatccctgcagccggagcgctcaggtcatcttcggtagtgatcagtatttgattgcctgcactgtcagcgcctacataagcagagtaaaaacggttgttacgcagaaagatctgcccctggtatacggccacgccaggctgcctggtgttagtaataatcaggttgtatttctgggcccggaaagacttatatcccgtattggttccatagcctatattgctggcaacagtgaaggtatccagcatcacattaaactgatcattgccgggcgctgcgtttacaaacaaaaagttaccgtgggtatcaggtaccgcactgtcactgtttttcttacaggcgcccagtatcaacaacaatattaaaacaggaatgatcaggtgtttcatgaaatccgcttctttttacgcactcaaatgtagtaatattaaaacaaaaagcgcctgcctttggggcaagcgcttcctgttttaatatctgtgtaatactattcttcttcgtcaaactggaacacttccttagaagaagccaggatgtcgtattcttccttggaacctacgatcatgttttcaaactcacgtaaaccagtaccggcagggatcaggtgacctgtgatcacattctccttcagacccatcatatcatcggttttaccgttgatagcagcctgtgataataccttcgtggtttcctggaacgaagcagcagagatccagctacgggtaccgagggatgccttggtaataccctgcaggagcggactggaagtagccggctgtgcatcgcggaattctaccagttttttatctgcacgacgcaacagggagttttcttcacgaacctggcgcagtgttactatctgacctgctttcaggttagcagattcaccggcttccgttaccaccttcttatcgaagatcatatcgttttcttcgaagaaatcaaacctgtcttctgtatctccttcgaggaagcgggtatcacccggatcttcgatgtttactttacgcatcatctggcgaacaatcacctcgatgtgtttatcattgatcttcacaccctgtaaacggtatacttcctggatttcatttaccaggtattcctgtacagcaaacggtcctttgatagacaggatgtctgcaggagtagtagaaccatcggagagtgaagtaccggccttcacaaagtcaccgtcctgtaccaggatatgacgtgttaacggcaccaggtatttcttcacctggccttcacggctttcaatgatgatttcgcggttaccacgtttgatgttaccaaaagctaccacaccgtcgatttcagaaacgatggcaggattgctcgggttacgcgcttcaaagagctcagttacacgtggcaaaccacccgtgatatctcgcagtttaccgataatacgtgggatcttcacgattacctgaccggctctcaccttatctccttcagagataacaatgtgcgaacctaccggtaagttgtatgatttcacctctttattaccatctaccatgatagacgggatcttattcttgtctttggtttcaattaccactttctcacggtgaccggtctgttcgtctgcttcttcacggaaggtaataccttcaatgatgctgtcgaaacggatggtacccggaatttcagacacgataacggcgttgaacggatcccatgtgcagagcatatcacctttcactactttctgtccgtctttcactaacagggtagaaccataaggaatgttgttggttaccagcagacggtcatttttcacgtccatgatacgcaactcaccggtacgaccgataacgatctgtactttttcaccctggttgttttcgtaagtggtagtacgtaagccatcgaattgaacggtaccatcaaacttagctggcaaaccggattcaacggaagtagaaccggcaacaccacccacgtggaaggtacgcagtgtcaactgtgtaccaggctcaccgatcgactgtgcagcgatgatacccacggcatcacctttctgtgcagtataaccgctggccaggtttttaccgtaacatttcacgcacacaccccgacggctttcgcaagtcagtacagagcggatctctacggtttcaatagcactttcttcaattctgtgcgcaatttcttcagtgatctcagcaccggcagcaacaatcagttcctcatcactatgaggatcaaatacgtcgtgcagggaagtacgtccgaggatacggtcatacagtgtttcaatcacttcttcattatctttcaatgcagaagtagcaataccacggagtgtaccacaatcttcttcattaattaccacatcctgcgcaacgtctaccagacgacgggtcaggtaacccgcatccgccgttttcaacgccgtatccgcaagacccttacgggcaccgtgtgtagagatgaagtattccaatacgttcaaaccatctttaaagttggacaataccgggttttcgatgatctcggaaccggtagaaccactcttacgcggcttggccatcagacctctgataccagccagctgtttgatctgctgcttggaaccacgcgcaccggaatccaacatcatgtatacagagttgaatccttgcttgtcagttgccagctcacggatcagggtttcagtcaccttcgtatccacacgtgaccagatatcaatgatctggttgtagcgttcgttgttggtgatcagacccatgttatagttatcccaaacttcttctacttcaccggctgcaccatcaatcatgtcttgcttaacatccggaatgatcaggtcattaatgttaaatgacagaccaccgcggaacgccatgcggaaacctaattgcttgatgtcatccaggaacttcgcagtttttgggatgtctgttgctttaatgatatcaccgatgatttcacgcagtgatttcttggtcagcagggcatttacataaccggctgctttaggtacgtgctggttaaacagtacgcggcctacagtagtgtcgatcagttttctttccagctcaccgtttgcatttcttacatcagctttaacacggatgtgagcatgcagatcgatacggtcttcgttcaatgcgatgattacttcttcagcagagtagaaagctttaccttctcctctaactactacatcaccgattgttttcttacccttcgtgatataatacaaaccaagcaccatgtcctgtgaaggcagggtaattggcgtaccattctgcgggttaaggatgttatgggaagacagcatcagtaactgggcttccaggattgcagcgttgctcaatggaacgtgtactgccatctggtcaccatcgaaatccgcgttgaacgcagaacatacgagcgggtgcaactggatcgctttaccttccacgagtttaggctggaaagcctgtatggacaaacggtgcagggttggcgcacggtttaacataaccggatgacctttcagcacgttttccaggatatcccaaaccaccgcttctttacgatctaccagcttcttcgctgatttcacggttttaacgatgcctctttcaatcagcttacggataataaacggtttgaataactcagccgccatatctttcggtaaaccacactcatgcagtttcagttcaggtcctaccacgataacagaacgtccggaataatccacacgtttaccgagtaagttctgacggaaacggccttgtttacctttcagtacgtctgacagtgatttcagtgcacgaccaccttccgctttcaccgcgttggatttacgggagttgtcgaacagggaatccaccgcttcctgcagcatacgtttttcgttacgaaggatcacctcaggcgccttaatttcgatcaaacgtttcagacggttgttacggataattaccctgcggtaaaggtcgttcagatcggaagacgcaaaacggccaccatccaaaggaactaacggacgcagttccggcggcaccacaggaatatattgcattaccatccattcaggacggttttccacacggccattagcttcacggaaagcttccaccacgctcaaacgcttcagcgcttccgctttacgttgctgggaagtttcagtagcagcctggttacgtaactggtaagaaagactgtccagatcaatcctggccagcatcatttctaccgcttccgcacccattttagcaataaacttgttaggatcttcatccggtaacagctgattgtcttttggtaaggtgtccaggatatccaggtactcttcttcagtgagcaaatcaccgtagttcatgcctttctcctgtttcatgcccgcctggattactacgtatctttcatagtaaacgatggtttccagtttcttggaactcattccaagcaggtaaccaatcttgttaggcagggatttgaaataccatatatgtacaacgggtaccactaaacgaatgtgacccattctctcacgacgtactttcttctccgttacctcaacaccacaacggtcacacacgatacccttataacggatacgtttgtattttccgcaataacattcgtagtcctttacaggcccgaatatcctttcgcagaataaaccatcacgttccggcttgtaagtacggtagttgatggtttcaggtttcagcacttcaccgtatgaacgctccaggataacatccggagaggccagactgatggtaatgctgttaaaatttgatttaggacgattttcttttttgatagccatctgtaattagcttttagctgttagccgttggtggtaagccagcgacaaaaattttattcctgcgaaatatccaagctatcagccactggcatcactgccaatggctggtagctaaaagctcttagtcaaatttcagatccagacccagaccacgcaattcatggatcaatacattgaaggattcaggcacaccggctttcggtatgttgtctcctttcacgatagattcatatgctttggcacgacccacgatatcatcggatttaattgtaagcagttcctgcaggatgttggacgcaccatatgcttccagtgcccatacctccatctcaccaaaacgctgaccaccaaactgggctttaccacccagcggctgttgggtaatgagactgtacggtccgattgaacgggcgtgcatcttatcatccaccatgtggctcagtttaagcatgtagataacacctacggttgctttctggtggaaacggtcgcccgtttcaccatcatgcaggtaagcgtgaccaaagctaggtaagcctgcttccttgatataatcagcaatttcgtctgtagtagcaccatcaaagatcggagtcgcaaaacgtacgcccagtttcagacctgcccaacctaatacggtttcatagatctgtccgaggttcatacgggaaggtaccccgagtgggttcagtacgatatccagtggtgtaccatcttccaggaacggcatgtcttcatcacgcacaatcttggctacgatacccttgttaccgtgacgtcccgccatcttatcacccactttcaacttacgcttgctggccaggtaaacctttgccagtttcagtacgcccgctggcagctcatcaccgatagagatgttgaacttctcacgtttgtaacgacccagctcttcgttgaacttgatgttatagttatgcagcagggtattgatctgatcgttcaccacttcgtctgttgtccagcccagcggattcacgttcatgaaatcaatatttaccaggttctttggagagaacttggaaccctttgagatcaacacttcaccgtaagtattggtaataccctgagaggttttatccttcagtaataccagcaacttgctcatcagcacttccagcaggtcttccgcattcttctggtgaattttctccagtttctcgatagctgctttctcgcgggttttggaatttttatctttcttggcgcgactgaacagtttcttatcaatcaccacaccttctgttgacggaggcgctttcaatgaagcatctttcgcatcagaagccttgtcaccaaagatcgctcttaacagcttttcttcaggagaaggatcagattcaccacgcggagtgattttaccgatcaggatatcgccttccttgatgtgtgcaccaacacggatgataccgttctggtcgaggtcttttgtagcctcttcacttacgttaggaatatccggagtcagttcttcttcacccagtttggtatcacgaacttccagttcatattcatcaatgtggatggaagtaaacagatcctcacgtgcaacacgctcagaaattacgatcgcatcctcaaagttgtaacctttccatggcatgaacgccaccttcaggttgcgtcccagcgccagttcaccaccacgggtagcataaccttctgttaagaagtcgccatccttaacacgctgacctttcttaacgcaaggtctgaggttaatacaggtgctctggttggtttttacgaatttggtcagtgtgtaaacgatcagatcgtcttcaaagctcaccagtttctgcatttcatcacgctcgtaacgaacatggatttcatttgcatccacaaattcgatcacaccattaccatctgcagtaatctgcaaacgggagtcacgcgctgccttgccttccaggccggtacctacaataggaacttccggattcagcagtggcacggcctgacgttgcatgtttgatcccatcaacgcacggttggcatcatcatgctccaggaacggaatcagtgatgcactcaaacctacgatctggttaggcgccacgtccatgaattccacttcttctctgtcgaggatcgggaagtcaccggtttcgcgggattttaccttatcatttataaagtgtcctttgtcatccagtggggcgttggcctgtgcaatcttcacagaatcttcttcctcagcgctcaggaactccactttatgcatgtccactttaccatctcttactttgcggtaaggcgtttcaataaagcccatctcattcaccttcgcgtgaacgcaaagggtggagatcagaccaatgttcggaccttccggtgtttcaatcgtacacaaacggccatagtggctatagtgaacgtcacgcacctcaaagcctgctctttcacgactcaaaccaccgggtccgagagcggaaatacggcgtttgtgggtgatttcagacagcgggttcgtttgatccaggaactgtgacaactgggaagtaccaaagaaggagttgatcacggaagacagggtcctcgcattgatcaggtctaccggcgtaaatacttcgttatcacgtacgttcattctttcacggatggtacgtgccatacgtgcaagaccaacaccaaactgagcatataactgctcgcctacagtacgtacacggcggttagacaggtgatcgatatcatcgatttctgccttaccatttgtgagctgtaccaggtacttgatgatggagatgatgtcgtccttcgtcagcactttcatgtctaacggagtaggaagacctaattttctgttgatcttgtaacgacctacgtcacctaaatcgtaacgtttgtcggagaagaacaatttatcaataataccccttgctgtttcatcatccggcgcatccgctccgcgcaactggcggtagatgtgctgaacggcttccagctcagagttagatgtatccttgtttaatgtattgtagatgatggagaaatcaccactcacctcttccttctgaacaaacacgcttttcaatcccatgtctacaatggtttcgatattcgcttcatccaggatgctatcgcgctccagcataatttcattacgctcgatgctcaccacttcaccggtatcttcatccacaaagtcttccacccagcttcttaaaacacgggcagccagcttcttgccggcatatttatcaagactttttttgtctgcttttacttcatctgccatgccaaacagctgcagaatatctttatctgtttcatagccgatggcacgcaacagggtggtaaccgggaatttcttcttacggtcgatgtaagcgtacatcacgttgttgatgtccgttgcaaactccatccatgcgcccttgaacgggatcacccttgcagagtagatcttggttccgttcggatgtacagattgaccaaagaaaacaccaggtgaacggtgcagttgggatacaacaacacgctcagcaccattaataacgaaagtacctcttggagtcatgtaaggaatgttacctaagaacacatcctggacaatcgtctggaaatccacatgctcctcatcattacagctgaggcggagtttcgctttcaacggtacagaataagtaagcccgcgctcaatacactcctcgatcgtataacgcggcggatccacgaaataatcaaggaattccagattaaagatatttctggtatccgtaatcgggaagttctctttaaatactttaaaaaggccttcgttgtttcgcttgtctggtgtggtttctaattggaagaaatccttgaaagattggatttggatagccaacagatccggtgtctcagtaacttgtttgatctttccaaaatttactctttcgtttgtttgggctttttttagagacatattcgaagttagcagttatatgacttgtaagaattagggaaattaagatttctttgccaataccatcccaatttatttatgccttctgcacgtggtcaaagtcacctgttagtgattcccccgttttgactctctgaaaaagacactttcccaaagggaataaggccaaaagtgcaaaagcacttttgacctttaaaagatgtatacttaagcaaagaattactgaatctcaacatcagcaccagcttcggtcagcttagctttcaggtcttctgcctcagctttgctaacgccttccttgatggatttaggcgcaccgtcaaccagttctttcgcttctttcagacctaagccggtcagatctttaacgatcttaacaacgttcagtttgcttgcacctgcagctttcagtacaacgttgaaggcagttttctcttcaacagcagcagcttcgccaccaccagcagcaactacaactgcagcagcagctggttcgatgccatactcagatttgagtacatctgcgagatcttgtacttccttaacagttaaacctactaattgttcagctaatgcttttacgtctgccattttataatgttttaatgtaatgtttgtaatgttgttgttaattatattgtgacttggaagccaattttgaatgcgggtagccaaaggccatccacactattctgctgcaggtgcttccaccccagcttcttctttcttgcctttttccagtaaagcagcaataacgcgctttgcaggagattgcaacagaccgataacttcgccgataagctcgttcttcgtcttgatgttggttaaagcaaccagctggttgtcgcctacgaatacttcgtcagcaacaaatgcagctttcagtactggtttttccagtttaccgttcgctttacggaatgcagagatgatcagagccggctctttcgggctgtcagagaacatcagggcagttacaccatgcagactgtcaaacacgcctgcatatttttcgctgtccagagattccaaagccttacggatcagggtgttcttagccaccttcatttccacctgcttgtcgaagcacactttcctcaggtcattcacctgcgctaccgttaatgattcggtattagtgacataaaagttgctgtattgagagaacttacttttcagcagttcgatcgcatcatttttttgatctttattcatattataacgtttgtagcaagccccatctttgcagataacggctacaactcgtgatcaattagttttgaacagatttagtatcgataacaataccaggactcatggtgctagccatagacagacctctcaggtaagtaccttttgcagtagccggtttcagcttgatgatagcattgatcagctctaaagagttctgctcaattttatcagatgcgaaagatacacgaccgatagaagcatggatgataccagccttatctaccttgaaagtgattttaccgcctttaacatcgttcactgcagctgcaacgtcgtttgtaacagtaccggtcttagggtttggcatcaggttacgaggacctaaaatcttacccagtttaccgatcttcggcattacagatggagtagctacgattacatctacatcagtccagccagcttcgatcttctggatgaattcatccagtccaacgaaatcagcacctgcttcttttgcagcagcttctttatcaggtgtgcaaagcactaacaccttcttagttttaccagtaccgtgtggaagcgttacggaaccacggatagcctggtctgctttcttaggatcaacgcctaagcggatatgtaaatcgacagagctgtcgaatttagtacagttaatatctttaactaagctggaagcctctttcaggctgtaaaccttatttttttcgagcttagcgtcagctacttttctctttttagttgccatttgtcaaaatgattttaagatcctgcctcaacagggtgaaacaattagttttcccaaggggctttaccatcaacagtaatacccatgctacgagcagtaccagctaccattttcatagcgctgttcagcgtaaagcagttcagatcagccatcttgtcttgtgcaatagcttctacctgagcccaggaaactttacccaccttgttacggttaggttctttagaaccactctgcaatttagcagcttccagcagctgtacaggtgccggaggagttttaattacgaagtcgaaagatttgtcagtgtaaacagtcagcaacacaggcaatactttacccattttatcctgggtacgggcattgaactgtttgcagaactccatgatgttcacacctttggaacccagcgcgggaccaattggaggtgcaggattggcctggccgcctttcacctgcaatttcacgtacgttgcgatttcttttgccatgtttcttaatttaatttggttaaacgccctctgccaaacagaagactcccaaaagtaaaagactaaaaataaccttttaaaggggatgcaaaggtatatattattatgaaattgtcaaaaagtatttgaaattgggcatcctttttgctctggatgggattttttttacaaatctattgcatttcccataaaatttccttactctccgaagccggcaaagttacaacttatctcccacttgcatataacaattctttccgcttccctttctccgtctttatatacttacctacaaacaactgctcatttcccaccttttccttcatcccggtaaccgcctgctgcaatgccgctatattagcgctcatcgcatcatcattaccttccagccccgaaagtgccttctccgctgctgccagcttccctgctatcccgtcgatcatcttcctcaatacctcatcctttacttccggtacaaactcacggttcttaaagtccacatactcattatataacctcaccacgtctgtgtaatcccggctcaccccgttaaactgatccacccgccggttccgcatctcaatttcctggttggccgccagcacctttatcgactggtccatccagtccagctccgtcataatgaacggattggccgctcccccaaaccgccggatcctcgcagctgcatactgtaaccgctgcagccgcgattgccggaaccagttattcagggtatcgttataagcaaaaacggggcgtttggccgcagctgcaaaagcctggctgcccaactcatcatgacgcagcggaaacggcaacatctgccacatcgggtcgtaaggcatgtgggtttttaccgctatctgcggcgccgactggaaccacgtccagttagtccgctgaataaaacggccgttatccaccaccccggctccccaggtgggatctgttatcgtccactgacttccgttctttaccaccacccagtcgtgcgaaccggttggcagcataatatcgttctgtaatccgtaacccgttaccaccacggctgtgataccggcctcccggcatacccgggcatataataccgcataatcagtactgagtcccttgcgggtacgcaacgttttcaacatcgccgctgcagaatcccggtaactgcttacacggtttacattctctgcatcataggcgatgtgcgtagccatccagttaaacaaagcacgttgcaatgccacaccgtttcctgtatgggctttcagccatttggccattagctcgggagaagtggtggcctcttccgggatggaaataatggccgccgttgcggccggcttaacagatttcccggactgggcgcctgcagcagtaaccagcaggagtccgagcattacagtaatcactgacttcatatcaatagatataggagctatattggataaacgagaaaaagcgttccgcataaaacggaacgcttttcaataaagagttatataacttactaagaaagcttttctacctgcataaagttcagctctaccggagtagcacggccaaagatctttacagttactttcagttttttcttgtcttcaattacttcctcaatcacaccattgaagtcgttgaacggaccatcaataatcttaatggtttccccaacaatgaaaggctcgctcatggtcagtccctgatcgctcagttcatccaccttacctaacatcttgtttacttcagatttacggagtgcgataggcttttcctttccgagaaagtggataacaccggatacgttgcgtattgcctgtattacttcatcggtcatcttaccatctactgcttcgatcatcacatatccgggatagaagttcttttcgcgcatcacttttttaccagcctgcactttataaactttttctaccggcaggaagatctggctgattacgttaccccaatcggagcggcgtacttcaatatccaggtattccttcacttttttttccttgccactaacaacgcggagtacataccactttgtttcctgagcaggaagattggctgcatccatttatttagctttgaaaatttggtaatagtgagttaacacgaagttggaagcggcatccataccccaaaccagcccggtaacaaatattgttgctatcagcacaatcatggtagaagactggagctcttgccaggtaggccaggacaccttgtaaaccaattcatgataagactcgcggaaatagtttctgatcttattcattatataaagttaactatttatggtcaattgtttaaagcctaaaaatggttgacttgttttcttgtaacaactcaaccatttaattattttctaaaccttgcacgggtactaggattcgaacccagatcaaaggttttggagacccgtatgctaccgttgcaccatacccgtgtataaagccattagcactcagctttcagcgccagcaaatatataaataaatgttgacatttaacagccaaagctaatggcttttaatataattcagatgcttacttcaggatttcagtaacctgacctgcacctactgtacgaccaccttcacggatagcgaacttcagacctttgtccatagcgataggctggatcagtttaactgtcaggctaacgttatcaccaggcataaccatttcaacacctgctggtaattcaacttcaccggttacgtcagtagtacggaagtagaactgaggacggtatttgttgaagaacggagtgtgacggccaccttcttctttgctcagtacgtatacttcgcatttgaattcagagtgaggtttgatagaacctggctggcagataaccataccacgacggatctgagttttctcaataccgcggagtaacagaccagcgttatcacctgcttcaccttcgtcgaggagtttcttaaacatctcaacaccagtacaagtagatttcagtggttcttcctgcagacctacgatttcaacgttctcaccaactttgatgcgaccgcgttcgatacgacctgtagcaactgtaccacgaccagtgatagagaatacatcttctactgacatcaggaacggttgatcaaccggacgtggaggcagtgggatgtaagtatcaacagcttccatcagttggtcgatagcagcaacccatttttcgtcaccagcgagtgcgccggttgcagaaccctggattacaggaacgttatcaccgtcaaaaccgttagaagacagcagatcacggatttcgatttctaccagttccagcagttccggatcgtctaccagatcaactttgttcatgaatactacgatacgaggtacacctacctggcgagccagcaggatgtgctctcttgtttgcggcataggaccatctgtagctgccaccacgaggatagcaccgtccatctgagcagcaccggtaatcatgttcttcacataatccgcgtgaccaggacagtcaacgtgagcgtagtgacgagcaactgtctggtactcaacgtgagctgtattgatagtaatacctctttctttttcttcaggagcagcatcgatctcatcatatcctctcttctctgccagacctttatttgccaaaattgtggtaatggcagcagtcaaagtagttttaccatgatccacgtggccgatggtaccaatgtttacgtggggtttatcccgcttgaaggtttcttttgccattgtattttctttttagatggtttgtaaagattgtattgattgttgttttaaaaaaacggttttacaaacttgtaccgttgatgagaattgaactcatggccttccctaaataaaaatgggttgctcttccattgagctacaacgctaagttttaatttcggagtgcagaatttacaaattcgaattccgaaattcgaattttatggagtttgttgaggcgattgaaaaattcactacaactattcttctaaaattcaatgagctgttgaagagaattgaactctcgacctcttccttaccaaggaagtgctctacccctgagctacaacagcttgaaaaattgctttaaaatacgagcgggagacgaggttcgaacccgcgacctacagcttggaaggctgtcgctctaccaactgagctactcccgcattttttaattcactaagcttccggcaaacaacactgcaactttccacttatagaattattagaataaaaataagagctttaaaggctgttgtaccacaggttagggtatgctgtctactacttctgaatttctcaccctctactcaacaactatgttccgcctctgcgaagggcaaaagcggaacacgctgtttttgtgggcaggataggattcgaacctatgaagacgtagtcagcggatttacagtccgccccatttggccgctctggaacctgcccctaactatcttttgattttgtcatccggcttaataaacaaccaaataaaaatcgatgagccagcagagggattcgaacccccgacccactgattacaaatcagtagctctggccaactgagctatgctggcatctttcaaaaaacattctttcaataaagtaactcgttgaaagagagcgcaaaattaagagattttttcaattctcaaaatctttttttcagtttgttacaaatatctaaaaatttatctgcttccccgaaaacgcgctaccataaagaactttgctacctttaccaaccctctttttgaatcgggatggcaaaggtagcaaagagattaatatttccaaaattatttcagagaattattgaaatttcttttccttctttctttttacctgctcaacgagggattcaaaggcaaggtcgaaggactcttcgaaggatttggactcgtgcttaacaaacaggtcctgacggggtattcggactcttatctcggctattttatctttaatttgatgcgctaaattatccacttttaaaaatacatccacgctaatgatacggtcataaaaagtgttcagtttctgaactttcttgttcacatgatctatcaatttggaatcagcatcaaaatgcacagtttgaatttgtacgttcatagcactaattttttaaatatttaacaatctaggttctagttagtaaaggaaggtcataggcattctcttttagcataatgaacttgattactaatatagtcacttttgcaatgcaatgctgtttagctgcgtaatattttgttaaaagcttaaaataactgctacgctttcgggtgcgcctgcttatacaccttcttcaactgctcaatagtattatgcgtgtaaacctgtgtggctgcgaggctcgaatgccccagcaactctttgatcgcattcagatccgcaccattgttcgcaaggtgtgtggcaaacgtatgccgtaatatatgtggactctttttctttaaagtggtaatctggtgctctgtgagatacttccgcactgtcaggtatacatatttgggatataaacggcggccgctctgcggatgcaccagcaataccccgctctcaaactcctccaggcaacggcgcttctcatccatgtatgcacgcatctgtgccaggagctccggactaaccggtatgatccgctccttgccccctttccccatcaccttcacagatttgttcccctcatctacccggaattcctgcaacgcaatcaattccgacaaacggatacccgtctggtaaaagatctcaaaaataagccggtgcgtaatgccttcgaaatcattggcaaagatgtgcagggcggtgactgaaaccgggctcacattgtcttccagcgcctgcatccccttctcctcaatatagccgggcaaacgacggctgatcttgggcgcaatgaccttaatcataggcgactgtttaataaggccctgacgcagacagaatttgaaaaaggatttaagtgtggagattttgcggttaacacttttggcggtcatggcatcttccatgagcttcgccagccagctacggatcataatatgactgaggtccccaaccggcgtactgccataactgagggtcacataatcaaaaaactggaaaagatcgttgcgataggcagtgcaggtgtgcgctgaataccgtttctcgagctggatataggatatgaatcgctctgctaaggaatataaagcttcgttcaacacaaaaagattgatgattgtaaagttattaaataaccttacaatcatcaaatattttgagttgccaacggcttatcgcctaagcaatattaatcttcaaatttacctgttgccaactgctgtttgtaaacggcttttaacacctggttacgacgtttaacagatggtttagtaaaagactggcgcgttctcagctgcaataaaatgcgagctttctcaaacttctttttatattttttaagcgccttgtctatgttttcgcaatctttagaatcaatgatcaacataatttttgcctcttatttttaggaacgcaaagataacacaagatttgtaaaaaaacaaaagaccaaaagaattattccatttccccgccttcctctccataaagatcacccaatcggccataaaattccggaaccggtgcgaggcgtccggcaggcacaaacaggaaatcaccgccctcagcctttacgaaggatatagcatgacggctggaccggagcacataagcacctctggtccagccgcttgtataataaactcaatttagtccttcaacttcttcttcaacaggcttacctggtcctgcaggtggctcaccatatccgccaggtggtttacactcatccggctttgttgtcctgccttactgatcacggcatccgactgccacaattccagcacttcctccatatccacgccgtaaggctcaaactgcggattgtcagacaccagcgtaatcttcgatttggaacggttgtttttcaggatccttttaaaaacaatgccttcacgggaggtgatcaccacataggtttcattgttcttgatctcgtcccacccctctaccttgtggcaaacgattacagaacccgaggtaaccggcagcatggaatctcccgctatttcaaatgccctgtaatcacccgcacccagcatgggcagtgtgaacgtgttcaattcctcgataaactcatcatcattataaccggccaggtaaccggcggccgcttttaccggcacaaactgaatcgcctgacgggaacttcccagcttgagctgccggcgcttctccaggaaattatctttctgggagccaagatcacgacgaagcagatcatcaatagacacccggaacatatcacttacctgttccaggatctctgtacggggttctgcacgctcctcctcatatgcacccaacagcgaacgcttgataccgagtttatcggcaaactcttgctgcgtccaggctttttgcttacgcaggtatttcaaattctgacatactacggacataacctaaataatttagtaccttgctaacaaaattagcaaatatttttatgaattaccaaatatattcggggcgcttcgcttatttttgcccggtaaaatccaactcgatatgttaataaactatgtacactcgttcttaagatgggctatattgctggcagggctctgggcggttatccgctccctgaaaggcgtaacaggcaaaacaccgttcaccgcagcagacagcaaagccgggcttttcttcatgatatgctgcgatttgcagctggtagtaggattgatcctgttttttatgagccccctttcccaggcaggtatagctaatatgggaggagccatgaaagaccctgttttacgattctttacggtagaacacgaagtaatggccatcatcgccattgcactggtacatatcggtaaatcaaaaataaagaaagcagccacggatgcacagaaacataaactgggcctgatcttctttggtcttgccttcatcgttatactggcccttatcccatggcctttccgggaagcgctcggcaaagcctggttctaagccttttccggtgaatccggcaactgataaaattaaatggcgcccctgtcagggacgccattcctttttccgatgtattgattgaccactgaattatcctttatccttattatataacctgaaggaataaatatagggtaatgccgccagtacaatcgccgcaaaaaatatgataaacaccccggtgataagcgagaggaaaaatccggctatgataatcaccacaccagcgctgatccacaggttactcgccatctgatgcgtttccatccatacctcggggctttgcagggtccacggcgttctcacccccacataattattcggcttcagcttgcgcaggtaagcgcctatgcccacaatcagcaaacccacacctataaaggcccagcgctccatgataaacggcttgccctggctgaccaggaaaataataatacaggtaaacactgcctggtaagaatggatcagaaagcggatcctgtaatactctttatgctccatctcaatggcagacggccgcagctgcgtttcgccggcacgcggaatatagcggaacagaaaataaatcaacccattcgtaaaaaagagaaagatcatcagcagcaggaagtcattttttgtccccatctcaggagaacccgccgcattaacagtattggataaaacaactggtaagtctttaaagacaaccgccagataaaccatcggcaccagcagcaaagcgaggataagtaattccctggtaaaatccggttttttcatgtgagatcagtttaaatgttctcatactccctgttttccttcattcccattctcttatctattacatattgattgccagatatgttgtactaaagttacgaaaattgaaccgaccggaaatttcaatattttttactaattttcttagcattactaaataaattagtacctttactccacatataaaagtgatcccggctggcaggcctgctgctatactatcctccctctgcccggtccgccatccgtaatcgcttttaacagcctgccctgttccgtcctttgtttatccataaaccattaccagtatgatcactttacaacagcgaacaatagcgcacttcgacctggactgcttctttgtatcagtggaatgccagcgggacagtcgcctcctcggtaaaccaatcctggtaggcggcagcagtgatcgtgcggtagtagcagcctgcagttacgaagcacggcggtatggtattcattccgccatgcccatgaaaaccgccctgcggctttgcccacacgccattgtacgcagcggggacatggaactgtacagcaccaaatccagggaaatcacggaactcatcgccggaaaggcaccgctttacgagaaatcatctatcgatgaattttatctcgacctctccggcatggataagttctttggctcattgaaatggacttcggaactacggaaaaccatcatgaaagaatccggactgcctatttcgttcggactcgcctccaacaaactggtttccaaagtagccaccgatgaagccaaacctaatggtcagcttgaaatcctgttcggagaagaaaaaaatttcctggcgccgctggcggtagaaaagattccaatggtaggccgtgaaaccggcgccctgctgaggcgccgaggcgtagaaaccgtaaagacactgagcgaagtgcccatctccctgctggaagcatggatgggaaaaaacggaatagccctctggagaaaagccaatggaatcgatgaatcgccggtggtgcctttttatgaacagaaatctatctcgacggaaagtacatttcccgcagatacgatcgatatgcaatttctccacgccgaactggtgcgtatgacggagaaaattgcattcgaactgcggcagcaaaataaactgaccggctgcatcaccctcaaaatccggtactccgattttgaaaccgtcaccaaacaaatgtcgatcccctactcctgcgccgatcatgtgttgctggaaaaagtaaaagacctcttcaaaaaactgtacgaccgccggctgctcgttcgcctcataggcgtgcgtttcagccaccttgtacatggcaactaccaaatcagcctgttcgacgataaacaggaaatgatcgccttataccaggccatcgatcagattaaaaaccgcttcggatgggaatatctcatgaaaggaaccaacgtcataccacccgggaagaaagacctgcacaccccgaaaaaagatatcatgccatactttaaataaacatcatgttccttaactgcaaaacatttttcagcctgcgctatggcaccatgcacgcagaaatgctggtgcaaaaggcgcatgaactgggcatcgggtcacttgcgctcaccaacatcaacatcacctccgacgcctgggagttcgtagacctctgccgtaaacacgatattaaacctatactcggactggaatgcagaaacggaaacgattttaaatatctcctgctggcacgcaaccaggaaggctggcatcatatcaatgttttcttatccaaacacctgcaatccgaaaaaccttttcccgatcaggcgcccgttatcccacacacctgggtgatttatgcgctgggaacccgcgcccctgaaacattagcgccccatgagctcattggtgtaaagccctggcaacgcaataaattattcagaacagctaccactgccctccgcgataaactggtgatccttcaacccgtcaccttccaggacaacacccattatgaattacaccaactgctgcgcgccatcgatcagaacatcctgatcacgcagctggaaccagccatgacaggccatccgcaggaacaatttgttacgcccgcttccctcgtggaacactttgcagattacccgtatatcgtacagcgaacagtggaagtgatggaagcatgccacatagaaatggatatccatcattccatctcccgtaataaaaaatgcttcctcggcagcgtggaagaagatcgcgcaaagctgcgggagcttgcactggaaggcatgatgtatcgctatggccaacatcatgaagaagctcttcagcggatcgaaaaagaactggcaattgttgcgcaactaaattttgaatcttatttcctcatcacctgggatattatacgctatgcgcaggaacgcggactcttttacgtaggccgtggaagcggcgccaactccattattgcctactgcataaaaattacagatgtagatcccatagaactggatctttattttgaaagatttctgaacccttaccgtacttcgcctccggattttgatatcgatttttcatggcgcgaccgggatgaaattatccaatatgtttttgacaagtatggtccgcaacacacggccctgctgggcaccgtgaccacctttcaaaccaatgctgtgatccgcgaactgggaaaagtttatggtctacccaaaaaggaaatcgataaaatcctcgaaaacggcttccaggttaacctggaagccgacagcatccaccagaaaatagcatacttcagtaacctgatggatcaggaaaaagcattccctaatcatctcagtattcatgccggcggcattcttatcagcgatgcgcctattcaccagttctgcaccacctacctgccacccaaaggttttgtaaccgcgcaactggatatgtggcaggcggaaaggatagggctgcataagtttgatatcctcagccagcgcggtctcgggcatatccgtgacgctattgatatcatcaaaaaaaaccgggatgtggatatagacatccatgatgtaaaagccttccagctggatccgctggtgcgtaaaaacctgtccggtgtaaataccatcgggtgtttttatatagaatcgcctgccatgcggcaactgctgctgaaactgggatgtgatgattaccttaccctggtggcggcaagttctattatccggccgggcgtagcgcaatcgggcatgatgaaacaatacatacaccgctaccggcaccccgaggaagtggtttaccttcatcctgttatcgaagaactgctgaaagataccttcggtattatggtataccaggaagatgttattaaagtagcgcacaaatacgcagatatggaactggcggatgcagatagcctgcgaagggccatggcagggaaataccgcgggtccaatgatttcagggaaatacaaaaacgtttctttgataactgcgaacgcctgcaacgcccgccggaagtatctgcagaagtatggcggcagatcgccagcttcgctaacttctccttttccaaagcccactccgccagcttcgcagtggaaagctaccaaagcctttacctgaaaacctatttccccgcagagttcatggtggctgttatcaacaacttcggtggcttctacaaccgggaattatatttccgggaattactgaaaaccggggtaacactgcacccgccttgtattaaccacagcgactatgccactaatattaccggccgtgaggtgtacgtaggactgatccatgtagagggactggaacaattactggcagaaagaatattgaaagaccgcgaacagtatggtccgtttctgcacctggaagattttaccagccggatttcgccgggcccggaacagctggaaatactgatccgcattggttgttttaattttaccggctacactaaaaaagaactgttgtggaaaagcagcttgctggtaagcaagaaagaaaccaatccacacagcatgtctttgtttggcaataccactactgttaattgtgaactgcccaccctcgcttatcacgcccatgaagatgcctttgatgaaatagatctgctgggcttccccctgcaatcaccttttaaagtattgcagcacgatcaaagtgcgtatatgcctgtccgtgagttcggaaagtatatcggtcagcaggttaccacacttggctacctggtaaccaacaaatttctgcggagcagcaaaggtgaaccgatgtgctttggtactttccttgaccgcgacggcgcctttatggatactatccatttcccggacagcctgcggcaatatccctttcaaaagggcggcttttatgtgctgcaaggcagggtggcggaggaatacggcgtgatacaattggaaatcaataagatgtggaagattggttattttgaagataaaaaaacataatcccgacaatttgttgtatttttgtgacaaatgtcgggtatatgaaacatgtaaaaggataccgcgtgcaggaaaatgcattattaatagtagaacagccaggaggagcggcgtatattgccagcagtggctactttgattttatacagctttcccgcagtggaattattaaaagagctttattgaatctgagcaggcagctgtctttttctttatcagaactggcgcaggtagtacatgtgtcagaaagaacgctgcagcgctatgcagacgacgagaaattgtctgccgacacgtctgaacgtgccattttactctctcagctttaccagcgtggtaccgaagtattcggccagctggaaaacttcaaggaatggatgagaactccgttacctgccttcaactatcaaacccctatttcgctgttagataccacctttgggtttcagcttatccaggatgagctggggcgcattgaacatggcatctttgcataatttacgaaaccattaacatggaagtatacaggatcagtaagtgcgcttacatcaatgatcttagtggaacaggtgcgcgcctgtatggcggccgctggaacagcccggggcatgctattgtgtatactgccggcagccgggcgttatcggcgctggaagtactggtgcacattccgctgaaaaacatagtacaggatttctgcattgctaccctgcagattcccgatgatatcgccatcaaagtacttaccaaacatgatctgccatccggctggcaatcactggcgccctcaccggagctgcaatgcattggagatgagtggatagatacggctaagtacgcagtgctccggattccatctgtagtaattgcagatgaatataactacctgatcaacccgctgcatccggacgcgacaaatattaccatcctgaatacacagccgtttgtatttgatcagcggttaaaaaaataaaaaagcagcgaagtaatctccgctgctttttttatctgaagcttttttctattccaggccaaataagcccttattcagcacctgcaatgttttctctttaaactgaccattgatcaggatagaaatattatgcctgctgccaccataggaaatcatgcgtaaaggaatttcttctatcgcatcaaataatttggtgataatggaaggagtagccgccacttcgttaccaacaatggaaacgattgtctgatgataatccagttccacggtaccaaacggttgcagctctttcaggatctgatcgaggtactgctggttatcgatggtgatagataccgctacttccgaagtggtgatcatatcgatcggggtgcggtatttctcaaatatctcaaaaatcttgcggaggaagccgtacgccagcaacatgcggctcgacttgatcttaatagcaatgatgccgtcttttgccgcgatagccttcacaccgttgccgttaggcatttcggtaatgatggtaccttttgcttcgggttgcatggtattcagcagtttcaccgggatattgaagtgctgtgcaggccagatagaagcagggtgaaggatcttggcgccgaagtaggccagttccgctgcttcgtcaaatgacagctgctcgatcggaaaggttttgttcaccacccgcggatcgttgttgtgcataccgtcgatatctgtccagatctggacttcatctgcctggatagccgcgccgatcagggatgcggagtaatcactgccaccacgtttcaggttatccacttcgcctctggcattgcggcaaatatatccctgggtaataaaaatacgctggcctttatgctggctgatcaggttagccagtttaattttaatctttggaatttccggttcttcgtattcgtcgatgctcatgaaatccaacgcaggtaacaataccgcaggaattccggcttcttcgagatatacgccaaaaagacgtgtagacaataattctccctgtgcaaggatatctttattcagtgcttcattgaaagatatcttcaggatgatgttcagaaattcgaagtgttcatcaacaatagccttggcatttgcgcggccggcttccttcttcaccaggtcgttgcaaaagttccggtagtggctttccagcttgtctatctgctgttttgcctgttccttcttaccttctgacagcgactgactgatttccacgagggaatttgtggtgcctgacagtgcagacaggaccacaattttctgatcattatctgctgtgatcagttgcgataccgactgcatacgctctggttttcccacggaggttccaccaaattttaacactttcatctgaatgtatattttgctttagctacccgaaacgctgcatcagcctcattccgggcgttttttatgaacgattgtaaattaaaaattcaaattaaacttagcggcaacttcctgcatgtcctttaccactgccgctattaccgggatacccttttccagccgctcgtgttgcatttctctttcaggatctccggggatcaatactttctttccggctaccggctctgcagcacggaagcggttgatccaggtatccatattggccttgaactcatctgccggccggaacgcatctacacgcatagcgccaaagaaatgtcccaggccctctcctaccggatccggcgctaatgggagaaagctcacaaaaggcggcgcccacgggccataattggcgcctgaaagaacggccgaaaatatatcaacaattgctcccaaacaataccctttatgacttccgtgctcacgatcgccgcccaaaggcagcaaagccccgccactcttgagttcatgaggattgttacttgggttcccttctttatcctggatccatccgtaaggagcttcttcatttttacgctgcaggatctccagtttcccgttggccgcagtggtggtggcaaaatccgccacaaacgccggctgctcctttgcaggaatagccactgcaatgggattagtacccagcatacgcacagtggaaaaggtaggcgctaccagcggactggcattggtcatggccataccaatcatatcctggtccagtgccttcatagcatgataacctgcaataccgaagtggttggagtttttcacacttacccagccggtacctacggcagccgccttctgcatggctatttccattgcgtatggggctactaccaggcccaggcctgcatctccgtcaataaccgccgtactgggcgtttcatgtactatccggatatggggtgtagcgttgatccgcttagcctcccataaacgaacatagcccgataagcgggctattccatgagaatcgatacctctcaaatctgccgataccagcacttcactggccagggctgcatgttccaggctgcaccccatgtggataaatacttccctggtgaattctctcaaatgatgataagaaaaaatatgttccatctgtcaacaagttaggcctgagcggtaggtccgccaaaattcaatggtacagatacctgctcctgatcctgaatggggccgtgtacagattcgtatttcttaatattatcaagcatggctttcataaaacgcttggcatgctgcggcgtgagtatgatacgggatttcaccttagcctttggcagaccgggcatcacgttcacaaagtctaccacaaattcggcattggaatgagtgatgatggcgagatttgcgtattgtccctcggcgatttcttcattcaactctatgttaagctgattctgttcttcatgctgattttccatgttgtatgatttagccgtacaaaaatagaaaaagaggactcaaatgagccctctttttttataaacagcggattgaccgggattaatagtcgtcttcgtcgaacttggtacgcaggatacccgccactacgtacttcttgccgggatcggaagatatttgcagttccatgtaaatactgtccgttatgtgcccgcccttcgattttccgccgttggggaaaacttttccggcagtgatggtaacggtcgcgtcactgttttcgtccttggcgttggtggcgctgaaggtaagatcagacaaattcacgtccaccttcgactggaagtcgaatcccagtcctgcatcctgtacccacatctgcttgccatcatcggcagtggtgttaaatgtattgatctgcacatggtccccatcgatctgcggggcgccgttgagcgacatggttacccaccaggtaccggccattttcactacctgcgtattctttacctccggcaaatccttttcacaggaagaaaaaagaacggtagccaccagcagtaatcctatgatatattgtttattcattattgttctcatggtaattattttaaaccgttaacattataaagcccaccaaaccttttgataaataggtacttccgctggtgtattactattccggctcctttccacatccgggaataccaggcgtttagggaacttaccaacgccggtaacaccattacgggaatataccagctggccggggatgtaggacggatcagtggaatataccgggctgtatttgggataacctgttctgttttgttccaggaagccttccagcgcatgtgtgccggggaaagaagcccatttctgtacaatgatggcttcgagcttcttatcaaaagtagctccggttgggtaagcatatacctttccgggcagaaggaaagtatcagcacttaatttaagctgctgaaatgcggcctgcacacctgcatcataataggcttttgctttagtgccaccgaaataacgctcatctgcctctgccagcatcaggttggcttcagccctggatatcaggtatgcagtatcaatagctgtttgcctgtagatagcagatttattgtaaatgggagacaaactggtgaaatcaccctggttaatgccataataaacaccgcttgccgcgcccggcgcgcggaatattttggttatccgcgaatctttatttttctgtaaccacgataacatggtgtaactagcccggatattggtagtcgtattcaggctgcggatatttgattcgtataacggattgtcctggcccggtgcatctttaaaagtactgtaagaagcatctacatctgtaaggaactcagcgccgctgttaatcagctccatgatctttgttcttgccagtgatggatttacattcaccatacgcaggtacattttcagtttcagtgtattcgcaaactttacccatttatccatatctcccttatagataatatcctgtgctgcattctcatcaaggatagtaacggtcagatcttttgataaggcaatatccaggtctctcagcaaccaggagtaaatgctatctccacggtcaaacttcggctgcagctggtttaacccgccaaacgcttcctggtaaggcacctggtcgtacaggtctaccagtatctggtaagaatatgccttcatcacggttcccatcaaaccaaagttataatcgtgcaggctgtcgcacaatttgagcatcaggctgtaatcctgcagtgcgcctgaaaacatctgcgtgtacaacgcattgtagtccgtccgctggatattatacgcatcaattgttttgtactggttggaggcgttgctttgcgtccagtattgcgcccagataccaccaataacagcgccatcggtgccggcgcacgatatggtagacattaccgccggcgggaacaacacataaggtgtagccttctctaacggcggattattcggatcgttgttgatatccaggttcttcttgcaggaagcgcctaacaatagcactgctgaaagtaggaggagaatatattgattgtacgttttcatgatatcagaatttaaaagattagaaggataccttcaatgaaacaccataagacctggtagtcggcatggatctgaattcaccaaactcactgttcaggtcattaccatagttggatacttcgggatcaatgaatgtatttccttccggcgtccacacaaacaggttgcgcgcaaaaacagtcagcatgagattgctggcagcaatttttctggcggctgatgaaggcaaactgtaagagagcgtgatatcacgcagtttcaaaaaagttttatcaataatacgctgtgaataagcgccgcctttattggtagtatgataccaataagcatcataattataatctgtgagcggaatggtattttcaccatataccggtttggcctgtgcatccgtacctacctgcattacagagttaggcaccacaaaggcacgtctgtcgttataagtagttaacaaggcgttacccacgaagtaggtcagatcagctgtaccagagtagaacacaccgccttttctccagtcgaaagagaagcccagcgttaaatctttataacggagtgtgtttatcagccccatggtaaagtcgcgctgagaggtaccataataaccgtcggtatctgccgccttaggcaagccggtagcatccacaattatttttccatccggtgtggtagcaggtaccggtgcataaaatacacccagtggatctcccttacgtgcaacaaattttgcatcgtaagcgaaattaagcactacctggtccaaacctgcaggaagctcctctactgtattgcggttacgtgcgtatgtgtagttcagggtccaggtaaaatcttttgtttctaccggtatgatgttaacagataattctatacccttattcctcactttaccaaagttttgcgtaatactcgcataaccggaactcggcgtggtaggcaccgccaggatctgccctttggtgagtttgttatagtaggcaatatcaaaacccaacctgttccgcaggaattttacttcgccacctaattcatactcattacttaactcaggagcaagatcaggattaccgatgttgtcacctactgtgtaaccggggataccattaaaaggaaaatccagtgtaccaaatggaagatctatgatctgtccggtagataaggtggttttagtgagatagggaccagcatcgttgcctgttttaccccagctggcgcgcagtttcgcaaaagaaacaccgcggtcatccagcttcagcgcttctgataaaatgaaggcagcattcaccgcaggatagaaatagctgttgttcttttccggtaatgtagacgaccagtcattacgggcattcaccgtgaggaacaggtattcgcggaagcctaaggtagcctgtccgtaaaggccataaattctgcgtctgaattcctgtgtttgtgacaccggtgtattgggtgagttggagatcacatagaaaccgggaattgcgaggcctttcacagccgaagtgaatatttttccttcccgctggttaacgttaaagcctaccagtccatcgatagtaaaatctgagctcagttttttattggcagtgagcaggagatcggagttgaactcacccctgtaatcgctgttttcccttacataaccaacgtcctcttgccgttgcgatccttccacattattaccatcattccagctgtcgagtgatggcctgtttttcgccttataggttttagactggctgttggtgatatctgcaccaaggcgccattgtacacttaaccagtcattgataccatatttaaggtcaatgtttccgaagatcctgttgcttttcaggttattcccattttcatacagggaatagtaaggattctccgcgtaaggcgtgaagtagttatcaacgttgtaatatttgtttttgtaatccttaaactgggaaatgttgatatctaccgggatctggataatatcctcaaacaaggaagaaccgagtccggattcactgcgggtagatactgctttcgcatttttatttacgtagttaaaggaagcagaagcagagaacctgccgtattttgtagaggctcttgcagagaacgtatttcttttataagaatctgcgtcagtgggcaggataccatcgctgtatatatttccataagacaggaagaaagtggatgtttcatttcctccgctgatagaaatggtgttgttcagttctttaccggtagtgaaataatcgcgtacgttatcatctacaaaagaaaatggttttgttaatgacacaccgtcaacaggtgcgccccactcgcggttttcgccggtcaaccgcggaccccagctaccattctctgagagaataaaagtaccgccccatccctggccaaacttttcctgcatggttggcaacatgcctacattagaaaaagtggcagcagaggccacatctactttaagttttccgctcttaccttttttggtagtgatcaataccacaccactggcggccctggaaccgtagatagcggtggcagcggcgcctttcaaaatgctgattgcttcaatatcatttgggttgatgtcattggcattattaccaaagtcgtaaccaccgttgttgactccttttccatcaacgctggaaccgggacggtcgttgttcaatggcaccccatctactacatacagtggctggttgttgccctgcagggatgaataaccacggaggattactttattggatgcgcccggagcgccgctggtggtggatatttcagcaccggcaatttttccggataaaccatccatcatacttacaggcgctaccctgttaatttgttctgtagcaaaattactggtggcgtaaccaacggttttcttttcacgcaccagtcccaaaccagttaccactacttcctgcaggttcttgttatctgcaatgagtgttacctggagatttgaactttctcccacggttatttcctgcgctttatatccaacgcttcttattacgagcacggtagcggcaccgggcacactcaggttgaatacgccattgtcattggcggtggtacctgtggtgctgcctttaatctggatggtggcaaacggaaccggattgccatcgttgcccttaacggtacctgtaaccggtcgctgctgcgagtaggccaggtgaatgattgccataaccatggcaaaaaggaggaacccctttttcataaaagtttcagattttggttgaagaagaaatgcatcgggtcttataaatgcttacctggcaaacaattgccggtagctgcttccggataagatgttttatttattgttgtatcatattagcacattaaaataatagcataaaaaatccatatcatgtctttgtaagcatgactaaccatacagaataccattcggttctgcagttacagcaaacaatcatcgcaacatacggtcaggtatattggcgaccggctatgtaaaaggagaagtgtttttcttcataaacagttctgattttggttgtacaagtcaataatagatcagcatgtgttctctcgtcggtaaattgttgtattcgctcgctgttgacaaacagctaatgatctcaatttcaggaatggttacgtgcctgttatagtttaaatcggtaaaagccttactaagtctctcgttgtgtcttattgatttgaatcatgacaagtatcctgctgcgggtttacagccattatcacaagctttttttcttgcagaaaggtctttctcataaagcaaatcagatttagattttggttgacatccacaagttagaaaaaaaaagtaaatcgtgatacatctacttaacattattttaacagcagataattttatcaccataacaaactgataatcaatttataaccagcctaaaaaatttcattttcctgctattaaatattgcagctgaaattgaagcaatgttttcttatctcctgcaacaacgtcatttccactaccaatacgggtttgaccaggataccggctctgatggcaacgtgcccagcatgccagccgccggcttactttccattttatgttgagataatattgccagccctcgccatacagctgcgataccgcgttttcgtataacacactgctttccgttgcatatatcctgctatcgtaactgctggtctgaaaccgggataccctgccgccgattgatacaggcaaatgtataaaacggtaactggcatcctggtaaatcatccatccctgctgcatatcccctgccacttcgtaactgctgtattctatcctggttttaacgtccaattgcttatttacttttatactccactgaaaacgtatgtgcctggacgttacctctgccggtactttgaccggattctccggcagcaacacgttctctgctccctgccggtagttgtaacgaagtaacagggtcattgttttcccgggaacatagcttccctgcacaaagaagtccttgccataagaaggtgcattactccggtacttcaaccaggggaagtgaaacacatctgcatatgcatccgcctttaaacgggatgttattttcagggtaaccgccgtgtatattccctgctcattaacggtccggtagccatccccgaatcctttggcatacagcgactggtagcctttatcataataccggtacgcaatagccacatccaccgcaggcgctacgctggtcagcaatccctgaactagggcaggtttgccgttactgcttactgctgcctccccgaataagtgcacatttttccagctgccggaataatcaatactggcagccgtcagctggttaccattaaagtcgaactgattatagggcgccgtttccttttgaagtaccggcgttaaatgatggctggttacgtttccccctacctgccaccgggcagcctggtagcggatatttccaccaacgctcacctgttgtacctgtccgcgtttggctgcttctgtgaccgtgcggtggtaaccactgctgataatactggccgccgttacttcgtccatcagtgtgtctgtactggcgtcctgtttacggaaagaggcaaaggcggtcaactcccaacgtttttgttgtaacgtaacagcagctcccctgaaaaaataaaactctcccggcgaggtgtaaggccgcaacacttctccttcccgttttacctgcatcaccgatgctcctttaccataagcctggccctgccagttcagcaggccctgtcccatattcaccgtataatcgcccaatgccagggcttttattttccggtagttccggataaaaatatgtgcactgtaaaaatcaaatccctgcttttgcgcgcctttaaaaaaagcttccccggcatctttctccatcacgatcccccagctcatataccggggaaagctataacggtaacgcataaacactttttccggacttcccctgtaggcaggtaaggtgctatcggtatgcagatatccctttgctttctccgctgcgcgggcataacgcagcaggaacgaatgatcacccttctgcgtataatcccgtaaagtataatgtggcgccaggtcatcgcctaccgttacgtaaggcaatacgcgccggataacatccggttcaaaccccggcaccgcctgtagttcataaatactgagcagatctcccaacagcgcgcggtaccgcaaaaactggctgatctgtaaaggcgtgagcagtcctattgactgcaacgtcgcttcatctgctgtattcaattgtatcttatgccgggccaatgcatttaaagtttgccattgcgcatcatcctccggtaccgtttccgtaccagccgcttcgttctcaaggttattttccattgcctgcggcaacgtctcttcctgctgacgggcccacgctttccgcccgcccagcagcaacaacaaacaaccagtgatgccgcaaatcgccgagcggatagttgccatatcaataacattgaaagtttagcttccctacgtgatctccggtaaaaccaaaggccacgcctggttaacaagtccataaacttatacgcatcactccatcaccggtggtggagaaagctgccatatcaatgaggtaacgggcgtaatacccagttgcggatgaaaccccgcagcgatatctatccgcagggatctcaggaataatatcactgccgcactgttataagcctgaccggatgcaatacccatttccagcgccagctgccggataacccggtaataagccgatgccttgacagcagtaaatgcacccatagaaaccacttcaccggttaacaggaaatcgcgcgatgcttcaaaaccgaggccgccactatatagaacagacgcgtctgcgggtttatacacatgaaggccgccatgccactgctcactgatatgccagagcattccgccgtcaaagctgatgttaccggtcgtccccagcccctgcacactggtggtctcataattaaactgcagcccgataccggcccgccttcccagctgcatgccatacgcgccactcagccgctgctggtgccacgctgcattgcccagccgggtaatacttccgccgaaagcgcctgtacccgcaggaatagccaccattgcagcatacaacgaagcctcttttaacataaaccggttctctgtataaatacccgctgcaaaagaagataaacaggataagccggcaggattataccaggcagataccacctgctggaaatgccggctgtaactgccgctgccagtgttctttccaaccggcattaacaatggttgtgcatacaacagcgctatccaccacgtgaataagacggttaacaataattgtttcatcagggaattgggtttaacaataaaattccgcgggctaacgggttaactacttgttgccggcgaatacaaaaataagcagcggaaaaaatagaagtgttaatgaaacataaacgcgcgaggtttgtctttctcaggattacgctgattatattgattttaaggatttgaacattttggattttaaatgattttgggagatacaagctgatattttcgcttataactcccaaaaaatttataaaaaaagtaaaatcaaaaaaataaaatcaggtatccgcctacatctcccaaaatcatttaaaatccaaaatgttcaaatccttaaaatcaatataatcagcgtaatcctgagaaagacaacctacgcgcgcgctaaaacaagccgtataactgtgaatcgatccgcgaaataatttcgcccaggtcttcatcgctctcggggaatttattcttatcaatatcaatgatcagcaacgggccttctttgtatttctcaatccagttgttgtaatattcgttcagtcgtttcagatagtcgagccggatgttttcttcatactcccttccccgcttctgtatctgcgctaccagtgtaggcacagatgcctgcaggtagatcagcagatccggtggtttcaccatgcttttcagcgtttcaaagaagttgaaataattatcaaaatcacgtttggtcatcaaccccatttcatacaggttgggcgcaaaaatatgcgcgtcttcataaatggtccggtcctgtataacggtttcttttccgttctgcacttccagcagctgctttaagcgcccgttcagaaaatatacctgcaggttaaacgaccagcggggcatatcttcataaaaatcgttcagataaggattgtgctccacatcttcatactgcggatgccatttataatgcctgcacaacatttctgtcagcgtggttttgccggcgccgatgtttccggcgatagctatatgtttgatcttattctgttttgccatgcgatgtgaggtggttaaaactgaaaatagctacagttggcgactttttcaataataatttataccaataagttttttcgcctgttgcaaagtttgtgccgcattcgctctggccttttctgcaccggctttcataatcttcttcaggtagtctgtatcccgctgtaactctttcgcctgctcacggataggagagataaacttcaccatgtcttcacccaattgctttttcagatccccgaaacggatagtcccggtattcttccatgcttcttcgtagaaagataccgcatctggtgcagacaccagtttcatcaggtccagcaggttttgtaccgtttctggaatcggcgaaccgggttcaccggaaccactgtcactctttgctttcttaagcttggcaatgatcatgtcatcctcgtctgccaggtataacgtggccatttcattctcgctcttactcattttacctttaccatccaggctggggatacgtaccaggctatcgccatagttgaacgcctccggctcggggaacaggtcaccataacggtgattgaaacgctgggcgaagttacgcgccatttccaggtgctgtccctggtccttacccaccggcactttcaccgcgcgctggatcaggatgtccacactcatgagcaccgggtaggtaagcagccctgcgttcacgttttgaggctgcaaccgcaccttatctttaaaagtaggtactttctccagctcacctacataagccagcatattcatcagcaggtataattccgcaatttcgggcacgtcgctctgcacatacagggataccttttcaggatccagtccggatgcgatattctctgccagtacccgcatcacgttccccggaagatctttcggatcgggatgggtggtcagcgaatgccagtctgccacaaaaaaatagcagttaaaatcttcctgcatccggatataattacggatagcgccaaaataattgcctaaatgcaaataaccggtagggcgtatgccgcttaccacaatttctttttcagtagccataacagggcgcaatttaaagaatagcttttagctttcagccattaacaccgggctgttttgtaaaaaaaacgccaaaagccaaaagcagatgatcaaaagcactttattctgtccgtttatccctaattttgagatactatcatatttaccatttatatttcattatcttttgatttaatttgattatggaagtgaacgacgtactggtgcagcaactggccgatctggccaggttggaattcaacgaccaggagaagattgaaatacgcggagacctccagaggatgatcacctttgtggagaaactgaatgaactggataccaccgatgtgaagccattacttcacctgacagatgattataatgttttcagggaagataaggtaataccggtaatcacccgtgaagaggccctgaaaaacgcaccttccgccactgaggaatactttaaagtgccgaaaataataaagaaataacccacatggaaaagtccgtcatacacctggaaggaatcaggaaaagttattttctcggtaaaaatgaattaccggtactcaaaggcgtatcgctggacattttcaagaatgaatatgtggcgctcatgggcccctccggctcaggaaagtctaccctgatgaacatcctcggatgcctggacacgcccactgccggcaggtacgttctcagcggacatgatgtgagcaaaatggaagacaacgacctggccatcgtacgcggcaaggaaatcggctttgtattccagcagttcaacctcatgccccgcctcaccgccctggaaaatgtggccattccactgatctacgccggcatcaacagaaaggacagggaagaaagagccatcgccatgctgaaaaaagtaggcctcggcgaccgctataaacataaacccaatgaactctccggcggacaatgccagcgcgttgccatcgcccgcgccctggtgaataatccgtcccttatcctcgcagatgagcccaccggtaacctcgactcaaaaacgtctgtggaaatcatggaaatcttcggggccatccacgactccggtaacaccgtagtgctggtaacacacgaagaagacattgccgatcacgcccgccgcgttatacgcctgcgcgatggcgtcattgaatcagaccgcatcaacgaaaaagcacacgcataaaatatttcgattactgcataacggcgttacaggatacttcccgtaacgccgttattcgtattttgcaaccgatcaacaccaacacccatgtctttcaaaatatatactaaaacgggcgacaaaggcaaaacatccctcatcggcggcaccaaagtgcctaaaagcgatgtccgcatcgatgcctatggcaccgtggatgaactcaactcctatatcggcctggtaaacgattacatcgcagacccggacaccaaaagcctgctccgcgaaatacaggaccgcctctttaccatcggcgccgcactggcctgcgaccccgacaaagaaaccaaactgaaaataccagacctccacgaaggcgatatcaccctcctggaaaaaagtatcgaccagatgaatgaagagcttcccgtgatgaaatcattcatccttcccggcggacatgtagccgtatctacctgccacatcgcccgctgcgtatgccgccgcacagaacgcctctgcgtaggcatgcaggagcacgatatgttcattgaaccgctggtactcaagtatattaaccgcctcagcgattacctctttgtgctggcgcgttggacagggcacaagctgggcgcggaagaaattccctggaaaccccgggtgtagaaaaatgcttaaatttgccgcatgtttacaggaatcatagaaacactagcagaagtagtatccaccaggaaggaaggcagtaacctggtaatcacgatacaaacaccactggcagctgaattaaaaatagaccagagcgtgtctcataacggcgtatgcttaacggtaaccaatatccagggcgatacctacgaaaccgtagcggtagatgaaaccctgcagaaaacaaacctcggccagctcacccctacacaattcgtgaacctcgaaagagccatggtgttcaacggccgcatcgatggccacctggtgcaaggccatgtggatagcgtaggagaatgcctctcctgccaggaacaggatggcagctggttataccgcttccgctaccctgccgaattcgccgcgctgattgtggaaaaaggaagcatttgcctcaatggtatcagtctcaccgtattcaatgtcaccaacgatgagttctctgttgccattattccatacacctacgaatttaccaacatctcaagtataaaaaccggcagcctggtaaacctggaatttgatattctcggtaaatacgtagccaggcaaatggcggtaagaaattaatcagccggttgtccaccggtgctaaaacattccaaaccgcatgctgaaatatctcctgctctgcaccttacttgttatcaccctgccggcaaatgcccaacaggccaaagtagcgcgcatagtggccttttacgatgcagatgctgtgacggaattgtacaacaccgcgcccctgggcatccggattatttataccgatagctccacccagcaaactaccggactcctggaaggaaacctccgctggaacaaactaaccgttagcagcagcaacgggcaaatacaaaacggcgtactccgttttaacagggaacaactggtaaaagataaataccgtataacccttaccgttactacacccgacaacacctcccatcaaaccaccctgcaactccccgccattaccgctatccggttcaatcattatgccgacagcataaaacgcgatatccgcttctacctgaatatagaaggaaaattcagcagcgggaaagtattcccgttagataccaatgccatcaggttcgctgcctccgcaggaaaaataatcggacaggatttattactcccaaaaaatgataccctgaaatcagtaacagtggaagcctggtacaaacacaacgaccgcctctacctgcgatccgtgataccagtaaaacaggcgccggacgcagactcccttattttgaaaaatacagacgacctgtttaaaaagaagagaagacattagccggtctaaaaaccaacaccttccgtgtttcttttgcgaatagcttcttcggttcccggaacaagcgtttctaaacccatgcgtatagcttctgcctgaacctcctcaataaacggacggaaatttttgttgtaatcctggaaggctaattcaaaatctccattgtgttgcagaaaagcatccgctaatgcggcagctccatctattgccaacgatccgccctttcccgcagcaggagaagcacaatagcctgcgtcgcccaccagcgccaccctgccttttgtccacgatggcatttttacctggcaaagcttatcgaagtaaaaagttgtagcattcattacttcgtccaataattccgcagttctccagctttgttcttgaaattgttccaaaatgatttttctttgttgttcttcatcacgataatcgtaagtaatttccttctctgaacgaaagcagaaaattatatcagttttgttattgtaagcatttagcattactgccttatcaggcacgttatagaattgcgttgtattttgctttatcagcaatttatttacgatggtgatagagaaatattgcccgagaaaatgcaggtatcccgcttcattgccaaaccagatcttccttaccgccgaatgtatgccgtcgcagccgaacactaaatcaaaagcctgttgtgagcgatctttaaaggtaacttcaacatcgtcgtttgtttcgtttaaggcggtgatgctgttgttgaaaatgaattcaacgtcatttttcaccgtatcaaacaagatattgagtaatgcgtttctttcaatctcgcattcgtcttcccgcagttgttcaccttccctttttaatatcatggttccttccgtaacatcatctgcatttttaaattccagcatttccatctccaatctggttgatttaatttgctcaaagattcccatacgcttaacaatatcaacagtattcccttctatgttaacaggcgttcctcccattttaaggccgtttgcgatttcaacaatagttactttgtaacctaacttattcatccaataagcggttgaaaggccggcaaaacttgcacccgaaacgagtacttttttatcttttaatattttcatttttatacgattttatttgaccatacaaaggaacatcgtataacagggagaaaaaataacaatacaaagtagatattggatcaaccgaggtttttattccggaaagctaaaggggttattcctgtgattttggtaaatagccgcgaaaaataagggtaatcatcataccctaatgcggtagcgatttcctttaccgatttaccggaatggtagagtaaacgttttgcttctaaaataacacgttgctgtatgtgatgcgatacagaatggcccgttgtatttttgacacattcgttcaggtaaggtgtggatatatttagtttttgggcgtaggctgccgggcgtttgtcagtggtaaaattatgctccaatgcttccctgaaggcttttgtaaccaattcaaagcgcggaaatttctctattggtgtagattgttctaaatacagggacaccaccaatgcgaccagtgcattacagctatctttcagcaaggagtgatatagtttgtcgcttgttcgttttgaaaatttcaggcaaagtgatacggcttcggaaataatggaatacgtttctttatttaaggataatggttttgtgggtgtaatgtcttctaataatcggagatattcagggttaatatctacattattgatggcccaggtgctgacttctacattttcaaatgttattatacggtgtacctgatttgggtgcatgtagatgatagacggagactggatttcatacttttgaaaatcaatttcgatcgtaatggcgccttcctcaagtaagtgaaatgaatgacgatcatgccgctcagattgttcctctccttcgaaaccggggaaatctttaagagatatccgctcaatggaaatacctggatgatattcacctccgaaatgatttacaggaatggatcttagtttttttggcattgcttgttgtggcttagatcaacatacgtgattttaattccaggtatttatttaccacgtttaacgtcaattgctccgggggactcagcaacgacataattccatatttcgccagctcttttacaatcaacttcttatcatacgcaaacttctgtgcaatggtctgcctgtaaattccctccacatcctgcaccgtttgttctgttaccctcttcagttctgtattttcaaaaaacaccaccagtaccaggtgataacgtgccaggcgccgcaggaagggtaactgccggtgcaaactggacatcgactcaaaattagtatagatcatgagcagggaccgcgtagataagctactgcgcagctgcacactcaatgcttcgtaatcactttcctgccaccgcgtttcctgtgcatacaacgtttccaggattttatttacctgcactttcttattgctggcggccaacacttctactttattttcgttgaaagtaaccaaccccgccttatcgcctttatccaccgccacattgctaaataccagcgacgcattaatagcgtaatccagcaacgataaaccgttgaaaggcatcttcatattccggcctttgtcgatgatggaatatacctgctgcgatctttcttccacgtaattattgatcatcaggttaccgctgcgggccgtcgctttccagttgagcatacgcacatcatccccttttgtatacggtttgatatgatcaaactccatgctatggccaattacccggcgcttatgcacacccagttcattcagccggttcatgtaggaatacaatgcatagtgccgcaactggtgataactcggatacacgctgatcgtttgttcattatcaaaaatgaaccggcggcttacaatgcccaatgcacttctaacaaatacgttgctgtagccaaagttatacagccctctttccagcggacgcaacacataccggaaaatatgagaacctcttgcggatacttttgcctgtaagagaaaatcacgctcctggaactgaaggggcaattcatctatcacagatacaaataccggaaaggggtaccggctgtgaaaatccagcaatacctcgttatcatccccgttgctaaaacggttactggttttccgttccatcgatacaatactggccggtcgcaggatcagcaggatcatatccagcaatacaatgcccaccagcacaataaatgcaatcacagcaatattgaaaatgcgcggaataaaaaacgaaatgataaataacaggatattccctcccagcaggaggtaaagcctgttggtaaaaaagagtatctggaataaattattctttacagtggctgacatactaatatcttcttgggagatgattatctcggtacctctatcgtttttacgatctgtgcaatcacgtcatctgttttgatgccttccatttctttttcgggcgtcagcataatacgatgacgcaatacatgcggcaccatttccaccacatcgtcaggaattacaaaatcccggttcttcatggcagcggtggcttttgcacagttcataacagcaatggatgcacgcggagaagcgcccaggtacagcgaggagttcatgcgcgtttcattgataatagacgcaatataatgaaacagcttttcgtctattattacctgccgtacgaggttctgaaattcgatgatctgcgtggtagttattactttgctgatcatttttgtaagatctgtttccccgttgaagtgatgaatactgcgcaacacagctacttcttcttccaggttaggataccttacttctattttaaagaggaacctgtcgagttgtgcttccggcaaccggtaagtaccctcctgttcaatcggattttgagtggcaatcaccataaagggccggtcgagcgaccaggtggtgccgtcgttggtgatttgtctttcttccattacttcaaacaacgccgactgtgttttagcgggggcacggtttatttcatcgatcagtaccaggttactgaaaatgggtcctttcttgtattcaaactcgcgtgtttgcggattaaaaacggaagtgcccaatacatccgccggcatcaggtcgggtgtaaactggatacggctgaagtccgcatccacgcattgcgccagcaattttgccgtgagtgtttttgcaacgccgggaacaccttcaatcagcacatgtccctgtgtaagcaagcctgctatcagcaggtctaccatctggtgctgtcctacaattactttccctatctgttccctgatggcttccacaccttcatgcaaggcagaaaaatcagtcctgggttgaaatgtattggtatccattatttatttcgtgtttatataaaattgttgaatgcggttataaaaatctttcagatcatcgtcgctgatattttcttccagctgtatattgtgtaccatctgcaacaacgccctgatatccgcttccggcaccagcgacttacgcgccagcgacgcaataaattcatcattcagcacattagtattgagataataactggaacgtatatactccataaaatgaatgatcattttatgcgccaggttgtagttgttatgttgctgatagtacaattgaccaatagcatctacaaactccagtgaagtattgtttacggctggtttatcggggataatccgttgccggcgtttgctttcaaacactacgtacagcagcagcaatatcaccgacagccacaacgcccaacgcatggatgcataccgcatcagcacctgccactcactgaagtcgcccgactgtgcgctatgctgactgttatagaaatcatcccagtacacattgccggcatcactgatcaggtacgacatctgcgtttccagcgcctttacattctgcttgtgcagtaaaaaataattcgtgaaagtatatggattcagcagcaggtaaatgaaaccgccgcgatacgcaatacggatgaaatcgggcttgtttttataattgtagccaagtatactggtagtattactatctaccgatgaaaaataacttccgcttactctgccaggataactgaaagaggtatccattggaatggtttcatcagcataccgttgtacaacaccttcttttttgagttgcatattattgctttccaccgtcacaaatttcaggtgtttttccagcagaggatccggcgtatttacagcaataaacaactcgtttccccgtgatacataatccagcatggcctctatatcgctttcagtggtgaacagccggtcggccaccaggatgtatacattgttcctgaatttcagctcactgtccttatcaaaagtgcgggcaaaaggtttcgttaccacctgcacagaattccttataaacagctggggcagcatcttaaaagcagcataggcgccgcctgcttttttatccttgctgtaaaaagaagactgggtcatatctgtggattgctcattttttttgttggcgagatttccactcaccatgaccagtactaccagcaggagcaaaacgaacaggacgatatatagaggtttgttcttcacgaagtttttccgattgtgttattaaaatccctgaactcctggttaatattcctgaaattctcttcactcacttcaaatccgccataccagatatattcataatccaacgtcagcgtagcaaattttttatagtagggagaactccgcatactgcgcaggtaatcgttattggttttttctctccccggtactatcagctcccggcctgccagttgaaacaaggtatacaggtaccaccagcggatagcttgtcttgtttccccggcagctattgccgcttttatcttttcttcatactcctgtgcactttgcaggtcttcttcctgtacttctgttaatccttctaccagttgcggtttacggaaaaagctcatgccattgcttttcataaaccaatacaccaggaagcccaaaccggccagcagcaatagcatcacaatgatgcggatagcaccgatcgatgaaaataaagccattaggaaacgttgcacccagctattatccgggggcggttccggcggtatttcctggtattgcagcttcttattttctttcagcgctttcaccagtgagtccggtacctcacgcaattcaaatggtggaatttctgtcgcatattcttcttcgccttccgcacgctcccgctctacctggatggtagcgaagctgtcttccgttatccttgcctgcaataagctatcgtattcttctttatttcgggctgtaccttcatattgcgccatgctttgcagggcacagcaaagcagcagtaacagcaggctgtatttaatccggagaaaatgattcatgttactgctttgaaagggtaaatggtgttaatactttcccttccgcactcagccggtatccttttttatgcaggtaaatgggataaaaaataaaatagcccaggataaaagccagtgatgccaggaggataaaaagacttaccaccagcggcatttctgtataccgggttacaaagctttccaggaaagcggccacaatgaataccgggatcagggttaccatgatcttgataccgtcttttgcacctttacgcagggaatcgatccgcttgcgtgtaccggggaaaaggatgctctttcccatgataatgcctgcacaggccgcgatcacaatactggatatttccagggtaccatggatccagatcaccaggatagatttccagccgaggccatgcgaaaagaagatatactggaaaacgcccagcatcacaccattgcgtatcaagagatataaggaaccaacacccaggaaaatgcctccaatataacaatagaaagataccatgatattgttgtaggcaatccggaaaaacatcatcaccgggttaccgtctttatacacgccgaaaggatctttattggcaatattgcgttccgtcatgtttacatattcatcgcccaatacgccacgcacaaacgtttcatcgtgtgctgatgaaaaggcgccaataatacagaacaataaaaagaaacagagcgtaaataataacaggcggtggtgcttacggaacaacagtggtaattcatatttaaaaaacaactggaagcgtcctacatcttccttacggttctggtaaatacgatggtagatacccgccgccaggccgttgatataacgggttactttactgaagctgtaaaaagttttagcgtaagacagatcatctagcagtgatacaaatctttccgccatttcatcagggtcatctgtcggttcctcctggtatttcttccagcgggacaaattttttttgataaacagcgattctctcatagtgagtcctttcccttttaaatacagatatcacctacagtaatgggttactaatgggggaataccggcaaacatactaaatcgttcaacaatatatcaacaaatatgtaaatttgagtatggcagatataaaaataccgacttctttcaatatagacctggaatttgaatcagcagacatcatgaaaagattcctggcgtggctcattgatttcggcatccgttttttttattacctggtggcgtatatgacattgagttctttccgtatagagatggaagggcatgtcggcatctactttttcctggtattgctgcccctgttgttttacttccctgtggcggaaatcggcatgaaaggacaaacacccggaaaaaaaatactgcacctgcaggtggtaagtatgaccggcaaccagccaagtataagtcagcacctgataagatggatattccggatcatagaaacaccgctgtattttttcgccctggtaccggtgattataccggcagtatctattgtgcgcaccccttataaccagcggctgggcgacctggtagccggcaccattgtgatcagcaccaaaagaaaaggcagtatagaagaaaccatcttccgggatctttccaacagcgattacaaaccgcagtttccacagatcatgaagctgtctgacagggatatgaataaagtgaaagacctgctggaccgcgcactgaaggcgaaagacgacgagctcgccgccagggtggccatgcgggtaagagaagtattgcatattgaaaccgacctgcccaatacctatttcctcgaaacggtactgaacgactataattactatactactaaagaaaattaatttgcgccttctgcaacgtatttaaatacttccgtaacatttatgaccggtagtaagggagaattattaaatagcacctgataagacttaatttaagctggttcgttcttaataattatctgatgaaaacattattgttttgtttgctggttcttctttccggaagtgtatatgcacaggaggatcttgcactggtgggcgccaccatatatacctctcccaaaacggcaccaattatatcaggtgtggttatcatcaaaaacgggaaaattgcagcggcgggcaaacaggtaaaagtgcctgcacatatgaaagtactggactgcaaaggcctggtgatgatggccggcttctggaacagtcatgttcattttattgaacccgggtgggaccatgcggacaagcagccggcagcgcagctcaataaccggatggatagcatgatcaacagtcgtggttttacacatgtatttgacctggcggcgctgaactatcccaatttgcttgccctccgggccaggattacatcaggggaggtaaacggccctgctatccttacggtgggcgttccgtttgttccgccgcatggaagtcctttctatattcagccgcttacccttccggaaataaacacgccggaagaagcggtggcttacgttactaaacagatacaggccggcgcagacggcatcaaggtatggtccgcatcgccggatgggcatgggattgtaccgatgcctatagacatcatcaaggctgctaccagcactgcccataaatttcataaaccggtttttgcccatcctactgccgataccgggatgaatatagcgcttgccggcggcgtggatatccttgcgcacgtggccccggatggttaccgcagctggacgaaaaaagaaattgatcaactgctgctgcataaggtagcgctcattcctacgctgaaactttacaaatgggaactggaaagaaagaacctcccggttagtaatccgttgatgacaaccgcattgcagcaattgggcgcctatgccggcgcaggcggtgaaattttattcggtacggatgtggggtatatcacggattacgatacgtccgacgaattccggctgatgtctgacgcggggttaagcttcgatgagatactagcggcgttaacaactgctccggcaaaacggtttggcatggcgcagcacagcgggcgtatcgcgaaaggaatggatgcggatattgtgttgctgaaagcagacccgcatacagatagccgccacttttcagaggtggcttatacgatccgtaatggtaaagttatttacaacggtattgaccggtaacatcaaataaaaagagggcgcctcaaaatgagacgccctctttactatcttatttttgatcaggccgtttttcctattgagttcaggtcttccgtaacattattaaaacgggtgggatcgcctgccggtcctttgtacacgatggtacggtcgaacgccaggataggataaaacacgataggcagtaataccaggcctaccgtaaatccttctgatttaccaaaacttttactgagcagattggttgcccaaataccccaaatggctcctacataaggaatacacatcaggagcaaccaataccatggtttgccaataatctgggtaagcacataaatgttgtagatagggataattgctttccaaccttcctggccggctttctcgaataccttccacatacagaaggcgaagaaaacgataattaccagcatgataattaaaaagacaccgctaaacatggcgctaaaaacgctgccgccttcataagtagttgtttccataattgaggtttatattgttttgaaaatgaatgatgacaatactttgggatatgtttacattccaaatatatataattttttccattacatagcattgtcagtattaaccttaaaagattgcgtattcctacggtgttaaaaaaagtttcaacatttctgttgctaatgtttggattttcaacgcattctattacctttgcaaccggcaagtcttatacgaccagctcctactgaactcccccaggacaggaatgtagcaagggtaggtggttgtagcggtgcgatataagtaacttgcctttttttctttttttattgtcattagttgcttgtcaatagtatctggttgctattttctccacctctttcactaatgacagcttctcccaaatgttcatttcctgacaactaatttatcatagtatgaaattctttatcgatacagctaatctggcgcaaatcaaagaagctcacgatcttggcgttctcgatggtgtaaccaccaatccttccctgatggccaaagaaggtatcaaaggcgaagctgcaattatcaaacattacgaagatatctgcgaaatagtagatggtgatgtaagtgcagaagtattatctacagattttaaatctatcattgaagaaggtaagaaactggctgctatccacccgaacatcgtggtgaaagtgcctatgatcaaagacggcgtaaaagccatcaaatggtttaccgacaatggtatcagaactaactgcaccctggtgttctctgccggtcaggctatcctggctgccaaagcgggcgcagcttatgtttccccattcattggccgtatcgacgataccaactgggatggtgtggaactgatcgcacaaatcgcacagatctacagcttacagggttacaaaactgaaatcctggccgcctctatccgtagcgcactccacattgtaaaatgtgctgaagtaggcgccgacgtatgtacctgcccgttagaatctattctcggtctgctgaaacatccgttaactgatatcggcctggctaagttcctggaagacgcaaagaaaatgtagtctccatattttttagatggtatatccccggtgcagtaattgcgccggggattttttttgcgcatgcggaggttgtctttctcaggattacgctgattttactgattggcttgatttttacttttatgattttacaaaggattaagatagataaaagcagatatattcgcttatatctacccgaatcatttaaaatccaaaatgatcaaatccttaaaatcagtaaaatcagcgtaatcctgctccaagacaatttaaaatcgccgaaggcgatcatattcgggaatttatctaaattcagtgataatatccacgtaaacccggtaacacacaaaatgaatagctaatgggaaaatacattctttcgctggatcagggcaccaccagctcccgcgccattatttttgaccacgatggcagcatcaaagcagttgcccagaaagaatttaaacagatattcccacaacccggctgggtagaacacgacgccatggaaatctggacttcacaagccagcgtggcggcagaagctatactgaaattaagagtaaccggtgaaaacatcgccgccatcggcatcaccaaccaacgtgaaaccaccatcgtgtgggacaaacgcaccggtaaacccatacacaacgccattgtgtggcaagacaggcgcaccgccgcctactgcgattccctcatcaaagaaggaaaggaacaacttatcaaagataaaaccggcctccgcatcgacgcctatttctccggcaccaaattaaaatggatcctggacaacgttcccgatgcacgcagaaaagcagaaaacggcgaactggcttttggaaccgtcgacagctggctcgtatggaacttctccaacggcaaactccacatcacagatgtgagtaatgcctcccggacattgttgttcaatatccacgacatgcattgggacaacgaactactcgctctcttcgatattcccgcctctatgctgccggaagtaaagcagtcgagcgaagtatatggctactcggaagccaatcttacgccctaccgcatccccattgccggtattgccggcgatcagcaggcagccctcttcgggcagatgtgcacgcaacccggtatgctcaaaaacacttatggcaccggttgttttatggtattgaataccggcgataaacccattccttccaaaaataacctgctcaccaccgttgcctggaaaataaatggcaaaaccacctacgcactggaaggcagtattttcatcggcggcgccgtagtacaatggctccgcgatggtctcggcatcatccgccactccgcggatgtggaaaagctcgccgctaccgtgcctcacagcgatggcgtatatttcgtgccagcctttgcaggcctcggcgcaccctactggaaccagcatgcacgcggtacgatggtaggattgacccgcggctccaccgccgcgcatattgcccgcgcagccctcgatagcatcgcctttcaaaccatggatgtcatgaaagccatggaagcggacgccggtatgcccatcaccgaactacgggtagacggcggcgctacaaaaaacaacatgctcatgcaattccaggcggacctgcttaatatcagggtagtacgccccaccatcaccgaaacaaccgcactcggcgcggcttatctcgccgggcttgccgtcggctactgggacagcattgaaaccattgcgcagcaatgggaaatagatgccaccttcgacgcggcgatggaacccgcagaaaatgaacggctgcgtaaagaatggaaacgcgccatcagggcggcccaggcatggaccgaagaataaatttatccacgtttatcaatactcatattaatttatgtcaccttatttagcagaactaatcggcaccgcattcctcattgtactcggcgatggcgtagtagccagcgtgatcctcaacaagtccaaaggcaaccagggcggctggatcgttatcaccctgggatggggaatggccgtattcatcggcgtatatgccaccgccaaatacagcggcgcccacctcaaccccgccgttacctttgcacaggcgctgcagggaaagctcgcctgggaggaagttcccggctatgtagccgcccaactggccggcgcaatgctgggagccctattggtatggctcacgtacaaaaagcacttcgacgaaacacccgacgccgacaccaaattaggcgtgttctgcactattcctgccatccgtaacccgaaatataacttcctcacagaattcatcgccaccatggtattcatcctggctatctcctatatcaccggtcctaccgctggcatcggctcactcgatgccctgcccgtagccttcgtagtgctggccattggcctctcgctcggtggccccaccggttatgccatcaaccctgcacgtgacctcggaccacgactcatgcacttcctcctccccattcccggcaagcgggacagcgactggagctatgcctggattcctgttctcggcccgctggcgggcgcggcagcggctgcgttcctgtatcaatactggcttcattaattcggagcggagcggagattgtagcgaaggttgtcttaagcgctgattacgctgattttgctgattggcttttgggattttagcggagatggaagcggaggttgtctttctcaggattacgctgattttgctgattggcttttgggattttagcggagattgtcgcggaggttgtcttgggcgctgattacgctgattttgttgattggatttttgtgattttgaaagaattttggaattttcagggaaattgatgggatgaattttaaagattgaataaaattgggaaagggtgggtggttgaagaaaggttgaataagatagtattaatattgaccgtggaatgcttcatttgtactttgcataggcttagcacatacttaatggatacttaatggatgcttgatacatgcttaatctatgctgataacccggaggtgatgtggaggtgatgtggacttgaagctaagatcttttatggtgcggcattacgagcgaaaaagcacatggcgtttagacgctgaagtgccatatagctgaaataacgtgccaacgtatcattcaaattcaatgaccggcagccaaatcaatcactgccgtcaaataccgcccatcttccataattatttagtgaaagcaaaccttttaatttccctaaattttccgaaaatctcttaaaagaacaaaaaacaaaccaattctatggacaaaatactgatagaaaaataaaaatccagtaatgcttttccacctttcaaaagtccataatcataaaatccaatcaataaaatcagcgtaatcctgaaaaagacaacctccgctcccatcttccaaaatctaaaaaagtcaatcagcaaaatcagcgtaatcctgagaaagacaacctccgctccaatctccgccccatagttttcatttttttctgaaagtttcgtaactttgagaatcttattaccatatcatcgcaactgcggcaatataaaatgacgaattatgattcagcccaacatcccggaaacaaaacaaccgcgaatcgttatagtaggtggtggattcggcggcgtaaatcttgccaaacaacttaaacatgcacccgtacaggtagtactgctcgaccggaacaactatcacctgtttcaaccgctgctttaccaggtatctaccgctggcctggaaccagatagcatcgccttcccgttgcggggaatcttccggaaacaacgtaacctcgtattccgcatggcggaagtaacaggtatccgctctgaagaaaatatactggaaaccggtatcggggaaatacattacgactacctcgtttttgccaccggcagcaataccaacttcttcggaaataaagatattgaggacaatgccatcggcatgaaatcactcatagaggccgtgcaaatcaggaactatgtggtgaaacaatttgaagaaagcctgttgctgcaaaacccggaagaaataaaaccaaagctcaatttcgtgatggtaggcggtggccctaccggcgtggaactggccggcgcctttgcagaactccgcaaatacattatgccgaaagactatcccaccctgccccagtcgctgatgaatgtttacctcattgaagcaggaccaaaactgctggcctccttcagtgaaaaaacatcacagaaaacactggaggccctgcaggaaattggagtccgtgtactaaccaataccggcgtaaaagaatacgacggcaaaaccgttaccctcagcacgggggaactgattcaaacgcaatcactcctctggagtgccggcgtaaaaggcgtcccggtaaaaggtatcccggcggatattgtcctgccaaacggccgcatcatcgtaaatgaactgaaccagctcaaaggattcaccaacatatacgccatcggcgatattgcccagatgaccaacgatccccgcttccccaaaggctacccgatggtggcgcaggtggctatccaacaaggcaaaaacctggcacacaatctcatgctttcactggaaaacaaacccatgaaaggatttaattataaagatctcggcagcatggctaccattggccgcaacagggccgtagccgaatttgccggtatgcgcatgagcggctacctcgcatggatcgcatggatgatcgtacaccttctcagcctgctgggattcaggaataaactggtggtattcatcaattggttttaccggtacttcacctacgaaagaggcacccgcatcatcatcaaacgcggcgccgccaatattgttaaactacgccaaagcatcggcgcataaataaaaagcaacagggagatgaatgatttcatctccctgttgctttttatttattccttacttacggttaagaatagaattcaatgtaattgacgataccagctcgtcagaccgcccacccagcgcccggtaatacaacaaaatggtatagttgttttccgtttcccaatgatcaccctctgtcatatcagtgctgaactttccattgggattggttttatctaccatcccataaatgtaattatagtatccctgcttgaggaaaatagtgccttcataagcgcgactggccccattatacgtaagcttattcgcgttgtttagctcatagttggtaaactcgccaaagatatacatctcatatcccgcataaggctccggcgccccaaatgaaaaatgtacggaagcataatccccttcaaaattaggatcatagtcatccagcgtagccaggtaatattttccgttgatatctttaataaactgatacggcttatccgccctttcctggtccattaccgcaaatacatctgtactgttgttatgatactcggaacgctgcaccctttcggtctgcaaccggaagctgcgcaggtcaatccagcggaattccttacctgccggcatgatacagtcctgttctgcattgtatttcaggatgttcccattaatgaactgcggcttcaacgtggtaagcgcattgtcccagcggtagttctgcaacaccaccactttgatctggtcaaaaggattctggatattcagggaaccggtatttacttcaaaattgatcttctggtgcgtacggaatagtttaggggcaatgggttgctggataaatcctgctatccctgctttattttccaccacaaacatccggcgggtaaatgccagctgtgaggtatcgctgtccagatataccttcagcaggtaattacctgatttcaccgggtaactgttggtacccggcagctgaatactgtaatgggtatagcgctgcagcgacacactggataacttgtaattcagtatcctggtttccgaaaatccccgcatataatcaaactggtttacctgtgcgggtgtccagtcagcattacaaagcacaaatgaataatagtagtttttcacatcattatccaggtcgtcaaacgacagttccagcttctcccctgtaccaattgtatacatgggtaagcttaacggatcgccgctctggttaaacttcacggatttgatgttattgtagtatacatggtccggggtaatagcattcacttgcgccgacgtgctgccgttaaacaaacaggaaacaagggctattgtaaaaattaatgctgctgtacgcatacgaggtaattgatagtattcaagttacgattaaaagcggaaagccgaacgccaaaagccaggtagcaaatgatcccggcgaagatagaatatttatcccgcccaattaccgttggcatccctttttgctttgcactttcagcttttccctatatttgttccatgcgtttatcattttttattgccagacggattgctttcaataagggatcttctttctcaaaattcattatcaatatcgcagtagccgctaccgcgataagcgtagcggtaatgatcctggcaacagcgctggtaaacggttttcagcaggtgatccaggagaaaatcttcagcttctggggacatattcatatcaatgaataccaacccaacgccggtcccctcacggaagaaatccccttccacagccgcaaaagcctgatagatagcattaaaacagcaccgggtattaaaaccatcagcaattacgctaccaaatctgccatcatcaaatccgaaaaggaaatagacggcatcatcttcaaaggaatagatcagggatacgactggccgcaactgaaacgtttcctccaggccggcaaactgctgcagttcaacgacagctcctatgcaccggaaattatgatctccgaatacatggcaaaagaactgcagctgaaagtaaatgataaagccatcatctattttatacagggaggcggattaccgccacgggcccgcaaactaacggtaacgggcatattcaaaaccggtatcgaggaatatgataaaacttatgtgatcggcgaccttaacctggtacgcaagctcaacgactgggaccccgaccaggtaggcggtttcgaggtatccatcaataactaccgcaacatggattccgtggcgcggtatatggataacaacgtattgccggaccaattgtttacccgcaccatccgggatatttacccgaatattttcgactggctccagctgcaaaaccagaatgaactgatcattatcgttattatgaccatcgtagccatcattaacatgatcacggctattctcatcctcatcctggaacgtaccaatatgataggtattgccaaagcactcggtatgcgtaactgggatatccagaaagtatttgtatatcaggcggcctatatcgttatactgggcatactgatcggcgactttttcgggctgggcattgctttcctccagcaggctaccggcatcttcaagctgccggaagaatcctattacatgtcggtagcagcggtatcccttcactgggtagacattctgctcatcaacgtaggcacattccttatctgcacattgatactgcaaatccctgccaggattatccggcgcattacgcccgtaaaggccatccagtttaaataactatttcttccgggtgcttttcacatagtcacgcaggtaactgcactggtcatatgcctgttggtaaaacttcgtttgcccgtaattacccaccagcaaagggaagtaacggttatggaccaacgcagttatatactgatcgccgttgccgttattggcagtatgtttctgtgaacaacgggcagccataaacgcgcactttgccctgaactccttatctgtactggcctgcgccgctttgaggtaataactctctgccgcatagcatccaaaatactgcttttcaaaaggatctttatcacattcgggagcgtaccaccgtgtagacgggcggtagtcttttacaaagttccaggttctgccataataggaaatactgaataacgccgtggcataatcgtagtatacttttgcaggtactggtgctgttttcatcttttcctgcaactgtaccatacgttcgcaaaactgtagttgtgtaatggcttttgtatagggcgcttcagcactgtctaccccgaagtcctgcaactgatcatggaatacctggtaagaaacagccagcgcacctggtcctgctttcttaaaccactcccgcgcattgctgaaatcgtgtaagcgcatatagctcacacctattgcctgatccaggttaataccttcgggcaggaaccctgcgaggtaagattcatacggcgttttaaccggttgatgcaggaaatctttcaggcgcatcagcgttgcggggttcatatcgttgttgatctgatccagcgacgtttgaccggaaacaaaataatcgttcattttcagcgaatcacaacggcccctgatcagcgactccttcacaaagtcgccctgctgatgataacgtggcgccagtatcgcaaacaacaggttacggtaggttttaccaaaggcgaaatttttgttttcctctcttccccagtaattcgagtaatttttattgccggcagttttcgtgtccagccatttaaaagacgccagcagtttcgattcaaaggcactgtcgatcgttttctgttgattgatgtttaccagcaagttcacaatttcccattggtcttttacttcccggtcttttgtttttatagctgccagttgttgggctgctgccgggtaattttttcggatataggaaaggtaggcagatgaaacccgccataagtccacatcttttaatttgccctgttgaaccaggctatccactacggtttgcagctcccttaatttgacaagcagcttactcttttccgcaggggaatagtcctgtatactcacgatgccggtattttgtccgtccatcagcaccgggctgaagtatgcgtcttccagcttattgatttcccttcccagcaatatattcagcgcaggagaagcagggtctgatgcatacacctgccggatggcggttacatcgggcgctggattggtaaagccataaatggctgctaccattgccttttcatggtcatccttgcacagggaatacacttgttcaggcgtggtattggcccacattaagctgacaaaacaggaaagccgcagggagggcgccttctcaaacacgcgggaaaacaaataagcgctctgcacggagtctttcaaacgcagtaaggcgccggatttcaacgccagtgccttgtaatacaccaatgatgagccttcctttccatcgaacagctggtcgaaagaagtaactgcttcccggtattgtttgctgtaatgctgcagccgtaccagctggaagctgtaacggtcgcggatatctttatcttttactttatcccgcaggccttgcccctctgtatataatgtagacagtaacgggttattgcgctccggcactgaccacggatcggcgttgattacggcaggctcgcacgattttgcaaacaacaggtagcgcgctgcttccctgttcttttcctttcccaggaactgggcaaaggtgtttttcttcacactatccggtaatgccgcactgccttctgcaatcgcagccagctgctctttcgggtaagtgtaaatgcattcacgtatatccttatccgttaccttattgccggtatagttttgccagtcggccacattggctgtttcctccgaaggcgttggatcgccaaaaaaattggtgagcgcggtgtaataaaatggctcgtagccggcgccctttgcatacggactaaaaaaagaaatgtagtagtcgtaaggatcaggggttggtccgcaggataaggtatacaccacattgccaaagaaaacggcacaaaagctaattaaaaaaacgacaaattttttgtagttcatccaatggatattttttcagggttgttgaatcaagatgataaaatataataaccggatcgggtgtctgcaactgttttgccaccaactgtgcagccgtttccaatgcctgctggtcaatggtttcacgccggatcacacttccttcttttaagggatatccatttaatgtagtatcctttctgatggtatacagttgtttatcaccggctgcaaagatagtggtatcctgcaattccgccgtaccaatgtttcttaaaataccggtatactccgttccgttccggaataaaacgctccagctgaataaaggcaaagcgatatccaaaggtaagggatacgctgcaacccgttgctcacccaggtaggattccatggcaggtatatcgaggatggaattatgcgatcccggcttacgcaggtcgcccatgttataacacatcagcaaccctctgtctaccggcggtatgccggtacgtactttatacttcacctggtacatccggatggtagcggatacccggcggtgccggaaaaaaggggtttggcggatttgttttataaaagagaagtaggcttcgctggtggtttgggtccagtcgcaatccagctggatctcttttatactggcagcgggtagcgagtcgcacagctgctctatcagccgggatacgttggcggccagctgagggcccgggtttgcccatacttcattcaataggaatactaccggcactatttccacgcctgcggggaaaggggctttctgccggaatatggctaccggtgcgggcgctttggttacttcgtcaacagctacatcaaacagttttatatacagtcgccctgcgggcaggtcgtgcatatatttcagttcggcggtgttgcctgtccatgtttgcttccagtaatagaatgcgggtgttacgttccgtttcgcagcgtggttacaggaaagcaataatatgatgagcagtatccgggggttcatgagcagttaaataagcaggcggccgcagataatacctgcagctactgcggcattcaatgattcggcgccaccgatccgggggatggtgatccggtgtgtagccagggcagttacatcttccgttaatccccttccttcattaccgatcaggataataccttctttgatagcgggaaaggtcgcgatattttttccgtggagggtagccgcaaaagagggcagctttgtttgctgcagtagttcgcggatatcgtattcggctatacgaacccgtatcatactacccatagtggcttgtatggttttaggattatatacgtctacgcaatccggtgagcaaatgatctgcggaattccaaaccagtcggctatacgaataagcgttcccatattgccggggtcctggatcgcttccagcgccagtgccaccgttccggctgcaggcagcgggtttgcggggacaggcatatccagcaaagccattgcccggttgggggtggtgagcgacgacagttgtttgagcacagcagcatccacttcagttacagtgcctgccggcatacgatctaccagggagcgatgctgctccagccaatcggctgttgcatatacccctttcacgggcatgcccgcctgtagcagctcctgcacaatcttatcaccctctgccacatactggctggatttttgcctgttttttttgtgctgtaatgattgaatatatttaatttgcgcctttgacaacatggggccaaacctacacgatttcttttaatcagccaagaagaggcatggttacccgttcgtcagtattggcttttaaaatttttaacaacgttttcgcccgtgatgcagctgcttcccaattcaaaaattttattgctgaaacaattgctgctactggctgtaatacttacgttggcggcctgctccaataccaaatatctccagaaagatcaaacactgtataccagcgccaaagtagatgtgaagggcgaaatcctcaattctgaaaaacaggatctgcgcagctccctctcttccaaatcgctgatgacgcagcaacccaataaaaaactgctcaacagccgtatcaaagtatggctgtataatcagaagtacaacgagaaaaagtcgaactggttctggaacctggtactcgccaaaaggaacctggaagaaccggtaatctatgattctaccaaaaccaaagaatcagtggcgcgcatgaccagctacctccacaaccagggattcttttatgtaacggtaaattatgaggaggaaacttcccggcgtaaaaccaatgttacctaccaggtaaatacaggacgaaacttcgtaattgataaaattacctatgcggtaccggattccgccatcctgcggatcgtaaaagccaatgaaaaattatcactggtgcagaaaggcgttgcttttaaatcggctaccctgggcagcgaaagggaaaggctcacccgtctcatcaaagatgccgggtactacaaatttaaccgcgacgccatagaattcagtgtggatacgctcaacaaggccctgttccggaataccctcaacccttttgaagggtttgtaaacatcttcaatgaaaataaaggcagggataaactgacgatggatgtggaaatccggattaaaaacccggaagacagcaccgctaactggcaacagtatcatatcggcaaaatatacgcctatcctgacttttcattgaatgccaatccaaacgacagtaccctgaaacaggacgagcgcaagtatattaccatccgctcccaccaggaactactgaaaccaaagattctctccaggtctatcttattgcggccaggagaaacctattccatgcagcggtataataataccgtcaataaattatacgatatcggcgtatggcagtttgtaacgctgcaatacaaagaaccgaaagactccgtaaatacactggatgcatatgtgtttcttacccccaggcgcaggcaggaactgggtttgacctttgaattaagtaacagttcggactatacgctgggatcgggcgtaaccctgaactaccggcacattaacctgaataaaacggctacgcaactgggtatggcgctcagtaccggtattgaactggtacgccaggagtcgggatgggagctgcagtcgaaacagtttgggggtgaggtgagtcttacctggccacgttttgcgctgccatttaacatcaaacaaagcagccgctccaatgtaaaaacaagattaacgcttggcgccaactacctctcccgcgtggagaagtttgatgtaaccagcatcaacgcctcctatgggtacgattggaatgaaagcctttacaaacggtggatcatgcggcccattacgctcaactatgtaggcgtgagcctggacccgactttccgcgacagcgtggtaaataccaatccgtatctgaaacgcagctttgagccggcgttaattggcggggaaagcgtttcgtttattttcagcaaccaggacctgctgcatcagcagcactacagctacttccgggtgaacgtggaagaatcaggactctggctcagtggcatcaacagcctcatgaacggcatcagcggcaaaaaaaccaacctggaaacgctgaccaacgtaaatatttcaaattttgtaaagatagaagcagattaccgtcacttctggaaactggggctccacagcgggctggccagcagggtttatgccggcgtaggtattccgtacagttattcacaggtactgccttatatcaggcagtttacttccggtggtcccaacagtatccgcgcgtggcgcttacgcacacttggtcccggctcttttaaagattcctctgctaccgcgcaggcattccccgatcaaaccggcgacatgaagctggagggaaacctcgaataccgcttcgacctgttgaggatgtttggcggtagcgtaaacctgaaaggcgccaccttcctggacatgggtaatatctggatgatccgcaaggactccacccggcccggctcggaattccgcttcaaccagctgtatcatgacctggcgatgggtacgggcgcgggcctgcgactggatttctctttcttcctcgtccgcctggattggggcataccgctaaaggttccttacttcaccggtaataaaaacggctggtatgtgagtgagtgggatctgaaagacagccgctggcgccgtgaaaatattatctggaatattgctattggttatccgttttaggaacggcgttggcagcaatgaaatcttccatgtcagtagcttccgacaagctgaaattaccgatgcgggttctgcaaagactactcaggtaggcgccgcaacctaattgtgcgccatagtcatttgccagggagcgtatatacgtacccgtactgcatactactctgaaatgtacttccggtaaatctatcttagtgatctcaaatgcggcaatggttaatttccgcggttctacttttacatctactcctttcctggccagcaggtaaataggttttccattttgcttgatggcagaatggataggaggcagctgcataatttcaccgatgaacggttgggtggcagccatgatggccgcttcatcaaggtggctgatatctttaaaattctccggctcagactccttatcgaatgtaggtgtggtagcgcctaaagtaaaagtgccggtgtattctttctcctgcgcctggtattcattgattttcttggtcattttccccgtacagcagatcagcagtccggtagctaaaggatccagcgtgccggcgtgacctattttagctttggtgagatttcttatcttacgcactacatcgaaggaggtccatgttaaaggcttattgatcaatatcacggctccttcctggtaatttgttttttcgttcgtttgcatgcccgcaaagatagctattagcagctagctgtcagcatgcggccgctaattataggatttatttaagatcctgaaaagctaaaagctaagggctttttactaaattcacgcaattttaaatacatggcattagaacatcatttagacgcaacgctacggcacaagcaacaggtggacaattcgcgcgactatgtgctgccattcatacagcaggagtttccgcaactggaaggcctgcgtgtaatggaggtgggatgtggggaaggcggtgtgcttactcctttgctggaaaaagggtgtaactgcgtaggcgtggatcttgcaccggaccggatagaactggccaaaacttttttgcagcaatacctggacaatggacaattaaaactgattgccaaaaatatctatgacctggatttcctcggagaattccggaattcttttgatgtaattattttgaaagatgccattgaacacattcctgaccaggaaaaaatcatcggtcatctgaaacagttgctgagtccccgcgggcaggtgtattttggttttccgccgtggtatatgcctcatggaggacatcagcagatctgcaagaacaaattcctcagcatggtaccttatattcatttgcttcccaggccgctctacaaaggtgtattgcggctatttggcgaaggagatgatgtagtgatcgacctgatggatgtaaaatccaccggcatttccattgaacgttttgaacgtattgtaaagcgccagcaatataaaattacgcaacgccggttttacctgatcaatcctatctataaatataaattcggcgtaagcgcgcgggtgcagtggaagcccattgctgcgattcctttcttccggaacttcgttaccacgtgcgtgtactacatgataaagccagcgtaggttgtcttactcaggattaccctgattttactgattaactggatttttacttttttgattttataaaggattaagggagatagaagcggatattcgctctcatctcccttagttattattaaatctaaaaatctaaagaaaatccaaaagaaaaaatcagtaaaatcagcgtaatcctgagtaagacaacctacgcgttccagatttcccacgaggcttctgcctggaggatcagcatttcgtggccgtttttgatggtggcgccctgtgcggcgccccgttgcaggaaggaggtttctgccgggttatacaccaggtcgtacagcaggtgcctggaagtgaggtactggtaagggatttcggggtaggtatctgttttcggatacatgcccaggggtgttgtattcacaattatggtgtgttgttccattacctgttggttcagtgactcgtaagatacggctccgttcaccggttgccggcttactacggtataggtaatgcccagctgttccagcgcatacataatagctttggcggcgccgccggtgcccagtaccagtgcgtgcttatgatgggcctgcagcaggggttgcagcgatttggtaaacccgattacatccgtgttgtagcccgttttttttccgtccctgaagtcgatacagtttacagcgccgattttcgcggcggcatcgctgagattatccaggaaggggattaccacttccttataggggatggtaacgttgaggccatgcagttgcggatgctgctccagcagggaggtaaattcagagatgcctggaatcgggaagttatcatatacacatcctgatatattttccttttcaaatttttctttaaagaaacctttggagaaggagtgactgagcggatagccaataagtccgtaaattttcatgtaccaggtaattgatcattaccaattatgaattacaaatcagggatttgtgttgatgttatccacaaatccgtcattcgtaattcataatctgtaattatttaaaaaactattctctgtcgaggaacaggttaaaggtatctcctctgaggccgatgcgcatggcttccagggagatcacttcattaggagccaggttgcccaggttggcattgcagcctaccagttccaggaagtaaagctgttgggctttttgtggcgcttcccagataattttttcggcggggatctgtgtcaggatttcctgtaccaggccttcgcgtacttcgccgctaccgcggtagatgcctacgttaccgctttcgcgggcttcagcaatcacataagtggcgccggcggagagctcagcgctcatcagttcaatccacttatagggagggataatgtgttcagcatctttggagcctacttcgctcagtaccagccctatttttgccagtttttcaatataaccgcatttttcagcatgcgggatagtgatagagccgtcggaaacttccatgtagctgataccgtaatcttttaccacgttgatgtattcttcaaactggttacggattacaaaggcttcgaacagggttccgccaaagtatacgggaatgtttgccgactggtaaagttcaatttttgcgcgcaggttgggcgtaacgtaagcagtgccaaaacccagtttcaggatatcaatgtgaggacctgctgcggataaaaaatttcgtgcttcttccaaactcagccctttgtccattaccatagtgagtccatgtgtgcggggcttctttgtcctttccgggatttgtgtcagattaaaattcatttgaaatatttttatcttcttattggtcagtaaaacacatgctaattttcgccaggcacttcgggatagcgtagatgcaattttagtaaccggaaatactattgacttttgtccatgacaattaaaagccggcgcaaaaataagaagtatactttattttattaaagtaaataacactggttaacgtttgcggcgatattgggcgatcagatctaccacactcacatgctgtaacacagcagggtcgagctctacgagctttttaacaatctttggagcctgttgcagggctgtttccaggtgcagtaacccttcttttgttttacccatggctatcaggatagcggcccggtaatagataaagataggtttacggcccgccttttcctctgctatggctaattgtacaagggcttcatcaaggaatccggatacatacagtccctttaacagttcctgccaggtaacggcgcttttgggcctggtacgtacggcattcataaaatgtaccagtgcatccttgttctttccgagctccaggtagcattcacccaggctcatattgtactctgcgttggttttatttattttcagtgcgctcattaacgatttaacggcattttcccagttggcttccatcatataggccaccgcaatcttgtagtacagcttatcatcgctgggactcagatgcgaagctttacggtagtaataacgtgcctgggtaaacttccgttgtctttcgtaacaatgaccgatagcttcatagatgacatcctccggcttggcgatttccaggtgtttctggagcacttctatggcttcggcatacttgcgcatccggatataggcatcgcccatattacggtaggcataatcgaatttctcatctatggccaccgcatattggtatgcgtctatcgctttttcgtataatttaagtccctggaatgctgtgcccaggttaaaccaggccagctggttatagggatgctcgtcgataatggcgctatgcaggcggatgctctcttcattgcgaccggtaaattctgtccagaaacagattttatgtaatgcttcctcactggtaggatcatattccagcgccagtttcaggcaatcaaacactttctcaaactcctcccagtcgtcgtatacgtcggccagttccagcaataattctgtcctgtcttcccctgaaaactgttcaatctgttcttccagcacagcagctgccttctgatgctggttcagcgccaggtaaacgtctgtttgcagtatataaagattgatatcagtacggtccagcacttctgctttctcgagcaagtccaatgcttccttatattttttggtttctatcagtaagttggcctttttgagaagtaaagtggaggaataggggaattgttcgatggctatttctgcggcctgcaatgcgatcggcatttcgtcatgctcgtcataatagtctatgatctgctcaaatgaatcttcgtccaaaaaagaatgagacttaccagccctgaggttttcaaactgctgcaacaagtctctcagatcatcaaaatcctcgtttaaaaatgaaaagtctttactcattactgtaaatatagtacttttatctatgcccaaatatggggtgaaatcaatgtgctaaaaaatttttaacaattctttgtgatttcttcgtatcttgcgttaagaatatgttatataatatatcaaaaagtttgtacatttgtgttacaatgaaagcgaaaacatacatatcacgcaccttttcattgtcttgcttgttagcgggcgcattagcgttttttgctctcaatgcggcggcaaataatggctttttgcccaccgataataataaagacaaagtgaaaaagacagctgacagccaacattttgtgctgaatacagctatgcctaaaaccaatctgagccttgatgctggctaccgcttttcgggtaccttcaactcagactttaagtttactactaccaataactataataatgtcattaacctgaaagcggtaatgacctatacgaaaggtaatgtcacttatgtagttccaaccaatgtccaggtgcagtcacaacctcctggaaacatgaactttcagaaactgcagattattctgccgcttaagaaagggtaataaacttaacgtttcttcaattacaatatgggccggttaaaaagttctacagctttttaaccggctctttttttgcgccggagcggaggttgtcttactcaggattacgctgattttattgatttaggggatttgaacatttttgattttaaaagattcggggagatataagcgaaaatatccgcttattctccccgaatcttttaaaatcaaaaagtgatcaaatcagcgtaatcagtgtaataagtttaatcctgagaaagacaacctccgcgttcccgcttatatctccccgaatcttttaaaatcaaaagtgatcaaatcagcgtaatcagtgtaataagtttaatcctgagaaagacaacctccgcgttcccgcttatatctcccagaatcttttaaaatcaaaaatgttcaaatcccctaaatcaataaaatcagcgtaatcctgagtaagacaaaatccgctcctctacatattctgcagctccttttggctcacttccttgtagcctgttttgggcacatcaaaataggaggcggggatcgggtataattctatctttgtggccactaccctggttttggagccggttttggtgataatctcgaactccagcggaatacctttcaggttcacaaaacgacggttgtattgtttattttccggcaccaggtcgagggcataatacacctcaaaggttttgccatcgggcatggtaccaatggctttacggcaatcgtagcctgctattttcttggtttcagactggtcctggaactggatgctttcgtattgtttcaggtccttctggtattgctctttccctgcgcgtatcaggtatttgttcccatgctggtctatcagtgtggtcattgtttctgttttactgttgatcaggtaggtgtagtgaacaatattgaaattcatatcaatcctgctcagtggtccgcgcatatattgggtaaaggtgctgccttcgagcatggcatccatttggagctgctcaggtggcagttccattttgtaaacgattttggcatcagaaataacacgctgcgccagcaatgagccggtgcagcacaggaagataaaagttaataacaaccggtatgacatagtgtggtgtattaataataaaatggcctcagtgaaccgttaccagttaagcttctctttgtttaaaaacgcagctattccgcgtttacaatcatcatgaccgcgggtggccgcattgagtatggctgcgtgcgccaacccatccgctaccggtaagtccaacactgtgccaatcaattttttggtcactttcagggagttggcagaagcttcattacataggctggcagccactttagctaccttttgggcgatttctgaagcaggaaccactgcggtgatcagcccatcggcggccgctttttccgctgttaccagtttgccggttaataacagctcccgggagcggccctctcctattttgcgaaccaggaaaacagctaccagggcgggaataaacccgatttttacctcggtatatcccatcagcgcttccggtaccgcgtaactgaggtcgcagagggttacaagcccgcaaccaccggccaccgcatgtccctctacctggccaattactatcttatcaagatcatagatctcccggaataactgcatcagttcccgggaatcagcgagattttcatcataggtattttgctgcagttgttgcaggtattcgagatcggcgcctgcgcaaaaagcttcgccgttacccttcaacaccactactttcacggcttcatcggcttccgccgcacggaatgcagcccggagttcagctaccatgggcccgttgagcgcattacgcttctcaggccggttcagcgcgatggtggccacccgctccaccactgtatactggataaaagaaaatgccataaacaaagaattacaaggccttgtttatggcaatctaagcaaaaaaaatttaatgggtaatctcctgtattacctgacctacattgccgctgggcatctggatatgcaacaaagcagccagggtaggcgtaatatccgtcataccaacagtacggttggttttacccgggcgaacaccccagcccatccacaccagcgggatatgcgcatcataaggataccataacccgtgcgtggtgcccacattggtaccatcgatataaccaggcgttaataccacctgtatatcaccgctccttttggtgttaaagccattggacagcatcgtgcgcatgggttccggcaaggtggtgcccatgagattatctatagaaaaggctttggcgaccgcgggtgatttaagcaactcccggatcataaactggcggatgtcggcttcacttttacctgcctgctcaatagcgtcgtggttcagccagagctggtagttatcggtggctttcaccgcatttttcaccccaaatttggctgatacctggtcgttcagggtagctactgctgctttgtcgtcccatgtgccgcccggcagtttgttttccgccataaaaccaggtacatgggcaacgccatgatcggctgtgataaagaacaggtactgccccttgcccactttcgcatcgagataggtgaagaacgcggccagatcctggtccaggcgcaggtaggtatcttcagcttccactgagttggggccgaactgatggcctacataatcaggagaagaaagactgacagccagcaaatccgttaccgggccttttcccaggccatatgcttccattgcttttttggcaaattccagggtcatggtattaccgtaaggcgatgcggaaatagcagtattggcgatctccgagaggttgtgcgggaaggaggtgttaccggcatttttatactttccttcgtaaggtttctcatcggctgtactaagggtataggtagatgctggatacagggtagtccacggtttgctgagatattgctgcgggaatttctgctggttgaattcctgcgtccatgcaggcaattcattcatgtaataggtgctgctcacccagttaccggtgctggcatcataccagaaagctgcgttggcactgtgcccggcaggaagaatagcacccctgtctttaatagcaacacctatcaccttactctggaaattattggataacttcaattcgtcgccgatagtggttaccagcatattccgggggctcattttaccggcggcggaggagctgccgacggtggttaccgtggtatcttccgcacaatacatcgtacgacccagttccgggctgtaccaggtgttgccgataataccgtggatagccggcacagatcctgtatagatacaggtatgaccacaggccgtgatggtgggggtgtaattgatcagcgtattttcacaggagaagccttcctgcagcaggcgcttaaaaccaccggcgccatacctgccggcgtagcggtacaggtaatcccaccgcatctggtctaccaccaggcctacaacgagtttggggcgggcagcgatactggtgtttttagccgcaggaagacgatgaagcggctttgaaggagcgttttgcgctttgccggccgtggcagataacaggaatgcgactgccaggaattgtgtaaatttcattagattgtaataatttaaaagtcactgtaatacaacaagatagatggttatctggcatcaacaacggcataaaatagctggtgccaaatgtaaaccaagtttacaaaaagtaatattttaatacctttgtgtccattttaaatggaatgaattaaccattacataatatatcgtatggatattttcgagaaactgctgaaacatctgggccctatcggggaacattcagacagagcccacggctattttgcctttcctaaactggaaggagaaataggcccccgtatgaacttccggggtaatgaaaagattgtctggagcctgaacaactatctgggtttggccaaccacccggaggtgcgcgctaccgacgccaaagctgccgcagactatggaatggcctctccaatgggagcgcgtatgatgagcggaaataccaactaccatgagcagctggagaatgagctgtctgactacatgggcaaagaagcaactaccttactgaactacggttaccagggcatcatgagcgccattgatgcagtagtaggccgcagggatgtaattgtatatgacgcagagtgccacgccagtatcctggatggtttacgcctgcaccccggcaaacgttatgtgttcaagcataacgatatggaagatttcgacaagcagatgaaacgtgctacggaactggctaaaacccagggtggtggtatactcgtggttacagaaggcgtgtttggcatggccggcgaccagggtaaactgaaggaaattgctgcatttaaagataaatatgagttccgcctgctggttgatgatgcccatggctttggaacaatgggtaaaaccggcgccggtaccggtgaagaacaaggcgttcaggataagatcgacctgctgttcaatacctttgcaaagtccggtgcttctatcggcgctttcatcagcggcgaaaaacagatcatcaattacctgcgctataacatgcgctcccagatcttcgcgaaatccattcctttaccgatcgttatcggccacctgaaacgtgtgcagttgatgcgtcagcatccggaaatgaaggctaaactgtgggagaatgtgaataaactgcagagtggtctgaaagaacgtggattcaatattggcagaaccaattccccggtaacacctatctacctgcagggcgatatccccgaggcgactgctatgtgcctggatctgcgcgagaattataacatcttctgttctatcgtggtataccctgttattccaaaaggacagatcatttaccgcctgatcccaactgctgcgcacagcgatgaagatattgaacttaccctcaaggcattcagcgaaaccaaagcaaaactggacgagaaagtgtacgaggtggcagagatcccaatggtataactgacacacgctatcatattaaaagccttcctgctttccaggaaggcttttctatttaaaatgggaaaaggccagaggggttatggcaaaagaaggtacggcaaaataaccgggaaaaacaaaaagggctgattttagtcagccctttacttcaaatcgttctttcactaggtgtaatttttcattagatttcatcaggacatggtagagaacaactggttttcatagaaattggaataaccaagtgattccaagtattttataagcgttcttttattttaattcggtctttttattcattgatgcttatcaaaaatagctcagatttcaccaaaaaatataacacatacgttggattttgttaatggcttgttaaagatttcaactgcaacaataaatcaccaggatgttaatgcagccatttttttcccatccgatcaataattttcccctttgcgtaaacggtttcccgcatcccgcggtaacttcgcggcggaagcaatacatactcaaccttttaaccattatggcggtgacgaggtgaggcggcaaaagtgtctatagcactttcgttaacgccgggtataattttttaagtcaaactgataaaagacaggtgttcaacattcaatggagcaagcaatttttccgcctgcacagaattaccgggctgatagccggcgctatgctgctattggtgagcattaccggcagcatgctggtattcagcgatgaaatagatcatgcggtgtatgcccatgcctatcacgttccgccgcaggcagttcccagaacattgcaggaacaaatgaaagacgcccgccaggcgcttcccggaaatccctacctgttttttgtaagactcccgcagtcgcccggcgaaagtaccgtgctgcgggccgaatattcagcagatcacaaagtatacatcttcctgaacccctataccggcaaaatattacaacaatacgccaatacagaccattttacaggctacgtcatgtatctgcacttcaccctgctaagtggcaaaacaggggctgtaatcgtcttaattacaggaataggactgtttttatctgttctcaccggcctgtttgtataccggcattcactgggcaaagtactcaccttccggcagccgctggaatggcataaccgcacccggcgctggcgtaacctgcaccgcatcgtcggcgtgtgggcgctgcttttcaacctcctcatctcttttaccggcttcatgatggaactgaaagtaattgacgcgcggaaaaacaccaaggcaggatatacggctgttccttttcccggtgaatatgaacccctgctcatcaaagctgcggctactatccccggcttccaggccaccggtctccgccctcctaaaaaagcaggcgacccggtacggatactcggtcatgcccatgaatccgcattcttcggagaatacgcttcgtcggtatccatcgatgaacaaggcgccgttaaaaaaaaggtggacttccgcaacgcctctttcagcgataagttcaatgcctctatcgctcccctccacttcggcaactacggtggcatcttcctgaaaatcatttattcactgcttgccctaacccccggcgtgttatccgtatcaggattcctgatctggtaccgcagaaaatttattatcaaaatacacggaaacagaaaatgaagaaggctttagtagcagcattaatagtcattgcagccaccatgcaggcagcagcacagcaaatacagggtactcccgcgcccacaactgacagtatcattcaaccatctgatgtaggtctgaatgaaatagtggtaaccgccagccgtaataaagaaacactgggcaccgtgccatcttccattaccatcatctccggaaaacgattaagggaacaaagcgcgatcaccactgatattaaccagctgctcagcatgaatgtacccggacttacactgggcaccaatacttccaccaacaaaggacaaaccctgcgcggccgcggcatgctcatcatgatcgatggcatcccgcaatccaccccgctgcgcaacggcgataaagatatgcgcagtatagacgtgtccgttattgaaagagtggaggtgatcaaaggctccactgctatttatggcaatggcgccgacggcggtatcattaacttcattaccatcaaagccaacccggacaaacgtttcagcggaagcaccgatatcagcaccgccggttcccttacaaatggcgccaacagcctcggtggccgcatctcccagaacttctccggcaaactcaataaatttgattacgtggtaagcggtacctatgaacaaacaggtgtgaacaaagatgcaaacggtgaagtaatcgcccctttccagtcgctcagccagaatgaaaacgtaaacctgtttgcaaaactgggatacgatatcaatgccaataaccgcatcgaagtgatgtacaactattaccgcaccatgcaaaacagcacctacgtggatgaaggcggcgaatttggcaaaagcccgatcattggcgtagtgggcaccaatcccggtgataaacaaggcaccccctataatcacaatgcttacgtgaattataccaataaaaatattttccgcaacacctcactgaatgtaaacctttactatcaagacttctacacggtatttgaatggtccgatttttatgcgcctccgggcaattctgccattgcttccaaaaaaatgggcgcgcggctgaacttcaacaccgttttcaatttccatcccaatttatccggagatgttacctggggtgtggatatccttaatgataaaacatcccagccactcaccgacggccgtccgtttgtgccggagatgaatatgaaaaactatgcgccctatgcacaactgaaaacggtagtcttcaaagatttcctggtgaaggcaggcgtacggtatgaaaatatttccctggacatcccagattatacaactatcaaatttggtaactatgccggcggcgtatttgtaaaaggcggcgaacttccttacgaagcgctggtattcaacgcaggcttacggtatacgaagttcccggtgttcaatccttttgtgagttattcacagagcttctcgctgtacgacctgggccgcacgctgcgactggcaaaagcagtcagcaatggcgccaccagtatcaataccattgaaactgaagccattatcaccaacaactatgaagctggctttaacagtaacatcgggaagttcaatgcatccggttcgtattttatcagcacctccgatcttggtaccagcctgaaagatgtaaacggtgtagcagtgccggagcgcgctcctgaacgggtacagggctttgaatttacagccggctaccagttcctgcctaacctgtatgccagcggtgcctattctcatgtagaaggaaagaaagaggtgaacggcactaaaacctatttgcctaccacccgcatttcacccgataaaatgacattcaacgtgaactattccccgctgaagcagtgggatcttggggtgtactacatttattccggcgtgcgcaaacgctttgacgtaaacgccacaaccggtcagtacgacctgggcagtggtcccgtgggggatttctacctggtgaacttatataccggctaccgtttcagccaggctgcatccatccgcctgggtgtggataacctgttgaatgccgattactaccctgttacctcacaaggaagggtgcgtaccgattcctatatcaaaggaagtggcgctagatttaacctgggattcaaatacagcttctgataattcaccgaaataaaaagggttcgcataaaagctatgcgaacccttttttatgttgttgaaaagcggacgattatttcttcagatgctcttcaatggcggtatcatatgtttttttccaggtacttacattgccccagtcatccccatttactttaatggattcaccggttacaacacctagtttctcgtagcgtacagagttatctgacgcatctaccaaaccgtgtaacagcgcttcgaacttctctttatctgccggcttaacggttaccactacacggctctggctttcaccgaagaggtaagcatctttacggaatttgttgttgagcgccagttcaaagcccaggccggatggcatagcgctttcgagcagggtaacaaataaaccgccgtcgcttacatcgtgtgcagactggatcagttttgctttgttcagtttggtgattgcctgttgcaggtgcagttcttcatcgagattgaaatgcggtgcagggctgtattctataccaatgatcttgtgcaggtattcagagctgttgatatcgttgcggctgcggcctaccaggtataccaggtcgccttcttccttgaagttaagggtgatacgctgatcgagcgtgtcgaggatacccaccataccgatggttggtgtaggataaaccggaccgtcgggtgactggttatagaagctcacgttaccaccggtaacgggtgtattgaatttacggcaggcttcacccataccttgtacggcgtgtacaaactggtagtacacttccggatcgtaggggttaccgaagttgaggcagttggtgatagcaactggttcgccaccggagcaaacgatgttacgtgcagcttctgccaccgctatctgtccgcctttatgaggatcggcaaatacgtaacggccgttacagtcggtagtcattgccaatgctttcttcgttggttttaccaatacgatagcagcatcgcttggtgcgttggtggtggcgtttgcagtacccaccatgctgtcgtactggttatagatccagcgtttggaagcgatgtttggtaatgcaaccattctttctgctacaaaacgcggatgttctgtatcagggatattctgaatatcgaatgcttttactttagcgaagtaggctggttctgtgtaagcgcggtgatattggggagcgccgccacccagtaccatactttctgcaggaacatctgcttccagttcgccgttcatatagaacttcaggtttttatctttggtaacttcaccgatctgaacgcagtgcaggtcccatttttcgaagatgtccagcactggtttttcttctcctttcttcactactatcagcatgcgctcctggctttcgctcagcagcatttcccatgctttcatatctttctggcgggtaggtactttatctaaccagatgttcataccatgttcgcctttcgcgctcatttctgcagtggagcaggtgataccggcagcgcccatatcctgcataccaatgatagcattggttttgatgatttccaggcaggcttccagcagtttcttttcctggaaaggatctccaacctgaacggcaggcaaatcttccacgctgtcttccgtgatattggcagaagcaaaggaagctcctccgataccgtctttaccggtagcagagccaacaatgaaaacaggatttccttcaccgtatgaagtagcggaaacagtttgacctacttttacgatacctgcgctgaatgcgtttacgagcgggttggtaccgtagcattcttcaaaataagtttcgccgcctacggtaggaacgccgaagcagttaccgtagtggcctataccatgtacaataccttttaccaggtgttgtgttttcttatcattaatattaccaaagcgaagggagttcagtgcggcaatgggacgtgcacccattgtaaagatatcgcggtgaatgccaccaacgccggtagcggcgccctggaagggttcgatagcggaggggtggttatgcgattctattttaaataccaccgcgtagccatcacctatatctaccagaccggcattttcttctcctgctttaaccaggagcctgtcgccttcgcggggcagagacttcagccaaacgattgagtttttgtaagagcagtgctcactccacattactgagtacatacttaactcggtaaaattgggggtacggcctaaaatagatttaattcgttcaaactcgtcagcggtaagtcctagctgttcagcaatttctacggtggtttgcatgtatttaagtataaaaaacgagatatttaaaagaagtcgcaaaagtacatgattttcctgcaaatgccaagagtaccctgtggtggcttttctgcagtttttttgcaggcaggtatcatattatttatttttaaattcatcagatttaaagtctatctgctccaaatatttaatgaaatgataaaaaaataccccttttaaagccctaaatgtaatttttcagttaaaatgaacaatttatttgcatttatagcgatggatgcgttcttttgtgtaaaataatttacagcatgcaatcgttacgtttcaaagcgctggaaggattagctggcgtagactccactctcaccgaacatgacggtaaaattaccgatgtatttggcagcaatgttttctctggtaaagttgttcgggaatatctgagcgatgaggcttataaaagcctgatgaactctgttaaaaatggcaccaagctggaacgtaaaatgtccgagcagatcgcttcaggcatgaaagcatgggcgatgaaaaaaggtgtgactcattacacacactggtttcagccattgaccggcactaccgcagaaaaacatgattcatttttcactttgaaaggtgatggcactgcactggaaacctttgatggtgatgcactggtacaacaggaaccagatgcttccagtttccctaacggtggtttgagagctaccttcgaagcccgcggctacactgcctgggatccttcctctcctgcatttatccttgagcagggttatggtaaaacactctgcatacctacgatctttgttgcctacaccggcgaatccctggactacaaagcaccactgctgaaagcactggctgcaatggacaaagctgcagtagacgtatgtaactatttcgataaaaacgttaccaaagtaaccggtaccctgggttgggaacaggaatacttcctggtagacgaaacaatggcgaacgcccgtcctgatctgatcatgactggccgcactgttgttggtcatgctccttccaaaggtcagcagctggaagatcactacttcggtgctattcctgagcgtgcttacgcttacatgcgcgatttcgaagtagaatcctacaaactgggtattcctttgagaacgcgtcataatgaagttgctccttcacagttcgagtgcgctcctatatttgaagaagtaaacatcgcagtggatcacaactccctgctgatggatgtaatgaataaagtggcaaaacgtcacaaactgaaagtgttactgcacgagaaaccttttgcaggcatcaacggttccggtaaacacaacaactggagcatgtccaccgataccggtgtaaacctgctggctcccggtaaaactccgaagaccaacctgatgttcctcactttctttgtgaacactattaaagcggtgcatgactacgctgacctgatgagagctgctattgcttctccaagcaacgacttccgtctgggcgctaacgaagcacctcctgccatcatctccgtatttaccggtaaatacctgtttgatgtactgcaggaagttaaaaaccgtgtaaacaacaagttcgacgaacaggacgaagctatcctgaaactggatctgcaccgtcatattcctgaactgttgctggataacactgaccgtaaccgtacttctccttttgctttcaccggcaacaagtttgaattccgcgcggtaggttcttctgccaactgtgcttctgcaatgaccgttctgaatactatcatggctaaaaccctggttgactttaaagcggaagtagattcactgatcgaaaaaggtgagaaaaaagagattgcgatcatgcaaactcttcgtaaatatattgtagattcggaaaagatactgttcgaaggcgacggatacagcgaagaatgggagaaagaagctgaaagaagaggtttaccaaacgtaaaaaccactcctaaagctttggatgcaatgatcactcctaaagcaaccaaactttatgctgacaccggcgtttacaacgaaaaagaactgcacgcacgccatgaaattctgctggaagattatgtgaagaaagtgcagatcgaagcccgtgtaatcggcgatctcgctaccaacaccatcctcccgtctgctatcagctacctgaacgacctggtagtcaatatcaacggtctgaaaggaattggcctgggcgacgaatcagtaaaagctcaaaaacaaattgctgctaaaatagctgaacatattaatgttattagtgaaaatgtacaggctatgatcgaggcgcgtaaggtaactaataagcttaccgacagccgtcagaaagcgattgactactgtgaaaagattaagccgtactttgatgttatccgctaccactccgacaaactggagttcctggtggacgacaaaaaatgggcgctgcctaaatacagagagctgcttttcttgcgataaaaccgtaagattgttttggtgtatgattagccccggattttcatccggggctttgttttgagatccacctgagcaagtattggtttaacctcagattatccctatcttcatattatacctatataccaataccccatataacgtttagattttcctgtaccgtacgcaccacgtttatttaatcagaattatttaaaaacaagttacccaaaatgaaaagacaacttttacaaacgctttgcgtcatggctattgccatccctttactgctccaaagctgcctcaaaccaccggtaatcattcctggccccaaccactacaggatcgtgcaactgaaaggtattcacgggtacgatgacctgctggattctgtccggatctcttacaacaataaaggaaacccggttagcctgattgccacacaggtgacaaccggttatccgcagttcctgataggatatgataacaaacacacgctcaaatgtattatcggcgcctattcagatgacctccccttttttgaaatagcccacaaatacatcaccgataacaaaggcagagtgaccaccgacagcacatttactattgggatctatgatcgtagtaccatgacagtcacctccgggtataataccgcagtggagtatttcagctatgacaataaggacaggattgtaaaatccgtcaggaaacaatttccggaagaatattacggcataaccaccgtttactatcattacaatgccgccggcaatgcatataagatttccacggttaacttctggcagggacaaacctctcctcccattgatgtgtaccccatttacgatgataaattaaacccgcatcagcttcataaaatatggatgttcaacgacagggactacagtgttaacaatccctttgtggcagatcagtacaataactacggcctgccggttagcatcactgcaaaagaaacacatcaggagttccaattcctgaatttcaacttcaaaaaactgttgattaaatataattaacaacaaacgaaaaagtccccctggtcaaaccaggaggacttttccaaatagtatatccgttaccgttataccagcttaaacgtttctgtaaacttcgtggtaaagttacctttacggaagttttcatcgcgcatcagctgctggtggaaaggaatcgttgtttttaccccttcaattacaaactcactcagggctcgttccattgtgttgatcgcttcttcacgggtttgcgccatcgtgataattttcgctaccatggaatcatagtaaggcggaattacataaccggcatagatgtgtgaatccactctcacaccatgaccaccggggatatgcagggtagtaattttaccgggagatgggcggaaatcgttgtaaggatcttccgcattgatacggcactcgatggcatgcatctgtggcgtataattttttccggagataggaatccccgcagcaattttgatctgctcttttaccaggtcgaagttgatcacttcttctgtaaccccgtgttctacctggatacgtgtgttcatttccatgaagtagaagttgcggtgcttgtctaccaggaattcaatggtacccacgctttcgtaattgatagcgctggccgccctgatagcagcatcccccattttctcacgcagctcaggcgtcataaacggagaaggtgattcttctaccagcttctggtgacgacgctggatagagcaatccctttcactgaggtgacatactttaccgtattgatcacccgcaacctggatttcaatatggcggggttcttccacgaatttctccatgtagataccgtcattactgaaggaggcacgtgcttcatttttagccatgttgtaggctgtttccagctcactttcttcccataccacacgcatacctttaccaccgccaccggcggtagctttgatgattacgggaagtcccatgtttttagcgatgactttcgcctcttccacgctctggagcaaaccttcagaacctggaataaccggtacgccggccgcaatcatggtttctttggcagtcatcttatcccccattttccggatcatttccggcgtggggccaataaatttgataccatgttcaccacagatttcagcgaaacgggcattttctgccaggaagccgtatccagggtggatcgcatctgcattggtgatttctgcagccgccatcaggtgagggatgttcagataagactctgagctttgtggcttgccgatgcatactgcttcatcggcaaatttcacatgcagactgtctttatccgctgttgaataaaccgccaccgttttaatacccatttccttacaggtacggataatccgaagggcaatttcaccacggttggcaatcaatatttttttgaacattgttttccttataagtttaataatagctgttagcatttagctgttagcctttagccatcagcgcactgccatttggcaagtctgaaagctaaaggctaacgggtaaaggctattattatggttcaactaaaaataaaggttgatcgtattctaccggagaagcgtcatctaccagtactttcacaattttcccacttacttcactctctatttcgttgaataacttcattgcttcgatgatgcacaccactttaccggaagttacttcgtcaccaacatttacgaatggtgctttatccggaccggcgctgcggtagaaggtaccaatcatgggagatttgatggttaccaggttatctgctttggcaggggcagcaggtgcagcggctgatgctgcggtggccggagctgctgcaggagttacagcggctactgcctgaacgggtgccatggttgcaggaacagtgattacctgctgaacttcattatccttctgctttattgtaatcttaaacttgtcctgttcaatgctcagttcactgatatttgatttgttgatcatttttaccagttcctgaatctgtttaaagtccatgtagacagtttttggtttagaaatatatagaatatgacaaatactttttcacgcattcagcaactttgtttcagaacatatctttctgaaacaaagttgcttttctctgaaaaccagtatttcagaaatgatttatttatgcttttactctttcgatgtactcaccatttttggtgtttacacggatcagttctccttcgtctacaaacagtggaaccatcacagtggcaccggtttcaacggtagctggtttcagggtacgggtagccgtatcacctttcacaccgggttcagaataagtaaccagtactacaattttatcaggcagttcaacagccatgtactgttcagtttctgtattgatctgtacacttacttcctgtccttctttcagaaactgaggtgcatcgattgctgtttccggcatagcgatctgctcaaatgtttcattgtccatgaaattgtagccggtatcatctttatataaatactgaaaaggtttcttctcaatacggattggaaagatagtatcacctgagttccaggtgtgctcaatggaacggctattatcaacgcctttcaatttagcccaaacctttgcggctgcacgggcggttttgttctgaccaaactctacaacagaatacaagctgttatccagcttgataattaatcctgttctgatatctgcggtggtagccataaataggttactgattttaagttaaaaatttatacggattgcaaaagtaaaaattttcgcatatgaacaagcaactaattcccaaaattagagagattagtcccttttcggctcaattttcggcttttttattcaaataatgacatttatccggtaattttaaactcaaatcaagaaacttttataagtatgcgctacgtgtttttcgttattttaagctgtttacctgtgtttttgatggcccaaacgcctgctaattccagcaccaaagcaccttatttacaatacccgatcatccccgcttttccgttgagccttgttgatggccacactatcaccaaaaacgacctgaagaaaaatgagaagaccatgctctttgtattcagtgttgactgtgaccactgcaaacacctcaccgaggaaatgctgaaaaatattgacaagttcaaaaaaacacagatcgtgatggtcactcccttcaaagtggaacaaatgaaggaatattacgatcattataagatccagaactatcccaacatcattatggcgagtgaaccttcccggcagatcatgtacttctatgacctccattatttccctggtttgtatatatataataagaaacaacagtttgtaaaaggttttgagggaacagtaaagctcgattccctgctgctttatctcaacaaataatgctttgtgaaaatgtagccgccagcggattattgtaaggccgaatccttacatttgttcaatcacattcattcttcacttttaaagctaaagacaaaatgaaagttacagtagtaggagccgggaatgtaggcgcaacgtgtgccaatgtactggcccacaaagattttctgcaggaggtggttttattggatattaaagaaggaacggctgaaggtaaggcgctggacacatggcagcaggctcccattgattattacagcaccaaaattacaggggtaaccaacgattacaccaaaaccgcgaacagcgatgtagtggtaattacttccggacttccccgtaaacccggtatgagcagggacgacctgatttctaccaatgccaatattgtgaaatcggttaccgaaaatattacaaaacattccccggatgctatcattatcattgtaagcaacccgctggatgtaatgacctattgcagctatctcactgcaaagaaaaacagcagcaaggtatttggtatggcaggcatcctggataccgcccgttaccgcgctttcctggctgatgaaataggttgctcacccaaagacatccaggcgatcctgatgggtggtcatggcgatacaatggttcctttgccccgttataccaccgttggcggtatcccggtaactgaactggtagccaccgaaaaactggatgctattatccagcgcacaaaagtaggcggtggtgaaattgtaaacctgctcggtacttctgcatggtacgcacccggcgccgccgctgcacaaatggtggaagccattgtaaaagatgaaaaacgcattttccccgtttgcgcatggcttaccggcgaatacggactgaaagatatttacctgggtgtacccgtagtattgggtaagaacggcatcgaaaagatcatcgaactacagctcaatcctgccgaaaaagaattattgaatacctctgcacaacacgttaaagaagtaatggacgtactggacaaaatgcaatccgctacagcgtaatgcggattttgtctttcccaggattacgctgattttacagattatacagatttgatcctgtttgattttttaaagattaagggagataacagcggatatactcactgttatctcccttaatctttaaaaaatcaacacgtaatcaatcaaaacaatcagtttaatcagtgtaatcctgagaaagacaatttaaaatcgccgaaggcgatcctgactataaatccacatttattcgtaattttaccccgatcctgtattggctaaagccgtctaaatgaagcagttctaattagtttcataaaatttggtttaactctgaatgtatgtctaacctggaaaaactgattacgcagaaaacatttgaaaacgaaaatcagcgcggcctgataagcctgattttcatcgggaactggataacgtcccgtcaccagcaattttttaaacgttatggaatcaccatgcagcagttcaatatactgcggatccttcgcggtcagcatccacaggctgccagcatcaacatcttaaaggaaagaatgctcgataaaatgagcgacgtatcgcgcctggtggaaaggctccgcaaagcagacctggtagaacgtaagaacagtgaaatggacaggcgcgcagtagacgtacgtatcaacgataagggcctgcaactgctgaaagaaatcgataccgaaatcaggcagctggacaacacactccagtcgttaaacgaaaaagaggttatccagctgaataaattactggataaaatgctggatagctatcattaattaaatctcttccaggtagttaagatctttgccaaatgtttcttccaccttccaggctgtaatcaacgcaacgccaatacataccactgccacaatagccccgctttgaaggaaagtaaaatatttctgtacttgtataaataatatagagatcaacggtagcattcccctcgcaaaattcggaacagtagtagccacggtagcccgcagattggtaccaaagctttcagctgcaatcgttacaaaaattgcccagaagcccacgctgaaaccgagtatacaacatacggtatagaacacccatgtttctacgccatgcaggtttaaatatacagttaccattataccggtgaaaacgaggaacaataacatcaccttccggcggcttctccatagctggctgatcaaaccggaggcgaaatcacctactaccagccctgcataacaaaacgctatcgcgtcgccggggctgatggcgccttttacgttcatcatagtggcaaacttgttggaaaaagcaatgaggatccctaccacaaaccaggtaggagtacccagcagcatacatttcaggtatttgataaaccgctcgcggttagtaaacaaagccataaaactgcccctggaagcggatgaacttttcaccacattaaataaatgggattccattacgctaacccgcaggaccagcagtgccagtcctaaaccgccgcctatgaaataacagatccgccagtcgcctaccagcttggcaatcaggttggcagccactgcgccggaaacccctacagtagccacaatcatggtaccatagccccgcttctcttttggcagtatctccgataccagcgtaataccggcgcccagctctcccgccagcccaaagccggccacaaagcgccatagcacatacccgttgatcccctgaacaaaaccattggcaatattggcaacagaataaatgaggatagaaccgaacaaaacgctcagcctcccctttttatctccgataataccccagaaaatacccccgatgagcaatcctaccatctggatattaataagcagcataccggcgccggcatcaatttcactatcaggcagccccagtgatttcaaactcggaacccttacaattgtaaacagcaggagatcataaatatctacgaaatagcccagtgatgccactataacggcaatgttgaaaatggagacgggacggttgtcggctttcatttcttaatttggttgacgataataacgggaataaaaaaaagggcctcatttaaaggcccttttaaagatataaaaaattatattggagaatcagttttttctgtttcagcaggtgtgtgcgccggctgttgttttaccttaccaaatactactttaataagtactggtaaagtagtgatcaccactatgaccaggatgatcagttccaggtgatctttcaggttggggaaggctttatccaggtagtgacccgccagcatcatggaaaatacccatgcaaaggagccgattatattaaagaacatgaatttcttaccatccatacccacaatacccgccactataggcgcaaaggtacggatgataggcaggaagcgggcaaagaagatagcgccgccgccatactttacaaaaaactcatgggcctggtgcaggtgcttcttcctgaaaaagaaagtatccttcttcttaaataaaataggtccggattttttaccaaaccagaagccaaccatatttcctagcacaccggcggtggcaatcaggaacataatcaccacaaatggaagatcaaagaagctgcggcaaaggtcttcgctgtagatacccgctacgaagagcagggaatcccctggcaaaaagaatccaatgaaaagacctgtttctgcaaaaataattcccagtaacaggtaaaggccaccatgttcaataatccacgagggattaatgaggtgtttaaaaaactcaataatctggtccatgctaaatacgctatttctatttctgaagtggtaaaataatcaataaactgttacgcatttgttaagttaggctttggcagcatcttctgttggcggcgtaagcttattttcccatttggaaacaacggcggtagccatcgcgtttccgataacatttgtggcagaacggcccatgtccagcaaatgatccacgcccagcagcagtataaggccggcttcggggatcttgaacattgacagcgtgcctgcaatcaccaccagggaagcacggggtacgcccgcaatgcctttactggtaatcattaataccagcaacatggtaatctgctggtcgatgctcaggtgcataccataagcctgggcaataaataaactggcaaaggtcatatacatcatggagccatccaggttaaaggaatagcccaggggtaatacaaagctaacaatgcggctgtcgcaaccaaacttctccagctcttccattgtacgcggataggccgcctcactgctggcggtaccaaaagccagtagcagcgggtctttaatcattcccaggagcttgaatacccgtttgcccaggatcaggcttcctaccagggaaataaccacccacaaacagagcagcccaaaatagaactgcaaaataaacttaccataagttaccagtacaatggggcccttcagcgcaatgataccggccatagcgccaaataccgcgaagggggcgaagttcattacaaaacccgttactttcagcatgatatgggcaacgctgtccagcagtttcactaccgggttggctttttcgcctatggctgccgccgctacaccgaagaaaatggcaaataccacgatctgcagtatttcattatgggccattgcatccactacgctatccggtactacatggcggaaaaatcctttcagggtcatatctgccttggcgatgccggaagaggcatgttcatcaggcagtggcaatgccagtgataatcctggtttcagcaggttaaccaataccaagccgagaaacaatgatacaaaggttgcactgataaaccacagcattgtttttccgccgatgcggccaacagcttttatgtcgcccagcttggccacacccaccacgagggtggaaaataccagcggggcaatgatcattttaacaagacgcaggaagatatcggtaagaatggagatattatcagcgaagatctgcggggtatccttggctcctgttgtaacaggcgcattgccataagtaaggaaaacaccataaccagtgcctattccgattaccatagcaatgaatatatataaagtaagcagattcgatgatttcttcatgctagccagaatttatcttgtaataattaaaagttgtaaccggaaaatttcccaaaaataaggttaagcagctaaacatgcgctttggcaggtaaaataaaactatctgtttttgattttagatattatatttggcgatcaacagaaatacaacaacaactaaactaccttaaaacatcaaccacaatacgactgcgtatgagcaaactctttgctaaaaaacaactgtctgttttattggccgaagctggagaatctgaaaagggtctgaaaaggacgcttggtgcaggttctcttatagcattaggtattggcgctattattggcgccggcctctttgtaagaacagctgcagctgccggtcaacatgccggacctgctgtcaccatttcctttattattgctgctataggttgtgcgctggctggtttatgctacgcagaatttgcgtccatgatccctattgcgggaagcgcctacacctattcctatgccacactgggagaatttattgcctggatcattggatgggatcttgtgctggaatatgcgctgggagcggctaccgtagctattggctggtcgcagtatctcaataagctgcttaccaatgtctttcatgtcacgataccgtaccagtggtgtcacagtccttttgaaacttctgatgccggtgtacagggtatcatgaacgttccatcgctgtttatcctgctggcgctcactttgctgctcatcaggggaacacagggttctgccattgtgaataacatcattgttatcactaaagtagccatcgtgatgttattcatcttcctgggatggaaatttatcaatcctgccaaccatacgccatttaccattcctggag

SEQ ID NO: 5 - DNA, 615908 bp, Chitinophaga pinensis
  source 1..615908: mol_type = genomic DNA
cgtgggcaatgtaaccataagcgctacacaggcaggtgacgccaattacacggcggcagcagcggtgagccagtcgttccaggtagcgccggccacgctgaccgtaactgcggatgataagcaaaaagcatacggcactaacaatccgccgctcacttataccatcgccggatttgtaaacagtgaaaacaacagtgtggtgaatggtacaccgggactcagtaccagtgctgataacagcagcgctccgggtgcatatcctattaccgtggatataactccattgacagcgaccaattataccttctctgctgtaaatggcagcttaacggttggactggcgccacaaaccatcaccttccccgctatcactgataaaacatacggtgacgccgcctttacactcggcgccaacagcagtagtacgttagcggtgagctacagcgtggtaagcggtccggctaccatcagtggcaatactattaccattaccggcgcaggcagcgttaccattgcggccgatcaggcaggtaatggcaactactcgccggccacgcaggcaacacaaacattcaacgttgccaaagccatactaacggtaacggctaatgataaaaacagggtatacaaacaaactaatccaacaccggattatactgttaccggttttgtaaacggcgaaaacagcagtgtagtaagtggaaatgccgccattactcatactgccgatatcaacagcgcaccgggtgtttatccgattacggtcactgcgggtacattaacagccgctaactacgactttaacttcgccaacggatcgctcactattacaaaggcggcgcaaactatcaccttcccggctatcaccggtaaaacatacggcaatgcagcctttacgctcaacgctaccagcgatccagggttaacagtaacttacaccgtaaccgccggtccggctacggtgagtggtaataccgttaccatcaccggtgcgggcaatgtaaccataagcgccatacagacaggtgacgccaattacacggcggcagcggcagtgagccagtcgttccaggtagcgccggccacgctgaccgtaactgcggatgataagcaaaaaacatacggcgctaataatccgccgctcacttacaccatcgccggatttgtaaacaatgaaaacagcagtgtggtgaatggtacaccgggactcagtaccagtgcgaataacagcagtgtgccgggtgcataccctattactgtggatgtaactccgttgacagcggccaattacatcttcacaccggtgaatggtaccttaactgttgggctcacctcgcaaaccatcaccttccccgctatcactgataaaacatacggtgacgccgcctttacactcggcgccaacagcagcagtacgttagcggtgagctacagcgtggtaagcggtccggcttccatcagcggcaacaccgttaccattaccggcgtaggcagcgttaccattgcggcagatcaggcaggcaacggcaactactcgccggccacgcaggcaacacaaactttcagcattgccaaagccacactaacggtaacggctaatgataaaaacagggtatacaaacaaactaatccaacaccggattatactgttaccggttttgtaaacggcgaaaacagcagtgtagtaagtggtgatgccaccattactcatactgccgatatcaacagcgcaccgggtgtttatccgattacggtgactgccggcacgttaacagccgctaactacgactttaactttgcaggtggatcgctcactattacaaaggcatctcaaaccatcaccttcccggctatctctaacaaaacatatggcgatgcggcctttgcgctcaacgctgccagcgatgcaggattgcctgtagcttacgctgtaactgcaggtccggctacggtgagtggtaataccgttatcatcaccggtgcgggcaatgtaaccataaacgctacacaggcaggtgacgccaattacacggcggcagcagcggtgagccagtcgttccaggtagcgccggccacgctgaccgtaactgcggatgataagcaaaaagcatacggcactaataatccgccgctcacttataccatcgccggatttgtaaacagtgaaaacagcagcgtggtgaatggtatagcgggactcagcaccagcgcgaataacagcagtgtgccgggtgcataccctatcaccgtgaatgtaactccgcttacagcggccaattacatcttcacaccggtgaatggcaccttaaccgttgggctgacctctcaggctatcaccttcccgactatcactaacaaaacatacggtgatgcggcgtttacactcggtgccaccagtagcagtatgttagcggtgagctacagcgtggtaagcggtccggctaccatcagcggcaacactgttaccattaccggcgcgggcagcgttaccattgcggccgatcaggcaggcaacggcaactactcaccagcgactcaggttacacaaactttcaacgttgccaaagccaccctaacggtaacggctagtgataaaaacagggtatacaaacaaactaatccaacaccagattataccatcaccggttttgtaaacggtgaaaacagcagtgtagtaagtggtgatgctatcattactcacaccgctgatatcaacagcgcacctggtgtttatccgattacggtgactgccggcacgttaacagccgctaactacgactttaactttgccaatggatcgctcactattacaaaggcggcgcaaactatcaccttcccggctatctctaacaaaacatatggcgatgcggcctttacgctcaacgctaccagcgatgtagggttgacagtaacttataccgtaaccgccggtccggctacggtgagcggcaacactgttaccatcaccggtgcgggcaatgtaaccataagcgctatacaggcgggtgacgccaattacacggcggcagcagcagtgagccagtcgttccgggtagcgccggccacgctgaccgtaaccgcggatgataagcaaaaagcatacggcactaataatccgccgctcacttacaccattaccggatttgtaaataatgaaaacagcagcgtggtgaatggcacaccaggactcagcaccagtgcgaataacagcagcgcaccgggtacctatcctattaccgtgaatgtaactccgctgacagcggccaattacatcttcacaccggtgaatggtaccttaactgttgggctcacctcgcaaaccatcaccttccccgctatcgctaacaaaacatatggcgacgccgcctttacactcggcgccaacagcagtagtgcgttagcggtgagctacagcgtggtaagcggtccggcttccatcagcggcaacaccgttaccattaccggcgcaggcagtataaccattgcggccgatcaggctggcaacggcaactactcgccagccacgcaggcaacacaaacattcaacgttgccaaagctgcgctgaccattaaagccagggacgaagtacgaacctataccggcagcggctatacaggtggtaacggggtagactatacgggattggtgaatggcgacggcgcaaccagtttaaccggtacgctggtttacacaggtacatcgcaaggagccattaatgcaggcacttatatcattacgccttcaggtttaacggccagcaactataacatcacctttaccaatggtcagctgacaattgcgaaggcgcagcagcaaattaccttcctcgcaacaggtaataagaaccagggagatcctgattttattctcactgctactgccagctccggactgccggttacgcttagcagcgacaacagcgctgccattagtatcaatggtaatacagcgcatgtgggaacagccggcaccgccaacatccgcgcgtctcaaccgggcaacagtaactacgaacctgcccaaacgatcacacaaaccattatcgttaccgcatggaccgcaccggtaatcaccgcgcagggcagtaccactttctgcgcacccaataccgtgacgttacaatccagcggcacaaccacccatgaatggtaccgcaatggaattttaatacctggcgcaacgggccggtcgctgacagtaaatgaaagtggcagctacaccgtcaaagcgatatacgacaacaacatcggtgtgctctccgcagcagtatccgtaaccgtaaatccattgccggcgggtgaagtacgcgcaaatggcaacaccaccatcagcaagggagaaacgatcagtcttactgcttccggcggcaatacttacgcatggtcgcccgccacaggactgaatgatgccaatatcgcatcccccatagcccgtccggcggttaccaccaactaccaggtaaccatcaccggtaccggtggttgcagcgttacaaaggatattacgattaccgttaaagaagattataaactggaagcgactaatatccttactccgaacggcgacggcaaaaacgacctgtgggtggtaaagaatatcgatatgtatccgcaaaatgaagtcaggatatttgaccgttcagggcgcatgatattccatcagcgtggctataccaacaactggaatggtacggtaaatggtcagcgactggcagaaggcacctactattatatcattgatctcggcaataacgtgccgaagtttaaagggtttatcactattgtcaatgcaaattactaagcaaacgactatgaaaaagtatgtgagatatatcgcactgctgggagctttcgctctcggcagtcaatatgcaggcgcacaaactgcaggcaatccaaccatgatgtatgagccactggcggcgcaatacttcctggatcagtacatggccaatgccgcgatggcagggattgacaccgggttacatgtatacatggcttatcagcgccagtcgtcagatatacctggcgcaccggtggccaaagcccttacggccgactatatgctgggaaaacgtgtaggcattggtatgaatatctttaacgacaaagctggtttaatcaacagtacaaaagtggcattcacttatgcataccacctgccactgagtttgagcggtgtgagtgtattgcattttggtttgtcggccgcatttgtaaaccgccggctggataccaaagggatcaacggcgatgtaaccgacacctatatcaatgcattcaacagaagagataattattttgaaggagacttcggtatggcctatacccgtaaaggacttacactgcagggatctgtacccaacctggtgagctttgttaaaaacaaagccgaggatgatggaatagaccgcgcactgtacttcgctgcagccggttataaatttgaaatggccgggcagctcaattcaatagaaccgaagatatgtatgcgcggcgtgaaaggatatgataatattattgatgccggcgctaatttcatcttcctgcaacaacaactgaatgcattcgccctgtaccactcctcgaaaagctttagtgcaggtgtgggcgtaagctacaggtccatagccggattccagctaatctacaactcgcagacggcaggcttacgtaattataccaatggaacatttgaggtaaacctggtggttcatcttttcagataagacttgcagtactacctggaaaaaaggggattgtatcaaaagcattttgatacaatcccctctcctttgtatataaaaaatcgtatcttaagccggtatttagcatcctgatgataccccatcttcaggaacattaaacggaacattgcaaaaagtaaaacatgatcaaaaaaattaacccgctggctggcgcgctgctattgctgttaaccgctacctctactgttaatgcccaatcctcccctgctatgttaatggtatatgatgattattccggtaaagaccctggtctcacttactggaacaatggaaaaacgatccggctaacggatggcaaaacacaggcgggagctgccgccattgcggtatcaggtaatgacgagtatgtagccggtcatgaatataacactgccggggagcctgttgccacttattggaaaaatggtaaagctataacgctcgctaacggggaaacatattcgaaagctgttggtatcagtgtatcaggtccggatgtgcatgtgattggaaacaatggcagcgatgcggtgtactggaaaaacggcgtagccgcctcactgggtaaagacacaaaactgcacggcattgtgctgggcggcggcgatgtgtatatcgccggctaccaggcaaatgaccagggtgaatatgttgccacctgctggaaaaatggaaatgcggtagcactgtcggacggaaaaacgagcgcggaagcacatgccattgccatatccggcaacgatatttacgtggcgggttttaaaattgatgaagccggaaaggaagtggccatgtattggaaaaacggtgagccggtgatgcttccggatggctgcagggcaaatgccattacggtgtccggtaatgaagtatacgtggcggggatcgacagaaatgaggccggcgcaaatatcattgtatgctggaagaacgggaaagcagtgaggctgaccgatggaaaagaagaagccggcgccggcgtaaatgtaattgcggtggcaggaaacgatgtttatgtagccggctatcttgatggcaaagccacctattggaaaaatgaaaagccggcaggtttgaatgacatcatcggcggaataaccgggttagtgatcagatagctatcttcatccggccgttgataaaaaaccgagaaccgttgcaataatagcctcaggcgcatcttcctggacaaggtgttttgcctggggcactacatgaaggcgggcgtttccgatacgcctgctcagttcctttccgcgctccaaaggtatccactggtcatcttcaccccataaaattgttaccgggcaacggatttcagaaaaatggttttctatttcgtcggtatattgatcgctcatctgtgcgatctgccggtagaaagccgcctgacctgtttctcccaaccagggttgcaggtacagctgcattacatcttcaggcagcggatgaaatgcagcgccactaatatatgcgcgaaggatcgcttcatgaatataagcgggaagccccgtaaaaacttccggatgattttttgcggcctgcacaaatggagagcccgacggtcctattgccaccggatcaatcagggtcagcgagcggtaatcccggccgtcgagcaagtgcgtccgcaatgcggtggtgccgccaaagtcatgcgccacgatatcaggccggtccagtccccaatgttgcagcaatgcagcgaaaactttattttgaataccaagcgatacatcctgcccttcttttttttccgaatatccgtaaccgggaagatcatagtaaaatacctgcctgtgttctgccagccaggaaccaatacgcctccatacaacggaagaaaaaggggttccgtgaagcagtacaagtggtgcacctgttcccagcaccccaaatcgtatttcctgatcctgaaatttgaatacttcggccggcgccggtatgtgagacatcagctgcataatcttcttttttaggttaacctttacatccggcgcaaagactatacccatctaaactgcaggcagcgctgcggtaaaacccttgtcaggatttcaaaccaatttgcattattttataaatcaaataatgtaaattacaagctatgatataatccaatccctcacattatgtcacatgaaaaccttaataccggagcgatacactcctctccctcagccgctgcacaccatcacagcatttcaggaatatcaaggccagccgttcagccgcttcaaaaaaaatcttcaaaaaaagatgaggaggaagaggttcctctgcaaatgaactcaacagccgttcagctattccgggggagaactggaaatgatgaaaacaggcaggcagatataaagccgtttcaattaaaatcaaataacaccggtttgcccgatagccttaaatcaggtattgaaaatttgtcgggttatgcaatggacgatgtaaacgtacattacaattcccatcagccttcacaactacaggcgcacgcttttgcccgtggaacggacatacatctggcgcctggtcaggaaaagcatctgccacatgaagtctggcatgttgtacagcaaaaacagggaagagtaagtcctactacgcagttgaaaggcaaggtaaacatcaatgatgatgctggcctggaaaaagaagctgacgaaatgggccataaggccgtacagcttgcaaaagatcccgcagccgtaccctataaagatttcaaaaaacaggcgcctgctttaactgttcccaccgcccaactgatgctgatcaacggtgtagacgttacagggtcgtccaaactggatgacctgaagcttgccatgggctggcatccgcattttgggataaccaagccactgaaagaaaatgaaaagacagaactggtaagactgatccggttacttaacagcgatgatatccaggttggtaatataattgaagacctggaggcagaatcatcagcagatgaaaaagaagaaaaagagaaaaaggatggaggggatgaagaagaattggaagaggacgagggatttggacctgaagatttcccgggcgcccagaacttttcatttgtccaggttccgcaggtatcccagcaacggcaacgccgtcagacgcctgaagagtttggatgggaaaatttccccgagactttccggggactgaaaaagctcggcatccacgaaactgaacatgcaaacgtagagagcctcgtggcgaacggccccgcagtggaaaaaatagattccgccaatcatataggcaaaggacctgggttttacgtatcacatgtagggaaaaagaagcttgctaccgtcgtgagcggcgtcgtatatggcgacagctttgttgctatatatatcaagtcaggcattgcggcgagaaaatcacctaacgaggagagtaatcatgtagatatcctcgataaggaatatggcgacgaattatgctattatatcatgtccggaggtggggaaattgttattccggaaagatgctttccctttgtaaaagcagtatcagtccgggaacagctaaatcagatcagcaacgagagaaagaagaaaacgagaaaagagaaggaagtagaagtagaagaagatgatggtcatggtgataatgaagcggcattaaacccggaccaccagttagccatgatcatctacgacgaagaagtggatttcgtacgcagattgaacctgttatcggatagatataacaatgcctccgccagcgaaagcctcagagcgcggattaagaaaagattcctgttcatgcaaaaaacggcctttaacaaatgggctatgaacagccggctgtataccgtttggtggaccatcaggccaattggtacgcatacgccaatgccgccgcatccatagcactgttttggaaaaacaaattcccaggcaacgggaacactttcgctattcgaagatgttcccattgtatcattcagcatttaaaatttgagatacccggcagcgcttaaacggaacggcatttgcggaattgtagttgcccatcctacccaatatttttcattattcaggttatcagcctttacaataacacggtaacgcggttgttcatagctaagggaagcattcagcgtggtaaaagcgggcagggtataaagcgaagtggtgcttacgtctacaatgttatcgtcggcataattacctccgaagcctatccccagtccttttagctgaccggcgggcacgcggtagctcagccagaagttggccaggttgcgggggccggcactgcctggccggaagccttccagggccggactgcttttcttaagcttgctgtcgttatacgcataccctgccacgatatgtaatccgcggaaaggcatggctgtaatttccccctcaattcctttgctgtactgtataccattttgaacagtaaatgcaggccgttccggagcatccggacgggtaacatccgacacgcggatggagtaataactcaggcttcctgctaatttaccattcgccaacccggctttaatacctccttcccattgattggcctggctcggcttgaaattgctggtggtgccatcgggctgctgcacaggtgctatattttgaaatccattgctgtagttcccaaacagggaaagctggtctgctatgatctggtaaacaagtccgaattttggcgatactgccgtttggttatacttgcccgtggtggtgtccctcgtcagattctttgtgccgggattgtcgaaatagtccacgcggacactggccatggctataagctgctccgtaatattgagtacatcctgcacatatacactatacatattttgcacagctttggtgcgggtatatgcgaggccctttatcctgtcctgtaacgccagccggttcagggcggaatacgctgcccctggcttggttacgcttaccacatcaaagacaactgttccgggagaactggacctggtagttgccgaatagatatccgttccaaccagcaggcggtttcgcaggcggcctattttaaaatcacctgtcagattatattgaaagtcggtggcatagctattcgtatattccgtataggtcatgttgcggctgagcgaatcattccctgctttcatacttaaatagccagttgccccgccggcctgcgaagtgagataggtataggtggcgcgggcttgccatacgtctgaaaaacggtgctgcagctctgcaaagaagttggtattggtgggggttacaaaaaggtcgtcgttgctgaaccgccttttaaaatccatgttcagcgcttcgggactccgcacgccgctattatagcttccatcagcgaaaagccggtaaaagctgtttgccttctccttcttgtactccgcttccactgtcagctttgttttttctgacagctgatacgtaaccaccggggccacgaaaaaataatttttaaagcctgcatcctgaaaactgccttctgcatactgggcggcatttactcttgccaatacccggtgtgccttatcaacgggtacattcacatctgcctcaaaccggctgagcccaaatcctccaccggtgaagcctatacgggtttgaaaggtgtcgagcggtttttttgtgacgcggttaaacaagccgccaaacgataccaggctggaaccaaacagggcgccggagggcccttttatcgcttcaatgctttcaatattggcggggtccagtgtaccgccgccaataatacccggcacgccgttccggagaaatgactgtgtggcaaagccacgggaagtaaccgtaccgcctgcactgttattctccagttgcatgattacaccaggaacgtttttcagtgcatctgcataaacaacattcagctggtcctgtaataatgcctgtgttaccgttgtatacacctgtgggttttcgaggttgttcaatggcatcttagccgcgaaaatgctttgtgttttaataaaccggttcctgccggaagtaacgtttacctcggcgagttgcttttctgatacctgtaattgcagggaaatagtttccgtactgcccgggcgaatggtaatactccgttgcaatgtttcatagcccatgagagaaatcaccaactcatagctgccgggcaggatccggtttatctggaaactccctgtttcatctgttaatacgctgcgcctggcttctttcatcacaatagttacataggcagccgctttcttgtcggatgtatacaccgtgccttttaaagcgccagggttaatgctttgcgctgaaatgccatttataaataatgtcagtgaaaagatagcaaaggcaaatattttggagatcattgttattttttgtccgcaaaaatggacaaatacgcagcggtaacccacgcgtatccggaatagtttttacgcaattgggaacttccatttgagtgaccgttattgccggaagtatcttatcaagtgcatattacttaatgatctcccaatgatatacgaagccggtttaaagcattcataagcgaaatgctggtggtcaaatctactatttcttttgtggagaaatgattttcaagatcccgctggtagccggttaaatcaccgtgcaactgtgtgatggcttcagcccattgtaatactgatttctgcctggcatcaaatgaggaagaaagtttccatccgggtaatttgtccagtaaacgctggtcatatccaaactcacggagctcattagcatgaaaactgcagcaataggcacaaccatttatttgagatacccgcagttctgcaagggcgattaatttaacatctatctccgactgtctcaacgttgcatgagatttatataaataaccaaccgcttcttttgaaatttttatgtaatccatattatctataattttggcgcaaattaaaataccatcacttcaatagacgatatgcacttttatgtgatatacttacaaaaacgaaagtgtgttgacattcaactttttactcatgcctgaattttttcatgataagacgctctactataccccaatggaatttgcactgaagcatattggcggcacctggaaaatgccgatactctggcgtcttcagtccaatgtgctccggtatggagaattaaaaaaagatattccgcatatcactcataaaatgctggcaagccaactgaaggaactggaggaaaagggattgatcaggcggaccgtttacccggttgtgccgcctaaagttgaatatgcgattacttcaaaaggattgaaagcaataccggtgattgaacatattatgaagtatggatatgagctgatccaggaagccggcattgagtatccgcctaagtaattataaagtcttcttcagttttatctctacattctctccttccttttctatggtcactacctttttaacactggcgccagcattaccagcataactcctgacggtggtgttctctcgggtgccctggtacaagccatttacataagtatcagtataacctactacttcggttctcctggaggtatgaacgtaaccaaattccgcaaagatcaggtagtcgcctggcatcaggtttacaaattcaaaatgtcccttgtcgtcatataccgttgccgtcttgatacactctgccgcctctttaggaagtggaacaggtcttccttttttcctggatgattcatttaatttcacccactctttaaagaaatcggtatagggaatcaaaacgatggaggtacctgtcggtgcgaattgctttttattgatattgagtacggcaatacctttcagcattccttcattctcgttatcttttgcaaaggcctgcccgctaattaccgcgctgcccgacttgatcagtttcatggtagccactttatcaaaagtgttcttaaagggattaaaatctgtctccctgtccaccatcagaatatgctgaccggcattggaatggatatccaccttccacaaccggcgggtttctttgtcgatgtgatacacgtacttgtctttggtggcctcctcaaatacggtcaccagccaaactttatgcgcaccggtaaggctgctggtgtacataccgctggttacttcctcaataagcgccttctttaaattattcgtattctcgggccggtaatcgtacaccggcatatttgcactgtacccggaagtaagcggaagtaatccaagtagatagggataacaataaccatcaaaaaatgcttctgttaccggttccttaatgacacgctttttgcggctttgtttgtcgtaatgataacctgtaacttccttcccatacttcagctgcaattcatagttgctgttaaaagaggaacggtaaagaggggtaaaggtcttcccgtcagaaataatggtatcaacccgtggatcatcagaaccggcctggtataatgtggtataaatagacaaggtctctttattcgcattaatatcaatgataaatgaactgatctccctttccatggcgccatctacaataaaacagcccatttcatacttcccggttttgaggaattttgtatcaaaaggaatgttccctggtgttaacgcgacttgtgctttacagaaacctgctgtaatgaggagctgcagcgtaaaaaaaatgccccgtacccgggaatgcttaaaactgatcatgcttgttcaatgtgctttgtccaaaatataggtaaccggttgtgattttcttgtaatctgcaagatactttgtgtatgtaattcctcgtcaaaagtaaacgcttttccggcttgttggactactggtaatcagggattttatgctactggtttacagggatttttcaacgcgctgccgttgtatcgggcaagactttccgggagctgctccattaccttcgattccttcattatcatccttttataggaaatcccgcttttatttatttaaattgccgtagtaaaacgccacgttgtgaatactatagctgctttgaaacaaggtaaccttttggtatttaatgaagtatattattcctgccacaaaaggatctactattttattctccggaaaacaaagtcttctttcatcgcagaggaggtagtacagcttacattcatcaaattctggaactaccgggaaagcctggcagacgacctcgacgtgcagctccagctgttccggattgcccgcactaccctgatcgactttctccggaaggaaaccgtgtacaaggaaaaggtgatccatgtaattgagcggtataccctgccggcggatgagctctggggcaagctggccgaaaaggaactgcagcataaactggcccatgcattggaggaaatgccgcctatgcgccgtaaagtatttgaaatgagccgttttaaaggcatgagctaccagcaaatagcgcatgaactttccttgtcgtccagaacagtagagtcacacatcttccaggccatcaggcaaataaaacattatctcgggctgctgctatcccttgtagcctgctttttcccgttttgaaaatatttttccattccgactaagtagttggcctttcacgaacgtattacttatctatcagccgtacataacatgataaatgacgaattactggcgcggttctttagcaatcaatgcacaccggcagaagcccgtgaggtagccacgtatctccgggagcatccggaagtactggagaaatatctgccggaagaagaattcctgcaaatacaggacgatggtaattttccggaaactgtttcccagcagtggctgaaaaatatccaccgccaaagtgcatctgccaatagccgtatgaaatgggcgaaacgagtggccgtcgcagcaataactgccggcgtgctgataggcgcaagcttgttactggtaaaccgtgaccatcaaaaggaaacaaccattgcttccgcagcaatgccatctattccgcgggaacaacaggaacgcgcggaaaacaacagtggcaaaaccatcaccaccgtactgccggacggatccgtgatacagctgttcccgacggccagcatagtatacgataaacagttcagggaaaacaggaacatatatctctcaggagaagcagattttaccgtagtagctgataaattacatcccttcgttgtgtatagcagcgaactgaataccaccgttctgggcaccttttttcatgtgaaagcaatcccggcggaagatataatcaccgtaaggctcaataccggtaaagtattgatacagggaaccgccaataataaaaaggtagtacttacacccggcaaagagctccggtattaccgcaaaacaggaaaatccatcgtagcagacttcaatactacgggcacggatatattagtaaaagcaggaaacaacggcacgagcagtgcaaagccggactggtataaattcaataatcaaccaatggcacaggtcctcgatcagctgagcaactattacggcgtagccatctattattatccgtcggatgtgacggaaatttatttcgatggtaagtttgaaaagacggactcactggtgaagatactgaccgatttaacgcttcccaataatctgaagcttatccggaacgatagcggatttattattaagaagaaataattcaacaaattacagttctattccacaaaaggcgcaaaggcgcccggggcttgctatgccccggattcaaaaaaaacacgtcccagttatgaaaatgttttatcgaccaaaatggcgtttactcctgctgctatgcatgctgttaggaggtgtatcgatgtcttctcaggcccagggccgcctgcaggtaaccggaacggtgcgcaccgatcagggcgaactcctccccaatgcctccgttgtagcgctgaatgaaaaaacaaagtattcggccggcgtaatcaccgacagcaacggcgtattccgtttctcgggattaccaccagaaggcaaatatttactcagcgtttcttacatgggttttgaaacacaacaactcaataatgtcagtctcaagccaggcgccacattaactttttcggtacgcctcgtgaaaacggtagcagccctgagcgatttcatcgttatcggctatggtaccgcccggaaaaaagatgtggtaggcgcctttaacgtggtgaccgtaaaagaagccggtgcagtaaatgccaccaacccttcccagctgctcatcggtaaagcagccggcgtacaggtggtacaaaacagcggcgccgccggtgcagatgcccagatcatcattcgcggtacgggcagtttcaccgacatcaatcccctgtatgtagttgatggcatccagggaacaaaaaacctgtttaatacactcaatccccaggatatagaaagcatcaccatcctgaaagatgcgtcttcaactgctatctacggttctgcagcggccaacggcgtagtgatcatcactaccaaaaaaggaaagcccggacctccccgcgttagctttacttcccaatggggtgtagccaaagcatggaaaaaactggacctcctcaatgccgcgcaatatgtagatgcgctgaaagacctcgcagctaccaaaaacgcggtactcccggcgaagttcaatacagcagcggtattacaggacagcaccgactggcaggacgaaactttccgcaatgcacttgtatctgaacacgatctcaatatcagcggcggcggggaaaaagtgaactactctgtatctgccacctatatcaatcagcaggctatcatcaccaacgctaccaacaaaagattccaggcccgcgtaggactggaagaaatactgggacgtttccggtttacacagaacctgatattcaggcagtatgtgggcaacggcaattatgccagcatcatcaacgccatccagtacgcgccctataaacccatactggacccaaatatacagggtggctactctatcctgtccaacatcgacgactacagcaacgccagcaaccccctgcaggatattgccatgaaaagtcaaacgagcaaatccctggccttctttccgcagctgtccggtgaggtacgcatcatcgacggactgaaattccgctcgcagtttgcagcagaagtgaacaccaaccggaacaacagttaccagcaacagtaccagtcgtccaacttcctgaaccaggcccgccagtcgatgctgggctttacagagaactcttattatatgctggaaaactacctgtcgtacgataaagtacacggtaaacaccagctctttttaatagcaggacaaagttatatcgatccgggaatcaccaatggctctactatcagaggtactggtcagcctaacgataatattaccaacgtaggcgtagcttcttcccaatcggttaccaactcctattccaattatgcccgcccttcggtgatctcttattacggccggttgaactatacttttgatgataagtatatcctcaccaccagctatcgcagggatggcgcttccaactttggtgccaacaaccgttatggtaacttcgccgcagcgggcgtgtcatggcgcttttcagaggaaggatttatgaagaaggcattccccgtgttatcggatggtaaactcagcgccagctggggacaaaccggtaacaacagcattcccaacttcctgaatacgtcgaaaacttaccagggtactcccggaggctcactggtatactccttcggcagtaacgaaacatttgtttccggcaccacactcaccacgttaaataatcccgatctgaaatgggaacaaacggcccaaacagatatcggcatcgacctggcatttttaaataaccgccttaccattgaagctgattggtacaaccgtaaaagtaccggcctcctggttactaccctcctgccggccagtattggcgtaagccctaccggtacccagccaaagaaaacggtgaatgcagccgatgcgcaaaataaaggctttgaacttaccatcgggtataaggacaagatcaataataatttcagctataatgtaagcgtaaacgggtctatcaacagcaacaaagtattgtcattgggcgatcagttctccgcacctatccaggccggcgcctttacaccagtgccggctaccacgtatactgctgccggttatgctatcggttccttttatggctaccggatggatcatgtggccagggatgccgcggaaatcaccgcactggaccaggaagccgctaaaaaaacaggccaggcaaacgctaagtaccaggatggattgttacccggagattttatctataaagatatcaacggcgatggtgtcgttaacgcgaaagaccaggaaatacttggcaatgccattccgaaatacatttatggtatcaacgccggcgtttcttataaaaacttcgacctgaacctggtactctccggtatcagcggattaaaactcctgaacggcttaaaattaaataccagcattatggccacgggtcacaacgcttctaccgacatactcgacagatggcgtaaacccggtgatgtagcggctttgccaagaatcggacaaaatgctaccggcaatggcaatctccgtccgtccgactggtggctggaagatggcagctacctgcgtctgagaaacattaccattggttacaacgcaccattggccatgttaagtactatgactaaaggcactgttaaatcactccgcatttatgtggcagcgcaaaacctgatcaccatcacgaattacaccggctacgatccggaaatatcgggcgactacctgtttgcacgtggtattgaccagggacaggtacctcaaccaaagactttcctggcaggtattcaattagggttttaatttttaaaaagtattttatgaagaagtatatatatcatttgctactaaccgccgcactggtcaccgttgcacagggatgcaaaaagtcacgtctcgaactggtggatcaaagcgcctacgcatacgatacttattttaccaacatcagtgcgcttaaccaagctaccgtggccagttacgccacattactccatccgggattatgggcgcgggagtactactttattttcgacctgctgggacatgatgccaaacgcgccagctttttgcagggcgcagaacaggaactgggcgactatagctttggtaccagcaatgcagatctcagctctttatggggctccctgtaccggatgatcttcagaaccaacctggtgattgaccgcgccgcagcctggaatcccaccgctaccaacgatcgcgcaaaattaaatcaatacctcgcagaggtaaagttcctgcgggcatatgcatattttcacctcgtaacattatggggagatgtaccactgtacgtcgactatcagtctaccgttaacaacaactatttatcccgaagccctgctgcggatgtgtggaaacaaatagaaaaagacctcacagaagcacaggccactgccgaattgcccactgtatatcctaacgcagaattgggccgggccaccaaaggcgctgtcaccgccttacttggcaaagtatacctctaccagaaaaaatgggtgcctgcacaaacagaacttcaaaaactgatgggtgcaccgtacacctatcagctcgatccttcttttgataatcttttcagcactaccaaccagaactcaacggaaaacatcttccagatcatgaaccaacagtggaccgactggggcattggttctccttactatatgtttggcaatggcgctgaacaggtaggtaaacaaacacattcaggccgtgccatggaatatggctggaatgattggaagaatgtatacatcagcaacgccgctgtaaaagcatttacttacacgaatcctgcaaacggcctgccgtatacagatccccgtgccaaatccaccttctacggcaccgctgcctccggaggagaaaccgaatactgccagcagtgcgctaccggtgtaaaggtgtatccgtttgataccaacgatccgcagggcgattatcgctggaagaaatatgagtactacaatctgatggaaaaatatggcgatcctaaaagccctatcaacgggcaggtgattcgcttcgcagacgtaatgctgatgctggctgaagcgcagatccagcaaggaaatactggcagcgcaccattggcgctgatcgacagcgtacgttcccgctcgaacgcatttttatataccacgctgggcgataaagcaaacgcgatgaagatactgatgcgcgaacggcagctggaattatgcggtgaacaagcccgctatttcgatctgttgcgctggggtattatcaaacaaactatcaacgcagaaaaggccgcagaacctggcaccggcacacagcccttccaggataaacacctcctgctgcctattcccgatgtagaaaaaaattacaatccgaatgtagccaaagctatcagcaatggctggaattaatctataaaaacagcagggcacaaccaccggcaggaaatattttatagctcgttagccgttactatccttcaattccacttatgtaaaaattactaccatgaaatggagcaaaccactatttctgtcagggttgttaacccttggctgtaacctactatccattgcccaaacctataactggtccgccgtccgcattgggggcggcggactggtttccagcgtacaggcgcacccgttagtacccaacctccgttttattaccactgatgttggaaacccttatcgctggaatgaaagcacacaacgctgggaaggtctgttgaacggccttccggcggtgtactggccatcatcggccggcaacctggccttcgtgcccaatgatgccacgggcaatattctttacgtttccatgcctaaaggtaccggcagcgccggtactattatgaagtccaccaaccggggtactacctggacggatctgaatatgcctatctggctggatcccaacaacgtggaggaaaaaagaaacggggcgcggctggtagtagatccgaacaacagcaacgtggtatatgttactacccgctttccggccagtgccaatgaaaccaccaatggtacctacaggagtgtgaacggcggcagcttatttacaaaaatcgatacgctgcatggccgctttattgtatttgataccagcggcggaacacttggcggacttacaaaaagattatacatcgccaatctgaatggtgtatatgtaagtaatgatgccggcgcttcgttttcgttgatgcccggcagtcccgctggtttgaggagaggcgtgctgcgcggcggtggtattttatatgccgccggcaatagcaaagtatacaaatggaatggcactgcctggagtacgattaccccaccttatagcggcagttttaccagcgtggaagtaaatccgaataacagcaaccagatcatcaccaatatcgatgcatttaccggtgcaatgtataaaagcaacaacggcggttccagctggacacctgtaaaaggcacgcgcgatttcagcgaagtgccttttcatggcggcaataccataggaaacactatcattgatttagcctgggatccgtttgattccacacaggtatggatggccgacctgttaaatgcctaccagggcactaacatctggtcggatgcttcagtgtggaaagtacgcgccgcaggacatgaggaagtagtggtaacagggccattgatttgtccgccttccggcaacaatttgctgctaacggttaccgccgatgtggcgggctttgatcacaaatccctcaccaatcccccggcgaaagctatctccgacgattttcaatattttaattcccagggagtgcatatgactggtgccgccatccaggaaaccaatcccaacttcattgtgagagtgggccgcaggggctggtcaggtaccggtttaggcggctactccaccgatggaggactgcattatacacaatgggtttgccccggtggcatgaccggcggcagggtagccgtatcggccaccagcgaaaccattatctggaccacgcagggcggttatacctatcgttcggtggacaggggtaataactggacaaaaataaattccattactaccagcgccgtcggcacttttggcgtgaccggctccattttcaccgtaccaccggatatgaatcccctggcggctgataaagtaaatggtaataaattctacctgtatttttttggtaagatgatggtgagtgaagatggtggattaacattcgttcagaaatacgctaaccttccaaacgtgcaaaatgtagcgtttgtaaaagtagaaaccactcccggcaaggaaggcgacatatgggtgtcgatagaaggcaacggcctgtatcactccaccaattcgggcgccgacttcacaaagatcaccaaagtgcaatccgccaaactgatggccattggaaaggccgcagtaaatgatccggctatttatgtggtgggcaccgtggatagcattcccaacagcattttccgttccgataacaacggcgctacctggacagtggtagctaatccggctatcagtgtgccacggaatttagcggctgaccgccgtatttacggaagagtatttatgggcagcgccggtaacggcatatatacaggagaaaccgtagccggtcctgtaaccggcattacggtgagtcccgccaccgtgtcggtagcagtgggcaatcgtgctacattaaccgcttacgtggcgcctgcatgggccggtaataaaaaagtaacctggagttcgggagataccactaaagtaaaagtaaacgatagcacgggcgttctcacaggagttgctgtaacggcaacgcctgtactggttaccgcaaccacccaggatggcagtaaaacagcttcggcaagtgtaactgtcactacacctgttgccgtttccggcatcgttatcacgcctaatcccgattcaataggcgtgggtagcaccgtgccgctggtaaccgtgattacgcccgccaatgccagtaacaaaacactgcgctggacttcttctgataccactattgcaaaagtggccatagatacgccgctggttaccggcatctcgcatggtactgcggtgatcactgctacagcgcaggatagcggctacacctccactgccaccatgattgtttataacgtagcgcccacagcgctcaacattaccggcacagcatcggtaggcgccggcgataccgtgatgctaagcgcggtattcacaccgctgaataccagtaataaagtactaacctggagttcttccgataccactattgccaaagtaaacaacagtggcctggtgacggccgttgcacctggtaccgttaccattactgccacaacagcaaaaggtggtattacgggcactaaaggcatcaccgccactaaagttattaccgtagtgagtgcaggcgtatgtggtatactgcctaacaatggctttgaaggcggtcttagtaactggatgattgtcggcgatattattaacggtctccaaccggccgccatcgtggccaacaacgcgcatagcggcaccaaagcagccgtgatttccggagaaggcggcgttagcactaccgtactgatgccggtagccggcagaaaggccgtcaccttttctgcatgggcaaagatccttgatcttcccgcatgggcaggttttggtatcgactatatagattcttccaatcataaaatcaccgcggaccagttcagcgtaaatgctacgtcttacacacaattcagcgtagtaagggctacgcctcctaacacagcgagggtgaacatctggacctacaaaaccagcagcgccggtaaattttacctcgatgatttttgtgtgaccgtagctgatgtggtagatgttaccagcctgtctattacgcctgatccggcatctgtagccatgggttataccaaagcattaaccgctaccatactgcctgcgaatgctaccattaaaacagttacctggacctcttccaacacggctattgcaacggttaacgcatccggcgtagttaccggcgtggcattgggcaccgctaccattaccgctaccagcacagagggcgggaaaacagctaccaccaccgttaccgtaacgccgccggtagcagttaccggtgtgaatgttacgccggatagcgttactattggcgtagccgattcatatacgctaacggccaccaccactccagccaacgccagcaatcagaacatggcatggaccagctccaacccggccatcgccaccgtaaacgccaccaccggcgcggtgaaagcagtagccattggtaccgccgtgatcaggggggtaacgcaggaaggaagttacaaagacagcagcatcgtaacggtgatcagccagggacaatgcggacaaatttccaacaatggctttgaaagcagcctcgtaggatggagtaatatcaacaacgctgctaccatcactacagatgcccacagcggtttaaaagcagtagccgttaccggtcagggtggcgtaggacgcgtacctgtattcagtttcgccgccggcgataccatcgtgtttaccgcgtgggccaaagtatccggcggacccgcatgggcaggcttcagcctcgatttccagaatgcttcctatgtgaaactggccaccgcacaatcaactgttaccgctaccgcctatacggagtatacgcaaagcgtagtggttccggcgggtactgccaacttcaacatctggtcatcaaaatccggcgcagcgggcatcctgtatctggatgatttctgcctaaccgtgaaaccggccggcggaggcatgttacgcaccaccaatctcatgcaaaccggccatgatgcatccgccactaaaaacggcattaccgtaagcgcttatcccaatcctgtacaaagtgatatcaacatccgcctgaccaattacaatggcagccggatcgcggctacgctgaccgatatggccggcagggttatacatcacgaggtgattataacgcagaaaggcacaacgctttaccggttgcataatgcaaagaagcctgcaaaaggactgtacattctgaccctgaaaggcgaaggactagtgagcagcttcaagctattggtgcagtaggtattgattgtttgataaagagcctggggccatgccccgggctctttgcgttattacatacctattacaatttcttgaaaagcccccctactctattatctgcgggaattaattaccttgcgtaagcagcgcagcaggagaaacctgcgtctgcgccattacctctctaacaataaagttacccgtcgttgtttatgtatcagttgctccgtgacaatatcgaacagcatgtccatctcagcgatgccgagttttcgcactttgccacctcattcgaagcgaaagagattgagaaaaaacagttccttttgagagaaggtgaaatttgcaggtttgagggctttgttaccaaaggcatattcagcgtgtatcatctcgataaaaacggagacaaacagatactttattttgcccatgaaaactggtgggttacgaacatcgacagctttaccaacaacctgccgtctcagctctttattgaagcactggaagacagtgaagtattgttgatttcaaaaagcgacaaagagtccgcttatatcaacctgcctaaaatagaaaagctgttccgggtaatgacccaaaaaacgcatgtggctttacaacgcaggatgatcgacagcctgagtaaaacggctgatcagcgttacatcgacttcatagaaaaatacccccagctttaccaacgcctctccaacctgcagattgcagcttatttgggcgtaagtcatgaatttttgagtaaaatcaggaggaagatagctggtcagaaataatacgggttcccattattattgaacttgttcaatttttttgtttcagaaggaacggatatttgcatatcatcccaaaagcaaaaaaatgaaacgaatcatttctatagcattattgaccactttaaattttttcaaaatggacatacaggcgcaaagcttcactactattgaagctaatggtttaaagctgcaggtatacaacgcttccgagaacagctttggcgtggcatctgttatcgtatcaggaaaaacagatgctgttttgatagatgcacagtttacattggctgatgctgaaaaagtagcacaggaaataaaggcatccggtaaaaatttaaccactatttatgtttcccatggcgatcctgatttttactttggcctggaagtattcaaaaaatactttccatctgtaaatgcttatgcttcccccgcaacggtagcacatatcaaagccacggcacaaaaaaagctggcagtatggggtgaaaaattgggcaacagcattacttccagcgttatcattccgcaggtgctcgaaggtaacagcattgagctggaaggacaaaaattaatagttaccggactggaggaatttccatcgcggacttttgtatggataccatctattaaggccgttgttggcggaataaatgtatttggcaccagctttcatctctggatggcagattcagccagtgaagatgcccgcaaagaatggctggcagtgttagacgaaatagcggcacttcatccggccatcgtggtgcctgcccatgccaaagcaggaactcccttcagcatggctgctgtaacgcacaccaaaaactatatacagttttacggagaagcgctgaaaagcaataaaacttcggaggcattgatagcggcgttaaaagccaaatatcctgaacttacttttgaaaccgccctgcagataggcgcgaaagtaaacaccggggaaatgaagtggtaagagcgatgttcatccacagcctgacaaacgctctttcctttattcctttctcaggctgatcaccgggttcatcaaagccgctttgatcgcctggtagctgactgttactatggcaattgctacagataagatacacgcaagcgcgaacacccaccagtgaatagccacgcggtattcatagtactgcagccatttatacatgctccaataggataatggcgctgctatcacaaatgaaataatcaccagctttacaaaatctttcgctaataaagtagtgatgccggtgacagaagcacctagtaccttccgcacacccacttccttgatcctgctttccgccatataggtagcaagaccaaataaaccaaggcaggatataaaaatggtcagccccgcaaataaagcagctaaagttccctggcgttgttcattatcaaatttcttcgcataagcttcgtctacaaatttatactcaaacggataatcggggttatacttgctgaaaatagcctccacctttttaagattttgagcagtagaatgatccccgtttaacttcatctgcaccacctggaaattcataaaagcacttttggcgccgcagatcaatatcggtcttgttggctcataaggactggtaagaataaaatctttaataacccctacaatgtgccagtcgatgccaagatcatttactacttttccaatcggatccttgaacttcaatactttcagcgacgactcatttacaatcagcccggttgaatcggtggggaattttttcaggtcgaaatcacggccttcaataaactgtaaccctgctgtggcgcccaatccctcatccgctaaataccggtcgaaagatgttttatcattcggatcctttccttgccagttctggccccacccattgctccaccgttccgtaaggggggaatttgttctggtaaccgacttcgcaacacctgattccagcaattcattttttatcagtgcatagtttttggatatatcacccgtcatgaaatggtacaccaggttatctttattataacctgtttcccggtcacgggcatagtcgatttgctgctttacaataatagtgcagatgataagaacggtggcgaatgtgaactgcaataccaccagtattttccgtggcgttaccagcgcattcgcttttttaaacgtgccctttaatactttaacaggctggaaagaggaaaggaagaatgcgggataactgccggccagcaaacccgtaaagaaaataaacccaataaaccctatccaggtatagatgttgccgaaatctataaacagttttttatccgtaagctggctataaaagggcaggcttatctgaacaataaggatcgccactattccggccagaaatgcgataaaaacagattccccgataaactggctgatgagggaactcttctgtgctcccactacttttcgtatgcctacctccttcgcccgcttttcacttctggcggtgctcaggttcataaaattgatacaggcaattaataatatcaaccccgcgataatactgaatatttttacgaatgtgctgcggcctccgttatcttccccaccatcgctgaagcttgaatacaaccgccacctttcaagcgggtaaataaacagctcccatttcattgttttcgcctcatcactgtaatgctgctttaaatcttttattttagcggcggcggcagcataacttacattgggcttcagcattacataagtaggcgtgctgttatcgctccagccataatccgtgccttccctgtattttaaatatgaccatggtaagaggtattcaaaatcgaatctggtattgcccggcagatctttcaaaataccggtaaccgtgaagttatctttattctcaattttaatgatcttacccatggcatcttcactgccaaataaacttttagccgttttctccgtaagcaccaccgaatgcacatcattcagcgcggtagcaggatcacctttcagcatggggaagctgaacatctgaaaaaaaccggtatccaccaggatgccggactttattatttttttatcccctacggaaagaagatacgcattattggaacctaccctcaccgcacgttctacttcaggcaaatctttttccaccgcacgggctgttaatgcagataccgtattccagtaagagagcttcccatcaatgggtacgcgattccatacttcgtatatcctgtctttgttagcgtgaaacccatcgtaacttctttcatcctgtatccacaggagaataaggattgcagcagccatgcccacagcaaggcccgtaatattgatggctgaaaaacctttgttgcgcaacaggttccggcaaacgactttgaagaaatttctgatcataatgcattgatgattcccggactgcaacgtacaggatttgcgggaatcttaccccaagacaatgccggatacctatttgcttgatttacaacgatgtggctgcgtcataaataccggtttgttcatttttgggacaaaacatgtccgcttttgaacacccggataatactaaaaggccggaatcatcacttatgataatataatatcaaaattaggtaatcctgcatagtgtacttatctaaagaaggggtaacttggtttggtcattattatgagcagtcaaaaccacgattatacttctttttgggtaacaggggatctttcatcgtttaaacaaatgatgaaggcattcactccttccctgaagcattttgcgggtaatattgttggtaatgaggcagaagcagaagaaattgtggcagatgtatttatcaaaatatggcaacaaagactgctggcaactgcccctgacgacatccggtattatctttttaaggccgtcaaaaatacggcgctcaattatctgaaaagcaatgaccgccgcacgacgcaccataccgcctgggaaatccaggtgaaccgggtaacctccaaaaatcccgaagacattatgatcagtaaagaacagctgtcgcatatcaatgccgccatcagttccttacccctccgctgccgccagatattcattctcgtaaaagaagaaggactctcctatgaacaggtagccaccctgctggatctctccaaggctaccgtaaatgtacagatgaccatcgccctgaaaaaaatatgggcagcactgggttcctccatccaatattcttattcctgattttttttctacccggtttaattgttttccttttttgcgttgtcttaatagggaatcaactgaaatcatactttctgtaaatgaccaaacgattatgggaattactggcactgcattggagcggtgagatttcctcggaagaaaaaacggaactggacaagctcctgctggagcatccgggagattggctccgggcgggacagctggaccagctgtcttttaaaacaataccggccactgacgaggatgcgcatacggacgcgctgatagataaggtgatgggaactatcactgccgaaccggctttaaccgggaaaagctcccgcaaaaagttcctgcaggcctataaataccagttgtcagtagccgtagccatgctgggcataaccgccatgctcacctttatttacctgtatcagcaacatcccgggtataagatcgtgtccaccgatgccggtatgaaaacaaagatccggttatctgatggcagcattatctggctcaacgccggcagcactttaaagtacccggaaaaactggataaagccaaaagggaagtatacctcagcggggaagcatattttgatataaagcaggcgcctaaccgcccgtttatcatccacgcgcagaaaatggatatcagggtactgggtaccgcatttaacgtcaggtcctataaagaagaggattttgaagaaacatcggtgatttcaggggccgtagaagtgaccgtggcggatgaaaataaagtgctgaaggttacgcccaaccaaaaagtaattctccggaaaacaatcaacgatcctgcagaaaaaaatagcagcgccaccggaccaggtaataataaactaacaaaaattgaacgtcagccactatctgttctttcatcaacagatactattcatgtgatggaaactgcctggatgaataatcaactcatattccgtaacgagtcgctgcaggcgctttcacaacgactggaacgctggtatggcgtgaaaattatcatcgagaatgaacaactggccacattaagattttccggacgggcagataatatttctattgaaaagctgctggaggtactccagaatattcaaccattcaattattccattcaggatgatatagtgacaatcaagtaaaccagaagttatgaaaaatagtatcataattggggagcgacctccctagcggacccgctatgcccggaacttccgttacggacctccacagaatccagatttattgatttataagctcacttccaggttatgaaaatagcaataaaacaaaccacgttcgccttacattgcaatggacgaaaattatttctaatgatcaaatttaccggtgtattgttcctgctgtttttccaggccactgcagcagggttttcgcagaatacgatatccgtttccttcgttaacgcagatattgagaaagtattccgctatctcgagaaaaaaacgacctacacgttttattacagcaacaacgaaacagagaaaacacccaggctcagtctcaccatggaaaaagtggatatccgcgaggtactcgatgcggtagcgctcaaaaccggtcttcattataccatcctggataacagcatggtggtattcaaaaacgccggcgagcggatacaaaccaaaaagatcagcggaaaggtagtggatgaaaaaggccgtccgctgcccaacatgaccgtgcaggtaaaaggaaccaccatcggtacattaacaacgccggaagggttatttacgctccaggtaccggaaaacgcgatcctggtggtatctgccatcggttttctcaggcaggaagtacctgttgccggtcagtcttccttcaatattatcctgaaagaagatgtatcgggattaaatgaagtggtggtagtaggttacggcacacaggaaaaacataaactcaccagtgcggtggccaccatttccggcgcagagctgaacaaacgggtagccaccaacccggcatcgctgttacagggacaattacccggattgcaggtaacccagggctcaggcgaaccgggaaatgaaaatatacaattacgcattcgcggcatcagcacgttcagcggcgcaggtaacgacccgctcgttgtgatagatggtttaccgggaagcctgagcgctttaaatcctaacgacatcgaatctatctctgtgttgaaagatgccgcctccgccgccatttatggctcccgcggcgccaacggtgtaattgtggtgaaaacaaaaaaaggacgcagcggtttttcgctgacttacgggtataacctcggtgtttcgcaggcaaccaaactgccggagacgatttccaactcggcagaatacatgcaactgtccaacgaagcccgcactaattccggtctggcgccgctctatacccagcaacagattgatttataccaacaggccaccgaccgtgtgaaatatcctaatcacaactggctggatgatatctttcgcaccgcatatacccagaaccattacctgaacatgagcggagggaaagaaagtactacttacagtcttggtttgggtatcagcacccagccaggtgtactgatcggcttcgactacaaaaaatatacgttggacctgggcctcagctcccgcatcaataaaagggtgaccatcggtaccaatgtgcagatgcggtacgccgacaggaaatatcctgaaaacggtgcaggcgacatgtttctgtctgcactggcacagtcgcccctctaccctgcctccagcgatggaaaatggattaaaaaagcctactccaatgaactgggtaataaaaacccggtagccattgtagatgaagatatccgggtgaagacaaacgattactacgcacagggaaatctctccctcgatgtggacatcgtagacggattaaaatgggaaaacagggcaggcatgaattatggcaactacaaatacagtgatttcaggcccgttatacctacctattatttcagcgacatgagccctgccggattacttgatgatggcactccggggctgacagtgggcaataccggcaatatctacaccgtttattacagccagctgacctacaaaaataaattcggcgaccataacctttccgcactggcaggttatcagcaggagcaaaataaagccgataccctcaatgccagccgcacgcagtttcccaccaatttcctgagagaactgaatgcaggccccacagaaggccaggccaataacggtacctccggcacctgggcgatccgctctttttatggcaatgcgaattatgattataaagataaataccttttcggcgccagcgtaagatacgatggtacttcccggctgccttcagatacccgctggggattgttctattcattttccggtgcatggcgcgcttcagaagaatcttttatgaaaaatatttcctggataaacgatctgaagatacgcgcttcctggggacagctgggcaaccagaacatcggtacctatccttatcaatccacactcgataacagaccctatgctttcggttccagcgtttctaccgggtttaccggcagccagattatagatcctacccttacctgggaaactacccgcgtgctggatattggtcttaatctcaccgcgttcgataaccggcttacctttaccggcgactggttcaataaatacacctttgatatcctccgcagctcccaggtgcccctgtggctgggattagccgcacctattatcaataacggagcggtgagaaacaaaggatttgaattcaacgtgcaatacaacgataagatcggcaaaaactttacctggtatatcggcgctaatttccaacgttataaaaatgtattggaagaatttggcaaacgcgagatcagtggtactaccatccgggaagaaggacatcctttggatgaatactacctttaccagtgggatggtatcttccagagcacagatgaaattgccaaatcgcccaaacaacctgtagacgccacccccggcgacctcaaaattaaagatgtgaatggcgacggtgtgattgatgataaagaccgcacttatacaaacgggaaatatcctggtttccagtatgcattcaatcttggcgcttcgtggaaaaactttgatctgagcgcacaattctatgcctcacagggacaaaagatttatgtcaacggatggggaatagaaccattccggcagggttccgtacctacaacagactggcggaaccgctggacgccggacaaccccagcaccaccatgcctaaaatatatgttgccgacggatatgctcctgttcagaactatgcctccacttatttcctgaaggatgcttctttcctcagactcagaaatgtacagttgggctataacctgccggctgccaccatcgccaggataggcatgaaatcgctgcgggtgtttttcaccgctgaaaatgtatttacgatcagcaaatttccggggcttgatcccgagcgtgtaggagacggtaactatgttacttatccgcaaaccaaaacatacacgtttggcgccatggttcagttttaatttctctgttaaaagattcagttatgaaaaagtttcagcaattaatagtaacaatcaccactacggcctttatactgtgcagcggatgtaacaaggatctgctggatgtaacgcctccggataaactggcatcagcttttttctggaaaacacctgaggatgcggacaaggcgctcaccggcctgtacaactacctctacgccaacagcggaggctatgctacctcacagtttaccgttttcgcctgggataatttcaccgacgactcctacggccaatataattacggaggaggtttaaacgcccttacttccggcattactcctcaatccggcgattttgtgtactcttattacagtaactgctaccaggcgatagcggcagccaattctttcctggcgaacgtagataaagtgctcagcggcgaccagctaacaaaatataaagcagaagcctatttcctgcgggcatttaactacttctggctggcgcagctctatggcaacaccatcatctttacagatgatcctttcaaggaagactataaatccaccagggctaaatccgaccgggccgaagtattaaaattggtattggccgacctggatctggctatcgcttcgctgcctgatgccggctataccaatgggcacgccgtaaaagctaccgcccagggatacaaagtaagagtacttctttttcagaagcgctacgcagaagcggccgcactggccaaagaaattatgacgggcaacaagttcagtctccttgccagctatgccggcaacttttataagcccgatcagaacaacagcaaagaaattatgttctccgtaaaataccagcgccctaacatcctccaccaggatgtggctatttctgtaaacctccagcgctggaaaggagaacaaggcacgcaggacctgatcaatgaatacgaagcagcagatggtaaagacaccgcctcctcggccgtatacgtgaaaggaaaaccgtttgaaaaccgcgatccgcgcatgcgcctgacgttcttcttccccggcgacaccaaagcacagggatggcccttcaccggcgccctggcaattgccacgcccggaaaagacagctggacggccggttactatgctgtaaaaaaatggctggaccccagtctcactgaccccgactacggcactatagacgacaacgactttgtactgctccgctatgccgatatcctgcttatgtatgcagaagcgcagaatgaagccaccgggccggacgcctccgtatatgccgctatcaagctagtcagaaaccggagcaatatgccagacctgccagccgggttatcccaggcagccatgcgcgaccggatccgtcatgaaagacgggtggaatttgcgctggaaggcatccggtatttcgacctgagacgctggggcattgcggtgcaaaaactggatggttttgtacctaatcctttgcaaccaactatcaaaactaaatacaaggccaattatgacttctggcctattccgcaaacggagatagaccggaatgcgccggaactgattcaaaacgatgggtattaaggtctttatataaaaagaaaaagccccggaataatttccggggcttttctttttagcatctcctgaatttgacacgcgcatctcgttgccaatgtttatttttgaagtcactggtaaattattaacggcccctgtaaagcgggcctccgtttaaattaacgaaaagccatttttaatatgagcagtgcaaaaccgcatgaatcacagaacgtcaccgactaccccaacaataacaccatattcgcggtctggaagtttaaggagggaacggaaattaaacctgctttcgaaaagctctgcgccctggtagctaatctcaatcacaccttcatcatacgggcgcccggtggccgcgccacctgcgtaatgggtgttggttacgaggcatggctgaagctatctttaccccaacctgttccgaaggaattaagaaattttgaaccgctggtgggcgcaaaacataccgctgttgccacccccggagatctgcattttcacttacggtcaaccgacatgtccatctgctttgatatgctcattgccataacagccgtattatcacccgtggcagattgtttggaagaagtacatggtttcaggtattgggatggccgttctattcttggctttgtagatggtacggaaaatcccgtgggtaacgaccggcagtatttcgcgctggtgggtgatgaagatcctgtttataaaggaggcagctacctttttgttcagaagtacctgcacaatatgggcggctggacaaagctcactaccgaagaacaggaaaaagtaattggccgttataagatcagtgacattgagatgcctgacgacataaaacccgataattcccatagcgcattagcgaacctggatgatgacaatggtaatgaactgaaaatagtaagggataatatggcctttggaaatcccggcaaaaatgaggtgggcacctatttcattgcttatgcaaatacgttcagcaccacctttaaaatgctggaacggatgtttatcggggtgccggccggcaactacgacaggatccttgatttcagtactgcccataccggaagcctcttctttgccccgtcaatggatattttaaagcaatatactgcggatgacacggcgtgattttatctgttaaccggcatgcagctgaagtgtataatctacctccggagaccgttgttcctggcactgaaaaataaagtgttaaattgacaattataattataattttcttattttcacccttcggtagtcatcttccacattagtcatcaccacgtagagatttaacatgatgcgattaacagcggttatcatccttgccacgatattattcgggcagcatgcacaaagccaggactttcataaatgggcgcccggcccgccaatgggctggaacagctgggattgctatggccccacggtaacggaggcggaggtaaaagccaacaccgactacatggccaaatacttaaaatcatctggttgggaatatattatagtggacatcaggtggtatgtcagcaacgataaatcgcatggctataatgaaacagatcctgaatataatatggatcaatacggaagatttgttccggcagtaaaccgctttccatctgccaaaaacggccagggatttaagccgctggccgactatattcacagcaaaggattaaagtttggtattcatattatgaggggaataccagtgaaagcggtaatggaaaatacgcccgtgaaaggtaccacagtaaaagcagctgatatccactcaaaagaggggcagtgcctctggctgcacgatatgtataccgttgtccctgaaaaagaaggcgcacaggcgtattacaattccctttttgaaatgtatgctgattggggactggactttgtaaaagtagatgacctgtcttcccctatttattttgcgggtgaaatagaaatgatccggaaagcaatagaccgcaccggacggaaaatagtgttgagcacatcccccggcgaaacgccaattgaacacgcagcgcatgttcagcaatacgccaatatgtggcgcacagtaggcgacttctgggacaactggaaacaattaaaggaacactttaaagtatttgagcgctggaataaatggagagcgcccggcgcttatcccgatggcgacatgctcccactaggccgcattgggatacgtgcggaacgtggacatccgcgtatgagcgggtttacaaaagatgagcaatacaccctgatgacattgtggacgatttttaaatcgccgctaatgtttggtggtaatctgccagacaatgatccttttaccttgtccctgctcaccaataaaaacgtactgaaagtactaaacacaagcactaacaaccgtccgctttttacggaagaagataaagctgcctggatggccgaagatccggcaactggcgccaaatacctcgccgtatttaataccgcggaccatccttcaacgcaggccatgcctgttactgttgatctgagtacactgggaattaccggctcctgcaagattaccgacctttggtccggtaaaaaagcaggcactttttccggtactttttcaccggttattgccagtcacggtgcagggttgtatcgtattgaggagaaaaaatagtgttgcagatccggccggctgtcttgtcaattcagattcctgaactcgtttggtgttataccggttttttgcttaaataaccgcgtaaaatgctgctgatacttaaatcctaactgaagggatatatcattaattgcgttgttcgcatcaaacagccggccattggcttcttcaattaccagccatatctcatatcaccgcatttgatatttcagaaaaactgcgtataccccatgtatcccctgaaatttaacaaaacctcttcccgccaccatcccgctaaaagtaaatcagtaaaactggtaaataaaacggtattttatataaagcaattcaatggctggtaacgacatttgtaatatgaatgactttagcagttaacacaataagctgaaattaatatactgattatgaattatatagatatttcagaaagacgctgtaacaccggcatctttctacaaataataattctttttgttttcatactaagtacaacgaacatgaacgcgcaacaacgcaatttaaccggtcaggaattaacggttcagcagcaaagcctggtagctgtttccgctttaactgccactggtgatttaaaaggattaaaagagcagctgaacgccggattagatgccgggctaacgattaacgaaatcaaggaggcattggtacagctttacgcctattgcggatttccacgaagtttgaacgggatatccacgttcatgactgtgctggaagatagaaaaacgaagggcattagtgacaaacaaggaaaggaaattgttttaaccagcgatagcaacaccaaatatgaacagggccggaaagtgctggaaacgctgacccaaatgccgcaagcaaggccggcgccagggtttggtgagtttgcgccacgcatcgacgcatttttgaaagagcatctttttgcggatgttttcgacagtgatgtgctgacctaccagcaaagggaactggtcaccattgctgccctggcggcaatgcagggagtggagccgcagttgcagtcgcatataaagatgggaatgaacaccggtatcacaaccggacaattagcacaagtagccggcctgatagaaaaaagcgtggggaggaaccaggcaaattcgttgcgaaagctcttgtcggagccagctattccggtaattgaaccggatatgatggtgcggatttcagaaattgaaattgtgccggaatacctggaagaatatacctccattctgaaaacggaagcagcggcatcggtaaaaatagaaccgggcgtaattgctatcttccccatgttccagcagttaaatccaacacaactcaggattatagagatatatgccaacaaagcggcctaccggtctcatttacaaacaccccacttccagcattacaaaaccagtacgcttaagatggtaaaatcactaaaattggtggatatggagagcattgataaagaaacaataccggagatctttagaaaaataaaatgagcaaattaatttaagaacagcagcggcctcctttctccttatctccgtactcatcatgacggcggaaccacatggtattcccggtttcattgcggcccagcggcgcccggtccagccattggtacatgccccaaagcccgtccagtccgcgctcatatgttgagtacgtgtggtaaaccaccccatccctcaacacaaaggcgctcataccgggcgcctcacgggtatacgtagcccaatctgtgcctacggtcgcagcaatccgttttccggcttccggcgcttcctgaaatgcttcaatttcattggcacgggaggtcacgttccctgtgcgatagttgtacgctacggcgcccgaacgttgctgctccgctgtgaatgacaccttgaaatcgtagttgaaatcactttccagggacgaggcccagggaaaatgccagcccatccgctgcttgtacacatgcaacttcgccagcggagcccgcgacacagcagtgagcatcacgtcgtggttagccaggtgaactgcgaaaccattaaaatcgtctgcaatcgacgagcacgacgggcacccggcctcatactccggcccaaacatgaaatgataaataagcagttgtgaccgcccgcaaaagagatcagcgagcgaggctttcccattatctgtatcaaagctatacgctttgtctaccttcacccacggcaactcctgacggcgccgcgctaccttatcactatgcctcgtaagctccttttcggcctttagcagttcgatccgggctttcagccattcttcttccgaaaccacgggatggtttttaatattgggctccataacgtttttatttatttaaaatatactaactcttatcacgtggcttttgttcagggtagtagctatttggtatcgtatgctttacaggcatcttacctcttttcctgaaataaacaccctcgctttgccaccagccttcaccagtacttttggccaacggaggaaggccgtataacccataggttgctttgcttccaggctggtttccgacataacggtcacactggcatcataagccgttggattgtgtaacaggatcaccagtcctttattatctttcttaataactgtcgcctccacgtggtcaaaaacatagcattttgatttgtcgctgatcacataaatccccggtagttcaagtgccatcagcattccgttggtttctgtccaggaattgcgggtgtatataaaattcccggtgctctccttcccttctgcatctcctggctgaatgcgctccatggaggatcccaccaggtaattgctggtaatatggcctggcatattaaccgcctccgtgtgtgcgtgctggatatccctgatcaaatctgcatacaatgattttccggtggcccggaacaatttaaaaagatagtcgccggaggaagtgcagatgcccggtgcggcatgtttattttgaatgctggcccaaacagcccccgtcatattggcctgtaatttcccgatggtactcgacggaggaaaaaccggtgcataagacagggtccagctggagcagagggctgcctgtacttcggccatcgacagccacttgtgatctccggtatatttatataatgccattaaagactccaggaatccaaaagccgattctgaattggcatcctgcgaaatatccccgcaatcgccacctgtaagcccctgccctgctacatcgcggcggtaataataatccgcagatgctgctgctgtttgcagccagtcggccctgttaaaatagttcgctgccagggccagcccagccgggacgatggcgcccgcagtagagttaaatactgccacctctcctgtttcaggcgctatatactggccaaactgaccatgcttctgccaggtttttacaaatgcgccagccagtctttttgctgcctcttcccaatctttgtttatcatggcagcatgcccgctttccctgaacaacaacagatgcttcatcaaccaaaacaaggcatccccgttcttccgcaccattgcctgcacttccgggaaatcccgtgacatcttctctcctgtgatttctccgtttgcttttatgccgccgtaaaaatagccgcttttaccctgcaatctgtgaactacaaaatcaagttcctcacagactcttttgcgttccttttcgtcgttcagcgatagcatcggataggtgttgatcatgccgctcacccatcccagctgaaaatcgttgctgttctccggtttataataattgccggcctgctgctgcgtaaaattactgctgcatatgcctgttcccagttccagtaacttgctcatcggtaccaggttccggggagcagcatggtccgggatatcttttcttacttttaaaaatttagtgagcaaagccgggatatctggcgccttaaacacatacaaccggaaacgcagcgatacttcgtcgccggccttccagtccggcgccttatcaccgctcaggtgaaagtcgccgaagccggcagccagcttacgcatggcgggtgctgataggtcaaaagaaaaatggtctttatgagcactctcggtgatggtaaccccgttgtttccccattttgtttgttgcgttgttaataggataaagcccctttgttcagccggagaaaaaaaacaaacggcgggggtggccatactacctgtttgcaattctaccagggaagcctgatcattttctatcgacaaacggggattatttgaaatcgttagcggcacctgcgggttataatacatatcacgcggatagtcgggattataaccattccctatagcgcgatagcggttgccgttataaagcgaagccggcaccagtacataattggcggggctccagttgctgaagtcaaatttcatcgctacggttgcagcgtttacctgtccggctgtcagcctgaaagttgccaccacatcaattgcatcgctgcattccttcaccgggctcactttcagcgccagttgccagttatccggcgcctctttcaaacgaaaaacgttttctgccaccaggttggtgccattatattgtctttgcaaaaaagcaaccgatccatatacctgttgcagcatcctgttgacctgcggatcccggaactgcgaaaaagtgctgtttgatatgacaacggccaccaggaacaataggaaatactttattttaatgcgatacatacttgctgtttaatgcagctaaaggtctgattccctttatatgaacccaacccttaatttgacaattacggctactatttttgccgcctttaacttcccgcgtattttattatctttggattgcctgtaacacacaaccagacctacaatccgatgcaatacatatacgagaattttacgtttccgccggaccagtcatttacggtaaggtcagagattcttgaaataaaaaagtatactgccttaaaatcgcatgttaattttgaaattgcgctgctggaaaactgtagtggcaaacggtttatcggcgatcatattcaggatttcgacgggccggagctggtattgctgggcagttacctgccacattgctggcaatattacaaggcggcagatccgcttatccccacccaggcggtggttattcatttctttcctgatttcctcggaaaggagctgcttgaaaagccggaagcaaaacaattgaacctgcttttcgccaaggcggcaaaaggcgtactatttacaggcaacaccctccgcgatgccaaaatgatcatgcaccagatgctctatgtgtcgggcttaagcagggtggcactgatgatccgcctgctggacgtgctcgcacaatccgaatcatcagtagtattatcatctccttactacaacaccgttgaaagctccggagaagcaaaaaaaatcaacaaagtattcgattacatctttcaaaatttcaaagacgacatcgtactacaggacgtagcagatcttattcccatgtcgtcggcagctttctgccgcttttttaaacgcaacaccaaccgtacgctgatcgactttgtaaaggaagtacgcatcgggcattccgccaaacttttactggaaggacatcacaacgtagcagaagcctgttataatagtggctataataacatctcaaattttaataaacactttaaggaaatcaaaggattgtcgcccagggactttgtcaggcaatacgaagacaaagagaaaaatggcattagcgccaaaagcctttaatcactcttttgtgaaccggtaaaaaggtaatgcctccacccatttttcatgctgcccggcgccggcaacgccggtctgataaccatccattaaccggttccattccgcacaacgcttatcataagattcagccgtttttcccatttgcccaagatctgctccggcaggcacactgatggtcattaccaacaggtagtcgtaccggtaaagcgttattttccggtagcctgctttcttaaagcctgcttccacttccggccatatatgctgatgatagtcgagataggctttcagcttctgcggatcatgtacaatattcaccacaaatacatgctcctgcagctccgcttcttttggggatgcattacaggctgtaaatataactacggcagtcaacagtaatatcctgcacaaaacagcgggtaatattttattcatgattcgttagtttaatactatatagatcgtgatcattattaaagccagtgctccccagcctgcccatagccatttatccatgcccgagccggcgttatccggaaaggtaaatgatacgtgatttttttcgggcgacttaaaaaccatcgttatcacccccattaaaatcaccaggaaaataaagatatagacagacagtagcaggaaatgcggccagaatcctttatacggatagttcaatacgtaacaaacgcccattaccaggcaaagaaatccgccgccaaacaatactgtttctgctcccacccggtgggtacgtttccagaatatgccggctaaaaaaacaaccgatagtggtggcgccagtatagacacaagtccctgtgttaattcaaacaggcttttatcagaataagaaaataatacagcgatacctcctcccaaaaaagcgcctgcggcggtcatccatctccccacccttgttttatccttttctttcaacgttacaaactgcgtaaccacatccaatgtaaaaacagtactgaaagaattcagccctgaagaaacggtatcgatcagggaagcaataagggccgctatacagagtccgcgaagcccggcgggcatcaggtttttgacgagcgtaatgtaagatttatccggcgtggtagtatctctgtataataaaaaacaaataataccaggcaatacaaaaataaatggcgtaatcactttgagcgccgccaggaaaagaatgccgcgttgtccctctttgacagtcttagccgccaacaccttttgcacgatcgtctgatctgcacaccagtagtaaacggctactacaggataccctgccacaatagcgagccaggaatattcgggatcggacctggcatgaaacaacttccaatagtcggcagggattgctttggccgcatcttccacatgaccaattttccctatagccaataccgttagtatcagggaagaaacaataatgatcaccgactggaaaacgccggtccttactactgcctttagccccccgatagcagtatagctggtggaaatgagggttgtcaacactactgcttccagcagggaacattggaaaatttcagagataaccaggccacccgcatacagtgcactgccaagccatacaaacaatatagacaccaggctgtaaactaccaggaaattataggacctgcggccataacgtaaaagcaggaattgcggaatagtgctgatccctgacgaaatataacgtggaataaaaaatacagacaacaacatcagaaatatccatgccagccactcaaaattgcctcccaccaccccctgcgaaaaacccaggctggataagcctatcaacatcatcgggcctacgttggcactgaacatggaaaagccgatctgccaccatttcaaagaacgcctgcctaaaaaaatatctccacccgattgtgaccgggaagatttaaggtaaaaaccaaaggcgaataaagcgattacatagacgacaaggacgagataatcaattccagttaatattatcttcacagaaaatgcttaaggatcacaaagatacgatcggcttgtattcaccgacgttctttttatcccatatccttgtcctggtcagttgaccggtgctttcacagtggccccaatttatcctgacaggcaaaccaggcatctccggcaggaaaaacttcccgttgctccatgccggttttacatcgaaatacgtttccagtcccgacataattgaatacaagtactccacttcacatggttcagacgcagtagccatcagggaagctgtaaacaatgaatatccgccggaagaaaaatcaatcttatgtttggctgccaggtctctcaccgccatccattctttcacgccggctaaatgaccgggcaccggctgcaaatggcttacgccgatgcttaccaacgtaggaaaaactcttgccgtccgttccgattctccaaaagctattttcaaaggcgtttgtttacacagcgcttcaatctggtcaaaagatgctgaatgcgtaggttcttcaaaccaggccaggttttccccggctgtctgatctataaaccggagcgcctgatcacaactccagatctggttggcatccacggcgagcctgacattttttcccaggagattacgtacaaacttcacacgctttacatcttccttcatgttcatgccaaaatccttacccaccttcatcttataacaatctacccctgctgtggtaaaataggtaacctctttttccagttgctcataactatagttggtgcctcctccgctgccatatacctttacctcattccggccggcgcccatatatttatgcaatgggacgccgagccggcgggtagccaggtcgtgcaatgccatatccacctgtcccaacagcgcagatgcagggcctctgaagccctcgttgcggatagaccagtataacctggaatataactggctgtaggaaaggttattggaatacagcaaatgaggcacgaggcatgcttccaggatattggtataactgctgtacaccggtgcttcaccaatattgtgattttcatcttcaatggtgatcatggacattccaaaagcatgaaacggtcccatagtggcgtcctgcaatggagtaaccacctgcaccggggctaattcccttatttgtatactccggatattaaagatctcgtgatcgatattacacatcttaacttcttttaccgttactgcaattcaaaatttctgtccggatggcgtccggtagtttaccctggttaaaattttcaatactggccaccagttccgctgtattggatggtcccaatacaatattaaaatcatagggtaaagacaggaggaacctatgcgccatagctgatagggaaagacggtgtttttccgctatttgttccagttctatggccatcttcagtgcctcttcgggcagccattcggggcgcatctgcttaaacgaccctatacatcgccccagcagtcccatgttcagcggactggcagcataatattgtatgttacgggataggcagtaaggcagtgaatccccgagtgaggttacatttgaggcattaagacggttaaactccatcaccacatcaaaaacgccggcatccaggtatgctttcagccaggaaggccaattacctcctacgcctaaccgttttgccaatccctgttccctgaacgctatcagcctgttaatgatccgcttcgcgtccatttcgggaatcgcatgaggatcatgtaaaaacaggatatcgagagaagagataccgatagtacggagactgttctccaggctttccgccattgtcctgtctgaataatcgtaacaggcttcgtcggcggcgtaagatttgagtcgccccactttggaactgatcacaggtgttttcccatcccattgctgtaatgcctgaccaagatagcgctccgcatctccataagccggagcggtatcaatagcgattatacccgattcgagtgcggataaaattgttaatacagattgatgtggatcaacctttccccaaacaccgcctaatccggcagtaccaagcaccaaacgttcgctgaccataaacaaataagtaaaataaactgttatcaacctgccttgctgcgcttcaatatttccgggctgcccaaaacaccatctggcgctaccttgtaaagtttccaggtattatcatccaattgttccaggtgataaacatttttttcttcctgcatttcttttttcaatgcgtctccaaatgcaccggcattctttgcgttttcccaggtccggaaagttttgaatatcgcctgcttgtcggttcttttctctacagcatcctggcttaaccccagcatataggtagcctcccaggcaatggatttacactggagattctctactacctgtatcgtccagtcacgctgcagattctgtatcccaaaagtagcgggaaaataactgccgttgaaagaataacgtatgtctttcccttcaattccccatttattatttaccggatcaaacatattattaccaccccctacattgcatacgctcatgtagtgccagtttccttcaaaaacgcaggatcccatcactctcacgtacggcacattcatttctttaaggtggtcaaacatgcctctcataaaacgtttgaaagagtattgtccatgtccctggtaagtaaaactttcgaagccgtcaaagtcgatatagttcatccctccgtcgtgcagcaggcgggcgtaataggccgcataatcatcctgcagcgtaatatcggggataaatccaccataacagtttacctggagtttggccagttgatccccggcgttatgcgcggcggcattggttttgagggcgccgcgttctacaccggcaagtgtatagggtttggtggtggtaacgcctttataccggatcagctctttcccgatctttaacacattcaccttgttgtcgtcccaaccgccaaattcgttcagataactggtgtccgccacctgtatcaatgtatcatttgcactaatccttttggtgatatgggtttttaacacggtacacaagccatcgttaggcaccggatgcacatcgctgctaaatggctgaataaattccgtgagcgtatgcaaaccataggcaacgccttctttattggttaaggcggttaagtcactgatgggccgtttttgctggttgagcgtcacttttttatcaccccaccggttggccggattcgtataatattctcccaaaccctcatcctgaacagctttcagccccagctgcccggcataggaaaccaggctgtcgtgcggcccccaccaggcgatatccgtttgataattggacggatcttttacccactttccattccgggtaatatagggtaagccttcattttttacaatctgttcaattgtttgtagtcccagtgaatcagggcaggcataaaaggcgatggcagaaccgatatagtctacatcaaccggcgtcagctccatatgccggggcgatttaaccccggggaaatcattaaaatgcggataaaaaatggtgtacggcttcttccggtcgcgcgagtgtaatacgatagacgatccgaagtccggctccaggctggcgccattaccattcatataccggtaatactcttccgggtgagaataaaatgccacatcattaatgccatctccaccgatacggaaccgttggccttcctgtagatttgccggcagcgggtacttcaccgggtcaggcgaatgaatgatataacaggactgatacatatcgccattacagggcggaccgctggtagtattgtcgttaagcgccagtatgccaatggcaaaattttcacttcttactactgacagtatttcgccgatggttttggagatattggttttataaggtccccatattacattgtcaacgccatttcgtggtaacagcgacaacagttcaaaacgcaggtagtcttttttctggtcgatctttaacgtagcaattgtactgttgggataagtcagctttaactgtttcccctgtagttttgcactgaccggataaatattctttccttctttctccagcgccagtaaaggtgagcttagtccccggggattgtattccctgcttgtttgtttatccctgatactggtaataaatccgcttttattgatgctaacagacgaatacctggttgtaaacgctatgtgctgtgcgcctgcatgcctgttaaaacccaataatgtacaaattattattccggccgttaaatacttcctgttacgcttattttctttcattcaattgctattgcaggggatcaaagtcgccaccccagttattgttttgttttaacaatgggtttctatccaacactgctttaggaatgccataaatatagtactgatctttaatagctatatcaacagcatctgttggaataacagtagaagtaaatttactccacactgtgtttatatccgacatcgggcttacatccgattgtcctgttttcagcaatacggcgattccatgacgttgagtaaggcttctcaggtaaccaaacatcttccagcggcgcaggtcattcaaacgtttaccttcaaaacaaaactcaacaaaccgttctttttgatatgccttgcgtatgtcgggctgcaacacggctgtaataccataattaccggcgatgcctggcagcacgcctgcacgggtcctgatctgttttaacacgtccagcgctgcagcagtattacctgtttcattagcgcattctccgtaattcattaatacttcagcataacggatttcaacccagtcgacgcctgcattgtaaacagtgcctttgtcaagggttttatcaaccgcttttatacggtaaaaactggagttagaccataaaggatccagtgttattgcattgtgaacgccttccagcccggtaccaccgttataattcgttattgaggtaaaatacgtccacaggtaggttttactgtcacgcattccctttaaatattgattgggagctccgttgtaataaatattggcataaaaccggtcatccctgttaaaaaacagtgtatcgtagcttctcgattgtgattcccaggccgagccatccttcatgggaaaggcattcaccagttccagggaaggcctgtcgtaacctacatcatccttagaccaatccaggggaattaaaccgccctggaaataagtggcctgcgggtagttgaaccggtggaccattaccacttctttgtttagctcatcatcccatattttactgtaaggactatataaccctttaccacgtgcatccaggaattctttggccgctttattagcatcgaatgctttttgccaggtggcaacgcctcccaaaccattaaacaacgggctggcataaaacaataatactcttcctttaaaggcgagggccactcctttgtctatccggcccatgtcatcatctgtaaaagcgtcgggcagtaatgcgagggcgtcatctatatcttttaaaatctgcgttacacattctgaagttttattacggggtttctgcagtgtagttaaatcagaagtaggcagctgtgcttccaatatcagcggtacgccgccgtaggtgctcacgaggttctgataagcccaggccctccagaataacgcctgtcctttaattttatccttatccgcctggctgaaggtagctttatcgatattacccaacaaaatattgatagttcgaatattattataagtactaaaactgttttgtgagtcgaaggtagcggtgcccctgaaccattcatttgtctgtttctgataaggtacgccttcgtcggtgttgttgccgctgccgtaaggattgcctggcatcagcgctgaatagatctgatttaaataggcggtggcaatatttacatccgaccatacctggtccggaccaactgcagagagattcgttttgtcaagtactttattgcagctcacaaataaaaaaggaacgaaaaaaaggagtactgctatatttaacttatgcttcattttcttgttttttaatttgaacatgcttttctacaaccttatatcaattcctgcggtaaaagttctcatagttggataactcatgaattgagacacttcaggatcatacaatttaaatttgctgatattaaacaggtttgatcctgccaggaaaatcctggtatctttaatcgctaatttattcaatacgatatcaggcaatttatagttgatgttcaggtatttcatccgtaaaaagccgccattatatacgttgaatgtggaggtccatgtataaccggcagaatgaggatctccccatgggtacattttgggagtagaaccattaggattttcggtgctccaggaatcagcgtggtattgtggcacttttccgccaccgccgaaattcctgccccaggcgtcattgtaacttattttatatcctgtgaggccggaaaataatgcttctaccgtaaatcccttatacgacagtgaaagattcaatccgtaggccatgggggcattgtcggctccaaaataattgcccagcaccatttggtcgtagctatctaccttattatccggttttccatccgggccactcaaatcggccagcagcatatctcccaaggctggggctactccattaatggtataaccgcttggcagcttattcaaatcctcctgtgtgcgtattacacccaatgccttgtaaccatagctatacgccagcgttttcccgatggggttagcatagtcctgcgtattggctgccacatctctttttatagccttgttggtagcataggtgaacaccccttttacattgtagctgaagtttttgccgatgttattgctgaagccaagctctacttcaataccatgggaactaacttttccataattctcaggaggcaatgatgcgccaaactcgtaaggaatagccaggatccggctgcctaatatatcataggattgacgtttccagtaatcgaagctgaagcgtacatttctgaataccgttgcatctacaccgaagcctgcggaatttgatttttcccaggttaagttgctgttaggtaatccgccatatgccaggcgtgatgccggggtaccggaagcgccaaggaaataggtgcctccttgtataatatattgctccatccatctccatctgctgtttggatcatccttatccaggatatcattaccggtggtagcgtaagatgctcttaactttaagaaatcaactgcatggccaagtgttgatgcctggaaaaatccttcctttgaaatcacccaacctccggacaccgatggaaaccatccccagcgcttatccggtgcaaagttggtagaaccgtctctccgtacagatgcgctgaaaaggtatttggcatcatagtcgtaattaacccttccgatataggatagccttccaatctgaccttcgttaccacttgttgaccaatcggcgttgttggcgctggtatataaaaactgatctgtggcaacgagcggaaaattataccggtacatgctgaaataattcgagtagccctcgtattgctcgtaaacagccagtgcgccaatcgtatgttttccaaatgtacggtcgtaattaacctgtgcatttagctggtaagtattggatttattatattcattgcctaaatactgggtgccgggatcgccacttaaagtagtacccaccaattcattcgtataaatcaaaccattgggacctgttttcttaaaattgtacagtgtttgttttttggcaaaggtttttatatagctgttgtcgaagtttttgctgtaggtaccttttatgctcagtccttctaccgtgggtattttgtactcggcagtcaccaacgcatctatttgctggttgttgttacgccagtagcccccgtttctcatcatctctataggatttcccagccaaccggggttatttggtttaccatctatataaggcgttgcaaatacatcccagtacagcagcttgccccaaagattattcaggtcatcggaaccataatcataggtaaagttgaaacggttgcgggtaccataacttgttcccaggtttaaaccgagtgtaagattttttacgaggttggcctgcacgtttccacggagattgtatttcttgtaggatacctgtggcaggaatccatcttctttaatataagaacctccaatgtaggctctcagcttttcattaccgcctgaaacacttaatgcataacgttggctggaaggattggtataagcgtctttgtaatagttatcgccgttagggttattttgaagcacccagttaatttcctcatcgcttaaacctccgttcacggctttgcttaaattcaatccatctttaaccggcatatattccggcagtttacctacccgttgcgtgttataggtggcgttgaaatttataactgccgtaccactctttcctgtttttgttgttaccaggatagcgccgttagaagagcgggaaccgtaaatagctgcagaagaagcatctttcaaaatggtgatatccgccacttcattgggatccagcgcatcgaaactggttttatcccgcactacaccatcaattacatataacggttcaacggcactgttactaaaggaagagcgggccctcactttaacattggagccaataccaggtgtacccgtgggtgaactgataaaggtacccgacatacgtcctgccaatacatttgataaattggttgcaggaatgagctgtatatccttcgcgcttatggaggaaacagcagaagtcattttagcacgtttctgtgtgccataccctaccaccactacatctgtcagttccgtggcaacgggctgtagtatgatgttcaactgggaagtaccggcaactgcaaaggcagtacgaaatcccgtcatcgtaattttcagacggctgccgggaggtgtgtttatttcaaagcgaccctccggaccggacactgttccgttcctcaggttcccctcctggctgatagttgcgccggggagcggcgtgcccgtagagtcagtgacaacgcctttaacgctaatcttgctttgggaataaatatgcgtggattgcagtatcaggcacagcaacgcaatcgcccatagtaacgacttggtttggttcataaaaaaaattgtacaggtgacaaatttgtggaatagcaattcattgttcggttgatgacatctctagtctacctaaagatcttactatcccttgccatgtacaacgcttaatttgaccattacaaatgttatttttgcaggaggacaattacttgttatgtcaataaacaaaactcaactggccggtaaagtggaaaggtctatcaagacctttccacttgtaaactttaaccggcaaactgatacgccattgcaaactctttagcaaaaccgggaaatttccggcttcccgatactccgtactgatctttcttaaattcgtcgaacaatccttccctgatggcctttcccgcgttcacgataagattttcagcagcatcctgtgaaaacccgttctgaagcaggcccgccaacaaggcatcatcgggaaactccacccaatttaacggcttgtcaatcgcgctgcctaacatttcagctatgccgttgccatttcttatatcgctgataacatattcgatctgctgaccggaaaaagaaagtgaatgtaagaacgtgaaggctgcatctgcaatatctgccggatgtgtcatgagcagatcaaccattccgcccacattgtgcccgataatgccctggtgttttgcgggccctaaaccaccataaaaattggtatagaacatggcggggcgtaaatgaacaacgttcagcccgggaatgccattaagccgttgttccaggttgtagtaccttgataacggagcaatgcccgccaccgcaacaccaatgctgctcaggttgaccgcataccggatattgtgctgttcaatagcccggacataattctggtgtatctggtccgcaaattcataatagtccgggacggaaaaatcagggggcaccatggtatataccgcatccgcgtcttcgaacgaccgggaaacaaattccgcatccgttaaagagccggtcaatggtacggcgcccagcttttctatttcctttgccttcctggaatctgagcttatcacttttatttcgtgaccacttgccaccaatctttctatgagaacacgactgatatttcccagggaacctgttactgttgctttcattttttatttgttttaaaattcttgtacaaaactaaacttgtacttacctttatacaagtacttacccaatggtaagtatcaaataatatgacagcaataaaagaaacatcggtcatccaggaaaacaagagcaatgcgtttgtcgcttgcccggtaacctttgtaatggaaaagattggcggatattggaagcccatcatcctgttcagtcttctgccgggaaaaaagcgctacagcgagctgaaaagatcaataccggcagttacagaaaaggtgctgatacagcaccttaaacaattggaaaatgacgggttaatcttgcgggagccaagacccgttgtaccaccgtatgttacctacgaactgtcggcgtcaggcagggcattaagaccggtgctctatgcaatggcagaatgggctgttagccagggaggggaactatcgggtcagttttcaaagcaaatggcggactttccgccggagtgagaggaagtaatagctaattcaattcgtcttgaagacatgttgatactttaattagatcaggaattattcgaaataagcacgaccactgttccaaaatactttctaacattattttttctgcgcccagatataagcccgcctgcttgcatattccacctcatcatacgggcgcctctctatggcatcaatgatattaaaacccgtctcatgaagtaatgcaatgatatcatctgatttaaagaagaacaaatcaacatcaatttctttatcatgcgctttgtcaaaatggacaatctcctctcctgcgtgaaaggaaaataaaaaatctcctcccgttttcaataccctgtttatttcgtcgaaacacttccttacctggtcattattaaaatgtactatcgcataaaatgcaacggcacttgccagaaatcctgagggataagcgatatccaataagtctcctgtttcatatttaatatggggagaaagctcccgggcagtactaatcatcgccggcgacaagtcaatgccggtgacgtcgtgcatgccgttgtcgtacagaaattttgttgtttgcccgggtccacagccaaagtctgcacagggtcctttatctttgttaacagctgcaaattccttcaatagcaaccggtcaaaatgcttgtgagtcagttcgtcccagcgctgcgccgcatagtcgccggctacctggtcgtaacagtgcagtactttttcctgtgaattcatcttattcgtcgtttttcaatactaactgaatgttgccttttcctgctctaaccttttctatcgcttcgttcatttcagagaacggcataacctccaccgcgctctcaatgttatgctttattgcgaaatcaaacatgtctgtcatgtccttgcaactacctacataatttccaaaaatagttcgctgagcataatcgtatagcaagccaaggttaacgggttgcttttccaaaggcgcggctaccacgcaaaacttcccctgtggcgtaaggatcttcaaaaaatcattcagatcatattgtacatttagtgtcgagataataaaatcaaatttcttcccgatcgttgtaagattattggcgtttgagcttagtataaactccgctcccaactgattaatcatctcctttttttcaggagaatgagaaaatacatacacctggtgtcccattttatttaaaaactggatagccaggtaaccaagaccaccagcgcccaatacaccaacggtagaattggctggcaactgcgctcttgtaattcctgtatatacagcaaggccagatgatagcaatggaactgaattcaccgagtgaagtgccggcggaagtttatatgcgaacctgttatcaacaacaatatgctccgccaaaccaccatagcaatgcacaccaattactttttgccgctcacaaaattgttctttccctgctttgcaatactcacagtcaaaacaagcttcctgctgataaccgatcccaacgcgatctccaactttcaatgtagctacatttgccccggttgctgctacaattcccacaatttcatgcccaggaacaagtgggaatttcgtatcgccccaatcatcacttatgaactggatatctcctcttgcaatagcacaataaataattttgacgctcacctcattgtcaccaacatttctttcataaaaaaatggttccggttttccacctttccctttaattccatatgctttgattttcataaatagcccgatgagtttttataggttttggaccctcagtatctcttcgcggtccgggtccgtgaaaagaagttacgactattttttggaagattttcgggggaataaagctatttaatggtgatgttctcggaaagctggtaattaaaattcaatatttcgttcatctccgccatacggtcgaaattaccgctgaattgcgaccggtatacatccgcataaataaaaacatgggtctggcccacttttttgtatttgagacagaaaacagagcggatgatagctttcccgtctttaggatcatagtcaagctcatacccggttacactgtttgcatcttctttgaatataaccctgtcggggctttccagtttatagcccgccaggtcgaaatctgcagggtctgtagagagccagatagtgagttgctttagtccataattcttttggggatgtaccaggtcgtatattttagcgttcgtcgtaaatgtgccgattttgataggcccgaactgctgggttttaacatgtccggatactttgagttcaatcccgcgcgggatctctaaagtgataggatttcctttgtcgtcctgtataacctggtttttgaccggtaatttttcaacctgatgcaagataatctgtggggctgtgcttaattgatttttcagcgtattgattttcgccttcacttctttttgtcgggcaatctccttattgatatcctcttcaaattcttctttcgatatccgggaaaactccatgatggtgtttttggcgttggagatagtcgcattatccctgaatttaatctggaaaacatcatcgctgaaagcatgatcatacatttcataatactccctgtcagcgatatggagttgcgaaagctgtttaaaactccggatgtctatcttaaatgtggaaggcagctcaaaatacaggctatcaccttttctgatgaagtggaaattataatcaagcacttcctgcataccttcaaccgtcatccctgtaaaaggagttttgtcttcccggtagatcttagtcatttcccagtatgttgggctgttctgagattgacaacttaagttcatcaaaaagagggtgatcgctataatgatattcctattcttctggtatttctccgctggtttcatcttcctgttttttgtttttcaatttcctggcgatactgaaccattgtactgcctgttaatccgttgttctggttgctgacataaaagatataaacaaatcagaaagatccattccaaaggtttcattagccggtaagttaaattggccatctgctcgttattgattttcctggataaattatatccgtacttatcatagttacgccgtatcacccggtgtaaccccggagaaaaatcctgcaccatttcctcaaaggcatttgcgatcagcaactgccggttcacgataatcgttcttccattcctgttacccaaccggaggggcttcacgatttttggatctccggatactgcaactgtacacagataatgccccttatggtccaacaccggcggatgcatctgctgggaaagccgccaggtggtggtttctgtgaaagctttgatcaatgaatcggtatcctggccaaacaaagtaagcaccgctgtaataaccagcaataacggaagtatcaggataatagaccacaatgttaaattgctttttttcccaaggaaaatattcaatttgttcaggaacttattggaataaacacgttcattggccgtagccatgtgcgttctcactacctgaagtataagcaggacggcaatcaatatcgccactgccggtgcaaatacaaaaagataaacatgtccggatttgtcatacatatcgatgctggccgtattatgtttcgatacctgccataaaatcagcaaattgatcacgatacctgttaccaggaaacccagcgacagcactttggccagtggtggcaatttattgcctttcaaccacaacagcaacaaagaaatattgaaggcaataaagtaaaaggtcagggtgatgatgtgcttcccgcccagcggaatataacattgatcatcaaccgggtctatggcggtataatattcgttactgtggatcaggaaaccgatgaacagcgatatcagggaaaagacataaacgttcgccaggatgacctccggaacagtaatggctggtttgatccttttcaaagtaaatatggtgataccggttagtcctaaaaaaaagaggagtacacaaacaataatcatgtattatttcgattaatttttacctgttgccaatctgataatttcgtttatacttaccagttcttcgtctgtatgctgatgatttctttccgaatggttccggttagttaccaatccgattccctccctgtgcgtcaatatattcttttcttcttctttaaaaaccacatgcctgcagatgaacttcacgacctcctgcagttgttcttccgtaaacgccagtgatgtatttctcaactcctccaggatagcatgctcgatttctgacgtttccctgttacgcccgatggtaagcggaagcaggagtaaaaacagcggagaacgctcatatttatctttagctacaatttgtttgaactcctgccagcttaacaacgaaaggtgaaaatggccaccggtattgcccaggtagatgtcattaaaaaaataaaccgtgttgtaaggatgaaattctgcatagaaggtcacctggggattgatctgatgtacgtacgtataaccattccagggttcggtttcctgtccgtctttgcctgtcttgccgcttaactcttctatccaatcctctgacggcattccgggatgttccattatataatcagacaacatcatttccttttcctcatcaacagcaaatggaaattgtgtaagcagataaatacaaaaatccctgtttgataacgtcaactccatgcttcaattgtttttacgggtcagtctgatagtcaaatggcacgccttcgcatgctgattttgtgatgttacacaataggtgagaacaatagcatcactcatccatcccatctgcatcattccctgcagtcttcttactattcgctaccagtgcattcaggttattcacttcctccttcgtaaaataccgccagctgccctgtgccaggtctttcagcgtcatattcataatccgcgtccgcttcagcgccactacatcatatcccaatgcttcgcacatgcggcgtatctgccggttaagcccttgcgttaaaatgatccggaaacggttggcgccttcctgttgcacaaagcatttctgcgtcatcacaccaaggatgcgcacgccgttacgcatatttttgaggaactcaatgtctatgggtttgtcaacggtaacgatatattctttctcatgctggttgccggctctcaggattttatttacgatatcgccgtcgttggtgaggaatatcagtccttcagaacgtttatccagccgcccgatcgggaatatgcgggaggggaagttcacgtagtcgatgatattggttttatccttgaggtcagtggtacaggtaatccctttgggcttgttgagggcaatgtacacggtggccttcttctttttgagcggctcaccgtctacttctaccacgtcgccatccttaacgcgattgcctttggaggcgatgttgtcgttgatcgtcacacgcccttgttcaatatatttatcagcttcgcggcgactgcaaaagcccgtttcactgatgtatttgttaacgcttatatccatatcagcgcaaattacttaaaaccgggcaaactatgcacccctggcggctgacttttgaccacggcaaatccaatacggcccaataattctgctttgatgttaatcgctaagaatgtaacttgttaccggcaatctgtcccgctgcccggcttcctgacatgaaaagaatactatgcctgatcaccggtttcctgcttcttaaaagttccccggttacgggtcaaacgccattgccatacatactcaatggcgcagctacccagcgcacctgcaactgctatgtgctcacaccggaccagcaagccaccagcggcaccgtatggaataaaaataagatcaacctgaatcagtcgtttaattatgtatttgatgtaaacctgggttgtaaagatgcaaccggtgcagatggcattggcttcatcctgcaaaccaaaggcactaatctcggcgctaccggccagggcattggttttaaaggcatttcaccctcacttgggatcatcattgatacctggcagaacacggatgaaaatgaccctccttatgatcatattgccatacaaatgaacggcatcacagatcacaacgatcccaccggcaatctaaccgcaccggtaaccgtactggctaacagcgataatattgaagattgtaactggcaccttttccgcatccggtgggacgcggtggcgcaacacatggaaataagcgtggatgatgagctgcgccttacactcgacaaagacattgtaaatgatattttcagcggagatcccagcgtgttctggggctttgccggatctaccggcggcagcagcaataaacaggaattttgcgccgccctccgcccggaatttaatttcaatccccaacagatcttctgcgatggcactcccatccagttcagggataattccagttctttcgggtccgtcacccgttggtggtgggatttgggagatggaaccctttcgaccgcgcctctgccgcctgctcacgtttatcctgcggccggtcactacgaagtaaaactggtgattgaagataacagcggctgccggtctgatactttaaaagcccccttcaccgtaggtgcgtacccggtagtggacttcggccccgatcccctttgtctcaatgccaaaatgcagatggaagatcgtacgaccattaccgtaggatcactccaaaaatgggaatggaactggggcgatggcactacctccgccggtcagcagccaacggctccctacactacgcccggtacccgccagatacaactttcggtcacctcggcgcagggctgcggcagcagcgctactaaatctgtcctcgtcagcaacactccgcaggtaagcggcagaggcgaagacgtatgcctcggtgttcccaccagtcttgaaggcgttaacctcacgccggctacacctatcagtcagtggcactgggatctcggcaatggtaacaccctgcaacaacaacaaggcaccttccgctttgcagatacgggctactatcccttacggctatacgccatcagcagggatggctgcgtctctcctgaagtggaagtgcctgtcagggttacttccgtattcgcacaggcggggaaagatactatcgtagccagcggccagcccctgcaactacaggctgaatggctcaatccgcgtatccgctacgcctggtcgcccaccaccggcctcaatgacccctatatacccaatcccgttgccatactgcaaaaagatcagacctatcgtctcaccctcacctccccggaaggatgcacggatcaggatgaagtgaatgtaaaagtttatgaaggaccggaattctatgtacctaacgcatttacgcccaacaacgacgggcgcaacgatattttccgcgtcatcgccgcgggcgtacccaaactggatttcttctgtatatggaaccgctggggccaggagatattccgcagcgccgatctgccgggtggatgggacggcaactggcaggggcgccccgcccccgcagccacctatatatggatggtgcagggcgtggattacaccggccgccgtttcagcagaaaaggtacggtaacgcttatacgataactacacccggtaacaaatcgcattgatgttcatgcccgctcccacagaagcaaacaggatcacctcgccggcatgtaccgcctggttggcaatatgccccttacgtaccatgtcaaataacgtaggaaccgtggctacagaactgttgcccaactcgtggatattcataggcataatgtccaccggtatgtctttaataccgtataataagtagaaagctttgatgatggcaatatccatcttctcattggcctggtgtataaagatcttttttacatctgcaatgtttacgccacccgcatccaaacaggccttcatcgcttccggtacatgcttcagcgcaaactcatatactttgcggcccagcatcttgatataacggacactgttatccgcttccggtgcgtacgacttgcccatataaatataattgagctcgtccatcgcgtacgactgtgcactcgcactaataatccccgccgtgccctccgtatctttgaaagcctctacaatcaccgctcccgcaccatcgctgaaaatcatgctgtcacggtcgtagcggtcaatcaccctgctcagggtttcagtacctatcaccaggcacctcttcgccagccccgctttaaagaatgcatccgcctggattaaaccctggatccagcccggacaaccaaacaaaatatcgtaaggtatacaggaaggattacggatgcccaatgcctgcttcaccctggaagccagtgatggcaccgcatccgactgaatagtgcctgttaaaacgtttccgaaattatgcgccaggataatctgatccagcgtttccgggtccactcccgcatctttaatagccgctgttgccgctgctaccgccatctccgtggcgttcatatctacatctgcatacctgcgttcagaaatccccgtaacctcctcaaatttgcggataatgtctgccgcctcagaagggattctctcctgccggtcactgtagaattcctgttgcaaaaaatcgttatttagttttttgttggcaggaataaagctaccagtaccggttataactgttcgcattgtttgaaccatagatcgttttttaagttgccacctgacaacccattacataaagatacaataaaaagctgccctgcatacacccttccggccttcaccagcctgtaaacacaaatggcgctgtcaaaaacagcgccattattatttttgttcattacttaacttataaattatcagctattcccttcaataattcgtacgaccgaagccgtgtgtcctggtcgtaaatgtgagcggtagccatcagctcatctacctgcgtctcttcaagaaaacgctgcaggcctgtttgcacagtagcagcactgccaataaaagaacaactcagcatctgctgtgcatgcgccgcctcatattccgtccacaccccttccatactgtctattggcggtccaagcctccgcagcttaccacggataattcccaggaacaactggtaaaacgaagtggccagccggttggcttctgcatccgtatccgcggctatcacattcacacacgccatcgtataaggagccgataaaaattcagaaggcttaaattgctgccggtatatttttaatgctgcatgtagctgtgcgggtgcaaaatgactggcaaacgcatagggcaaacccattgcggcagccaggtaagcgctgtcggtgctggaacccagtatccagatcgggatatcaaggccctcgccaggtatcgccctcacggcactggtatggttgtcgaacgataaatactgttgtaattcctgtacctgctcagggaaatcatgaccagccccaagccggtcgcggcgcaatgcccgcgctgtaacctggtcggtacccggcgcccttccaagccccaggtctatccggtcgggatacagggaggccagagtgccaaactgctcggccactaccagcggcgcatgattaggcagcataataccacctgaacctacccggatcgtatgagtgccgccggctatatatcccagcaatacagccgtagccgaactggccacactcaccatattgtggtgctcagccatccagaaacgcttatatcccaacttttctacgtgttgtgccagccgcaggctattccggaatgcatctgcaggcgtacttccttctgttaccggtgccaggtccaaaaccgacaacggccgtcttaatccatgcttattcatgggtacaaatttacagcattgcggcccacggaaacggggcgatatactttaggtaagcacttccccccgttaagcatgctccagcatatggataaattcggccgaaaaacggtacgcatcgcccggccagcgggccgacaggtaattccggtcccgcactgtaaaaccccgctccggatgtcgcgcatcatccaggctcaaaggcaggggaccggaaaggaactgcgccggatcacccagcgccgctgtcacttccgcctgcacggtaaccggatacgtgagataatagtcctttaaccaccaccgggtaagatgatacgccatgcgctcctggctggccagtaaggccgtggttttataggaatgtaaaacggataaccctgttcgcggatctttgcttcgtgcagccagcaccacaccatgacaaatagccgccaccggcttctgcgccgtaaaaaaatgggctaccacctcctgtaacagggaagattcaatatacgccttcatcttcttgtcatgcccgccgggcagcaaaagggcgtcataatgttccgcacggatttgcgtatactttaaaggcgtacaaaaagattcactgttcgacatccggtgataggccatcaccgcatcctcacgcgcctgcagcaaccatttccatatacccagctgttctcccctcagtacccggagatccgccatcccgctgtaaccacccggcgtggcaaattgcacgtcgtatccctttgctgtcagcaacaaccaaggtattgccgcttccgtaggatcgaaaccataatcaggtagtggcaccagtaccttcttcattcaaaaatgtttaatgtgcaggcagtaacttgaaaagaaagataacaaaaaaagcattctgctgttagcaattgcctactttcagggtattatgatccgcgatatcgacatttggtatgaatcacagccggaaccggccaaaggctgtctgctggcgctacgcgcttatatccggcaatacaatccccatattacagaagcctggaagtaccgcatgcccttcttttgttacaatggtaaaatgtgctgttatctctggatccagaaagaaaataaacatccctatctcggcattgtggaaggtaaaaatatcccgcatccccagctgcaacaggataaacgcgcccgcatgaagatcctcccgctcaacccctcagaagatcttccgatggaagtgatcaatgatatcctcggcaaaatggttcgttggtacgaacaatcccgtaagtaaatgctgatgggaacaaattattttataaagatcaataacgacagtaatataagaacgacagtaatataagatagatgaccagcttggtgatccgccaccggttggtacggaaatgacgggggcgcgtaaaatcaacattgatacgcttcataaaataatcgggcttcccctgccctatcacggttttaaacatgccccactctgtactgcaccgcagcaaggtcatgtaataggctactttcaattcccggtaacccataccggcagcccttatataattaatacccatgtcaattaacggaatagccgctaaaaagatcagccatttctgccagctgagaaacatgaaaaataaaggcgcgcaaagcaatgccagcaccattccttctacaggattaggaaacgcataccaggtaaactttttaaaccgcggcaacaacaacgccgtgcctacgccgtaacgctcaaagcgtttatagtgcggctgcccgtcgttccaccagggatgtgttacccttgcttcttttatacaaataaaacgtgcattattccgcaaacagatctgcgccggcagatccacatcttctccaccgccgcttttcggaaaaacggacgaaaaccgtaactcctgcatggcggcacggttatacatcatatttgccgttacgccccacataaattcttccttcctgttggcaatcgtaaaaatagtcgttaaccctgccgccatcaacgccctggtaaaagtattcatgggagccgggaaatctgttaacccaataaatccaatcgcctcccggtggccttcaatcgccttcacgtattgaaaaagtaaatcctgctccgccacaatatcatcatccagaaacaacatccactcgccactgcctgcattgatacccttattccggctttccgcagcacccaggttctccgggttaataaacaggtgaatcgccccctcccccgataaacggagtatttccttacccggctgcacctgcggattgtctaccaccacataataggtgaatttccagccaccaggtttcggcaaatggatcaggggtagcagatactgttcatccaaccggaaagaaggaatgataatatcaatcgaatttgaaaatgccaacatagggcgcgaagataaataacattttatttgctttcataatgcaaatgaaatatatatttgcagccattattttacgctgaaggattattataaatacgcaggttactatgctgataacgtatagggctaaacgaagtaaatttatctcccaaacaaaaaaaataaaatccccgcaatcagcttagtcactttactcctgagaaagacaacttccgctgtatgcataaaaaaaaggggtggcaagactacctcccctttaatattttaaccatatcctatgaaaaacctaatgcaaagatatattcatggtcgttagttgcctaccttatttcgtgaacgcataattattgcccgtgaatgcaacaaatcagccgttgttaaccggcagttaacaaaataataaaggtgttcccaacgcttccattagttgcccaaagttttcagcgcgaggtaagacatcaggccagcaccggtttccagcgctttttcatcggcatcaaaggtggccgtatgcaaaccggatataatacccctgttttcattgcgtacccccaacctgtaaaaacaggcatccgccacctgtgaataggaagcaaaatcctctgccgccatccagatgtccaggtcctccacctgcgcttcacccaggtagtcaacggcgtatgccttgctggcagccgtcagtttatcttcgttgatcagcacaggatatcctctttctattttaatatcacaggagccttccatactttctgctatggagatggccatctttttaatcttatcatgggccgcactacgccaggtttcgtccagcgaccggaaagtaccctccagcttcacttcatccgggatcacattactggccccgttggcgtgcattttaccaaaagacaacaccgatggcagcaacgggttggcacggcggctcacaatctgctgcagcgctatcaccatatgacaggcaatcaccaccgggtcaatacccaggtgcggcatcgcaccatgaccgcctttccctttcaccgtaatggaaatttcatcattgctggccatatagcgcccggaacggaagcccaccttgcccaccggcagctccggcatcacatgctgccccaggatatgatgcggccggggattttccagtacccctgccttgatcatcaaactggccccaccggggattacctcttccgccggctggaatataaacttcaccgtaccggaaaactcgtccttcatccggctcaggatacccgccacgcccaacagggaagaagtatgcacatcatgcccgcaggcgtgcatcaccccctcgttctgcgaacggtaaggcacattattcagctcaatgatgggcagggcgtctatatccgcccgcaaggccaccaccttgtccgacggccctgcccctccctgcagtaaagcaacaatcccggtatcagccatcctttcaaatggaatatccagggcgcggagcttctcctcaataaaaagcgccgtctggtactcccggtaggaaagttctggattcgtatgcaggtggcgacggttggccgttgcctcctccagcagtccgctggctaattgccggattctttctttaagcatgtaacagtagtttttattacgctcctgcgccaggaacgtttttacgaaatcatcagtcaggttcggatacgcccgtcgtctcgccccttataaccctcaagtatacaattttttatccggtcgaagcgagcaaacgcctggccaccaacagcgcctgtgtggtggtataatatttcgccagcatcccctgcacttcccaggccggcatctgcccggatttcacgtataccaggaattgctgcatcactttggcaaataaccgttcatgcccctttaccaattcctccggtatcaccacttcccagccatacgcgctttcctttaacccgatgccgggatacttttgttccagcgtgcggaatgccgttttcatttgcacggtatctgctgataacggatggatatataacaccggtttgtactgttgttccttgtcctgcagtatcatcagctcggccttgctgccacgcagcagtgaataatgggtatcgccggtacctgcaggcgcttcataatcccactgaacggaaatacgcgcatgtaccccacgtatcgtataatcaaaggccccgttggcatacacctccagcaggccgccggcatcggcaatttcctccaggtcaggcgtaaactgctgctctcctgtaatggcgctgtactgcggcaggctcatcccggtggaccacgtaatggcggtatctatatgaatatcttttttataatccagtacctgcccgggaaaacaggtccactgcaccaggtctaccaggtgcgtggtcacatctgtaattccttctccctgctgctttacatccatataccaggatggccggatcagtgttttcccggctaccgtcttcttaaagtgatgtacgctttttttgatcacagcagggtccccgaagctgccctcctgcagtgttccaaacagttccggtaattgcaacagctccctttgtaacacgttatggatgtcgtaacgctctgtcatgatatcatacaactgcaccttgttcgcagcagccatcgcaaatgatgattgcagggaatcgaaaccctccacatcaatcgccataggtttgtcggccagcacatgcataccggcgcgcacggcatggctgatataggcaggcttcaaacggttattacctgccagcaccacaatactccccggatcacacagcagcatcttctgcagatagtcgctaccggcgtatacctccgtgcgccagcgcaccgccgggctgtactgctcattaaaggcagctatccggtgcaggtattgttttacttccggtccgtccggtgcatatacccggatcacgtcatctatttccgggtacatctgctgatgtaccagcgaagcgtggaaatgaccagggtcaagcgcaatcagctgcataggcgtttgcattttagatggatgaataaagataatattttgcttcatccggttattttttccgtttccgcatttccgttacaaagtcattatatttgatacatctccaaatatctaacacccaaatatacccgctatgagaattattttcgtactcccgttcctgttaatttcatttttcagctacagtcaaacggctaccattaaatccatcctgctggaccagctgcgtactacgcacgacaaggcccacgcacaatggtttgtaacagccaacaccgcagtagaaggactcacttccgaacaggccaattggaaagacagctccggtaaccactccattgcacaactggtaaaccatctcattttctgggacctggaactgctggagaaattcaaagggaaagaaaagtcagctttcaacggtaataacgacgaaaccttttcccccgcaacaccggcgcaatgggaagcttccgtgaagcggatcgacagtgtgctcaccgcctgggaaacggctattgagcaggccgatgaaaaaaaactcgcatcacaatacgctaccatcgccaatatcaacacacacaacgcctatcatattggccagattatttatatccgtaaattgcgtggcaactggaatcctgaaaaaggggtgaaataaaaatcagtaacctgtatttatgaagataaatcccaatagaaagggcctcgtgatcggggccttgtttaccgccatctcactgatgctggtcgccaccgtaatagcgcctgccctggcagtgcttcccggctacccggtggaaaaaatggtggcccgtatcgcaggcggcgtatcagatcatcacgttcaattgctcaccatcctggtactggcggtcatctttcttttaatattaatacccgctttaatactcatccgttcatccacccctcccaacgaggctattgtcagcgggaaaatcatcctcctgatggtactcctgtacatgattgtacatccccttgtcttctatatcttttcctatgcgaaagcatggaactccaaagatgcgcaatacctgatggccgctttggtaaccgttccgttcagcagctttgcctttgtgatcgtgggcgccgtcatcgacgccataaaaaaaagaaactagccgtaccggttgccacaaaaccttgtaaaaactcccggattcctttatattgagtccttatttccagcccaagccgccggaaataaggattttgcagcgtgtaagatttaaaataatgcagaccaattcccgttttattacaataaattccaatcaatggcagtgacaagaagagctgcgctcaagcagctgctgtatgtttcagccggtatggccatattgcctgcctgtttacaacataccagcagaacatcattaacattaaagaacatttcggtagacggcgaccaggaaaaaatgctggccgaactcgtggaaacaatcattcccgccaccaccacgccaggcgccaaagaactgtccgcccatctctttaccctcattatgatggacgactgctataaaaaggaagaccagcagaaatggctcagcggcatgaaagcatttgaacaggcctcccggaaattaaatgggcataccttcctggaaagcacgccggcacaacgcgagtccctccttagtgcctttgaggccgctaaagatgataaggacgatgccgcttttttttaccgcgctaccaaacgtcttaccattgaggcatacaccagctctaaatatttccttaccaaagtagatatctacgaactggtacccgcacgataccacggttgcgtaccgctgaaacccattacccggaagcttgcctaactattaattgtatgagtaaagataataccagcctgcaaaaccgtacgttcgatgccattgttattggctccggcatcagcggcggatgggcagcaaaagaattcacagaaaaaggtttaaaaacactggtgctggaaagaggccgtgatgtgaaacacttaaaagactatcccactaccagccagttcccctgggaatttccccaccgcggccaggtaccggaagccattcaggccgccaaccccgtaatcagccgctgctacgcctataaagaagatgccatgcatttctttgtgaaggataccgaccatccttatggtcaacccaaaccgttcgactggatcaggggataccaggtaggcggtaaatcactgatgtgggcccggcaaacacaacgctggagcgacttcgactttgaaggccccgcccgcgacggcttcgccaccgattggcctatccgctacaaagacattgccccctggtatagctacgtggaaaaatttgtaggcatctccggaaacaaagatggccttccccacctccccgatggagaattccttccaccactggagctttcctgcgtagagaattattttaaggactttgtaaaagataattataaagacaggcacgtgatctatgcccgttgcgcccacttaacgcaaccacagcagatccacctggaccagggcaggggacaatgccagaaaagggatctttgccagcgtggatgcccgtttggcggctatttcagcagcaactcctccactattccctgggcagaaaaaaccgggaaccttacactccgccctttttctgtagtgcattccatcatctacgatgaacaaaaaggaaaagccaccggcgtacgggtagtggataccaacaccaaagaaatgatggagtattacgcaaaagtaattttcgtaaacgccgctgccgtaaataccaacgcggtgctgctgaactccacctcccaccgcttcccgaatggcctcggcaacgatagcggcgtgctgggaaaatatttcgcctttcataattaccgcggtcatatcagcggacaatacgacggattcaaagactctaccaccgatggccgcagccctaccagcgcgtacctaccccgcttccgtaatgtacacaaacaggaaacagatttcctgcgtggctacgcagcaggcttctccaccggcagaggctcgcataccaataccaacggctttggtaaaacactgaaagaccagctctttaacagcgaaacgggcccctggtacgttggctcccacatgatgggcgaaaccatccccaaagaaatcagcaccgttacgctggacacccaaaagaaagatgaatggggcatcccgcaaatcaatatcaacgtagactacgacgataatgatgaaaaaatgctgaaggatttctttgaacagatgaccgaaatgtttaccaaagcaggttttaccaatatacataccggcgactccaaacaggcgcccggactggatattcacgaaatgggcggcgtacgtatgggcaacgatccgaaaacatccatgctgaataaatggaaccagatgcacgcatgtatcaacgtgtttgtaaccgatggcgcatgcatgacctctacctccacgcagaacccgtcgctcacctacatggcgctgacggcgagagcagtggattatgccgtgcagcaactgaagaagggagagatataaacaggtttgatattttttgaaaaccgggtgcagcattgcacccgcgtttttttatttaatttgcgcaaatgaaacctgttaatgaactgataaatacaaaagaaccaggctgggacctggtaaaggaatggatcaaagatggcaacaaccatatagaaattctccctaaagataacgcccgcgcagagcaggctttatatcaaacccaggtaaccacccgctccccgatgggcgccatcatctatgaaaccggcggactactcatagatcatggatggatacgggtactcggctccggtcataataaactggatcgtacattgcctgcctggaatgatggaaaatcgtatacgcattcaggtgagcaaccgggctttttattaatagcagatgatgtggtaggcggcttcttcgccatcaatgccggtggcattgccgcacaggaaggtattggcagcgtgttttactttgcccccgatacattggaatgggaaaatatggagatcagttacagcgattttatttccttctgctgctccggcgacattaatggtttctatgaagccttccgctggaaaggctggcgtgaagacatagcagccctgaacggcaaccaggcattcagctttgtgccattcctgtttacaaaagaaggaaaagacatggacaacgcgagtaaaaaagccgtgccggtggaggaactatggttcctgcaaatggatctgcaaaaacaattcgggcattaaatactacctgaaaaaccagtacagcactgccatcagcagcagcaacaccgtggataatactttgtaattggcaagacccggccacccttttacccgcaagggcgccaacgggctttcccagtaaaggcgattgctttcagcggtatgctgcacagggaatacaaatgacaataccacctgcagtaccacacaaaccacgaacaggtaaaaagccaccatcagcggcggtatgttaataggataaagtttacccgtaagatatacccccgctcccaacgccgatcctatccacaaagtatattgcgccgaaagggaagaggcttttttccagaacacccccaacaggaacacgcaggtgataggcggcgcaatatgcgatataacgtcgttaatgccgttaaaaaggctctcatacctgttcagtaatggtagtagcccgatggatagaaacagggctaaaaccgccgcaatacggcctgttttcacgagctgccggtcggttgcctgcggacggttccgcttgtacagatcataactcaccagcgtggcaatagaattcagcgcaccggaaatctggctcatcaggcccgacagtaatgccgctaccagcacacctaccagcccggtaggcaccagccgcgtaatcataacggaataaatgcctttcgtatgcagctgcccatccgcctgccgcaatacttccaggtccaggtgcccctgtttgaacagcacatacgccagcaacccggggagaatgaaaatgaaaacaggtaacacttttataaagccacaaaacaacgcgccagtacgtgcatgatgctcgtccttcgcacccagtacccgctgcacaatcgtttgatcggcacaccagtaccagatgccaataaccgggtaacccaggaataccgcataccagggcaatccattcggatcgcccgccgggtgcaacatcgacaatttatccatctggtggccttcctgcaatacctgcactaccggctgccagccgcctaccttccaccacgacaataccgtgatgatcactgcgccggccagtaacaccaccgtttgcacggactccgttaccaccaccgcccggagcccgcctacgatcgtgtacgcgcctgttaccagcgcaatgagaataatgctggtaaacatgtttatgccaaacaacgtttccagcacaatacctccggccaggaacgaaaacgcaatatgaatcacaatcgccgacactacagaaacaatcgccagccagtcgcgacacgccctgttgtaacgccgctccaggaaatccggcaatgtagccacccctgaacggatgtaaaacggaataaagaaaagagccagcaatatcaacgtaaaggcggccatccattcaaagttacccgccagcaaccctgtatcaaagccgctctgggcaagacttaccaggtgcaaacaggaaatattggtagcaaataaagccatgcctatcataggccagcgcaatgattttcctgccaggaaatattctcccgccgcggaatcattcttcttgccggataacccggcccagaagcccagccccacaataaaggccacatagcagatgctgatgataatatcggtagtagcgatcatccgggaaatgtattaagggaaagcagatcacaactgctgcccggtgtttcaggcgtctggtaaaagccgtctgtaataagtgccggatgaacaaaatgcttacgcaggtgcggtatatgctccaggaataacgcctcatgtcccatcccgatatgattgaacaatacaagatgctgatgcagctgtcccatatctcccacgtgcggcaccaccggcactccaaactttttacacaacaggcttaccgtaataaattcactcacaccccctacccttactgcatctacctgtataaacccggcactgcctgtttgcaggtaatttttgaagatcactttattgggtacatgttctcctaacgccagtttcacggggttcaatgcatccgccagcgttttatgcgcaaggatatcatccgggtgcgtgggctcctctatccagtaaggattaatatcggttagtcttttaccaatagcaattgcctgcggcagattccattgctgattggcatccaccatcactttgatctcatcgccaacggcatttcttacaatatgcgctcttcgtatatccgtttccgggtcttttgcccctacctttaatttcaatgcccggaagccattgtccaatgcacgtttgcaattcgcctccagctgatcatccggataattaaaccacccggcagaggtatcgtaggcgggataacccgtgcgcagcacgccttcccgcgcgcccctggaagcctgcatctccgttaacatccggatcgcttcttcgcgggacaatacttcttccaggtaggacaggtccagcgtgttcaccagctgttccggcgtaagatccagcaacaatttccataacggcacctgctgctgtttggcccacaggtcgtagcacgcattggttaccgcagcgagcgccaggtgcaccactcctttgtgagggcccagccagcggaattgctgctcatcggaacgttgtttaaaccaatcgccgaacgaagccatcacttccggcagttcctttcctacgagtttttcgccgtagaaccgcgcagcagcgcataccagctcgttacccgctcccagggtgaaagccaggccggtaccacaattacctttatcgtcgtataaacaggctaccgtgtacgagtatacgggattctgatgtatggcatcactgccggcgccacctgttaaagggaaccgggcatcttttacaactatcttactgatcattttatttttttcattttatgggtgcaacactcagcgccggcttatccgtttccaataccaccacgttgtcattggcatcgggtaatacagcaggcagtgttatcgtgaactgatcggcagctgtagtcagcttcactgcagcgcctttcagcaggtatgctttagtaattttcacacccggcatagccggaacttcaatggtttgctgtgccgcatcaaaaacatgcaggtatactttattgccactccgcgtagccgcatacttactgttgggattgtaaggaccgccatgcgtattataaatagcagcgccatacttacggagccaatcgcccatttccttcaaacgtgctacctgtgcaggttctatggcgccatcggagcggggacctacattgaataataagttgccgttaccaccggctacctttgccagtgtttgaatacaggtttgcagcgacttcattttatcatccggcttccaggcccattgctcacaaatggtcatacaggtttcccagggcgtgttcatgtccaggtcgccgatgcgctgctccggcgtatcaaaatcacccaggaaggtagcagtacccgatgcaccggtgccggaaaatgctttcccaaggcggttattaatgataagatctttcttcagcgttttgagataagcatatacatccagcgccatctccggcgtccacacactttcccagggaccatcaaaccacagcatataaggatcgtagccctctaccagttctttcagctggtgcttcatatacaccacatactgatccatgcgtgcgtttttacgtatacccttccccgttgtatcatcggggttgtctatcgggtattccggatggtgccagtcgatcaccgagtaataaatacagaactttacattatacttcttgcatgcttttgccagcagccctactacatctttcttaaacggggtagcggtaatattatagtcggtataggcagatggccataaacagaagccatcatgatgcttggcagtaatggtcaggtatttcatacctgcctcgctggccgtttttacccattcctctgcattaaatttcacgggattaaactggcggtacaaggtgtcataatctgcagccggcaccttgctatggcgcgaccagcctatttccgtaccccgcagggttacaggtccccagtggataaacaggccaaagcgcaggtccataaactggtccataacttttttgctggtcagtatcttgggatccagctgtgcatttgtctgggctttgccctggaatgccagcaacaacaaacagaaagtagctaattttttcattgttcactttattttataaggtatgcttatatccaagttctgccccgccgcttaccggcattatgcaaccggtaataaaccgcgcctgctcagataacaggaacgcacacacgtcggcgatctcatctgcttcagggcaatatcccaacgcgtggatgccatcaagatactgctctatacgcgccggctccggctgttcgctgctccaccggcgcaacattggcgtccatacgcctgccggggccactgcatttacccggatgccatctgcggcatagtcgagcgccattgctttggtaagggcattcaccgctcctttactgcccgcataggctgcgtggttttcctggccgatgtcccctaccatactgctggtgttaaggatgcagccacgggacgctttcagcgcagcaatgccataccgcgtggtatagtagataccccgcacatttacattcattacctgttcccattcttcgtcggtggtatcatgtaaaggtttcgagggactggcaatgcccgcattattgtgaatggcatgcagtacgccgaacgtttgtaatacgttgtgaatggccagctctatagcagcaccgctgttaagatctgcccggatgaaaatatgcggcgctcccatcaactccttcaaacgctgcaatgctgctgcgtctttatcaatcaccgctacagtcgcaccctgttttgcataaacctgcgcacaagtctctccaatgcccgatgcgccgccggtaatcagcactattttatcttgcagtatcatcatttttcattttccgtggataattcaaaagtaagcagggataaggtaggtcatcccggtgaaattgacttaaatcaacactattttgacttatttactgaatttacctattttagatggataatatgaagcctctttttgccataccgggcgataaagccctcgaacaaaaggtatacctgatcaaggaaattacgcaaccgtatttttccacggagtttcatttccatcacgaatgccagctggtatatgtagtggaaagcgccggccgccgtatcattggcgacaatatcagctactttgaaagcggggaactgatattcgtaggctccggtacccctcacgtatggcataatgaacaaaagtattttgaaggaaaagataaactgcaggcaaggtcgctggcattgtatatttcaccggacctgctggtagagcatcttagtccctttgccaataccagcaccgttaaaacctggctaaaaaaggcgcagcggggcatccagtttcatggcaaagctaaagcggaaatactggcattaatgcggcagatgctggaacagcaggatttgctgcaaaccatctcctttatgaccctgatgcaaaagatgatggccaccaaagaatataaactcctggccggcaccaactatgtaaacctgtacaacgataaagaccagtcgaggatggatgatatcttcaaatatattttccgtcacttcaaaagagatatcccgctatcggaaatagcggctgtagctggcatcaatgtgcactccttctgccgcttctttaaaagccgcacacagaaatcatttacccattttgtaaatgaactaagaatcggctacgcctgcagactgctgcaggaaaaagaaatgtcgatggtggaattgtccaataagtgcgggtacaggaataccacgcactttaaccgcttcttcaaaaaaattaaaggaaaaaccccgagagaatacaagagagaagttacttcgctggattaacttatttgttcaccaggaaatacaccacgcggcaaacagtagcatccccttctttttgcaaactaagtatatgcctgcccggcttcaggttatcgcccaatataaggtaccacggcaggtacaggtttttactccactgcgtgcgcagatccttttgctgaacagcaccgccatcgatacgatagctgattacacctgcatccggaccggaaacaatgctgatgccaatagtcctcccggtgaaaggatagtcaacactggcgcgcgccgtgtccgacacaagcatcggcactttcacaaatcccgggcgggtacctacgttatcagatggctcccaggaagcagtaatgcgaaagccattctgatgaacggcgtcatgaatatcgccataggcgccgttttcataattgagcggatccgcagcgcggggcagtttcacggataataaacgttccggcgccggtgcgctgaaatcttcttccagcaaacgttttatagcgttaaaatataactgctgaccaaaaggagcaggatgcaggtctttaaaatcatctttccaggtaaactcacgggcatcaatgcgggtcgtaatttctttggcaagattgataaacggcaggtggtattttttggcaagatcttcatgcacctgcacttctaccggcactttaccggcgtgatagtcggccatcttatcctcatcaacaaaagccatcagtacaatattcacctgcggattcgctttcagcgcatgacggatgatcccttccatagcacggcgctgcgttacttcattggtaccattcacccggtcgtttaccgccgcttccaggaatagcaggtcggtcttccccttgcccagcacatcttgttcaaaccggaatgcatgcggcaagctgcccagcgatggaacacctgcattgatgaaacggaaatcagttgccggatacgccgccgtaaggtagtcgcacaccttcgtacgccagccttccatattggtgatagaaccgcccaggaaagtaacggtagctcttttatctgttttgatgtgataccttacgttgtcaaggcgaccgtaacgtgtgataaatttatcctgcgcctgtatactaacggtaacgactatacttaatataaatcctgttattttcctgatcatattttcactggttgtatctcttttatgaccccgttgatctttacttttactttatgcgtggcggcgccgcggatcttgtaattggtaaccaggccgtttttccaggtcatatctaccgtataattaccgcgtgctttcagtcccgttaccgtaccggaagccttccacgcatcgggtaaagcaggcaacaggtctataaagccggcatgactttgcagcagcatttcagccagtcctgctgcaccgccgaagttaccatcaatctgaaatggaggacccgcggaaaacaggttggcataaatgccgccacccgcgccatagttaatgtctgtattataagtgggtttgatcagtcctgcaaacaatttaaacgcgcggttgccatcgtgcagtcttgcccaaaataataacttataggcaatggaccagctggggccgtcgtcgcctctcacttccagcgtttttttgcaggcttcggccagttccggcgtggcttccagtgtaatcagcgaagccgggtacaatccatacaaatgtgaaatgtgacggtgcgtgggttctgtctccttgtactcttccagccactccattaatcgtccgtctttccccaccctgcccgcaggcggcagctgttttaatttctctgtcagcgtgttggtaaaggccgcatccttcccgagtgtccgggcagcggtgatcacattcatgaacagctcgcggataatctggttatcaatagtaggaccgttgcagatactggcagtttggccgttgggcagataaaaagaattttcaggagaagaagagggcgaagtaacaagccatcctgttttatcatcttttatcagcatgctgctgtaaaattccgcagagcccttcaacaccgggtatatatcttccaggtattttttatcattggtaaaagtataatgctcccaaagattattacacaaccaccccgacccggatttggtaacaccccaggaagcgctttctcccggttccgtgaagccccatatattggtgatcacatgcgccacccatccttctgcattataataggctttggcagttctttcgccgggtttcaccaatccgtgtaccagctccgccagtggcaggttcagctccggcaggttgctcacttccaccggccagtggttcatctgcacatttacatcgaggtggtagtcaccattccagggcgtctggatctggttggcccacagcccctgtaaattaggtggcagcaaacctacgcgggtactgctgatgctcaggtaacggccatattggtaaaacaatacaggcaacccgttgtccgccgccggcgctttgtgaaaattgatgagccgctgatcggtaggcacctgctccgcactggcgccgcccaattccatgctaacgcggttgaataaacgctgaaaagcagcgatatgctgttgcttctgctgcccataacctttacgcatggccgcagccagcaattgtttggtttgttcccggtaaccggcatttctgaaatcggtcgcagtggatacatacaggatcacttctgtggcatcttttataaccagtgtatccctgtccgttagcagccggccatcttttaattttgcccgtaccctggtcaggtatttcataccagggttggcagtaccactttttaattcgccggacatttgcagctcctgcccttctgtgccgatggtggctctttccgggcgactgatagctacccgcatattcagctgtccgcctttaccagctgttaggcggatcacgcctacatcgccgttaaagtctgtaaaatattcgcgcgtataggcgaccccgttaatggtataagctgtagtggcaatggcctcattcaatgataaagccctttcataacgggcaggggtatccgctgcaggataactgaactgcagcgataactcgcccagcatctggaaacatccgaaaggcacatccccggagcctttgccggtacacacaaatgatttatccatcagcgcctgcgcctcgttattcttaccctcagccagcagctgccggatagcaggcagttgtttgtacgcctcgtaattgttggcgtcctggggcgcgccggaccagagcgtgatatcatttaaaacgatcttctcccgggcgataccgccgtccggcatcatacccaggcgtccattcccaagtggtaccgtttcctcccaaacctttgccggcttgttataccagagccgtaaaggccgctgctgcgcttcagcggttgatggccgaaaaccggccatcaacacgatgccggcaattacaatacgcctgaaagaaaaaagttgctgactcatgtttttcggataacgtttttgatgtagcaggctgtgtccccgcttgctattaataatctccgactgcggcagatcataggtatatgattcttccgtggaatttgtatgccatcaaaattaacggcaacggggtaaccgtgctccctgaaaattgactaaaacagacactatattgacttaatatagtatttacatactttcagacgggtaaaatgagtgcgttatttattcctcaccagcgcgcggatctttaaacaggtgggcatggtggaaaggtagccattggcggcaataaaagtgaagatgaaacccgtacgctttttatcgcggtttacccaggggtggctcccaaaggcgccggggctgctgttttcaattaatgccccacccggaccggttacatcccgccagttgccggtgccatagaaatcttttgtatttagcagtaccgcgggataaggggaataggtaacggtagcgtgggcagtctgactttcctccatcgctgttaccgctgcttcgctgagcacacgggcgccgtttgcagccacgcctttgttcatgatcatgtcgagaaagcggatatagtcgtccggtgtactccgggcgccgccgccaatctgcggattggcagtaagaccaaaatcagtattggtcatgccgcagggcgtaaatatcttatcggcagcgaggtccttccagcttttaccggatgccacttcacagatacggccggctacctgcatacttacgccgccataataaaaggtagtacccggcggattcaacagcgctacattccgcgctatcccatctgccgcctgtgtaagcgtaatcaatacattggattcatatccctgggaagaatttccggggaaaccggatgtatgggagaagagttgcgcaatggtgatatctcccttatgataagtagtaaaaacgggcaggtattttcccacactgtcagtgagctttatttttccttcgtccaccaggctcatgatcaccgccgcagataaccatttggaacaggaggcgataagctgcctggtactcccggtataacctccaaatcctttggcatataccgttttcccattttcatgaatcactgcataacacttaccggcgaaagccacaggcacagaatcgctcagcacctggtccacatcactgtaaccggtggcaataatggtttgggattcacttttggtgcatcctgccagtaagaaaataacggtaatagcggacagggagttccggaagaaatcattcatgtgacagttgtattcagttgtaagctaagaaataacgccaacttattcaacgtcctctttttaattatattgcggttgttatgaaatacagcaatattttatttgacctcgatggtacgttgacagatcctaaaaccggtataacgaaatctgttcagtatgcgttggcaaaggcaggcatcttcgaaccggacctgcaaaagctcgtgccgtttattggtcccccgctgcagcaatcgttcatcgattattatggctttagcgaatcacaggcctgggaggccgtgggcgcttaccgggaatatttcaaagaaaccggtatttatgaaaatgaacaatatgcaggtatcccggaattactcactgcgctgcggtcacagggacggcggctgtttgttgccacttccaagccacaggtatttgcggatatcgtgatccggcactttaacctggagccttattttacggcagtgtatggcagcgaactggatggtacccggtcagataaggcggaactgatccgctatgtaatgtccgaacaacaactgagcgccggcgacaccattatggtgggcgaccgtaaacacgatattataggcgcacagaaaaaccgtttacccgccattgcagtgggctacggttacggcagtacgcaggaattacaagctgcattaccggattacatttttaacaccgttaacgaattacacgccgggtttccctgatcagcgccagtagatctcgatttatatccgctacccggagaccgcattacggctccgggtaaaaaaaatcagccctaattgatttattagccctttattaatgcactgattagtgcctctccccttaattgcaccaggaaacttccacgtttcattatctgtagcccggcattattctaagaaaaccacggtagcaaatccgatagtaattcctaatcatcatcaattgttccacacatgaaaaacaagttgcatcttctcttcgcaacccttgttgcattgtctgttggctgctccaaaaaagaagccgtcaattcactccagtcgctcgatggcaaaaaatcaggcgtcaacgcgctgggctctcctgtaggcgacgtagtcggcaaaattacggtaggctaccagggctggtttgccgccaatggcgatggctcccctatcaatgcctggtggcattggacgcagaactggggcgcatcgccttcttccacgaataatggcattaagtcctggcccgatgtaagggattacagcagcacctatcaaaccgcctgggccaacctgggaaatggtcaacccgcgaaactgttctcttctttcaacgaccaaaccgtaaacacccactttctgtggatgcagcaaaacggtatcgacgccgccgcactgcaacgttttaaccctaatggcagcgaaggacccgtacgcgacgccattaccgcaaaagtgaaaactgccgcggaaaactatggccgcaagttctacatcatgtatgatgtgagcggctggactaacatgcagtcggaaatcaaaaccgactggactactaaaatgtcggcctacacctcctcctccgcttacgccaaacaaaacggcaaaccggtggtgtgtatctggggctttggcttcaacgattccaatcacccctggtctgccgcggtatgcctggatgtgatcaactggttcaaaaaccagggctgctatgtaatcggcggtgtacctacgcattggcgtaccgaaaccagcgattccagacccggcttcctcgccacctacagcgcgctgaatatgatttcaccgtggatggtaggcaggatcggcaatatcgctgatgtagataatttttataccaatgtaaacacgcccgaccaggcttattgcaacaacaatggtatcgactatcagccctgcgtactgccgggcgatttgcaggaacaccagcgtgcacatggcgacttcatgtggcgccagttttacaacatggtacgggcaggcgcccagggtatttacatttctatgttcgacgaatacaatgaaggcaaccagatcgccaaaacagcggaaaacacctccttcattcccgcaggttccaacttcgtaaccctggatgaagatggcgtggtttgctccgccgattactacctgcgtttgaccggcgacgggggtaaaatgctgaaaggccaaatcggcctgactgccacccgccctactgcgccggtagtgggcggaggcggcggcgcgccggtcggacaaaccattaccctcaaaagcgccaataacctgtacgtgtgcagtgaaaacggcgcccagcccatgaacgccaaccgcaccacggcgcagggatgggaacatttctccgtggtaagcgccggcagcggcaaagtggccctggtaaacagtggcttctatgtatgctcagagaacggaacccaggccatgaactgcaaccgtaccgctattggtccctgggagcagttcgattggatcagcaacagcgatggcaccatttccctgaaaggcagcaacggtaagtatgtttccagcgaaggcggcacacagcctatgacctgcaatcgtactactatcggggctactgaaaagttcagggtaaaccagtaaacattcccctgttttaaatatttggttatttggatatggcgttacatcatgccgggctatcacaacaaaatatccaaataaccaaataaaaaaacaaacaaatagccctaattttagccccggtaatcaactagtatatcgaatgaatgaacgacccggtgatgtattgatcagcataattatagcgacatataatgccggtcagcacctcagagaatgcctgcaatctgtgaaggaacagactgtgaaaggaatcgaggtggtgattgtagacggaggcagcacagatgataccctgactatcgtaaaagaatccggcctggaaatgttgaaatgggtgagtgaaccggataagggcatctatgatgcactcaataagggcatccggatggcaggcggaaactggttatattttctgggcagcgacgaccgcctcctgccaggcttcagtgaactctcggcacatctcagcgatgatcacaccatttactatggcaacagcaccgggttcaatacaaatggccccgttgaatatccgcttttacagggcagcttcagtgaataccggctcgccaagtattgtatgaaccatcaatccattatctacccgaaaagcgttttccggaaatattcctacgacctgcaatacaaagtgctggctgattatgcccttaacctccttgtttggggcgaccgcacctttaagaagcagcattatcctgttaccattgtactgtataacatgacgggattttcctccggcaataaagacacacaatttttaaaagataaattacaactgatccgcaggggaatgggctggtggatgtatgtgcgtatgctgctgaaacgttacaggaaaaagctgctgcgggaagaagacctctgggcgccgtaaggaatgtagcccgatttatctactgttatctgttaagtatgaaactcaccatagatgttgtaatgccttccttccggctggaggaaaaatatgtgctcccggtgcttcgcctgccgaggccggataatgttgtcattaagttttacctgatggcagataaccccaatatagtacctgccgaaagtatccgggaactggcagacaacgaccaggtgtttctttatatcaatgaaaaaaatctgggtgcttccggtacccggaaccgtggtataaccgtttcaaaaggcgactggatcctgttcctggacgatgatgtaacggtaacagatgacctcctgttcaggtatgccgctgctgccgccgcatatccggatgaaaccgggttcattggccttatccatttgccgccaccacccagtgattttgccatggcgcttatcgttaacggcaatgtaaatatcttttctgtggcagcgaataagccctcctttacctggggcgcaacggcgaatataatggtaaaaagaagtgcagtgggcgatgtgcgcttttctaccgactatccaaaagccggcggcggtgaagatgtggatttcttcctgcatgtacgcgacaataacaacaaacggaatttcagatcactgccggaagcggctgttacgcatccctggtgggatgatggccgcgctaactacaaacgtccttaccggtatggccttggcaacagccgtttgggtaaaaaaaatccaccttatacctaccgcaatttgccgaatacgcccgaaacaatattgctttgcgttggaataacattggtgttgctgtttactgcaccctattggaccattccggtgttgctgcttgccattggtaccttacccgtggaactggtggcaaccgcggtgatgaccaggaaacgtttcccgggcagttcctttccggtgatgttttatgtcaccaccctgaaattgttaaacgatacaggggaactatggggaaagctcacccacggcgagctttccaggatcactgaacgttttgatgataccggcactattaagaagaatatcttcttcaaaacgaatacctacaaaatagtaaagtgggtattatatctcttgttgcttatgctgatccttattatctggcgtaagccctgatctgcaaagacgatggattaggcaacgttacttccacacctgttttctttagcagcccgcttttctgatcccttttaaaaacaacaatattccccgttttctggttggctaccagtaaaaacctgcccgtaggatcgatcacaaaattccggggatgtttaccctgcgtggattcaacgcctatttgtttcagtcgtccgttccgctggttaatggaatagataaatatactgttggcatcttccctggtagaagcatacaggaagcggccatcgggggagatatggatatcagcgctgccataatcggcctgttttttttccaggcgggcatctacccgttggaagctatccagtttaccggcgtggtactggtatgccgcaacggtgccgctgatttcttcaatacaataagccattggcagccggggatgaaacgtgatatgccggggaccgctgccgggagtggtacgggcaaacggcggactggccggctgcagcggctcagccgcttccggtgccaattgataggcatggatcttatctgcaccgaggtccgggaaaaaagcatatttaccgtcaggagaaaaaaccgccgcgtggatatgcgagctcagttgccggctacgtacaacactgctgtctttaaaagcaatggtttgtttggcgggcgctatatgtccgccgccggtgagcgggaaaatggaaagactgccaccgctgtaattggcgcagataagccatttgcccgttggatctactcccacataggcgggattatcgccgccgctgtcctgccggtccaccagtgtcaccgtttctttaacactgtcgaaagcaaaactgcttacaccacctacatttggcgtttgcgcctccgagcaggcgtaaatatatttcccgtcaggcgataacgtaagaaaagaaggattgagaatgcctttcgtggcagatacctgttgtaatgtaccggtctgatcgttaaacctgaacaggtatacgccatctttctccttgttgtgattgtaacttcctacaaagagatagtactgctgcgcatgtgtagcaaggccgccgaaaaacataataacgaaggtaaaaaatattttacgtagcaatgtgatgaggatttaagcatgaagatatcctctaagataattatctcccgaaaaaaaacagggaaaatgtataatagacaaatttgtctattattaaaaagatgcactaactttgtatcattatggcacgaccagggaatccgaaagaaaaaatactggctaccgcagcgcggttgttttacgaacagggatataactccaccggcattaaccaggtactggaagaagccggcgtagccaaagccagcctgtacagccattttggctccaaagaagaactcggactggcctacctgaaagaagccagaacggcctggtttgccgggattaccgccatggtggagaaaaaaaagacaccggtggaaagacttctcgccgtattcgattttctggagcagcagctgccacaacaggattttaaaggctgccgctttataaacatgctcgcggaaatcggcgacagccagccggagatgcggctacaggtgttggaacacaagcgcaaactgcggaagtacctgcatcagttgttagtggctgtaccaggacaaacagctgcacaggcagatacggtttacctcctgtttgaaggtgctattgtggaaagtaaagtataccgggagctttggccggtgaaaacggcgaagaaaaccgtccggttgctgataggccagccataatatttatcatcgccctgggatcagggctatttttacaccctgttatagacaaatttgtctataactaaatacatattctcatgaatacaattcctgtcttatcagcagcaacggccgcaccggaggcaaagccggtactggaacaggtagcccgctcactgggccgcattcccaacatgtacggcgtgatggcccaatcgcccgccgtactcgaagcctacgtacaattcagcaacgcactccgcaaaggaagtatcggcaacgccctggcggaaaggattgccctcgccgccgcggaatataacgggtgcagctattgcctgtcggcccacagctacctcggcgcccgtaccggcttaacagcagcagacatccgcgatgcgcgggaaatgaaagcggctgacgaaaaaacggatgccgccatgcagttcgcccggcagctgctcgccaccccccaaagcctgtcggaagccaatgtcagcacactccgcgcggccggttacaccgatggcgccatcctggaaatcattgccaacgtggtaagaaatatcttcaccaactatctcaacgtagtagccggcacggaagtcgactggcctgaagtggtaacgcctctaaaacccgctgttcatgaaaacgaataacatcaccgttaccgtccacaaaccttttaacgagttgttggggagcgccagggaagccattaccagcagcggcttcctgctgctgcacgaaattaacccccaggccatactggccagtcatggcatcaccaccgcgcccgtccgccagctgttgtttttccacccggtatatatgcagtcgttgctcgaaaatgaccccgaagcagtgatagaggcgccccttaaactggtattgcgggaaaccggtgaaaacaccacggcagtaagctactttgaccctgcactgcacctccagggctaccgcgggctggcgcctctccgcacccggctgcaaacagcaatggaaaaggtattggcacatttattttaaagactgtgtaaggaaaaggcggctcatccgactaacaggatagccgtctttattacggatttaaagcggtaattttgggttattgtattattcaccagtattttttagcgagatgagaataatatttcttttaacactgatcctggctacacagattgcctgccatagccagaacagcgacaataaacaagcgccagtgaaaaatccttactactccagaacggatacacggaaactgcatattactaatgcagaatggaaaaaaatattgccgtccgacctctacgccgtcgccagggaaaatgccactgaacgggcatttacgggcaaatactgggattccgaggtgaaaggcagttactattgtgcggtttgcggcaatcctttgttcaggtcagatgccaaatttgccagcacctgcggctggcccagtttttttgaaccactcaaagccaacagcgtgatctacaaggaagataattcctttggcatgcaaaggacggaagtgatctgcgaacgttgcggctcgcacctcgggcatatctttgacgacggcccccctcctacgcacaaaaggttttgcatgaactctgtatcactggactttgagcccgatccgggcgcacattaacccggattcactccaggaactgatccaggaaagcttccccaaatgcggaagcccgcagtgttttgttcagattgcgccggaaaggattaaacatcccgatccccggcaaaggtttcacaatgtgatagaaaggccggctcagatcctgggaattggccagtacaataaatgtcagatccctctccggaatcttcacaaacagggctgaatagccggtccaccagccggtatgccacaccacttttatgcctttgtaatactttacataccatcccagtccatactggatggttttacctttgggggtaacataaggcgtgaacactttctcccaggtgctgtctgccaggaacattttcttatcaatagcagtagaataaaccgccaggtcggccacattgctcattatacccgccgccgggccaaaaccatacgaaaaagtaacaggctgccactgctggtgcttccagtcgtacggcctcgctacccgctgcatgaatgccgctttatcataaccggttaacgtgaagttcaggctgtcgtctgtactcggtactgtattttccagcgacaacggcgtaatgatctgctccatcagcaactcaccgaaactatgccccgacgattgcgcaattaccttccccagttgattataccaattgccgttatagcggaacacataaccaggcttatagctgttaaacatgttgcccatcgcggtatgggtaagcaggtgctttattttgatccgtggatcactaccccagcgggcgcccaggttgattccgtatttgccgataggatcatccaggcttaccttcccggcctgtacctgctgcatgagaataatggaaccaaacgttttggtaaccgaagccacctggtaaacggtattttcatccggcgccgtttgttgctccaggtcggcgtagccaaagccttttttccataccagcttttgttcatttaccacgcccaccgacaacccagggatatggtatttttcccggagatgttccagtttcttttcaaaacgggatattgctgcagcactccacacggtatcacgggaggtgaccgctgcaaccttttgtgccggccgggtagtgcggcaacccaataataaaaaaacgatcatcaaaaatgcgtagaacgaaaaagttgagcgagatgccatccgggttattttttaatggcaaagctccctgtttacagcattctcacctactcatatccggatttgagacaaattaaagcaccgctttttgtgcttcatgcgcacttttccggaattcggagggcgacatgcccgtgaattgcttaaacacccgctggaaagtagcaggtgaagaaaatccgcaatcatatgcaatgccagcgaaagttaattggtcagcatcctcctgtaacaatttttctttgaacaggttaatacggtagccgtttacatactcattaaaatttttatgaagatgctggttcaataccgccgaaatagtttttggcggtaaaccggtatgtttggccaccatttgcagcgtaagggccgcattcagaaataaccggtcttcttccatcgcttttttcagcaacaatactgcaggcgtggtagtcgattccggcaatatcgtttcagctttcttagccgttaccatttcctggtaagaaataatatatcccttaatacccagccagtaaatcaggatagtaacaggtacataaataggataccagtcaaatttatcgagtatcacgtcggtataacggggaataatatacggcaccaggtataccagccagatagtgaggaagccggcaaacagccaggtgagctgctgcagccagcgcaggccggcgtcagccgggcgattgcttttatataccgccaggaatttaaaagacaaccccgtataaatggccagcgatatccatcgtggaatatctgaatatacattgtaagtatctataaagatgccccacggctgcgggttattcttcaatacacctgttaacacacctgccacaaatacgatagctgcaacgggcgctccgaggtcgatgaccaccggccagaaatgcctccgccgttgccgtgtgagcgtaaattccggatcacaaaaagattgtatgtaaaaatacatcagcggccccacgggcattatcacaatgagcggtagtaattgcgacagcaaattgagcagcggaacgtcgaaccagtgataataggaaccgcacaaacaaaaactggccatactgagcaggaagatcaaccctgctaaaaagcggttcgccacccgtttcctggtggagaaaaacagtagtccgcctgcaataaaaccctggactacccccagtaagataactgtttggaataaacgctccatagtgccaattccctaccaaaataagataaaatatgcttcctgccgggaactgtttaaccaaacccggctagaaatatttctctatagtgagaccataattcatcaacaggttttcgcggtcggtacggtttagcttattataggtcatggccgccgtgatggccagccaggaacggagtttcacggaaagggcattattgcatttaatgatatagtcgttgccgtgggacagggagttttgcaaaaaattggagccttccagcacaataacatccttgatcacccatttataatatacccggaaggaattccggaaggtatgatacacatcagggatcgtatcgtgcagaataaggtcgctgttttcaaacaggagcccatcactcaggttgagcgtggcgttcttacgtttaataacgtcgtaagctgcgccgccgccgccctggaagcgatcgttgatctttaaggaataacttttatcgtagttggccagtccccagaaatacaccttcttttctccccggtaaatattaaaatccagtgcggtagaaacgtcattattggtgatgtcgtggtcctgctttccatacacatagctggcgcccatgttcagattcattctctttttactgatcttaaagcctacattattattgagcaggtacgaattaccatcgttagtcatattcaccgatcccgtggaagcgtatttaacgtagtaatgcaccgagtcgctgaactgggcgctggagcttaagccgtaaaacaatgccatccatagtaaaactaatctcttcatgaacaggtgcttaggtgcgcttcgggcgccgcaattaacgtgcctgaacatatgcagggaatccgtatatttataatattaatatcgtcatgatgaaaagattgatactatctcttcaacaacgcccttacctgttgttcctgttaactgccattgtgctgatcatctattccttttttatccgccatcaaatgacggacatccacgtgcacgataccatgctcattatatccacctacctgatttactggctgatctctttttgctttatagtcgccgccgggctatatgccggtttaatgcgcttcctcccaaaccgggcgctaacatggacgcacatattgctaaccttactgctattattgtctgttaccgtaattgttcaccactatgataatttgtataaaaataccgggcagaacgactcccccgcttcggtcgggcaggcaatacactacatacaaaccgctgaacttatttaccgttggctgatcctgctttttttggcaacacagttaatttttgttggtcattttgtttggggaatcaccaggcactttcagaaaaaacactaaaaaaaacaaagttttttagagatcttagcccatgataccgccggagcacatttttcgggccactacattttgctaaaaaccacgtaaacaatctacatatgtcatcaagaagaaatttcctgcttcagacagcgctcggcatggcagccactactatggcgcccttcaccgttgccgccactgctgccggcccggcaaagaaagcgctgctgcccatcgggatggcgggttacacctttgccaaatttgacctcgaccaggccatcgccatgatgaaccgggtgaatatcaaaaacatctctgtaaaagatattcatcttcccttaaacagttctccggaaaaaataaaggaagtactgggtaaattttctgcggctggtattaacgtatatgcagtaggcgttatctacatgaaaacagaaaaagcagtagatgaagcattcgattacgctaaacgtgtaggcgttcccttgattgtaggcgtgcccaatcccgaactgctggattatactgaaaaaaagatcaaagaatataatatccgcctggcggtacacaatcacggtccggaagacaagctctatcccggccctaaaaacgcctacgaccttattaaaaacagggatgcccgcctgggcctctgcctggatataggtcatgccgcccgcgccggagaagaaccgtccaaagccatcctggcctataaaaacaggatcttcgatctgcatattaaagatatttcagcggcagtcaaagatggcaaagccatcgaactgggccgcggcgccattgatttcaaaaagctggtaacggcactggagaaaatcaattacgcgggcgtatgcagcctggagtttgaaaaagatatgagtgatccgttgccgggcattgccgaatcggccgggtttttcagaggcgtgatcagcacggttaacagctgatcatgtacatttattgatgcaggttgccggaagtatctcttccggcaacctgcttttttttagaactttaaagttacgcttgccaggatgttcaccggcttttgcgcaataccattggtatcccagtacttttcatttaagagattattgcctttcagtgccagccggtatttcggttgatcataaaatacagaagcactcaacagggtatatcccggcaaaaggaaagtgttgctggattcaaaccaggagtcactgacataattcccaccggcgccaaagcccaaccccttcatctttccagaatgcatatgataacttacccagatgttggctacctctttagggctgcctgcgatcagcttattctgcaaagcaggagacgctttcgtatacctgttctcgttatgggcataaccagcaacaatgttcagtcctgttacgggattggcggccagttccagctcatatcccttgctgcgttgcgtaccatcctggaacataaaagttttaccgtccacgatctccgtccgggtaacattggttacgtcaatgttataataactggcggaaccgcttaatttgttgtccagcagctccacctttacaccaccttcccactggtcgcctttctggggcttcaggttcaggatcgtattgtccggctgcacaagcggcgccagatttacaaaaccgttcatataattggcaaacaatgataccttgtcttttacgacctggtatacgatacccagcttgggcgacaaggaagtctggttataatcaccggcatattttcctgtggcaacggtgtaagtaccgctggtggtaaaccggtccacacgcaggctcagcatagccatcagcgccggggtgatattgagtacatcagaagcatacacgctgtagctgttggatttggtacgggtagctgaaaatcctttctgataagacaggtcatcaatcaaaccagcattcagttctttcacaggctgattgatattaacaacgtcatagttgaccgtaacgcggttcaggctattataattatagttatagtcgataccaatcaccagccggttccgcaacgacgcgatgttgaaatcgcccacgaaattctgttgcagctgaatgttcccaaaagtttccggcttttgattcctgacgctgcgcgccatagtagaatcggtaagcagggtcatgttggtccagtaaaaatgtttatagaagccttctgaaaacaggtaattggtttgggaagtccaggcatttgatattttgtattctatcctgccttgtatattattgatcccattactgatatccgcgccgttattgatatacgaccgcttatacccaattttaagatctttaaaactcctggctgtcacatttttgaaatcgtttaccgcataggtgccggtggcgaagttgcccctggtgatgtccacatctaccaggaacttcaaccggtcattcacctggtaagagaaactcggcgcaatcgtataatttttagcatatccctgatcctggaaagagccttctgtttgaccggcagcattgagcctgaacagcatggtgtgctcgtcattcaacggggtgttgatatcagcggtaaagcgtgcaaactcaaagctaccgccggtaaagctcacgtttccgccaaaatgatcatatggttttttggtgacgtagttataaagtccgccgaaggtgatgttgcggttactgccaaacaaggtaccggaaggtcctttgattacttctacgctttccaggatagccgggttcaaaggcacaatcgcactggtcaccattccattccgcatacccgtggcattggaaaaaccgcgtatagtcatgccctgggaaccgcctacggcgaaattaggcactgcgccgggaatattccggtaaatgtctgtacgctccgtgatcagttgctcctgcatcagggctttgcctaccgtttggtatacctgcggattttcgaggttcttcagcggaagccgtgctacctggtccgtattcttatcaacaaacctgttacggttcgtattaacaacaatttcccgcagctgcgtatcagacaattccaaccgcagcgatacgtctgttgtacggcccttttccacggttacgttttgtgtaagcgtctggtatccaatcagcgaaatttccagctgccaggcgcccgcaggtacgcggtgaatggtgaaagtgccatctggtcctgtaatagcgctcttcgatgttccttttatcaccacggttaccgatgccgcagtttggttatcgctggtagttattattccttttatagtccctaaatcagtttctgtattggagaatgcgtacagtggcagtaataatatcaggcagtatagcaatttcttcatggttggatgcgaaaattttcgcaaagataccccggcggcaactgcatcattttaacattccggaaaaatatttatcagaaaagaaatattacccgcattttgatattagtttgcaggcaaagatcccttacatgaaaattaagcttatcagaaaattcctggaatacatttacaataattacgtgggcaactttttaggatttgtgatcggaatggcctctacccgcctggtatcccattatttcaccacccgcagcatccggaacttatggggcctcaccgcccataaaactgtggtagacaaacacacctacaacaccatggaatggaccatctccatcgtgatcggctttattgtttttgaaatagtttccaagtggctgaagaaaaaactgagcgaaatactcccaaaatacaaattcacccaatggctcgtagaagccgaagataaggcgccaccggccgataccacggagcgaagattgtagcggaggttgtctgaagcactgattacgctgattttactgatttactttttttgattttactttttgattttactttttgatttctactaaaaaataatgggagacagaaggcaaactttgctttcatctcccattatctttaaatcctataaaaatcaaaaaaagtaaatcagtaaaatcagcgtaatcagtgcttcagacaacctccgcgacaatctccgcctagaatttgagggcaacactacccgcgaagttccgcggcttttgagggtttacggaccagtagcccgtgtagtaaacggtgttggtgatgttattcacgttgaaggataccctgaaatgttttgcattgtaaaagacgccggcgttcagcagcgcataacttggtaagtagaacgcgcctgttttgctgttgtctatcactttgtaccggctggcatagttgcctccggcgccgatgcccaggttcttcagcgttccgctggcaaaccggtaggtggcccagaggttggcgaggttctgtggtccttgtcctcctggtgctctgcctggctcactgtagaaatcatccttattcccttccagtacttttgtatggttgtagctgtagccggcaatgatgttcagttgttgtaaagggtgggcgttcagatctatttcaaatcccctgctgccgaatttaccaccctgggtagagttcatcgggtttttgctatcgggcaccactttgttgcctactttaatatcatataccgataacgtggcgtacaatttatctgcgaagatgtctgttttcactccaaactcgaactggttggcatgttccggcttgaacgattgcgtgcgctggtaatttccatctgtatcataaacagaagacggagatacgttgaagaagccgttcatatagctaccgaaaacggataccttatctggtaccacctggtataccaatcctaacttaggcgataaggcaaactggctgtagccgtcatcatcagtggcgtttttatcgcctttggaatcgaagtagtcggcccggagacttaccatcgcaatgaacgccggcgtaatattcagtacatcggatacataagcgctgtagatgctgttggtaacattcgtgttgctgccttcggtgcctgcgagcagtgcatataccgcatcttttgtaaggggcaccgcaggatgtacttcttcgttagacgggtctgtatagtcggtaacgtcgccctgcggacttacgttcctgccggttgcccagcccgaccctttatccaccacgttgcggcggaagtaatcaaccccgatcagcaggcggttacgcagtccgccaatcttgaaatcgccgttgaagttttgttgtatatcgatggttttggtggtttgatcttcaatgtgaaaatcctggccaaaccatttatcccccgggtcctggtcccacatataggtatacacaccgtcggattgtaccctgccaccggaaacaacggtctgggaagtccatttgccggaaagcttatacagcatttgcgcctggaagtttatccggggatttttaatagtaagttcgttgctggtgaatgattccttcacgttgagattaagctcgtcgatatttttgaaatcgagtggagcagcacgatcggagtgaaagaacaccggtggtacagctcttttttcctggagtatttcggccatcacctggaacgagagacggtcatttacttcgtaggagaaagacggcgcaataaagaagcttttccggaagcctgcgttttggaaagagttttcggaagtataggccgcattgagccgcatggcgatcttttgctttttgctgagaagggtatttacgtctgccgtaacccggttgaggccgaagctgccgacgctgtagcccacttcaccaccgaagccatagtaaggttttttggtgatggtattgatcataccgccgtaactataaaaactgccgccgaaaagcgtgccggaagggcctttcatcacctgcacttcttccacatcagcgggatcaaggttgccgctggtaagaccagggaggccgttgatcagtgatggctgtgcatcgaaaccacggagggcgaaataagaagcgccgtcgccggctctcccggtcgactgccacgtttggaagatccccggaacattgcgcattacatcgtcgtaggtagtaatgccttgttgcttcatgatctcggtggaaacagcattatatacctggggattctccaggtttttgagcggcatcttagccactgccctgctttcccggttcatgttgcgtgacgaaaccgttacttcgctcaactgggcagcgctttcgttgagggtgaagttcagttgctgcgtttgtccgggggctacagtcacttcttttaactgggtagcggagccaacagaggtgatgcgcagcgtccagttacccggtttaatatttttgatggagtattcacctttttcgttgctgatgctacctagtttggtgcgctctacgctgatggtaacattaatagccggatggccgtcgctggtggttaccgtaccatggatggtgccgttctgcgcgtatgctgctgctgaacacaaaagggtacctataaataatagaaatctgttcatctacattaaactggttgattaaaacttccgcaaaggtccggcgacgaaaagggaaaagtttacgcaatcgggaaaattttgttggtaaccacgcaaaaaagaggatgcccttccggacaccctctccttttcttatttagaattggctttagaacttaaacgttacgtttccggaaaaacgtcttggcatttgaggctcaatagtgctccagcctttgtagtattctttattaccgatgttatcgagtttgaaggctacattaaatttgttggtgttataaaacagggaaccatttaacacggtgtaggatggcaacgtgaatacgcctgtggtaagcctgttcaggatcatgttttcgctggcatagttgccgccgaatccgataccaaagcctttcaccggaccatcctggaatttgtacgtaacccagaggttcgccaggtttttaggtccggcttcttcgggacgtctgccttcgtaatctttattatctgttttaacgaacttgctgtcgttgtagctatagcctccggtgatattcaaacccgctaccgggttagccactacctctgcttccacgccgcggctggttctttcgccgccttgtgtaaagctggctgtaggaccaccgcctatttgcataatgatatctttcactttgatatcataatagctcacagaacctgtgatcataccacccaacaggtttactttcacaccaccttccatttgattggcttgctcaggacggaaagtttgccatacattatcgctgggacgttgtcttggtgcgctgttggtgaaaccattcatatagttggcgaaaacagacaatgtattcaggataggctggtacacgataccgaacttaggcgacagggcagtttgttcgtatttctcattggtgccggcagtaagacccccatttttaaaatggtctacccgcaaactggccattaccgataagctgggcagaatgttgaatacatccgacacataagcgctgtatgtttcctgtgtaaggttagaattatccactgaggtagcgttcagcagtgagtcggtgtgctgccttgaaaggatgccgttgtcgttaccggccatatctatcagtccattcatcacatacccggtactgttgccctgtgttttacggctgaaataatccaggcccgctacgagtctgttacggaactgcccgatcttaaagtcgcccgtaaagttttgctggatatcagtagtgttggtactaccgttctgatagctgatatacctggcaaaagtaggcgaaatattggggaagcccggcatagctgcagagccttcatacaggtaggaatagtatccgtctgatttggcggttcctcttgacacaatggtttgcgaggtccaggtatcggataatttatagatcgcctgtgcctgcacactggaggtaggcgttttaatgctgaggttattgctggtataagagcgtttgttatcatagcccagctcctgcaggttctttgcaaacaaggcagtaccacggtcgaggaacagcatggtagggttggtactttctgaagaaaggaattcggtattcagcatcagcgtaaggcggtcgctcgcacggtaggtaagcgacggcgcaatgaagcgtttcttcacgaagcccgcatcctggaaactgttttcatcgtgataagcaccagttacgcgcaacaacactttattatctttatccagcggggtattgatatcagccgtcaggcggttgaggccatagctgccgccggtatagctgatttctccgccgaagtggtcataaggttttttagtaacggtgttgatcaaaccgccgtaagaaattacggagctgccgtacaacgtaccggaagggcctttcactacttcaatcctttctacgttggctacatccaggccgccgttggttaagccgggcaggccgtttaccagcgtaggctgcaccgcgaagccacgaagcgagtaataaccagcgccatcgccatcgcgaccggtggaggaccataatttgctgataccgggcgcattgttcagcgcatcctcataacgggttaccacctggtctttgatcagctcgctggaaataacgctgtatacctgcggattttcaatattctttaagggcagttttgccacatattcgctgcttcttttggtatacttgttccgggaggcagtcacctctacttcattcaggttcttctcggaaatattcagctgaagatccacagtaatagctttatctttttcaacagttacctgctgactgctggtttcatatcctgtgagtgatacctggatagtataatttcccggggtgatattgcgaagtaaataagtaccgttatcgtctgtgagggttgttttcttagtgcctttcaaaactactaccactcccggcgccggcttgttatctgatgtggtgacgagtccctttatactgccaccgttgtctatttcctcggcggataaagtgccggatacaattgttgtcaggaacagtaaacaccatgctgttctttttaaaaattcccttatcatagctttgtccattgtctggttccctaaaatttgcagccgcaaagttcggggcatgtgatatgctgaggcagacggatacggaatttgatttacgcaatcgggaaaaattcagcggaggttgtctttctcactgattacgccgattatgctgatttgccggatttacttttttgatttttatttaaatgatttggggagataaagcagatatcactgctttatctccccaatcttaataaatgataattaattatttatagctttcaattaagcaggtgctttaagttaatcactaaaaatttcggtcaatacaatccgcataaccaggtaaccgcagatgaatccaaaacttaagaaaagtaccataatagcgccggagaaaactgctgcaaatgcctcgctatttactacaccaggcaccatcattcccttagccatttttattgatacgttctcgataaaacctggtattttcgacaactcaaccaaccccgctccgatgatcactttggttagccaatccgatatttgtgtgagattagtattcgcctgtactattttttcggcctttttattgtctgtcagcgttcgttgctgcgcatcagcagcagtaggcaggccgctggtaataatagtaggcacaccaaaaataaaacccgtaactgcgcctatcattagaaaggcaaatgcccagagaaaggccggcgcaagatacagtttaccaaccaggttggcatagaacaaaggcgtgagcaggattaaaaaggccacgagtaaccagaatgtagtccagaaaaacttttgattaccaccgatagcattaataattttttgccagataggccgggcttggggaacagaactttccagattatgtgcttccatgaggtttttgggggtttaatgatgaagggattatcttaatgaagataagacattagaatgcttttttttgttaatctacctcctggctaaataaaaaaagccacccccttgcgggaatgacttttctctttcatccactatctatctacttaacttttacattaggggcgggtgcatcgttccgtacttcttctgtggcggtagccaccagggtatcgccggcgttcagctctccaaacacttcggttttaccgttttcactgcgaccggtagttaccggtacccatttcgtctttttatcctgtattttcaccacgtatacaccggtggtggaattgaggacggcagaggaaggcaccaggaaattgttggcattaccggtgagtggaatggctacttctgccaccataccgggcaataacgttttatcattattggctacgtcaatttcaatatgctgggaacggagtttgcggtccagcgcaccggcgaggcggatcacttttcctttaaattccttattgttcagggatcgtactttaaaagccacttcgctctggttggtgagataactggtataggcttccggcacgcttaccactaacctgagtttcttttgttcctgtaaggtgaagatgggcatttcagaaccttttccggaaggtcccacataggcgccggcgcttacgttacgcgcagtgatcaccccgctgaaaggcgcgcgtatctcgaggtagttgcggttatcccctacttcacggtgcgcggctttggcagcgtcgagctgggccaggtcggatttctgccgggcaaaggccaggtccaggtcattctgtgacacggtacccggggttttgctggtttccagcaggcggtcgtaggtggctttgctggacaaatagatcgcttcctgcgactttaacctggattcagcgccggagagctgcgaattgatttccggggcttccatggtagccagcaactgaccggcagatacttcactgcccacatccacactcatctttttaataaaactgctcactttggcataaagatctacctgctggaaagcaatcagctctccgggaatttgtatagaagaagacaagctgccctgtgtcagggagaaaacttcaacagtgggcgctgctgcaatggcggatgtgtcttttccctctttggcgccggaggtactgcaactgtacagtcctgcgatgatcaccatcgctgacaataaaggaaatgtaatacggaaaccgctgttcatatagtatattttattagaattagataatggtcaggctttttcgtctgatgggatatagtgaatactttcttcatctcttggatgcagtgatacgctctgtgtacctgctttaccctgtccccatgcaaacgccaggggcaaaataaacagtgccgcaaaagtggacgctatcagtccgcctactaccgcccttcccaatggggacgactgatcgccggcttcacccaaaccgctggccataggaatcatacctaccaccatcgcgagggctgtcattaagataggccgtaaacgcaatgccgccgcttctgtagcagataacagcgcatcgccgttatgcttccgcaactgctctgcattcgtgatcagcaatacggcgttggaaatagatactcccaccgacatgatcatacccatgtaagattgcaggttcagcgtagaacggcatagcatcagcaacaccagggatcccagcaacaccgccggcaccgtagccaatactacggcagatactttgaacgactggaagttggccgccagcatcaggaagatcactacaatcgccaccagcaaaccactctgcaaactatccagcgtgtccgtgagcgtattgcttaacccaatcaggtctacattcagtccgcgcggcagcgtacccagtccggcaatcgctttctttacatccactgcagccgtacccagatcggtattattcaggttagccgttaccgttagtgtgggcatggcgccgaggttatctacctcgccgtaagtggtatctaccgacatagtagccacatcactcagcaacggacgggaattattcctcagcaacggaatttcaccgatctgttctttgctgttcatcttactttccggcacctgcacctgtacgttataacttaaaccggctttttcatctacccatatattcttttccgttaacctggaagaagaagtagaagccaccagggaacgggatatatcgttcatatctactcccagctgtgcagcccggatacggtctatatttacgttgatagccggatatttaatggactgccctaactgtacatcgcggagataaggcagcttatttaattcagtaatcagcttctgcgcatattgctcgctcagtttccggtcgcggcccgcaaaccgcacttccaccggcgtgggcgacccctggctaaggatcttatccgttaactctatcggctcaaaagaaagttttatcgttggatcaatcacctttgccttctccctgatcttatcctttaactcatccaggttagtatgataatgttcgctgagcgacacctgcaatacggcttcatgcgggcccgccatccacaggaagataggtgccgtggaaaacaactgcgggtgcatacctatgtaggcggaagtaatggacacattttcctttcccacaatctggttaataccatccagcaatttgatggtttgctgttccgtgcgttcaatacgggtaccatccggcactctcatcctcacctggaactggctgccattcacctttggcagtacatcacggccaatgttggcaagcagcaataccacgatgccacaaaccaccaccaggtagccaatcacaataggcttccggtaaggcatcatccttttgataaagcgcaggtagcggtttctcaggcgttcgaagcgactaagcttaccattgccgttaaagtcgccgcgctctatcaatactttcttttgttcccaggtatctttttcaccggaaagaccagcagccgcaaattcttctgcatctgtcatctcgccgccatctgctttcttgtgatgctttactttcatcacccagttagccatgataggcacaaatgtttgtgccaggaaataagagatgatcatgctgaatcctatagccaaagccagcggcaggaacagtgatcccgggataccgcccatggtaaaggccggcgcaaataccgcaaggatacaaaacaggatcagcaatttcgggaaagcaatctcctggcaggcatcccagatagccagcgctttgggttttcccatatccaggtgctggtgtatattttctatggtcaccgtactttcatctaccaggataccaatggccagcgccaatccgctcagcgtcatgatattgatggtttgcccgaacaggctcaggaaaagcacagctgaaataatggaggtaggaatggtaaggatcacaatcatcgccccgcgcggatcacccaggaataataacaccattaagcccgtaaggatcgcgccgatggtgccttccgtgagcaaactttttacggagttgatcacgtaggtcgactggtcaaattcatagctcagcttcacatcttccggcagctgcgcctgcatcttcggcaatgattttttcaggttctgcactacttcccaggtagaggcatcggcgcctttggcgatgctcaggtataccgagcgacggccgtttaccagcgcataacctgcggtaacatccgccccgtcttctaccgtagctacatctctcaggtaaagattttgtacatctcccttaaataagggaatgttttcaaaatcttttacgttacggatcgtggtattagccggtgtgatgtaattattattcccgatacgcacgttaccggaaggagccgtttggttattaagccgcatggcttccaccagttgatccggtgtcatattatgctgacggagcagctcaggatcggccttgatcaccacggtacgcatattaccgccgaatggagtggaacctatcaggccaggaatggaagtaaaggaagaacgcacatacacgtttgccatatccagcaattcgttattactgcgtttattactgctcaataccagctggcctaccggcaaggtggaggcatcgaaacggataataaacggcgggttggaaccaggtgggaaaatggcctgtatcctgttggaaaaggcactcacttccgcagctgcctgcgccatgttggtaccagggtaaaagttgatcttcatcagcgtaagaccctggatattttttgtttctatacttttaacgccatttacaaacaggaatatattgatgtattgtttagcaaagaaggattccatttgtttgggagtatatcccccaaaaggatgcgacacataaattaccggcatgtccagcttcgggaagatgtcaatcttaatcgtattgactgctttaatcccgaagaagaacaggccggcaactagtaccaggatggtaataggtttttttaatgcgaaactgattaagttcatggtaatgaagtgttgataaataaagccatcaatggcgtccgtttaacgaaaagctaattttcaaagatgctgaaatcacctactgcggcggctttcagcaataatgcctgccatacgttactatatgcaatatccttgtctgtttccgccctgatgagtgcatacagcgcctgtgttacatctaccaggttggtcagtccgtttttatacaatactgatttctggagataggcatctgaagcggctttcacctgtacaggcgattccaggtaattatctaaagcatttttgattttgatatcagagaggtccagctgtgcgcggatctgctgatccgccaggttgtattcttcctgtaatccctggctgatgagctgttgcgacttcacctgccgcgaaatgcggaagggctgcgtaatattccaggtaacgcccacgcccaacaggtagttggtacgggtaggcttaatgccatcccagtagctatgggtgaagtctgtttgatcggtagcataaccatagccgaagcccgaacctcttgtctgcaatacgcccaccagcgtaaacgccgggtaataaaaggttttagcatattttgcctgttcatcgctaacagcgatcctgctcttataccactgtaacagcgggtggttttccggggaaaatgtttgctgcggcagcgccgggatgcgggctacataagaagtgtccagtataaattgccgcggcgtgatgcccagcagctgtgccagttcattgctttgtgtttgttcaaaatccctcgctttggtaagcgcaatttttgcattggagtattccgcgttggcctgggaggaatcaacacccgctatcagcccgtttttcacgcgggtaaccactaccctcctgatggtatctgcacgttccaggttttcctggtaagagcgggttaattgctgtgctgctacgaggtttaaataagtggccgccacttttatcttgtgcttaaaaatctcctgttgccagtctttatcgttctgagcggcggccgctaatgctgttttaactttttcctttgccctgccgaaagcaaagaaatcccagttgatattagtaaggtataatgcgccgaaggaggcgttccagttctgatgatcgagtggtaagccggaggaagccactgctaagcctccgaagccgtacagcgggccgttctggccgtttacggtaccatagtcctgttgtgctgccacattgaaattaggcaggtaatcgcggcgtgcctgggacacctgttccctggaagctgcggtgtagctggctttggcacggatcgttccatagttggcaatagccgtgtcgatagcctgctttaaggtaaatgcctgttgtgcatataaatggtagcctgaaaacagggatacaagcgccaacagcaaatatttcttactccacatgaataaatagattttacggttgaaatatcctgaaggatattcaactgcaaaatttctgtatcattttgaagtaaacttgaaggaaaagggaaatacggatttttttttgtgagatggacacttaaacggctactgcggccgctacaggcaaggcatcactgtttactgtctgttttttgtaaaaacacacctgtattttatgccatccatcgctgtaattataatccacatcatagccattcacctcgcagatttgctttacgatggccagtccgagcccgatgctgtcgttgctctggttacttttcttaaaccgctggaacagttcacacgtggggatttgcggcggtatgccggtattgctgatgcttaactcacggtgagtgagcaccatttttatttgtccgccgtcgcggttatgccggatggcattgctcagcaggttgctgataagcatttcagcaagggccgggtgaatattaagcggaatgtttttatcaagattagtggtgatggcgatttcacgcatagtgatccagtcttcataagtagcaatcacatctttcaccacgcggcaaaacttgaggctctctgttactttaaactcctggttttccagcttggtgagcaaaatgagggagcggttaatatgtgacagtttctcaatggcattctgcatatccccaagcagtgcggcctgcacgctatcgatgttggtttcggacaacagttctatcttactgcggatcacggccagcggcgtttgtaattcgtgcgaagcattttcgctgaactcttttacggcagcgtaatcttccattgctttatcggtcatcttgctgaggaatacattcagctctttaaattcggtggtgctggtttccgccagctgcagtttattcttttgtttcaggtcgaagctgtgaatcgctttcatggtgcggcgcagcggggaaaagatcttaccggaaagcaaccttgctgtaacagataccgcaaagatcatcaacagcattttccatactaccgtgctgagcataccccggaatatttcttccgatttgatcacataattataggacgatattttatattgctggtccccgattttataccaggaatctaccgtgatgcggcattctttctttccaagatcttctgctacaaaattatcttttgttacaattaccttcttctccggcagcggacccgccacggtggtaatggcaatgggcctgccatgggtgtagcggtctggtttttcaccggccatcatctgctgggccacccggtcgttgacggcggtcatacgcgctacttcggcgtcatcgaggtgccttttgatattattgcgcgaaatcaccatggtaacaggcgttaccaggaacacgatccctataaaccagagtgttattttattaagcagcttcatgttttggatgtattaaacttgtaccctaatccataaaccgtttctatatagtctactccttctgcggcgctgatcttctttctcagatttttcacatgctggtaaacgaagtcgaagttagccaggttatcggtataatcaccccagaggtgagcggcgatagcctgtcgtgacagtacacggttcttattgaccacaaaatacaacaacaggtcgaattccttgcgtgttacgtccaggagggagttattgatcagggcttccatggtgtcggtattcagctctatttcattgaaaacaacgaggttattgccatccagcttcttccggcggtaaatagctctcaggcgggcatgcagctccggtaagtgaaaaggcttggttacataatcatccgcaccccgttcgaggccgttcaccttatcgtcgagggcatctttcgcggaaatgatcagcaccccgctgctgatattctcctgccggatgaaattgagcaattccatcccattgccgtcaggcagcatgatatccagcagtatacagtcgtaagtgaaaagagaaagcttttcccgggccgtttccacatcataagccagttcgctgatatacttttccccgttgaggtaatcggaaataccgctggccagttccttgttatcttctacaatcaatactttcatataaacacacctggatgcaaagtgcgtagtaaatttatagcaaatttgaagttttgccgcggattttgtcttggctcaggattacgcggattttgtctttcccgctgattacgctgattttactgatttaggggatttgatcactttggatttttaaatgattcggggagatctaagcggatttcgtcttggctcaggattacgctaattttattttgggattttagcggattttgtctttctcactgattacgctgattaggctgatttttttgaattttagcggatcttgcttatctttataatatctgtaaggtattgataaccagtttacttctccgaaggatgcgtctaaagaatatttcaaaacctgctatagcgcattgatacacaatacattaccgatcaagtccacgtcacctccacatcaaggccagcttcaaagcacattaaaggcagatgcaaagtaagtccaaggcatgtccaaagccagtacaaagcataacctatctcctcttcacatcatctttaaataccccatcttctccttcaaaaaaacaacatccgcttacatctccccgaatcctttaaaatcccaagtgatcaaatcccccaaatcagtaaaatcagcgtaatcctgagaaagacaaaatccgcgtatctacgcgccgaaaagctccgccagcttcttattcatcgcctcgtcatcctctccgccgccaccgtagcggccaatgatcacaccattggggtctatcaggattttggtggggagggaatggatgccgtagtagtcgctcaaatcttcggggttgggcaggttcttttcccgcttgctccaatccaggccgcggagtacatgccgccagatgccgatgccatcttcgttaacggcttttttccatgcttcaggcttggagtcgtcgtcagaaacgccgatgatttcgaagcctttgctgctgtatttaccatatagctccttcaggtgcggattgcctttgcggcagggtccacaccagctggcccagaagtcgagcatcacgtatttgcctttgaaatcagcaagactaatggttttgccttcgatatcggttttggtgaaatcatgagcaggactgccgggagagccggcgcgcagggcgtccagttcctgtttgatttcaaggccgctggcgctttgctgcatctcaggcgacatctttgcataaaaggcctctccttcctgcaaaggcatattgcctatacgaaaacgaagcagctgtgcagatacgtaggagttgggatgctcagtaaggaaggctttatccgttttctccatttcctcgtaatagggctccatctggtcttttattttgtccagctttgttttgtaggcctccagcgcagcttcggatttctttgctttgatggcagtaatgtattctttattcagcttattaaaagcatcagacagtggctggagctttttcatgataggtgcgcgggccgcatcaagctggtcctggtccagctgggctttggaacccgtgagtttcgcgtccttcaggcgcccggtggaagactttaatttcatgggcgctgcctccatgaaaaaagaggccatgtctccttctccgtacatggcagtctttttatccacgaagatacggccttctaccggctgcaccagtttaccgctgaaggtaaactgcccgtttttcgacaatacgctgtcggtccggtattccttgccgctttccgcataggcgaggtacacgtagcgattgggaagacccttaatatctcccgcaagggtaaatggtaacttttcctgcgcctgtgccccaaattgcagggctataaaaggaagcgcaatgagactgtatttcatgctgctgttttttgagatgattataatacttccgccagtttcttttccagctcatccccatgcagatctttggcgataattttaccggaaggatcaaccaggaagttagccggaatgctgcggatatcatactgttgggcgatggcgttgttccagaatttcaggtcagacacatgcgtccaggtgaggttgtcctggtgaatggcgttaagccacttctctttgccggtgggctgatccagcgatatgccgagtaccgtgaagttcttgctgctatacttttggaaggcggccactacattcggattttcttcccggcagggatgacaccagctggcccagaaatcgatgagtacatacttaccgcggaaatcctttagggaaacgggtttgcctaaagtgtcattctgcgtgaagtccggcgccatgctgccgatgccggtgagtttatttacacgtatgctgtgcgccagtcgttttgccgggccgttttctttcgcagcggcagacaatttattaaagatactttccttttcatccagcggcacgtcgttcaggtgcgacagcaacgatgcgctgataccggatttcggatgttgcaggatccattgtttggtgaggctgtcacgctcttcctgcatgcgtttcattttaggttcgagggctgccaggccggcggagtcctttgcggcgtataatttattcgcctgttcatagagggctgcctgtccttgcaacccgggcgcctgtttcagcagggccgtatattcgttgtaatcttttatgtattgcggacctgagaaagtggcattcttaaacataggtccatctccttttatggcgacgtttcctttatcgaggtagtaaaagatcatattattgtctccatactttttcccgatctggataatatagaaatctgcttccccgggggcgatgtttgttttgatggtaaacccgccggcagtggtttgcacggagtcgcggcggtcatcgttgccctgtgagcgccagtatacccactgaccagccggcagatctttgatggtagccgtgatggtggtgttttgctgtgcgtaggctgctgctgtagttaatgcagcagccagcaatgcggttatttttttcatacctgcgtagtttttactttaatatttcagccagctttgtatgcagtgcagtacctcttaattctttggcgatgatgatgccttgcggatctatcaggaaagaagacgggatcgcctggataccgtattcctgcgctacttcattgcggaagcctttcaggtccgacacctgcatccagggcatgccatcctgcttaatcgcttctttccatttatcggctttatcatcgagcgatacgccgagcacggtgaagtttttatctttgaatgtgttgtaagccttcagcacgttggggttttcagcgcggcaaggaccgcaccagctggcccagaaatcgagcaatacatatttgcctttgaagtcggataagcgaacgggtttaccatctacatctccctgagtgaaatctatcatcggctcaccgatcgcactctttttcagcacagcgaggcgtttggccaatcgtacgccggtagcggtttgttgtgccgccggcgtgagtatacggaacatactgtctaccggtgcatattctcccatcacggccatatctgccaccatgttcaggcttacggcgctttcaggatgtgctttaatataggctttggcgcgggccctccgctgattacgcagggattcgaggttcgcttccaaagccgctttggcggtatcgttaccttttacttcatcgtactttgagtaaagggtatcttcctggctggtgatatcggagatcgattttttatacgcttcgtaagcgtcctgcgtggcggagccggtgatctttatctggtccgttgaatccatatttccgttcacctgtatagcggcattttccacgaacaattccaggtagcgtgtggaggtaccgatatatattttttgcggctcggtgatgttgccggtccaggtgaagcggccatcctttaccggcaccgtgtctgttttagcagaatcggctaccggtatggagatgaaaacaacggagtccttcaatccgcgcagctccgccgtgatactggcggagggagctttaggctggctgcaggcggcggccagcagcagcatggcaaacatagtgggtgtgtggatcttcatactgaatatttaaaagttattattgttgatagcccgggttttgctcaccgatggtcgggttgttcaaaaattcggtgtgcgggatgggcatgatatatttcaccttatcatttgcggtgggccgcagttcctgtaccagcgaagatggaaggcgcagcagcgacatccactcctgtccgtcttctcctaccaggttgcggaccgtttccaggtacagttgtttgagcatttcattaacgcttccggcattatctactgcagaaaaatctgttacacccgcatggcccatgatgtttttcaggatagtacgggccgcagcgaggctgccgccggaacgtacaatagcttccgctttcagcaggtatacttctgttaaacggatggcataggcggtttctgttaaaggtgtgggcgtatttccttctttgatatatttcaggaagtaaaaggtgccatccgaataatcattggcggaacctatcatccaggcgccgcggggatcattcgccagcaatgttttcagcgctgttttggctacatacagggaagatgcaccgggccagtactggcggctgagcacatagtaatagctttcctggttttgctgtgatttaacaccgagtataacttccgggctggcaaggccttttgtgtaaaagatgtctttcatctgcggctccagcgtatactggctattgaggatgatactgtctgccagggctattaccaccgggtaatcggccggctggccgtggctcataagcaccctcattttcagcgccatggcggcccagcgggtagcatagaacgctttattttgtgccggcgcattggcaatggcatcatcaatatcagcgaggatagcggtgtagctgtctttcaccgagctgcgtgcttttgcggtagcgcccactgttacaaattcatcgcgcagcaatgcgccgtaagggctgctgagatcgaaccactggccgaagtaactgagcactttaaaatggccgtaagcccgcaggaaccgtgcttctgccaatacttcttttttacggttgttggtaaacgctttgtcctccagcagggaaacgccttttataacgccgttggcagcatttaccaactgataggctgaagtccagtatacgccgctgaaaaaggaattggtgtagtcattgagttctgctccatcttcgccataaccatatcccatataaccggcaaatacggcggggggcacttcgtgttcaaaccagtccgttacattattagtggcatccacgttggcaaagcgatagtaaacaccattgagggcgatttcagaagtacgctggtcgatgatggtattaccatctacctttgcattttccggtaattttcccagctcctttttgcaggaagttcctgctattaatagggtgccgagcaaagtatatatgatccttttcataaaatcttttttgttgttttaaaatccaaaacgaagaccgatgttaaactgctttgtagtgggaaaggtgcttacatccgagctgccgttgataaggctgtaaggattgttgctcacttccggatcggggccagggtagttggtgatcgtaaacaggttggtagcagatgcgtacatggaagcgtccctgatatgcagcgaggaagctactcttgccggcagctggtaggtaagcgtaatggattttaatttgatataggaaccattgtacacatcgtcgctggcagtgttgctcacattttccccgagcagcaggcggggcctgttgctatttggattttcgggtgtccagcgatcttttatagatactcccctgttggcatagctatcgaaagatttattctggatatctgcgagataaagcaggtctccgccgtaggagaacgtcagtaaggtgataagactaaaatttttaaaggtaaaagtgttggtgaagccgccaaagaagtccggctgcgactttcctatcacatcgcttttataaaatccattgtcgcctatttcatacatcggatcaccgatgccgaggtagggagccatgtaccgtgctaaggtgaattctttcttgtaatcgtccagttgcttttggttttgtataatacctttcattttatagccatagaagaggccgaggggttctcctttgcgtacgatgctgttcccctggatataggagctgacttcacctgcattggtgaaatcgtcgttgatgtcggttactttacttctgttcctggaaatattaagcgcgcctgtccactggaattgtttgcttttgatgaagtccgtgcgcaggtccagctccagtcctttgttattgatagtagcaaagttggagatcacactcccataagatgagctgggggccagttgtgtagccattaacaggcccgtggtatttttttcataataaccgatcacaccgcgcaggcgggagccgaacagttcaaagtcgaggcccaggtctttctgcagggtagattcccatttaattttttcatttccgagctgggtaggaacgagtgcgttcacaccaccgtaagaaccgggcgtatacaaagtataataaaggttatcaccaaaattctgtgtaccggtgtaaccgccactagctctcagtttcagttcatttacccaggttacttttttcataaagggctcttcagaaatacgccatgccacaccgccggaagggaaataacctacgcggttatctttcgggaatttggaggacgcatctgaacggccggtgaaggtgaacaggtatctttctctccaggcatagttagcgcgcatgtagaaactcagcagggagttctgcccggaaacaccggtgccgggtaaagtaatggctgcggaggaaaggttgttcaggtatttatcatccgggaaaccctgcccgctggcggaaaaggagttataacggtatttctgccaggaggtaccgccgaggaggtttaaccggttgttttcattaaactgtttgtcccaggtaagggtattttcgaagaagaggtttacatcttctgtttgtgactgtgagccgacgccgccattggagtcgtctaccccgctgggggaagcgataacggccgaactggacacatagttcagctggtggtagttgttgtagttaacagaaacagtagacctgaatttcaaatctttcagcacatcataatctgcggagagtgatcccagaagagaagatgtttttccttcgttgataccatccaggaggatcatcgggttttgatttccctggtagtcgtacccaccgatctgcgagcccaggaaccggtaatagctgccgtcggggttgcgttcaggcaaggtaggcggcgcaaagaatgcggccggataaataccattggtgatattatttttagtgaagccataatccaggttggtgatgatccggaaccggctggtgatttcattatccaggctgatcttaccggaaatacgggagaaatccgttccgagcaccacgccctgttgtttgttataacccagggaagtatagtaacgggagcccgagccgccgccgcgtacagagatatcggcattctgcgaggtagcattacggagtacgaggccgagccagtcggtgttagctgtaccaagactggaaggatttttaataatattatctgccttggtgctggatgcctgacctgcggctgcgcgggcggtattcaggtttacagcggcttctgttagcagcgagagataatccgttgcgttgagcagtttttccttgataggtgtgctgacacccgcatagtaattggcttccagcactggtttctggttcagcttaccttttttggtgttgatgatgatcacgccgttggctgctttggaaccgtagatagccgtggcggatgcatctttcaaaatatcgatgctttcaatatcattgatatttaacccggcgaggctgttcagtccgcgggagaaagaaccgctcacggtattattaggatcatcgctgccggctctttcaatcgggtttaccacttctgcctggttctggatatacctgttctggatggttacctgtacgccatcgatgatgtagaggggatcgttgccgccgagcagggaggtaccaccgcggatgcggatcttggctacgccgccgggggagccgtcggattgtgtaacctgcacacctgctgctttaccggccagggcctggtcgatgctcacgaaggaaacattctttacttcgtctacatttaccgaggccaccgagccggtgaggtcttttcttttagtgctgccgtagcctactaccacgtattggttcagatcatccactttggctttcagttccacctccacagtgaatttaccacccatactgagcgttttggattcaaagccaacgcatgaaatcagcagcaccgcgcgggcatctgtattatgcaggataaagaaccccgtttggtcagtgatagcggcggcgttgctgccttttacccgcaccgatacgccgggtatgggattgcctttggtgtccactattttgccgcgcacatcttccgggggaagcgcgtcgtcgttcgccggaggggttaccttccgggaaataacgatggtgttgccttctatatcgaaggttaacggcttatccttcagcagttttcccagtgctgcctttagcggcacttcccggatctctgccgaaacaggactcacatctgacaaatctttactccggtaaaaaaacacatacccggtttgttgtttgatgacgctgaacagctgctgcagcggcatatccttgcaggacaccgtgaccgtttgtgaaactccactggcacaaacgtgtaaagccagtaccgttaataaaactgcggtcattctcattactcgccagattttggtgacataattggtccctggttgaggggaccttccgttatcaagtgaacgaaccaatgacatggaaaacccatgcgggttgcgaacaacattaattttcataccttagattggtttttggttgacaaaatgtttctcatccgcctttgcaggcagtgaaaagctttcctgaaacgggttaaccattgatcaaaacctggtgcggacgccaatcttgacaccaggttttttttatggatgaacataagacctccgcgtccggtggacctcatcaattcataacatgatattactggatagctatctgtgcaggcgttagcaagcctggcaacattggttgtttcgctgacgttggtggtatcagctatggttggttattgatttagcttatggataaataatgatccgtcttccctcctctactttaaagttaatttttgcctgtgacaatacttttaacaattgttcctgtgtaagacttctccctatttccccggtaaatgtttctcccggtattttatcgctgtattttacttctatattataccacctggataactgacgcatgacggtagggatatctgcctcctcaaaagagaaatacccattcttccaggcgatggcgctgttcacatctaccctgcccacttttatgatcccgtcgccgctggccgtggcttttgcctgctgccccgggttcaggtgacgcatagcgctgcttgtttttaccagcaccgccccttccagcagggtggtattgatggtgctttcatctccataggcattgatattaaaatgcgtgcccagcaccattacttccatgttattgactttcaccgtgaaaggccgttccacatcgctggccacttcaaaataggcctctcctgtgatcgtcaccgtccgctcctttcccgcaaacgccgtaggataactgatagaggaggcagcgttcagccatacatccgttccatccggcagggtgattttatactgtccgccgcggggcgtgcgcaatacgttataagttaccgcagatgcctcggcttcctcgtttttatatacgatttgtccgtgcgtggttttctctactttactattcccttgtacagtgagtactcccgtgccggcgctgtccaggtttaccaccgttccatctgccagcgtgagcgtggctttatcgcctccgggcataataatcgccggtttatctgcgaccacctgtttcttacccgactgccacacatagaagctgctgcctgccgttaccagcaatatgactgccgctgccaccttccagccgctacggcggcgtatgggcactacgcgcggctctggcgccgttgccagcatcaggcgattacgcatccgttgttccatggctgtttcggtttctctttcctccacagttaaatgggctgttaaggcatgctcgtcataagcattataccatcgcagcaaacgatccttctcctcgtcactggccgcgccggcaaggtacttttttgacagtatggccagttcattcatttccatccgtgatataatttacagggtcctatatagtaatgtctggaaataagggtgctaccctacctccgtcaaaaaaaaattatagacatttttaaaaaagggcgtgaaagtagttgcggaattggaggcgcagtcgctgcagggctttggtaatatgcttttccacggctttttcggagatcttcagttccgtggcaatttcccggttgctcatacccatattgcggctataatcgaatacaatgcggcatttttcgggtagttgctttaattgttcctgcatggattgctggaggaaatgtaactgggcggtatcgtctgtcaccgcctgaacagcttcggggagggcttccaccgctgtaaccgggaccattttcgataattgtgtaaatacagcgtacctattggccgtagccaggtaggcaggcaacgaccggatgatagtttgcgtcctgcgctgccaaagaccggtaagcacgtcctgcaccacatcttccgccagctcccgggaacgcaggcgatcgtatgccagtacgtacaaacgtttccagtaacggttgtaaatttctgtaaaggcgttgtgatcatctttacccatcagctgaaccagctcatcatcagcatagtaggagtactcggtcatcatctcttataaaaatgcctgcaaaaattaatgattggttgatattagagattgttatgaacccaaagctaaggtatacggggatgagaaacaaggggtgagaggaaattggaaaattgttgattgaaagaaacagattaacttatctgtacatttaaacgctatatatactaaaatgagaataagaaccattacggtagtgttttcttttatcttatggggtattggtggctatgcccaaccagtagctgataaggtagatgctttcataaagtatgagatgagagaacgttccattccgggcttgcagatggctgttattcaacatgggaaaatcgtcaggatgagcaactacggtttcgccaacgttgaattctctgttccggtaacagatagcacagtattctccattaactctattaccaaggcctttaccggggtcgcaattatgcagttggtggaagaagggaaagtgaatattgaatcccccatttcgcgttatctcgacagtttacccctgacctggcaaaaagttactgtacggcaactgatgggccacatttccggtctcccggatattacagatactttaaccgatgaattgtaagtaaaaaaggagaagattcctcctgggtgaaagtaaaaagcctgcccctgtttttccagccaggtgaacgctttaattataataccaccaattacctccttttgggaaagctcatcgacaaattaagccggcagccgttcgtgagctttattcaacacagacaactggatgtgttgaatatgcagcaaaccacatttgggaattcttttgatgtattccataggaaagcgcctacgtatacttattaccataaagatgataaaggagaacttgtaaagcagaatcatttgatgcagacatacgaggaattcccggcttttttgttgactgacgcagggatgttcagtacagcgggagaaatggcccgttggattatagctttgcaacagggcaaactgctgaaagacaaaaaaagtattcatacgatgtggacgcctgtgcgtctcaataacggatctcttgacggttttggcggtatcctcaatggttacgcacttggatggccggttgtggaccggcccaggcaccctgctatagcgcccattggaggaggacgagcttctttatttatctatccccaggatgatatttcgattataattctaacgaacctgacaggatgcagcccggaatcattagtggaaggggttgctaagttttatatagctggttttgattaggtattttcaggttctttgtccttaaatttgcatgtcgactacaaaattcgacgtaaaaacatcataaatttacttattttacgctatatttgtaatatacttacataataaaggcataaaatgatagtcaattttagtattgaaaactttggttccatcaaggataagcaaacgctttcttttgaagcaactaaatcatcgcatcttgaaaaacaatatgtggtaaatactggtggagttaaattgctaaagctggctttaatttatggcgcaaatgcatcaggcaaaaccacgatattaaaagcactggattttttaagaaatatagttttagagcctgtagggaaaaaaacaaaggagttagattttcatccttttctttttgatagccaaacacctaaacaaaacgctgttattacgataacgtttattcaaaatgaaataagatactattatgaagttgaattttcccccaaggcaattgtagcagagaaactggatttcttccatcccaacaaagcgggtgttttcaaaagaaagacaaacctggaaaaccaattcacagagatcacttttggtggcaagattaaaatagataaaacttctgaaaagatattagaatcaaacactctttggaacaatactgtattgggtggctttttaaaaacaaacattgaattaaaagaattaaaggaggctacagattggtttagagaatatctgaaacccctgattcttacaactactgcattagaaggcgatgtaacgtcgcacattgacaacgctaacatctcaaaagaggatattgtgagtattcttaaaaaagctgattttaatatttcagatatactcattcaagaagaagaaagagatattcctgaaggtttcatcacatttattgaaaccaagttgaataccccaaatgataaaataaatgaactaaaagctaaaggcaggataacctcccgaaaattagcattcgaacacaccacagaagatgacaaaaagtatacgctgcatttcgacctggaatcgcagggtactaaaagatattatggattagctggcatactggcgctgctcattaaaaactcagttgcatttcctatagatgaacttgaatcatcattacatcccgaattgtatcgtcatttcttactttcatttcttttgaatgcagataaatctcaaataattgcaacaacgcataacagagaaatccttgacagcagggatatactcagagatgacgctatctggattaccgataaagatgaatcctgctcaacttcgttatattcactagcggactttgacagttcggtaatcagggacaccacaaataggctaaatgtctataaaagcggcaaacttggtggtgttccgcatttaggagattactacattgacatcgaaaaatgagacaaaaaagagctactgcaataaaggccaggaaaacatttgcggttgttgtggatggagatactgaagtgtggtatttgcaaatgctaaagagaaacgaaaggtccattaatgttaacattgagcctaagatacctcaaaggaaaaggctttcagaacaatttgagatggtaacggagctgtccagagactacgacaaggttttctggataattgattttgatacacttgcaagtgagacaaaaaatacccaaaaaggagtaaaaactcccgttcaaacattttcagaatatcgaaggaaaattaaatctgaacatgataatgtaattgtgatagttaacaacccgtgtcttgaattttggttattgctccattttgaacgtacatcaaaatattttagctcatgcgaaggcgctgaaaagcaattaaaaaaacatctcaaagattataaaaagacacaaaagtattataccaaacagaataatgatatttacttgcaactaaaatcaaaattagctaccgcaataaacaatgcaaaacaactgggatgttttaatcctgatacgcctcaaagcgcaatatcggagatgccattattttttgaagtaaataagttggggcagcttttttaagaatacccacaggcaatccccactccattttcttaaaaaacatatactattcagtacgcaatctttttattggatttgcattagcagcccggtatacctttgttccaataacagcactgcagcagagcaatacaatcaggaatgcaccgatgtaaggcgttgctccaatattagcatgataccggtaaataactccaaaaataaacttgttcgtaaacaagtagcccagcgctgaaccaaccacaaatgcaatcaggagaatacgtataaactcccggttgactaatcctataatttgcagcaccgatgcacccagtactttgcggataccgatttctttacttcgcttgtctatgttcaatgaaatttgcgcaaataagcctgatgctgacaaaagcaacgtaactatggccaggaaaaatgcaatcaacttaaatgcctgcgtcatccggatctccttttcaattaaatctgattgcaaatatccccggtagggtacattgggtatcaatttacgccaggctgcctgcaagtgctgggttacctgcgacaatctatctttatctgagcgaacaaccacaaacttatactccgctggtttggccatacgtaacgcacaaggtggtacaagaccatgtaagccgtattctttgtaatcgttcacaactccaacaatcgtgtaattgatgctatccagggtgacccggtgaccaagcggttcctttatctgtaaccgttgcagaaaggtctgattgaccaggatagattcatcggcatcagcgccattatcgtaaaaatgacgcccctgaagcaaacggattcccatcgtgttaagataggcctcccctcctacctgcgcgacctgtacctgggtttgcccattttcagctttggccgtctgggtgtaggtgccgtcaccaatttgctgcacacatccggccacgcttttaatttccgggtactgctgaatggcctgggtaaaaaccccgtactcccggggattgctgatctctacaaccgccacctcattgacagcatagccaaaatcgactttcttttgaaatagggcgttttgagacatcacaatgccaactaccaatgcgaagcacgacaagctaaattgtgagatcaacaggaaacgtgtaaaacggttggaagccgcaagtgaagttttacctttgagaatctgaaccggctgaaaagagctaacgtacattgccgggtacagaccagaaaaaatggcactgactacgggaattgataccaggaataaccaaaatccataatcccggctatagtcaggtgaaagttcaacgtttgtaagttgactaacagccggcaataacagatggacaaacaacaacgccaatacagatgccaacaggcataaaacaatattctccgttaagaattgacggattagctggctcctgaaacctcccattaccttacggataccaatctcttttaaccgtccactggcaaatgcgatggaaatattggtaaaattgaaacaggtgataattaaaataaacagcgacatgatggccggaactataacaagcacaccacgtggattaaccgttaattggttgccatatacgtatcccggcatgtcaatatccgaggtggtcgccaactcagagaaaggttggagggaaaagcctgctatgggccaattggaacgattacggttatgaaccgctacatagttattaagatcagccattacaaaacgggccgcctgtttatcctttaatttcacaaatgttgtaatgagatccggattggcccagtcgtcgggggccacctgcccattcacaaatccattatcaaatgaagtgatgatatcgaactggatacttgaatttgccgggattttctgtgttacagcagcaaccgtatatatcttagaacggccttcggatccaatgatcgtcaatgactggcccaccggaatttgctttggaaagtatttgtctgcaaaatcttcgctgatgattacctgatccggttgaccaaaaccggacagattaccggatttcagggggaaagtaaaaaaatcgaatagcgttttgtcagcatagtgaatatgctcatcgaaagtattctccttaattttcacaacaactgcagcgctactgaaccgggccacctgttccgccccggcaggttctttctgcatggcctgggctaaaggtaagggcacaacggcccagggctgcctgcttccatcaaccaaccgcacactgttcagccggtaaatttgctcggtgtgaacgtgattcagatcaaagttagctctgtagttatagttgagatatgccaggatacaacaggcaatagcaaagcctaagcctactacgttgaggaccacataaatcttgttgcgccaaagaacacgtaaagcgatcttcaagtagttcgagaacataaggttaatttaaaaagaccgttaaacagtttagttccatagcgccaacccggaaatattgaagtcagcgccggtattttacctgggcaacaactaccataccacttgttgcctatttgttcgccccgctgtggtggctatgtttgcctttctgtggcggatagtttaataagtaatatgtacggatacggacatacctgttcagttttaatgatcaattagcgaacctaatgggatgtagcccggaatcattagtggaaagggggttaagttttatatggctggtttaaattgagtagatgtcgaatggctcaggtaaacaataataattgtaaaaatcagaagtaaggcgttcagggtaatagttcaggaattattattcaactttttatcttccgcaatcttgtatagcttctcatttattttgtccagataaaatacaatatcatttattctcaatacccatctgataatcattatctgaattacgaaaaacaaaattcctacgatcaggaaaagtataggggcactgagattgttcataaatgtgtttttatagattgtttatataataaagtaataccccactccggaaaggaaagtactataactaatacagaaatctactaaaaatggtaaatgaggagcctttcacagtaattcggctatttgaggatttccaataacgagttaaaatccggatagctaagtatatgttagttatatcgagatagaaatacaaaaactatttgaattttgtattcactgggcaactttgacagttcagtaatcaacgacgcaacaaacagactttaaacctactggataatttcttgaacatttataataaataactattaagataatttggacttttcttttttgtattatattattgcgcccgaaatactatttgcaatgaaacatcttaagtacaagtaaaagcttcgttaatccataaggtgtaatttttcaaaccctatttcacgaatttctctattaacccggttaaaacccattactcaagtctttgcaattcacatatattttcatctttaaaacgctatttatgaagcaaccaatcgcagcatggctaattggatttactattcttatgtccagttgtcgaaaagacgaaccagcaacactccaaaagttaaattcaaatgcgttcgctaacgttaacgccaatacgatgacggaagattcggatgaggtaaccggtagtaagaatgatgtcgttgttggaaaccatgattataattggggcggccctggcatttactacagtattgtagacgggcaagtttcccaggtagactactactatggcaagctggaggttacagggcgttacaggacacgtaatttgcaggtaatggttacaatcccttatcaatatgactacaacagatataatggtcgtgtttacaaaatcggtcccgctgaacaaggtgacgggaatccagtaataagctttattggaactcctggagatatagtaggtacatattcatacggttctgtgggaacagttcaggcaaccagccatacgcagacactgcaaacgaatgggaatgctatttatggcgccagcgaaaaaagaaccattgttacatctgtgaacggaggtacgaaagttatggccggctttaatgccgaagttatagaaattggttcggaaattgaggcgggatttaccgttcaaagtgcgagaaacgaaaccggcgttcactctggggaagtaagctatactttaaaggtggctgtgagcggctggacatctcaataccctaattttcaaagaacagcaagtttaaatggtgcattctatggtacggttagagattaaatacctactttcagttatatttccggcgcttatttccaatagctgctctactgatcagtataatcaaaagggctttatcagtgagatatcccacacttccttttttgatccaaaggctggttggggcaaagtatatacctttaaacctatcggtattgcctatcagcccaaacagcagctcatgatcataagcaggttaaaggtcccagacactttgcatttgattcagctttcgaaagccgatcaagataaaatcacagcaaaatatggagattttcgtttcctgggagcatttgaagatcataatctcccttttgagctatcacacctgatgtatttaaatccttttaacctggatattttgcagatcgacagaatgactgcagatgcacaaggaactgagaaactcacacgggcaatactttacatgaaggatagtgtcaactatatgagagaaaacgcactttttgttaaacaaaacaaatagttttcttttcatatcggaataagaaattggcgataccggcaacgacaccgccagttaccaaaaagcccccgcagcacacgctacaggggctttccttatcattaacccattttatttaatttcctgtaacatctccttcactgccgcttccagctgggtatccttacccgccaggaattcttcataccgaagcggcaccctgatgtccggttccagctgaaggttttccgtagggcggccttctttaccgatagtgccaaccattggaataccgaataccatggttggatcgatctgtgtttcccaccaaacggcggttccggtaccgggtaccggcataccgatcagtttaccgaggttaccttgtttatagatgtatgggaagatgaatgcatcgctgtagttcccttcgctcatgagtacacagctcggctcctgccattggccggagggttcaccgcctttaagcttttcaccctgtggcgcaaactcaaggtattttttaccactcaggaagttgtacaggtcgtcgtgcagccatccgccgccgttgaagcgggtatctacaatcagggctttcttatcgcggttgcgacccattacttcatcgtatacagaacgatagctggcgtcgttcatgccttgtacgtgtacgtagcctacttttccgttgctgagtttatccaccatttcgcgggtattttccacccagcgtttatacatgagcgtactttcttcaccggcggatattggtttcacggtttcatcccagcgggctttagtatcagggttgtagatgcttaccaacacgttgttgcctgctttgcggttcagtaacgatgcccagtcggttttagcggtgatgttttcgccgtctattttttcaatgatgttacctttcttcagtttgctggaggctttgtcgaagggaccaccggcgatgatgtcatctactttgaggccatcgcctgtggaggtttcatcatacagcaagcctaaagatgcagtggcgtcgccattcatttgttgcggcgagtagcggccaccggtgtgggagccattcagttctccgagcagttcgcttagcagctcttcaaaatcatagttgttgctgatatgcgggaggaagcgggcatagttatcgccatacattttccagtcgatgttacggatcgtaggatcataaaatttctctttcacctgtttccatgcatgccagaaaatgtatttacgttcctcgtcctggttcagcgacagctctgtgctgatagacaccggcgtaattttgccgctgttggcgtctacctttaccacgctgccacggttaccgacaaagagcgtgttgccatctttgcttaactcgatgctgccgggtgtaccggctaacttggcgaggatctttgtttcaccggttctcggctcagtcatccacaggtcgtagcccttctcaaaagaggccatgtaatatagtttgctggcatctttgctcagcacgtagtcgctgatggaggcgctgttgatagtaagttttaccttcctgttttcaaggttattgaaatcgggatgaaatacttttttcgcgtcagcagaatccttggctttcagcgtggagtctttggctgctttgccgccggtggcttctttttctttcaggagattaaattcgtctttcgacagcttatagttatcataagcttcctggtcgaagaatacggcgaagatatctacttcgcggctgccttgtttggcaagtgatttacgtccttcgcgactgctggcccaggtgagcatttttccaccggcgccccatttggtaccgccttcgccaaaaccgctgttcacggggtaaacgaatgctcctttaccatcggcgggaataagcgtggcatttttcgtggtgaaataaccctgctggtcatctgcagctatccatttgccatcggggctccattcaaagctccagtcgccatccgagtaggaatggttacggcctgcgggcaataaggtgcgacttttaccggaggcgatgttgaataccttcaggacattgcggttttctatataagcaatttcttttccatccggagagaacagcggctggaattcttctgctgaggtggcgatcaccggttcttccttcagcagggtggcagcaaaaaagtaaggttcttctttgcgcactttggtagtttgaaagatgtcccagttgccgttgcgttctgctgcatagatgatgcttttgccgtcgggcgaccactgcaccatcctttcctgttggggcgtgttggtaatacgtttagtaagattgccttccacgctggtaacaaacacttctcccctggctataaatgccatttccttaccgtcggggctcatggcgaactcggtggtgttgccgctcacgggtacatttttcacaataccggcccgtccatcattaaagatgcttacttccagcttacgcggttgttcgccttctttcagcgtatatatttcaccgttataggtgaagcaaagggtattgttatctgctttggacaggttacgcaccgggtgtttggtaaaggtggtgagctgctgcatgctggctttatctgtgagagaacctttgaagaggttctgtgagataccgcctttttcgctgagataataaatatcgttgccattgccgaatacaggttccctgtcttccccaacatactccgataccttttcataactgccttttgcaatattcattacccagatatcgcgggtaacagaagatacgtggtgtttacgcatcggatcttcatatcctttccggtcctggaagatgactttatcgcctgctttgttgtaatgcgctacatcggctcctgcggcgctgagcagtgtggcgcggccaccggttaccggaacggtatacatgttccggaacaggcggtacggaaatcttacgctggcggcaggtgcgttgcgtgcgctcccgaaaagtacctgtttgttgtcggtggtgaagtcgtacggaaaatcgccggcgctgttgctggtaacgcgtaccggtgtgccgcctgcggcgggcatcacaaacacgtcgaagttgccataacgatcgctcgcaaacgcaatgaatttgccatcgtggctccataccgggagcatgtcatgggcttcatgaatggtgagtggaacggccactccccctttggtatctacccggtaaatatctcctttatagccaaaggcaatggtgttgccgtcgggagagatagaagggttcctgagccatagggcattttcctgggcataggcagtggcggccatgaggatggctgcacatccgaataataatctcttcataagcgctgattagatatctgttgttaagcagctaaagaaagctgacgcgccaatgtataaaaataaccgctttttatcaagcaggatagtgaccagtggttatttgaaggtaagacggataaaccgcgggcggtacaactgtggctgggcggccagctcatgaaggaaattgaacgcattgacattgtagctgatgagcagttcacccggctttgataagttggggtgcgccttggcgttatatacaaggaaatgcttgttttcctttgtttccgggcattcccatattttgatgaccggtccgaaaggcccggcaggactgagacccagccgcagcccgactacaggacttataccgtccacctggaagatgagggcataacggccatccttcaacggcgttacactcagttcattggaggcatgtgcggttaccgcagccgcctgttgaatgttcgccgtccattgctgcccgttccagtagcgccatcttccgaaatcctcgatatccgctggcaacacacgggctacgagcacttctttctgtaatccctttacgccataaacgtacacgtagccatccgggttgggcgcgcctgcccggcgggtattcacgaagatgccgactccaaaagtgatatgctgactgctatccaacggctgaaacaagggcgtatccagttggcggtggttggcaaaaggaggccggctaccgggcggcaatacaataagggcattgcctgtttcaacaaaaccgaaaacttcgctgccaatattgcgaatacggtatgctactatgtaagtgctgtttcctttttcatgattaacaaaaccgtcgcccagccagtaatagtcgcctttaactgcggcaggtgtgcggggttcaaacatcgttgcatccgaatagaagcggatatttttctccagcggctcattacctttcagcatcgccacggaattgtggatcatggttacatccgactgaagtttgccatcccggatagttccggtcatggtgtcgctgaaaagcagcagggtactgtctgccgcgccggcggtatctaccccattcaccggaatgctgaaaatgccatcgccgccaaaccagccggattggcggataaagagtgcattccagtcgttcgccggcgccacgctataagacaggtgcacggtatccctgctttgcaggggcacggtgtccaggcggttttccgcgcaacagttgctgatcagtaatgccagtagcgttatcatctcccgtaaatttaataaaaaaagcccttgcagtacaatatgctgcaagggctttagtcaaactatttattactaccaggcgcggttacgacctacataaatattcttcgcgttataataggtatctccggcggggccattgctgccactggagccttccatctgcatgttgatgataatatacatgggcttgcccacaaagttagccacatgcattcccttccatacgttgtcgatgtaataatgaatattcacatcggtagcgctcaccttagtgatccaaacgcggtagttatgccagttgccgggagatgatacactggttaagatactggacacatcctgccaggttctgaaagtattctgccagttggtggcgttccccttaaactccaggatatcgctttccggaggccagctgttaacgccggtaagccagaaggcaggccaggaaccggctacagacggcgcctgaaaatctccttttacttcccattcggggaactggtcgttgatcaacacctgtgctttagcatgcacagcgccactatggtagtgaatgggcagataagggtcactgctgctgttaccttcgttccagttgatgcgggcggccttaatagtaaggactcctgcattcaggtaaatgtgattatggtctgaactgctgccatacatacgtgcggtaccgttatgatccgatccccagggatagagatagttccaggccgcttcaaaggcactgtagctggcaaacgaactgttgtccagtacggtttcccaggtgagtgcagcagctgcctctgttttggccagcgctgcattttcaaccggctgaagtttgtcggacgcctgcttgccgcacgacaggatcacggagctgctaagcgccaataggattttcatacttgttttcataaagtggagtttttatggtgaataataaaatacttccctattttccatccacgcctatattgggaggtgttaacaacaatggggtcccatatagatcttttactgttttatccggcaatgcggcgcccttgtgcagggcaggcgaacccggttgcaaacgaaatgcttccagcgcctccatgccgtgcatgccggttaacggcgctgcccggaactgcggatcttttgaaaccgccgctttatcggccggccggttaagatgcctgccaaaataaaggttgttgctgtacacattccgtttgcttttattcatgatgtagtctgccgtgccgagggtataaaagatattgttggcaaaataggtactgtcggcataaccaaaccagttgcccatttctaccaatgtgctatccattttaatatctctttctggcaggtaaataacgttgttgtatatacgtgtatttactacggggccggttatatgaaaaaccggcgcgaagcccgcgtgtttaccggtggtgcgcaaaccatcgttcatgctaacgttgtaacggatgatggttcctttattgccgcagctttgcggagctttggcacttccatcgtcacataccagtacaaagccaccgtcgttatcatgactgtaattatattgtatcacggtattattgcagttccagtcggagtcgaatccttgtccatcccacggcgctttatgatcgcttacttcattgtattgaatcagtgcattatcgcagctccagggccatatgccggctgccgattctgtatcaggcaataagcgggggctgtcccgcatgatgttatattccaccagcacaccgtcgcagccggtaggcacaattccatcgccgggcacgccttctatcaggttaccgcggatcaccacatgctcattgggaaaccagtctgttctggaccagttgccgtttaccaggatgccgttgcgttgacaacgtttaatggtacaatctgccaccaggatgctgtcgaatttcgagcgggtgtgccggccgccgttactgaaaataatgcctgccccgccgccgtctttctttaccaggctgccgtttacatcatgcacatctacatttttgagatagatattggaagcaataccgtagtcggataactgcaccagtatgcccgcgcgatgtgccttcacatccgggccgtagttggaaatatccaggttacggatttcccagccttctgcgttcaacaggtataacgttgccggcattacgccattgccctggatgcgtggtttgtatccttctccatactggtcgatggtgatcagctgttgcgcgtggccgctcccctgcggcttcagctgcccttcataaatgcggcctgcgtggaagcggatctgatcgcccggttcaaaaacgtggctgttcacctgctgcaaactgcgccaggcttgttgttccgacaacccactattggtatccttacccgtaagggcatctatataatatgtattgggcacagcagcaacagcaggtaaacccgccatcatggagaataatacggcgctctgaaaaacctttctaatattcatttcagttatcttttaaaatacatttaccagcctggtgtttgcgcgagggcagacgatttcattttctccgcctgtggtatcggataccagtacatctttggttgaaacacccttccttccacttctgctttttcataagtaaacgtattagcgttcacacgggtgatgtttacaccatacaccggtgtattgaacaaggctacccccagttcccagcggcgcacatcccaatagcggtgttcttcaaaggccagctccacccttctttcattgcgcaccttatcgcgcagggtggcggtgttccattgaccagccagcaacagcggcatcttaacggaagcccggtcacgtaccttgttgatggcttcaagggctgttaagccgaaaccctgcggatcctgaccggggccatatgcctcgttcatggcttccgcataattgagatagatttcaccaagacggaagaggatccaggtgtgcacgctggttttattctgtaccaggtcgaggttttcatccacatactttttcaggtaatagcctgttttggtggcacggtctactcccctgccttcacggccaccggtaaatgcctctacggcacggcctttccactgcgagttattaaggatcacggtcatggctaaacgcggatcccggttatcgtacggatgcgctacctgagctggattactccagttaaaagtgctaccgtcggtcatttcataggcatctaccaggttttgcgtgggcgtggtgccactgccgccgccatcataaccaatgggatagttggcccgttcaaagccattgccgggtgcatagcggtgtgcaaaaatgatctctttgctggtggtgctgcggaacagtccacggtaatcattttccagctgatacgcattcaggtcaatcacctcttttgctgcctttgcagcggctatccatcgctcctgtaaatgtcctttgttattgaggctgctcgcataataaaggagcatgcggcttttcagcgccagtgctgcgcctttggtagctcttcccagatcgttatcgggaactgttaccgccaggtgcgcagcagcagaatcgcattccgaagtgataaactgcacgcattcatcgtaggtgttgcggggcaggttgaggctgtccgacaaggccagtgttttagtaatgagcggtacgccgccatagcgggttaccagttcaaaataaaagtaggcgcgcagaaaacggttttcataacgccagcgctccaggtcggccgtcatattgcggtaagtttgctgcgcggtggcgtcggggttcagcttatacatgttgaggtccacattaccggattgttccaggtaaagattggtgcggcgtatagccgtataagtggtattccagttatcgtccggatttatgtaggggttccagctgccgttattatagcgttgaatggcgctgccttcccaggtaaattctgcatcatcggtagctgcgtcgagcatggcattatccagccggttaaagccatcgggcaaaaagccataagtgcctataaggaagtcacgtgttctggcgtaggaagaaaatacttcatccttcgttagctccgtacttatctgcctgtccaggaaatctttcttacaggatgcggtgatgagtgtaactactcctgtaaaaaataaccaaaacttatatttcataacttgaaattttttgttgagatgatgatcataattgcacccgtacaccagcgttcatggaacgcatagcaggatatccgctgagtgtttcaggatcagcaaaatgaatatggtccagcgaaaacacattggtggcgttcacatacagccgtagttgctgcatccggatgcgcgacaatagcgaggccggaaaagtgtatcccagttcaatgttgcgcagttttataaagctgccgttgcgctgccagaagtctgtggagcggtagttgttatcattggctgcagtagtaagccgcggataagtagcggtagcggcagtttccggcgtccaccggcccatcgcaatgggcgctgcttttgcatcatttacaaaagcccataccagcgggccggataacataatgctgcggttggtgacgccctggaaaaatgcatccaggtcaaaccctttgtattgtacgcccaggtgcaaaccgaaagtccactccggcaatacaggtttgccaatggctacttcatcataaatatcgatgatgtggtcgccgttctggtctttgtatttgatatcgccgggttttaccggtgcgaagatctgttgcgggctgttgttcacatctgcctcatctttaaagaacccgatagcctgtaatccaaaaggctgcccgatgctttgaccggtgcggttaagataggcatagggttgttgtgcttctgccatatacaatattttattccgggcgaaagctgcggaggcagtagcaaaataactgaagctgcgttttacttcgctctggtatcccagttgcaattcaaagcccctgttttgtacgctgcctacgttttcggctggcaggcccacgcctatgtagccgggaacagcgccgtatctttccgccaggatatctgttctcttttcgtcgaagatatcgagcatcaggctgattttattattcagcagcgaggcatctataccaatattggccctgcggtctttttcccaggtaatgccggggttcgcgagactcccttcatccataccaccggcataatgattatccgtgccaaagtaatatcctccgccgctgttgtaatactggctgtaaggaaaccggcgtccgcccacctggtcgttgcccacctggccataagaggcccgtagtttcaggaagctgatccactctgcctgttgcaggaagtgttcttcagataagatccatccggcggatatggccgggaaaaagccaaagcgtttgcctttggggaaattctctgaaccgttgtagccaaaggaaaaatcgccgatgtattttcgtttatacgcatacgttatcctgccggcagtaccctgatgtgcatagggaacgttattaccggatatggtataaacatcctgctggtaaagtaacaacgcatcaatgctatgatcgccgaacgtacggttataggtaagattatactgggtgttggtgcgtctccactggtcgttcaccccatcgttttccacgatagtggtgttatcaccaaacttgttgtagatggtgtctcctgccgggttcctgagtagttgaaatacggcgaactgcttggttttatcgtcatttccctggaaccagttattgaaagatactgctgcaccggcttttaatcccggtgtaatctgatccaggacatagctgaggcgcatggtcgcctgcaggctgcgggcgtgcgtggtagctacaccacgacccagtaccagtcctacggggttaccgcggtataccgaggtgccgccgtaagagttatcgggattgcgtaccgggaatgcatttggcggtatcagcatcatattgttccatatttccggggcgccaacgccgggatagctgcgatcctccacccttccggccaggtccagtgaagtacttaagcgccgcgttactttaatatccacgttggagcggaaattataacgcaggaaattggcgttggagctttcttctctttttttatcggtgttcttatacagcccggtgttcttcagtacgttcagcgatacaaaataggtagcgttgctgttgccgccggtgaggttcaggttgtactccgacatgggcgcggacttcttcagcacttcatcataccagtttacatcgggatgaaaatatttatcgttgccgcttttgtaggcgtccaggtctgcggatgagtacttgtctgttttactttcattccgtaatgcctcgttgtagagggtggcgtagtcgtacgatccaaggaaatccggcagtcgctgcggacgctgaaaaccggtttgcgcgcggaaggagattttaggtttgccgttgaagcctcttttggtggtcaccagcaatacgccattggcgccgcggataccatacatggcagtagcggtggcatctttcagcacggtgatgctttctatttcatctgctgccagctgatcaaaaggactttcaaatccgtctacaaaggtaaggagtcctgaccctctgtacgaactaacgccgcgtatggtcatggatggcgcatcatagcctggttcaccgctgccctgcataacggtgagccccggtacacggccatacaggccattgctcagggtggcggcggctgatttccgtaacacgttgccgttcacccgtccataggcgccggttactttccaccacgcctgttctccatatgccacaggtacctgccgggaggtatccgctgttgccgaggcagagtcggcagcagattgtgccaatgccgcaacggacaatagtgtgcccgttgccgttagcaaagctgttctttttattttatatatgcagttcattgtttcagtattgaagtttacaatcgggcgtggcgttaccagcctgggttctggatcatgtattgtttgtagatttccacattggggaaaggatacaggtacattttatcgttccacaccctttgttcaaacactacctggtcgaaatggaattcactgctgccggtaataggcttcaatctcaggccatacatctttccgttcatcaccccttcgtcgccggcaattttccagcggcgtacatcccagaagcgatgttcttcaaatgccagttccacggtgcgttcatttcgtatagccgtcctcatttcttcttttgttttacccgaaagtgcaggcatgccggagcgggcgcgtaccgtgttgatggcagtatacacttccgtaacggggccctgcgcttcattcagcgcctctgcatagttgagataaaattcggcgaggcggaatacgggccaattgatggtagcgccgtaggttgaccaggtaacactgcggggcaggaacttatgcagccactgtccgccgccacggtcaccgccatgcagggcaggtttgccatctgttttgatgtacatctgcacggctcctatttcgctattccagttggcgccgttgtatcctattgattgtgcaaagcgcgggtccagcgaagcgtacatggcattggcgttatcgccggattccggccaggtttgggcaccaccggttttcttttcatacagtttcacgaagttcattggcacagaaataccataccatcctccgtacatattcaccggcatggtgaagttgaaatagtcgccataaatgccccaccagccgctcgatttattcgcgaggatgatttccgcgttatccggctgtgaccacacgtactcataattcttatctgcgccaaactcggtgatcaggcggcagctgccggtgggcgcccagtcgagcactgctttggcggcatccgcggccttctgccagcgggcagcatcgtagttatgatagcccaccaatgtagcggtagcgtcggtggtggctacatatggggtggcgctgttgaacaacgggcttgctgcatacaacagcacgcgcgatttcaatgacagcaccgcgcctttgctgatgcggccccggaggaaaccttcctgtgcaggcggcagcccggttacagcagcatcacaatcggccacgatgaaattgatacaatcttccagtttgttacgcggcagtttcagatcgtcgctattgagcaaacgcctgtctacaataggcacgccgccataacgcttcaccagttcaaagtactgcagggcgcgcaggaaacgcgcttctgctttcaattgtgttttatattccgcggtggcatccggcacaccgtcgatgcgctccataaaaatattagccttgcggatggctttatagtgcgtattgaaatcatcttccgggttatcgttggcgttccattgcccttcgttaaaacggttggcgcctggccagctgtccgcaatatccccttcatcacaggccgccgccagcacaccggctacgatgccgccgctgctcgaagtactccagccggtaggtaatcctgaaggcatgctgttgccatatacatcatacagaaatgtttctgcattcctgatctttgaaaagatagtatcttctgtaatatccacggatggcggcttctcaagaaaatcccttgtgcaggaaaagaatgcgcccagcagcagacttaatatgatatagtattttacttgttgcatagtttgtattttttagaactgcagattcaaccccacgttgtataccttttgttgcggataaaactggccgcggccatccggcgcttcagggtcgtatgttttcagggacgaccaggtaacgaggttcatgccattggcatatacccgtacgctgccgatctttgcgcgtttcaggatgccatctgtaaaggtgtagccaacttccacgttcttgagtcgcaggtagctggcatctttcagccagtagctggaacgctgatagttgttgccggcagggctttgcgacaagcggggaaacgtaatgttttcaccagccttataccgttcttcgttccagcgctccatgtgtaccgacattgcattgcgccagtcggtgtcaaatggccatgccgccatttgctccaggtatacggaagctttgccggcgccctggaacagcaccgagcaatcgaatcctttataggctgcaccgaaggagaagccataaatgatttgcgggagctgcgagtaaccgataggcatctggtcgtcgttgttgatgacgccatcaccattcacatctttatagcggatatcgccgggctggagggcatccctgccattggcgccgggcgcataggacgactgtggtctttttgcgtcattgatctcgtcccaggtattgaacaatccttctgccaccaggccaaaatactgtcctaccgggttaccggtttcgttttgataggcgtataagcgcggagcttcatctttaaattctattttattacgggcaaaagagtagttcgcttttacccagtagttcactttgccagcatagtcgttgtagccggcatccagttcaaaccctttgttgctaacccttcccaggttatacgctggcaggtcgctcactcctacaatgcccggcacggcgccgcgcatagccaggatattattacgtttttcctggaagtagtcgccggtgaaagacaacctgttgttcagcaatttcatttcaaggccgatgttggatttcttggctctttcccaggtgatatccgggttaccgagtttgccttcataagaaccgccataccattggtaagaggaacctacttcgccgaaattgtatccaccgccgtatgcgaaagaagaaggaaggtagaggaaccgggagccgccattgaagatatcggagagtttatcgttgcccacttctccataagatcctcttactttcaggaaagtgaggtatttattttttggaaagaaaggttcatcagaagctacccaacccagggagtaagcagggaaccaaccaaatcttttgccctcggggaagttttcagagccgttataacccatgttaaactccaccaggtagcggcttttgaagttataggtcacgcgtgccgccattccgaggtaggcgttgggtactttataggtgagcgtaggtgcataggctttactctgattatacagcagtaagccggtaacgttatgcgatccaaaactgcggttataatccactgccagctcaccatatattttgcggcgcttgtcgtatccttcgctgaagccgagggtggtttcttcgccctgcggcacatagaggatattaccggcgttggccgggtcttttacagcgaggtaggtaacgttgtttttagagcgcctgatagagtggctgtaccagctatcgtaagcgatggtaccacgggccgataatccagccgttataaaatccagtttgtggttcaggataacggaagaattcacattgcttttaaacaactgctggtagcctgcgttcagcatggtgagcagcgggttcctgccgtttacggcgccggagattataaccagcttaccatctacaataccaggactgctgaaaggattagccgacagcacatcgaagaagatatcaccggcagatttggccgggtaattctgattctctacctgtccgccgaggtttacttttacggtaaacagcggggttacatcaaaatcgaaattagagcggaagttataccgtttgtattttggattggcgctgaattcggggttatagtcggcatagcggtaagccccgttctgttcaaaatagccgcctgaaataaagtatctggccagcgaggtaccgccgctgatattcaggttgtgctgtgattgaagggaataaggtttcagcatcatatcaaaccagtcgatgctgggatgaaacacggggtccttgccggatttaaacaattccaggtcctcttccgtaaaataaggctccttgccgtcgtttttgagcgcttcatttttcaaggtggcatactcatagctgctcaccattttgggcagctgggtagggctttgccggcccaggttggaagttaagctcagcttgggaggccccattttgccgcggcgggtggtgatcaggattacgccgttggcgcccctcacaccatataccgctgtagaagaggcatctttcaggatattgatggtttctatttcgttgggatctatctggttgatgttggagcgttcaattccatccaccatgataagcgggtctgacccggagccggcatccagtgtgccgataccgcggatcttcaggctggaaccatcctggcccggttcgccgctgcgttgtaccgcaataaggcctggcaggcgacccaccagcatgttggatacgttggcaacgggggattgtaacaggtcttttgtaccgatggacgccacagcgccggtaacggttacctttttctgcacgccgtatcccaccaccaccacttccccgaggttcttttcgtccggctgcatctttacatttaaaactgctccgctgcccagcgatactttgcgggtaatgtacccgatacaggagaacaccagcacccgtttgccctccggcacatcgatgcggtaattgccatccgaatcggccgaagtggatttctgggtgccctccaccacgatggtagtgcctatcagggcgctgcctttttcatcggttaccttaccagtaatgatgacgccggccggtttaacggcggcaaaggtaaagagaggtaatgaggtcagggacaggaggacaacataagttatccgtaaaaaagaccgcacactacagtagctttttttcataacgttgggtattgacttttgagaatgacgtggctgtatgccccgcattacattggttgacaggggtaaaattcggatgaatcatcctgaatcatgggggagagattcgcctatttagggggagaaattgggaataaggcgctaatattcaagggattttgattccgggagatagcaattcgcatttctatctcccggaaatttatacctgcttctggttatcaaactttttacggtatttccggatataggcagatgggttcatctcgaacaccttacaaaattgctcccggaaatacttcatgtcgttaaatcctacctggaaggcggcctcatttacattgcacccggtattaatgagcagctctgctgctttcctcaaccggatgaaacggataaactcatttacggagtggccggaaatggatttcacctttttataaagggtggagtggctgatccctatttcgagggcgaacagtttgatgttgaagtcggggttatcgagatgcttctcggtaacagcaatacaacggtgcaggaactccttgtattctgctgatattttctggttgccggtgttcagcgtgatttccttgtaaaaatattgctgcagggtgttgcggctgcggataatattggtaatgcgcgctacgaagaggtctttgtcaaatggcttgctgagatagtcgtcggccccgccttcgatgccttttaattttatttcgggagaagagctggccgtaagcaataccacagggatatggcccaacgccggatccgactttatctggcggcacaattcaataccgctttgtccttccatcagcacatcgctgataatgatatcgggcaggtggcggctggccagctggtagccttcccctccttctgatgcttcataaatattgaaggtagccttgaaaatgcttttgatgtagtcgcgtatctggccattgtcgtctacaatgagcatgctggggcggggcgacaacaacacgtccagggtatcttccgcagcagcttcttctgcttccatcagtgccaggtcatcttcttccaccagttcttccaacagggattccattccggcggcttcttcaaaaatcgtatagccctgcaggtggtccctgcccttttgcagggtaatcgtaaaggtggtaccgttgcccggctcactttcatatgccacggtacctttgtgcgcctgtacaaattttttaacgagatataatcctataccgaagccatttttcagggaggtatctttttctgatacctggtaaaagcgttcaaagagttgattgcctacctggccggggatgccacaaccactgtcggcaacacggatgacaataccttcggggagatctgacagcgaaaaatggatgctgccgccgtcgggcgtatatttaaaggcgttagacaacaggttaaacaaggccacttctattttctcgcggtcggcgtatgccattacctgttccgcgttacaggtgaagtcgaactgcagtttcttcatgcctgcctggtgagtaaagcagaggtacacttcccggcagatagcggccatgtccaggggcacaattttcagctggtcctcttcctggtcggcctttctgaacagcaggagctggtctaccaggctcagtaagcggcgggcattgcggtatacgatggtgaggtccttgctttcgatttgcctgccatcgctgtaaaggagttcttttacaggattgatgatcagcgtgagcggggtccggaattcatgcgacacattggtaaagaacgagagccttttttcatgcacttctttttctttttcagacctgatatgcgacagttctatttcataccggaggcgggcctgcctgcgctggtaaaagcgataggcgtataaaaggccgccggtgagcaaggcatatatgatgtatgccagccaggtgcggtaccagggaggcagcactttaatttttatgatccgttcctgcggattccagatgccatctgcattggtgctttttatacggaaggtgtaattgccttcatgcaggcgggtatagttggcggttcgttgtgcgttcacatagttccagtcgttatcccagccctccatataatatgcataggcaatcttatccggggaagagtattccagcgctacatagtcgagggaaaatacggccttatcatagggcagcaccagttcatcaagataacttagcgactggtggctgcttttggcatgttccggatcaaatggcgtgttggaaatacgtagccctgcgataagcagcggcgggaagtcgtttttttccgcgatggcggcagggtcaaaaatgttaaaccctttgatgccgccaaaaagcagttctccggacgacaggcgcaatgatgcgttgtagttgaactggttgctttgcaatccgtcggactcataaaagtttttacattgcctggtggacgggctgtagcggcagatgccgttgtaggtgctcatccacaggtttcctttgttatcttcttcaatattcaggacagcgttattgggcagtccttcctgttctgcgatggtagtggttttaccggtgcggcggtcaaactgcacgagtcctcctccttcggtgcctatccagaaatggcgggcattatcttcgcagatcgcccggacgttgaagtccatattataatactggtgctgccggtttttcgtgtccgcttttatgagcctgttgaaagtgcccagccaaaggtcgccggctttatcttccgcgatggtgataatatcgcggaggccgggatcaaaacactcgaagcggttggcagttttgttcagacggtagatggtgcctcccatgcaggcgcccgcccataggttatcctgactgtcgagatagagtttccagatgaacttatcttcataaccattaagactgcacgggtatttttcaaaggtatgcgttgatctgttgtagcggttgattccgccgccgaaggtggccacccagatattattatcctcgtcttttacgatactggtaacattattattactgagtgaaccggggctattggctttgtggacaaaggcggcataggtgttttgtttccggttccatacagagatcccgccgccgtcggatcctatccagatatctttattatcatcttcacaaaatgaaaaagcaaaattcgctgccgggctattaccgggtaagggattgggggtgatggtagtaaaccgggatttctgtttatctataatattaatgcctccgcgcagggtaccgatccatttgcgttggtcacgatcttcatacaccgcatacaccgcgttgctggtaagggaagatttatctttaccggtttgaagttgccaggcagtatctttttgtgcgggcataacaaaaataccatctccatcggtggcgacccatagctgccggctggcgtcaatcgttaagctgatcactttactatcctgccggcgggtggccgctaatgaccgggaaaggttattggtggcgggattgtaaaggtaaacgccttcgtcggtgcccatccataattgcccggacgcatcagcgatcaggcaatttcctcttttctgttgtccgtttaccaggatgatctgctgtttatcttcatcatagcggcaaagtcctacgttttgtacaataagccagcattgcccgcgggtatcattcacgatagcgggaacgttgttgttgacaatggtattgacacctgccagcgggatttgccgggcgaggttgccagctggcggataaacaaggagaccatgattggcggtgcccattagcaccagtcctttccggttggtgacgatggtatatacttctgaagaaacgggcagggtatcgccttttgtccagctgcggtaatacaccggctggaatacgcctgttggactattcaaccggttcgcaccatgtttggtacctacccacatatagcctgtagaatcttctgcgatggcaacgatgcggttattgatcagggagttcggcactttgagctgctgccggcttactttgaagctatagccgtcgaaacggtttagtccatcgtaagttccaaaccacataaaaccataccggtctttatgtatgcaggtaacggaattattggacagtccccgctcaatgccgagatgactgataggctgttgctgtgcccgcgcttcactgcgtatgagcagcattgccacgaccagggatattacgctaaccagaatatgagtacgtgaattggtatagatcactgctttcttctttgaagatgctgtttaataggcctcttcaactaaggtagcaattaaatgtaaacctgacaataatcggatcccctaatttccggcaatgccgcgtcagaacatggtaccaaacacgcggtcccacagcgtagagcttacgccaaaacccagttcctcgtttttatagtgatgcaggtggtggttacgccacaagggcttcagccatttgaaaggtggcgcccaggcgtggatggcgtagtgcatgcttccataggcaaggtacccggaaataaagcccgggaaaaatacccaggcggcgttgtgcatcagtaaataaaagacagcaaaaagaaaggaagaaatgataaggcttggcacgggcggcataaacagccgttggcggtcgcgcggatattcatgatgattgccatgcagggtataggtgactttcctcgccagcggatgttcgctgacccagtgaaagataaaccggtgagcgaggtattcaaagagtgtccagccggttacggcggccaggtaaattgcgccaatttcccaccaggaataatgtaatgaagtgcggctgtaatatatcatgtagctgattacgggcagatacatcccgaagataatgacgggatgggtttttgtaaggaactccaggtacctgttactgaaaatctgcgcctgacctttgttgtgcactttttcaaatttcatatgcggctgttttatgcgtagcatccgccgtaaaaatgcaacagcaaaggtttacggccatctattttatcatgagctgcggatttaaggggttgaattgttgaaaaaaggggtttacccggaggagcacaaccggctattattacgtttgaatttcataactttggcgctatgaaagcaaaggaaagtgtagcctccttttttgaattacatggaaaggaatatccaagtggacagttcagtgtaaaccggctggaggaatttggctgcagtgctaccaatttgccttccaacaggagggatttttataagatctcgctcattatacagggcggtggtattttatcttattcagataaaagtatccgtatagaaggcgcctgtctttctttcatgaacccgatgatcccttactcctgggaacccactaccaacgtgcaaaccggctatttctgcctgttccaggaagactttatagatgcgcatttgaagaatggaagccttgcgcaatcgccgttgtttaaaaccggcggcaatcacatcttttttcctgataaagagaaaatggattttctgcggcagatatttgagaacatgctgcgggagatgaattccggttatgccaacaggcaggaattgcagaaaagctatgtgcagatcattatgcatgaagcgctgaagatgcagccacctgaaacctattaccaggcgggcaatgcctcccagcggatcagtgaattatttatcgctttgctggaaagacagttccctcttgatccgccccaccaggtgatccggctgaaaaatgccaatgagtttgccgaacatttatctgttcataccaatcacttaaaccgggcgttaaaggaaaccaccggaaaaaccactaccgagtggatttcggagaaaataaccgccgaagcaaaggcgctgctgctgcacagcaattgcgatattgcggaaatcggttactgcctgggcttcgagcatgcttccaacttcaacatcttctttaaaaaacaagctggtcaaacgcctaaccagttccggaaggcaactgtttccatttcataactacctgtttgattcgcataattccgggcgtacggtgccggctatctttgtgtcataaataaaaatatatggcacaggaagcattaaaagacaaagtagccctgattacaggaggcactaccggtataggtttggcaacagctgaattatttctgcgcaatggcgccaaagtggtgattgcaggacgccgggaaacagaaggacaaaaagcattacagcatttacaacagatcagttccgatgtacattttattgcggccgatgtgtcgcagggccctgttgtgcaaaagctggtagttgataccgtgactcgtttcgggcaactggacattgcctttaataatgcgggtattgaaggccggtttgggctgattgaagatacaccggaagaagaatttgataaggtgatcggcatcaatttaaagggtgtgtggttatcctgcaaatatgaaattgagcaattcaaaaaacagggtactggtggggcgattgtaaatacttcgtcgtggctggcccgcggagcgggagctggttcgggtgtatattccgccagcaaagcgggtaccgatggcctgatccgggcgctggcgattgaaacagcggcggcgggtatccgggtaaataatattcagccgggttatatccacacgccgatgttcgaccggtttttccctacggagaatgcggaagctttacaggagccttttaagaaacatgcgcctatgggccgttttgcgaaacctgaagaggtggctgaactggtgttgtggctgagcagtccggcagcatcgtttgttaccggggagagcatcctggtagatggcggtttggctattggcggtcaacggttataagcatcagggggctgtctttaccggcagccccttgttataccagcatcgacggcgccacgccaaacgtctttttaaaagcaaaagaaaaatgtgacaggtcttcaaatcctacttccaggtatacatccgatatttttcgtcctttttccttgatgagatagtaggcttcctggagtcgtttctgttgcagccagcggctgggcgaggtatgaaagatcttttcaaaatcgcgcttaaaggtagccaggcttctgccggttaaataggcaaagcgtttcatttctacattgaagtgatagttttgctgcataaaagcctccaggtctattttacctggttctgtaaaatcgaagagaatatttttgagtgccggatctactttcagaaggatgaggatggcctctttcagcttcagtgcaaacaggtgatcgttgcccggttcattcagcttctcgtaaggctgtaaggaggcaacataactttgcagcagcagatgggctttcagttccatcacggtttcgctgtccacctgtttatccgctgcatagccatattccatactgaaattacggagcgtggtttcatcgagataaacggagattgttttaaactcaccattttccggtggttgtttgaagaatttgagcagcttattccgcctgcagaaacggaaagttccctcatcaaaagtttgattgcgttgtccatcgttgaatgtgatggcgcccgcgatctggtaactgaaaacgtgtaccggaacaaactgttctccttccctgctcctgtttacgtaacaggaataaacaatttccttcgacataatattatagaatgatggttttcggttctacatattcttccaatccatatgcgccaaattcccttccgatacctgactgtttaaatcctccgaagggcgccagtggatcatgatgcagcgtattaatcagcacccgtcctgctgcaatttttcctgcgatatcccttgctgtcttttcgttggatgagctgatgtacgccatcaggccgtatgttgtatcattagcgatatcgatggcttcttcgattgttttgtaagtcatcaccgacattaccggtccgaatatttcttcgctggcgattcgcatgttccgggtaacgccggtgaacacggttggttgcacgaagttacccgcttccaatcctctgggatgtcctgtaccgcctgtcaggagttctgcaccctgatcgatgcccagttgaatatactgctgcacgcgatcgtattgtttcctgctcacgagcgggcctatagtcgttgttttgtccatagggtcgccaactttcacgtttgccaccgctgatttcagcaggacttttactccttccagcctggcttccggtatcagcagcctggtgcctgcgatgcatgcctgcccgttgttcataaagcaggcggctacggccatcggaatggcggtactgaaatcggcatcatcgaggatgatattggcggatttgccgccgagttccagtgtaacccgtttcatggtatctacggcgccgcgtgcaatcatttttcccacggctgtagagccggtgaaagagatctttgcgataccgggatgccgcgtgatttcggcacctactacattgcccaggccattgacgatattgaatactcccggcggcagtcctgcttcatgaagcgcttctgcgacgatctgcgtttgaatggcgctcatttcactcggcttgataacagcagtgcaacctgccgcgacagcggtagccagtttattgcaaatatagctggcattcgcattccagggcgtaataattccaactacgcccaatggttccatgaccacatccgaggtgcctgctttgcgggtgaaggagaaatcttccaatacttttttatagtgaagaaagctatcggcggcgagttgattgctggcgagggcccgttgcgcaggggcgccgtattcgatgatggaggcttccaccaggtccggcactcttttctgcatggcgtcgtgtaggcgttggaggtagttgctccgttgttgcaccgtagtttttgaaaagatagtaaaggcggcttttgctgcggcaacggccctgtttacatccatttcatcccccagtgctactgttcctatttgttgattggtgctggggttgatgagatcgaaggtagtggcgccatgtggtgttacgaaggcgccgttgatatatatctggtctattgttttcatgttactcggctgtttttgtggcgaatttatctgctgcggttgttccgaagaagtcgacagcatcatcgtgatcagtggaagtactaacgggcagccacttttcaaattccgcttgtcgcgcggcatccgcctgttttaaaatccctgcggcttcgctgcccaggatgagatgcacaggtggggcgggatggtttgccagatccaccattactttggcggctttttcaggatcgcctaccggcacatagtttccttcgcggagatattttatcatccagccaacggtaggttcataatcttcgatgggtgttgcgaaggtcatggatgcgccgccccagtcggtgcggaatccgcctggctctacagatgtaacgaagatgcccagcggtgctacttctttggccagggcttcggtgaatccgccgaggccgaacttagccgcctggtagatggtgagaccggggtttcctacgcggccgcctatggagctgatctggaggatgcggcccgcgcgttgtttacgcatgtgcggaagaactgccctggtgatagcgatgggtgcgtagaggtttgtttccagctggctccgtacctgttcttcggtgaaggcttctgcggcgccggtgataccaaagccggcattgtttaccagcacatcaattttaccaaagtgtgtgatggctgtatctattgcctgttggatctgttggttgtttgttacatcgagttgtaggggaaggagctggccggggtattgtgcggcgaggtcatttaattgtgcgggggtgcgggcggcagcggcaacctgatcgccctgggcgagcactgcggctgtaagactgcggccgaggccccgggagcttcctgtgataaaccaaacttttgtcatgagtattgttttttgtttagacaaaggtcgggtggaaattactgccggattttgttgcagggctcaaatatagtttgccaggaagctcaggtatttcttattttttccagtactgcggcgctgccttttcccagtcgccttattattgtgatagtttccgatacactgataggcaggtaacggacatcctgcttctcccgggcacagatggtaccagaagagggagtgggcgccgaaggaaagaatatagagcagtagtgttctgtttcatctaccacaaaacaaatcacttcattaccatctatcagcacagcagccggcttccagttagaagcctggctactggtaagtttgtcggtggatagtgcctgcagataagaatatcctggaatatgtaccaggatatcatcttccaggatccttttaaaacggcgggcaatgccggtgtgcataaagatccctgccaggaaacaaagcagcaggagaatgaggatggttagcagcgtttctttcccgatgccggggacctgaacaggtagcttgtgtgcaatggggaccaccacccgctttatgaggctacctgctttcacaattactgctatcagcacaaacaggggaatcagtaacaacaaccctcctacaatggttatttttatatagtggaagaaatttttcattgtgcaccatcttctacctgtactacttcatactggcttttgccgtcgagatttaccggctggtaataagtttctcctactttgacgtaggtttgatctcctacttttacttcttcgccaccggcgggcaggttttgcacaacggctcccgcaggtggagatacaacggtatacttgctgccatccttctcgtaatatgctccgccgtaatagtagttagtaacattatttaccactaccggttgcgcgcctgaaggcaccgtagtgatagtagctcccaccggcgcctgtacaacagtgtagccattattggcctgctgataccacacgccctggtcataatgatactttgcattattgatgctcacgatgatagcggtagtagccagtgtggcgataaagaatccccatggatgccatactggtccccaggcatagggcctgtaggggtgataatagtaaggatggtatgaataatatcttcgtccgccgtaagcatatggcggtctgcggtaggtgttgatattgttgcgccttacgaccgtattgcgattgttatgtacattgatatccctgctgttatcgacattgatatttacgtttctgcgactattattcacgcggttgccagagttattgacacggttacctgagttattccggttaatgttattccggttaacggtgttgttttgcggtcgattggccggtcgtgtttgctgccgcgtgggccttgctgtttgagcgggtcttgctgtttgtgcagggcgggttctggcgggtgctttctgaggtgtacgtgcgggcctgttccttgctggtgcagctcctccccgtctcctttcctgagcaaggccctcaaatggttgtattgcagtaaaggaaataaacaataaccatatggtaaagttcctgatagctttcatatgtgtggtttaataatgagggaaatgttattttcagggtaccgtccttttataacaccggaagtgatcaatttgttaacgaggttttgcggggggatgtaaatcagggagaagaacagcttcccgttttcccccaccctgaaatggatggaggaaagggagagcctaccacttgattgcgcgcccatgcaaccggaagtggcaaagtgggtggttggttgggttatttaatggatgaatgaaattcttattccatgcgattgcctccttcaatatatggtattgaatcaatgtcctgtcaaccggaaataaataatgaatgtagcgactacgggatttcgttttttaacagataatggatttgttgctttgataatgtttggtaattatttagcgcttcgggatcaaaattaggggatttgttttgaatttttaattgataattatcaagaaataaaattgataaatatcaataatcagcgttgataaatgtcaataaatggcttttattcttgagaaggtttcctgtgtaatccccagataggatgctatatactttgaaggaactctctgcgccagatcggggtaattctgtataagaaattcgtatttttcaaaagcagtttgctttctgattgccaacaaccgttcttcacttttacaatagtagtgttcagtaagcttccttccaatgatattaaactccagggaatttgcatacagctccatgaggtcatcatatgtgatgtatattagttcacagctttccaatgcctcaatggattcatagcttttaattctcctaaaaaaagacaaaacggaaatgataaagtcattctccatcataaaccaactggtaatttcctcgttatccttttcataatatgctcttagtaatcccttagatacaaaaaagagattatcgcaaacatttccctgccataatatcgtctgttttcttttaaattttgcaaactgcagtttggcagatatttgtgatttcaactcctcagaaacaggacctaactgtgataataaagcgaataaggtatccattgtggttagttattttgaggtagcaataattttagtgtctaaatataatgaaaattaagtcaatacatatatttgacatatatcaattttttgaataaaggaaataatttaaattgataagaccaaaatcaagatcctaatgaaacctttttactactgtttagcttttctcgtactcatatctggctgtaaaagaaaggacctcggattttcaaacaaaattactatttcagaggcaaagcaaagctacaacactacaaaattgacatttgatttgaaaaattctattggtttgaatgatagccttcctaaagacttaaactgggaagcttgttatgaaagacaaataagtggagaatcttgtttgatattagacattcacccaacttctaccaggcaaatcaaaagccaggacaataagcattcctctaatgtcgaaaggtatcttttattccgcaagaataagagtgggactgtggttttcgagcttgtaacattttttgtcaatagcgatgcacaaaacagcctgtcaattctcgtctttgataattcaggaagattgtcaggtaactttgtttcggacggtgtcaaattattccccacaaatatggataccattcgctatcaaaatcacgtaacaagaatgccgggaggttctttgtgcgttgaaacggattggtatacatgcttgtcattcaggggagtaagctatggatgtacttacaattatagcacccgtcaatgtgtagatataccggacaatggcggtggagcgcctataaacaatcctattgacccaataggtagcgccaattttgactataattccgttccagctataaggtttacaagatggatggttgcaccggctactgatcgactaatcgctgatcttaaaaaatatttcggctgcttcaatataaatagtacttcgacttacaatattacattgtatgtaaaacagcctatccccaattcccgcgtcattgtttccgatggttatggaaataagttgcctagctcattagatctcaattctttgagtgtaggtcacactttcctgggattttctcaatctggaggtgtatcaacaacggttagccgatatgcaggcttttacccgtcaacaatggtatcgccttttctacctgaaactcctggtgccattgctgataattccaatactgcatatgatgtttccgttacattcaaggtatcaggtgcccaatttaaaacagcaatggagcaatttgcagcagcaacaaaaggcaactataatttaaactggaataattgtacggatatttgcatctctgccttaaatatcatcggcttaaatgtgcctaaaacaattggtacatggccattgggacaaggggccaaccccgcagatttaggcgaagatctcaggctatttaactccacatccatagcacaaaaaaatctcacaggtgggacatctccctccaatacttttcagtgtaaataatcaccactatgaataacatcatcttatatcttttagcatttctttacttcaatacaaatgaacaacaatgtgtcaattggaaggaagcccgtacgttccatttttataatttacccagaaatgtcaccacagaaagaattaagtggccagatatagaaaaattaaaaccagtaaaaataaacaatgctgcacgaattttgagtaattcagaatgtaaagaacaaacaatggctatctggaaagatgaatatttgctcattgtagaattcaatgacggcaaaaagagaaaattcaaagtaagtgggtacggcggcttcttatatgagcccggaggtaaattctactttgttcaggaaaaagacagagacgaatggcagtctgttatacaagcgttaaaagcccaaggtctaccagacaattaaattgatcgaaaacacacgcatatacttccaacatcaataatcatcaacacataaaatctacacatttacgatataatcttgtaattttatcgctaaaaaaatatagattaacatgttagccctgtgttattccacaaacagagaataacagaaaataatctcaaatgaagaacctcttgtaccgggtcagcttttctgccatcacccggatggtattgggtatcgctcttttgttcacagaccagttgtctgtaacgtttagatatcttattgttgtcatttttttattaccggtgatcaggtatattcttcatgcgtggcagcaaacggaaatggacgtttttttcgccggctacccgaagctgggagtagtcagccatttttttatccttgccggcatagcagtgttgtatgtattggtgttagcacacgtacttgagatttacactacctcctatttctggtggatactcatcatcattgcacctgcgataggctggtatcttttgtttggtaaggatcctgttccaacagaagtacataaatataacaaacgggcattgctgcgaacattggccttttacatcattccctttttctttgcccttaattatgcattcgacttctctacgcccacgattacaagatattacatcacccgcagcgatcatactactcatgtctttaacgatccggatatcagcgaaatagacatctattacttttacctgttgcccgcggaaagtatgaccggccccacgcgctggcagaccgttcccgcaaatgactactatggcgttaaagactatggtccttacaaaggcaaggatagtgtaaactacctcgtaatggataagtggaagggacgtgacagcgcagcagtgcctttcagggagcgtttccagctcgaattactccctacaaatgtattgcctgtacggcaaactgttcccttcagcttatacaagcggtttaaagatggagattatctgaataaagaagaacaccgcggcctgtttggaattcaatgggtcagctatcattaatttgtacccctactccgccttcaacgacctcacaggattcatcctcgcggcctttagcgccagcacacctacggtaagtaaagcgataatcaccgcccccagtcctgccaggccaaatgtccaccaatggatatccacccggtaggcgaatccattcagccagcgatgcatgctccaccagcccagcggtgtagctatcaggatggcaattaataccagtttaataaagtcgccggatagcaggccaacgatactcgtgatagacgcacccagcactttgcggatgccgatttctttcagccgtttttcggtggagaaagtggccaggccaaataaaccaagacaggcaatgaatatagtgagtgtgccaaaagccgcaaagatttctccgaagcggaggtctttcagatattgttcattgaaagcctggtccaggaagctgtatttgaatggcctttgtggttccagctgattccatgtttgttccaacgctgaaatagtcttgtttatctccgttgttttaatgcgcagggaaagcctgttcaatgcatcggagggcgccattcttaacgccagcggctctacttttttatgcagcgactgataattgaaatcttttacaacgccgataacggtgcctttacggccccattgctcaaagttcttcccgataatttcctgcggattggcatagccccattgtttcgcagcagcttcattaatgatcatcgactgctccaggtctgccgggaaatcacgggagtatgccctgcctgcggccatctttatttcatatgccggtataaaatctgcatctatttcatacagccccggaccaaaaggctgcatttcaccactgggcgaagcaataacggtatgtgcgttgggaaaaaattctcctggcactgcacgggaagctgttatggctatcaccgccggattattggctagtgtggcctttacggcttctatgttcttattcacttcattatcgccaccatagtcaattaccagcatctggtcctgccggaaacccaggttatgcgaccgcaagtgatcgagctgggaaaacacgatggccgtacaggcaatcagtgcaatggataaagtaaactggaataccaccagcccctttctcagctggatacccttccctgaggaataaaattttccttttaacacaagggccggcttaaaacgcgacagcaccaacgccgggtaaataccggcgggaatccctacaaaaaaaggcgccagtattaaaacagatatcatctgccacgacagcaggtcaacaaatggcaacggctttccggatatattacgcaccatcggcaataaaataaataccatcgcaaatgccagcacagtagccaacatggaaatcaccacagcttctacaaggtattgcagaattaaactctgcggatgagcacccacagcctttcgtacgccgatctcctttgccctttccatagaacgcgccgtagtaagattaatgaagttgatagccgcaatgaaaagaatgaaagcggctaccagcgaaaaaatatacacatttgacaaactcccggtagctccgggctgccgcattgcctccgaacgcagataagcgttcttcaacggttcaaaagcaatagcatagttgctttcattgggaatatgccgttttaagaattcaggcaacttccctcgcatcatgttgatgtctgcattttcattcagtaagaaataagtgtagaagtcaacatatccccattcattaaagatctccggcctgaagcgataaaaagtactcatcgacaataatccggaaaacgtaaagtgagaattggaaggcacatcttccatcacacccgtaactgttaaaggattatcctgatcggttttaaatacctgccctaccgggttactatctccaaaatatttctttgcagtactctcggttagcacaatgctgttaggcgcttttaacgccgcttcccggttaccatatatcagcttccagctgaagatatcaaacatggtagaatcagcgaatgtcaggttgctttcctggaaccgcttatcgccatgttgcagtaacagggtgatcggactggtgaatctggctgtcatttttatttccggaaaatctgcctgtaaagccggcgctactggcgcattgccccatacctggtattctcccggtgctggtgggggcaacttctgagcagatttttcgcggtacgcatgcagtacccggtaaatttgatggtaatttttatgatattggtcatacgacaattcatccttcacatataacacgatcaggatacaacaggcaataccgacggtcagaccaatgatattgatcaaagagtacattttactcctggaaaggctccgccaggcaattttaaaatagttgctgatcataattgtaggaataacgacgatatatatttaaatagttatacctggcgcccaaaacggatgccacgtagaagagccagtaccatagccaattttaaaaatcaaccggctcctttttgttcaaaaatgaacacttttcttacaaaaatgaacatggcgtctccatccaattgttaattttcgctgaacataagcctgcttaaattgttcatccagttattggcagtaatttcgtactaatctgtttgtaccaaaacacatgcatatgaaaacaatgctcatcctgacggatttttcagaaaatgccttccgggctacagaatatgcagcgcagctggtaaatccccttcaaatcagccggatcgttttgtatcatgcttaccaaagcactattataggtactgatttacctgtagcaaataccaccaatgatcagcagatatatctcgaaagtatggaaaacctgggcctgcaacaggatcgcctgtcagcgctcgtaaaaaatgtaaggatcgacctgatggcggaagatgtttcacttcccgtacacatcagcgggctttgcaagagtgaagaaatagatattgtggtgatgggtgtttccggtcgttccgggctggagaaattattactgggcagcactacttccatgatgatccaggaaagcagcgtgccggtacttattgttcccaacagcacgctgattggtaaacccataaattctgtggtatttactaccgacctgaaagaccatgcatccataccggcgcatcagctgtatgagttcctggatgcctttcccggagccgctgtgcaggtcatcaacgtagataaatcagccggtaacagctatactgtagaaacaaaagaatccattaccagtttacatgaaatttttgacaagtacaatgcagccttcgattatattaatacagataatacggtagaaggtattttatcatacgccaatacccaccatgcttccatgatcattgtggtgcctaaaaaactgggcgcagtagcctctttcttccatagtagcgtctccaaaaagctggcgtacgattccaatatcccgctgttgtcattaccagccgtaaaggcataaaaaagctccggttgtggccggagctgctagttgtttcgttttccctacgctggcattacccagatcaggtgcttgagtatgatctcagatctgttttaccagaccaccccattctgaaacatctgataataaatgccgaaaaatcgtgccagtgaaaaaggacggtttttagctatttttctggtaaaaatctctacaggatgtaaaaaatacgcgccactgctgtgacgaaaatccctggttatatgcacgagcctggcttaaatcagcactttattatccacggcgcattttatgagcatcgcggtattccgtgcattgaatttacccagcaggttccggcgatgactatctaccgtatctgaactgataaacagcttctctgcaatttcatgattggtatgaccgttggcaatgagccacaatacttccttttcccttttggtaatatgtaacggcagcaggtcttttttaagcgactgttttaattctgccgatagataggtgtgcccggaatatacgtcgtgtattgcccgcagcaattcttccttatcggcatttttcatcaggcaaccgcttgcgccgctgtccagcatcccggcaatgccgctgtcgtttttatgatagctcaatcccagtaccgcaatatccgggtaccgttttttaatgctggcgcagagttctgccccactgatatcaggcagcagggtatccagtaatacaacatcggcagtgtgctgatctaagaagtgaagacaggaaattccgttcctggtttcacctgctaagtgaatatctttttccatactgagtaaagatcgcaatccttcgagtatcaatggatgatcatcaacgaaatataaacggatcatggtttttctgtttgctgtaacgtctgtatgcgatggcataaataatatcgggcgaacaactgaaatgctcatttactatgtatgtaatatagtaaaaaaatcaagacaagtttaatctatcagcatacattctccccatgccggtttgatagaggtatccgcaaaactgatcagcgacagcccgatgcccgcaataccttccaatacattatgactgttaatataatcgggatgatgataaaatttatacccggcaggtccatcatcccaggtattcatttgcagggtattttgcagccaatagcgggaggcattcaataaagcggtatcaccaccggccagtccggcctgttgcaggatatgggcaatgcctgcgctgccatgacataagcaaccgtcatgcaccgcgccattttttacattccggtgtgtggcaatgtgtttaaacagctgttgagcttcctcctggtaatcggttctatttaaacgtttgccggctccctgcaatgtgatggcaataccaagatctccatagcaccatccaagcctgctgtgcgcgtcgcccattactttattggcggcatttacaatagtaggatagcgtgaatgcgtggcttctgccgcggtattttttgtatgcagcaaccattgaacactgttgttgattagcctgccggcacgttcctttgcaatcccgttttcatagcacctcgccaacaccgagatgatggcaggaacaccatgtgccagtccgaggttaaacaggtcttcatcaggatgctgctggcttctgctggagaaatgatctttccaggcaatgccgcctggtaacaggatggcgctttcttccaggtgcgccacgaggttttccagttgggcaattgcagtggccgccggcagccgctccaggaaataaagtgctgtgccaaggccatgatgcaggaaatcatttctgccttccgctaactcggacgccataaaatctgctaccagcagatcgatgtctgcaaaggtatcttcggtatcatcggcttcaataaatcccatggcgcccaggtgctgaatacaccaggatacgcctgcaattccactgcagtgagaaccattcatgggctcttcagataatgcctgcaggcatttttctatgatgtaatggactttgtccaggtgttcttccttaccggtgagctgataatagtaggcataaaacaaggccacgccggtatatccccccagcaggctggtattggtatcttccaggataaatgggtccagcgctgcgcagatcctttgcagcgcggatgtagcctcttgctgttgatccatataataaattgccgttataaatatataatggcaaaacacgtatgcatactgcaatacatgttttgccatacagtcaggttgctgtgaaaattatcgatctgtactgatcagtagcgacaagagtcgaggctgcaaataggagcgccctgactgatgttgtcagtacaaatccggagcgaacacagaacggaacaggtgccgacggttgccgccatctgttgtcctgttgcattggaaagactggccacttttattttacccagactgagttttttgcctgatgtttttttcatgacacaatttttttaacagtacaatgatgaaattagaaaatgcaggagtcttcactacatacaggtgcaccctggctaagacaagtgatcttaacacttggaacacaggccagtgatggaatgaattgagcagctcccctgctgtcattattgactttgctgaggtcggccactttaattttaccgagactcagtttcttaccggattttttcatggttgttcagtttaattagaagcaaggatctttggaaataggtggagtacatttcataaacaggctgcagccggtatatgtaggtgctttaccatcggcctgttcctggctgctgatactgagtttagccacttttaatttaccgagggccaatttctttacaggtgtttttctcatttcgcaaatgtttatggttgaaaaaataaatagacaataagtttggcaggttcaatataatagggtcattcgaaatacaggttttataagattacaggattgatgataaatgtaggtagaaagtgagaatatagggatcacgtaaaaacgtgattttttacataaagatgtttaaacatcctttttaccggttttacgtgatactatactgtggcagaaaaaattaccttcatttttttaatgttgaccttgcgccatgatcagagctgaaaacttctatgtggtaagaacaccgctattaccggtgaatattgtcactcagttacaccatatctcccaagcctccctcgctcctgttatcaaagctattttccgggatgagttcctgcaggaagctatttatattgcttctccggaattataccaggagttgcagaagtggctggccaccgacagcgacaaccagaaactggcatcagcactgtatcgctacctgctgcggatgagcagcagatgcacgccttacggtctctttgcaggctgtgccaccggcggattatcggatcatacggctattcaactgaatgataaacagttgcataaaaaacattgccgcctcgacatgaactatgtggcagagcttaccgccgccattactgccataccggccatccgggaacaactgctgtattatcccaacaactccttgtatgctgccggcagccaatatcgctatgcggcctacagcgttaaaaataaggtccgcaattattatctcaccgctgtaaattatagcagctacctggaaaaaatgctggaaacagcccgcaacggcgccacgctggcggacatacgcaacagcattgtaagtgaagaagaagacatcagcgcagaagatgctgaagttttcacagaagaactattgcagaaccagctgctggtaagtgaactggagcccaccgttaccggtgacgagttttttagccacctggtgaaccggttaaaaaacctggagcataccaccgaaacaaccgcattgctgacgaccatacaaagtatgcttaacctgcaacagacaggcaccggcaagtataccaccacccatgagctggtgcagtcgctgctcacggaaaccagtaacaaagacctggtacaaacagatctgtttctttcaaccgcaaaaaataccctgagccataccgttatcaatgaattgtccgcccaggtagcgcagctgtggaaactggccagcaacgataacaacagcgacctgcggcagttttgcgatgccttccggcaacggtatgaagaacaggaaattccgctcagcctggccctggacagtgaagccggtatcggctatggcgcccatagccagagcaatacagaccatacgccgctggtagataatttacaccttccaccacgtaataccacatctgccgccccccgcagtaagttgcaggactttcagctgcaacagcttcatcagtgcctgaaggaaaacaaaaaggtgatcaccctcacccgcgagcacctggaaagcttccgggaaaaagaaacaccctccctcccccacagcatgtacctgatgggaagcatactgagcaacagcgccgcagctatcgataacggcgactacctcttcgatatgaatggctgcagcggcccttccgccgccaacctgctgggaaggttttgtcatggtgatgaagaactggccgcccatgtaaaagcctgtttaaaagcggaagaagccagcgacccggaaaagatctatgctgaaattattcacctgccggaatcacggacaggcaacattcttatgcggccacggttacgggagtacgaaattgtatacctggccaatagcctcgccccggaagcgtaccagctgcacctttccgatctgatggtgagtgtacaacgtaataaggtagtgctgcgctccaggaaactgaataaaattattgtaccacgcctcagcaccgcacataattaccggcagggactaccggtttataaattcctgtgcgatctgcaattccaggactaccataccggtattggctggcactggcagatacccggtgaggtctctttctatccgcgcgtgcagtatggcaacatcatcctcagcaaaggaacctggatgctgcacaaaaaatcatacccggcactggctaaagcaaccccggaaaagtatatggaaattttccgggacatcagcgcacaactggagcttccccgttatgtagtggtaaaggaaggcgacaatgaactgccggctgatcttgaaaacgaagtggcagtgcacctgctggtaaccaccctgctgaaaaaagaacaggtaaccctgcaggagttcctccatacacccggaaattgctggatcaacggccccgatggcgcgtataccaacgaatttattattccactcaggaacatatcttccgaaaaagaaaacaaacaaacaaaccaaataattaccacacctgccggtacgcccgtccgaaaattcagtaccggcagtgaatggctgtatgttaaactatacgccggtacacggagtgcggaaaatatcctgaaagaaaagatcctgccgttaacacaggaactgatgcaggacaacatcattgaccagtggttttttatccggtacaccgatcccgaacatcacctgcggatcaggttccaccacagcactaatccacatttctggagcaccgtattggaaagattgcacgccgcactgcccaccgatagcatacaccggcttcaaacagatacctacgaaagggaaattgaacgctacggcgcagataccatgctgtttagcgaagcggtgtttcattacgacagtacatgcgtcatcagcatactggatctcctggaagaagaagaaggtgaaaactaccgctggatgctggcattgagaggggtggacatgctgctgaatgatttcgggtatacgctttcagccaaatcggccttattgaaaatgctccagaaaagcttcttcgaagaatttggtggtgaaaagtccttgctggtacaactcaacgacaaataccgggaagaaatgcggaaagtgagcagtatacttgatcctatgcaggacagcgaacagggtattgaagcggccgtggcttgctttcaaacccgctccgctcatatacaggaacagcttgcaggcatacagctcgccaaccgcgacgatctcctttgcagctacattcacatgttccttaacaggatcctgttatccaatcagcgcaaacatgaactcgtgatctatcatttcctcagcaggtattatgaatccatgatcgccatctctaaaaaacagctcaaagcaattactcactaaatacatattggtatgaaaaagaagaatgagcaaaaaatgaagctgggcactattaaagtggccaggttaagtgcaggtattacatccacagatcaacagcagaaaaagatcactcatcctaccactacggtaatcaggactttcgactgctaactgtttcaccggggtgccggctattttttacaccggtaccctcttttaaagtctttctacttcactcaagggcaacctgatttccccaaccgggtttaccaccttcagcatcagttctccataatgcaggtagagatcggccactatggcgccatcttttactttccatttggtgtttgtttgcaggtagcgttttaatttctcctccagctgcgcggttcctttccatttccggactttcagtaacgctacatacactttatatcctttaggttgtgaagcggcagtcatcagtttcatcatctcttcctggttagcggtatggtaaatgccttttctacaatccgctgaaatatgttgcaggtgctcatttgccagtgcaagatgcttatagggggtaatgagaaaagtttcaatgatatccgtatcaaaatgatctttcccacgcggataactttgtcttacaaaagcaacaaaaccatgctttgccaaagacatcactaattccggagagagcagcgccaggggattatgcatgaactgaatttaacatttccaggaaagatactaagatagttagtactaatataaaataaaaaagccctgatggccactacagcatggttctcaaggcttttttacattattcatttgctttctgaaacaaaaatactaatatttttagtaaatcctaatttattttatccacggcctcaactgggccccacataactatcatgtttggtccatatgagggcgccggtatcatatcccagtgcggcggcggttgccaggaaacggattttgatatcttcggggatagtccgggtacgcgataaaatccagatatagttcaggttgttgccggccaccagggcatactgatatttttcgtcgatatcaatgacattatacccggcgtaaaacggtctggagaaagatacttttaaccgggcttcgtcaggtgtactcacaaacgcagctttaccttcactttctttccaacggtatttcttggtatcataacccttgttgtccacttttatctccccgttttcctttaatgaataggtggcagaaacattgctgagataatgttcaaaccggtaatccagcctggcgatttcataccaggtgcccaggaatttttgtatgtcaaaaggagaaacagctttggcccccttaggaatggacactttggtattattatacaacaaatatgcggcggcagcagacgcagctgctcccaggaccagcaattttttattcataaagcatgatttttaaaaatgatgtgtctgaatttgcgggaggtaccgcaaaaaggctgcctgaccggaagtgactgctggcagggagttttaaaataaaaggcggaccgggagtgttgccaaattgctacaaatagaggtaagaaattgagaagggcaaggaaagtgagctcgtctacagggcagacatttccatccttcgttgaaacccttccaggaactgcgccacatggaatccatccatcaacgcatgatgcacatgcacagatacaggcattattttccggtcgcccacttcttttactttaccgaaagtaattttagggcagctatctttaaatgaaaaactccgcgcatgggatacggcggtaaagttaatccagggcagggaggaataatgaatcacattctctcccgacacagctggtatcaatcctgtactctgacgtactctttcaatttctgctttgctgctggcttcaaatgcggctgcatcttcataaaaattcatatatgcaaaaccaaaagtaccgtcgggccggttaatggtgggtgatgcatgtacctggtcatacacccatacttcatcaccggcgatacggtaacggaaagggggaacttcgttggcggctgccagcgacttatgcaggtagcttaaaaagaaggagtccccgctggctttggcgttgttaaaggcagtggtgcagtcgatgtcggtggtgatcccgaaaaaaggttcttcgaactggcggaagaagttaaagtgttcctttctcgcccaggtgtccagatctaataattgtttcataatatcaggtgcggcaggatatctgccattgtagtaaactcataaaaacggggatcttcgattgtatgatcgatgtgttcatgctgccaggtggtatggtacggaatatggatagcatgaccgcccagtgccagcaccggcagtacatccgatttcagggagttgcccatcatgaggaattcttccggcttgcagtcgaggtgctttattaatttaagatagtcgcgttcctttttgtcgctcataatttcaatatgatggaaataatgctccaggcccgatttccgcagtttgcgttcctggtccagcagatcgccttttgtagccactaccaggcgatacttgccggagagcgcctgcagcacctcttctaccccatcgagcagcacaatgggcttatccagcatttcttttccatactggagcaccttatggaaaacttccgggccggcagtattttcggatacgcgcagtacggtttctatcatgcaaagcataaaagattttatgccataaccatagagttccaggttggccatctccgttttaaacagctcctgcgatacggtatgatgcggcaggtaatcttccagcaggctgcaaaaaagggcttctgtttcctggaagtaaggctcgtttacccaaagggtatcgtcggcatcgaatgcgatcacgctaatgtcagagatcattgttatttttacgtttttccggatgcaaaaatagaacccggcagtttataaaacgggacatttgtcccacttcttaaaagtatgttacggaccaatcctgcttttcttcatttcatggaacaattcaccgccagcagcgcggaaggcgaagcagtggccattaaaacctttactgccggcacacggctcatccgccagggtgataccatcagtcatgtttatattatccgggaaggtattacaaaatgttatattgaagaagataacgggaaagactatattttcgaattcctgggaaagggtgaaattaccggcgacctggaaggcatcaggaaagaaaaatgcctgtgtaatattgaagccattacgcccgtaacagcatatgccattccgcataccttgtttagctggctgctggttaacaatacggagttcaacaggctgatgttggaagaactggtgatccgtatccgccaaacctgtatccgcgcgtcttaccagcaactatacccggtagaatatgcattgctccggttgctggcgctggaagcggaacaagacattgttattcccaaaaaggatatggcatcttacctgggtattacgacccggagttttaacaggaccctgaaagaactaaggtccaaaaatatcctggatccgcaggggatgaacattgatcttagccggaagcaactggaagaaatattgcgccggtttgaggatatgggataacggccacctgtatacgaaaacaaagggctgtccctttttacagcaacagcccttctgttatttacttgaataacctccactcgcttagctggaaatccacactgccattggtggcggttacatacacggcataatatttatacgccgtagtattggaaatggcaaactgcctggtttgatttcggacgccaaacacctggtttgtttgggtatcgagtaccgtccacgtagtaccattattggagcctttcagctgccagtttttaggatctcggtctgtagcgtcgttaccggaagtaagggtatatgatttcacggtttgcccggtgacaaactgcagctgcattttaaaatcagcaggcaccgcattcacaaatagtttggtgctgtatacattatcggtgagcttcaaggagccttctgccgcggaggcgccaccattgttttctttactcacggtaatcgtgcccgaaccggtaatgtcatccgaaggataagtgatacccgggaaatccgtttttgcctgcttcagctgtgcggtccagtcgttgcccccttcgtctttattgccaaaggcagtgagggccaattgcttcagatctttattggcagcgccgctccagtaatgtacaaattccccgaagttaaggccgcgggtgtattcggggtaagtggtgatgccgttattgtacgtttgtttggggaaatgctgcgccagcagtgcgaagaatttattcagtggcgctacaccaccgtagttagtatagattggataaaaccaatccctgaaccagtaagtgcctgcgcggggataagcatctgtttgggtgatcttcatgttataccagcgggtaacatcggcactgcggcccagggccaggtacacatcgtactggtagatttccatccatttgctgtcgtgccagatgccaaacgccggggagccgtgtacgcctttggaagcgccttccacaatatgccccacttcatgggtggtaaggtcaatgtcgttgcctgcaccggagatccaggcattgggatcggaggagcctacatctattacgttgcggtaatcatgactggcatccatatacgtagacggatgcccaccggaatatttgccggagtgcaggattacaaagaggcgggaatcgtcgccaaaagcaccgtaagtgcttttggtatagttccatacctgcgcgaggtaggtgttgggccaggtaatgctgctgtttacatcattatcaaaataaactgctacgctggtatcataaaaaacgcggttaagcagctgttggtgttcaaaccaatgttcctgccaggtgacgggtggtgtggctaatacctgcaggttattttttccggaaacaggttgaagatcaccgccgggagcgcttttcttttcgcatcccaacagtatgcccagcacaataaatgccgcagcaaacaatgaagttttcatacgtttttttttaagatgagtgaatgaagggggtttcgggttttcaatcatgcgcaactgctcctggtgaagcagttgctaatcaatgcagttttggttgttcaggtagataagttaacacatctttttacagtaacctgtcaacggattttaaacaattgtaaacagatattaaaaggatacataaaaaaaggtgcgcagtacgctgcacaccttttttactttttattgccgctgctattctgttgcgcgggtgtacaatcccctgtccatcctcactcccaggcgtttcatcatgcccggcatatcaaatccttcttttttgtattccgcctgcacctgttctttggcgctggctaccgccgctttgttttcccactgcgcaatggtaacatacaccaggttgccctgctcatcaaaatattcataggcagcatctgaaataaagccggggagcgttttaatgaggcgccggttcaccgccacccgctgcttgaattccgtgatgcccgcagcaggcactacaaatttatcaatgaactgtacctgttcttttaccggtgccgtggcaatatccgcgggtaatacgcccagcgaggttaaaaacccgaggcggtcggtctgtacttctgatgcgatgatttttccatctttaaattcatagatggctacgccgttgatatgaatagctttgccggtagcaggaatgtttttgtacggccctgtttgtgtgccataccaggtccatttcgccactaccttattcccatctgataccagtgacgataatttccactgaatgtccgggaaggcggcgatgagtggtgcaatgggggcagtaaaccccgccacgcccttgtgtccttccggaccggtatgcgcttcggatacaatggacggcaacaggcgcatgtcttttttgttcatgacattttcatatagttcctgtataatggctttgttcttttccatatctgttattttaaattccttttgttgatgaatactttttccctgtgaaaatgacatcgctggcagcagtgtagtgaccaggtatatcgtaagatgaacggttttcatttgtttttctttttacaaaagtatctctcccgcaaaacccggaattgtaaaaaatcattgatttaccaaaaccacttatccttattcatgtttttcattacggtcagtttttctatcttagctccgatctattatcagtaaaacccacgtctttgaaatttctgattaattttttcctgataagtattatcagcaacggcgtttatgcgcaggcggtacttacaggcacagtgaacaattcatctcatacgcccgctgcttatgccattgtacgccttcaacggttacccggggatccgcagcaggtattgcaaacagacagcagcggcagcttccgctttaccaggctgtctgcaggcgaatacacgctgaatgccgttgttaccggctaccaggccgccacgctgcatttcagcattcgccgtgatacagtggtaaacatcaccttacaaccttccaatacccggttgggtgaagtgaccgttacggccggcaaacccgctattgaaaacaacccggataaactggtgtacaatgtggcgtctaacattaccgctgccggcagcaatgtgctggaagccattggcaaagtgcccggcataaaagtgaacgacaatgaaatcagcattaccggtaagggagcggtaaaagtgatggtaaatgaccgcctggtgcaactggccggcatcgacctggtacgctacttaaaatctatgtctgccagccagatctcgaaaattgagctgatcaaaaatccttccgcacagtatgacgcagaaggaaatgcaggactaatcaatatcactacccgtcagcgtaaaaacgaaggctactccggcaccgtgcaggccaatgccaaaggatggcttcacaaccccgccgtagtgtatggcacccgtaactatgaggcgttgaatgtaaacgccacgctgaactacaacgccgcgcggtggtcggcgtatgggagcattaacctcgatcaggatcagcacctggaaggcttccggaccaccatctattacccgaagcaaacctggatacagtcggacaccggtaaatatacctatctcaatgcgaatgtaatcgccggcgctgattacaggatcagccggaaggccaccatcgggctgaattaccagggcggtaaaaatgtgtatgatggcggcgaccgcgtgaacaacccggtatttgacaatgccaccggcaaacaggattctatcatgaaaacacacgccacctaccgccctatcgccgataatcattctatcaacctgcattccgcgatcaactttgataccaccggccgcaggctgctgctgaatgcagactacttcagctactaccgcaccgaccggtccgattttgaaagcaataactacctgggtgataacaccacccacccttccggcaccacccgttactacgacgataacaagcaacgcattcatatttacacgctgaaagcagatatggaactccctacccgttttgcaaagttcctggtaggcggcaagctgagctttatcgataactacagcaatgctttttattataacaaggattcttccggcagattggaatacgacaaaaatctcagcaacgagtttgattaccaggaaaacacgcaggagctgtatgtgagcatgaacaaggaacaggacaactggaagtatgaagctggtttgagaggggaacttacgcaaactaccggttactcctatacgctggatcagcgcacccaacgtaaatatttccggttattcccgtcgctgtcggtatcatggcaggccaataaagacaacagcctggcttttacagcaggccggcgtattaaccgcccgtcgttctggaacctgaaccctttcaaatcgttgtatacctcctatagttatggcgaagggaatcctgcgttaaatcccgagtataacaccaatattgaattatcacatactttcaggaacaggcttacttcttccttattttttaataaaacagatgatggatttaacaacgttaccatcgccagtgcagacaccaacctcgtgtatacggttccgttaaactttatccggacttaccggtatggcatctctgaaagtgtgtcgtttactgtttttgactggctcgacaacaataaccaggtaaccctttaccataccgacgcacattctgacattccgcaggtgagtagtatccgtggatggggaatgtatcttgccacaaataataacatctatttcaaccgcgataaaacttttgcaggcgccatcaactgctggtaccagttccccgaaataaatcatattggcagatcagatgcttattttaagctggatatcgggctgaaggcatcggtgatgaagaagaaagtagacatcgtgttaaccatgaatgatatttgccagagcagcgccatgaccattaattccaccatcaacggcgcgcggcagcagctgagcaacttccagttgaaccgttacctgcagctaggcatcagttaccgctttggcagcagggccgctaagcagccggccggcgacaccggcaaccaggaagagagaggccgtgttcattaactgatgatagaaccggagatttatacacatcccttttttgcacagattccaacaccgattcagtgctggcctgcgggccagcgcatagagcatgccagaaacagcactcgcaacctgagaatttccgcaggtgcagaatggctgctttttggtagcttagcggccgggaactgcatatccgggcttgtaacacccgggcaggaaagctagataagttaaaaaaccaacttactttattaccaatacattaacaggtggttttgggtttatatgaaagataaaatcctatattaggaccttgaaaaaaagcgggatgcaggcttttttagtattaacccataacaaactgattttggtaacaaaaagattaaacaggagctgctaaatattacttatattaacccttacaggtatgctggtacagggaaccgggccgactaacaattgccggagtgacgtaaatgattaaaaagtacatgaacatataccaacattattcttttgatctatggttaactttaataaaatcgaatcctttatttaaacaggaaaggacgcgctttttttacaaccatttcaatcaacaccaaaaaacactggaagaggtaggccgcatattccgcaaaacagatctgctatgcaatgccatcaatgaaaaaacaggcggtaatattgatgcggaagaaatgtacctcatggtgatcagtgaaataaatgattacgacaatgccttcgggagcattgatctggcaggactttaccaggaaatggacgccctggtgctcaaatacctcccggttatttattgttcggaaacagtgaaaacattgcgcaggataaaagcatcgtccgatagtaccatcagtttactcagtaacaccgcttttataaaaggcagcacattaagacgggtattacaggagctggagctggagcattttttcgatttccagctgtattcagatgaaaccggcatgtcgaaacccaatgaaaaaatgtttcgcctgatgctggaaaacgtagcgatagtaagaaatgatacggcaatcccgctaagtaacatcatacatattggcgataatgtaaaagcagatattaacggggcgcaggtgacaggcattcgtactttactggtcaactccaatcatcaatgtatttcaagtttacttaactgatgacaacaacctattcacttcataagatcacccatgccggccatttcgggtttagccccgatgattacagccgtttcaagttcggggacgacgccgttgccgaaaaattcgggaccagcctggcggaagggtttattgagcatcacctcaaaggacaggaagtgccacagtttgtggtagtgtcaagtccatattcctttatcccaacggctacctttgcgatgaaaaactatttcgtttttcatttgaacaggtggctggcagcgcacgggcacccggttttacaggaaaccaaagtacaccgtaccattacctacaaggaggattacggcgaactggatgcggagcaacggttaaagctgatcggcaacgacagcttccatatcgaccgccacttcctgaccgggaagaaagtgattttcctggatgacatcaaaattacaggaggccatgaaagaatgatcctgaaaatggtggatgcctatgacctgcctaacgatgtgtacctgctctattatgcagaactgcagaataaaagcattcatcccaacattgaaaaccacctgaactatcattttgtaaagtccatcttccacctggaaaaaatcatccagggggaacaatttttcattaatacacggattgtaaagtatatcttgaattatgatttcgattcattttgtattttccttcaaaatcaatccgataaatttgtgaatcttttgtataatatggccctgggaaacggttatcatacgatagaagtttaccagaaaaatctgaattttattaataattacttatttaacagaaaacataaaagcatacaacatggcaattaatttgcaaaaaggtcagcggcaaacgattaatgcgcccaaattcgtaatcggcctgggctgggacgctaatgcttcatctaccggcaccagcttcgatctggatgcttccctgttcgtaatgggagagaataaaaagatattatctgagcagcactttattttttataataacctcgtatcacccgatggcagcgtagagcataccggcgataacctcaccggcgatggcggcggcgacgatgaacagattaaaattgacctgtctaaagcagatccgaaaattaccgaaatatgcgtggtggtaaccatccacgatgcagaagcacgccgccagaactttggccaggtaaggaattcctttgtacgtatattcgacccggttaccaacgaagtgctgctgaaatacgagctggaagaagatttttctattgaaaccgctgtggaattcggaagaatttacaaacgcaacgacgaatggaagtttgaagcagtaggcgttggcatgaaaggcggtctgcaggactacctgaacaaatacaactaatctatacaccactatatctaaatataagatcaacatggcaatcaatcttcaaaaaggtcagcgtataaatctcgaaaaaagcaatggcgccaaacttcagaatatctgtgtagggatcaactggggcgctattgaaaagaaaggcctgtttggcctgtcaaaaaccaaagaagcggtagacctggacggcagctgcgcaatgttcaccgaacagaaacaactgcaggaagtggtttactttggtaacctgaaatcaaaagacaacgcggtaaaacacagcggcgatgatctgaccggtgacctgaacggcaacgacggcctggacaatgaagtgatcacgctcgatttctcaaggctggacgctaacaccaactacgtagcgtttgtgctgaacagcttccgcggacacgactttggtacgattccttttgcgtctatccgcatttatgaaggtaccccctcccgcgtgaacgaagtatttgccacctatgatatcgccagcggccccggctttgcaggacacgtatctatggtgatgggcgttttctacaaaaagaacggcgaatggaaatttaatgcgatcggtgaacctacaaaagataaaaaactgcaggaaaccgtaagcaccgttgcgcagaactacctgtaggatcacttttgataagataatatcaatttataatcagataccttatggaagcaaacccaaatatcaccgaccaaacccttcccgcggtaaggctcgacaaagagggaaatgtggatctggcagttattacgccggacgatgcaaagaaatacggggaaataagtaaaacattggtaaccaccgatgtaaattccattctgaattatggtaccgatgtacagaattcaatggaaaaatacagtaatgagttcctcacttctgtacgtacctataactcaggcgaagtaggcgggctgatcaacgatctgcttacagaactgaattatatcgacgtagatgaactgaaccagggcgccgtacagagctttatctccaaaatacctttcctgaaaaaactggtatttgatgccaagaagcttttccagaagtacgataccgttatcagtaacattgataagattaccaacaagatcaaagcgggccgcatcaattcactgaaagacaacagttctttgcaaaccatgtttgatagtaacgtatcttacatcaaacaaatggaagatctcattatttcaggtcagctgaaattcaatgagctcagccagaagctggccgaaatggaagtgaatgccgccaattacaatgactatgaaatcgctgatttaagggacttcattacccgcctggataaaagactggcggacatgaagattgtacgctttattatgctgcagtctttagctcagatcaggctggtacaaaacaacaatacttccattgcggaaaaggcgcagtcgatcatttccaccacgatccctgtctggaaaaaccagctcaccattgcggtagcgctgcaaagacagaaagccaacgtggaaatgcaaaagaagatttctgataccaccaataccattctccagaaaaatgccgatctgctgaaacaaaacagcatcgaggtagcgaaagagaatgagaaaacagtagtatctattgaaacattgaagagaactacccagtcgctgattgaaactttacatgaagtgaagaagatccacgatcagggcaccgaaagccggaaagtgctgaatggtgaattgcagacgctggaaacagagctgaagaaaaatgtaacaaacgttagctaacggaggataagtaatggaggataacctggcaataatattaaatgactcaaataaaactatcagcaagttacaattgctgtccactttttttgaagaagagataatatacaagatttatctccgaagccaggttgtccataaattatttgaaaccaatccggaacttgatgtcaataagctggaactgtttcacctgcaatacaccgccacggtgattgacctgttgcgaaaaataaaagccagcaatgaaagaaacgtgagtattttatacgacgaaatacagatcaacaaagacctgatcgccaatatcaacgactccgttttttcagagaaaaattaccagcaggataaacagaaacaatccctgaagatcaatttatctttgcggaagctgtaccaggtgctgtctgacaactccgaagactaccccttctccaaaaacattaacgctttcagcgcacgcttctcccaggatttttatttcgatatttccaccgaagcgctcaatgaactgattaaattcaacccggcagaagtgtaccgcaacaactccgccatcatacagcgcaagctgatgggattgttgtgcaaaatggattttaaaaccgagttcttttgcggactcagtgccggtaacctgatcctggaagtgtaccgtttccttaatatggaccgttactatctcttcttccccgctaaaaatttattcctgttctgcgatctttcaaaaatcacagatgttgactggtccaataccctctccaaaaaaacaaggattgtacaggagttaacggataagaatgataacctgatgagccgcgccaacgtactgaaaacggtgatcccggataacgtgcatgccctcctgaaagaatactatgagaaaatttccgacgtcgatttcctgcaacagattggtcgctttgatgtgcagacaaacatcctcaaaacgatgctgaacaccaatgtgatttaggcataaaaaagacgccagtccgcaaactggcgccatagaaacctttattaagctaagccggtttgttaccggcatcattttttctccaactctgcagcaggggttcttttaggaacatttaacagcgccgatgtaatgatcggaacgataaacacgcctacggtgatgatcgacgtaatgatgtctgcttttgaactttccaggaagtgggtaacaggtgattccgggaagaaatgttcgtagatagacaacgtcagtttaatacccaggatcgcaataacgatgtacgccgctgcttccaggaaggtaaacttcgtcatcagtttcacgaaagcctgtgccacaaaacgcatggcgaggataccgataaacacgcccaggcaaaccagcagtatattatcagtaaaagctactgcagcaaaaatattatctatagagaaagccatatccattaactccaccagtgccaccgtagcccagaaaggcccgatagcccccactgtggccttgtatagccagttctggcctttgtcgatgctctcttcttctttctctccttctgttttcttatttttccaccagctgaataccaggtacaggagatataaaccgcccaatggtttcagccaccagatcttgatcaggaaagacgcgaacaacatagccagaccacggaacaggtaagcgccgaaaatcccgtatttaagggcgcggtcacgttgtttttcgggcaggtccattaccatggtagccagtacagcggcgttatctaccgacaataaactttcaataataacgagattcccgacaatgattgccgaaggtattgggttgtcaataatttgttggattaattcattcatttcactttattttttatataggtttctacttgttggcaatcgttataatgactactcttccaccctcttccctcgacagcaatagtctttttccatccgttagttccaccatctcaccgatggcaatttctttatcttctgtaagatcttttaaagaagtgagctgctggttgaccagcacccatttgccctggtgaaaaacaaaatacccgaccggcactttttgcgcggcggtgatccgttcgttgcggatagtattcctgtttacatgccattggaacaggtattgattattatacaccatcagccggtggttttccggtttccataccgttggcttaaactcgtaatacaggtccagtacgggcagggtgcctttatgcggcgtaccgcagaaagggcatttaggagaatgggtgttatcaaaaacgtaccatttctgttcgcaggcggcattgctgcagggctgcatgaggtctgttgtttttagtaacgcctgttcccacatttctgccggcggccgctcggttggctggtgcaaaccggttacaaacgcctggtagaacagttccttcaggtaaggccctgtaatggtgtatggtaacttatttacatctgcccagggcaattccttcggattaatgtgattcagttttggccggttggaagtatcctgcggatgttcaataaacagcgccttctctcccattgccagcaggtcgtctttttctgcgtcgagatcgtggatcttccctccttttaagggatgacggtataaaagatacatgtagatcattactgccagcgcatgcaggtcggtaagacggttgggcagcttcctgcccgggtctttcaggcccaggtgcttggtggcgagtacttccggtgcgatgaaatcggctgtgccaattacatccggtggaaacaggcccggtaccacgaggccatctatatcgatgatagtagccgatttacttaccgggtctaccagcacatttttatacgacaggtcggaatgtgcgagtccggctgcatgcaggcgtttcacacctcttgaaatatttacacagatctggaaatagcttaaccagttgcccagttctgcttcatccaggcgcagcgtaaactgcttgttcctgaatttgggtgaagcaaaccatttcccttctttctcctttcctttaatcaggtcgtttgatgcgtatcctttcttgaaaaaaaagttagcatggtaacacggtactacgaggcctacctttttatctgcttccaccatgtctgttggccagcaataaagatcccggtagtagtcgccgccttcccggttaaagaagctgttatagtagtccgtcacaattttccgcaaccgctctttcgaagcgtagtcctgtgtgtcccggtaaaatgccaccacgtatgatttatccggactgaagtaaacgtccttcatgccaccccgcataggttctccgttatcaacgtattgataacttttccctgcattgatgacggaattcaccgtttttgtactcatatagtccgcatacttaactgatgatcattaaagttctgtcgtcatgattcccggggctccagaagtccatccaggcagatagctggctggcggtttccggtgtatggctggccaggtctacttttacattgtcatcgtttttaccgccgaggtcttccagcagtgctttccaggctgtcagcttctccaggttggcttctacttcaaacttgggatcataaataccgtcggtcatcagcatcaggtacgagaaatcaggcaccagcctgaacccgaagcgggttgcaaatgtatcacttttaaagatttcctgcatggtaataaaccgggttcccccgctaaattctcccacatccagccggttcagcaactggatgtctgtaaaatccttattaatcaaagcaatggggcaatcgcctacgccaaagctcatgatcacatagccggattcgtacttttttaaaagtacaaatataagtgtggaatgaagatcttttactggcgctgcgcaggcgacagcaaattcttccagctttttatgtacggtgaacgctgctttgccgaggttatcgtatacaaagcgggtgagttctttttgtgttttgtcgcttccggcggtagcgtgtgcggcaatcagcgcatcaaatgcgctccttagtaccggcgtaaagtgctgctcaaagtattccacgatgccggtgcaggcgatcctggaccctgcgcgggacagccttgcgctgccggcgccgtcagaaacggccataacgctccagccggtgtcgccgaaatgtttaaaggcgaaatcatcttcccggaagccgccggtattggcgtgtgagcggcctcttttggaggctaccagcaggtgcctgtcgcccagcggggcatattccgctacgttgtcttctttccagtagggatcatttttatcgctgtcaatatttttccagagcgatctgggattggggttgatgaccagcggcacctttttttcgtttggcgcggtggtttcatcttcgccgttgatgcggtatttcaacgttagtttaaaatcgccgcttttaacgggtgtgccccggatcacttttgtttccggatcgtattgcagaccggtttcttccagcccctcgatatgaaaataggtaaagtcgttccatttcagcagtccgaaatccagtgtcacctcgtaaggctttcctgcagtggcattcgggatgctgacgggttgttgctgaatgtcggccaaccggtttttaaactgccaggtatccattagtagctttttattttccaggatctgccttaccgccagcctgtttttctcttcattcacaaaagcgtcgaacaggtgctgccggttagtgccgaccgtaatattatttgctttaaataattcccggataaaggatttgtccatgtttctcttttgtcggttagccttgtgcccggtttacatcaaaaccaccgtcgctggcgccgtatgccgcggtgtttccgcaggtggggcaggtactgagcttttcttcgccgatgcaatgaatctggccacaggagcacagggcgaatccccattggttgccgcagcaggggcaggtgggattgcctatcagttcttcactgttgataacagccggttttgtgtggctatcggacagttcgtgataggttttatctacctggaacgcccctaccagccggtaatacagccggttcaggtttagtccgtatatttctgcgtcctgttctgcgcggcggtatttcatgaggtaatcgcgttgcaggtgctggcatttacccaccattaccacgtaattgctatcggtgtaactgcggggtggtgatggttttgagagatctattttcgataaggtaacggtatcgtgtattttcgacagttcaaatcctgaagcgtttttctctacactttcactgctggttttgatagagtcggtaatccacctgaagaactgcttataggctgcgggagagctgtttttaaaatgcactacgttttccgtcagctccttcagcaggttggtatctgcttcattgccgaaagaaacggccaccatattggcagtgcgttgccagttctgtttccattccgcgatggctgcgctggtatcgtctgtaggcacgccatccgtgaaaagaaagatgatcggtttccagtcgccttttatttcataggtggttttcacctggttttttctcagttcatacatgaggtgtcccagtccccggcttaaagaggtgcctccgccaataggaaaacgcggcggataaaagttgatgatttcctgcagcggtaccagtgttttcgcctggccggcaaaaacaataatagagatccaggctgtttcaatggcgtagggatctgttttaagtgcttggatgatttgtcccagcccttcttccacttgttgaataggttctcccaccattgattcggagacgtctatcaggaaataaaccggtagtcttctcattatccaaaatttacagaagtgatatatacggttcccggaccggtaattttcagcatacttaatccttctcctcccaggagattatttccggagaaatgggatgacatccggtttaccatatctgcattcatgcagataaagcttttttcatccacaaaaacggtttgcccgggtgtgaggtccagtgtaatgggtgtacctatcacatctaaaaataccgtacaaaatcctgttattttctgcatgatcaggcctgtaccacctatgagggaggtcaggttcattttcacatcaatatcaattttgtcggaggaggccacaaaagcgcctgctttacaaacaatgccggaagtaagctgcttgaggttaacgggcaacagccccactttgccggctaccaccagcttgcgcggatttaaatgggtattgcacagttctacctggaaaatactttcgccggtgagttttctttttatcagtccggctacgcctttatcgaatacattgacctttgaagtaattccttcttcatgataaatcagtgcacctttctcacagaagaatttctcctgttgggataattctacttccaggcatttaaaatcgtgtccgatcaattttacgttcattctttttattatcagatgactaaattcacttcgttgggaggcggcggcagtgttacctgctcggtggtgcccatacttttatttccctgttctatggtgtcggatacccacttgaaaaattgcttcaatgtggcgctgtcggccgtatcgagatgcaccacggtgtctgtcagttccttgagcatgccgttgtctgctgcttttcctgccgcgcaacctacaatggtggcgaagttcaggtcttttatcagcgggatcattttgcggtacagctgcagatccgaaggtttaccatcggtaaaaaggaacagcaacgggcgccagtcgcctttttgcgtgggagtacctttgcgtacttcgctgttcacttttgcgtggagaaattccagtgcatagccggtgtgtgtgggcccgctctgcggacaggtaatttccggcaggtggaaattggccagttccaccagcggggtcagttcttttacttcccggtcgaaagtgatgatgctgagccacaacgaatccattgcctgggggtccatccgcaaagtgtttaccataccactcagggcgttgttgagtgcctgaatgggctcaccgtacatagatccggaggtatccaataaaaaaaataccggtaatcgtcgcatatcaatattttaatttcttacaccacgatattcagttctgccggtggtggcggcagttcgtttaagcctattaattctttgccggcatcttccacttttgtggaagtaacgccaatggaagcggttacccatgcaaagaagcgggcgatgctctgactatcggcggtatcgagactgagtacattatcggtgatttgtttcagtatgacggtatctgcaccggagccggcagcacaggcgatcgtatacgccactttgcgttgtttaaatgcggtcaatccactttgccagttatcggtgggaatgccgtcggtcatgataaacacgagtggtttccaatcgcctttcttctccgtagttgttttggccacttcgtgatcgatacagttgcttaccagctgcagcgcttctcccagtgcggtggtgccggtcgcttttatatccaccatctggaaagacgcgaggtcggtaaggggtactacctgccgtgcggagctatcgaaagtaatgatgctgataaatgcggtttcaatggcctgtggattctgacgtagtgagttaatcattatctgtacgccatttttcactgcctcaataggttctccattcatagaaccggaagtatctaataaaagatacacgggtaatcttctcatactgcattaatttaataccagtgttggcatgttgaaaatgggtaacatttcatcctgcgttttccgccggatgaggttatgctgaatataggttttttgtgatcaggaataggttaactttttcaattcgtccacaaagctatcggattgatgtggaataccaatggccctgaacttccaggcgccatctttacgataaatttctgcaaatgtcatggagcacatcccattgtaggtgctgtcgcccgacaggctaaatttagcgatctcttttccgcggctgtcaaccgcccggatgaacgcattatcgatcataccaaaatgctgattggtggcgcggccattgtaaatggtgaccataaacaggatcttttcatatttattctccagctggtccagcttgatgatgatttgttcatcatctccatcaccagcaccggtccggttgtcgccggttaaccagatattgccggaagggtggcgcatggaattgaagaagatcacatctccctcaaacaatcctactgatctgccatcctttgtttgtacggttctgccaaggttcgccactttgccgctgctgtcgagcagcatggctacggcatcgaggtcgtattctgcttcttttttttctccgccgaataattttccaaagaagccttcgttgcttttcgtttgccgtacatcccagcccaaaccaatcgtgaccgtggataaatcgaattcttctcctttgtcgtttttacggaggtcgatcgtttgaccttttactaaattgatagccataggtagtggtttatcaggggttatttaataatctgacctttgaaatatttggataagaagtaagccagatcttccctgtagccaatcccggatgcttcaaatttccatttcccatctttcaggtaaagacggccaaactccacgccggtttcaatggagaaatcttctcccagttcatactttgcaatttcattgccggtgccttcatcaacgatacggatatacgaatctcttacctgtccgaagttttgtcttctgctgatggcttcatggatagttaccacgaataagatttcccttatgcggggatctattttggtgaggtctacctggatggtttcatcatcgccatcagcgctgttgccgccggtagggtcatcaccggtgtgatgcagtgcgccgtccggagaatctgtatttccgtagaaaataaaatattcttcctggagaatatgcctgctctcatcgatcataaatgcagaagcatccaggtcgaaagcggagcctgttccttcattaggatgccagcctaaaccaatactgatttttgagaggccgatatcgatcctttgtcccttttgtaagttaatcgccattattcagaatttaaaccaggggtaatatagcatatttatttcagaggatatatggcgatattacagtcaatgcttagtaaacttttcatgtatcaaagatgaagctaatattgcttcatgatctccaccagcatatccgcaataacggcaaatcctttatcagagggatgcaggccatcgtacgtcatatcgatcgctgacaccggataagggtattcatctgtgtccggatggaaaggaatacctttataatccggccagcgatagtctttatattcaccggtggcggggtctttcaggcgtttatacttcaccatattttccggggtgatgccgctgttatgatacaggtctaatttgtcgaagtgttcatagccggcaatagaatcaatggcggccaccacctgtgaaagctgttgcccttttctttctttataagagccccaggcgttgttgtgcatatcggcgatgtatacaaaatcgccgcgttgcagcggggtgatcaggatgatatgcgcctttttattcagtgatttcaacttgtcaatgatcgtccggaatgcgccatacacggtgctgttccccgttttatcgagatagtcggagaaattaccaacagggcgcccgccccaccagtcgttggtaccaagaaacacagaatacacatccgcttttacaggatccagtttttctatggcatcggcgataccgccggaagtccagccgttataacctttattgatatactgtatgtgcgggagcttttcggttacgcgtgtcaggtatcctttggtgatcctgttgccggtttcaccggggtgatcattcaggtaggtaatagaatccccgatggccacccaggtgattttgcggggtgtaaaggcagtagcggccactattgcggcgatgagcagtcccaacaaccatttcttcatgataatatattttgcccattgaaagtagtaaatagcatagataataacaacgctggactatctcctgattataaactggactaccaggaggagctttacctgtattatttttgcctgtcaaaaataccaggcaatgaatattaaacaggatatcatccagctttttctgcgggtggcgttaggtgccagttatctgtgtgcggggctcgacaggttcggcgtgtggggacctccgggtggagcgaatatcgggtggggcgactggcaacattttatgcagtatgcacataaactgatgttctttttcccctatgcagtggcggaagtctttgctgcattagcttcgggggcagaaatactttttgccgtaatgcttatcacgggcttttggacccggtgggcagctattggcagcggcgttttgctacttggctttgcactggccatgacagtggcgctgggcatagccgcgccattgaactattctgttttcaccgccagtgccggcagctttttattgtctgctttacctgcctatcgctggagtgcagaccagttgcggaaaaaaactaatcccgcttccctttaaagtacgcgaatatcgccatcgcatgaccgtggcccagttcatattcttctttcagccagtttacaatgtcgccggcttttaccttgggggccagctcgccgttttgtaagaactttttcttctctgccagctttttaaagtcttcacctgttttgccggtttttgctttgatattgtctaaataagcctggaatgacataatacctgtttttattttgaatgatcttgtaagatgtatctcttaaaacaaaattattcattccggggaacactccgggggtgtggttccgacaaactaaggggcgatttgcggcgtctttcaggcggcttttttcacagtccccatgatccacctggccagccagttcattttctttacgcggcaattgtgaaaggcagacatctgccattggccttccgggctttttacccaaaccgtggtgttcaccgactgacggctttcaggcacttttttctgccagcggaaacggatagcgccggtggctaccacgatggctacattctcattcaggaaacgtacctgttcaatctgtccgtgcaaccgtgcgcctttgaacataaagttattcatcagctgctcgtgcagtgtgatgtactcctcccgcccttttaagtgcatgccgttaaacgtaatgtaatcgcaatcttccgtaagatatactgcagcgccgcggaaatccagtgtccggaatgaatgatagatggcgttgttcgcctgcctgatcgcattaatttcatgtacctgattcatacgatagttgttttaggaatgaatacgaaaataggcagccgaactacggcagcatagtacaaatgggttaatgacacgatcatgccggtaaaaacacatttttaccggtaaagtaccggggcgaaataaaaaagggccgtctgtaaaagacggccctcttctctattattcagcatctatttcttttgatcccaccaaaccttcgacaggtaagaatctccgttagttaaaccagatacggcagtcttataattatccgtattcagcagggcttccagtgatgaatataccgccctgcggggaatggtaccgttggtagatccctggttagggcccggcgttaaaacggggtagccggtgcggcgccattccgcataggcttcatagtcacggccaaacagcaggatccatttctgggtcatgatcttctccagctgtttttctgatgtaagtccggcgagtgaaaactccgcatcaatgtacgcctgcggaatggtagtaatattatacggctgcatggccattgctgctttgataccatcctggtaaaatttctccgcttctgcgggcgtagcaccccatcccatcaacgccgcttctgctttaaagaaacatacatctgcataggtgaatacataagcagggataggcgtagccaatgttttattaaagtaggtggtcatagaagcggtggaataatcatctttaatgataccggacaacaacgcatccgttaatgccacaccaatacctttgtacacaggcgttccgctgttttttgaatttacggtaggcgcggaaataaaggtaaggcggggatcatgcttatcattcagtgtggccacaaaagccgatgccaggtaacgcagatcggggctgccgctgataaactgcgccaggataggatttgcgttggtagtttgtgcatcgttgaaagtaggtaccgcggcattgtctttattatctgaaaaaagtggttgactcatcgcctcccgcaccgttttttccgccagctgcggcgcggcatacttaatgcgcatacctaaacgcagtttcagtgagttaccgaatttcttccagttgtcggtaacgcctttgtagtagaagtccgcgttgccgtacgatacatcgctggcgttgatattggcgatagcggcatccaggtcggcaatgaggtgttcatagatcgactgctggctgtcgtacaccggtttgttatttacgtcggtagcatcctctgttgtttgtgaaaacggtacggcgccgaagagatccgttaaccgttgccatataaatatttcgaggatgcgggcaatggcaagctttgttctcccggttggatcattttcttttcctttcaatgcctggttgcggatctggcccaggtttctcaacaaggtataatgtgcggcccacatgttattatccggctgctggatataacgggaagtaggcgccaccaggccaccggcccagtattgcacccaggaacctacctgtatattggcggtttctgttccttcagcaaaggccgcatctttctgtacttttgataacaacagggcgggatcaatgtttgttaccgttgttggcggcgtgttcagatcgctgaagtctttggtacagccacccagtaacaaccccaccgttaacaccagcacttttctatatatcgatgatttgtttttcatatgcttcgtttttacagattaaagatccaagcttacattcacaccaaagctccgcatcatcggcagcgccgttgactccaggccgagagaggagttgtttacgttgaaggaagacgcttcgggagagaagccatccgttttccgctggaagtaaaaaaggttcctgccatagatgcctacattcattctgcggatcattttaccggagaataatttcgatggcagcgcgtaactcaaactgatttcacgcatggctacgtagctggcgtcattcatcatttcttccgataccacattttctttatcgctggcgactacgttccagtagtcctgcgccaatactttcatcgtattttctttaccggtgctaacccagttgccactgctgtttttttccgcaatcataccggaggctacgtagctgccgtccctgcctgccagtgtttttgttgtggtaccataaatcagttcttcccggttactttgggaatataccaggccgccctggcggatatccactaatgcggctaaagcaaaacctttgtaacggaaggtattggcaaaaccgccggtccagtcgggcatggcatttcccagctctgtgagctgacgcccctgtgtgcgcaatggcaagcccgtagcaggatctatcagccggttgccggcttcatctttcagccaggcgaagcctgttccgatcatagtgccgaaaggcttacctggtgcagctattacgttgatccccctatcacttcccaatacaaatgtttccacaccttcggtgagtgataccacttcatttttgttgcgggaaaatgtaaaggtgctttcccaggtaaatccattggccagcttcacgggtgttccgtttaacgacagttcaattcccttgttgcggatttcgccggcattgatcctgcgcgcttcaaatttgctggaaggcggtaagggcacatccaggatctggtttttcgtagcggcgttatagtaagtaaagctgatgcccaggcggttgttcaggagacgtacgtcggtaccaaattccaccgaggtagtcagttcatttttcaggttaggatcgggaataatagaagtaaaagatgccagcggctgacccccatgtgtgaactgatccaggctgtaggcgccggtgagctggtaaggattaccagagctgccagcctgcgccagcgatccgcgcagcttccagaaactaacgatgttgctgttcatcttcagcaggtcggtcatgattaaactggtgcttacagaaggataaaagaaagaattgttacttgcagacaaggtagatgaccagtcgttccgtgcggagaaatccacgaaccagtagttccggaaagccagctgcccgaagccgtatacggagttgatctcagattcctgtaaatcgaaaagataggaattggtaagcgtgttattgatcacatgcaggtccggcacaataaactctttcccggtattgccggtcatgcgcataaactttttctggtgactggcgcctgcattcagccccagggtgaagtccttgctcagctccaggttgccggccagcaatacatcatagttatcttcccggacccttattatccggtcttcaatatcaccattcctgttctggctctggtacgtgcctttggctctccagcgcaggcgttcttctgtataaaaatcggtaccgccgcgggcagttaatttcaaccatttattaaaatcgtacgacagccgcagcatccccaggagccggtcgcggtgatcggtgttttgcgttttatggatggtccagtaaggattggcggtagaactgttggtagcgtatgttttctccagtccgggtgttacgccgctgtagccgaactgccgggccacatcctgggcggtccaggtataatcggcgaggatgctcagcggcatgctccgcggctgactgataaacaggtaagccgggttatcggatgcatcggagagtgtgggcctgtttttacctttctgggagatgtagttgagcttcgcatccagctgtaatttgggcgtaatagacgcctgtgtgcgaagggtaaaagtgttcctgtcaagcgtgttagtgggcacatacccgtttacatgcgtgttggaataagagaagcggtagttcactttatcatttccaccatctgcggcaatattatttacgaattgtttttcctggtcgaaaaagtctttataggtattgggttgcggcgtcagcttcaaaatatttccccactggtcttcatactcctgcccttccatttttgggccccagctgctgcgggcaatcctgtcgcggccggcgctcattttaggcatgccctgcagcccttgtgctttggcttgcgccatcgtatacactttaccgtcggtggcgcggaagtgcgtgaaatcaccgtttaatccctggccatattcatcctggaaatcgggagttaccaatgcgttgccgatggcataatcgctgctgaatttcagcccgatgcctttgcgggagctgcccgatttggtggtgatgagcactacaccgttactgccgcgctggccgtacaatgctgcagcattagggcctttcaggatggatatgctttcaatatcttcctggtttatattggagatgccatcgccatagtccacaccgccggtgctgccggcagcaccgatgttctggttatcgaggggcactccgtcaactacgtatagcggctgactgttaccctgcagggagttatttccacggatcaggatcttggaagatccgccagcaccggaggctggctggctcacctgtacaccggccactttaccggatagcgcattggctacattcacttcctttccttccgacaggtcggcgcctttcagctctgctacggtgtatccaagcgacttactttcgcgcttgataccaagtgccgttaccactacctcagacaaaccctttgagctttccgttaactttacatcgagcgtggtgctgccggcagtttccacccgttgtttgttaaacccgataaaggagaacaacaatgcgctggcgccggagggcagctggatggtgtattttcccgtagcatctgttacggcgcctcttgcagatccttctactgtaacggttacaccgggcagtggcacacctttttcatcggtcaccctgccggtgatcaaggtatcggccgccagttccgtggcagcttttttcaccggcacctccttcagggtaatggtgcggtcgatgattttatattccagcggctggcctgccaggcattgattcaacaccgccgttatttccgcatcctttacgttcaaagaaacgggagtggtgtttttcaggatatcattgttgtataaaaagtagtagccggtttgttgtttgatagcgtcaaacacctgctgcagcggtactttctttaccgacaacgtaactttctgcgcataagcagtggctgctgcacttaatgcaaaaagaaaaagcagcagggtggtcagcttcagggccaccttcatttttacaggcaatgggagtagtataccccgcccggaagcggaaataaatctgttcatcatcggtttaatttttaattaatagcgattgattcgtttaaattctggtctttgtttattacaggtacttttttaattttcgtgtgtccgttccagttatacttatttattttgacagtgttacagtgacgtcttttccatttaccctgaagttggccccgctcacgaagttgagcatttccagcacctgcgacaacttcgcctggcggctgatattgccgctgatgcgttttgcgggcagcgggccttcgtaatgaatgtccaggtcgtaccagcgggccacctgttccatgatttcccggaaatcgtcatctttaaaaaagaagatcccttctttccaggcgatagctttctcagtatccgctgcggcgatacgtacctggtcgccctgcacattagcctgctgaccaggcgccagctgccaggaacgtttatcctttacctggatttttacagcgccggtgatcagcgtagttttcaccactttgctgtaagcgcctacgttaaagtgggtgcccagcaccagtacttccatctgctgcaccattacccggaaaggtttgtcaggactggcagctacttcaaaatatccttccccggtgagttctacccggcgttcgccattagtaaagtgtacggggaaacgcagggaggaggcggcattgagccatacgcgtgtgccgtcttccagtgtgagctggtattgccccgcctttgcggtagacaaagtattgaatagcgcagccccgtgcggttcatttgatttattgtatacaagtccgcctggttgctgcgcaatagtggttccatccgcctctttgatgggcccttccggctgattgcccaggtgtacggttttcccgttgcccagttgcagggtggcactgttgctgccagggaggacatcattttttatttgtgaagaagtagcggccagcattttcccgggtttgctatccggtgtgcgccaattgtaggcgaggatcacgcctcctaatatggcggcagcggcggccgtccatgcagcgatccggcgccacgctaccctcctacccggagttgccggagtggagcgggccagcacggcctgccagtcggcatccacatcaatggtatcatgaaaggcgatcgcatcgcgcagggtttcctggtctttcagggattccagcagctgctgatgccgcacatccttttccagccaggcttccagctcctgctgttcggccgccgtagcctgttcccggagatattttaaaattaagccggcgtatttatacagatcctggttttgctccataaaggttgcttaccaggtaaagaaacgcgggacggaaaaaagggtgaaagaaataagaatatttttttgaaagcaggatttacaggaataatacggcgtaaatttcggggttaagccgttgtcttaacaggtgcagtcctcttttcttctgggttttaaccgtattaatgctgatgttcagctggtcggcgatttcctggtttttaagcccggagatatagcccatcctgataatcacctggcaggcttcgggcaacgtttccagtgcgcggttaatttcgccgatcacttcggaccggatcatcgttaaaattacagaaggatcattttctgacgcgccttcctgtgcggctgcaaatttctccaccactttctcatgccggatggcatttaaacaggcgttacggacggttgtatacaggaaatttttgatggcccccggatgcgcggttacctgcccctgttgccccaggtagcttacaaaggcttcctgggcaatatccctggctgcgtctttatcgccggtaaactgaaaggcaaagtagcaaagcctggtatagtaagttttgaaaagtatggctggctccagtgcatcggatggcgttgacataaaatatacctttcgtgatcaattctgacaatccggaaaccatagataatggcatctcacttgaaaaaataagacatttattcggaaaataataggaaaacaaatatttcgggcagaaagaaagcctgcggggtgcgcaggctttctgatatcggggatcgccttcggcgatggaaattgtctttctgcctgattaggcggatgatgctgattacgctgatttgattaacttttattttttgattttaaaagatttttatcaggatttgtcttcgggattgttttctaccggaggcagaacagaggtatctctgttttcttcagcggtgtgtggttcggtatccggttcatttgtaccggtgttgaaaacaacattttccttctctgcttttttgcggctgaacaggcgtctgaaaaatccgatgagcgctacaaacccaatggcaataaatttccagccggcagcaaggtattttaccaggatggcaaagaacccaactttcgccagcaatttaccagctacaaggccaccaatagaccatgccgccacgttatccaccttcggatcgaaatcgaaataagtattcccctgtgtgaaagtagccatgtgtaacaccttgccgatatccgcctttaccagcgggagttcactcatcgtgcaaaccgcattcagcgataatacgccatggcgccccagtatacggatctcgtaattcagcgtatgaccgccttcctggtcatcgaaacggatttcctttgcccagtgcagtaccttattctttttgtcgtagaaaggttgctgcgcccatccaatcaggtgaataccagagtatccctgcttggcacgttcctcattggtttccttctcgccttcctgcatgtttttcatcatttcattgtagtcaatcttttcggcgtcatcatccttcacataaccaatgtcttcgaattcaataataaaggcataactgctatccgcaaaaggatcagaatttgccgggaaaatcattcccagcgtattgttggcgttttccggcggattgccccaaagcgtagtgagcacatactggcttttttccttgttcaggaatttgaaacccgcaggcacattaatctccacctttccacccggcaatacaatagtgccggtttcatatttaaaagacttgttgacagaatcaacataattatcaagctctttttgataaagctccgttgaatcttcaatgggggcggctttagggacagccggggttgcatacaaacccagggctgcaaagagcaaccctgacaggtacaggtacttgaacataagttattaatatttacggggaccaatttgcgataaatattccatatccggaagaaaggaaggaatattacaactaatgttggagcagaggaaactatctatccctggtcttttttacataatttttcaattgcctcagcgcccccttatgtcctttccttccagctttttcaaaataatactttgcccaccggtcagactgcattacaccgtctccccatttataacaaagcgctaaattgtaaagggctttgaggtcttgttttctggcggccattctataccagtaaactgctttccgatgatcttctgtcacaccctggccgtagaaataactatatcccaattctctccaggcctcaatatctccctgttttgctgaaagtgtaaaccatcttattgctttctcataatcctggtttacatattctccggtcctgaaaaagagtcctacattaaactgtgcatccatatgcccctgcatggcggctttcaggtaccagtaaaatgcctcttccgtatccttccctacaccttttccataatcatagcaggtccccacataaaactgcgcctttttatgaccattcgacgcagctgaatgccagaaggcaaaaacctttttccagttccgccttccaggcgaaccttcaaaagcatagctgtatcctaaaagaaatcttctttgctgttcttttttactcaatacttcgggcatccttaaagttattatatatttttcctgctctctctataattttctttcggtgaaaagtagtcaaacctgtttacccgatattatttttctgctttataaaacaattacttaatttagttcacctgaatatgtgaaacgccaacagcgtaatctggaaaaccttaaaccaaaatctgtcgattcttactgtctttgttaatcataaatctgaacaatgaaaatgaaaaaccttcattccctgctagcaggtatgctattgctgcctaccctttttatggcctgcaaacgatctcccggcggggaattgcagcccatgaaagataaaaccaaatccggcctggaaaactttgtacccagcgcatatgccttaaacgttgtttactttgtgccttccgatggcgataccatcacaaactaccgggcacggctaaacggtattttacagcaggggcagcgcttctacgggaagtggatgaactattacggttatggcgaccgctcctttggcctggcgctcgattccgcaggtaaagtaaagatcaccgtagtaaaaggcgcgctgccaaaaaccggttatccttatgaaggaggcggcaacactgctatcggtgaactgaacacctggtttgctgcgcatccggcagataaacgcagtgaacacacgctcgttatcatgcccgccagcacctacgcttccgatggtgatcccggtggcgtacccttttacggcttgggccgctggtgctttgcactggactatgcccaaatggataccagttacctcggtcagaataccacgctgggcaaccgcgctaccaaatggataggtggcctcatgcacgaactgggccatggacttaatctcccgcataacaaagagaaagtatcggaagccgctgatccggctaaaggcacggcgctcatgggcagcggtaattatacctatggtaaaaaccccactttccttactgccgccagcgctgctatcctcaacaactcgcaggtattccgcaccagcaccgccacaggtatttacggcggaggaaataccactatcgatatcatcaaagccagttataccggcggcaacattgtgctgaaagtgaaattctcttccacacaaaccgtgaataacgtaaacgtatataatgatccggaaggaggaaatgattatgatgccgtgccatgggtggctgcgccttccggcgatagtttccagctgagtatgcccatcagtgaacttcatacgaagacaggcaactacgccctgcgtatccgcttcctgtataccaacggctcctctactgaaatctcttacccgtattcttttgtaaataatgaacctgtactggatatcagcaccaaagatgaactgaataaatcttcctggagtatcacgtatgtaagcagccaggaagacgatgggcccgccactaacctgcttgacaacaaccaggctaccgtatggcatacccagtggaaaacagtacagccggcgcatccgcatacagtgattgtaaatatgaatgccatcaagtccatacaaggattggcattccttcagcgggccaatcttaatggttcgctgaaagatatttcggtgtttaccagtactgataatgtaacctatacatcgaggggaaactatacactggcgaatgtaaacagtaagcagtatatctctttcggggcagctgtttctgcaaaatatatcaaaatcgtgaccgcttccaattactcaggctcacactatgcagtgctgtcagagttgggtgcgtggtaatcacatctcccaaaaatttaaacagggtacggtataatttccgtaccctgcttgttttatttcaattgctgcgccacatatacccggatggcctgttgcataaaactgccaaaagccggattggccaggccattcacttgcatataccgttcatcggtggcaagcagatcacccagcccgttgtaggcttctgcctggttaccggttttaccccagaattgcaggatatacctgtaatgcagatctatttcctgttgcacctgctggctggccggatccaggtgagagagcgatgccagcttttcccagttggctttaaagccttcctgtagctgttgatagctgtctttgtccatttccagtaattgcttttctgcatgcgctacctgaccgggccacttttcctgtgcttcccgccgccaggctgctgcctgttctttgggcagtcctgcatatagatcttctacgttcatgtttacattgttttttagatgagagatggttttctctactgtagccaccagggtttcgatgcggtctttcttcgacaaaagcatttgccggtgcccttccaacgcatggatcaggtcaaagccaggatcatccagtatgctggcgatatccttcagctctacatccagttcacggtaaaacaggatctgctgcaaccggagcaattccgcttcaccatacacccggtaccccgcggaggtacgcacagagggcgtcagcaaaccaatctggtcgtaatagtggagcgtgcgcacactcacacctgccaattttgccagtttatttaccgcatactgcttcatcatcctggtaactattagattgaaaacgaagttagggtatgacgtagcgttagagtcaaatctttttccggatttttttttgggagacaaaaaaacagccggcacattggccggctgctttatcttctcattatatcttacctctttttcctagaacccgtaccggagccccagctggatctgccatgggttaccacccggcaccaccacgcctgagttcacgtttacgttatacttataagtagaggtaacaggatcgaaaccacctaaagaataaatattctgtttgcccagtaatttactggtaccccattccttgttaaacacattggcgaggttaaagatatcgcaggatggttcaagatattgcttcttgccaaaccggatctttgtagcaatcctcagatcccatacgccatagaaaccgtttacaccaccatttctttctgctactttcccgctgcttttgcggatataatcttttacgctttcatccgccaggggattatctaaaatcgcctggagatccgtgcgcatcttttccggcacgctgggattattcacatcaaatacataggccaggtcgtttgagtttacaaagtcgccattcacgttaccgcctactgccagcgaataacgtgtgccgcctataccggaatagcgcacgcccacattaatgccccagaaagtaggcagggtgccgtataccactaccttatgacggaactggttatcggaataactcatggtgctgagattacgcggatcgtcttttaccatcagcgacaaggtagcagtgttggccacgtcgccgttgtaagaggtattgtctttcgcatcgttccacgtatagctaacggacacctctccgtctctgaaataacggaaggtaccatccaccacaaatgcaaactggtttactttaccatcgctgttcagttccagcacgcgtcccacattggtggttttacggcctttggtccagtcggtagcgccattggttacattgatagtagatgcgggtacatatacaccgcggttatcttcattcgacaaacggaagaaaggctgatcagccatgttcctgtctacatacatataattgtgacgcgcaatagtggtgaagaacgtcacgcccattttaaagcggtcggagaacaggtgattgtaggagatgttcgctttgtacactaccgggatcctggcatccttaccgttcatattaatggtaccctggcgcggcagcccgagcttgtcgaacatttccttgcctggtgcggttgacggatctttacggtatgccgggaaatcgggaacgggtacaccggcgccctggatatccacggtgagtactttggttccatcaaacagcatgttgttgatcatggcatagttgtttatgtctgatccaaagatggctgcaccaaagcgcaggtaatccgtatgcttttctttgatatcccagttgaactggatacgtggctgcagctggaaagttttcagcgagttgtcggtgctcagtccaagctcatcatacaccgtttggttaaagtttggcttgttcaggtaagtggtataatcggcacggataccggcgatcatttcaaaacccgggaacaggtaggtttgcatctgcgcgtacaatgcgccgctgagaatattctggttcacgctgggatcatctgccagtgccacttcgcgggcataacggtaaggtttcaggttattgaaattatccataccggtgaaataataacgcccgttcatttcactgccatacagtgagttcatgtggctgtacattatatctgcgccgaaagtatagttggctttattggtattataataaagattgtctaccagctggaatacgttattatagaagtgctccggtgaatagcgttgtccgccgagctggatagaggtaaataccggtttgttgtcaatagtggactgtaccctttccacgatggcgcgcggaatattctgcgccggcagttgatcgccgggtgaactctcttcaaaagtatacaggtgctgcaatttcagctcattcgtaatccggggatttaccaccgtacggagcgtggccagcaagctgttgttaacggcatgtgcatccgcatatacttcgtagaggttgatggcagtgttatcgtcacggcctaatggtgcgcggtcgtttacatagttatcgcggatagtgaggaggttccgctcgttgagctgccagtcgatacgcgcaaaagccgcatctgtaccgcgtttcttattaaatgacccgaactgcggcgtggaggccactccatatttgctgcgggcaatatcgaggtaggtatccagcgtagactgtgtaacgttgaaccgtttttcatccgccggcgttttgatatccgccagttgcagggggcgtgagtcggcctggtgatcccatgccaggaagaagtgcagtttatttttaatgataggacctcccagagagaagccatactgataggtggagaagtcgttctggcgcctgttaccgcgggcgtcgtatttactggacaacgcatcggcccttacgaaggtgaaggcgctacctgaaaaggtgttggtacctgatttggttacagtgctgatggtaccgccgccgctgcggccaaaagtaacatcatactgattggtgaccactttaaattcccggatggcttccattgaaatagcatatgggccgccgatacgggtgttggtgccactgctggaagttggattcttcgcagaggttccatcaatggtgatgttggtagaagagccgagctgtcctgccaggttgcttccgctgctcagcggcgaaaggtctatgaggctgctgaagttacggccattcaccggcaggcgggcaatatcccttgccgatacagtggtggctgcaccaaagttctccgttttgttgcggagtgcggcgccggacacagtgatctccttgatatccaccgcagatgtttgcatctggaagttggcgcggattacatcgccctggttgagtgagtagccggtacgtctttgttctgcatatcccatcgctgttacctgaatggtgtatggtccgccgagtggcaactctttaataaggtattcccctttggcgtttgaaatagtgcggctgctaaatccggttgattcgttgcgcaccaatacggatgccccgggaatgagttgtttggcattatcagagacaatccctgaaatcgaggcctgcgttgtttgtgcaagcaatggctgcctgatgatgcagcataataacagtactgacagaagtgtgaagataggtttcatgagcgcgaaaatattacaggataatttgaatattaagtgttcactgcattcgtaacataaagttcatatccgggaggatatgtctgcatcacactacgagcgatatggttgaatgctgctctctgctgatattaagatacgcaaatagttgggtattcacaacgcgtattttgtcttactcaggattacgctgattatattgatttatgggatttgaccacttttgattttaaaagatttggggagatataagcggaggttgtcttactcaggattaaacttatttcactgattacgctgatttgatcactttggattttaaaggatttggggagacgtaagcggaggttgtcttactcaggattacgctgattacactgattacgctgatttgatcacttttggattttaaaggatttggggagatataagcggaggttgattttattttttgagttttttaatcgtttgtctttctgcctgattatgtttatctttataatgtgtataaagcattgatatccagaccatttctttgatgcaacgcgtctaaacaatattgtaaaacccactctagcgaattgatacacaatacattacggatcaagtccacgtcatcttcacatcaacagcaggttataagcacgtataaagcatatgtaaagcaggcgtaaagcatctgtaaggtatgtgtaaagtatgggctatctcatcttcgcgccatctttttaaatataccagaaaaaagtataatccccttaaaatcaaacgtggtcaaatcagcgtaatcagtgaaataagtttaatcctgagtaagacaacctccgcgtttccgctcatatctccccaaatctattaaaatcaaaagtgatcaaatcccataaatcaatataatcagcgtaatcctgagtaagacaacctccgcgtgaaccggtccatcagctccattgagagtatagcctgctcagcagagcagggattgccgcctttgcccaggaaaaaggcggttaccttttctatcatgggttgctgcacatgctgcagcggatcaaaaatgaattcttctgtatgtccgtctttgcgcagggttattttactgccaaatacggggaagctgatggtgccggatgatccggtaatctcgcagcggtcctgctgatcagcgggcgataccgtgaagcaccacatgccgttgaacaccacgccgttttcaaataagatatgaccggtaacaaggtcgtcggcctggtttacaccggcctggtttacggcaatgccggcggcgtgttttggttggccgaagaaatagatcatcaggtccagctgatgcggggccagatcatgaaacaggccgcctccggaaatagcgggatctatccgccagttaaccgctgaatctgcaatgagggcagaggccggcggttgcagcatctgcagggatacaaaacggatatccccgatggcgttctccgacaacagctcctttactttgaggaataccggctgctcgcgccggtagtgtgccacgcttaattttacatggtatttgtctgctgcggctttcatcctgatggccgacgctgcgttcagcgtcattggcttttccacgtataccggcttgccctttgataaggccagcagggtgtattcctcatgctgcaaaggtggtgtggcaatatatatggcgttgatctccgggtcgttgatcagttgctccgcgttatcgtaccatttgggtacgccatgccgccgggcatagtcctgcgcctttgcggcgtccctgcgcatgaccgccaccagggaggaatgcggcactttattaaaagccgggccacttttgacttctgtcacatctccacaacctataattccccattttatttcttccataatggtgcttataattatgcaaataacataaattcattttttaaaacagggatatttatttcaatggccaagctaaagaaggaattttatcagcagcatgaggtaactactattgcgaaacaattgctgggcaaaatactggtgacacgtatcaatggcgttcgcaccgccggtatgattgtggaaacagaagcctatgccggtgctggcgacagggcatcccacgcatggaataaccgccgtaccaaacgcacggaagtaatctacaagccgggaggatttgcctatgtatacttatgctatggcattcactatctctttaatgtggtgaccaacatcgaagatacgccccatgcagtattgatcagggcgctacaacctgtagatggtatagaagtcatgaagcagcggtacaacaacaagccctccgccaaactcacagcaggacctggtagtctttgcaaagcgatgggtattgatgccagcctgaatggcgagagcctcacgggaacgaaagtatggatagaacccggcgaagacatcccggaggaagcgatgaccgtgtcaacccgtgtgggcgtgcaatatgccggggaagatgcatatctcccctaccgtttcagcattaaaaataatgattgggtaagcaaagggaaagggctgtaaagattattgccccatcttcttattaatttttccttccagcgatgaaatgatatttacacaatctcccaggcgcgaataagccgtgctgccatccagcgccaggtcctttttagtaacctccaaaccgccgaggaatgcttccaggtatgataaatactttggctgatcgccgtataacgcgttgtaaatttcttcgttgagcttatctccttccgcctggagtgcaggattcaccaggtcggttactccgcgcagcttttccattactgcactcatcctcactttaagcgcttccaggttataatcgtcctttttcccaggagcaatattgttcctgaacaagctatctgacaatgttttccgggctttccggtaattatccagttcctgtttcagggattccaactgttgattgagctgttctcctttttcacgtttgaaatatttatcgacatcactatccaggtgtttcacccaggtgagcatatgaaaagtgatatctgcaacacccggtttttctgattgtgccaatgcgctgaaggaaaagaacagcatacagcaaagtgctgatacggtaagtactttacgtaatttcattatgatgatttaatggcctgtgccaattaaaataagcaattttttgttatttctaatgagatggcgcatccgccgtgtaagtttctgattttatgttatattcggccatgtgttgcgagtaatatataatatacctggtgaatgttcaagaagatctgttttcgtgccgcactgtttactgttcttaccggttgcctgtcgtcccctgcccccgtgcataagggcaaggtttatatcagcaaagagggcggacaatacctgctgtaccgcgagggacaaccctttgccataaagggcgcagctggttttgaaaatctccgggaactacatgcagcaggtggcaataccatccgtacctgggatactttacaccttgataaaatactggacgacgcatataccaatcatatagcagtaatagcgggcttccccatgcctgtcagcggattcttaccctactataatgataccgctaaagtagcggcacaatacacggccttcaaacgtgtggtaaaccggtataaatcgcatcccgcattgctgatgtggtgcctgggcaatgaaatcgactttccctacaaaccggaatacagcagcttttacaatgcttataaccacctgctggaaatgatccatacggatgatcccgatcacccggtgaccaccgcgctgataaacttcaacaggcggtgtctttataatatccggttaaaggtgcagggcctcgacctgatctccatgaatatttttggcgagctgcgcgacctgcaacataacctggaaaaattttcgtggtactgggatggtcctttcctggttacagaatggggaattaacggcccgtgggagtcgcagttcaccagttggggagcgcccattgaggttaccagtaccaaaaaggcgcaacaatacctggagcgctaccagcaatatatgccggtgaaagacccgcggttcctgggcgcctgcgttttttactggggcagcaaacaggaggtaacagatacctggttcagcttattttcaaaagaaggcagcgcatcggaaacggtgtccgttatggagtacctgtggaccggcaaatggccggccaacagggcgccctcgttaaaatatatgctgctgaatggcaaaggagccggtgacaacatcttattaaatcctgacagcctgcaaaccgcggaggtactgttgcaggatactgctaccggcccgttacatatcacctgggaaatactggcggaagactggtacaccaacaacaaagatgcgtccaatgggcagccccctgttgcttacaacaacctgctgctgcctgcccaggggaataaaatcgcattccgttctcctgtaaaagaaggaccttacaggatctttgcaactgtttccgataataagggacattttgctactgctaatacaccattttacgtagtcagtcgataatgagtagtccatcacctattttaccaccctcccggcgcgaacgctttacgctacggctgatgatcctgctgggtgtatgcagcatgggttatctgctgttttgccttttaaacagggcgcagatagggtatgctcctttttactggatcctgatggcgggtcttttttttaactgcctcacggtactccatgagtggtatcactatttttccatttcagtaccggaaacaccggaaatggaacacccattcacggtagacatctttactactttttgcgcgggtgaaccctacgccatgatcgtggaaacgttaacggctatacaggccattacctacccgcataccacctacctctgcgacgaagccaatgacccttacctggtagaagtatgtaaacagctgggcgtaaaacatgtaaccagatttacccgtgaaaatgccaaggccggcaacatcaacaatgcgttgcggcaggccagcggggagctgtgcgtggtcatggacccggatcacgttccttcgccggatttcctcgacgtgatcgtatcacatttcaataacccggaagtagggtttgtgcagattgttcaggcgtacagcaacctgggcgacagtctggtggcgaaaggggcagcccagcaaacgtttcagttctatggccctattatggctaccatgaatagttatggtaccgtactggccataggcgccaactgcaccttccggagaagcgcgctggatgctatcggaggacatgccagcggtcttgcggaagacatgcacaccgctatgcagctgcatgccaaaggttggaaatcggtgtacgtgccggcagtactcaccagggggctggtgcctgccaccatgtcggcctattacgcgcaacagctgaaatgggcgcgtggcaccctggaattactggttacttcctacccgaaattgttccggtcttttacctggcggcaacgcctgcattacggcactattcccttccattatttgtccggcattgttttcttcatcaattttctcatccccgttctctccctgtttaccgggttgataccgttgcgggtcgactttatcaactttgtatggctgggattaccggccgttacagcgattatccttatccgtcattttgtgcagcgatgggtgatggaagaaaccgaaagaggctttcatgtggtaggcggactgctgctgatcggtacctggtggatttatatccttggacttgtatataccgtgatccggaagaaggtgccgtatattcccacccctaaagacgacaccgggcaggataactggcaactgaacatccctaatatgctggtgttgcttacttcgctggcagcgattgtttatggactgtcgtacgactggaacccttattcccttgtgatggccggcatagcaggcgtgaactgcctgatcatgagctttaatattattgccagtctccggctccggcgcttatccgtaaaatatcactggctggggatcgtgctcgtatacccgttactgttaaagaaacagttatggcttttccggcatcttcatttatatgccggtttccgtaaactggggctgcctttattgctcgtggtggtgttattaaccggttacatgatgacaaacaaccccgaaccggctgctgcaacgcatccacccacacataaacaaaccacattttataccggaatattcagtccagctgatacaaacggcctcacggcgattcaacaggtaaaggattaccagcaacagtttaacacccgctttaacatcatatcgttatacctgccctggggagatgcgccgcaatgtaacctgcctgactcactgatagcagccatttataacaacggttcgttgcccatgatcacctgggaaccctggacttcattgtttaaaaacgctgcagccggtaaagaacaaaaagtctttgcccgtatcagcgcgggggactttgatcaatacctggtgcattttgctgcgcagatgaaatcgttgaaccgcccggtgttcctccgctttgcgcatgaggcggataaccccgcctatccctggtcaccagccggcaacaacacgccggaagaattcaaggccgcctggaaatatgtacatgacctgttccggcgtaacggggccggcaatgttatctgggtgtggaacccgtggcgtgccgccgcagcggagcaatacttcccgggcacgctgtatgtcgactggatcggggtaacctgccttaattatggaccacaaaatgagaacgggcaatcctatgctttccgggagttatatgcgccgttccatcagctgccggtattccattcaggcctgcccgtgatggtggcagaaatgggctcactggctgatgccggtaaccagcaactatggctggatgatgcatttaacgccatcgaccatgcgttcagcgaaatacatgccttcgtattatttaacagcgaccaggataaaaacatactgcgtcctgttgcaggaaatatgctccgctggaaattacaggaaccgggaaaagtatttgccgccgcaaaaaagtatacccgtatccgtgagtccgaaaaacccgttgcttacgccagcatgatcaccacccctgcagccgggcggatggcggcagccataccgctgccggataccatcaggggaatcaattaccagacaggagaaaactggttcaggaatttacatgcccttacccggcgggaaatcatcaaagatttcaccggtatgaaagctgttggcgtaaataccatccgccgctttggccctggtgtgtacgaccgaaacatcctgcatgtggcaaaagaaatggatctgcacatccattacggcttctggatacctgccataacagatatggataaagatgctaccatgctttcggatctccggaaaactattcttaaacgggtagaagaattgaaacacgaccggagcatcgtagcctggaacattggtgatacggtatggcagcagctgtcaaaagattattttaaaccggagctgctctatcagcaacaaagctttcttacctggttaggcagcctgatggccgccataaaagcgatagatactacccggccgctgaccatagatgtagccattaacagcaacatcgccggcacactggaaatactgcaccagcaactaccgcaggtggacgcttttggcatcgtagcaggcaacgacaccacgggtttatcgcagctggccaccgtaaacgttccgcattatttcagccagatacctgtaacggcttacacccatttacccggtcgccggcaaccggcttttattaccagctggcaggaccttgaaacacgggactacgtaacatttgatggcctcacggaccaccagggaagatataaatcctctttttaccagctgggacgctactggcagcattccttccgtgaacctgccattccgcgtattcatatactccggccggcaaggactaattatcccggcagccggctcacatatcatgcgcttctttacagcaacaatgaatggataccggccaccgatgatacccctttaaagtttgaatggtacctggtaaaaacggatggttatggcaacagtatttttctgaagaaactgggcaccggcgccgatgttaccatctccatacctgaaaacccggaacactaccggttatacctggaagcaacaaaagatgatcaggtggctactgtacaatcgcagctgaatatcccgctataatctttacgccagataagccgtcattctatcacattcataatttctataatgaaaaaactattcataactgccactctgatactgacatgtatgctgtcgttccgcagcatttccatagcgcagcacaacgaccagcaactatctgcggtaatcctgcataacgatagccttttctggcgggcgtataatagctgtgatataacaaagatgatggaatatttctcagaagatatagagttctatcacgacaaaggcggcatcaccctgggaaaaccggctatggcccaatcatttgaaaagggagtttgtggcaacaaggaacaattcactttgagaagagaggcggtcgacagcaccatcaaagtgttcccgctcaaaaaagacggcgtgatatacggcgctatacttacaggttcgcatctcttttatatacataataaaggaaagaaagaatatgcagatgggttggcaaagttcaccgatctctggctgctgaaaaacggtagctggaaaatgacgcgggcactgagttacgaccacggcccggcgccgtatgtcaataaaagaaaggcccttacattaccggcggatgtgctgcgtagctacgctggtaaatataagggacctcaaaccacatccgaaataaaaacggaaaatggtttactcatcatgctgataggcgataaaaagttttcgctttacgcggagaaagaaaatcttttctttacgaaagaacgggacctcacctttgagtttataaaaaaaggaaatgaagtgataaagctgattgtgcgtgaacgtgacgacgtaacggaagaattacaacgggatagccaggggacggacgggcgccccgctcgcgcctcttaacttcagcggcagcccgataaaaacgaacgtgtttatttttgcggcagataattcttcgagatacaacaactctataaacattacccctttttgggccagcaggtaggtatgccccggcagccagttatgattattgccggagggcatcacctctacgctcaggttatcggcgcccagcgtcattacgcctttttcttctatcagccactttatggcttccatactcatacccggcgtgttgctcataaaccgttcggtatcgctgtagaaatatttcatgagccctgttctgatcagcacaatatcgcctttgtgaatgtcgaggtgttgggcctgtaccagttgctgcagttcggccaatgtgatcacatagtttccgggaagcacctccacgcctttccaggcgggaatgtcaatgagcacagcccttccgataatcggcggaatattttcggcaccgcctttatcccagccgcggtcgcccaggtgttcatctgcggtgtacccgttccagatcttaccattcaaaccaaagtgggaaagcgcatcgatgtgcgtaccggtatgcgtgtacatggagatggcatcaccggtatagcttacttttttgttcatatcatcacccagtttggtgacgttgcccacaacagtaccgcggggtgtatgcgtaagccagtattgataaggaggatcgcccagtgctgtgaatcctggcatccccgtaaaatattccacaccaagatcataaacctttcccgttctgatgttggagaacagggaaaggttattactgtcgctcatcatattcagcgtgcctatttcatctgattttccccaggggctcacccctgcctgttccgttgcatgcgtgctttgtcctgttgcggtgatagttcctgccaatggcatcgccagcagtaacagcttataccagctgtacccgtttcgtgtattcatcttcgttaatttttatgttacgcacacaaaattaaaggggaagatggccatgccgcaggtacaatgcggggattgtgctgtaacttccggggttggttttaccggtaatatccatgatgataataatgatgatggtgacgcggataatatccgggcctgtcgcgcacaaccaggcaactgcttaatccggctataagtaaaacggtaacgataagatattttaacgttctcatgatggcaaaatttgaatgtgtgatgaatagatggaagtttagcgactgcaggcggtttaagcttcttgttcatctatcataaatgataaaactatgccagagtgaaatgagaactgttatctattgttaacgccttgctgataccgggttacacgaggctgtacagcgcttccctgttgaatccctgcaattcatccaaccggttttctttcacctttcgcacccagtaaggatctgtaagaatagaccggcctactgccaccaggtcaaattcgttatcatccatcctgcgcaccaggttttcaagagatgccggcgcggagtcctcacctttgtgcagtgaaataatatctttatccaaacctacggaacccactgtgatagtggctttcccggtcagtttttttgcccagccggcgaagtttaatcctgatcctgcaaactcaggttcccagaagcggcgcgtggaacagtggaagatatcgatgcctgcatctgccagcggcgttaaccaggcttccatttccgccggcgtagtggcaagtttactatgcaggtcggtgagtttccattgcgacaatcgcatcatgatggcaaaatcttctcctacctgccgccgtatttctttggtgatggcaacggcaaaccggctgcgttctgccagtgttttacccccgaaaaaatccgtccgcgtattggtgttatcgcggaaaaactggtcgattaaataaccatgggcgccctgtacttccacgctgttaaatcccatgcgttttgcatcggcagcggcgcggccaaaggccaggatggtatccgcaatagcggcgtcggtcatggctacaccgttgcctatcccggaaggaccttcaaacggcgccggcggcagccatccggaaacatggttctcctggatgccgcagtgccagagctgtggcgccatctggccgccggcagccagcacactgttgatcacctgctgccagccggccagcgactcctcaccataaaatttagggacacttgcttcattcgcggatgaaggccggtcgatcaccgttccttcagaaatgatcagacccacttctccttcggcacgtcgtgtataataatttgctacgtcgccggcaggaaccccgcccggagaacaggaccgggtcataggggacattacaaagcggttctttgtatgcaatgatttcagggcaaatggcctgaataagctgctggtattcatattgcgttgtttatagcctatgacgaccgacatcgccaaagggggacaacgcatgttaatattcgccgaacaatttattgatctctccataaggctttgcctccgctgcatagctgaaggtgccctggtgaagtatttcctctgccgcccggaaaacggcgccatatgctgcccttatgagcgaggagccaatgcttacacgttttacgcccaggtcttccagctgccgcaatgaaaagttaccaccggaaagtcccatcaccacgtttattggacggggtgctaccgctttaaccacagcggctatttcctccggcgttttcagtcccggtgcaaacagcacatcggcgccggcgtctgcgaaagcttccagccgcctgatagtatcttttagatcggggcggccataaatgagattctccgcccgcgccgtaagcataaaaggatgaggtaagctccgcgctgccgctacagcggctttcacgcgcgccacagcaacatcaaaaggatatatcggatcttccggtttaccggtggcatcttctatagaacctccggccagcccggcttctgcggcaagcaatattgtttcggcacataccgcaggatcgtcgccaaatccattttccagatcggcagctaccggcaaagcagtggcgctgataatgtcccggacgttttgcagcgtttcttcgcgggtaacagccgcgtggccatcgggtttacccaaggaaaaggcgaggccggcgctcgtagtagccagtgctttaaatccaagcgtttccagtatccttgcggaacctgcgtcccaggggttgggagcgataaaaataccggcgcgccggtggagtgcctgaaatgcttcggcccgggcgcgtaatgagttttctgctgatggtttcatatcggatatttacccggtaaatataatcactcctgctctcccaacatatgcgccaatattgctgcgcatttctcgcggcagggagcataaaaatgaccatgttgccagtagtcggatttgggcgattgtccccaccagaattcggccagtgccaatggctccatcccatgctgaaaagcatattgcagcaacttcggggcggcgcattcgccggcgcccgctggtggtttcccggaaggcgtatgcgcaaaaatctctgttaaacttttagatgtccctgctttattcagaaaatgatactgttcaaaaattttgtgctgcagtgcggtagaatggtttttccttaatattttgagcagacggacctgcgctgcgctttcgtcgtcggtaaacgattccaggaggctgatttctttgttgatagcggtgagttctaacatgccggtattcacaaacccgcccggttcaagcccatcgaaaacgggtggcacaaatttcgcgtggtggttgccacctgccagtttacccgagaatgccgccaggtaacccagctcattatccctggttctaacgatcaacacgccgaacatctttccaataacggtacctgccgcattacccggcaaaccaaagttatgctcccactcctgctgctccaaatgcgcctgcaaacgctccgctgccagcaggcaaagcgggtgcggcgcatcgttcaatgaaaaagtaagccctgctgctaattcactaacggttgttgattcgtcgaaagggctgaatgccgatggctcataactcacactatccattaccaacgttgtaaaatttaataaaaaaagcttcagtataatctgaagcttttttatctatgacccttacgggataatatatgtcttaaatgcagctttccgggatcgcctcccggaccagcgtcacctgctcagacctgaaaaaacttttaatcgccgcaaaggtactaaaatacaggctgccaggctacatggattctttaaaatttaaaggcaatgccaagcatcagccgccgtggcatctgcgggttaccactggcatcccagtagcgctgatccgacaggttatctgccttcacagaaaaacggtaacgttttgtattataaaacaccacggcgtttaaaatggtgtatcccggtaccgtaatggtgttaagatcattccagaaagcactgctgctgtagttgccgccaaagcctgcaccgaggccgtttaagcgcccttttacaaagctatagctcacccacaggttggctgcatgcgccggcgggccggccggccgcttgccctcataccctttattggttttcaggaaaagaatatcattgtaagcatatcctgccactacgtttaaaccaggcaatatggtgccggtaacttcggcttccactccacggcttttcttggtaccatcctggatactcgccgccgggttaccagggtcctggcgcaccacattctccacgagtatattataataattaacggtactgctgagccgtccgttcaacagctccattttcacaccgccttctgcctgccgtgcattttccggtttgaaactgatcccaaaaatgtcctgtccatacacattattaaacccggtctggtagttggcaaacagggaaactttgtcttttatcacctcgtaggtggcgccaaacttcggtgacagcgacgtttggtcgtaatcgcccgatacttcgccggtttccagtacttctgttccttttttgttatcgaagtagttgatccgtaagctgagcaatacatttaacctgtcggtcagggaaataacatccgttacataggcggcataactcaccggcttgctgagggtggttactgctgccgcttcgccatctgccagcactttggcggcatttatcggcggcacaaaggattttgtgtaatccagtccgtctaccagtacggtatttcccaggggcgaataacgggtgtcgcggtgcaggtaatccaggcctaccagcaggcggttacgcagcttaccaattttaaaatcgcccgtcaggttaggttgtatagccagtgatttggtggcattggaaaaagcgccgtaatagcgccagagactatctttcttaaaattcaggaaaacattaccgatttcgtagttgtagtcggagtagtttacattcacatccagcttccagtcatccgaaaagcggtgggtgatctttgtataaaagctccggatattaaatacgccactcagcttattagagccataggatttaaagtaatcgcgttgtaactggttgatgtttgtaacacccggcacatcgataccgcttacccgcaccggtgaattggctttcatgttgagaaattctgtactaaagagaacatctgtgcggtcatccagcttataggaaaacgacggtgcaatcgtataggattttttaaacccataatcctggaaaccgttgtcccagctgccggcggcattaacgcggaagagtgctgttttatcttcattcagcggcgtgttcacatccacggttaggcggctgtagccatagctgcctagattggcatcgatctcaccggctcttctgtcgaaaggttttttggtaacgcggttgatcaacccgccataagaaacaccgttggcgccaaacagcgtgccggaagggcccttgatcacttctattctttctgtgttcaccggatcagcgttcactccctggtccacatacatgccatccctgaagttatcgctggcaacaaatccacggaggtatacccagctgttatatccgggtcttattaacgcaccgctaacgccgggaatagccctcagtgcagatacatagtccacgatggcctgctcctgcaataaagccctggatgccactgaatatacctgcgggttttccaggttgcgcagctgcattttagctacatactcactttccttatctgctacgcggtactggtttcccaccactaccacttcccccagcgaggaagctgtttcttccagctttatagcgggaataccggtaaccgctgcatcggtgattactaccggctgttccaggcttttagcgccgataaaagaaacagttaatgtataactgccagcaggcgcctttatttcaaaatgtcctttttcgttggtaacggtataataccgggtggactttaaccccaccgttacgccgggcgcgggtttaccgtcggccgacagcacatgcccctttataccggtaacgccattttctgcctgcaggaacaacggtaacaggaataaaagaaaggtagagatgcaaaaaaagatataaggttggcaatgttgcttcatatttaaaatttagtattgcaaagagaatacatgtggcgccacggagtttatctaatccggaattttacggcggaacaggtttgaggcaacagatgcctgaaaaagcaatactgtacctgtattccttgaaggaaaccggaaattgcaaatgctcaaatcagaaaaaaaacgtccggggctttcccgtcaaaagagcttacttttggtaaacaaatcaaccgccaggccacagcaccccaaaacactgattgccggcaaacgccaggcatcaggcactttcactatcaatggcacaaggagttaagacgaatgattgtaatcttttaattaaaccccacattatggaacaagtacttgaacaaatccgtgatcagcaaaaggacgcctggaataagttctctcccggctggaaaaaatgggatgaacttaccatggacttcctgcagccaatgggcgatgaaatcatccgtgcgctccaacttaaagacgatgatacagtgctggacatagccgcaggaaccggtgagccagggctcaccattgcctcaaaattgaagaacggtaaggtagtgatcaccgatcttgctgaacacatgctggaaatagcccgggaaaatgccgccaaaagaggtatcaaaaacgtggaaacaattgcctgcgatgtttgtgaacttccatttgccgacaacacctttgatgctatcagctgccggtttggatttatgttcttccccgacatgcagctggcggcgaatgaaatggtacgggtacttaaaccaggcggcagattagccactgcagtatggaatgttccggagaaaaacttctggattaccgcaattatgggcaccatcaaccggaatatggaactgccgccgccacctccggacgcaccgggaatgttccgctgcgcaaaagatcagctgatcgctggcttgtttgcacacgcgggactaaaaaacatctcccaaaaagaaattaccggaaaactgaactgtaaaacaacagaggtgtattggagtatgatgaccgaaataggcgctcccattgtggcagcgctcagcaaatgtgatgaggccatgaaagaaaaaataaagagagaagtatttgctgccgtagatcagaaatatccctccggagaggtgatgatcgaatccagtgcgctggtgatttatggagagaaataatgatgttgttttatattgatgaaaaaattattaaaactcgcaggttttaatcaagccattggccagtgtaaacttttttgtttcgccgtcctctttaatttcaataaacttttcgagtcgttgtgaacgacccactatataatcctcatcatagtagtagttggtggtttctcgcaccgggccgttctgcgaggtataagaacctgtatatacccgcgcggttttccgttgattgaaactgtggatcagttgtacgaagtatttaccgggtttaagtccttcgaaagcaaatttaccatcggagttggccactgcttcgatagagtatttgtttgcttctttcgacatataaacgcctgttttcctgctctctttctgatcgcgcaacttatgccattcttccaggtacggcgtaaccgggaacagttttacgatcaccccggcggcagggaatatcagcccgtcttttttggtgcaggctttccctacaatccttgataagccccggcctagtgcggcttccgccaacttagcatcaaatgttccctgtgggaatatttcgctccgcgttttcccggcagacgcagtgatctttccacccaggtcggcatacttcttccggtcgaggtccgcctgcttcttgctgccgatggcatcgtaagcatccgcgcggttgaggtaagcgaggatatttgccgggtcggcttctatggcttttgtataactggctattgccaggctatatgcttgtttgtcgtggtgaacaacgccaatattcagatacccattggaatagccagggttaatttcaactaccttattgaaatcggccagggccaggtcactttgttttttattattcaggtaaatattaccccgttccaggtacgcatcggcatatttcggatccagtgaaatggccttgttatagtcgttcagtgcggaatcccactgttcccagcgaacgtaggtattaccgcggttcacgtagtaaagcgcattctttgggtccagctcaattgctttgttgtagtcgctgaatgccaggtctcctttttccaggataaaataaatattcccccgattcccgtacagggaggcatctttaggggaaagctcaattactttggcgtagtcggccagcgcttcttcgtactttcctttcttcttatacatcaccccccggttgaaataggcattatcatctttagggtccagttcaattacttttgtgaagtcggctattgcctgatcgtactgctgctgcccgtaataggcattgccgcgggcaaaataacagctggtataagtggggttcaccgtaatggcttttgtaaactctgcgatggcagcatctgcctgtttcctgtcggaataaatccagccccgctttacataggaaagggcaaaacgcgggttcagctcaatggacttactataatctgccagcgcggcttcctcattctttgtgttttcataaacaattgcgcgggcatagtattcaatagcagattttggtgaagccagtaaccccagcgccttttcaaatgtttttgccgacaggccgtcattcttctgaagctgataaccgattgcctggaaagtgtaatagacgccgttatccgggctaagtttgatggcttcattaatatcctgctgtgcggaggtcacctcatttgtagcaatctttgcccgcccgcgaacggcataggccaggccactgttcttgcctgagctgatggcttccccggcaagagtttttgcttttgcaaagtttccttccataagcagggttaacgcattatctgctgttgagctattctgaccggaagcggtggacagcattccactgataacaaggacgacggctggtattcgtttcacgaaataacggatcatatacattggcttaagtaacttacgtgggtaacaagaaatgttgttcgatgattaacaaaaatgcacaacattttgcccgcaaatataatgcataatcttaaacgccaaagtactcccaagaggctatcgttaaccaggtatatttaagtacccggaaagcactaactgattattaagtaaaaataaaggggacctgatggccccctcttaaaaaaacggttatcttcttttccttcttatcatcattatcactactcctgctacaatcagcgccgggaggaatcctaccagacccattttgagatagttgacaccggtagcgctgatccgcaggtcgctatctgttaacggcgggcgggaagtatccaccgggaacaatccataagtgaaccaacggaacaactccgtggtaaacagaaaattggcggtgcggatattatttctcagcagttcggcattactcataaagtcagcatctgccgaaacaatgatccgttgctgacggccattatgttctcttgttaaagcgactgtcatcgggaaagcgccccgctcatcgttcagttcaggcgtgaataccgcagtacgcaggctgtcgtcgataggcgccgtgcgtttgaatgtattggcggtgttgcttacaatcagcggcgtgatgtgataatcattgttggcattgccggcaatactgcctgcacccgaaaagctaataacgatatcatcctgttggaaggcaggtgaattacctaacagtttcaatcccggtgcagagagcgcgcattgaacaaaccgcggtgacagatcttctgttttctgcaatatagtgccgggttcaatgctcatgcccagtgttgacagcagcggattgaggtattcccgcctggaaggctccccggcaatcagcaggttaccaccgccatttataaacgttgttacctgttgcagctgctccggtgaataaggcatccccggatctgcaattaccagcaccgctatatctgacgggatactatctttccccaggtaaatttcctgtacggaaaagccctggttgagcaaggcgtagcggaaagttttttcaacggtagatagtttgtaatcattatctgccatgcgcttaatgcttctttcattatgccctgttacaaaagctactttagccggctctgttaccagcctttttatagcggcggtaatttctttttcatcgggctgacgcatcaggtcttcataaattctaaggaaggtggttttaccgttgtattccagcaggcgcagggtcctgttcccctctcccgacagatcgatttttttatggatttgcgccggcgtaaggaaatcgttgatatccagtttatacgacgaagctacgcgttgggccaactgttcggtgttcagtcctttattcctgctgtaaaggtcaggattgctggtgctatcgtagtagtaaatatatttcatgcggatatccggtctgaaacggaagtacttatcaaatctttccaggtccgaattacggaaaatgggcgccaaagaaaagtagttggcatccagcaggttcacatatgccgtgatcgtcagcgggcctttcatctgtttcagtacatcctggctgccttttgttaacgtgcggccattgttggcggtcatgtccttatacgccactacacccgggcggctggtaacatagccggccagcaaggcgcatactaccagggcggtatagcgcgccactttcaccagcagcggtttcgattccttaccggcgcggagttttaatatcgttaaccccacaaataaaagtatcacgataataaaatagaaaacatccctgctggtaattaacccttctacaaagttttctgccctgccggagatggacaggaagtaggtcaggtcgcggataaaatccatgtcctgccataacttacctatatagttcaatccacctaaaagcgcgagcgtactaatagccgccaccacctggtaggtagtcagcgacgacataaacagtccaatagccgaataagcgcagatgagcaggaacagcccaatgataccggaagtaataaatgacccgtccgcgtctttcacgatataggaagcaacaatacctaagatcacgaaacagcacatcagcaatacacaataaaataccatggcgaggtacttaccccatacgactgcacttaattttacgggcgatgaatataccagtttgatagagccgctgcccgtttcccggctgataaggcccatcgttaaaagcgggatgtacaggtacaggttttcctgcatctttgtaaacaaacctgaaaaccctgcaaaaaaggtgtgggtcaacccactgcggttcattcccaactgctgtaccctttcgaaacgttctaccatgctggtgaactcccaccccgactgcaccataaaaatgaccagcacaacccatgcaacgggggaataaaacagattgcttagttccagttttgcaatccttaatgtaagtttcataagtactgattataatgatttaaccttgtttgataattttgcaaagatttcttccagcgaacttctttccagctggatttcccgcagcttccatccgttgcgggcgctgagttccactactgtttccgcgatttcaggcgctgtatcaaaatgcaaacgccaccagccgttgtctgttggcaatgcgccggtaataccaggtatcgctttgagtacagacagctccggtgcattgctgaagtacagcagcatggagttgggagcgatataattattgaagtcgtttacggtaccggtaaaaaccaccctgccctgctcaatcattttgatggtatcgcaggtagcctgcacctccgataaaatgtgcgacgaaaaaataaccgagcgttcctccccgatttctttgatgagcaggcgcacttccgcaatctggttagggtccaggccattagtgggttcatccagcactaccagtttcggtttatgaatgatggcctgtgcaatgcctacccgttgtttatacccgccggaaaggtttttgatcagtcgtttgctgaagtgcgcaatcccgcaccgttcctttgcctctgtcatagccgctttgatacggtctttcgggatcagccgcatatgcgcgcaatgtgtgaggtattcatctacggtgagatccaggtagagcggcgcattctgcggcaggaaaccgatcagcttcttggcggctatcgggtgttcacgcagattgatattatcaatgagcaccgatccttctgtttgattgagcacaccgcaaaggatgttcatggtggtggatttccccgcgccgttagagccgagcaaacccgttattcctttatgcctgatgtccaggttaatgtcttttattgcccaggcggtactgtacctgtgcgataaatgctcgattttaacaatacttgtattcataaatgattgcttagcatggtaaaggcaaagtatggacaggggcggccggaaccgcccacaggcacatactttggagtgatcagtatcggatgttagttataatccggattttgcaccaggttaggattggcatccacggcagattgcggcaacgggaaataagcggcgcgcgcctgccaggtactctttttggcgcccagcaccgcattgatccggccggtacggcgtaagtccatccagcggtggccgaattcattaaaaaactcgcgccggttttcgtcttcgatttcaagccggactacgttttctgcggtggaaatgctggcagcagtattagcgcgtacacgtaccacgttcagatcggtccttgcatcagacaggttctgctgattaagccgggcttctgcacggatcaggtattgctctgccagccgtaatgcggtgggcgcctcctgtttgccggccgctgttgcggcagcgatcgacgtcaggcggtatttataggactggtgatttaagacgccgctgaaggtggtatcttttatccattttgttctgcgcgcatctgccgcatcgaaaatacctgccaggtcgtctgtgagtgaatattgagaagtattggcaacgaaagtgtagccttcgtaagtataaccactggtgatgctgagataaggtccgaactggaaaatggcttcggcagaagcttttagaaaggtattctccaaagtagcggcgggtgtcatcgcataaagcgaaccggcgttgtctattactttggatgcttcctgttctgccagtgcccactgtttattatacaggtaaacccttgccagcaaagcgcttgcggcccagcgggttacactggtgcggaagcctgctgctccgctgtaatcaagcggcaaatgatcacgggcgtccagcaggtcagtgatgagctgcgtattgatagccgccacattggttttaggcagcagcgcagttttgcttacatctgtttgcagtaccaacggtacttcgccatagagatttacaagataaaagtagcagtaagcccgcatgaatttcgattccgccaccacccgttgtttaaccgaatcggataaagcggcactcgccgccgctccttctatgaggctgttaaaacggtaaatacccgcgtacagatctatccagatcccattgagcgtactcaccgccgatgtgctggaagcaggtacataggtgttgctggtaagctcgtcataattggtgttggcgagatagatcatatcgtcggatgccagtgacgtcatggacgtaaggttaatagccaacgtttgtgaaccgaaggcactgctgaatgcgccggataaagccgacagtgccagcttatcagacgtaaaaacacgtgcagaagaaatctccgttaccggggcaggaatgtctatcagcttttcacagccagccattgccaacgttgctaccaaacctgcgattatttttatagaatatattttccttaacatgtcatcaatctttttaaagcgaaagtttaaaaccagcagacagcgtgcgcaaaggaggcagcgaagtacctcttgattccggatcgaagcctttgtaggatgtgattgtaaagaggttctgcgcctgcataaacaacctggcctgattaatccgcgcacgtttcagcagtgacggtgaaaaatcgtaggaaaaggaaaggttcttcaaccttacaaaagatgcgtctacccaggtagcatcggagccaaaatagttattggcaacagggctataggccgccagcacatggcgttgaccggggcctccatcggccaggtaatcatccagtacatccctggaaagattataactaaatcccggcggatacgtcatagaagatccgagactgcggcctttctgttttacaaactgaaaagtgaaatccagtgtaaagtttttataactgagcgtattggtgaggccaccgaaaaagtcgggatagctggtacctacgtaataccggtctcccctgccaattgcctgcagcccaaaggtgatggctttatcattatttaaatctgctacaatgggaagatcagtagcaggatcatacccggcgtatttatacaggtatacactgcttaccgggttgcccactacgtaactggtgtagtaggaagttttctgaagattggggaatgctttcagtttatttttgttggcggagaaattaaagttagatgtccagctgaaatatttgttccggatattcacggtattcagcgagatctcccatcctttgttctgcacatctgccggcagatttgcctggtagttgctgaagccggcctgtgtactgatagtatagctgataagctggttgctggtaatattattatagtaagcggctgttaactgcagtttgtcgtccaggaagcccagttccagcgccccttccagtttgtccgtttgctcccagcggtagtcgctgttggcgatccgtgagggcaccaggcccgtaacgccgttaaatacataaccggtggtactgtaggaatcgagataggcatagttgccgatattatcgctgccggtgataccataactgccgcgcagtttaccactgcttaaccatttcaggcgatttttgaagaatgattcttctgtaaacaaccaggcggcgcccagtgaaccaaaattaccaaagcggctgctgggtccgaaacgggacgagccatcgcggcggaagataccgttgatcacgtagcggtcgttgtacacataattaagccgcgcaaaaaccgatgcaaacttataatcggtagaactggagcgggtaaagatactcgcagcagacgccaggttctcgataaaatcatccgaagtaaaatccgatgcaatggtataataaggctggcgtgacatacggtattgccaggagccacctattaggccggaaaaatggtgggcgcctgatgttttagtataacttacctgcggctctataatgtagttattggtataactatatacaaaagcagcacgggcagcgttggtggcatttgtctgatcctgcgacgactgcggcgtaagctgtacctggtccatatctgaacggccaaaaccaagcagcgttttaaactccaggcccttcaccggcgtataactcagattcagggcgctgttcaggttagacgatttattacggttggtccgcatcatcacaccgaggggattttgcgaaaagaaatcggtggaccagtacaggctgccatcaggcttgtataaaggaaagttaggcgctaactggtacgcacggctcgtaagatcttctatcgccaatgtattattatctgccacatacatcgctgaaaatccaagtttaaattttctatccaaactgctgtggttaatgctcaggttagcggcaccacgtttgtaagatttatccaggtaatacaccgtggtttccttgtggtaggtacctcccagcagaaagttcgttctgtcgtcgccaccggatatactcacgctggcatctgtgaaattcgcggtgttcccgatcagcaacttctggaaatttgtataagcatgctggtcccataccagcaaatcctgtgcattggcggtggtgggcgtaatattggaatttttaaacccctgtttacgaagcgccagaaactcctctgtatttaaagtaggtacgaaatgcgctacctgcgacatcccggtattgagattcatgtcgatcctggttttacctgcacgtcctttttttgtggtgatcaatatcaccccgttagcgccccgcgaaccgtaaatagcggtggcatcaccatccttcagcacttccacactttccagatctgccgggttaatactgttcaacggactggtaggcccgttggcgccattgagcacattacccgtttgtgcattgatggcatccgataaaaacggtacgccgtctacaatgtacaatggctgcgaagtacgcagcagggagtttacgccccttacctgtacatcgatcgatgcgccggggtaaccattattctgtacaatggatacgccgggcatacggccctgtaaagcctgcaatacgttggtgacgggctgttgctctattattttagacgttacccttgttacgctgccggtagataagcgctgtgattctgtgtagtagcctttattgatcaccacctctgaaagcctgctggtaaatggttccagcacgatgatgcccatgttggtactggtgatctttacttctttggtagtaaatccaacgaaggtaatcatcagcacatcccctatttccgctttaatggaaaaccttccgttaacatccgccgttacaatgatcctttgccctacaatatgcaccgttgcgccttccagcggctggttggtatgtgcatgtaccagcgtaccggatatttccgttgctacatttacgggtgctgctgcggttacgggaacaggaagcgggttttctgtaatgaatatggtgttgttctgtatcttaaatttcaatggctggtcctttaccagcagctgcataaattcttccagcggcatattacgcacatctatggtaaccggctttgccgcggccagtacttccctggagtaggccgctataaagctggtttgttttctcaccgcgtttagcgccttttctaccggtatatttttaccggacaatgtaaccagctgaccataaccttttgccgcaacattcaggatgacaacagtcatgagtacaaaagttaacttcattgcgttacctattgttttattcgccgggccctgaactgtttggaaaagccttgcagtggagcatccgattttggttgagcacctgtacaaaaggggcggaattgcctcgctatgggcatgagcagtccccttctcacattggtagcaatgtggtttaatttgcatagatttgcaatgtttgggttgatgtaaataatgattaagccaattgttgtgatactgaatcccaatctctttaaacggtggcgggtccaatcgccgccgttttttattggaaatcccggtgccttcttttaactacgttgcattcatcatacatagatctggttgatagtgtttgaaaaaaataatggttggtatctgataagtaatagtataggctattgtgtgatgatcagttttttgccgttgctttccagcttataatgtacccgcgaatcccggagaaagtcgagtacctctttcagatttacatccctgctcatgccacctccaaaagtgatatcaggcactttgccgggaaaaaccacatcgatatcataccaacgggaaatctctttcatgatctcttccagtgtttgtccctcgaaactaaaggcatccgaacgccatgccatttcctggtcgaggttcacctgtttaaccagctgcatcgtttcttccgcagcgcttacctgtgcctgctggccgggccttaactgcacttcggataccttacccgtgctgaacattaccttcacggcgccatcaagcaaagtggtttttgcgatcagctcatcatcgtaggcttttacattaaaacttgtacccagtactataatggaatgatgcttactcactgtaacccggaatggccgggtggcatcttttgccacttcaaaaaaagcttctcccgatacctgtaccagtcgttccgttccattaaaatctgtcgggtacctgagtgagctggcggcgttgagccatacattggtaccatccggcaactgtactttaaactgtccgccacggggtgtgcggagtgtattaaattccggctgactggtatgcttaccggccgtatataccagctgcccgccttgtttctgtatagaagcggcgccttgctgcatggtttgcgtgctgttgctgtccagcgctactacgctgccatcggccagtgtaagcagtgctttattgccgccgggccgtacatcttccactttcaccaacggcgttctgccggaacgcaccggccagtaatagtacgcggtagccaccacggctgtaaatacagctgcggctactgcagcgcgcagccagccacgcctgctgcggacgtataacgccggttcactgtctgcgaaacggatagcatccagcacctgccgggtcgactggtcatccatccggtactctaccggggcatcttccagtgcctgcccaatcagctccccgagcggcgcatcgtcctgctgctgctctatcagtatgcccaactcctgcttttccgccggcgacaaagactgatctaataattttttaaacagatatgataacctggtttcgttcatataaaaaggagcagcgttagtgcttctgctatatgagaggctcagaaaagaaagaagggggtataggggcaaaaaaattatgaaataagcaggtataccagaacgggaataccaaggcgtaccatgcaataagccctgacgctgcgcatagccagcgccaggtaggctttcaccgtttcaggggaaatccccatgatggcggctacttcttccctttttagcccttcctgtttgctcaggcggtatacttccgcctgttgtgccggaagttttgcaatggcctgctgcaggatgccatcatattctttttcacgaagcagcctgtcggccggttcctctgctaccccatcgttttcagacgcctgggtaaaaatgagacgggcattgcgtttcatatagcgggcaatatagttccgggaaagcgtaaacagataagccttaaaatgctgtacatctgccataatactccgtttcagccatacctgcaaaaaaatatcctgcacaatatcatccgccatcccgcgggaaccggtgagcttataagcaatgttgaatactttgtcgcggtaaaaacggaataccacttcaaatgccaggtggtcaccattggcgatacgccgaagataaacggcttcgtgctctatgtagatgttggctgcgatcaccttctttagctaggtaagaaggtaaaagtaagaaaaaatgttattttactacttcaaaacctcaacaggcatctttttaaatacacagttatgaataaagaagtatataaaattacaagaaacgacgcttccaactatgaggaacacctgggtcctctcatttttgaaccatcggccaaagcgttgctgccacatattataacccttcccgcaacgtctatcctggaaatagcatccggaagcggcaggctcaccaaacacctccgggaaaactttcctgcatctacccgtatcacggctaccgatatcaaccctgatatgctggagttggcgcaacagcaattaaatcattctgctataacttttcagttggccgatgcgcaggcattacctttcgcagatcagtccttcgacctggttgtaaaccagtttggattaatgttcctgccggataagcagggcggcgtgaatgaagcattccgtgtactgaagcccggcggtcattttgtgttcactacctgggatcatactggcagcatggaattatttaaactgctgatcgacgaaacaattattcccttatttgaaggagaagatacaagccgcttccatacaccgttcgcgctgcatgatccgcaagtgctgaacaactaccttaaagaagccggttttaccagccataaagccgtgtatctgaaaattaaaggacatgcctcttctgccaaacatgtggtaaacagttattttcaccagcatccgctgggccggcaggtaaaggaaaaggcgcctgcttcctacgatcgcgtggcaaatgaactggagcaacagcttattcaacggttcggaccagcggcttttgaatttgaattgagcgcgctggcaggcatcgggcaaaagtaagtccgtttattttaacaggtcaattaagtccttatcggcctcctcaagaaattccaatggggtggtgccgtctatattgggaacggttttgtcggcgcctgctgctatcagcaaccgcacgcattcaacctggtgatgccggttttccgggcctccatgtttgagcccgtgaacagcccacaaaagcggggttcctttaaaatctatacatcgtttatgaatgtctgcgttttccctgatcagtcttgctaccagcttatcctgccctgtccaggcagcccagtgcaaagccgttccgccatgacaaccggcatgatcaataacggcgccattttctatgtataaaatacctacttcctctgcaagcaaactggccgctgcaatcagcggcgtgtcgcgtccttcggtgaactcattaccattaacgtttgcgccatgcgctaaaaatatccgggccatctccacggcttcctgatccgtataagtatgggcaaatacgccgtcacagatccgatgcaacggatgggctttggtcgtattcttttcatcaaaaggaatcccttcattagccagtgaaggattttgagagagcgccttttcgattccctcatagtctttattgctgatcagttctttcatgggagtttaaataaagttactaaagcaatggaaccaggtgttcccaaccaagctgctttgcaaaatccaatgctgcttttcctttaccggttttaatggttttatccgcccccagctgcaacaaaatttcaactgaactccggttgcctgatattgtttccctgtgcaaaagtgtatacccggcttcgttctgattagttatttcctgcggatgctcatgtagaaatttcactaagctatccttcatattaatactcatagggtgctcaataagatgttccgggtgttccttttgtccataaacgagctgaatatcctggtagttcccaaaattcaatccccaggcctcatcatgttgcttacgttccgacttgcccatggtggaccttaacagctgtatggtaaatcctccataggtatctccctggctgctgaataaccagtcgctgacctgacttagcggtatttccacaaagtctccattcttgatatttgtcagctcagtcggatcatttataagtacgccgctaatcatatcgccatcaaattccacttcattaatccacatatgctctaccagcggagttgtttgatgcgccacattttgcatgaaggctacttttacacaagccaggtctaatgcaggaacaattctccggtactcccaggaaagttctctccagaaatacttaaatgtttcctgtgctttatgaaaggctttaatcatttccggattatctgattcggaataaaagatggtcttctctgccatatttaaaatatttattttttcttactaacagtatctatcagggcaacggtgtccgcggatgattgaataaaggtatctttcttatatccctcaggattgggcaccaattcgcggctttcatcatagccttccttactattgtagcagctgcagaaaccggttagcgttatggctatcaataatattttcatactgcaatataggaaaagattgatttgaactaatcccgaaattccgcgatgatcagactgcggagcagatgcttaatgactgttccaaaccggataataaatgacgttttaaacaaagtactttgacgttttaaacaaaacggtttcatcgggctgtcgctagctttgtttcataaaatttaaaacgatgaatttaaaagacaattataacggcgcctttcagcaaccaatccactccgggtttaacgccacctctaccgtacacgacgtgataaagggtattgacctcagcggtaaaacagctattgttaccggcggctatgcaggcataggacttgaaactgttaaaacgtttgttgccgccggcgcaaaggtgacagtacccgcccgtgatatccgcaaagcggccaataatctacaagggatcagtaacgtaaccatcgaagcaatggatcttatggaccctgcgtctgtcaatgcttttgcagaaaaattcctttctgccaataatacactggatatactggttaataatgcaggtattatgtgggtacctctgcaacgcgataaacggggttatgagtcacaactttccaccaaccacttaggtcattttcagctaacagcaaaactctggcctgctctgaaaagaagcagtggtgcgcgtgtggtgaatgtatcatcatacggtcaccagatggcgccgttcaattttgaagatccgaattttatcgcccgggagtatgaaacattgcagggctacggacaatcaaaaacagcgaataatctttttacggtggaacttgatcatcgcggcaaagtgtttggcgtacgtgctttttccgtgcatcccggatcggtaaatggtacggacctcggtcgtgttgcgcccatggccctgttccagcaaatgggtacgcatgatgaagcgggaaatatccggccggaggttgcggccacactcaaaacgatcgggcagggcgctgcaacatccgtatggtgcgcaactaccccccggttaaatgacataggtggcgtatactgcgaggatgcagacgtagccggactggatgaaggaaatattgcacacaactataacgatccttcttccctgagaggcgtaaaaccttattcggtggatgctgaaaatgccaggaagctgtgggcgttaacggaaaaactaacgggtattgcatttcctgtcaactgataattacccgcaattaaaatcttctctcacaagccgaattcttatattcggcttaaatctattgttgaaaaatggagtttgaaacaaaatatatcacaccggatatcaagctgtcggagtttaacggcaaaggattcaaaacggaagtaatatttgagcaccatatcctggtttggtttatctctggtgaaacaaaaattatacaggctgatgctgcctatacttttaataccggcgatattttcctgattccacgtaatcaattgacaacggtgatcaattacccgaaaaacgggatgccgcataaagcagtagccatgcatttaaccaaagaacggctgcgggatttttattcccggcataaagcagccggacgaacagcctcccattcaaaaatatatcacttctccaaacacccgttgctggaaagttgtcttgcttcactgatcccctattttgatctgggagaaaaccttccgcgggatatcgctgccattaaaattgaagaagccatcagcatactgaggtctatcgacaaaagcgtggatggcctcctggccgactttgacgagccggggaaaatagatcttcccgattttatggagcggcattttatgtttaacatgacgatggaccggtttggctacctaaccggccggagtctggcgactttcagaagggattttaaaaagacctatcataccacgccgcaaaaatggctgacagaaaaaagactgcagctggcgcattaccagatgtcggaaaagaagcggaaacccattgacgtttattttgaagtaggctttgaaaacctgtcgcatttttcaagtgcatttaaaaattatttcgggtatccgcctaacgcgttattcaataacagtgccccccgttgacctttttgctttaaactgtccgtttccggacaccccgcgcccgtgtatgaacaattacagaaaacaattatacataagtaatgtatgtgcatactgcccggatatggcaaccttcttgcggaaacgcttgtataacaacaacaccatgagccacatcgtgattcctattcccccactcccgggtaagcaggagattgaagttgaagtgaccatcaacaaccagaagcagcagctgcactaccgggtagaattgttttactgggacgattgttccaatcccatgggccaccgggcagattgtatcagtgaaatgctgtcgcatcacgatccggaatggaccgtatattatatcggcgcacctacagacaagtttgtgccgattacttttgtgagtaaagaaagcaggaagttattgcagcgggttacggtatagaaagctaaaacgctgctacagcaatcgttccagcacgcctttccgcctgacgatatttttataatcccattggatctttgtgcctttttcgagccagcgttttagcagcccggtgtctatctgttttacatcggtgtaccgggcctctgcggccttgaaagtgccttccggttgcagatcttcttcctcaaacgattgtccgctccaaaataacaggcgcacactgtcttttaatttactgtacccaacaatgggattgccattcaggaaccacaccgggtgccggtgccatattttaccttctgcgttggccagatgcttgttaatttcccgggccagcttatcgccaatagctttatctgcggctgacagtgaatcgttgtaggcctgtatttctttgttcatattgcaggttttgtaaacgaaaacaataggctcaaataaaaaatacaaataaattattcaacaaaatgccagcacacacctgctatatcaataatattcacttcttttccgtaaggctgctgtgttacttcaccgatccgtatcccgaacagatccggcagttttttatcgatcacttcacttctgaattcacttacgctttcaacctgtacagtgatcataaagttttgggcaaagtcaggaacatcgtagtcctgcaaaataaaccggcagccgtctttctcaaaaccggcataaccaggcgcctcaaaactgatactaaaccctaacgctgaaaataactgctttgatctctcaaaatcacttcccgaaggaacaaatggttgcagggaaagaaatttcatacattactttttatagtgtaatcaataaagcctgggatgaaatcgccttccggatagtatttcccattttaatctcacatctaaatataagactatctggaaattaccgacagatcttttgaagattttaattgcccagcaactccaataatgcactcacgggcaaagtatcctttatcaccatctgctggtgccctgtaacgttacctgtatcgtctttaatcatggatcccagcggcatggtagccgaaattattccaacaagattgccacgtttgtccaataccggtcccccgcttgaacccacgccatagtcggcggtaatctccatccggatgggcggcttacccagtggattatagccggccgctgtctgccgggcactgatggccacatttcttgctaccattcctttactgaaataataaaaataaccggtaggatgggaaatgcagtaaacggccgcccctacttccgcaggcttccctatcggtaccggcaggagtttattaccattggtattcaccttgaaaacggcgagatcattgttttgggaataggcgagtatcttttctatgaaatagagctgtttgtcccaggtaataataaagtaaacgctgtctttcacagcatccggactatcacttacaataatgcttttcaatacatgatagttggttacacatatcccatcggcgtttagcgcgaaagcagtgcctgttaaagcgaacgataacgggtctgtgccgttcccggtcttctgcagtttccccacaataaatacactgcttttcctcctggcataaatttcttcatcggccagtaccttggtggtggcggaaaggagtttgattttatttcctgccggagatgcttcgtcggccagcagtgctgtgctgtccttcaaatcctgtatcatggcacttttaccgggaggcataaatttcaagccactatagtagtgttgatagctggtgtatatatcggcggtagacgaactttgcgccccggcccgcaataatccggatactataaggatgcccgttaataagcatgtatttttagtcatgatgatttgttgtacaacagttctaagataccttcgttgcggataatcatcatcccttgccggtcttccgtaatcccttcctgcagctggtaagtataacggggataagcgccatccatcaccgtaggcatgtatacaaaatgaatattgtcgcggtacttcaacgcttcgcccacttcaataatatgtgtagaaacgatgaacaggcattcttcgtaaccggaaaaaccctccgttacagcaagtgtaccgtcgtaagcatcttttacattcgttcctttaaacagctcatcaaacatgagcagcagccttttgccgctcgccgccgcttccgcggcctgttttactcttactacctcggcgtaaaaatggctgtagccgagacctatattatctgccacattgatggaggtatacaatccttccctcacggagaattccatgcgctccgccgccaccgggaagcccatgtgcgccaggtaacatccgatacccaccgatttcatcagcgtggatttacctgccatattagctcctgtgaggaataatacattactgtctgcatccatgaagatccggttgcctacagccccgtcgatacatggatgggcaagcccggaagccgataacacattggcttccggcggcagcgcccgggcatagctgaatgctttttctgccgccacagcgctcacggaaatgtatacgtctgttgcataaataaattgtaaaatatcttccatctgccggagcagccttcccttcaacagatgatcgtaactggctaaggtttttatcggcaatgcctggtagatgtcgatattccgaaggatttcaatccgcctatccgataagatatccttcattgcctgcacacgggaataatagggattttccgcgggatacatagctgttacgaaagcatggcacttgttcagggtaatgatagttgcctgtaatccctgtacattttttttatactgttcgtcccttgttagcgtagaaagccattttttaattagtgtgccagccaataccagcgcagcatttttattcgcctgcacatcaaggtactcccgcataaggcttacctgctgcacatcaaaggggaaagagagctttgcctgctggaaatactgaaaaatactgctccgctcattgatcgcggtttcactattcaagggaaagcggaacatgttgtcaagcagctgctctccgccgcgcgtttttacgcggttaaataaatgatatactgatccttgccggaacttacccagcaggttcagctcatcaagggtttgtttgtcgattccaaaactcatacgaacagttattttttttaccggtgattaattcccaaacggctcctggctgatttatactggcttcaccctttgagctgctgactccggcgctcttttcttcttccctttctccagtatgttcaggatatcttcattacggatgatcaccatgccgtgccggtcatctgtaatacctttttccagtgtgtaagtatattccggtacatggttgttcattcgtgtgggcaggtaaagaaagtcgatgttgctttttttcttaagctcctctcctgcttccacgatatgcgaggaaataatgaacatgctgttttgttttgttgcaaagccatttgtaacggcaacagtggcttcatgggcgtcttttacattggtaccgcggaacagttcatcgaataaaataaaaaatgattgcccggagcttaactctgtcgccatttttttcaccctcagcacctccgcataaaaatggctggcgcccatgcccaggttatcgggcaggttcaccgtggtataaataccatccataacggagaaggtcatcgcttttgcggcgaccggaaatcccatatgcgccaggtacaaagcggtactcaaggaacggagaaaggtggacttaccagccatattggcgccggtcagaaaaatcacattctgtgcagcgttcatcgtaatatcattgccaaccgggttctttaatgcgggatgatatacgccttccagtttgagttcgcacaatcccttgtccaacgcctttgggaaaataaaattcctttctgtagctgttttggcaacagacatatacacatccaggtagtagatatagcctaacaatttttccaccttgggccggtcgcttaccctgaacagggcatcataagccgtaacagcgccataagacagttttcctttgggttgttctttgagtgcaggttcaaaaacaggatccgccagcaaccgggtaatggcttcacactccgatgcgtaggcaggtatattttttacatcgggctgctcaacaaattttttcgtaagccggataagctctattaccgctcccaccccgttttgcacctctttttcaccgagtaaggttggatcgtttttgctttttgcatttttttccccgctgataagatacttctccgccatgtcaaataacgaagcattgtaagggaaggacatgcccagccgcgcaaaattttcgatgatgctgctgcgccggttgatagtatccttatcagacaaagggctgcggaacatctcttccagtaaggcctcgccgcccctggtgtgcgagcggttatagatatcataaatcccgctgccgcttttctttccaaatattccaaggtcgtctatggtttgttcgtcggttcgtaacatctgatgtgtatttagtagaagtatgcttatttgcgtttcctgcggatcagtagtatggtgcccagtagcagtatcacacccggcagcacccatatgtatacgattttctgtacaccggcaatagccgcattgatctgtaaacgggtatcttccggttgtggacgcggcgtataaacagggtactggttatagtttaaccagctataaagtgccctgccaacagagtggtcccccgtctggttgttactcaaaaaatcggcatcgccacacacaacgatccgttgctctttcccatgaatggaccttgttaattgcaccatggtgggaaaggaagcttgttttatatcgcctgccagcgggttaaatggaggaagcgtggaatccgctaccaggtcgcccgctttcagccatacacgaccaggactggtcatagccaagggcgccaccttaaaggtgctatccccggcgcaggaaattcccgcaaccccgcgcatctgcgtttgtactgaatcacgggtattatgcgcctctagcatcttccgtaagtacagcaccagaggctcttcagcaagaccggcagctgttgctgtgagatagggcattaccctgtcaggggtttcattatacgttggctgcaccagctgcccattcatcagttgcacgccgatttgcttcagcaatgggttgagtacatattgtttgccgggttcaccggtgatcagcatattaccacctgcatcgatatagtttttaagtttatcatgcacagcaggactcaggtccattttgggatcggccagtataagtgccgtaatcccctccggaatatgctgcgtggcaaggttgatggtatctacgtcaaagcccatattcaccaaagcattgcgcgctatttttaacgtggtatgaaaagcatattcccgctccccttttttataaatattgcgctcaagctcgccgcttacaaataataactttggtacatctccatataataaatgcctaagggccgcattcatgttctgctcatcggaccatacaaaattatcttcaaaagtgcgcaggtattcggtgcgtcccttgtattttaattgcatgatcaggcgatagccctccggtttaagatcaatcatcctgcgcatttcttccggtgtcttaaacatcgacaagtccatgtccagcgattctgcaaactccgttgcaatctgtttcaggcttttaccaggaagcattttatacaatgcgctgtccgttgctttagcgtcgttatcgtaatagtattcatacttaaatgagataccgggcttaaagcgtaagtaggcttcccagaaatcgcccaggtaatttacattccgcacgtcgggaagtccactagataccatgcggtctaccaggttggtatacagcgtaacctccagcgtagtatcacccatttccttcaggagctgctgtgtacggggatgtatggtattcattttggtggcggaggtatcccagtaaccggtgagtgccgggcgggaagtgacatagcctattataagggttgccgcaaaaacgcctgcaaagcggcctgcttttatgtaccagggtttaacttccctgccattccttagttttatcagtgtaaagccaacgaacatcgatgaaaccactataaaatagatgacatctttagtggtgaccaatccctgcaacattttcccggtacggttttgaagagacaggaaataggtaaggtcccttacaaaatcatatttctgccacagtccaccgatccggctgaggataaaaatgatcgtaaaactggcgagcgccgatacgatctggtaagtggaaagactggacataaataacccgatggctgaataagcacatacaatcaggtaaaaacccagggcggcagaaaacaatatgccgtaatcagcatctttaatattaaaaattccggtgatcataaaaattccgatgatccctatcagcagcaggctgtaaagcataatacccaggtattttcccagtacaatctgccgcagttgaaccggcgaagaatacaataacttaaccgtcccgttattgatttcccggctcaccaaccccatagtgagcaaagggataaagagatacagatttcctatcgcacgggagaatatgccacccatcaggaaaaccttgagggttaatgattccgtcgccatcgatattctgggcatgggattgtttttcagcaccatatcctggtaaagtgccaggtcataaacaggactcgtatacacgagcgcacattgcaccaggaacacgatgatcagaaaccatgcaatgggcgagtaaaacaggtaccggaattcattctttgcaattctaaataataacttcatgggtgcgcttatttatttcctttttctcctgatcagcaatacagtgctcaggaagattaatataccaggcaatacccacaggtatgctattctttgtaccgttgccctggccgggctgagcagcagcatattgtcgctggcatacggatagattgagtaaagcggcatacggccatcactcagccaccagtagaatgtcctgctcacccaacccgcgtatgataccctgtcgctaagaaagtcggcatcgccacacacaatcatccgttgttccctgttattgatttgtcgcgttagctgaatacaggtagcaaaagcgttaaactgaatgtcgccttcctgcggactgaataccggggcaacggagtccgtcacaaattttccggcttttgaccatacggctccgggaaccgttgcaaacaatggttttgcggcaaagccgctatccgatgaataagcaattcccatagcggaaggcatctgtatttttagcgtgtcgtcatacacgccgttggaccataaacgattcatcagcaaggcgggttcttcatgcgcaatacggaggcctgccgccgtcatataaggcgtcaccatatccggcgcgttattatagccgggctgtgccagcttgccgttcacgtactgaacgccggtctcctcaagtacggggttcaaaatatgttgtttaccgggttcgcccagtatcagcatattacctcccctgcttatatagcttttaagtttgctcaatgcagcagtgcctaattccatttttggatcggccagtaccaccgtggtcacatcaggcgcaatgtcctgtgtagacaggttaacggtgtccacatcaaagccggtattcaccaatgccccggaattatcgttgtttattacctggaggaacaactcccgttctccacgcttgtaaatactacgttccaggtctccgctaacaaaggctacttttggcattttaacaccacgcagcctttccagtgctacatcgatatttgcagggctgggccattcgacactgccatatgtccgcaggaaaacagcgcggtctttatatttcagttgcatcacaaggcggtaaccttccggtttaagatcaatgagcttgcgcatctctgccggaggcttaaaggaggatacatccactttgagcactttcgctacttcccctgctatctgttccaggctctttcccggaaactgtttgaaaacagtgttggtcgcatcggtgctgtcaacgtcgtaataatattcatacttaaaatcgatgttccagttaaaacggagataattttcccagcagcgcttcaggtaaatattgcgccattccggaaggccatgctgcgcagcggcaccaagtaaattggtgtacagcgttacttcaagcggactatcgtcgaatgatttgataattttctgtgagtgcggaaggagtgtattgatttgcccggcggtggtatcccaatacccggtaaagcggggacgcgaactgatgtagcccatcaacaggcccaccacgatcacagccacgtatctgccggcttttacaagccagggtttggcttcacgcccggcctgcagttttaataacgtaaaactgataaacaggtagatgataataaggtagtagatcacgtctttcgtagtgatcaggccgatcaccattttttcggtacgtcccgcaatagaaaggaaccaggtaagatctcttacaaaatcatactgttgccataagcgcccgatactcatcagtacaaaaaataccgtaaaactggcgatggcagacacaatgggataagttgtcagactggacatgtaaaaaccgatggccgtaaaagcgcataacaacaggtaaaacccaaacagtgtcgataatagcgggccatagtcgagcgatttgatatcgaaaaacccggagataataaaaatgctgaggataaggaccagcagcaggttataaatcatcaaagcaagatacttcccaaggatgatccggcttaatttaaccggtgaagagtacagcagtttaatggtcccgctgttgatctcgcggctgatgatccccatcgtaagaaggggcacaaacaaatagatgctctgtaatacattgaccaggataccgtcgccatccaggaaaatactcgaagtcccggattgcgtggcacgccaaacccagttaggatcattggaatacgccaggtgggccagcttggcccaggtataagtggtgccggtataaaaatacgcgcacatcaccaggaaaacaatcagcagaaaccaggctattggtgaatagaacaggttacgaagctcattctttgctatttgaaatatcgtcttcattagttgcgctttattgtggagactgggaggatagttgtttgaaaacatcatcgagcaggcccttgtcaagcgctatctcttttaacttccacccctgttccacactcgccgttatcagccggtccgagatatcttcatgactgccatcgaaataaaccctcgcttgtttgtccgtcataaattccacctgggtaacgccctgaatttttaacaggtcgcttttcggcggagggttgtccatgcgtaaaagcataattttcgactgcacataattattgaacgcatccatactgtctgaaaacaccatccggcccgcctctatcatgatgatctctttgcagagcaaattgatttcggacaagatatgtgaggataaaagcacagaatgatcgatggctatttccctgatcagttttctggcttcaatcaactggttgggatcaagcccgttggtaggttcgtccatcaccacaagtttgggcttgtgaataatggcctgcgcaataccaacccgctgacggtagccacctgacaggtttttgatgagccgggagctgaagtgtgtgatgccgcaacgttccttggcttcttccacagccggtttgatcttatcattttccatcagcctgagttgcgcgcagtaggtgaggtattcgtcgatagtgagatccgtgtacaacggaggattctgcggtaagaacccgatctctttcttcgccgcctccggatgctttctgagatcaatgccattgatatacacgcttccttccgtttgattcagcacaccgcaaataatattcatggtggtagatttgccggcgccgtttgagcccagcaagcctactatgcctgattgccccacctcaatattgatgtcgcggatggcccaggtactggaataccggtgagaaagattttccgttcttaaaatggaagtcataaatttattcgtttgacaatttgcttgttaaatacgttgcgcaataacggcggtttgtacggtacaactaacgggtctgaggaccgccggcagcaggcgtatttaatttattcaattcttccgcgtgggcctgcaggttgctactcatcatttgcgccgattccatctgtaactgggcagcagtggtcagctgtttctttccggccgatgttttgtaaaatgctgtcagcacttctatttcttccgtactgtaatattttgcgtacaacttcagcaggtcatttttgcaggccggatacgacgcgtatttgataaaaaaggcccgcacttcttccttctttccagccagttgcggcgaacctgcagcggtttggtcggccgccacaatagctgattgcttataggcttcttccaggttcatcgcagcaaacagctgctctattttctggtactgttttgtattatcctgttgtgcgtgtgcagcaaatgttccgcagatcatcatagcggccagtaagagtgttcttgatctcatattttttatattaattgttgaataatttctttttctttaggcatagcgaatcctgtttcatgaaatgctccatgaattcattcacccatccggatcaatgacggccttatttcagcgccagtttcattaattcagacacacctgattttaaagggaatattggtttgccgtttgcctgttgctgtatagtatataaactatcagacttcacttttgtactagtgcgattaaaaaatatattgttaaaaacgaaaaataaaatgaagagggtaaccccgccaatatgttcttttatatattgaacggctctgcccagatggttcttaacagtatgcggagagatcttcaaatgatgcgcaatttcatccctggagagcccgcccactttgctcaggtggtatacggcctgttgttgttcaggtagccgggcatatattttatttaaaacaatcctgttttctttttgtaccaaacgctcttccacttcggtagaaaattcctgctgcgatgtacgtaaagaagcatataccctggttttgcaggactctcttttcaaatgtcccatggccaggttagtggccactctatataaccagccgcccacattacccggtgtgattgccacccgtttttcccacaaccgcaggaaagtttcctgtacaatatcctccgctgtttgccggctccgggtgatataagtaacaatggtgagcagcttcgtggaataacatcgtacgatttcattaaatcctgcttcgtcttcaaaacacatacgatctgttcccgcttcattgccgggacgtaactgattttctatcgactggttcatcgttatcatgacgctgattttaccgtgggttctgtataatagcggggttattagcaataatgaggggcgaaaaaggcatcaggtaacgcggtgaattagcggttaatgtggccttcagcgtagtgccgttatcggcgaacctttgcagggtttgtgcaaagcggttatccctgttcagccttttcagatcaaagagccggagccctccgtgataaaagagttccctccttctttcctctaataccgtggtcagcacatctgtactgctgttcagcggggcataggtaaccaggcggttttttctaagctcattcaccaacgccagcgctcccgctgcatcctgctgcctggcgaggcattctgcttttatcagcattacttccggtacgccaaggctataatcataggctgttccactaaaggcgaggccgttaatataaagtcccccatccgcaaaattgttgagcaaccttatatcgttgctgtccagtacggcacgaaggctgggactaatattaagcccggtatgccggatgctgtagaaatcataatcgatgcacagcctggcaagtaatatttccggattcttcgacaggtcgagcaggctggaaaatggtgcataatcccgggtatatttcagcagctggctgttaatggctaatgctgattgtgcggcgttgagtgcatcgggatatttagccatgttcagataaattcttgccagtaatgcatatcccgctgctttgccgggatgcaccacatcctggcccatacccggtaaacccggcgtggctactgcagccgtcagatcgctgataacctggtcgtatacctgttgtacggtagccctcaccggttgtgcactggcatcaggaaacaataccaaaggaacagctagctcggcggcagctgttgccgcctggtaatctgttccatacaaactggctaattgcaggtaataccatgcgcggttaatttgggcctgtgcacggatcacatttttctgttgttcgctgcctgctgaacggcctatccgttccaatataatattcatttgcaggatacgggtatacgacgcgttgtacataaagtccgcatcacccggtttccagatcgattgttcccataaataagaacgcgtataggatgaagcggcatcggcagacaggtgcgcatcttccagccgtacatcatcgctcatgaagtcggccaacaggtaattgcatatcgccatggaatcattattcagcatctcttcaaaatcccccagcgtagtaggattgatgctggtagtgctgggacgcacatcaaagaattttttgcaaccagccgacaggagcaggagtacgcaaagcgcagcgatcatcactgacaggctactatgccgtaaaaattttcttttcatattcgttcgttgtcgcttgtttaaaatttcatattaacactgaacatatattgccggggaaccggcagccctatctcccctgtatttgccaccgcctggggatccacatgcaacctgttgctggtccataaagcggcattcagcatttgcagggataccgtaagatctttgataaaataacgccgcagtatttcgccggataacacctgccagcctatctgcacttcctgcaaacggatattgtctgcagacataatactgttcgatgagttctggataatgaatttccgtgtactgccttcatctgcatttcccgacatggccgcgatatctgtaaaggcctcgtctcccggtttccgccagcggtcgcggatcaggagactgttgtcagccgttctggagggagacggcaggtattcccgcatcacgtgaccaaaattcagcagcaatgttgctctcaggaaaaaccctttatagtcccattcctgtataaggccacctgtaaaaggcgcgcgggtaaccccgctgtacaccagcgaggaagccagcgtagcgctgtcggggctggctgtcttctgccctttggcgtcatatatcatggggcttcccgtagcatccagtccggcccagcgataactccagaggttctctgtgctgtaaccgttgcgatagtccgttaaataacgagcggattgtgaaaaattcaccagcggcacttttttcgcaatattcttattataggcgccattgagcgtaatcacatacttaaaatctttctgctgcaatacttttatttgcaggtacatctctactcctttttttactatctcactataactgatttttgttcctaagccggtagaaggatcggtaggaaccgggataaaattattgagccccgaagtgtttgtctggtaatagcggaagtcgaaaagataacggtcattggctaatcccagcgttgtatgcgcttccaggtttcttattgttggcggaagctgcccgaagttgctatttacagccatcgtaaatccgccgccggataacggcgcattggtgcctgtcattatttccatgccttgaaaaccactgatattttgcagggtaaaatccgccattaatttgctgatagcgccggcatgaaaataagattccctgccgatgtcataagcaaccctgatatttgtttgaggattcccgtccaacgaatagccataacccgcatataaatgcaggagcccttctctcagtctcacccgtgcgtttgcgcccacataattctttatttcaaggccattggtgcttttatctccgctattattattgatgcgtaagctgttgtagctgatatcaaaagtataacggtcgtccaacaggcctatcccgagtttctcatacacgttgtacgaactttgtccgctttgctggggcaggttaaaacgggttacccaaacgccatagttattccagttgctctgacggttacgctgcgcggcaatttgcgtggataaaccgggtatgctgattccgtttacgccggccgacagtgctacgttactgacccaggaaggagcctgaaaaaaatggttcctgcttaaccgccaggtggcatccgcggaatagttagtaaggttggtatagggatgcggattgccatagtcaggatttaatgttgtattgtacttgccgctcagtatataagtaccgtcataggaataagaaaagctgccgttccagttgagcccccgtgagatagtagtatcgcctgcctgcggcgttagtaatgtattcggataaaccattctgccataggtaccttcccaatacctgtcgggcaggctgaataaattgaggacacctgcagtagggtcgggcgatggcaactgcacggcctggccctggcgggtttgtttattataaccataaatggacgtataggaaggactgcgtgatgcattaccaaaaccgccgccacccagtgttacagcaaggcggtgcttcccgaaacttttatcaaacagcaaggcggatctcagattccattccctgttttttaaagatggcttttgcataatgcccccacggggcacataaaaatcgatgccggtaagggcgccgaagtcgtcgaacacagggctgccgtattcatttaccaactgcctcgccccgctggaagctgcgtcctgcaggtcctctgttctgccattcagcagatcatattgcagtgaagtggaccaccggagagagggcaggatatcccagtcggtagtcagcctcgactgcacctggaggtttttgctgatctggctgtttatccgagcatcctccagcatattggcgccatgatcttcatacccgtatttcttaagggcggtattggcatccgggttaaaggaagaataatcgtatacatactttccggtttccggatcaacaagcagctggtaaggttgcaggttgcggaagtcggcgttggccccggtcctggctgtagtttgagcaacattcacataccattgcgcgcgcagtttattcttaaataataagaagtcgttgttcatattcaggctgaaggtccggccataattgtccagggcgctgctacggtcggtgttgtaaataccggcagccctgaagcgccaggcattgctgcctcctgaaagggtaagcatctggttttggttaaaggaattttgttgcagcagctttaactggctttcattggatagcctggccagcgaatccagttgggtgttatagtcatgctcagacagtgtgcccagctgccagccataaaatatacgctcagcaggattgagactaaaagctacacgtggatcatttttatttgccagcaccataaaccccgaatctgatgcagaccttaaatagtcgatcatatcggcggaagaagccaggcgtagtttactgcggttaaaccggggcgccgctgcataaccgaagttggaactataactgagctgcagttttcccttcacggcgcgcttgctggtgatcataatgatgccaccggtggcggcaggtccccatttggtcagttcttcggggtctttgatcaccttcaccgattctatattggtcatcgggtaattggcaggaaaaccatcctgcggaaaaccatcaatgatgaccagcatacccgacgtgttcccactaaatccacttacgcctcttaattggggaaccaggccattactaccaacggaagtgctgtaattaaaacgaatgccatccacacctttcatagaattgatccacgaatcaaaggttggataaccggtcgacgaatagatgctctgatattgattatagtgtgcccgtaaagcttcaatagtgggtgtgtaagtacctgttatgggtactccccgcccggtaaagtcgatggactgcaatgtttgctgactctgggaagaattttgcaaagtgaggccggggatactgccctgtaacaactgcccgaggttcaggtgcgtccggtgggtcatgtcgatggtatccgtaaaaggtgtccttttccggctcatgtcaatgtcgtcaatcaccacggcattcatttctatgggcgccactttcatcgttattttcaggctcacttcaccattgtaccgaacttccacattcctgtgcccgatggcgctgaatataagcttgtcgcctttttgcccatatatttgaaaggtgccgtcggcattggtaacggaaaatgttttctggtgcgacccgccggatatgctggtaacagttacaccttgcttaggaatgctaatggaatcaaccaccagtcctccaatcaggatatcttcgtccggcgacgccgccggcgatgcctccctgccctcttctgatcctacagattttcttttaatgccaatgttattaccggaaataatgtaagataatggttggtttttcaggcaaatttcaagaacatcacggatcccggcattgctcacctggatgcttacgggcgctgttttatccagcacacctttctcgtaaaagaagatataatccccttgttttttgataagattgaatatcttttttaagggcgcattcttttcattcagcgtaatctgttgcgccgctgctatagtacttgcgaatacgcccgcaaataacaatactgataccgtaatcgtctttagcagaaaaatcttcgtcagctttttgtgatgtgtaaaaaatacagggacctgtaatgaataaaaattcatagttttgaactgttttgggttcataattaaattactttttcaaacgccttgttggaaaaagggttgcccaaagccttgccggatgcgccgcgaacgcttccggcttttttttgcaagccttttggttgatattagttattcacatgactaaaaaaatactttcggattatccgtgttgccggcgaagggaacggccacgggatatgctatggttttacgacaatcttcttcccttctactacaaaatttacattggcaaattccagtacctttaaaagttccgccaggctggatttgcgggagatgcctccggcgaattgtctttgaggaatgttcccttcaaaaacaacatctacattgtaccagcgggatacctgccgcatgatggtttggatgtcggcattttcaaaaacggtgtacccgtttttccaggcaatcacatcttccacattcacctgttcaatgagcctgagcgtattatttttttctaacagcgcctgctggcccggcgcaagtattttcacctggttgccggcgttcacttttaccgcgccttccagtagtgttgttttagcatcgggctcgtcgttgtaagcattaacattgaaatgcgtccctaatacggctatattcatttggttgacctgtacattaaacggtttaccgggatctttcgctacttcaaaatatgcttctcccgtaatggccacatcccgcttcctcccggtgaaaaccgttggatatgtaatggaagaagccgcgttcagccatacattggtgccatccggcaattgcagcttgtattgccctccccgtggcgttgacagcgtatgatactctgcctcattggcttttccctcgtaattcagcgtaccgctgtcgttgttcactttaaaattgccatgctgaacaatattaccatgcgcactatccagggtgatctcctgcccattggccagcttcagtacggcgcgattgctacccggcggcacatccgccatggctattaccggtggactcacctttgcattgccggcgcgataaaaccaccaccctgctcccagcagtatggcaagcattgcggctactgaccaccatcttctgaaaagaggtactaccttcgtctctttctctacctgcggatacttcaggatgctatccagtaccggctgccacttttcagaagtaaacgctttatcggcaacggcatccgtaaatgcaggcgccagcagggcataccagtctatctcaggccgggagtcgatgatgtccaatagctgtatcctctcctcttctgtggacagatcatttatatatcgttctaacaactgttttatatggtcttcctgtatcacagtatacgttttgtcccggtccggccaggtcgttcttagtaatagacaccaaaaatgattaccggtactcctccggaataaaaaaaaatttaagcgtaatacataggaagtgtttgttgcagcaaccggcaggtggtgggcattgaccggtgatagcagggcgttaatgcgtgatgatctctataaaaaagatacccgctattaaagtgccctggtcctttagtatagattcctgtatgtggcgtaacgcaatacgcagttggttctttacagtattttctgaaatctggagcaggtcggcaatttctttcctggataatcccttttccctgcttaactcatatatcctgcggcgttgcccgggtagcccgtctaccgctttgtggatggattttctcagttcctgtacagtaagctgttcgtccgcggtagcatcatgacccggcacatccaggtacatatcctgtaatacatgcgcctctgttttgttacgtttcaggtgattgatggaaaaattggtggccatgcggtaaatatagccggagagattggtaacagcggtgagcccttttctatttatccagagcttcagaaatacttccgctaccacatcttcagcagcagcttcctcttttactattttaagtacaatgggatgaataatagccccgtaatggtaaaacaggcgggtaaaggcctcttcgtctccttctgagatctgtataactaacttctcttcatcatatgaaaaagtacccggcagcaaagtggcttagatgttgagataacaagataatcctttgccggaaaatatcaaactaattttatcggcgccggcaaatgaaaaagcgtgataccatccggaagaaggtatcacgctttttcatcgctgtggcactaatatcttactatattatgatttgataaaggccagcagatccttgttgatcgtggccgcttctgtagtgggcataccatgagggaaccccggataggaaatgagctttccatgctttaacaggcccactgcttttgcgcctgaaatgggaaacggaacgatctggtcatcttcaccatgcagcaccagcacgggaatgtctacacttttaagatcttctgtaaaatctgtttcagagaatgccttcacgcaatcgtaatgcgccttgatggctcccatcataccctggcgccaccagttatccctcacgccctgcgatatctttgccccttcacggttgtatccataaaatggcagcgtaaaatcctggaagaactgcgggcgttgtgtggccgtattttttctgatatcatcaaatacagacatcggcacgccgtcggggttaccggctgtttgcaccatcaggggcgttaccgcgctgatgagcaccgcttttgccacacggcctttaccatatttcgcagcataacggattacttccccgccgccggtagagtgaccaacgtggatggcatcttttaaatcaagcgccttggtaagctccgccacatcggcggcataggtatccatgtcatggccggtggcggtttgactggatcttccatgacctctccggtcatgcgcaataacccggtagccctgctccaggaagaacatcatttgcccgtcccagtcgtcgccggacaaaggccagccatgatgaaatacaatgggctggcccgttccccagtccttataataaatttcagtaccatcttttacggtgattttactcatgttgtttggctttatttatttggttaaaaatttttcagatgtcatcaatttaagcttgtttagccggcattcattcctgctaacaaagatttaatagatgttgttcgtctgaaaaacaaaaaattattccgctgatctgtatcatgcttcttctccattttacattatttctgaaaaatatttgggtaactcaaaagttacacatacctttatgtaacttcaaagttacttatcatgaccagatcaattaaacaccagttcttcttcccacacccggctgaaacagtttggaactacctcaccaaacccgaactgatggagctgtggcttatgaaaaatgatttccagcccatcgtgggactcgactttcagttcagaacaaacccgatacccagcctcgacttcgacgggatcttctactgtaaggtattggaggttgttccctttaagcggctctcctactcctggaaaagtggccccggcgatggtaagatcacactggattctgtagtattatggaaactggaaccaaccgataaaggcacagagcttttcctggagcatagcggtttcacgaaagatgaaaacctgaatatgttcaatgctctgaccgacggctggctgaagaatttgcacaaaattgcggaccgtataaacgcagcacaacatggcaacaccaacacttgacgcattccaggtaatcggagatcccagcaggcggaaaatgctgatgctgctctcagaagatagtttgaccatcaacagcctggcagataactttgatatgagccgccccgccgtttcaaagcacatcaaaatactgtataacgcaggctttatttccatcgaggatataggccgggaacggtattgcacactgaaacaggacgggtttaaggaattgcagaactggatctcctacttcgataagttctggacatctaaactgaaaaagttagaaactttattaaataacaaattacccaactaaaaagtcaacaacatgtctgcatcagattttaacactaccatcctggtagatcaaacgcccgcggaggtattcaatgccattacgaatgttcgcggatggtggtcccaaaacattgaaggcggtactgcacagctcaatgatgagtttacctaccagttcaaagacgttcataagtgtaccatgaaattgacagaagtggtcccggataaaaaagttacctggcaggtgctggacaactacttcgatttcacggaagacaaaacagaatggactggtacaaaaatcgaatttgagatctctgaaaaagaacatcagacacagcttcacttcacgcaccacggactggttcccgcatatgaatgctatcatgtttgttttgatgcctggagcaactatatcgggaacagcctgcgcaacctgatcactacaggtaaaggccagccaaatcccattgagaatgccattaaaaatactaagccatgaatataggcattatcggcgcaggcgctatcggaagctgtctggcatcaaaatttgtaaaactgggacataccgtttcaatcgctaattcccgtggtcccgcatccctgcaacaagtggcagagaacaccggggcaaaagccgttagtgtagaagaagctgccaggaataaaaaagtgattgttgttactattccccagaaaagcatcaccgatcttcctaaaaatatttttaaagatcttccggaagatgtagtggttattgacacgggaaattattaccctaccctccgcgatggcatcataccggcacttattcaaagtggcatcgacagcctgtgggtacaggagcagttaggcgttcccgttgtgaaagtttttaactctattgttgtggaaagcctggaagccctgggccaacccaaaggtgctcaaaaccgcatcgcactggccgtttcgggcgataacgacgccgctaaagaagtagtatttacactggtaaacgatgtaggttttgatcccttcgatgtgggtactatcgcccaatcatggaagcagcagccaggttccaccatttattgcagggatattaacctggaagaattaaaaaaaagggtacatgcaatgggaactgcatggacagacatgcacaatgtaatcattggaaaacggaacagcgatgaagtactgatgaagacagactatcctgcttatctggaaagcctgcaggatgaacggctatttctttaacaggtcgttgatgatggcagtagccttctcttcaaacccctcctcatacccttcaatgacctgggcaatttttccatttttgccaatgaaatagaaagtcgggaagcttgctacatggtatgattgcaccacctcctttgcatcaacatacatgggatactttatgcgataattcctttggaatccaagaacggatttccggctgtccctttccgtcaggctcaccatggcaacgttttggttcttatatttttcatgaagacgattcaatggtttcagggaaagcatacagggcgcacacccgataaagaagaaatccagtaacatcactttacctttcatttgtgcagatgacatcttcctgctgtgcgtgaacatccaaatgcaacaacactaacaggaggcaaataaatggccaggtaaacctttttatagtataaatcatcttatggtggttagcgttatcgacttgttttaacaagatagggcaaattcccttttttatgcttaaattctctctccgtgcaggaacacactacaaatagattttaactattgaaacatagaaattaattgattgtgattattctttcaataccataactttatcattatgcacaactaaaaggtgcaggcaagtgttctttcaataccataaaacttctaaaaatgggaaaagaatcaaacgacatcagtaaatgtccgtttcataatggcagtatgaagcacaatgttggcggtggcggcaccaggaaccgggattggtggcccaaccagttaaaactgagtatcctgcgccagcactcctccaaatcaaacccgttgggtgaagattttgactatgccgaagcttttaaaagcctcgacctggaagcagtgaagaaagaccttcatgcactcatgactgactcgcaggactggtggccggccgactttggtcattatggccccctgttcatccgtatggcatggcacagtgcaggcacctatcgtgtaggtgatggccgtggcggcgcaggctcaggacagcaacgttttgccccgcttaacagctggcccgataacgtaagtctggataaagcccgcagattgctctggcccatcaaacaaaaatatggtaacaaaatttcatgggcagatctcctgatccttaccggcaatattgcactggagtcaatgggcttcaaaacatttggcttcgccgggggacgtaaagatgtatgggaaccggatgaagatgtatactggggctccgaaaccacctggctcggtggcgacctgcgttatgcgcacggctcccccggcgtggaagaaaatcatggcgtactggtatcagacgacgacgcagatggtaatattcacggccgcaacctcgagaagccccttgccgctgtgcaaatgggccttatctatgtaaaccccgaaggccccgatggtaatccagatcccatcgcagccgccaaagatatccgggatacttttggccgcatggccatgaacgacgaagaaacagtggccctcatagccggtggacacagctttggcaaaacccacggcgccgcacctgccacccacgtaggcgcagaaccggaaggagctgacctggaaatgcagggcctgggctggaaaaacagctatggctccggtaaaggcgcagacaccattacaagcggactcgaagtaatatggacgaaaacgcctacccaatggagcaataacttcttcgaaaacctctttggatttgaatggcaactttctaaaagtccggctggtgcacaccaatgggtagctaaaaacgcagacagcattatccctgatgcatacgacagctccaaaaagcacctgccaaccatgctgactaccgatctcgctctaagaatggatccggcctacgaaaaaatatccaggcgtttcctggaaaatcccgatcaatttgcagatgcttttgcccgggcctggtttaaattaacacaccgcgacatgggccccaaggcgcgttacctgggccccgatgtgccggaagaagaactgctttggcaggatcctattcctgcggttgaccatgcgctgatagatgagaaagatattgcggccctgaaagcaaaagtactggcatccggattaagcgtatccgagctggtttccactgcatgggcgtcagcttccaccttccgtggatccgacaaacgcggtggcgctaacggcgcccgcattcgcctggctcctcaaaaatattggaaagtaaataatcccacccaattacaaaaagtactggatgcactggaaagcattcagaaagaatttaacggcgcccagtcgggtggtaaaaaagtttccctggccgacctgatcgtactggcaggtgcagccggtgttgaaaaagcagcgaaagatgcgggacaaaccatcacggttccctttacccccggccgcatggatgcttcgcaggaacaaaccgacgtggaatcagtaggctacctggaacctgtggccgacggcttccgcaactaccgcaagtcaaagttccccgtgtctactgaagaattgctgatagataaggcccagttgctcacccttaccgcaccggagttaacagtactgctgggtggtatgcgcgtgctgaacactaactttgacggatctaaacatggcgttttcacttcccgccccggccagcttactactgacttctttgtgaacctgcttgatatgcgcattgcatggaaagcagtgtctgaagacagggaactctatgaaggcagcgaccgcaccaccggcgaagtaaaatggaccggcacccgtgccgacctggtattgggcgctaacgcagaactgagagctaacgcggaagtatatggcagcgcagatggccaggaaaaatttgtgaaagacttcgtcgcagcctggaacaaagtaatgaacctcgacaggtttgatctcgcttaattaaattaaaagaataacaggagcctccttcaccgggggctctttttttatgcccgtttctcaccagcgaaacgccctctaaacatactgcagcagccattcctttgcctccgcatcgtttgtaaacgacttcatgggaataggcggcgtttttaacttaaacagtatattcatgatcagcttcgacaagcccggctttgaaaccattgccatggcagtatatacatgaggtaattgctctgttgaaaattttcttgtggccttatcgggaacaggagaattggaaagataaatcagcaagggtactttcttattcccggtaatctgtttcaccaatgcaatattgcgcgaaatattctctactgttcgcagtgtgcttttcgaataggaatataaaatccccgtactatcataataatagtccgctatttctccttcaataagtggaatgttattgggcgggttcatgaaatgactgttttattgtacgctgtaatttactttcttaattccatcatcgataattgcagaccgggccttaatgggtactgtacccgccatggcagctttattggaaaaatttacggtgacttttatctggttgccgtatatcatttgttgcacctgccggtcatcagaaagaatattaaaagccgtcaccggcagaaccactgctttttcatgcaatgggctccacacttttatatgatcgatgatccgtgttttattgagcttccattcagcctgatcaatatggtataaaggtggcgtgttatataaaagttccgacagcatccgggtccccacttcatcctttaatttaagagaaccattttcccagtgtgcggtggttatcaccgcatcattgtaaacaaggcggaacagcggcagtgaataggttggatcaacatatattttttcatagcgttccttgatgggtattactttggtgtagatagatggaatggtgccgccttgtccccagtaactcccaacataataagggctgtttttattttccctcagatcgggatcgccccagaacagcaccggcatttccaaaccctgggcaaatgccagtgatttagccgtaaaatcatttccgccttcagatcctactaccatcgccacttcattaccgatgtattccatccgctggagacgggccttaaagtcttgctcctttgtagtaacatgacttggcgagtaatcatcaaacacctcaccggtagcatcacaatctacaaaccaggaattgtacggaatacgatcgctcaaaatggcggctacccgctgttttacagatgaaaatgccagcgtgggattcagctgccttcctacccctataaaaccacctgtttttttccccgaggcattggtcacagtagcattgtcgtataaagatgaatcaggaaaccagcaggtacgccattccctgtcctcttttgaatgaatggaatgatagctgtcgtatgggccaatgagataaccggatttattagcttcttctaccaaaagcgggttcttcaatccatctgcccaatcagataaaccgatccacgccttctttattcccgactggtacatatccgccatcaggctcacattttcttttccccagtcgccgggatcatctataacatctcccagtgccttttttattaatcgcttattccaaacatacagttgctgctcgctcagcgcgcttgctgatgtccctggcatgctgccaaaaacatccggctgatacagcgctttcgtccggagtgctttattcagggcttcaaggataattcttttctgataatcattaatgggcgtttgcttcttgcattccagccacacctggttaaacgcattggcagcatcgtcttcttcattatcttttaacgattgtataagccgggaaaaaaacttttccttcgctggccaggaggcctgcaactgcttccaccggatattttttacggtaataagtccgtgcggccaaaaatagacatgtggtgcgccgtataatttccggacgttaggatttttagccgctttctcctccagtgtttcaaacctgtttttttcccggatataatttttatatacggtacttacagctacgggatcatttgcagtaacataaatgctgaagccataggttttgtccgggttaatagagggaaattgatggaagaaggaaaaactgatgtccgggttcacatcgaaatgcaggtcgctgttaaaaacatttttcagtacatacacaattgtatactccggcttgttggcagcaaaaaatcccattgaaaaacttccgggaaaatctaacgactgatgctttaaaaaagacttccaatagttatccttagcgggaatatatttcccctcccacaaaggcagcatataactttctgcccgaacatgcggccatacaaatttgccggcgccttccgagcggatattaacgtcgaggtagttttctttctttacaatgtttaccgaaacaagaacatcaggatagaaccacgataccgaatcagcggtctttttcaaattggctacccgcatgggaggcagcggatcgcccgctttctccgctattccgttgtaataaagattcagctcaaaggtttccgggataacctcaaacgtaaagtttgcaggtactaccggtttaacctgctgaaatgcgaatagttgcccataagataagatacaaacaagcaggttaacacttattatgatccgtacagttaacatccattcccgtacttgtttcatgctatttatttaagcgatttgctcaaatatacaatttcgctaaaataaactgccctgtattaccgccggcggcatcgtaggatgaaacaagccaacgatcgtaaacggttgcctggcacttgcatgtacattttgcgtagtacccaggaagaaatacaggtcgctgttccttgcatattcgtgcaggtatttctttctcacctcgttaatggctttcagttccttatcagcgccacgctgcttttgcaggcttttcaaatacagggacgccagttgccagtcttccaccggcagggtgatttcttcgttcttgtcatcaataaaacggaaagaaaatttgtacggcagctttggcatcgcggcaaaaggatcttccggctgctcagctaccacgccgcgcagcagctcttcctgcaatgcattcaaacggttgcggttccattcccgctccgtttcctctaccacaaaatccagtatcctggcaggtttgaataccaccagtgaagtataaaatgcttcgtgtttcgcttccatgatgaccgtagacaggttacggtatacattcttcagcacaatggctttccgctcactccaatgatcttccgttcccaggtgcccggtcttttttaccggtgcatccgggtttaccggtctgaaactttccagccggaaatcccgggtattcctttcgagatccagctccacccaatcgtagagctgatattgttcgtcataggttttctttgaaaaagggatgggatatatcctgataaaaacgccgtcttcccggaaaccggcaatgctaacctgctcctcataatgggaagatacggagggataacttttaacggtaatcaaaacttttgtcgaaggcatgcgcaagatgttttataaatatgcaaatccaatggtttccgccagggttattttaaatactttctttcccctggtgcaacgatgaatgatacggaccataaaacaattcccggtaacctttttctattatgcgctgtattaattctctcctgtaaaacatccggcgaaaataggtgaatcgttgaaaataaaaaagttagcaccggttcagttcatatttttcctggtggtttacccaccttatagatttcctccattcccccgatcgaaacattctatgcgtacaatccggcctattttgtgtaatttgtacgcataaaattttaacacatgagttttcaagatgagctgaagaaactttttgttgaagaaaatgaaatacccgaggaattccgtatttccgaaattcatcagaaagagtacctggtaaacggggaaatgaaacaatgggatgggccggtgagtgaagtgtactcccctatcaacatccctactgcaaatggcctgaaacgcaagctgataggcacttacccgctgggcaccgaaaaagaagcctttgaagcgctggatgccgccctcgccgcatatgataacggccgtggtgaatggcctaccatgcgactggatggacgcatcaactgtttgtctgtatttgcccgcaaaatgacggagcaacgcgccctgatcgtaaagctgatcatgtgggaaatcgggaaatcctttgctgactccatcaaggaatttgaccgcaccatagaatacatcaacgccaccatagatgcgcttaaggaaatagaccgcagctcttcccgctttgaaatcaaagaaggcaccatcgcgcagatccgccgttcgccattaggggtagtactctgcatgggaccattcaactacccgctgaatgaaacctttaccaccctgatcccggcattgctgatgggcaacaccatcctcttcaaaccgcctaagcacggcacattggtgcattacccgctgctgcgtgcattcatggaatccttcccgaaaggcgtggtgaacaccatctatggccgcggcgcttctgtaataccaggcattatggccacgggtaaaatcaatgtactggcctttatcggttccagtaaagtagccaacgacctgcgcaagcaccatcccaaactgaaccgcctccgcgcggtactgagcctggatgccaaaaatgccgccatcatcacgcagcatgcagatatacaagtggccgtgaacgaatgtatcctgggtgcattatcgtataacggtcaacgttgtaccgccatcaaaatactgtttgtgcaccgctccatcgccgacgaattcaatgcgcgcctgggcgaatctatcggcaaaatgaaattcggcatgccctgggaaaaaggtgtacaactcacgccggtagcggaacctggcaaacccgcctatatccgtgaagtgctcgacgacgccattgcccacggtgcagccgttgttaatgaaaacggtggcgctaccaacgaatcctttgtgttcccggcagtggtatacccggtgaatgataaaatgaaactctaccgggaagaacaattcgggccggtaatcccggttgtgccctatgatgatatagaagaaaccattgattacctgatcgaatcgccacacggccagcaagtaagcattttcagcaacaacgctgatgaagtggcgacactgatagatccactggtaaaccaggtaagccgggtgaatattaacagccagtgccagcgcggaccggatgtattcccgttcaccggccggaaagacagtgcagaaggaacgctctccgtgcatgatgcactgcggtcattctctatccgctcactggtggccaccaaaatgaacgatacgaataaaaaactgctggaagatattgtgaatgagcatagctccgacttcctcagcaccaatttcattttctaaaattactttatgccttgcagctgcccgctgcaaggcatgatacccgcttttaagatttcaggaacctggttaaaacagacaacaccacttctgccgcaggcatatgatcctggcctttcagcatggtgtaggtaacgttcgggatggcagcattcaattgtttggcgacttcctgaatagattcagggcttttttcccccacaataatttgggtgggcgtagtgagcgttgccacctcctttacgggtgctaagctactggccaaagtagtgtcgtaggcaagcgttggcgccaaagccaccatggttggccagtcggggaataagctatcaaatgcctcgccagggataccaataccttccaggaatccggtgatcgcggcctcgtttttaccattctccagcaattggtataaacccctgctgagggttttaaattcctccaggtaggcttcattgtgacaataagccgcgtcgtacattaccagtttactcactttgttgccgagtgtcatagcagcctttagcgccaggatagcgccggaagaatgaccatacaaaaacgcccggcctccggcggcagctatcatcgcctcaatatcttctatttcacgctccaccgcataaggcaaagtattgccactgtcgccacggccgcggcgatcataattgtacactgtaaattcttccgaaaaaaccgatgcatcgtacagtaccgggttaaattcacggtggcatgtagcccccgtaatatagattaaggcagggcctttgccagtcatattgtaagccagctttgttccatctttggagtgtgttgttttcatcgtgatctgtttttaaagatttgtttaatgttccgatgtaatttcaacacaaagatagatgggccacttacgatagctttgtccaaaaaccgctttgaatggtaaatttacctgttatactgatttctgaattccaaaggggtggcgcctgcatttttcttaaagaatttattaaaatttgccggatcagagaaattaagctggtaacagatttcagccatatccaaatcagtatataggatcagtgattttgcctcggctactattctctcgtgcattaagaacaatgcattcttcccggtggtggttttgatatactcggaaagatatttaggggtaatggaaagcatttcggcgtattcattcactgttctccgttctatataattgtcgttgacaagctggagaaactgcttcagcaaaattgactcaggtctggtgatccgctcctgctgctggttaagctggatgaaactttttaattgatacagaacagccaatatcttcaaactggctactgtgtgcagtttatcgtctgcgttttcatatgcaataaaaaaatcctcaaacgccagggagaactcattatatttttcctgcgataattcaaaaaagtgcgtttgttgtacatcaaaaaaagaaaactgcttttcaaagtccggtctgaagaaagaaaaacagggcagcttaaaataaacaaaatatccataagcaagtcctgagttgtaaaagctggaaagcagtccgggcgcctgacaaacgagaaagctgttcatccgcacttcattcatattgtcataaacaatctgcgactgactaacaccactcatcagccccataaaataaaatgatcttctgaacgggggtttatagaatttttttacgtcttctcctttcctcacccggaaacaaaacagatccggatcatttgttctatcaggaaacggcgtactggcaaagaattcattaatatcatcgtaaaaaggaataacacctttggaattgcccattacttagagatggtttttaatcaaacagctaaagcaccttatttttactacactattgaagataggaaaaatatagtaagctcaaataacaaagcggcgcttcatcgtgaagcgccgccatattgtttataatttcaccactttaaatgtttgccggaatcctgttccttccagcaccagcaaataaacgccactgccggttttcgcagggaaccgcagcggctgccgcacctgcccctgtgttaacatccaataatgaactacccttccctgcaaatcaagcaggcttgcatacattttctgtttcaatgcccgcggacataccacataaatcacctccgctgccggattgggataaacaaaagcatccgcctcgtgcgtgctacttacggaaaccacggcgggcctggatgtccgcagcatagtactatcgttcagtcctgttgaataccatcccgctccgtagctacccattgaactggtaacagcatcggcggtgctggtatcggtgggtattacattatacgcgcccgtacgcgtagttgaaaatgcgagccggttttgtgtggctccgtcatctgtgccgtaagcgatactgatggccgtgaaaccagcaagactgccactgcgcacggcgcaacgccagcgtcttgcagcagacaaactgctcatgcccgtacccggcgtacccaccgcactgtcagcagacacctgcatcagcagcgcgccggtaacagacgacaatccagttaatactactttcctgtactcccccgcagatccggttgggaaagttttggtaacaggcgttgcacctgcagtaagcgccactgcgccattcacaaaactactgctgctgcccgaaataccattgtatgaagtattggtacaaatcagcgctttgcctgccggcaggtggatgatgccttccgtcaatgtgatagccgcattgctcgacttcagcgtgagactgtcgctgagcattacgccaccggggttgttgatggtgatgttatgcagcgaccgggtaacagggatttcatggccttcggtcatgacttgccccggcgcatttacatcatggttataaacaacatacaatgcagcggtgcttcccaatgtataattattggcgagcgacgcatgctgcgaacgcctgatctggcagttcacagaactggcgctgccgcctacctgtgtattgtccatggtgagattactaccgttatgaaacacgccactgataagcgttagcaccgacgggatgcttacaggtgtttgcaacgtcacaccggcggcattattgattgtaacactgcggatgataccattcgtataacttcctgttccgccaatcgcggtgctatctgctgccggccccatgatcagggtggtgctcccctttgaaaagtcggcggtgccgttgtttaccaggttgccgttcaccgtaactgttctgccaatggtgccgtttcttgcataaaatgtaccggtgttgttcactaccaggtcgccggtagtgaaggtgtgagtggtagtggtattgaagcccagtgtgccggcaatttccgtgcgtgttactttcaccggcgtattgatcgtaatggtgctgcctgcgatgatcacagcggtatccgcatctgcgggtaccacaccaccctgccagctgccaggcaaggaccagctgccgccggtggaagcagaccttatgagttttccgataatagatggtgttaccttaaacgggatagacgcattggcaatcttcccgcgctgatcatgtacgtatacatataaccggtagttgccggcggccgccggcgccgtaaagcgggcgctgtcggcatgctgcgaaacaatcaaacccgggagcgcaggcaaactggccgtagcctctcctccggccataatactgttttcaggaatgatcagccattcgtaacgcaatgaatcattatcgggatcactggcgcgtacccacccggtattaagagaatttgcttccacgatcacggtatcttcggcgcgcttcccgttgaaaagcagcgaatccctgttgcggatcaccggtgcgtgattcacaggatactgtcccgtccatacatactgcatttcatcagcagctccgaaagcttctcccagccggttatacagcccgaaccaggtaactacgtcgccggaagattgatatccccatacaaacacaaagccaccaagacaattattggacgcattcgcagcaatatgatcctggtatatttgtcggtacactaccgccttttctgtactggtttgttccaccaatccgccccagggcattttccgtgaaggctccggattcatttgccaggtgcctctcggcccgaactccgtaatcatatagggtcttgtccagccagcggtttgcaggttgcccaacacaccgggaatattaggcgcatagctgttaatggaaagtatgtccaatgctgtaaatctttctttcagcaacttaatcttctttacatcggagttcaccagtaccgcagtggtgaggtggttggtgtctacctcatggatcatttcggcaatattgttgagcgcatcccagaaaaggatattggcagctgtatccaggctgttatagttggcatctgtttcattaccgatcgcccacatcagcacggcaggatgatccctgaatgcgagtacctggctccgcatattttcaaattgcaaccgcacggcagcggtatctccgtaattcatttcctgctgcttcttaatacccaatcccaaacaaacggtgatgccatgcgcattggcgctgtcgagccacgctgcggtggaatcgttgatactgtaagtacggatggtattgcccccataggtagctacctgcacatgaaaattgttggcggcggcgcctttaatgtaatacggcacaccgccgcgatgcagggtatatacgcccgcagtttctgtcaacgtggttttgacggcctgcgcaatcgcgttgcccgcaacggccagcaccgtcagcataagtatcagttttttcataagtggaacgtggttttaaaaagtgagtatatctaccattcctccaggtaatccaggtctttatgaaatgtttcctgcatgccggtaagcgaccagaaagccagtgccaggcatatcacgcccacactgatgccggcatacaccagggatccgttaaaaagcagttgcatggattgaaagagaaaggtgagcggcactactgcgccgcgcacaaaatttgggacggtagtggtcaccgttgcccggatattagtgccaaattgttcggtggcaatcgtcataaaaactacccaatagccaaccgaaaaaccaagcaggccgcatatccaataaaagagctgcaggctgatacctgccgccaggaaataaatgctgacagcagccatgcagcaaaacaggtaaacatatactacccggatcctgctttttaataactggctaagggcgccgctgaaaatatcgcccactacaaggccgccataacaccatgccaccgccgcaccggcattcacatcgccctggatatgcagcactttcccaaattcaggtgagagcgtgatcagcacacccaccacgaaccagagcggcacgccaatgaggatgcagcgcagatatttaaagaatctcttcccatttgtgaaaagcgccaggaagttgcccctgttctccgaatgcttcgccgccccgaacatgcccgattctgccacaccaatgcgcagcagcaataataaaaggccaaggccaccgccaataaaaaagctggttctccaggtgaaatactgtgcaacaaaatatgccgccaccgcaccgctgatacctaccgccgcaacaatggtagtggcataaccacgcttttctttgggcatcagttccgccaccagcgtgatgcccgcacccagttcaccagccaggcccagaccggcaacaaaacgccataacgcatagctccacacgctgtctgcaaaaccattggcaatgttggccacggaataaagaaaaatggagccgaaaagtacagacaaccgccctttcctgtcgcccagcacgccccagagaataccacccagcaacatgccggtcatctgcacattgagtaataaaatacctttgttggttacatcctccccacgcagtccaatcgactgaagactgggcacacggacgatgctgaaaagcagcaggtcgtagatgtctacaaaatacccgagagaagctactactacggcggctaaaacggcgcccctgttcgactgttgtatgttcgtcatctgctataatttattccgctcaattgaaagtacctgcccgtctttcagcaataccggctgtaaaacatcataagacaattcctgcagggtaatattccggtcgagcgcaagtgcggcagctgtgccggcagattgccccagcaccatgaataccggctccatgcggatagaactgtaagccacatgtgaggccgacaggcataccggcaccaacaggttgaccgcttcggaggactttggtcttaatgaacggtaactgatcgtgtaataagtgttcttctgtttaccataactgccttccgcatgtactctcccctgcgcgtctaccacgcgggaaacatggtgacaatccagcggataggtggctactgccacggcatcttctaccggctcctctccattgcagttcctttctgtcatcacataatcgctcaccattctcctcgcctcccgcacatacagttgatgagggaagttgccattatctgtaaactcatctttcggtaaaccccagcgcttcatttctgtgcgcagggaatcgggtacccgcggatcgttacccaggaaccagagtaaacccagtacatagtccttatgcatttgagcgatcttgtcccgctctgcataattgccttccggccatccgtaattggcgccaacgaaatcggcctggttggtatccgtttttttattgggcatgggggtgaaagaaataatatttttcagcatgtagccgggattcatttccagcatcctcgccaggaattcataccagagcggctgatagccggcaggttttacaatgtcgatacggttcgccggatcatcggtcagcgtcatccggtaacagtacgattgcgtgcggtgatcaccttccccgtttgcacccggaatttttggttccaggaaaggcagcacaccggaggaaggctcaccttttttaatataaggatcgatagaactactgcctttgccaatgatatcgttcagtttaataccattcaacgtttcattataaacactatttgcttccctgcccacgatgttggaaacaccggcggttgccatcaggtctccttcgtaggtagcgtcgataaatatttttgcatgatagcgatggccattctccatttgaatggaaactatgcgggcatctttttttcctacgccttttttcagctgcagcctttctttatataccacagccacgccggcttcttccagcatttttttcaggatattttccgctacgcgggactcatacacccactgcattttcagggagtcgttcttcccggagaaggtgcgctttttggaacgttcaaaaaatacgtctctcgattcgcaacgccatgcgctgctatcactgtagtacgtatacaggcgctggtaaaattggcgtgtgagcccgccggcgctcctgaaattattcaggtcggtggccgtaaggcccgaagtagccacaccacccagatgtcccgtgttgctgatcagcaatacctgtttattcattttcgccgcctgtatggccgccattatgcccgcgggcgtttctccatacacacatacatcccagcgcttctgggcctgcaaccggttactgcccagcaaaatgatcattatcaccaggctacggataattgaagtcctcattttcgttattatttaagcatgagtatagctgcacgaacaggtaccttcctgttcgtgccagccggaaaaaagttatctgatcagaatcccgggttctgttccagcagcggattggtatccatttcctgcgacggaatagggaaaagcgtgtcggaatccctcactgttatagccggatcctgcgcgttcatggcctgtttcagtttgccggtacgcaacaggtcgaagcgccgctgcccttcaaacgcaaattccagccgtctttctttcagtacggcatcctgaaatgccgcagcgctcaaacctcctgcaagatcttttgcagacggcgtatttaccggcaggccatacgcacgccttcttacctggttaaatgcctccagcgcttcggtgctgccggggctggacatatacagcgcttccgcgaacatcagcaatacatctgcataacggacaatgtaatagttattaccgccatcattcacattcagcgctgcaggatctttaaatttggcaacgtaataaggattttttatcgtggcaggcgctttgggatcagtggtataggaatacttaatcacgtttacatccctccgcagatcgccctcagcataggcttcataatgattcttagtaacaggattatcgccattgccgccgaagccgggacgcttatcaaacgacggacgatagaaacccgcaaagctgctgggaatattaccggaaccgctcaggaattgcacttcaaaaatggattccgttttattttcattagcgatcaggaatacatcctggtaagatgcccaaagcgagtaacgccccgatgtgatcaccttccgggcctcttccactgcctttgtatattccttccgggtcaggtaggtttttacaagcattgccgtagcagcgccactggtggcccttccggcgttcaccgcatcgtaatccggcggcaggtgctccgcaccaaactggaagtcggcaataatctgcgcatacacttcttcttcagtagctcttttaacggcaagattattcaacgaagtggtaggtgcaagctgcaatggtaccccgccaaaaagacgaacgaggttaaaatatatcagcccccgcacaaaacgggcttccgcctgcatacgttgctttttatcgctgccaacggccgtcatggccccgatattttccaccgctgtgttggcgcggttgatcacctggtaagaagtgctccagaactggtagaacaaattagtaccggcatcgaaattgaatttatccagcgccgttttatcggtattgctggtgttgcggccaaagccccactcacagtcgtccgtgccttgcgactgtatcacttccatgaactggttgtagagataagagctggtcatgccggaatacacggcattgacggcagacaccgcatctgcttctgttttataaaagttgtccgtggtataagtgccttccggaacgccgtcgagcttggcgcaacccgctgccgccagcgtaaaaaatatgatgatgaaataaaatgcagatctcatgacaaatgattttgattagaagctggcattaataccaaaagaaatcgtacgtgcgttcgggtaagcgccggagtcgaagcccgggcttacattgtctgacccataacggcttacttccggatcaagccccgagtagttggtgatggtgaacaggttctgtacattcacatatacctttgcagcgagtttgatgcgttgcaggtttgcctgcggcagattgtatcccaactgtaccgttttcacccgcatgtaagagccgtcttccaccatccggtcccacgaacgggcggttggcttcacggtggtagcacgcggaatattcgtattggtgttatcgggtgtccagcggttaagcgtggtagtgctctggttttgcaggccggtaagattttccagcgtactggtgttaacgttatacagcttgttaccgtaaacgccctggagcagcaccatcaggtcgaatcctttcagtgaaaatgtattgctgaatccgaaagagaatttcggctgtgcgttacccagtaatacgcggtcgtcgtcgttgatctttttgtcgccgtttacatccctgaagcggatatcaccaggtttggcagttttttgggcagaagcatccacttcttccttcgacttaaaaatgccatcactggcaaagccgaagaaagtgcctagcggctgtcccacctgcacaatggtggattgattaggtccctggcctgcaaagaggcgttcggcaccggcaaggtccagcactttgttcctgttgaaagaaatattaaaaccggtttcccagcggagatccttttccagcggcgtagcatttaccgtgaactctatccctttgttttctacctgtcccctgttttgcagtgaagtggaaaaacccgacgtggtaggaattttcacatacaacaacaggtcgcttgtttttttatagtacacatctgtgataaaagtcagcctgttatcaaagaatccgaattcaagaccgatatccgattgcgcggtagattcccagcgcagatccgggttgcctacctgtgaaggcgtaagccctatcacgttcacgccgccgatggaatagttagccttgcccatcaggtcgagtgaaggataattgccgatgccgtcctggttgccggtgaggccatgactcacccttaacttcaggttactgaaaacatgcaggtcgcgtatgaaaggctcctggtccagcttccagcccactgctgccgaagggaaaaaaccgaagcggttgtttttcccaaaacgcgaagagccatcgtaccggccggtgagtgtaagcaggtatttgttccggaagctatagttgatcctgccgaggtagctgagcagcgcccacctggcaatgctggaagaagaaggttgcacagaggccgcattgcccaatgcgttggtgccgaggttatcgttcaggaaaccttgtgcttctgcaccgagcgactgataagaagaactttgctgggtgaaaccaccgagcaggttgagctgatgcccgtcacggttcatcgtgtagttaagcgtattttcgtttaaccatgtaaaggtttgattggtggatactgctgcatttccgcccagctgagatccggaatacacggcttgcggaaggtatgtatcattgcgggcgaagctaacgtcggcgccccagagtgttttgaaagtaagccctttgatgatgtcaatactggcgtatacatttcccagcgtacggtaaacgttgttatagttcttatagttttcaatcaacgccaccgggttatcgaaaggcgcgccctggttgttcacttctgtataactgccatccggctggtatataggaaggttgggagcggtagtggccattgtaaacagggaggaactgttcacccggttggtgcgcacattactgatggtaaggctgctgccgagtttaacattatcccggatatctttatcaagattagcccgcaacgaataccgcttcagatcagacgcccgcacaataccctgctggtcaaagtaattggcagtaacaaggaagcgggtctttggatcgccgccggaaaatgacagggaatagctttgtatgggagccgttctgaagatcgcgtcctgccagtcggtggtggcgggcgttttgctgagatcatataattcagggccgttttcagcaacactggcttcattggccagctgctcaaactgccccgcattcagcagcgaatattttttgagcacctgctgcgagccgtagtaggaatcaaatgtaacgcgtgaatcgccgcgttgtccgcgggaagtggtgatgagcactacgccgttgcccccgcgtgaaccataaatcgccgttgccgaagcatctttcaatatttcaatggaggcgatatcggtaggactgatactgttcagtgggttaagcgatgtaccatcgctgccctgatccgcaaataccggcacaccatctatcacatacagcggttcattgctgccattgatggagttaccaccacgcacgcggatagaagatcctgcgccgggcataccggagttctgcacaaaggtaacacccgctaccctgccctgcaatgcctgatccacagagcggataggcgttccttccagcgttttggtatttaccgaagcgatagcgccggttacatctccccggcgttgtgtgccataacctaccacgatgaaatcactcagggcagtattctccatcgtgataactaccgtaatagttttacgtccatttaccgcaacatctgttgccttatagccaatcatgctgaaatgcagggtggctgtaggcagcaccgataatataaagtcgccgctatcattcgtaaccgtgccttgttttgttcccggcaccgaaacggatacgcccggaaccggtttgccatcggcatccgttaccttaccacgcacctcaatggcgggatcggccgcctcgtacgttttttgttttacaacaatcgttttgcctacgatggtataagtcagcgcaaactgccggaaacaaaggtttatcgcgtcctgtaatgtgccctccgtaatatctacgctgaccttttttgcgggatccagcagtgcatagtcaagaaaaaatacgtagcccgactgccgctcaatattcctgatcaggtgttcgagggatacgtttttttcatgaagcgtgaccttttgcgcgtaactactgctggcgtgtacctggcaaaaacatgccagtaaaagaaagtatgtcagtttcataatgagcctgatttttctgcccggtaaaaggcggaatcgcctggtaacaggaaaatgtttctcgctcaggtttttgaagagacctgataattgcataaattggaattgtttaggtgagataatcaatctttcatacacggaattattgtaatgataacctgaacaaaacggaggtggtaacgacacttccgtttttggttatattaccattgctgtcatttcataagtggacaatgttggttgttgatcgtttttattggtgaataataatggtatcgcctttcatggaatattgaatgctgctaagctccagtattttgagcgcttcactcagcggcacattcctcggtatcttgccccagaactctctttttccggtattgccttcataacgaacttccacatcataccatcgctgcagctgccgcattacatccgtcagcggcgccctgttgaactggaaatagccttctttccaggacactgcttcgtcggtatctgccggaccaacggtgatactgctgccaccggccgcccaactggcctgctgcccctgaacaaggcgaacacgctgactgttatgactcactttcaccgcgccctgtaacaaggtggtttttacgtttgcttcattctggtaagccataatattaaagcgggtgcccagcacctctactacgccgctgcccagctgtactttaaacggcatattatcccggtgtgccacttcaaagtagccttcgccgttgagtatcaccgtgcgctctttcccgttaaacgcagtcgggaaacgcagggatgatgctgcattgagccataccatcgtaccatccggcagctctattttgaactgaccaccccgtggtgtggccagtgtattatacaccacggcagcatctgccacccggcctgcttcatattttaattgtccgtttatccggatcacttttgccgtaccctgactggggatcacttcatgagcggcactgtcgagcactactgtggcgccattggccagggtgagcgtcgctttgctgccgcccggcatagcatcctttgcggcgctggccagcgtggtggcgggcgctgtaatttttgtggtacgggaatactgccacgcaaaagtggcgactgccagcaacagcaccgccgccgccactttcggcagccattttttatagagcgggattaccttcacgggttgcgcggcaagcagcagtttttctcttacccggtcgcgccagggcccttgcacttcaggagcgggcaggccaaacgaagcattcatttcccccagcagcaaacggttggatgcgtcctgctgcaggaagtcgaacagctccctggtttccgcgggagtgcagttattgtcaagaaagcgccgcagcagttgctggtaatgatctttttcctgtggcatgtatcagttttgtacgcagtacgtggacctgcttgtaatatatactgtcgccggaaaaaagagggtgggtgggtgaataaataatttttattattatataaacagccggtgtcagagccggtgtaggaaaagcagtatggccagagagaggtcgccgtgccggtagaaatacgctttgatatccttcagcgccatcaccatgtgttctttcacagtattacgggaaatgcccagctcctttgcggcctcctcatagcttttgccttcctgccggcacagcacaaacaccttttgccgctgggaaggcagttgggtgatagcgttgttgagcatttgctggtactgggcccacagcgtctggtgatagggcgattctgttatttcgccgatccgctgcatgatctgaaggcgggtagcttcgtcggaagcattcttttttaggaaagtaaaagttttgttacggctgattttataaagataagcgggaaaagattgcgcagggtccagccggtcgcggacttcccatattttcaggaatacgtcctgtacaatgtcttccgcataagcgggtactttcacaaaacgaagcacccatccatacacgtgcccattgtattggtcgtacagctgcatatatgcggctacatcgcccttccggagccgctccaggtattctgcttcagtgatcgtggaatcccccatttggcataaatgtaataaaattgggaattagaaaagtggattctacggaaaattggagcgggcatagtgtataggaagtgcatggggagtccatgagtagtgcattggaagtgcatcagaagtccatgcgaaccccattggttacccatagcctacccatggtataggcattcgtaaagtattcgctacattatttctgtgtccaggaaaccaggaatcattgccatgagtaaatcagtcctttgggttaacgcggtatgcatggttccgggcaatatggccaattgcgatgcgggcatcgacaactcccccaggctcccaccgcccaataatctgtataactccagcacatgctccggccgaacgatatccgcgtcgccggctataatcagggcaggggtcttaatattccttatttcttctaccggccagtcttgcaccttttcttcaaaggcccttactttggcaagaagtgcgggccagtcttccggccgggcggctgtacgcaggtactccgcttcataagggctccccttcagcgcttcgttcatcacttccggggtaaacaggatgctaagatccggatggcgcccgctgctgttgtagctgacggaggccaatatcagttttctgacggcgcccggttggcggatagccacctgcagcgctacacctgctcccgtgctatagccgaaaatatctgtttgtgatatattcagcacactgagtaaagcaatcacatcatccgcaaattgctcataagaaagcggacgctccgggatgtcagtggtatgcccgtatccctgaaactcaacggcgatcacctgtctctccccggcgagtagcggaattagctttccaaatgcagtgccgattccggaaagcgctcccggtaacagcaggagcggctttccttctccgtgtatttcataatacatctttagtccattcacctccgcataattcccatggatcgtatatttttctgagatctgcatagctgtttatttgcctgctaaattcgcttcttgccggcaaacaaatcttggtatacaccaacatcagaatataacgttgttaaacagcttgctgaaattagtgggatctatccccaggtaagacgcgatgtacttgtggggcaccagttgaagcaggtcggggtttttcctgcaaaacgttttataccgttcttcaatggtcatggcacgcagatcgatatgcaggtcaatcatacctgctaacatggcttccgtcattcgcctgaaaagcctctctatttgctgcgactgatcgatcagtttctgcaggttatcgtaagtaatatactcgagttcactgtcggttaaacaggttaaaaagtatttcgaaggttcctggaacgaaaaagatgctgcgatggcgcatagataagggaaataagtaaaggcaagtgtatagatcttgtcgcccgtatcaaagtacgacatctggacgccgcttttcacaaagtacagctcgcgttgaatctgccccggtaccgtaatgaactcccctttcttaaacaaccttacgccaagactatccgtcagcagttgataatcggctatactgatatcatgaaattgccggaaaaactcatatcgctccataaattcaattcttaatatatagtatattcactttttaacgcaggcgccttatgaatatagacaatataattgacagcatatatccgttaccggaaaaatcaaaagtcttactaaaagaaaatatttacgaaataacctatcctaaaggacatgttttatttaaagtgaacaggatagaatctaaaatgtatttcatagcgaaaggtgtggtacgggcatacgccaatccgggtgaggaagaagtaactttctggtttggaaaagaaggcgacgctgttatctccatgaaaaactatgtggacaatcaaaaaggatatgaaaccatagaattgctggaatcatgcgacctgtatgaattaaatacggatcatttgcgtaagctgtttaataaagatattcatatcgctaattgggggcgaaaatttgcggagcaggaattgataaaaattgaagaacggcttattttcaggcagtgcagaacagccatggaacgctacaaagaactaatgacaactgatccggaattactgcagcgggtacaacttggtcatatcgcctcttatctcggtatgacacaggtcagtttgagcaggatcaggtctgaattgaaatagatttcaaagtttttatcatttgtaaaatttttactgccggcaacgtgcgaccttagctactctaaatcaattatcatgaactggattattttaatcatcgctggcttgttcgaggtggcatttacctccagccttggaaaagcaaaagaatcaacaggcaccaccatgtatttgtggtatggcgctttcctgttctcactggtggccagtatgcttttactgatgaaggctactcaaaacctgcccctgggaacggcctatgcggtatggacaggtatcggcgcagtgggcactgccttgatgggtatttttgtttttaacgaacccgctcatttctggagactgttctttatagcaacattaataggatctattgttgggctgaaagcggcctcacattagcgatatcagccggtgaaaattattgttgcaaagaagcgtctaataaattgtgaggatcgttaattcttctttattgaacaggaattgatctcccgcttttttttgcagcaataatttcgccaggggtgtatagggagacaggaaaaagatggtctgctcatctatcagttgcctgcccagtcctgctgcaataaaaaaagactgctctgcacattgtaccagggcgcctgtttgcggggtggtataaatactatccgtatttacctgctgcaaccttgccagttcctttacatgctccgcctgttgccgtgcatacatatctttctccaggtggcccattgctcttcctgtttcatatttatcccccgccgaacttttatcttcaccattcgctgcctcctgtgcgcggtccccggccgatttagccatggcaatacgttcggatattaactgcagccctgcctgttttaacctggctttaaaagcgatcttctcctggcttgtcataaaggttcattgaatagcaagtataatacaatattcatttaacattacaatcaacaggtaaaaaactatctttaataattcaaatagataaaatcaggcgttaatggaaataccagcaaacttcattaaaatatttccggaatatgaggatgttttttatggtgatatagaaaatcacaggaaatatttcctgccgttgtgttctgttaatttgcagttcctgccccagggaaaagatcagtggctgcattttgtatcggtaaaagagatatacaacggccggttaggcgaaaacaccacctcttttcataccgactataccaggtgcgatatgcttggttttgatattatcgatagtaaatataagtttgacgcgccgtgggaatactttaccgtttccactgaaatttcgccggagaattaccacctggaatatagcgacgaagagatccaatttaattttaatgatgcgatgtatcagttaaagaagtcgtattataaaaaattcggagaattatacgaccgggatttccaccggccgggattaacggtagacgacatcaggagattagaacggctgctgaaacttactgcggatgatttacggaacgatgcaccttcggattacatgtcagaaattatcggcaaaaaaaccaacggggtaatagatgaaattaataccggtcatcttccacttgaagaatgccaatacacgggtgacaacctgatggaaaagcctgtgaatgcagatggacacctttttaactacatagcctgtatggaaggataccatttccaggaaaatgccgcagatcagctctatttatttcataatgatgagataaagaaggcggtaatttgttttgaatatacctgataaccgggatttttatcttgacccggttgctataacgaacgcctttaatgcagccatcttaccatcacgaaactgccatacgtcgcagtagtcgtaatcgaccatcgtgccgttttcgtccttcatgcttattttgccggttgccgtaacaaactccccttcggcgatgagggcttcgaccatgaacctgggcggctccaggtatgctgtagccatgtattgtcgaacagcttcctttccccgcagggttttgtcgcctacaaatgtccattccgtatcgtctgtacagaacgacaggaacccctcattatcgcctttagtgatagctgcatttgctttttccagtatggctttattatccggattcatgtattactggtttacttatttaacaggatctaaagaacaggtaagcgtaccatatcccaactggtcataaccgccactgttgggcccatagttaccaccaccgccttccggtcttactgcctgtgccatccgttggcagttcggcgccgcaaggcctttacggttcacatagtgattatataccagttcccagatgggccgcatattacctcttcccccgctgctgattaccggttgggtaacgcctacgcaattgctgtaggtaacgtatggtacggaatcgccgagattatattttgctacgtattcagcacctttgagaaagcggttatcgtcatagccgtacaggtcctgcccctggttccatgccatctcacaaaaggcgcccatcaggccaatacctaatgttgcatggccctggtcgcggccactctcctgccattgccccagccctcccgggtgaataaaatataccgcatttccaatagcaccattaccggccccggatttaaaataactgatggcgtcattgtagatgtcccggttatcacaaagcacaccgatagccagcagggagttcatcacgcaaaggtcccagttggcgtagaaatggctcatacatctctcctttcttgtaataaagttatgatttaacggataaaaaacatgcagcatcatttgctggaaacgggtgaaatcggccgctgcccagccattatacgaccgcatgatttccgctgcattggcaaactggtatccatacaaaccggcggcgaggttcacatcattattgccgccgagtcctttcaacctggctgaccaggcattcatgatctctatggatttatcggcataggatttttctcctgaaatcttccatcgtaaggcagtggcgtaggctgcggcgatatcattatacagccgtgggtaattttccgggtgaacaccgtctctgcccctgtaaatggtatcagccggattcggctgccaggtgagggctgcgtgtgagttggttagtaacttgttccaaccggacatccagggctctgccttctccgccacttttgttttcatacgatccaggtcggcttgtttatgcaatagcccgggatgtacaaaagcggtatcatggtcgttaagcgccagctgctgcgttttcgttgacatatctttcctgcatgccattaaatataacaaggtaaaaactgcagtaaaccagcaaagtcgagttgttctcataggaaatgaactatatatgtgcggcaaatataattgtaataatgacaattaaaaaaacatgataactatacgagctgttttctttttactatagccgacatatagaatgggaatttaacgtaatgattatcaccaaagaacccggtttggcagaaactgtataatttttgtcattgcagccacgccgattcggttgtatttttgtggtcacaaagcaacgcatcatggctaccaatacttccaaacttgttgttattgttgtccttcccggcagcagattgctgacgctggcaggcccggcagatgtgttttcctttgcgcagcagatgctggaagcggaatccggggggcattccaaaggatatgaagtagtgttggcaagtgccactaacaagaaggacctgcaacttaacagttccgccaggttggtggctgccaccacggtgcatgaaatagaccgggagatagataccctgatgctgattggggcgcgactggaaaaccaaccggattcagatcagttttatcactggctgaccacgcatgcaccgaagatcaggagaatagcaggcgtatgtgtggccacatttgtgctggctaaagccggactgttacataacaggcgtgctaccacgcactgggagcgtaatgatgacctgcagcgccaataccctgatattatagtagatactactccgttttttataaaagacggcaatatctacaccgctggaggtgttacctccggcatggacttgtcgctcgcaatggtggaggaagactatggccgggacattgcgctgcgggttgccaggaaactggttatacacctgaagcggccggggaatcagaaacaatttggcggtttgctgccgggctatgagctggtgtctccgttgctggtacaattacgtccctggttactggaacacctgcacgaaaacatcagtgtggaggaaatggcagctcaatgcaatatgagtgcccgtaattttgcccgggtatttctgaaagaaacagccttcactcctgctaaattcctcgagaaattaagagtggagatggcgcgcaattacctcgaaaactccgcgctctccctggaggaaatagccgtgagatgtggtctgggcggcctcgtttccatgcgcagggtattcctgcgtcacctggaaatatcgcccggcacttatcgcagtactttccgtactgcactgcataccgattaatttattcatcttataaaattggatatcatgaaaattgctatcaatggattcggccggataggaagaatgaccatgcgggcactccttgcccaaccaggcgctgaagtagttgccatcaacgatctcgcagatattaatacgctggcacatcttttccgatttgattcggcacacggtaagtttcccggaacagtggcagtaaataataacgacctggtgatcaatggtaaacatatccggttattgaatgaacgaaacccggaaaacctgccctggaaggagctggaagtagcggttgtcattgaatctaccggacgctttaccgcgaaggaacaggcgcaggcgcatattacggccggtgcaaaaaaagtgttgatcacggcgcctgcaagtggtggtgtgaaaaccattgtagatggcgttaacaataatatcatcagcccggaagataccattctgtccacggcatcctgcaccaccaactgtatcgccccggttttacatgtactgcataacgcctatggtgttgaatccggctttatgactaccatacacgcatttacgatggatcagatgttacaggatggtccgcataaagacctgcgcagggccagggcagccgcccaatcgatcatccctaccactacgggtgcagccaaggcaataggagatgttttacctgatcttaaaggtaagctggacggcttttcctacagggtaccggttatagacggctctattgcagaactgacgcttaacctgtcaaagtctgcctccgcagcggaaataaatgagttgcttaagcatcatgctgacactgatctggcgggaataatggaatattccacagaccccatcgtttctgttgatatccttggtaacacccattcctctatcgtggacagcctgctgacaaaaaatataggcaataccgttaaagtggtggcatggtacgataatgagatgggtatctctaatcgtatagctgaactggttagtacgttataagattatagatagaatagaaaagccgcgcgaatcttaggatttgtgcggcttttcctgcttttatctcccctgttttaatcctgatcaaattaattattcccgttttgtatgtataataaaatccttttacatacatttacgtaattaatatcggaaatgaaaggtacaaacctcggagaatttgaagaactggtgctactcaccattgcagcgttgacaaacgaagcatatagcgtagcggtatgcgacgaactctcaaaccataccggccgttctgtgaaacttggcgtagtgcactcggtgctcaaccgtcttgaagaaaagggacttgtgaaaagtgagctgggggaagcaacgaaagcccgtggcggtaaacgcaaaagattctatcaactcacgatgcacggacaggcagcattgatcaacgccaaatcgatgcgggatcagctgtgggccaggataccggcgcttgcctggaaaaaaatgtagcatgaaagaacaacggcaacaccatccgcccgcctgggcgcagcgctttgtagaatggtattgtaaacccggacttgtggaagaccttacgggcgacctccacgagtgcttcgaccggaatgtacaatccatcgggccacgccgtgcgaagctgatctacatcattgacgccttcaaattcttcagaagttatacggtacgaagatcaatatttgtcaacctttttacgaaccgcattatgatcggaagctacgttaaaacatcagggcgcaacatcatgcgcaacaagctgttctccttcatcaatatcctgggacttgccatcagtatgtccgttgggttactactgatcgcgtttctgctcgacctgcgttcgtacgacaggttccataaaaatggcgacaggatctatcgcatcaccaacgtattaacctccaacagtgaagaaaacggcaagtttgcgtctacctccataaagacgggaaagctcatccgcgagaaggtaagcggtattgaagaagtgactacgatgcgcaacaacttttcgggtgatgcgaaggtaggagacaatattattcccatccagggctactgggcagagccttcgctgttcagggtttttacttttccgatgctggaaggcaaccccgaaacggcactgaaagatccgtattcggttgtgctcactgaaacggcagcaagaaaactgttcggtaaccaggcggcgctcggaaaggccatcaggattgataccgccgtttaccaggtgaccggtattatgaaggacgttcccttcttttctcatctcagttttgaagcgctggtgtcgttgtccacagctgagcaaaccaataaaggtgataaaaattttgacgcatggaccaacatgtggtcccattcggtgtacgtgctcccctcaaaaaatgccgacatggatgccatccggtcgcagctcaacgcacttgcaggaacggaaaatctcgctgaagaaaatacaaagattcagctcgaactgcttcctttatatcacatcgtggttggagagagcctccgtcaatccgagggtgggcctggctttgcaggccctcacatgccccctgtggtgctttggatacttggcgggctcgcatctgttgtgatactgtctgcctgcttcaactacaccaatctttccatagcacgcgcaatgcgccgcattaaggaaataggtctccgcaaagctatcggcgccggaaagagccaggtgaggctgcagttcctggccgaggcggtcatgatttccctggcctcccttctgctttccttcctcctgtttcttatattacggccgatgctgatcaacatggcccccgagatgcagcataccgtaaagctcgatctcacaccatccatgattgcagccttcatcgtttttgcggtggctgtaggtgttatcgccggattcattcctgctatattcttttcgaaagtaagtccgatcaatgcgttcggaaatgcttcctccgtgaaaatgttcaaacacctgaccttcaggcgcgcattggtggtgattcaatacaccgttacactgatctttatcactactaccgccgtcggctatgtgcagtataaaaacatactggcattcgacctgggattcagcaccgccaatattctgaacatcaacatgctggataataaacccgacgccatgctccaggaactcagtgagctgccggaagtaacggcgctgtcccggtcgctgattacaacaggcgttgggaatgcatggggcagtaatatgaaatacaaagactcgcgggattctgtgctggtcatgaccaaccacgttgatgaaaactatttgccgctgcataactataaactcgttgccggcggaaatttcattgcccggccggccaccgcccaggccaccggcgaggtaatcgttaatgagcaggtggtaaagcgatttaacatcggcgccaataatccccggaaagccatcggggaacaaatcatattgaatggacgcaaaatgaccattgttggtgtaatgcaggactttcactacggcaaagtggacaacctcatcggaccggtagccttcaccttctggatacctgaagacagggccatcatcagcgccaagatacatagcaccgacatgccggctaccttagccaggatcgaatccatatggaagaagatcgatcgtgttcacccgtttacggctgaattttataccgaagaaatagaagatgcatacagcgaattttccactatgatcaagatcattggtttcctttcggttttggccatttccatcgcatcaatggggttgttcggaatggtggtattcactaccgaaacaagactaaaagaaatcggcatccgcaaggtgatgggcgccagcataggcaaccttatatacctgctgagccgtggctttctattgctgctctccgtgtcggcgatcatcgccctgccggtaacttacattttcttcagcgccgttgtgctcccgaatttcccctatcatacacccgttcatatcaccgagcttttcgcaggcttactcgcggtgttactcatcgcgttgattatgatcggatcacaaacattaaaggccgcgaggagcaacccggtagcggttttaaagagcgagtaacaggagaaatatcattaaactaagcataatatggttagcaggagtgaaactgaaatgatggaattaataatgggagtggcagaaagaacacctcagatactggctgtattgcaggatggatcgcgatctaatcctaatgtaacaaaggatatcttccaggattacgatattatttatgtggtagagagtctcgacccattcgtacaggatcatagttgggtggatgtatttggagaaagaatgataatgcagatgccggaagacatggaactgtacccaccttcaccggaactggcaggcgcattctcttacctgttgcagttcaaagatgggaaccgtattgatctggtaatagtacccctggaaatactggatcacttcaccagtgatagtctttgtaaagttatatgggataaaaagggcgtgttaaatgatcatcccctccctcctgcaagcgacgggagttatatcgtacaaaagccatcagcacgttcgttcatcgattgctgtaacgaattctggtataccaatgccggcctggcaaagggattgtggcgcgaagaagtgatactggtcaaggaattactcaaccaggttattcgccaggcattgatacagatgatggattggtatattggctgccgtcatggatttacagtcaacccaggcaagtttggaaaattctaccagcgttacctggagccggaagtttacgaaaaaatgctggccacttattcagatgccgacctgcaacatatatggcaggcagtgtatactaccatggatctcttcagcaattccgccaggtttgttgcaacgcagctgggttatgagtatccggaaagttgggatagggatgtaacggcttatatggtgcatgtgcggcagttgcagaaggatgcggaaatgatttatgcaccggaataaatgccttttccttttgcataatctaaaaaaaatacaggcttgctggaaaagctgttgtgtattacctttgcgacttacaagcaaaatacatgagtcaatttccgcatataaacctgtcattaaagaacaaactgacattcacggccaacccggtaaacgtagtaccattgccggatggagagatcctgatgaactttgcaagtcagccgctgattacaaagctcaatgccaatcttgaaattgtctgggaaaaaatcatgcagggacggaatgcgaactatgtcagcagcaagctgtcggcctctcctgatggccgcctgattgccattgcgggtataaccgatatgcgcattctcgatgcagaagggaccatggtattacattcggtggaacataagtcctggggctggttcctgggtgcggcctgttatttcgccagggataataagacgatctggtatgtactaccaggcgatgaaaatgaaactgacaagctgcaggtaatggatacggctacttttgaagtaattgctgcttaccccctgctggaaagccagcaatacgcctatgcttttcacacgacgcccaacaatggtattatcctgctcgaagcctctgctggtcaggagaaaaccatcctgatgcagttacagctgaacaacggcgtcatttccctcgctgaacttacccaatgcagtgatatgatcatgggcaactttgccccatccgggaaagagtttgttatggctccgcattatgatgggccgttagccatctactccttccctgaaattgccaaagtagcagagcaggatcaggaggctattttcgacggcagtaaagattttcccgctgctgaaccggataatatcaactacagtgtattttttgtagatgatcataacatcctggtggtttcgcagtttggacgattgctgttgctggacagaaaagatttacgatgtaaagcagaggtaatgccggagggtattgaatttacagcgtacaacctggatggcaatccgactaccaacccggattatatctttgattacagcagtaatattatcaatgtaatgattgtgcatgacatgctgttgatgacgaccggtgagggtgagttgcgcagttatgggctgcctgtctcataaaaaatagagtctcccggaaaaagataatcattccgacctcaggctctttaccggatttgcaatagccgctttaatagcctggaaactgacggtaaatacagtgatgaggatagccgccatcgccgccagtacgaatgccacggggctgattgtgatccggtattcgtatttagtcagccagttttgcaaataatgataagcaaccggggatgcgatcaggcagctgatcaacaccagcaggagaaaatcttttgaaagcagtaaccatacctggggaatagaagcaccgagcaccttgcgtattccaatttctttggttcgtttttctgctatgtaggaggccaggccaaaaaggccgacacaagagatcatgatagccagcgaagcaaagatgcctgcgagctttccaatcagcgattcaaaatcgaattttgccgcatagctttcatttacaaaacgatattgaaatggaatagttggattataacgattgaaaaccggagcaagttttgcgagcgctgcttgtgtattgacgtgaggtgataaacggtaggtcactacatttgaccagcctggctcgtaaacaaaaatggttggaaccgagcctgaaaatggcgacaacattaacgcatctttaactacgccgatgactgtagcccgttgttccactgtgtgccaggtaatgatctggttgattggatccctataccgcatacgcttaacagccgcttcattgagaacaacgctcagggaatccgcaccttgatttccggtgaaatttcgtccgtttaccattttcatacccagcgttttaaaataatccgcatcggatacaccgataactgccaggctcagcgtctcaccaggcaatctgcctgaccaatctgttacgctgttactggcccaaagctcagtaacgggactggacgatttagtgacgctgctaacaacgcccgtacccattatttcgtttttaaaggcctcataattacgcgtcaggtccccggtagcatcagtcatcaataaacggctggcatcataccctacaggcctgttcctcgcatgctggatctgctgataaataatgatcgtgctaatgatcagtataatagaacaggtaaactgcaccactaccaagacttttccgggaaggttgccgccttttcctgcctgcatggatccttttaaaacttttaccgggttaaaggaagacaggtaaaaagctggccggcttccggaaagcaggcctgtaaacaggacgtagcctgccatggccagccaaaacaagccattagcaaaaggaatgctgatggtggtatgggtaagattgttaaaagccgggagtaccaggacgactaaaagcagtgaaagcaaaaatgccaccagggttaaggtcatggattcggttaaaaattgtaaaatcaagtctttacggcgggagcctatggctttacggatgcccacttcgcgcgcccttttttctgaacgtgctatggagagattcgtgaaattgatacaggcgataaccaggatgaggattccgatgagcgcgaacatcttcacgtaatctatcaggccactagttgctactccattcctatactccgaaaataaatgccagtcctttaaaggttccaggaacagcgccgcttttgtctgtccaaaatacttaggactgtgcttaaccagtactccctttattttaggtgccagatctgcataagaaatattaggctgcaaggcaacaaaggtctggaaagaattattgttccagtcatcaagtgaatttttaaccccttcatcagtagctgaatagtaggcaaaaggcacaataaagctaaattgaaatgtagaattagctggcaggtccttgagtataccggaaacacgtaaatcatgcgaattatcaatgcgcaccatttttcccaccgggtcttcctggccaaataaggcaactgccgtagtttgtgacagcacaatggaatatggatcactcagcgctgtacctgcattaccctgtataaacggatattgaaaaattttcaggaagtcacttccggccattgcgccattaacgtttattcttttatcaccaacgctcagcggatgcggccccatccagtccgtttgtgcaacatacttaatctccggaaattcttctttcagtgcctgtgccaatggcaggttggtggaattggaagtattgatctcaccgttattatttgtattatatcttaccttgtagacctgttggcaaccaggtagaaagcgatcatacgaaacctgcacataaacccataagccgatgagcaaggccgcggccattccggaagccaatcccagaatattcaacgcactgtatactttattgcgtatgataccgcgccatgcagccctgaaataagtctttagcatttgagccgggtcgccaaaaaaatgccaggaattaagcaatatgataatcaataaattatagtagtgctttcggttcacctgttcgataatgaacaataaatcgttcacttgtagaacagttactattaaccagcagcaaacggccttccaaaaacgcttccgctaaaaactttctctaaaattatccgacataccgctacaggaactgaccgggtatgctcccgaataagtaacaaaaaaattagtatgaaaaagttgatcttattactttcactcgtttccttttttaccgggataaacgcgcaacaaaactattttaatcccaccgtaagggtgaaggactaccttgaacctgctatccctcatgccagccaggacaaagaattacgtaataagctgtcgcgccttaataagaaacccaatatccttatcttcctggtagatgatatggggtatggcgatatcggtgtttatggaggaggatatgctgtgggcgcccctacccccaatatggacagacttgcacatgaaggattacaattaacctccacttatgcccagccaacctgtaccccaagccgcgcggccctgatgacaggaaggatcccggcaaggtctggtctaacaagaccgacattaacaggtgaacatccaaaagtaaacccctgggcatccgaaaatacgaccgcgaaaatcctctctcaaaatggatataaaacttctatttccggtaaatggcatcttggtgaaaccaaaggaagcttgccaaatgaagtggggtacgacgaatggcttggattctctgctgtacaatcggaatatgcacagtttgtaaatgaatggatttatccggatctgattaataaaccggacagatttgaagccatgaaaaaactggttgaccaatccatactaaccggtaagaaaggtgaggataacaaggtagtacagcctatcgccaatatcgaagaactttccaaagttgatcagattttcgctgattacagcgaggacttcatcaaacgctccgtgaaagaaaataagcctttctatcttattcactccttttctaaagtgcataatgataattatgtttctaaaggctacaagggtaagagcccggcggcatttccctacaaagatgccgtggtggaagtggacgacattgtgggacgaattatgcaactgttaaaagaaatgaatatcgaagagaacacctttgtattcctgacttcagataacgggcctaatgaagatgtttggcctgatggaggctacacacctttcagaggaggcaaaggcactacctgggaagggggggtacgcgtgcctggtattgcatactggaaaaacatgatcaaatccggacgcatcagcgatggcttatttgatctctgtgatctctttaacacctcactgtcactcgccggcgtagcagataaaataccggccggcaattacatcgatggcgtggatcaggcatcattcttactctcggataccggccagtccaacagaaacgcagtttttatgtactcagaaaccaaatttatggccatcagatggcaggaatacaagctgcacatgaaagtatttaatacttctgctccaagaaaaaacctggatcaatcaactatcgagagtattggaatgagtccatgggtatataacctgtatgttgaccctaaggaacaactgagtagcggtcatcgctactttgaatggggaataccagggatgatggggcttatttcggcacatatggctacctatcaaaaatatccgatgaaagatatcgggttgaagaaacccggagccgattgacttgtcgaacttcaatacttacggagtattcataaaaagaacctgcgttatacgcaggttctttttatgtgcaaaccccaaacccattacttaccgccccggatcatatccaatgtatattgaatctccggatctttaccagcatggatatattgctgaaacgcttcaaaagtcagctccttatctggctgactcccccggccgttatcctgctttgccttcataaaatatacttcgctcatcggaacggttaacttacttttcgttttaggcagtatataggtattgaaccatgcggctgttgtagacgcttcgccgctaccggtttcggtgcctaccagcacaccacgtttgttattcttcaccagcgccgcaaagtaggtggccgcacttaccgtaccgccgctgatcagcacatatacgttccctttaaagttattcttatctggcggatagttggaaatggaaccttccgtcaggcgtgcattgccatagtaaaaccccgccgcgctgtcgtaatcgaaccgttgtttcaggaagttctccgtctcctttacttccgtttctgccatcttggttccgtaaccattcaacaggttttcgggatcatgcatctgtatgttctttgtgcggtaattgaatacattatcgaacggacgtaacgccacaaaggaatacaacagggcagacatgttcgggttaccacctccgttcgaccggatatctatgataacgttactgatattccgcttctttacttctgcgaaaaagtcgttcagctccttatacatcgcattttcctgcagcataaatgtaagaaccgtcaggatggcggtagattccttctcctggtattcctttgttacgtaggcacgcttcaggaaagtattaaagggcagctctcccaggctccggttatgataaccggttttggcgtctactgctttcagctgtatggtcgtggaatttttagcgccgtactctttgtataccacctcatagctggtggcttccggaaaaatgaggctgataaacaaactaagacttgttccggtgcgatcggcgcctgttctgataaagccatcactataagtggcgtagccaatttcgctcagcagctttgcggcaggcactttattaatactcagtatctctgcaccaaaaggaatggtttctcctttcgcattaacaatgatcctgtctttaaaagtggtagtcgccaggggaaagtgattcatgccatataatacattcaccacgcgttcctcatcataatccagtttcagatgcacatcattgaataactgtacgggagaataccgcaaaccgcttaatatcgatggatctttatccagcctgttcatcagggaatccattttacggttaaacgtaacagtgtccgtgaacttataaggattcggatgttgcttcttcaacagctcaacggcatatttaaaatcatctttcaaatcctgcctggtaaacccggtaaaaggttgtacctgggccataacagaggtggagagcagggacataagtatccctgaggcaaaaatttgcttcatgctatttgtaattttttaaatagttgatatgttcaggtgagcgtttctcccaggctacattttattgataagcgcaataattccttcgttttcgatgatcatcatgccttgccggtcttcggtgataccttcgtgtaaagtgtaagtgtacctgggcacattgccttccagcacagtaggcatgaaccggaactgcacattgggaaggtcttccagcgcttcccctacttcgatgatatgagtggatacgataaacaggcaattgttgtattcggagaaccctctcgtaacggccagagtaccatcaaaggcgtctttcacgttggtgcccttaaacaattcatcgaacatcagcagcaggtgttcgccggtggctgcggccagcgcagcatccttcacccttactacttctgcgtagaaatggctgtaccccatcgctatgttgtcggccacgttgatgctggagaagatgccttcccgtaccgaaaacaccatttcggaagcggccaccgggaaaccgatatgcgccatgtacataccgatgccaatagatttcatccaggtagacttacccgccatattggctcccgtaagaaacagtacattgctgccctccatcatttgtatatcgttgcccactgcttttgaaatacagggatgcctcagcccccgggcatggaacaggttttcggttttctccactgccgttgcataacaaaaatgccgctcccgcgatacattgctgactgcgatgtatacatctgtttccgcaatgaactgcagcacgtctttcatagcttcattgtgccggttgcgtagcaggaaatcgtactcggataccgtccccgtcgacattgacttgtagatgtcgctgtccaggattctgcgaatatccttttggtgcatgatggccagtaaaccttccacacggtcctgcaaaggactgttttcgagcttcagcaactccagcagtccgaaacacttcttcagtgttacgatcgtcgcctgcaactgcagcagcgtatttttgaaacgaccgtctttcgtgaggcccgccagtactttttgcagttgtatatccaccgctaccgcccattgcgattttcctgccgtagtatcgatatattcccgcatcagggcaacctggtcggcctcaaaaggaaatgcaacacccttctcttcaaaaaactcaaaaatcgctacccgccggttgatcgcgttggcatcattcagtggatggaaaaacatctcatccatcagcttctccccgatccgtgttctcactttattgaataaaaagtatacggacccctgacggaattttcccatgaggttcagctcccctatcgattggcgatctattttaaaactcataattgcttatttaatttttttccgcctttgtttccgtgcttaagaatgtccagtataccttcgttattaatgataatcattccatgcttatcattggtaacgccttcctcgagggtatacgtgtattcaggtacagtccctttcatcacggtgggcagaaaataaaatgcggcactttcttttttccgcaactcgtctgccgcttctataatatgggaggagatgataaacttactgtctttccggttggtaaacgcattacacacagccagggttccttccagggcatccttcacattcgtaccgcggaataattcgtcgaacaatacaaacagtgattttccttcactcagttcctgccctattttcttcacccgcaacacttctgcatagaagtggctggccccgatgcccaggttatcaggcaggttgatcgtagtatatacgccgtccatcacggaaaattccatgaaggccgcggccaccgggaagcccatatgcgcgatgtaaacggcggtactgaacgaacgcaggaaggtagacttcccggccatattggctcccgtaagaaaaaccaggttacgggaaggtcccatatgcagactgttagccaccgcattttttaaaagcggatggtatacaccatccacttttaaaatgctggtgcctttcgggtgcaccacggggaataccatgttatgcttcagggtaacctgcgccactgaaacatacacatcgatatgataaataaaatgcagcagttgcagcacctttcttttctccttactacggatcaacacatcaaaagccgtaacggcagcgaatgaaatcctggcattcggtttttcgttaaacaccggtataaaaaccgggtcattcaataccccgatagccgccagccgttcttcctccagctccttcacccccgccatttcgggcgactccaggtattttctgagtgcatggaaaagatcgatgatggaaataatcccattctgtacttccttctcgctgagcgacacttttgttccgccatccgggttatcgtcaaaagagatgtatttctcggcctggtccagcatagcgccatcaaaaggaaagctggccttcattttcacgaaagcagtaatgatgttgatccgcttgatgatcgcttccctgttgttcagtggcttcctgaacatcgcttccataatggtttgcccgccacgggtaaacgaatgattataaatatcgtaaataccttgcgtgtctgctttcgaaaacaaccgcagatcatccatcgtctgcatatctgtctgcaaatacataattatactttttatgaaacagttaaagtacccgctatttgcgttttcttcgtatcagtatgatgatacctgccaccaggatcagggaaggtataacatattgaagtatcgtcttcaatgtttgcgccggggcctttttgatcgtcagccatatatctgtaggcactttgaaattatggtaaaccgggtatttgttatcaaccgtatagctgtagaacgcattgccataatcccttccatcccctctcgccgcagacatcatgtccgcatcgctggaaataatgatcttctgcaatttgttgccaattttgcgggtaagctgcaggcccacaggataaggcgcttccctcctgtaatccccttccgcggtactgaataccggcgctgcggagtccactaccaacaagcctctttctacccaggtattttcattgttatgtaaagtggtaatctgttctaccttaaatccggtggtatcagaatagcttaatacactggcgccaacgatagcggtatagcaagctttgacgataccgtttctcaggtagaaaaacggctgctcatctgccatatccgaacctttcttagcaatcaatcctaaaaacttgtgcggcatatcctgcgggttcacctgtacaatggtgccttcatccgcatttacccccacatgattcagaatagggttcatgataaactgcttgcctggttcggaatagaacatagcatttcctccattgtcgatataccgtttaacgctatcgataatggcattatccaataatgatttcggatcggaaaccaccagtacatcgttgggcttaaacctgccggaacccaccgccgggatggtgtcgaaattcaatcccatattaatcatcgcgcccctggaagctttattgactgcatggttcccatattcccgttctccgaacttcagcggcgaacgctcatagtgcccggtaagaaatttaaacgtaggtgttgtatcattcactaaacgcagcaagctgccggaaacatgtttctcatacggaaaaacctccgggtcggggtacgttctcaggatcgtctttttccctttatactccacctccatcaataagcctttcgcttccgattccaggttgatgatcttcctgatttctgccggctttttatatatcgagagatcggttttatacatttccgcatacttctccgcgatttcatccagcgttttacccggatatgcctggaatattgaactgtctccctcgtttacatcgtaataatacacatatttaaactccatattgttataaaagcgtcggtacctggcccagaagttccacagatatgcattgcgcgcagtaggcaaaccactgccgaggttataccctaacaggttagtatacagcgttaccttcagtggcgatccatccagctgtttcaatacgccctgggtattttcatgcagtgtatttatcttgcctctcgtcacatcccaatagccgatcaacctgggcagggaggtaacaacgagtacaacaaccgttatcgcgaacgccaacaggtatctgcctgccgatacacgccacgacttcgactcagtaacggatttcgttttgatgatggtgaatatgataaaaagggaaataatgctaaagaagtagacaaggtcctttgtggtaatcaggccagacagaaagctctccactcttcccgagctggaaaggaaataggtgacatccctcacgtaatccgttccctggaacagcatacccagcatagtaaacatgatcagcaccacaaatgttccgatcccggcaacaatcggatacgaggttaaactggagatatacatacctaccgccacatacattgccgccagtaaaaagaacccgagcaccatggacataatatgcgggaattctgcattcttaatagaaaaggtcaatatgagcacctccgccaggaaaatcaggatcatcaggcatacaaaactgtatacacccaaaaacttacccaagacgatctggcgtgttttcaaaggcgacgaatgaagcaacttaatggttccggcagaatattcacggttaatcacacccatagtcaacagcggaatgaacaaaaagaagatcatcatcaccgtatcgagtcctttgccgatcaccacccgggttaacggcaaattgagaaaaccattgaaagcactcccctgcaactcaaggaaggtgtcctgctgtaacgcagtttccgccaggtttcccataatgatgcccccactggacatcaggaataaaatcaatataaaccatgcgatcggcgaaaagaaaaaatatcgtaattctgcccgcgctatattaaaaactactctcattagtgtaatgttgaagaagaatttgatgataattgtttgaatacattgtccataccggaagattcgatatgaatagaagtgagcctccagtttttctctgcactcttcctcacaattctttcagccagatcgtcgttgggctggaaatagatccggcatttgttatccggcagcaactctactttctgtacatcttccatcgccatcaattcttccggcggaggcatatggagcattctcaccatcatggtattgggctgaagaatattattgaaagcatcgagggtatcagaaaacaccacctgcccggattcgatcatgatgatctctttggcgagcaggttaatttcggacaatacatgcgacgacaacaataccgcacggtcctgcgcaatttccttgatcagtttccttgcttcaatgatctggttgggatcaagaccgttggtaggttcatcgaggattaccactttcggtttattgatgatggattgcgcgatgcccacccgctggcggtatccgcccgacaaattctttataagacgtgacctcatctgtgtaatggatgttttctccagtacttcatccacggcgcttttgataagacgcctgtccattaacctcagctgcgcggaatactccaggtactcctgcacggtaaaatccagatacaggggcgcctgctgcggtaaaaagccgatctgctttttatattcaataggatcatctttgatgttcaaaccattgatggaaacattcccttccgtttgcagcaaggtgccgcaaatgatattcatggtggtagacttgcctgctccgttcgaacccagcaatccgacaacaccggtatcattgatctcaaaatttatttcgcgtatggcccaggaactggcatacttatgcgataggttctccacctttaatataggctgcatataatgttacttatgattaaaaacttggattaaaaatgaccgatagtttttgccctggccgaaaaaacaccttctgaagtccatgttccggttaccagcatcgtacgtgccttaaacagccattgggtattcggcgtagtagtacccggggcaatattttcgctggacaaggtggtcagtgtgaagcctgttgcatgatccctcacttcaaaacggaagttgtttacggatacattagcaggaacctttataaaaccggacagctgttcataagcgagatcggtgaccatagtgcccggtaccggctccagctgtaccacatcgatcggcctgttatcgaaaagattaataatccggaggttcaccacactgtcattcaggctacgggaaggaagttgttccttcaccgttttttgttgcactttcgccggactaccatacacaaaatgcgtatagatcccgccaggctccagttgcagcgtggttttcagaaagggattattggactggagcgtatcgtagtttctgaataccgtaactggttggttcattttatcggtagcataatcaaaagagccgccgctgacaatatatgacagcctgttgtagtattttggctgtgaatttccaaaataggctaacagagaggaggtattgtcgttaacgccattcacaatcgtcaaagacgccggaaatatctcttcccgtaactccttcttacaggaagtaccggcaatcagcatccctccggctaacaggaccgctttgaaacattctttatagctgaattgaaacatcttgcttgatttatatagtgatcaactttttattagtagccggcattctgggagagatggttgtccaggagaatttcgtccggcggaacggggtatagcaactgatgctgactccacggctgtttgtaaaatatctccgaaagcacctgcgtggccttgttcgtccttttcaggtccagccagcgatgtccccactctgcaaacaactctatgcgcctttcctgcgcgatggcatccgttacctgctgatcggttaaagtataaggaagaccattcaatccggcgcgtaacctgatagcgttcaggtcatcgatcgcagcatttttattgcccgcactccgcaacatattcgcttccgccctgatcaggtacatttctgcaagccgcatcactacataatattcggacctgaaccctcccaattcgaagttggtggtattgatcttatacttggccggagaaaaaccggcaggtattgatgtaccgccggtgatagccgtcgtccatgccgctttcctgttgtcgcccgcttcgaaagcattcatcagcgccggcgtgagataccggcctgtcatggaaatcgcttctggcgtggcattgcgccgcgtcgctgaaatattggtctgcttcaactggaaaataacttcccggctggatatactgaacacgttgttcagactttccagtttaaacaagtctgtccggctgatcacgtcgttcgcctgctgccaggctttttcataatccctggtaaagagagatacccttgccagcattgccttaacataccatttattgatccggatgcgctccgtgttgttgccatcgtaattttcggaaagataccctgacgcctcttccaggtcgttgatgatttgttggtatacagcgccagggctggcagaagggagttttactgtattattataatcgatggataaagcgagggggattttttcgaacaggtttaccaggtagaaatatcccattgccctcactgccagcgcttcgcccagcacccgtttccggtagtcctgcgtaaactcatttgacgtagcagcttttacaccttctatcagcgcattggcattgaagattgccttataggccgtcttccatattttcgtggaatatccagggttccgcaatgtaatcctggcggccatctctacatagtactggtagtccccgctgagcgaaggctgatataattcatccgccgaatgcccggcagccagcgtaactcccccggcgctgtataaatcgctgcccagctgctcgtacgaattgacttcgagttctcctccgctgatcaggtaagaatacaaaccattgagcgcaatggatgcctgatcatcgctctggaaaacctggttggtagtaatcgaatttaccgggtcctttatatccagcaatttattgcaccccgttaccagcacgccggacaacagcataccggttgcatatatattgaaagcaaatcttttcatacgattgattttagaaacttaatctcaggttagcggcaattcttctgatctgcggtgtagtacccaattcaacatccgacatcctgtattgcgagaatttgaaaatctttgatgaattcacggagaccgttccctgcgtcatgcctactttctttaaccatgctgccggcagcatgtacgacaaactaagattgtccaggctgacataagcccctttggcatagtaggcatccgacccggaaaatccgccgctgttgaaagtggaatacttggtgtaaagcgctttgtcgcccggttgctgccagtgcctgtcctggacctccttatacatcaccatgttggccacattcccgtacccgagattattcaactgatctgcgaccagggaattttcgaagctgaattgtgcatccagcgacaacacccgcttgaaatctacccggaagcccatcccaccgaaatatttagggttcaggtcaatcacccggtaatgatcgtccagctccgtatcaggaaaattcgtggaagatattccaacaggtttcgccccatccccgttataatcctcaaactcaggtgttcctttcattgggttgatgccgatatagtgcgagtaggacttggcggttacagaagtccctatcctgtacatatccttgtaaggagaatcttccaacccttcgaaagctaccagcgtattattgttcttacttacctggaaacgtgcggtcaggccccaggtcttcgtgttcaaaatcgttccatccaacattagctccacccctctgttccggataacagcgggccagtttcccaccacagaagcaaaccctgtgaatgccggcgtggtaatgcttgtcagctgctttccgtccctgttgatgtagaagttaccttcaatgttcacggtgctgttgaaaaatcccaccctggcgcctacttcaaacttgctggcgctggaccagctgtatttctggttaacgggttgtatgagcgtataaatagtctgatcgtcataatccggcagtttgtccagaatgcccgttggaatgttcgaccagcgcgagaggtattgataatcgcccacattggcattccccatcacgccataggtagacctgattttggcaaacgagaaccaatccatgccggcatttttaaaccattcttcattagataaaacccatgacacccctgcagatccgaagttcccgaaacgggccccgtcaccgaagcgcgaagagccatccctcctgccgtttaaactaacgatgtacttattttcccagtcgaatgccaccgttgccagcaacgaagcaactttcagctgggcataattattcattgcctgcagcacctgggcattcgagtagcttttgatgaggttatcgttcgagaacatcatcgctatcgttgttatcacatcctgatcggcataactgtagtctgctgccagtgaagccgacaccctggcgccgccgaacagtttaacatagttgatacttggcctcaccagcaggctctttccggaaccattaccaaaaattgccatgctcatgggaaaatacatgggatctttcccggctttaggcatatagtagccggatttattggagaaaaattccccgctaaagcgaacacccgccgtcaggtccttaaatatttcgtaagtaaacccaacattggtctgacttttcagcgtttgattctctccccagtttttaatatccctgaatggataaatgctcccatactggttcctgtacggctcaaaattatattgcccgttctcatcataaatcccgggagcattgggcgccagcgagtaaaagtccaacgtagcggcagtttcattgttggaataggtactgttggaagaaagttccaccatcagcttgccgttcggactgcgatggttgaaagacaatcccactgttaaacgatcgttccctctcccctggttatacatctccgttgtggaggtatatcccacactcacgcggtaggtattctgcagcaatccaccttccacactcagctgtacatcattcgactgctcatttttgaagaagacacgttgccagtcggtataggctttgggatcccagatcgtgagatccggggcattatcccgggtagggagaactgcatcattcagcatcgcttcccttctcaccgccaggtactgttctgtgttcatcatatccatgtagcgctgcacgcccgaaaacactttggaatagcttacgttaaacctggtaggacctggctttccttttttggtagtgatgatgatcacgccgttggcgcccctggagccatacaacgcggtggcatccgcatctttcagtacatccacactttcaatgtccaggggattgatcatatacaaagggctttcagtagttgaatacccgccgctaaccggtgtgcctgcacccaatggattaacggataaagtagcaatcggtaatccatcaaccacatacagcggatctgtaaacatgttttcgttcagcacattccgtccgcgtagctctactttcctcgctcctgccgtgttggccgattgactgatccggaggccagggacgcggcctgcgatcgcgtccagcacatttacgacgggttgcctttcaatatcactggctttcaccgtggcgatattagcggtgccgattcttttattggtagtacccaaaacagtgatctgcacttcatccagtttgttttcagaaagcaccagctccgtgttatatgccctggcagcaaaaatgggttcagttattttaaatagatggtccacatagccgatatagctgatccgcatctggtcgcccaccttcatcggcacctggaccgacccattccctgcggtcagataattccgcttgtcggtaagattgctaatggtagcgctgaccaacggcgtgtaaccggaagaatagacatagaccgtgatcgattcctgtttcgccggcaccgtatcaacgggcggactggctacagccggcctggactccttctgggataccaggatgtttttgtcgatgatcttgtaggtcagtgactggttctcaaataccttgttgagaaaggctcccaggtcaattcccctggcagtgatggtgaccggttttgccactgataaggcagtagccttgtacaggaaaacataatcggtttgcgattctacagctgcaaaaactttttccagtgcaacgtttttaccattaaaattgatgctctgtgaaagccctctggcagatacctgcaacagggcagcggtaaggagaaagaatgttagcttcataactaacagagatttggttgagccacgtttccatccatagggaacccgtatgcaataagaaataattagcatagctttgcatcgtccgtccttttcataaagggcggaatgtttaagtgaataaataagcagtctttaacctgattgtgatgattacattacttgaacatctaccgggagtgtcgcaagcacttccggtttcgttttaagcaacctcttttattacttgctatcttacatacaaaatatttcccttcagttcgaaattcacatccatcgtttccagcacttctaatacattagacaaattggtattgcggtgcattttccctttgaagatgacattatccggcttcccaacgtattgtacatctatattgtaccatctttccagctggcgcattacactgtataaatccatgccgtcaaaattaaacaggccgtttttccatgcgatcacgttgcccgcatcaggcgtttccgttacggtcagcgtaactccctccgatgcatccggtttgcttaaaacccctgtctggccgggcacaagtacctggggaggcgtggtgtgcttatcgcctgccagcggcgttattttcacagcgccggtcaacagggttgtgcggattgttttttcgtcatcatacgtgttcacattaaatgaagtacccaatacttccagtttcatctgaccggtttccactacaaatggctgccagctcttgctggctacttcaaaataaatctccccgctgattttcacccttcgttcccccgctttgaaagcgaccgggtattgtatagaagactcggcattcagccatacttccgttccatcgggaagagtgacgtggtactggcggcccttaggtgtggtaatggtattatgggcctccccgtctgttgcggcggaagcgtcgtatttaagctcgttattgctcagcgagatttgcgttccgttctgtgtagcgatttttccttcgcccaggctgtccagtaccagttgcgtaccgtctgccagtgtcaggatagcgccgtttttacccggtggaatgtcgtgcagggcggatttccggccaaaaggatcagcattttgcgcaccaggtgtgaggaggaaataagtggatatgcctaaccccagcacaagtaccgcggccgcccatttccaggtgcgaaggaactgcatccggcgtatatttgattttgcaggtttgttagaaagaaaacgttccatcgcagcggtttcatcaaaccgggccatggcccgcacattttgctgttgtatgtcggtattgttcaattccatccataactgccggttctcgtcgctggcagcgatccacgcatccagctgatcctgctcgtcggccgtaagcgtgccctgttgcgaacgggaaataagcgcagctatgatgaatggatcgtttaaagaagaccccatgtctgatgtgtttatcttattacaacatggtgtcccgatcgtaccaaaagaaccaaaaaaaaattatgagtggagggaaaacgacaaaaataaggctactacagccggcgacacgcgcattctcagcagcttcatgcccctggttttctggtttttaaccgtttggagtgaaatagaaaggatttcggcgatctgttcgttcttcagtccgtcgatgtaactcatacggacgatcttcccgcattgttcgggcaggttgctgatctcgcggtaaattaccctgaacacctccatgcggatgatatccaggtcctcacctgtggtggccttttcctgctcgtgaaggaatttagcctggcgttccttgctatgctgtgcccctttcaggaaattaagggctgcattacgtgtagccttgtacaggaaatccttcagatgccggagatcctcgaacgcatatggcttctgccataatttttcaaaaacgtcctgcacaatatcttctgcatgcccaggctcaccgatgatagattcggcgtaatggcaaagggcattataatactctttaaagatataagaataatgcaatgtatcccccgaagtcaagccccgcaaaagctgatactcattattaaaagatttccgcgacaagtttgcaccccgattttagttgaaatgtaaaaatagtcaaaaaatcaagctataaaaatgcaattgaggagtgggattttttccggtcttaaccaaaaaactatatccacatcaacaaaaatcgtaaattgatcatgatagttctgttcctgtttgtaacttaaagttaactgatcatgaagtttaaactaattttatcgttttttcttttaaccacctgttttgtttcatttagtcaagatatgccatccggaaaatcccaaaatcacgacattgctgtcactgaaaaaggcttaataaagatatccgtcatgtatccatatgccgagggtaaaactttcaatatggagtattatgaaactaagcatatgcccatggtggctggtttcttaggggcaaacctggttaaatatactattgaaaaagggctttccagcggtattcctaaccaacctttaccctttatggctattggtacgttctatgtaaaaagcctgagtgaatatcaggcggctattgctccaaacagggatgcgattcgtgcagattttataaactacaccaatgtcgttcctgtcattttggtgagtgaggtggtaaaataagctaacatagcgatttatttccggcatgtatttataaggaaaaacaaataaatttgtggcaaaaaaaatggaaacccaaacaagccaggttactgtagaagaggaaaagcaattgatcctacttacacttaatgattatcttcaaggacgcccggtactggatatcgaaaggatccgggcggcgtttcaccctgatgccaacatcaggaccgtcatagatggaaagttggttcagtgggcgctgccacaatacctggacctcgttgcccaggcaacaatacaggaatgccaacccgaactcatttcatttacctgggacggagacactggctcagcccacgtgcaattgacttttgccacctttcggttcattgaccggtttaacctgataaagttagacgggaaatggctgattgtggataaggtttcctatcggcaggaattaccgtgagaagtcgttggcaagagcccctcctgcttctatagaaagaattataggttaaaaacaaaaacccgtttctactgagtagagacgggtttttctaaaatccagtgatcacagcactactttccgccaacactaagtgaaaactccactacttttgacggcaaacattggtggtcgtcacaggccataaattccacgcatcctttaatcttagtggccgccttcccctttagcattatctgctgaataaaattaactcttctctcatagtacttcaattctgttttaaaattatcgtcataagctttcttcaaagttccggattcctcaacttttcccacgaacgtaaccaacggattcttattaaaccggaatgaagtaggaatggggccttctccggtttcctgagcatagatatgccagcgtacatcaatattcgctgtcatttgcagttcgattcgcttttcatcgattttctttgcactaaatgtccattttacggggttctcgatttgcgcactggcaagatgggatagtaaaagcaggaaaactgcaaccaatagatgtctcatatatatgtttattgattcaacattcatttttagtactgtaattagacactactcactaataaagtatcaaaacagccgttcgtccctaccttcattaaaaaaaatttcaggtcattccataattaatctaaactaccatattggattaccacaaaaaatactactttcaaagtaatttcaaattgccatcaaaaaagattcaatggttaaggcatgtcgtacaaaaagtgctatacctgctgtatatgcagtcggagatgaaaataaaaaccagtgccgttaatcaatgaagaaagaaaccggtaaaaaaataatgtatgtgcttgcagcgatgctaccagtgctaaccggggtattgttatatctggtggtcagtgcgctgccgtttattgataaaagaatgcgactgccggcggtcgccactggttacctgctgattacagtcatactttgcatggtctctatttacaagcccgcatttaaattctccatgatctgggcaggtgtattaatattcgtgtcgctttttatgaccgaagacctgctctggccagccgccatactgtggcacaagcctttggcccttattattgctatcgaaatcatgttgctgctggttctcgttatcgctattatccgggttttccgtttaaccccggcgacacttcgcaaggagcttactaacaaccatgagccacttttttataagatttttgcactaccgatgctggcattcggagtgtttctctgttggagagcatgggataaatttgtttgcacgggtatctacctgttacccgggaaaaaagttcatatcacagcggtggttaccagcaatggtgctgtaagaggaaaatattactatcaccggtattggaatatgcaattcccgaacgggagcagggagaaattctgggtgtatgccgctgccaatacagaagatggttataaatgcagcaccaaccctgatcccggaccaggtacggtagtatacatcaccggccgggagcactttctcggttttgcctatgaaagtgttgatagcatcaaaagtgaaaagggggaacggatttgtccccattgagaaggaagattgaatcaacaaaacattcacccagacagacatctcacgacagatgataacaccgtacaatcatggcaaaattgaaaaaactatttcctatcttctgcatgctgatcgttgcactgtcgtgtgatgaatcaaaattgtctaaaggccctgtagccagcctctcgctcatccgcgcagaaatcaatatcacacaacgtttacatagcaagatcgaaaaccaggtggtggtcattttgtccgatgaagaagggaagaccattaaaaacgattctattaaaatctatgtgaacggggccgaagtaaagtacacggtcagacaaggactctattacacatccagcacttattatttaaaggatagtgctaatccaaaaaacaatcaattcaattttgaaatagcgcttccggatggtaaaaaatcattcctggccgaggtggatgcccttgacctggtgaatggtcaaaacatcagttatactgaaaaagggaatctcaataaggattatgaaataacctggaaagagctgaccggcgtaaattacctggccatcgagagaaccctgaaagtaaaaaaacaggaggagcccaatattactacctatgaggagcatatgccagatacgatcagcattcattctgaagggcgtcatgtggtatctaagtcaacttttgatagtccaacgcaccaggtcaacatactctcgttcagatttattgctcaaaaaattggaaaagtaagtcctgagctggccaaaggtagtagtatcagtattatagggagtattgaaagaagtgcgtcatttgagtagctgcgtaagcctaagagaatactatacattaaaggatacagctgagtatccctcatcatacgaagcttctataatggcagtagctattaccctttcgccagaatacggattcctgccatgtgaggtaagcatgttgtcgagaaaaatgatatctccctgctgataagaaaatactactttatttttttcatacgcttcccatatgctccgatattggttatagctgatatctgaaccatccccgaaaaaggtatcagagctgagataatcctccggcagataactattatgatcaagccctacttcctcgtaacgggcatatttattaaagaaaaggacatgattgaaccacatctcctctccggaaacaggatgacggtaaacagcaggtttcacccattctataacagcatcgttcctgcccgtaaaaacgcaggtaatgtcatttcttttacatatacctaaaacctcctctttgtcgtttgtctgaaacacttcctgccagggcattccaagtccctccgacaaattccggcgatactttacccctgtttcccggaacctggtcagcagctccggaggaatatcggacagtacaaggcgagaatctgccaggggtgtctccccgcccttttcagcaggcacaagacaacagaaaacgatcttccttccccatacgcgactgtatgaagtttcattatgcatgttaatgggcctctcctgcggatatgttgtagacaggtaaatatttttgatatcagatgaaagttcttttcttggggaagacctgaacagataaggaagcggatcagtgttaaaacaattcatgaattctttaaagtccgcagaggtcctgatattaaaacctctgaacagtatgcctccgtgttttaccagatcggattcaaaaactgtcttattggcgttcatccaacttacaagatccccattaggctgcgaagaactgattacaagaggcatgagcctggtttcatcattcagggatgatctgttcacaccggaaatgacggtgtctatggtcgttgccggacctgaaggtatgttgtccgaaaaattgctttccattattttactttaatgatgatcaaaagccaatagccccgccaaatattattgcctgcgtatcccatcttgcaaaattatttactccatatctatcttcatttcgtaattgaagtttctaaaaacacgtccttgcccaaacatcccattattcactgcaactgccttgcgttccatattattaatcataattgtacgattacgataatccatctcaaaatagcttatcatattgagtacatactcgtctgtcacatgatacaacaacacacttccggcattattatcgggtaatcgtatattgcagccatcaaatatagttgcgtcatatacaacatcgcgggcttcatcctgcaacttcagatcgccaccctctttttgccaacacccttctgtccaataattttcttccagatcaaacaggtactcgaattgctctccttttctcttattatttatcacagtaccatatttgaatctgtaatcctcaaataatatcaacacctttgtagtaaccgcattaacgggattggcttcacttacataagcagcttttatcctggaaaggagtttttgcctgtcatacttctcttcatgaccaatggcatcaaggtagaatttctccctgatcttccattcctctacgcctgcaagccggagacggtttctgaagtctacatcttcccatccgtaaacagacatcctttcatcgaacccacctacctgcaggaagtcggccttgttcacacatacaacgcccgctacaccgggatgtaaccccaaaggtctcataaacacctttttattcgtcctgaaaacctcatcgatataatatacaaacctgtttcctgtgaaattgtccgcatttatattacaaacaatatcaccggaggcaagtttgaacgccatatttttggcatggctatggttgaactccagaggatcaaatgttttatagtaaactaatgcgcccctttctatgtgatccgataaattgtttttcacccattgctccatatcatcgcccgagttatagtcaagcaacagtacttccagcccaggatacccggtattattagtaagattctttaacaaggtttcctttaaatggtataatctgttcatacagataatgcagaatgatattttccacggaccatattcagagagtgctctttgtttaacaagctcgttctccagcatattttagattttaatacagcagatcatactattctgaaatgctgctgtttactgccagtaaatgattagccggaccattgttctctggcggcagctcttttccaacaatataattgccgatcaccaggtgatctaatttacaggagtgaaagaagtcaagggcctctgccggcgtttccacaataggcattccccgtttgttcagcgatgtattcagcagcagtgaaataccggttaatgctttaaattcaaccaggagctgataaaactcaggtgaccaatctgctgttacggtttgtatcctggaagtattattgcgatgcacaatactttgtatctgctgatgccattccggctttacatcatctaccaggatcatataaggactctcccggtcggtcataaaatatgttcctacatcttcacgtaatacagcaggggcaaaaggacggaagtcttccctgaacttgatctccgtattaatataatcccgtacgccactattccggggatcagctaatatgctgcgtctgcccagggcgcgcggcccaaattcagcccctccctgaaaccagccaatcaccttccctgctgccagcagttgcgctgcctgtttgatataattatcactgtaaataacctgctctataatacttctgtggagcgttccgttaaaaagctctttgttgccaaatacttttcccaggtccactactttaccgaggaggccaatagacggaggatgagaaacctgtacattgcctgcatccagtaaaataccggaatataaaggatccataatcacagcacccaactgatgcgcatcaatgtttacaatgcaatccgcacggccttcaccatccacttctatataaaccccgctgtcactgaccttcagctggtatctgcagtaatcactgatgttgaattcaatcaggcttaccgctcccttcgccttcccggtggcagcatgctgttttatcaaacggaaaaagttgtcgatgcgcgtcctgatattatcccggtgatgcgtattggaataggagtagatggccttctttacttcttcctgcgaataggtttggccaaagcaggtagacctggacgcctttattttccgctcccttttcattacttccagccagccataataagcacacccgatagcaataccgttgtcaccggcggcaggctgaatatacaaatcaccaaccctggtatttttcaaaataaggttattggctaccgcattcaatgctacgccgccggcatagcataatttgtttcccactcccctgtttagccggtcttccaccaggtataaaattgccctttctatctcctcctgcattttatacgcaatattggcatagtaggtaaagtttcttttaaattcactatgcgtaccggccggtctgttcagtgacttcatcaaatcatagttaataaaaacccggccgccccgcagatgaaatatatcctcctttatcacaccaggattcccatatggggcaagtcccatcagctttcctacgtcactcatattcctgaagcaatagtgactgatagcctgataggcacttcccagagaatgcatggtataaggtgctaccggcgcatttttatagaaaaccccgtaaggggaaaaatcttttataacaggtgtaaggcacccgttctgataggtataaaagctatctttctcaaaatacaagtgggatacatctgcatgaattttttcattgtcaggaatgaatgctccttccagatccatgcattcgcagaaaggacttcccgatccatctatcaccagtacattaaaatctccctcaaacgggctggtaccaatggtactataggcatgcgccaggtgatgagaaatggtgacaacaggaacttttacatcatccgtaaaaatcctgggacctttgaaacttccattaccataatcgaagcttccgccataaagcgcattctgaacaaccaggtccacctcatttatggtgatgcctgccgcattcaaacagtattgaatggcagcggtgtcattcattccgtcatgcttcttccttgttatcctctccttttcaatagcaacacaaatctccccatcctttaacaggcaggctgacccatcgtgcgaaaggtttgtaccaagtacataaattggtttactcatacgatttgataagttattgactcttctattttgaaatagcagaggatgatttaatacagtccgtgatgatttccgccattttctcaggatgctgatcgataaagaagtgcccaccgggcaaaatactacccttaaaccccgccctggtaaatgccttccagttggtgatattcccggcattctcctcttcgttccccatgatagcccagataggtgtattaacaggtggaatcctgcttagctggcaattttcagataaatggaagtctgctctcaaaatgggtaatataaaatgcaggaagtccctgttatcgagcaactcagccggtatccctcccatcttcctgatcgcttctatcaaatccttatccgccagcaggcttttagtttgctgagcttttatccccgggccggcattgccgcttacaataagatgcccgggcgactcccctacctcttccagcatactgcatactttaaatgcaagagaagcgcccatactatgcccatatagcaggaaaccgggatactccacactgtccaataccttattaaaaagatcaagggcggcggcttcaaaatcaaccagaaggggttcagccatccgcctgcctctgccaggcaattctacgggaataatatctatatcctccagcaaagagaggatgggcttgaacgaataggagcttcctccggcaaaatgtataacaaataactgcgttcctgacatatgactgaaatacgatgaaataattaatgatcttttagtttaacatcatccaccaacctggaataacactgttccataaactgatttatgtattgaatagaaaagagttcctgcggactggcagcagtccgtaactgaacatgaacggcatcaacgaaccgcggccagaacaacccggcctccaaccccagggccctcgcttcctctgcataaatatggtacccattcacattgtcaatcagcccgtcaacatcccataccgctttgttatctactatccatacacaatccacggcttctccccattggtgccacgacaagcccggtattgcgttggttaactttcttccggcttgtggtcccaccatagcgatgcagctggcgagaaagtatgctccctccttttccagttctttcaacctgctgctgacttcctcctcagatcttgactgcctccagtattttgcctggacaatgggattacggataccttcgaaagggcgcattatcacgtttctgtcgaggcatttcccgatcaatgcttcaaccttcactttgaattccggaataagatgctccaggtatttatttgacatatttttttattagatttcggagattattacatactaaaaaaacagacccataggattcaatcaacacaccatgaaacaataccctctatccccaaggcaactggaagactggaaatataattataacctgaagcccggtgttccacccaccatcatgagaattgaaactgatctggccggcatcgatatcggcacactgaaatccgccttctcttcgttaatacaaaaacatgaaagtctgcgcaccaccttccgggtaattgaaaaccaggttatacagcaggtagaagaactttccggcaaatttgaactgatgtatgtggatgaatataccccttcctctctgcacacgctttctgaaatggttatcagggaaatgaaggacctggaaaacggacctctgatcaggggaatagcctgtaaaaaagaagccgggctttacaggctacacattatcgtccatcacatcatttcggaccagtggtctgtcaacatcatcaaaaatgacctgcagcaattgtacctcaaacatgccaacaaccaggtaacacattatgaaataccatccgaacagctcggagcctatatactttccaaaacagcgttctacaatgaacatcacgacaacgtaatcaggtactgggaatcaaaactgcaaacaaaaagctggcattcagactatgatatcattcaccggaacctgctgtcacctccgccagccgaacaggcttttccatggaagggactgacaggcacagaccttatcgcaaaccccacgggagaagcatatactgctgctatcagcgaacatctctacgaacggctacagcaacttcgctataatgaaaaatccagcatgctgaatatcctgcttactgccattaacctgctaggtgcaaagctgaccaataaccggcaaatactgatacaatgtcatcatgcctgccggcaggaagctattaccgcgaatatcataggcaacttactgggtaagctgcttatttttaccgacatccatcctgatgaaagcatttcagcgttgatgaaccaaacaagccaccgttaccaggaagcaacctctcatattatattcagttcagaaaaactaaatcctcttgagctcactacaggcaacttcctgttctttaactttctgccaaaggaaatgcagaataactccctgtataattataaagaacccgcctttagcagcaatgtctgggcagaatctcctttagtttgccaggcgtttgaatacaagaataccgtggtgctgaaatggtcttatcatcttcaatttttcaaccggacacttattgaactcctggcagcgcaatttgaagagatactggagatgatgaccggcgatagtcaaaccgatgttaaaagcttcttaaataacctggattaggtcaggggaatacctgccctgcgttgctccagttcaaaattgagatctcttgcggtacatgacataaacacttccgcttccgggatgttgtgcttttggaggaaatataacttgttgtgatgctcctgacgcagtttctccgttgtgtcactgaaatgcgggcaatgcagtgaagctgctttcctgttcagtacaaagcgaacattattcttgtagatacggtagcccagatcgatatcctccacgccccatcgttgatcataagcagtatcaaacacaccggtccgttgcaattcacccgatctcacggacaaatttccagtccaaaacatagcccatggcgcctgcagggccataatatcatcaccacaggcagcataaacggattccctgatatccaggtatttatctccggcaataaacctgttgatcgtatccctggggttcagcagatcaatctctttcaaaagggtttcaccgggatcatatacttcttcaatacccagcacatagccgatcacgaccacgttctggtctgcgtgcgacgccaggtgtgcgctgatacagccgggatccagtacaatgccggaatcaataaacaacaggatctctccttctgcattggcaattcccaggtttctggccgttgccaccctgtagccgtcatcctcctggaacaggtacttcaatggaaaattgccctcgtatttactgacagtctccctggtgttatccgaggacccgtcatccactacaatcacttcaaacagggatttatccagtgtctgggcattgatactcattaatgtgtagtctaacagatatgccctgttgtacgttggaataataatactgatgctgggcgcctttttgttcatgatgctatatttaacttgttttcaaagcgaaagacgggtgattgttcaatttttttccaccaagatccgtcaggcgtttcgaccagcgttgcacatccgaatgcctgactttcaggtaaagtttacgattcctcgcttcctgatcctgtacagacatctccaatgcctgatctatcgcattgtccatgctgttgtaagagtaaggatttgtaagtactgcttcatgaagctcaacagcagcgccaacaaactcagacaagacgagtacgcctttcccaccttttttcacggcgaggaactctttacacacgaggttagtgccatcccgcaacgagggtacccacataatatctgtagcggaaaaccaactcaccatttcctcaaaagaaagggctgcttccgaataaataaccggggtccagtctgcggcgccatgagcgctgataatccgggccacctgttgcctgatttttatctgaaactgatcataagcggttatgccggccgccggttgcaccgctacgagagacagcaccactttaccttttaattccggccgcctgtccagcaaacggctgtagcactccaacagtttatccattccttttacataatccattcttgaagccgcgaaaatcagtatcctgtctttgaactggctcctgatagctgatacgctgctttttatgcgccggtttttaagtagctggtcaatacgggcacaactcgtacccaccgggatagcatccagctgaacggttctgttatcaaacaacactttcgatgttactacaggctcgctcagggcgttaccggattgcgaaaaataaggtgttaccttcttacgttgcttaatcgaaatattggtcactgatttggctaccgctataaagttctcgatgtacctggggatagagaaaacgatatgattacaacataacaggctttctatgattttttccctccatgatataacattgaagatatccggtccggggaaaggcgtatggagaaaaaaagcaattttcacatccggcgccttctttcttataaagtatggagcaagccacaaattataatcgtggatccagacagtggtattgctatcggcttcttctaatgcagcctcagcaaaccttttgttgatcattacaaaattttcccagttgatcttctggcagtcaaagttttcgtggaatgaatgcagtatgggccaaaatccttccttcgatgttttatgatagaagcaattaagctcttcttttgtaataagcacccgtttaagcgtacaagccgccgctgcttccggcatatcaatcctttcataaaccggaacggacgggctatccacgaattcacttccggcaatccacatgccatcaggcactacagaaaaaaatcccttcagcaggggaataataccatttggtttaccagcatcccgcctgtaaatggtgctgccattaaccatcacctcttcatatggctgacgatgatacagcactattatttttctcttcataaatggtaaaaaatttgagtattacatgccatcagatcctgctgaatgaggaggctggtatttccacggaaatggagtggttaagcaccggaatttttaccccaaatcttgtttttcctttcttttgaaaaataacaccttctattccaatgaaaggtccttctgtgatcagcaccttattgccactttgcagttcctgctcaactgtcacctccggttcaatcattagttttttaatggtgtttatctccttttccgatacaacaacaggctttccatcaaaggccacgtaacgtgatacccccgtaatatccaacaacctgaaccttgcctgttcttccacatatacaaaaacgtaattcgggaaaagcggttcatcgacaatctttctcctgtcgctccattgcttgacaactttttttgtaggcagaaaacagtgaatacctatctttttggattgattgagaattcgcttctcatagtgtgggtatgtgtaaacgacataccaactgcatacagtttgctgaagtgctaattcgcgcatagggtgtattttaagctgtgtaaatgaatatgctggcaaagaataacgctaccggcaaattgagtcaatccccatttttgatgatggaatataggtgggttatcaaatatagcagatggattaactaacggtacttttacttactaatcgcgtttattcaataatggtcttttacgtggcaacaatttttagtacatacgtgatttttaactgtacttctttctcaacagcttgttctcaagcgattgcataatcagaaaacaggtcaatacaaatacagcaataaacagcataccgggcgtagcaatggaggccaatgggaccgtatccatacctatccaccctatcatgctcacagccagcaatacgccaataacggagagggaaactacaataacaagttcttcccggcctgtcttcaatttcttaccggatgcggctaatgcggcggtaacattccgggcaaaatccggtggaggatcagcttcaggcagttttttcagttcatcaaataataactggtacagttttacatctgcactgaatcggggatcattgcaaggcgcctgttcaccggccccctctcccttttcttccagcattctctggatactttcatcgtttgtattgctcatactatatccttttttaaactacccgttaatttatccttcaagagcttcctcgctctgaaaagataactctttatcgttcccaatggcattcctgttatctgcgtaatttcctcataagaaaattcgttcagatgatataatacgatcactgtccggtactgttccggcatctgatctattagctgattcagataagctgctacatcttttctatctaaaagttcttccgggttttcgctggcctgctcaatggtttctatttctgtgattttttgtctgtgttcccttcgttgttttctattatggttaacagcggtaacccaggcaatgcgggctatccaggttgacagtttcgactgaaatttaaagctacccagatgacggtacaccttgatgaatacttcctgacaaacatcttctacttcttccctgtttgttactattttacctgctataaaaaacacaagccgctgatactccttcaccagtatctcaaatgcatgtaaatcaccctttaagataacaggaatcagttctttttcatcaaccataatttctctggaattcggcgttggtgggtatgggtatcatcatatggatattattgattaaagtcttcattggatacatcatcattcttaattccacgcttattcttcctgatcgtttctctgagttttccgaaattataatttaagttaaaactaattgctctgaaatacaaccgtctggtaatattttgttcaaaatcatttccaaaagtgcttctgatgtcgttccggaatttaccaaaagggttgatgagcgcggctgacagggacagtttatcattcagcagggattttgttaagccaaatgaagatgtaacaacggaattagaagtcccctgaaaggttactttcggactgatcacatttacattactgcttacgcgccatcccttatcaaacttataccctgctgacccggcaatagtatacatgaaaccctgattatcaatattggctcctttggaaacactttttgtccatatataaacgaaattattattcagggttaagctcaatcgcttcgttgcaggatagctgatattcaggcttccgcttaatcccttgccgctgccggcgttttcaaatcttgtccgcactacatttgtttccggaataaaaaatgataccggtatcgccagtttattaaaataggcatagtccacacctgttacaatgaccactttaccggaataagtgtatcccagctgaacgccgttgagcaacgccgggctgagctccggattaccggtatgttccacattaggattagaacggtctataaaaggattgagctggttcacacccgggcgctttatccgctgcctgaatcccagcgtcatcatacttttcttacttaacttcttgccaatggaaattgcaggcatcacattaaagtaattctgcttaacatttgaggcgttggaaataaagtctgcatcaatagtagtttgttcaatccgcacccctcctttaaatgaccagccattaattccatactcatatgtgttgtaagcggccagtatattctgccggttgcggagtacgttgccgaggctggtatcctggttaaaatcacctgttaaatggtcaaatatacttgtttgaaaatccccctcgttctttctgaaaatagctttcactcctgactcgacagccactttacctatagtgaacacgtaatccacctgcactgtttgctctgaggcgctttgcctgttcgattgtttataatctgataacgggtagttaatggtatctaatactgatacatctgtctgctgcctcgagtcatatgtaaaataacgataagaaaatgtcagcaggtcttttttattccttttgaatccaagctgataattcagggaaatatcttttccattaccatgtgtttctccctccccggctatatcgtacccttgcagatagccatcacttgccgtcagcacggattgttgcttattattatccttatccttgttgccattgatattcagctgcaccgataccaggttaagactgtccgcttcataactgatttccgcaccaatataaccattgttgctattggatttctgtgttccgttctgaagcagatggtcttttttggcgccggtcgccgatctgtctatcgtagtttccgtttccggggaattataaatactggcggcgccggaagctgatatgccccatttcccacttttcagggaaagggagccgcccattccgggaccacccaccggggtacgcccgttgaggttgatggtgcctttgtatccatccgccgggcgtttgttggtgatgatattaatgattcctgcaaagccttcaccgtcatattttgaggaaggcgttgtaatcacttcaatcctttgaatagtggaggctggcatggatcgcagaatggctttcggatttctttctgccatactggaaggtttaccgttgatcagtattttgtaccctgcatctccattcagcaagatattatcatcggcatccagcgaaatatgcggtactttccgcatcatctccagcacattactgcccttactatccggatcggcctgcaagtcataagaaatgccgtcaatttgctgggtaatgatgggtttctccccggtcacctttacttctttcagggtacttgatgctcttacaatacttattttgccgagcccggcatgtccgtttgccgcagccaggtttacctggagcgtttgcttacggaaacccatagccattaccgttaatgaataactgagcggtttcaaatcagaaaatataaaagaaccgtcttccttcgtcacggcagccttaataataccggtatcgttttttaatccgatagtgatataagcaagaggtgatcctgtagcagaatcaaccacaacaccagtaattgttgaatcattcaggggagcctgaccaaatacgggtaacacaaacaagcaacatacagtaaagaacaaacaggttttccgggttaatttattcattgccttgagtttaaaactgatgatgaacaaattacctgtccttttgtacgatgaaataataaagcccaaaacccaatgcaatgaaaatagcctcgataccatatggcaccggggattcagcatcagcaaaagaaaggaacccgatcaccaccaggcccagccctccaaaaaagagcaccagcgcccatttaagtgcctcgcggcgggaagcagacagctgcccgagaagctctgctgcggcagcatctgttatacctgaatctataatatgtttttttagcttatagttgaaataagctactatcaccaccgcaattgttatgaaaagcgctaccggtaaaagaaataccaaagttttaggatgcatgtcagttcgtttataaaatgatcttcccccagtagacacccataaaacctaaaaagttgcagcgttcacaaatttcttttttgtggttaaaagtacaggggaatgctcccgtcagatttcctgtttaccagctcctgtaaacggattttcagccaatgcctccctgataagagcccgggcaaaagatgccgtggaatcgactataatcatctcatctatcgtactttctgtaaataccagggacaagtccgtgcaacccaggataatggcatccacctgttgctgtttgaaataactgagtgcctgcccgctccattgctttacctggtgtgttatattaccaggacaagctttgataccatcgcggggatcataaatcattctatggataatatcattctgaaaacgggcatccggtatcaccacttcaaaccccattgtttccaggacggttttataaataccggatctgtaagtaccattggtggtcatgagcccgatacgccgcacgcccagcaggttatccttaatatgccggcaggtttcaaaaggcatattaagcaaagcaatacgactgtcggggtgttgtatcctgccggcaataacatcaaatatggcgggcgaatacactgtattgcaagccaggcccaccacctccgcgccggcagcctccagtttccggatcatcttaacaatactgtacgcagggtttactgagatatatccgtccaggtattgggtcctgtcgccgatagcatcgggaaatgacatcaatataaccggcaaatgttcctggtcaagcgttgcgggcgtcatcagcagaatgctcttaaaaagggcaagccctgcctcaggccccattccgcctactataccaattaccttgtttcgtccgggcttcatatctgttgcaataaatattataaatgtaatttcccgatcagttctgcagccggcgcttcctgccggaaaccggcactgctgatacttacctgcctgatcagggcttcctttacctcttccacttcaattagcttcatacaatcattacccagcgggcatgaccggccccacaaataatgaaagcagggagaacacgccacgcctttataaatattaacattgttttcatgtccccagtgctggggactggtatctccaaacaataccacacctggcagattgaaagcattggttgcatgcgcaaagcttgattccacccctacaaatgaagtggcatatttaagctggcaaagtgtttcgcgaagcgataatttactcctccagtcaatggctccttccacggttggttcatttggcatcccaatctggataaacgtcagctccggtaactcttttaccaggcggttccattttttaatatcccataaatgattgacggagcatttggaataggtatgaataaaaacaacgtttttaaaatgcctgatccgctccctggcctgttgttcctccgctgctgtgaaaaacagctgtatcttacgatccccactcagcttcacatcgaaaacatcagccgcaacttctttataattcttttcgtatatccatgtagccggaacatggttcagatacatgtgataatactttctgtctttgatccactttttccttttaaaaagatatacaaacaagtgacggggatacctccacatggatgtaacatgcaattccctcaatgaatcaatatgaggattgttcagtaacacctgcttatgtcccggatgaaagtgctggtagtacacgatgatccttgagtggggattttcctctttgagggctttcaaagcgggggtacagagcatcagatcaccgataccaccccaggtaactacaataatttcttcacgcatttaaaatccagttcaattgttctaaagctgctgtacatacctttttattctggtccagtacccttgaccggaactggcatctgtcaagaaacggccgggagagttccttctctatctcgtggttaatgagcgccaaacgggttttcacttcatcagccctcgccgtgatttcttcatacgtcctggtcttcatagaaaataaaattgccggtgtattaatcatttgaagcggctccgctgctgctgccggaataaacggcctgcttctgaagctccttctcacatttcctcaaattaaaatccaatgtaaattcttctgaatggagggcttttgctttgagaaaatcctggtaggccgcgttaaaatctttctgtttcatatccagtgtgcccagcaggtagaaagccctggatgcatccgggtacaggatggtattttccgttagtaatttccgggctatggcagtatctattcctataaaaatatgtcccagctcattcaacgtattaacacccagcttttgttcgctcttcaatcttcctgcatctgctatcatcgcatcccctcctgcctgcttgtactttttcagcaatgtaatggcattactgggatactgctcatagtattgtttggcaaactccgatttgatatccagccggacagacatatccacgagtcgctgcgaaataagcttaccccggtcagagttggtcataaatattattccccgtttatgaacaacagaatagaaaacctggcatttataaccgggattgctacctccgtgtgcgatgatggtatcttttggcgtataaataacttcatatcctcctccgaagtaatggttgggaggaaaataatcatccaggctggtcgttttgtgcaggatatcgtttatgcgatcccgtgataaatatttaccattgaacatgcctatcagcaaatgggcgtagtccagggcagtagtgttaacgcccccggccggaaaaaccgacttatttttccatttgggaatttttctctccagcacatcatgtccatttgaataattacccggaacactatctttaaaactggtaaaggtcctttccagctccaaccgggataaaaccatccttttttcaatatcctggtaaggctctttgagtatggtttcaattacccgggcgaggtaatggaacccttccccggagtaaataaatttctcacccgggttggaaacaatatcgagggtatcgggattaaaatcggatttccagttctcaatgccggagcaatgacccagaatcatccggggagttatcaggcgataacgcgcatcatgtttaagccgctcgtactccaggtactggtacatgggcttatccaggtcaagcttatgctgatccaccaactggtataccatgaacaacatgaaatttttcgacagtgaacaggcctcaaaaagagtttcatcatctacagtttccggctgccccgactgcttgtaaccataggtatggtaaaaagcaaccttattattctcgataacggccagggatacaccgggaatccccacctcttccatcatgtggcttacttcagcattaaatgcattgatattcacctttcttccatcggttttaaagtatttcggtgattgacccaggctatactgaaaacaagcggtgagcaataacattgataccatcgttgcattcaaaaccttccgggcatatgccgctgaaaaatcaaatattctcataaaaaataataagatgaatgattacgtggagccgtttagaatttctctattttcatcgtgagagatgtaaaggaacgttcgtcattataaatttccagcttgccatgttccattttcaggatcttatccgccacatcgaaataatggtcatcatgagtaatggctataacgatctttcccgcttccctcatttgtggcagcagtgttctgtagaaaaaattacggtatgcagggtcctgatccgctgcccactcatcaaagaggtagatgggggcatcttccaggtagcattgcaacagcgccaatcgctttcgctgcccgccagacaggttaatagtggtgtatttgttatccaggataccgacgatattttcgaggttcagcacccgcaggtatttttctatctcatttttcttactgacagtgtcaatattgtacagttttccaaagatgtacaacggggaaaatactgcagaatagtattcgctcaggtcgcagcttttaagctctttttcattaatagtgatcgttccttcagagggctcatataaacccgtgagcagtttagccaacgtggatttaccactgccgtttcccccaatgataaagagtatttccccgctcttcacttcaagatcaatggctcctacctggaacccctcctggctgttataggcaaacttcaaaccctgtgcctttatactcatcacttcgggctccaaaggagggcaaagttcatgtaagtcgagattggagggtatttcggacaaaaattgctggatccggttccaggcaatcctcaactgtaatatagaaggtgctgccgtcagtaacctgtttaccggtccgataagatataaaagtacgatcacaaaattcatgatggtacctgacttagtatctgtaaacaaacgcgggataataaatgccaccgtacccagtaaaagtatcagcatggactctcccagcaaagaggcatagaggaaacgcatggctgcgaatgatattttctggcgatagctatccgctgcatctgtaatgtccttatagtactccagcttctttttccgttgcagggagatctctttaaacccgtcgatcatgccattggtcagtcgcataaaaatattcctggtatcacgggcttcttcataatatttattggtgcttttgctgacaaaataatagagcgtcgccaacgcaataatgagtatcaatgtcatgagtgttgcccagaaaaccatggtagccaggtacaggaaggcgaccacagcagtgaatacactggtcaccagcgtaatggccatattggaagaattgccgatggtgtccacatcatcatttacagaggtgtatacccttcccctgtccatgttttcaaatttctggtaagaggtagaaaatattttctcaaagactttaatccgcagttcaaatccgatacccttggagagctcaattaaactggattgcacaaacttcctcccgaacatatgcacagcaacagttaacaggaaataaaacaccaggtactgtaattctactttactgttaatggcagatacaatcaagagtatcaataccatgttagacattccggacacgatgcttaccagcaatattttgggaatcacccgtttgtacttattctgttgcgggaacagcaatgtgataaagtatgccaggtaggttgtcaccagcgataataacgcaagacctaccattgccacaaaactaaccgggctccagacaataacgggctgccagctcatccctaacagggcgtgcggtaacatataaaatccatataaaaatggcaatgccagcacaattgaaagtcctatccgtcccacagtgttgatgttccctccctccaggcgccttgtgccggtgaatatctggtatatcaccattcccgtgaagcccagcagcaccagcaggtagatacacagtgccgcacatacaatgctataagctttatcattaccatctgcaaccgtaaattccctgtctcttatttcttttgacaccaggtccagcagtgaggcgccaataatacgcgtagcgccgctgtttgaattggccatcactactacaccggttctttccccaggatcaaatgcagcgtaagaagtatagttagggttcagtcccccgtgataaacagccccatcccccatcaatgaaacctgccagcccattccataggaagacatatcatgtatgggcacagtcacgtccccttcatgcgtttttgctatcagcggataaagatttgaaggttgcagccccatttgcagcttcagccacttcgccatatcccgtatatcggatatgatgtatcccgccgcattatttcccctatacacaggtgcatcatatctccggggtttaaagaagccaatcttataaccggcagacataaaggtgctgtctttcggcgcaccaatagtagtttgggtaagaccgagggaatccaatacatttttctgcagataatcctcaaaggaacctccgctgcgcagcgcaataatgtaagccagtatatcatagttcactgtggcgtactcgaagtacagacccggcttattcgccagtttgacgccggaaagattccgtatggtcctttccagggcgttgctgctatcaccttccggaataagtgaaattgttttccagggtaatccactcgtatgatgcaataaatgcctgatttttatttgcgccggcctcccgttgtaactcacctcaaaccagggcaggtagtccctgacattcgcatccaggtcgagcaatccggcctgttgcagcttaagtgccgccaatgcagtgaaagccttgctgcatgaacctatctggaataatgtggcgggggtgaccggtgtttttttatccaaatcagcaaacccgtagttcctgaaaacggttgtattccccgagataatagcaacactgagtccaggaatgctgccgtctttcatcagcttactcacaatggagtctaccgcatgtaatggaatagtgtcagccccggggccggcaaaacaaaggtggccggagtataccagtaaaaaaacaaaaaccggtataggtcttaaggcagtcacgataaaagatgcgatgaatttgctcattctgctactttgtgcggtgaggtttggctaactttttcagcaatctgtttcagggtacagttaaaatatatactgaaagggagatccacattaaattgtttcttcattctttcgttattggtcaccagtaacaacgagtgtccgcccaaaccaaaaaatgtatcatttagtgtcacctgttccagtcccatcaattccttccatatcagtgcaatctgtttttccacagctgtttgtggctgagcggcttcgtctatcacaatggccgatctttccagcaatgcaggaatggcatcccggtccactgttccagccgctgtcaatggcaggtgtccaaattttatgacgtcggtaggcatcagatgcctgggtagctggcttctcaaatactttttaatctttccaacagtgaccgacttatcaggcagttccaccaatgccagcagccgcttgccaggttgctgattcccgggaataatgactacagtattggttacctctccatgccgcatgatcacagcttcaatttctgataagtctgcccggtgcccgctcagcatcagcggcccggcttcccttgcggaaaattcaattcctttctccgctaagtatcttgcctgccagggagttttgattacacttacttccagttccggaagtggaaaatatagctggtggcacagttcttcttccgtcagataatcactcgccaggccggtaccgcctatacacaaactgccatataagccatctgcctgtaatttgttgttcctgtcaacggtgtataaagcagctcccggtaaagcctggtatagtatcctcgcatttgtggtgccaggtgcaggaagcgtacgtccgcaggcaaaaattgcatactccggtactccaaacatgtcttccagcaggatgcccgtattcagctggctgaatttgcggacaggatctgcccacgcgcccataccggtgagaaagatatgctgaagggatttaattttctcccgtccccggcgtgttagcacgtcagtaaacacattgaataccggcgcttcaaaatgtatgtgtgtgatgccataaacctctatccagcttatgatcttatctatttcgctttcgttttccggagggagaatggacaagcatcctcctgataaacaccaattgaatatctcctgcagggaagattgcagactggtattcgtccttaataagtagccgcctgtttcctgtacagggtatgtatcctgcattcctgcgagggcgctgaagagtgcctggtgactgaacatgaatccaacaggatttgataaagattccaggctatacatcacgtatgccagatcatcggcggttacaccggatgccggtggaagttccctgcattccaatatggaggtccactcctgctgtatgttaaggacctttacatttatagctgaaacatcgaacgtggtgttccccgttattaaaaccccaacacccgccttgctgataagcgtaccggaaataccgggaggataagcgggatccaatggaacaaaggctgcaccggttttgagaatgcctaatatagtgggaaccaggtattcatcccgctccatcattacaccaaccagcatcgatttcccgagacctgtattttctttaaggtgatatgcgatctgactggagatgcggtcaacatccgcataactccaggaaacatccttgtatcttatagcggttttttcctgaaaacggctaacggatttttcgaaccgggagagaatcgtttctgttggcacactattcccatttccggggaaacgacccaacagcgctttccgttcgtcttcgctgactacatcaatatcggcaattttaatgtcaggatctgctaccaccgctgctactatttttctgaagtaagcggcaaatttcaagatagtttccggtttgaacaggctatcctggtaaccaatagccagtcttatttcaccattattttcaaacgcagttaaagacatatcaaattcagctacaagatggctggctttgtaggaggatatttttaaatcaggaatgacaaacctggtttcttcaaaattctgaaatacgaacatgacatcatacaatgcgctgtgcgctcttgcccgcctgatctttaatctgtctaataaccggtgatattcataggattgattctccaggaaagcgaatgtcctttccttcacctcattcatgaactgccggaagcttagttgttctgccggaaaatttctgaagggcagtattttaacaaacatgcccaacatatgctgcaggtcactatgatcccttcccgatgcggggataccgatcatgatatcttcctggttagtaattttttcaagcaaaatattgtaaacggaaagcagtacaatgaacaaagtagccccttctttatcggcaattgccttgagatgaccggtatgttcctcttcaattctgaagttgacgtttcctgcatgattgttcttttgttccggccgttcaaagtcaaccggcaaatctaattgcggcatgtccctggaaagctcctggtaccagaaatcattctgcttgtccatttcggcccttctctcctctgtatccagccattccacataatccttatactgtaaggttaacggcgcgagtgtgccattattaaacaatgtcttgaattccctgataaatattccccaggacgtaccatccattaccaggtgatgggtatccactaccagtacatgcttttccggttgcacttcaattaatgctactcttaacaacggtgcgcgggaaaggtcgaaacgtgcgatgacctgctgcaccagctgtttaacatcttcctctgctgccacataatgtgttatggtaagcgcggcactatctgcaatctgctgcaccacctcttcccctatcacctggaaagaagtacggaatgcctcatgccgggctaccagttgctccattacctgtttcaacttgtctttatccaggtttccttccatcaccactaccctgggcatgttgtaagcgagggtctgtttgtcgtattctgagaaatagtatatcgctttttgtgccggcgagagactataataaggcttgggggttgctttgggcacacgggatacctgcattgcccccacctgccggatatactccgccaggctggcaatcacgcgtctttcaaaaatttctttgagtggcacctctgttcccagctcgctcaatattttgttcaccagtacagttgccctcagcgaatgtcctcccaggtcgaagaagctggaatttacgctgatgacatctttatccagcttcaatatatcagcccatatttccaccagtttcgtttctactattccggatggtggtatatactcatccgtagcggatacatgaggctccggaagcgctgccctgtccagttttccgtttgaggttagcgggaagtgatccaggtaaacaaagtaagaggggaccatgtagtccggtattttccctaacaggtaagtacgcagctctgataccctgatctcctgatcagcagtataataggccaccaggtatttgtcgtcttccttttcacgggcttccaccaccacttcgccaatacggctgttacctgataaggcatgcgctatttcccccagctctatgcggaaaccccgtaactgtacctggtggtctttcctgccaaggtattcaatttcacctccgggcagcaaccggccaaggtcgccggtgcggtaaagccgccctcccattttatacggatcctgtacaaactttgcagatgttaaggcttcgttgcccaggtaacccctcgaaacgccggatccacctacgtataactctccggtgataccagccggaaccagccgctgatgctcgtccagcaggtaaactgataaagtagggataggtttgccgatgttgctgatattactgccgatctctttttctgtgatctctttgtaggtaacatgcaccgtcgtttccgtaatcccgtacatattaatcagcttaacagcaggatacagctcccgccacgactgcaatttcccagggctcagtgcttctcccccgaaaataacatagcgtaaagacagacccattacagacaattgtaaaagattataaaaagcactgggcgtctgattcagcaccgttactccttcttcccgcaataatttaagatacaaacccgtatcacgcgctgtcatcttcggaacgataatcaccttacccccggttaacaatgccccaaaaatctcccatacactgaaatcaaagcagtggctatggaacatcgtccaaacatctgccggaccaaaggtaaactggaaatcatcgttgcagagcaaccgcactacattacgatgctctaccatcacgcctttgggatttcctgttgttcccgaggtataaataacgtaacataagttcgatggtaacggcttgtcaggcaaaacagcgctgaactgctccctgtcttctattaacaccaccgctatacctggctttaccaggtctgcaaactcctttgttgtcagcaccaaccgggtctgactattatccagcaggtaattcctcctttcttccggataggtaatatcaaccggcaaataggcgccaccggctttcagaatacccagcatgcctaccaccatttcaatagaacggtccatcaaaagacctactaccgcatcccgtttcactcctcgggccgtcagctgcgcggccacctgcccggcctgctcatccagctgtgcataggtaagagcggcgccttcatattgtacggctgtattccccggccactttgttacctgttcatcaaacaggtcgagtatcgttttatcttcaggatagtggctgctggtatagtccaggctatccagcaatccctgcttttctgcatcatccaggatatctatctcccataattgcagcgaaggttgcagaagcaaactatccaacaacctggagaagcgttgcatcattaacgcaacagaagcctggtcgaagtattccgagttatacagcatcttaccttcaacctcatcttccgattgaagcagcaagagactgaggtcatacttaccgtatccatagttgctctcgtataaatcaatatgcagatcgtcaatccggggaatttcgtaagatttattttcatactggaacagcacgtcaaacaatgctgttctgctcatatctttttcaggagcgagataacttaccagcttatcaaaagggatatcgctatgcgaaagatccgcattaaactgattgttaagccttgtcaggtattcctggaaactatctgaagggaatatctggctacgtactggcagcagattggccaacggcccagccacgtcctgtaatgcgccattgttcctgttatctgtactggtgccgataacaatttcttcgtgctgaacatatttatagagtaagattttaaaagccgccattaagatcagccggggtgaaataagccgttgctctgcataacgcagcacctgggaagaaatgtgccaggataaactaacatcaattgccgcacctttataaatatgaacggcagaccgtggacgatctgttggtaactccaatgctttaagtcttgttcccaaccgttgtttccagtaagggaaaagataaaaatacaatttagataagggtccccgctgccattctgaaaactgtgcataacgcagtctctctgtttcttccaggaaaagttccccctttaaccttctgcggtagttctctaaaatatcccgcgctatctgtaaggtagtatgcctgtccaccaccaggtgatgaaaaatgagcagcagcttacagctatctgtgtctgcttcaaacagcacggcccttaccggcggtttggcaggatcaaaaggcttgtctctctccgacataattgcagcttccagggaactgtctttgtgccggtgggtccttttttccagctgtataccggcatcgtttacaggttgctggaagatgatgtctttcacctcaacaaaacaggtacggagtgcggaataatgtctgattacgctattgatactttcttccagccattcaacattcaacgttcctttcaggtcaatctccaaagggatattgtgataaacagggcttccattgtacaggtagtccttctcgaatttatcaataaaccataatctttcctggtgataagaggtgcgtaccagaaccgactctgcctgggaagtatgattgccggacaccgtcaattcatcgaatacctgcagccgctcctgttcagtgagcagcgggatgttttgcagggaattcctgctgttctgtgtaatcctggaaagcaggctcaaaaaaactgccgtgatattctgaacaaagttgtaagtgaacctgctatgatgataccagacatccagcttctggtcctcttctgcatgaaaagaaaagtaaagatccagtgagcagccatcaacatcgattggtaaagcaatccctttcatacccaaacctacacctgatatgcgtttgatagccggactacccgccaggattctttccagcggatacctggcgtgccggaaatcactgaataaattttccttaacagcgttgaccagcgtgctaaaatctgtgtcgggagcaatgtcaatacctacgggtatgatgccttttcctgcatcctgtttctcttcttcggaataagtatgggtgaacagcaatactttgctggttgatgaatacttttgtatcagtaccgacagcgcagacaacagcacgatatgcttcgctttttctgacgaggcaataccgttcaggttcccgctgacacgccggggtatttccactgtataaaccccataggtattccccgaaggcagctgctgatcgtcggtagcgccatcgaagtagttttcagccctgaagttctttaatcgctgcttccagtaattcctggcagatatatttttgttggactctaaagctttaatatttagcatataattttcagacatggccagatacattttagggtaaaggacactgcagcgaggataaactgcggcaaaaagagaggaagtgccgggttaaaaattgaaggagatatcatcctccatcagatctattgcctgatccgagctttgtatgatactggcaagatcttcatccagcctgcccaccacgttctccagcaatgctttgaactgttgggccagcaatattatatcgggtcttgtaaaatagtcggaagaatattcgaaacggaaagtaaatgactgatcgctgtcgtatacatacagtgtcaacggatatttggagctgttgttttcaaacggatatataataaacccgtcttgctgccggtcctttctttcctcgaagttctggaaaacgaaagccacatcaaaaaggcttttaacaggattggtcctgttattattcagctctcttacaatatctcccaggtcatatatctgcctgctgttggcttgcagcatataattatgtaattcagcaactgcatctttaaacggggtatacggatttatctggaagcggaccggcaacatcttcacgaacatgcccaccacattttctgtttcctcctgcatcctgccggaagcagccgttcccacaacgatgtcttcctgcccggaaagctgggatagaaacaaaaaatatacagtgaaaaagcctgaaaatgcggttacatgttgctctttcagaaaatcagtaaaaggctttaaaagatgattgtcaattttgagcgtaacattccctccgtgatgagataccccatcgatgatttcttttgttacaggaagcgtaagcctcggtacaccgtcttcaaatgtcttcagccaaaattccctgtgcgagaggtattcttccgtaagccggaatttatgctcccactcagaatagtccttatactgtatttccagttcgggcaggtgcttaccgtaataactgttcaaaaagtcgtgatgaagaattttctttgagatgccgtcacagatgatgtgatgacaatctattaccagtattttccggccgccttcctggtgaatgagtgtgcaacggaaaagaggggctttatccagttcaaatggatgtataagtttagaaatagtattatggaggtcgggagcagatgtggtaatatgctccagggagaaatctactttatcatggagatgctgatagagttccccatccctgatatggaattcggttctcaggccttcatgtcttttcacaagtacgtgcagcgcctgttcaattctgtcctggtcgaatgattgtgaaacatcccaggccataggaagattataggatgtcacttttctatccagctgataactggcataaacacgccgctgcgcggcagaggcatgataggccggctttatatctgctttgggtataacaaatacatcatccttcatcagtgatccgataagggttgcctgcttctttaccgtaagattttcaaacaactcacttaaagaaacccggacaccaaactctttgaagagcctggatgacaatctcattatacttaatgaattccccccaatgcggtaaaaattttccttaacagatatcgacttatctgctaaaatatctttccatatctccagtattttttcttccagttcattctccgggacggaaatttcccgggctactattttactttgcagcgcctggtagtctacctttccgttgcgtagcaacggaagctcacttatttctacaatggatgcaggcagcatggatgcgggaatcagttcctgcaaatgtttcatggcagcgtcagagagctgttgtgcctcttcctgaaaattcttcctggtgatataggcaaccagtgcatcgtcaatattttctcctgcatgctttgtcactactgcctcctttataaaggggcttgtcagaagcatatactcaatttcatccagttcaatcctgattcctcttattttcacctggcggtcttcccggccaatcaggtctacatttccatcaggcatccaccgtgccctgtctcctgttttataaactgctgtttcgtctccggcagcagatctgaaagtcaggaatttctgtgcagtcagctccggattattcaggtatccttttgtgagataagcagaagcaatgtacagatcgcccactatgagcggatcgcaggattccaggttctcatccaggatcaacagggctgcaccatccatagcagtacccactgaaatccttgcagcgtttacatcttccggcgtaatccggtagcaggattttatcatggtggcttctgttggaccgtacagattcaccagttggatgcgggcgccaaacacctcataccatccccgcagttccaatgggttaattctttctcccgacagcaaacaatatttcaggtgctggaaaagatccggtgataatgccgctgaactgattatcctgaacaaactgggtacacaatgaatatactgtataccagcatcatttacccaggcaaccatttgttcgggcaatgaaatgtcctgtttaggaggcggaatgcagatagtaccacccgttagcagcggcgcaagaatatcccggagatatgcatcgaagtagggactgatgaattgactgaacctgctgcctgcggtaacctggaacgcgcctgtttcccattgcaaaaattgtatcaggctgctattcctgccaacaatgcctttaggtatcccggaagagccggaggtaaagtatacatatatactgtcattttcctgaaaagccggatagttcaatggctgctcaatgttgtccgcagtggattccagcagctcctctgcaaggataacccgggcggaacaataattgccggacgtggcagcgatgttgtctgtggtggaggtgatcagaaaagcaggttgcagctcatccaggacggcctgcattcttttctggggaagcgatgcgtcgataggaacatacacgcatctggcattgaatatgccaatcatggcataaatattcagcagcctgttgtcggttattaccgcaacgatggtgtcagccgggcatgcctgctgtataaaaaaaccggagattttatcagagatggataacaacctggagtatgatattttctcctcgtctacttcaatcgcaattttgcctgcatgggcacgcagacttttgtttaattccgcttgtagaatcatgataaaattattatgggaaaacagatttacaaactttcagcaacacagtatgttgcgtctgtaaagagaagtgtgtgcgacagcttcaggcaggttggcctggcatagtcccgggttaaaaaaagtaataaggcttcagttgaatattcaggcaaatatagcttcgctaaaggttgtcacaagttacagttaacaacaaaacaaaaatgagggcttcatgaaaattatttgcctatcttctcacaatataattatttacttcaggttttcgaaaatattttaatgcttttctaatttttttatattcgcttcctgctcagcatgtttcagtaatagcactgcgatatccctgcgcccattcttctgcgcacattcaacaggggactctcctttacggttcacagacgccaggctggcgccgttacgaagcagggcatcaacgaaattcacatgccctttatctactgcgcgcatcaacaatgattcgccctcagcatcaggttgatctatatccacccctttctgcaggaagcgttgcagaaaagatgacaactccggaacactaaacatatcaatgccctttccaataggaatgtcaaaccggtgccaccagaaattaacgctgacggacatatcaagcgacaacacattgtgccaccagcctgtgggtatataaataatgtcacccggctcaacaatgcaatgataaggctgcgcctgtaaaaaaagcggaaattgttctacatctgcatcgtgcagttccacttcactcatatgccatttacccggcaactgactcggatacaataacggggtatcttccggagaaaataacaccatgtcttttcttccgcatacctggtaaaagaaattatgactgttatcatagtgcagtcctgaatcgcaaccggccccgcccatccataaatttaccttatccaggatgtccccgtcccggatgaatgcaggtatttcaagatcatccatcaacattgggaagaatcccggtattgataactgcgccaggtaataagaggttcccttgctggctggcaaggtgaataaatcggatacttcatcgaaagggccgccgatccacttaacttccctgatagcatagttataactacccttctccgtataggccacccgcaccgtggttgatccgatcttttccttcagataatcaaccgaccatttactgaagcaggtggtaccttccaggccgcctttgattactaccggcttcctgttatagtagaatgtattaaaatctgcgtcagataaagcgctgacggtgtcgatgtttcctgcgatattcatagcattatatattttgatggtgatgaacaggcgattccatagtccacttaaagttagactgacactaaaaatataaatcatgcaaaatgccaaatgagatgacggtcattaacaaatcatcttcaaatggggcattgatataaaaacctggttgtttgtaaatatcaacaagccgctgcacttctgccggatcaaaaacgccttgtctcttaattgtttcaaaagacaacaattcattgatatacgcgatattccgttgtatcaggtagggacttccgggcgccacaaaaccaaacttctcccggtctaccaccttttgcggaacaaaccgttccgccattttcttcagtatatatttttctgtgtaatcctttaatttcaattgagcgggtatcctggtagaaaactccaccaggtctttgtccaggaacggatatcttacctccactgaattcgccagcgccatcctgtctccatgatctgagatcaggtgatccaccagccgcagtttataatctatgtaggcccttttatgcagcacatccctgttcctgatccggtctgtattcacaacaggatgctgaaggcagtcaatgtcgtcaaaaatggccctgagttcttcggaatataattgtttctttaccttgttaaactggagaaaatcacgctcgtaaaaaaaactgctgtcattccagacatgatgccgcagacgctcttcagccatagtagccgggcttccgcctccgttctcatgcctcattttatcaaaacggtaacccacataaccggcaaacaattcatccgaaccctcaccggataatatgaccttgacacctgccccacccgcagcctcagataaggaaagcgaagctgtattataggtttcctttacaggacattcacaatgatacaccgcatgtttcaggcgcaggcttatgtcatcataaaaaaaagtcttctggctcagccgggcattggcacgatccgctaccaaccgctggtacattgactctgacaaaccggattccacgaaatctattgaaaacgcatctatgtgcatagaaggctgcaggtgtcgcatcttcatcaggatcatggaagaatccaatcccccgctgagataaagcccaacaggaacatcagagcgcaaacgcaattttaaggaagcctcgaacagcgactccagctggtcaatataccatgcttcatgctgaaccgggatgtctgcatgctgttcaggataaacaaggtcccagtattcgtgttttgtcaaacttccgctggcaccgatttccaggtagtgtccgttctccaggctgtaaatatcccggaacatagttctggggctaattaatcccgcaaacgtcaatacctggtcaagccctacaaaatccacctggcggggagcatccggatgttttaaaatggcttttatctccgatccgaaaatgaaactatcatccgtttctgtatagaagaagggaataatacccatatgatccctggcacagaacagcgagccggacttcttgtcataaagtgcaaaagcaaattgtccattgagcatattcagaaatcccatgccgtattcctcatacaaatgaacgatcacctccacatcggaaccagtggcaaagcggtgtcctttctccatcaattccttcctgatttcaatataattgaatatctccccattgcatataagtacaacagagttgtcttcattgtgaatgggctgcatcccgttttccaatccgataatacttaaccggctaaatccaaaggcaaggtttccggacaccagcgtgtcctgtgcatccggccccctgtggatcaactgcgcattcatgtgctgaacaatggcctgatcatttccggaagccgggcgtttaaaatttataaatccgcagataccacacatttgctaaagaatttaatttgtgagttagatagaaatggcaacaggtacgttcaggattttttcatatttatatccaggatacgaccatggggattattgagaacattcaccaggatgttctggtagtactgcataaatatttgaatagtggcatgttcatacaactcactgctgtatacaaatgcaatacgaatgccttctcctttaccggggtatacttccgctttgagttcgtactgggttagtttccgttcctttctcgtgtctattgtagtgaacgccagctgatccagctccacttcattgtcaagaaagtttgcataggaaaaatgaatatgaataagcttttcatgtttatctctttttatcagcgacaacatctcatcaaattgaaaatcctggttatcaaatgcatctaaaacgcaatctttcactgctgccagaaacccgtcatatggcagttccctttccacctgcactcgcagtggcagctcatttacaaatgtgccgactatatcgcggaactcaggcctgttcctgccgatggtatcagacccgactatgatatcagtgttacccgacaccctggctaacaggatataatacacggagagcaggaacataaattccgatacgtttgcactggcggtaaattccctgatccgggcataaagttcgcgatcaattaccagctcgctgctggcggcggtgtaaacagtcactttatccctgttcatcatcaccggcaggtcgggagcacgcagctcgccagacaactgcctcctccagaattccctttgagcagtatatgcaccaccatcagcgtgctgccatactgcatagtcgatatacctgtagggaagctgtttcagttcttcacccttatacgccaacttaaattcattcatcaaaatgttaagcgaaatgccatcacacacaatatgatgtatgtcaatcaacaaaatattcccgagtctttcgtcctgtaacagacctactcttagcagcggagggctggacaaatcatgtggtttcacaaaatcagccaacgcggcggcggcatcgttatatttcccggcgtccagcctggaaatcctgaacgttaccgtttcttccacttgttgaaccactgtatcacctgcaataaacaagcaggttctcaatgccccatgtcgccggatcaggtattcaaatgtctgctgtaagttgtcaggatctacttccccttccagcttgtaggcactgttgatgttataagcgaggttgtctctttgggacacctgttcataatacagccggcgctgcgccgcggaagcggggtaaaaaggtgcttcactggctcttataaaagcaggcaggagatttttatgatggttctcaataaggctggtaagctcttttacggtgggatgttcgaaaatatcccttaaagtaactaccgaagaaaatgtactgttaatggcgttaatcaggcgatgggcgataatggagtgtccgccgatagcgaagaagttgtcctctaccccaacattatttttctccaggtgcaaaacatccgcccaaacttcgatcattttttcctccattgcattcgcgggcggcacataactttctgatggcagtaattcaggatccggcaaagccttcctgtccagtttgccgctggctgtcagcggcatctgttccagctgtacgaaagcccccggaatcatataaccgggcaactgtcctttcaaaaagtctcttaactggttttcattgatctgatctcccgcagtataataagctaccaggattttgtcgttccctctttcttttacggtcaccgctacctctttcagcatacccggcaaaagcagttgattttctatttccccgggttctatcctgatccccctaatctttacctggttatcggcccggcacaaaaactccacattaccatcaggcgtccatcttgcaaggtcccctgttttgtaaattctttccccttttataacagggtgctgtataaattttgaatctgtcagctccggattattcaggtatcccctggccagtccagcacccgctatgtgcagttcaccggcaactcctaccggtacaggtttaccatttgcactgagtatatatagcctggtgttatcaatgggcttacctatcggcacaggcttcgaggtttcctccattgtgcagttgtagtgcgtaacgtctaccgttgcttctgtaggaccatataaattaatcagcgagctgccacaattcctgaataaagattcccggaacatggcaacatgttcagccttcaactcctccccacttgaaaatacctgtttcagggtatgcaggcgggtaaaatcgaatgaggcatccagcaccgggagaaaggcactcaacatagatggaacaaagtgtatggttgtcacaccattttcggatatggcggtaactattttcgcgggttccttttctgctcccggttccagcaggcaaagcgaagcaccggtaaatgcccaccagaagagttcccaaacggaaacatcaaataccagcggcgttttctgcagcagcacactctcttcctgcagcgggtattccttttgcatccagaataggcggttgataaccgaatgatgttcaatcatcacccctttgggttttccggtggaaccggatgtaaatataatataggcaagatcctgacctgataaccccgcattttcaaatccggccggctgtgaaagtatttcaggaatcaccctgttcagatccagcagctggtaatcattgctgcattgcatgtcgccggaaggattccgggctaacaccatgcgaatacctgcgtcttttaaaacagactttatcctttgcgcaggatgtccgggatcaaccggaacatacacacctccagctttaaggataccaaatacagccgggatcagccactcattgcgatccatcattaccccaaccagctctcctttcttcaggccttttacttcactcaaataacgggctgttttgtcaaccctttcctgaagttcctggtaagtattgctcccattatgaaaacgaagcgcaatattatccggcgtctttctcacctgctcatcaaataccgcggtaatggtcttattggggtaggctgtggcagtatcattaaaccggtgaagcagcaggtgctgctcatcggggggaaccatttcaatatttgccaggctgatgttgacattattaactacctcgctgattatctgctgaaaatagcctgcccatctttcaatcgtctgcctttcaaataaatccgccgcatactcaaactcaaaagtaaatatagactggtgttctgtcactaatagagagaggtcgaatttggaaatttcctttgttgctttcagcctcgacaacttcatccctggcagtgaaaactcctgttgttcaaagttctgcaccgccataaaaacatcaaacaggggattacggccgctgcttctatctatctccaggtctcttaccagcatttcataatcccagtcctggtgatcgaaagcctcaattgctgttgattttatctcctgcaggaagtcccggaaagagcgattcgcacggggaaagtttctcaatgcaattgtattgacaaaggggcctattgttctttccacgtcttcatgaaacctgccggaagttggggtacccactacgatatcttcctggttcgtcaatttactgagcaggatattatacacagccagcaacagcatgaatatagtagtacgctcctccctggctatactcctcagcctggccgactgaagttcagctaactgaaaaataactgcgcttcctttataggtcttatgaagcggtcttgaaaaattgtatggcagatcgattaccgggggaacgggcgaaaatttgttaacccagaatgcccgctgctgctgtatttgatcttcttttatcttatcctgctgccattccgcataatctttatactgcaatcttaccccgggcagcagctgatcatgatacagggagaggaattcctgcataagcacactgttggatattccatcggaaatgatgtgatgaatatctacaatcagtattttttccacgtcagattcaaaaagccccaccctgataagaggagcgtgcttcaggtcgaaaggccggataaatccctgtacctttgcttgcatatcgttgtgttcctgctcatagcgttcgatggaaaaaacgggtgctgccagcacgctttgcattatttctccatccaccacttcaaattgtgtccgtaaagtttcatgcctgccgatcagctgcctgaagctctcctccagcttcagcacatctaatgcacccacaatccttaccccctgcggcatattataagcgagagacgtcctgttcatttcatggagaaaataaagccgcttctgaacagccgacaaccggtaactgccggtgccggacgttatgcgaacaggaggggccagctcacttgaacttactgaactgaaaaagtcaagtatctctggtttccggcgcctgatagatgcaataatttcctgtgtaagggccgccttatcgccacgaacttttacatcgttatcagcaacagaaattacaatgttattctcttttcttaaccgggtgatgtactcatctattctcataacgatatttcaattacgtcatcatcgccttcgaacgcatgttcagccggcagtatggtggcaatataagatgcaagctctgctatggtctgtcttacaaaaacttcttttagcgtaatccgtactccaaaagttttattcaacctgtttaacatggtaattgctttcaaagaatgtcctccaagctcaaaaaagcttgttcttacccctatctgttgctcatccagtttcagcacctccgcccagatgatgaccagtgctctttccaggtcatctgcaggcgctgcaaaatccattgtttgttgtatttccggaggaggcagtgcattgcggtccacctttccattggaagacagggggaactgatccagttgaaccaggtacgttgggagcatatatcccggcaataggctgcttaaatattttttcaggtccgatttatctgtttcctgtccggcaacataatacgcacataaaaaaggcgctgcaccattgtcgcttctcaccataaccactgcatccgttatgccatcataccggagcatattatgtttcaggtcatccggctcaatacgtataccgcgtattttaatttgctggtctgtacgacccagaatttcaagtttaccatcttcatgcaggcggccaatatcccctgttctgtatatcaggtcattgttgtttacagcaaacggattctgtataaacagggcattggatatcccggcatccacgaggtagccggcggttctatatggcgtacgtatatatacttctccccttactttcttcggacaagcgttcagtgtatcatccaataccatgaactgggctcccggcatagcagttaccgggataaaggaagcgaggtagtctgccggtttgatgaaataaaatccttttaccagtgttgtttctgtagcaccatagagattaaccagctgaatactgtctccgaacctggcataccagtcactcaactcatagggcaaaatcttttcgccagccagcaatatccatttcagctggtggaaaaccggtccggacagatcgcctgttctgatcagtttaaaaagactggggacacaatgaatcaggtttatccgctcccgctctatccaggcaatgaggctatctccgtcggcaaagatgtcttcatccgggatacaaagcgtacccccggcacaaagtgccacgaaaatatctctcatggatgcatcgaatcccaggctggtaaactgactgatcctgcaggattgctctactttcaatgtgctgatttcccaaccgatgaaatgcgaaaggcttccgttcctgcccgccactcctttagggataccggttgtgccggaggtaaagtaagcatatataatatcctctattgtataatcgtttgcccgctcaaacagtgaagaagcacgctcagcttcctctccggtaacagacagccactccgtacggccagcaaaaggtaactgcgccaccgcctctgattcctgatcagtaaggatcaatttcatttgcacactgttcaccattgcagccagccgatgatccggcaaagccgggtccagtggcacaaatgccagcctgacttttaagagtgctaccatcgaacatacctgcaggtatttgtttttgcaaaaaacacccacaaatgaacccggcgctaacctcaatgatgaaatagtattggcgattctgttgatggttgattccatttccgcataggaatgcgtaatgcctttatatactaccgcatcgttctgggcatgttgacgaaatgatgtgtggagtcgttcctgtatggtcatcctgccatgcgctacttcaatgtcagctgaaaacgttgctttcatcgtggcatcagccgcctcatcgaacacactgatactgctcaaagcggacaacggacgggtggcgatactgtgaataatatgcttcatcccactgagcacctggtcaatagtagcctgatcgtacctgcgctgattaaaatcgagttgtatagtaaagtcattttgcggcagtatgcgtacaataaggtcataattggttttaacattataggccgcagagatgatatcaaagcctttcccgtccttctctgcagctgacatatcttccagctgcctggcaacagggtagttttcaaataccatgatatgatctatcagtttcctgcccaacttactgaaagactgaagttctgataaagaatggtagtgatactgctcgctccggaggtcatcctcctgcgctaccttcagcaattcgctcaaactgcagtcctggtctaatttaagcctgacagggactgtattaataaataatccaaccatggtttccaccccttcaatctccgcagggcggcctgaaaccaccgcgccataaacaacatctttcacattgttaaagcgggcaagcaggataccccacgccactcttataatggtgttaattgttacaccatatccggctgaaacctttgccagtgatgcgaccacttcctgtgtcagctttaactcactgatcaggtgactgccctgtaccacttcaccggccggaatttctttttcaggtaaacgtgccagcagatcgtatccttccaggtaagttttccagtagtgtgcggattcgttcctgtctctgctctccagccagtctatataccgggaatacggtttaacggcagcattgataagagattcattcaattgcagctttgtataaatttcgttgaagtcttttacgataataccaatacaccagccatccatcagtatatgatggtgactccatatcaattcatatttcctgtaaccagtttggagtacggtcagtcgcatcagcatatctttctgcaacaggaaaggtttcaacctgtcgtggttccggtaggcttccagtacctgctccctgcccgattccaggcattcatcctgcacatcgtgatagtggaagtccatcttcctttcttttagtactacctgcaacgggcgatggtaccggtcatgtaaaaactgtgtccgtagcacggcgtaacgtgctaccagcacattcatggccgattcaaccgcggtaatatccagctccccttcaatatgaatgacggtttgaccatgataatcttccgcatcaggattcaataacgagtgaaacagaattccttcctgcgtgggagacaacggataaatatcttccacctcctgctgctcctgtaattcgtccagcagatctaccgggatactcttacaggtaagatcggacggacacagtaatagcctttgcccggagccgcagtaatcgattacctcacctaggcactccctgtacgcattcataaacgagctgattgtatccgggcgatactgtgatgtgctatagttcagctgtacctgcagctggccggagctgatcattgcaacaatatcccaatcatacaatcgcacatcttccggcgagatcgtttcgccatgaggatccgaagagatcttataagatctgcctgcagtatcactatcgaactggcccaggtagttaaacgtgattccggcgccttgctcctgcccttccggacctgacctgcgctgctgcatgagcaggtagtccattcctccgttcgggacatttctgagtgtttcccggatatcgcggatgagtacacccaggtcatcgctgtcgctggttagtactacaggataaatactcgtaaaccagcctatagtgcggctcacattaacggtaccaccaatatccgagcgtccatgaccttccatgtcaatgcgtagtaccggcgccgcatactgcctgcgtatactcaggtaaagggcggctaacaatatatcattcacctgcgtatgttgcgcatggtgtatcagcttcctggtaacgttactgtctaatgcaaaaacctcacgacgtatggaggcctgtattcccctgacacctggataatctttaggtaaacggaagaccggttgttcatcaatccggaaccaatgcatgcaggctgaccggaaggcatcactttccgcatacgacaacaaagcagcggaccattgctggaaggcatctgtcttcaacggtagtgatagtgtttccccctgtacagcctgacgatataatgtttcgatatcctcgaacagtatccgccaggaaacaccatcgatgaccaggtgatgaataatcaacaccaggcggctgccgtccggtacatgaaacagcccaagctttaacaacgggcccgtggcaaggttgatacctgattgaaggacattacaatgtgatatgaaatcggcctgccagtcatctttcttatacaggtcaaccacctccagtgataccggcataccagtaacctggttgcgctgaaccactgtaccctcctgttcttcaaacaccatacgcaatgcatcatgatgatccgtcagcttcctgaatattttaagcacccggtctgcggccagctgctccgggaagtgaagcaccaccgactggttaaagtgatgcttttgttccagtggaccatcaaagaaccattgctggattggcgtcagcccaacctcccccgataccgctgcctgagaagagatagcggacaaacgtctcagttttaacgacaactcacggatagtctgactgccgaagatatccctgattgttgtttcatatcctgcggaacgaagacgcgaggttatttgtatagatttgatagaatcgccacccaaagaaaagaagttgtcggtaacgcttacctgtgcgatgcccagtacacttaaccatatttctgacagcagtttctcttccggggtaacggctggtaaaaacgctcctgatgatgacacttcaggatcaggcaaaccacgcctgtttatttttccgttcggagttaaaggcatggattccagttgcacaaacaaggcaggaatcatataatccggcagctgttgctgcaggaaagcacgcaatgaagctgccgcaacaggtgaagccgatacgtaatacgcaatcagggatttcgttccattcaattccctgataatcaccgccgctgcctgaacctgttcgtgttccagcaggcagttctcgatttcacccaattctattctgaacccacgcaactttatctggttgtctattctgcccaggaactcgatattaccatcaggcagccatacgccaaaatcgcctgtcctgtacattaatcccgacccgctgatagtatcaggtaaaaatttcgtgttggtcagatcgttattattcaggtatccttttgacacaccgatacctgcaatacaaatctctccttttacaccaggcggttgcagttgttgacgactatccagtatgtataacagggtattgtctaccggctttccaatcggtataatgtgattcttctgtacatcataatcttccactacatagtaggacactacatccgtacattcggtagggccgtaggagttcatgacctttgcctggaagtggccggattttatccagccggcaaaagcacccatattgatattctctcctcctaatacaacatatctgatgtgtttaaggcgatcatatttattgggagcacattcttccagtaaaggataaaaggctgcaggcgcacagttgaccacggttactttttcagccgctattgtagctgacattttaagataatcatgctgtatctcctctgccagagtcaaccttgctcccgttactaatggtgcgaaaaagttcttctgtgcaaggtcaaaggcgataggggcgatcagcaggaagttatccaatgtggttgtatccagcgccctgacataccagttcaccaggttcaggaacgaaatatttttaatggcggcacctttcgggtttccggtagaccccgaagtatagatcacataaaacaggtcgccggcagagacccgcgggaaagtcccggtcacgggaacatcctttatgctttgttccagtgcatcataccgcaaaatatttgtatcagttatgctatatacaccttcttccggaatatcagtgatcagtactttcattccgctatccctggccataaacctgatcctttcaacaggcgttttgggatcaatcggaagatagcaggcgcccgaccgtaaaattcccatgatagtaaacaccaggcgttctgatttttgcatcagtacccctaccacatgatttacgccgataccatgctctttattcagacacagtccgatccggcgggctttgtacattaattcaaggtatgtcacggctatgttaccagatgtgactgcaatattatccggcgtttttgctacctgtttttcgaacagtgaaataatattttcttcctggtcaatgtcaacagcggaatcattgaactcaaccagcagctggtctatttctgtttgattcatcaggttgcctgtaattaccagggcctgaggggacattacaatattattcagggcgctttcaaaatattgaataaaccgttgaataaaagtttgtttgaatttctgtgtcgagtagtttatgctgatttcaaaattcccattcctggtactgatgttaaaatcaagatcggtatttgtaactgcataagatttgatatccaggtcggcggatatcgctgcgggagcatttctgtcagtctcgtataaggcctcattgtaaatatggaaatccacgtaattgaagatcgaatcaaatagcgggttttcgttaaatcctgcgcggtcaatgagtttaagtatgtcaaataatgacaactgctgatacctgccaacatcaatcatctttttatcgaccaactgcagcaatccgttccaggaaagctcattggggaacctgaatctgtaaggcacggtattcaggaagcagcccagtacctggtctccgccttcttccgcgggccggttgctggataccaatcctacaattacctcgtcgttgtaagtaaacatcttcaggacggccaggtaagccgacaccaggattgtttttataccaatccctttatccctggaaaaggaggtcagtctttcatatagctcgcctgaaagtcgttgctgttcttgtcctacactgtgccgttttacatgccctgtatccgccagttcctgtttggcgacgtcatgcaattcctcctgccaatactgggatattgccttattacgtttggcaagcagttcctgtatcacataatgtttataggaaacgttgatggctgccgggcggaatgagcgatccgccaataatttcagataagtattattgagttccgtcatgaatgaggcaacactccatccatccataatcgaatggtgacatacccataccaggaagtaattttcgggagacaatctgaaaatattcattctccagagaggaggttgttcataattgaagggcgcctgcctgtcggatgccataaattcaattacagtggattgctgctcgtttttctccaggtgtgaaatatcagagaaacggatagctgcatcaatgtgtttgtacacaacatgcaacggcacttcatcatcactcatattgaaggcagtccggagcaccccatgcttttcgaccatcaactgcaaggcatgctgaaacaaatctgcgttgaatgagatatagcgaacattgaatgtactctgatcatgatacaaagcgccttcactggcagaaagagaatgatagatcattcctttttcgatatcactcatcgggaaaacttccgctacattttcacggtccataaacctggcattcagctcatccagctcctgcatcacctggctggcagcagcaacggcaagcggctcctgctgctttgtttccaatcgtttagccaacagggagatagtaggacactcaaatatgtcaattaacccgatacccgtagcggctcgtttcctgatggcaggcagcagccttattgccttgatggaatcgcctcctatagcaaagaaattatctgttaaagagatggcacgcgtaccaagtacttcttcccacgcatccagcattatcttctcactttctgtttcaggcgcaatacccgcgtcctgttttccagcccccggcacgggtaacgctgctttgtcaagctttccgtttgaggttagcgggaagtgatccaggtagataaaataagaagggaccatgtagtccggtattttctccaacaggtaagtgtgcaatgcggtactgcttatttcttcctccgcggtataataggccaccaggtatttgtcgtcttctttttcacgggcttccaccaccacttcaccaatacggctgttacctgataaggcgtgcgctatttcccccagctctatacggaaaccccgtaactgtacctggtggtctttcctgccaaggtattcaatttcacctccgggcagcaaacgcccaagatcgccggtgcggtaaagccgccctcccattttatacggatcctgtacaaactttgcagatgttaagacttcgttgcccaggtaacccctggaaacaccagatccccctacgtataattcaccggtgataccagccggaaccagccgctgatgctcatccagcaggtaaactgataaagtagggataggtttgccaatgttgctgatattactgctgatctctttttctgtgatctctttataggtaacatgcaccgtcgtttccgtaatcccgtacatattaatcagcttaacagcaggatacagctcccgccatgaatgcaatttcccagggctcagtgcttctcccccgaaaataacatagcgtaaagacagacccgttacagtcaattgcaaaagattataaaaagcactgggcgtctgattcagcaccgttaccccttcctcccgcaataatttaagatacaaacccgtatcacgcgctgtcatcttcggaacgataatcaccttacccccggttaacaatgccccaaaaatctcccatacactgaaatcaaagcagtggctatggaacatcgtccaaacatctgccggaccaaaggaaaactggaaatcatcgttgcagagcaaccgcactacattacgatgctctaccatcacgcctttgggatttcctgttgttcccgaagtataaataacgtaacataagtccgatggcagcggcttgtcaggcgaaacagcgctgaactgatccctgtcttctattaacaccaccgctatacctggctttaccaggtctgcaaactcctttgttgtcagcaccaaccgggtctgactattatccagcaggtaattcctcctttcttccggataggtaatatcaaccggcaaataggcgccaccggctttcagaatacccaacatgcctaccaccatttctatcgaacggtccatcaaaagacctactaccgcatctggtttcactccacgggccgtcagctgcgcggccacctgcccggcctgttcatccagctgtgcataggtaatagcagccccttcatattgtacggctgtattcccaggccactttgttacctgttcatcaaacaggtcaagtatcgttttatcttcaggatagtggctgttggtatagtccaggttatttaccagtgctgctttctccaattcagaaagcagctcgattccggatagggttaatgcaggtgcggcgaccatccggctaagtacctgttgtaaatgatgcaacatatttctgataatctcatcagcatatacgttattattataactgattttcagcaggatgtctttgccgggatatatcgttatccaaaggtcatagttcgttttctcgtatgtttctaccgctgtgatgctgagtccatcactgatgttctttacgtcttcatcaagcgggtaattctcgaaggccataatgtgggtgaacaaacggctgcccaattcatttgcgccctgtatttctgacaacgggtaataatggtgcaaattcgcttccaggtcctgctgctgtgtatcttttagtagtttttccactaccgctgcattatccagtatgattcgtaccggcacagtattaataaataaaccgaccatagattccacaccggcaatttcaccggggcggccggatacgaccgtaccaaataccacatcgtccaaattacaatagcgaccgagcattattccccaggctactttaaatattgtattaatggttacccccacttttgcagaaagtgattcaatggattttgtcagctccgcactgataggcgcctgatgtgtaacgatcgtataggatgaactatctgaaatacgcaatgctttcccaggcaaatccgcctgttggctatatccccggagatactccttccaataggcagctgattcattcctgtttctcgtctctaaccacgttatataccgggaatatggcgtaaccatacccattgagatggattcaccggacaacatcctggtataaacttctttaaaatccctgacgataataccaatacaccaaccatccatcagtatgtggtgatggctccataaaagctcatactccctgtgtcccgtttggagaactgtcagccgcattaacctgccttcctccaacaggaaaggttgggacctgtcaagatgccggtaagcttccagcacctgctttctgcctgattccaggcattcctcacgaacgtcgtgatattggaagtcgatttttccacgctttaacaccacttgcagcggacgatggtaacgatcatgcaaaaaacgcgtccgcagtactgcataacgtgctaccagcgcattcatggccgattcaaccgctgcaatatccagttcgccatccatatggataagcatctgttcaaagtaatgatcggatcctttatccagcaaggcgtgaaataaaagcccctcctgtgtgggagacagcgggtatatgtcttctacctcctgttgttcctgtaattcatccagcaaacttaccgggatgcttttccaggtgagatcagaaggactcagtaatatcttctgtcctgagctgcagtaatcaatgacttcacttaaacactccctgtatacatccatgaacgcagctatcgtatccggatgatactgtgacgtgctataattcaattgtacctgtaactgacctgagctgaccatcgcgatgatgtcccaatcatacaaccgtatttcttctggtgagatggtttccccatgcggatctgaagagataccataagatctgcccatggtgtcgctgtcgaattgtcccaggtagttaaagctgattccggtgtacttgtcctgcctttccggagctgacctgcgctgctgcatgagcaggtagtcgatccctccatttggaacactgctgagcgtttgccggatgtcgcggatcaatatgcccaggtcatcgctgtcgcttgttagtactacggggtaaatagtcgtaaaccagcctacggtgcggcttacattcaccgtagcgccaatatccgagcggccatgtccttccatgtcaacccgtaacaccggtatcgcataccgcctgcgcatacccaggtaaagggcggctaacaacatatcattcacctgcgtgtgctgcgcatggtggagtaactttacagtggtattactgtctaaggtaaaggcttcacggcgtaaggaagtgcgtcttcccagcgcaacgggatagtcccgctgcagccggaaggcaggctgctcatcgatccgggaccagtacgcactggccgaacggaaggcatcgctttctgcataccgcaataaagtagccgaccactgctggaaagcatccgtcttcaacggtagcaatagtggttctccctgcgcggtttgacgatataacgtttcgatatcctcgaacaggatccgccaggaaacaccatcaataaccagatgatgaacgatcaccaccaggcggctgccgcctggcgtataaaacaagccaagcttcaacagcgggcccgtggccaggttgatacctgactgaagaacattacaatgtaatatgaaatctgcctgccagtcgtcttttttatatagttcaattacttccagggacaccggcacaccagtacccaggttgcgctggacaattgtccctccctgttcttcaaacaccatgcgtaaagcatcatgatgatcagtcagctttctgaatatgtcaagtacgtggtttgtctctatcctcccggggaaatgaagcactaccgactggttaaaatgatggcgttgttcaaatgggtgatggaagaaccattgctggatgggcgttaacccaacctctcctgttactgctgtttgggaagagatggctgataagcgtctcagttttaacgataatcccctgatggtctgactgtcgaagatatccctgatcgttgtttcatatcctcccgaacgaagccgggacatgatttgtatggatttgatagaatcacctcccagtgaaaagaagttatccgttacacttacccttgtgattcccagtacacttacccatatttctgacaacagtttttcctccgctgtaacggctggtatgaactctccggctgaagatatttcaggatcgggtaaaccacgcctgttgatctttccgctcgaagtcaaaggcatagattccagttgtacaaacaaggcaggcatcatgtaatccggcagttgctgctgcaggaacgcacgcaacgaagctaccggaacgggtgatgctgatacgtaataggcgatcagtgattttgttccattcccttccctgatgatcaccgctgctccctgaacctcttcgtgctccagcagccggttttcaatttcacccagttctattctgaagccacgcaactttacctgatcatctgttctacccaggaattcgatattaccgtcagcatgccacatcccaaaatcccctgttctatacatcatttcaccgggataaaaaggatttggcacaaatttctgcgaggtgagattttcattatgcaggtacccctttgccagtccatacccggaaatgcaaagttctcctggtacgccaacaggttgcaattcattattcaatccaaggatcaatatcctggtatttgctatcggctttccaatagtaatctgcgccggcgcctcatttttcatagcaagaatggaagtacaaactgtatactccgtaggtccgtatgcgttcaggaaagtccgcccaggcgtccattgcaatgcaatcttcctgtcacaggcctctcctgccgaaatgatggccctcagctggtgcaggccgtcagcgggtaacacccttaaaacagatggaggaagcgtaacaacatcaatagcctgttctttcagcactgaatacaaaacatccgtagaaaaagtatcagatcttttgaagatgactaaggtagctccggaagatagtaccgggaaaatttccgcaacagacgcgtcaaatcccagggacgaaaactgtagcaacctggtttcaggagcgagtgccaatacgtttgtaaaaaccgttgccaggttagccaggcctttatgtcccaggagcacgcctttcggcctgccggtagatccggatgtataaataatataagcattatccccttcctgcacttcccggccaccaggcgtaccggaaaacagatctccttcaatgagtaaatcatcctgtaataaaaaatccggcaggaggctgtctggcaggccttcctggcctgttataatccctgtgcctccggaaagaaagtcacgatgtagcctgtctgtaatacaatatcccggtttactctcttccaggattgaccagatcctccccgccggccaacgcggatccagtggcaggtaaacggctgccgccttcatcacgcccagtatattggcgatggtagctgcggagcattcctgcaggatgcccacaatgtcaccatgcgatacccctttctccatcaggaccccggctacctgatcagacctctcatccagccgtttataggtcatgctttcatacagcttccggttgcctgttgttgcaacggcgccctcttcgccaaaaattttatggtagaatggttcactacggaaacgttgcgggaaatgaggcaaatcggtatcaaaatcaattttctcaccggagatgcgggtcaaacaacctttgatgctaaagtcgggattaatgccgttatcattcagccgcctgtcaatcaccatctcaatcatatcgcccttgccaaccggaagcccggggtaaaaaacaggcacgaataccggcagccagcaatattcatattcaagtgtatccagtacttccccatttgcacccggcatcgttaaccataccaggaatccctgtatagtgtcctccctccggatataaaatttcacagcatggctatcttccggttttaccgctcccccgttaaaatccaggtcttcaaatgtttcagcgccggataaaagatattcctgtgaaaagttcctcagacaaagccttatatcggcacttctaccgatgtaatcaaatgttttgcggacataaggagccgaaacatcagaaaaaccgggtgtatcaataaaatatccgggtaagctaaccggcgcaatcctggtcagatttctgccgggaatcataataccgtcttccttcagaaaacgcctggcattattcaacactacggcggcgccttcgcagccacctataggacctaccaactccgacaaacatacatcagctttctcgggtaagtctaccagcatggcatccccgtgaatcaggtgaattttctgatccaatccggcatcctttaaaaactgttttgctttgttataggtttcttccagtatttcgatggcatatactttttctgcaccagcttctatgcataacctcgacaatataacattaggccctgttcctatttccaccaccacctttcctttcacatgtcttctgatctccttttcataccacgcattccttcttacatcgttcgtcatcgcatggtacaacatgtcgtcataaataaaatattctgccgtagaaggccataactccatcgggttagctacctcatcccgaatggccacggcatccggatgttgtgctgcctgttgcttaaaccgttccagcacggtagccgccggtgcgccggcaggggcaatactattgaattcgtgcaggatctgatgctgctcaacaggattaatcagctggatcgcagcgatactgatgctgctatcggaagttaccgccgatactacatttgtgaaaaaatgtacaaacctttttatggtggcttccttaaacagatctgtcgcatactcaaaacttaaaaacagctgactgtctttctcgtatgcccgcagggtaatatcgaattttgaaatggcatgtgctgttttaaaaacagaaatcttcagaccagggagtaacagctccttttctctgtagttctcgtaagaaagcgccacatcaaacaaaggattgcggttcgtcttcctttcaatactgaggtcatcaattaactgttcatatgggtagtcctggtgatcgaagcaggacaacatcttatttttcacttgcagtaaaaatccgctgaaagatttgccggcagcaggatgatttcgtataggtaatgaattaacaaacatacctaccatcgtttccaggtctgcatgctgtcgccctgctacccctgttccgataacaatatcctcttccccggttagtttgctgaggaatatgttaaagacggacattactgccatatacatggtagcgccggccttttctgctattgatttcagctgctgcgtttcccggatggggatagaaaaatcaaccgcatgtccattaaagctgttaattacaggtcttggaaaatccgccggcaaatccagctgctgaggcgattctgaaaattccttcaaccaaaaatcccgctgggtacgcatctggcgttgttgtacttcgcccgcctgccaaactgcaaaatctttatactggtgttttagttcagggaggtgcactccgttatacaaggacataaactcatcaaaaagcacctgctgggaaacaccgtcgctaacaatatgatgggtatctaccatcaggatatgctccttctccgataactcaataatacctaccctgatcaatggtggattttcaagatcaaatggtttaatgaagttttttactatctcctccacatccggaaactgtgctttataatatacacaattcatcgatacatccggaaacacacgctgcacgggttctccctctttcacaaaaaaaccagtccgtaaaatttcatgacgggatacgagtgtttttaatgactgctcagtcctcagtttgtcgagggatccctccagcatcattacgataccaccattgtaagcaatggaatgcttatcatactgatataagaaataaaggcggttttgcccggatgaaagcttataatattcctgcgccggcgccttttgaatgtctatatgcttacgggtttccgactgtgccagtaataacgctaaactccttaccgtctggtgttggaagaagtcttttatggaaacagatacctgaaataccttataaaccctgctcgccagcactataatgtgcagggagtgaccgccaagttccgtgaacgtacgatcgataccaatgtcctccttattccgtttcagaatatccgaccagatctcaatcaatttttcttctgtttcggtggtgggagcggtataaccaagttgttttacagatggcgccggcaaggcgttcatattgattttgccattcgcagtcaagggccacgctgtcagatgaacaataaacgcaggaatcatatagtccggcaacagatcagcaagaaaatctttgatggccacttcgctcaacaggctttcagagagatagtaggcaatcaaaacagtatcgtcatcctgcgcttccgccttcaccaatacctggtccacgccatcaagcgacagcatcgccgtttcaatttcagacagctctatccggtatccccttacttttacctggtgatcctttcttcctaaaaattcaatattcccatccggcagccaccgggcaacatcccctgtcatatacattctggcgccgctttcaaaaggattagcgataaaccgctcatcagttaagtcctgttgctccagatatccaatggctactcctgctcctgcgatatacaaatctcctttcatgccgataggaacaggcataaggtgctgattcaatatataacaccgggcattgctgattggttttccaatagtaggtgctttctgaaagtccaacagctgatcgcggtgaacatatctcgctaccgcgccaatagttgtttcagttggtccgtagtgattgataatttcgatagacggatgcagtgcgaatgtttgttctattgccctcaccctgatcttttctccgcccagtatcaccagccttaagtccgtggctgttttaaaatcaggatgatctgttacagcgccatacagggaaggcgtcagcttcaggtaagtaatatgattttgccggaggtaccggagaaaaaaggcaggctgcatgtaaacttccgcaggcaatatatgcagttccgcaccggacaatatggaggaaaatattcctgtataacccaggtcaaacgcaaatgatgttaccaatgcggttttatcggtatggtttattcttgcaaatttgttgatccaggtggcataattaatcacattctcatttgaaatcatcacgcccttaggcaggccactggttcctgaagtatatatcacatacagcagatcaccgggtgtaatggtcaccaacggattttcaggagaactgttattcaggtccggatgatccatcgccagttgatcaattccaacaggaacatcaaccaatagttgttgctgcgtcaatattaaccggcagcctgcatcctcacaaattttcttcagcctggatacggatgtttcagggttcacaggcaaaaacgcagccccggcttttaatatccccagcatgccgatcatcatttcaacggagggttctacccgcaaaccgatgatatccagccccggatgactattgagtaccacggccgccacctgattggcccgcttattcaatgcggcataggaaagccttgtttctccaaaaacgaccgcaatattatccgggtaagcagccacctgccgctcaaacatttcaataacagactgataagatggtacatcggccttcgtatcgttaaaagcatacaggatggtatccttttcagcctcgtttaacaacaacacctcactgacaagcctatccgggtaagttagcacatccccgataagatgaatgaagtagcttgaaaatcgctctatatagtccgttgaaaaaatactgcttttgtagttgaagtcgatcaccaatgcgtcatcggtaaaaacctggatagacagcggcaggtttgtattctcataatacccgtgcagcgctatgttcagcccctctacgctgtcgaggatgttttgatcaaccggataattttcaaagccaatactcgactgaaataagctttcatttgcagtgatgccaactgcctggttaatttcatgcaaagatgaatgatgaaattgacttctctctatcaatcccgtattcacacttttcaccagcgcttcgagcgttatccgctcatcaacatgaatcctgattgggacagaattgataaaatttcccactaccgcctggcttccctgcacaaaggggttcctgttagatacggtcgttccaaacaccacatcatttgtattaccatactgttgcagcagcaagccataagccgtataaataactgccgctttggtaactttattctttttcacaaattcattaaggccatccaggtttttattgatcctcagcttgctgacatcctgcgacagttctccctggttagcagcctccgacaaggggtgtccgatttcatatccctccaggtagttcttccagtaactttctgacgcctcgtgatccaccagttgccagctatccgcataaacagcgccgaaggcaggtttatcagtgtgttcaggcgtatcccccttattaaggctgttataataccggagcaagtcttttatcactatcgccgtactccatccgtcatataaaatatgatgatgcgtgatgacaatgataaaatcttccgctgccttctgaaatatcctaacccgcaggggcaaggctgtgaggtcaaatttctcctgctgatcgttcaacagttcctgcgtgattataccggcagctgtctcagggctatcttttgagtagtcgtaatatttaatgtcgaggtcacaggacttcagaattacttgtatgggagcctttatttcctcccatctgaatacagatctcaatacatcattctccgattgtaccagggagaatgcctgtctcaggatgttcatattgagcggccccgataccgcaaaggatatctggacattgtaaagattataatctgcttccttcaaataatgatacaacatgcctttctggaccatactaagctcgctgatctcctgcacatttgatttctcaagcttctttttcaagggaataagatttaagtgggtaatatttttgaagaataaccggtaggtattaattaaaaagaactgacaactcatcgtcgtcaagtccatccgcccctgcgcccagggaaaaagaagtaactggtaactcttcccggaatttattatatgccatcatatggagcagccatttcaccaggttgtccgcaaatgattgaatggtagccatttcatgggccaaacgattatactgtatatctatttccagtgaatcctttaacacaataacattgagttccagtttagccgtcattacattgtccggggctgtgttacttcccctggtgtcatcagaataagcatacagatcattgtcgaattcctggtcaaattgtccgaggtagttaaacctgatttcagacaatttctccctgctaacctgcagggcctgatgcaggtacctgaaaatgccgtatcccagcccattgccgggaacattggtcatttgctccctgaccccccatataacagcttcaagggacccctcatggagttgcagttgctgtggatacatagaagtaaaccagccaacagtcctggagatattcagatcatcgagatatcttccatgattttcctgctcgataacacatacattctttcctatccagtccctgacagacagtgccaaagccgcatttagcagaatggtgatgtccgatttatatacctggtgtgcaagcttcaataacgcccgcgtgcctgctttatctatcgtgcgtttctcatttgcagcattcatcgtgcgccagtctgccggccgcttatccaggggaagtgaaaatggaacatcggccactgattgccagaatgccagttccgccgcattgccatcaacatgcggatatcgcagcaaagcatcataccactctctggcagtggctgttttagcggggaattttaccgggttattgttcttcagacttttgtaggtagtataaagatccttcaacaaaattctccaggaaataccatcaacaattaaatgatgtgcggtgataaataacatcctgtggtttcctcccattttgaaaacagctgctttcaaaagaaggtcccttgaaatatcaaagctgcttttaagagacatgcatattcccttcatttcctcgccctgaacatccagttcaaacgatgttatggcaaatgggctatcgcggtgatgcttgttatagaataatgttttccgccggggatcatagttgattctcattccgtcatgttgcctgatgagcgcctgaaacgacaactgcagcaaatggagatcgatctcttcatgaaacgaaagcaacatagaatgattgtagaaatcaggacattgaaaatcctgatcaaaaaaccaggcttcaataggcatcagctcacgggccccctctatatatccctgctcatattcccggcgactttctgtattctgcaggttagaaacgatctgccggattgtttgatagataagaatatcctttatggtcagcataaaaccttcatcagccaaccgggataatatctgaatagccttgatagaatctcctccgagttcaaaaaaattatcactggccgaaatattatctaccccaaatacctcattccatatggctataaaagttttatcgcgtgcatctatctcctgaacattcgaagcttcagaaaattccattgccggaagtgctgcgtgatctatttttccattagaggtaagcggataagcatccagttgaataaaataagccggcatagcatagtagggtaatctgtctgacaggtacgacctgagcaacggttcagctatggtctcctgcatccccgaaacaatgtaataagctattataacaggtgacttcttcccttctcttatgatggctaccgaagaagcaatcccctcgtaagttgccacctggtgttcaatttcagtcagatcaatcctatggccgctgatcttaatttgcttatctgtccggcctatatactcaataaggccggaaggaaggcgcttcgcaatatcgcccgtcttatacatccttaaccctgccacaaaagggtcgctgatgatcttctgcccggtgaggtcctggctacgcaaatatcctcttgccaccccttcgccggaaatatacaattcccctttaactccaataggtaccggcctaagcgaatcatccagcacatatatgcgggtgttagcagcaggtatgccaataggcactgccacggccttgtctgccgggtcaaattgatgaatcatacatccaacagttgcttctgtcggtccatattcattatagatctctatatgatcgccaaaaagcaggtgtatttccgccgcaatggagcgggtcaattcctcaccaccaactataaagcgttttattttactgttgcgcgcaacttccctggaaatgcaggaggcgatcaatatcaaatgcgagggagtggctttaactaccgccactttattatcaagcactactctccgcatcaaaaattcatcttccgcggcgctataaataacgatcctgttaccggttaccaacggcaaaaataaagaggtgatggttaaatcaaatgaaatagaggtatacagcgggaaagcagctttctcttttttcacatacatgtctgaagcccaggtaatataattgaccaatgaatgatgctcaatcattacgcctttgggattgccggtggtaccggaagtataaatgatataagccaggctgtttggctcagccgggctataagtagcaggaacattctccggcagtgtcagcgaactgatatccaatacctccaacaagggcagctcagaaagcagcaaagctacctccggcaggtctttgcctgtgatcatcatgcttgccctgctgtctgtaagcatgtagctgattctccggacaggcgttgatatatcaatgggcaaaaagcaggcacccgctttcagcactgccagtatggccaccatcagttcaggacgcctgtccatcagtactgccacaatactctccgtgttgatacctttgcttctcagaataaatgataaccggtcagcctgttcattcaattcacggtaagtgatagtgtcttccccgtattctatcgcaatcgcctctggcgtggcttccgcctgccgccggaactgctcatggatagtggtatggcgcgggaaatctgtggcggtgtcattaaaatgatgaatgatatcccggtactctacctcacccaacaaatttatttcatgaaggctgatgtccggcttctgcgttatttgttttaccaggttggcaaagtgaccggaaatccgttctgctgtttcctttttgaagaggtttgtgttgtattcgatgacgtactttaatgtctggtcataataaaatacttccatcgaaagatcaaacttggcaattcccggatcgaagaaatggcgctgcacctgcagatcgccggtcgtcatatgatcgtagccaatgttctgataaacgaacatggtatcaaaaaggcgattacgactggcatcagcaggtactcccgcctgttgtatcattctttcaaaaggataatcctggttatccaacacggccgttaacaggtgatgatgtttttccaggaggtccggaaaaaaagtgctggcggaaatatcgcttatcacaggcaggctgttgacgaacatgcctactatatttaatagatcggggtgagttctgcccgcggcggcaatacctattgcaacttgtggctgtccgctgtactttgataacagcacgctgtataatgtgaacaggagtgtattcagtgagcaggcatattgtgtggctatccgggaaagactggcggtaatatctttatccagcagtacttccagcttttttcctgtaggattgaaaataacgggacggttgaaatcaatgggcaggtccagtaccggaacggattgagccaattgctgtttccagaataattcctgcctttggaggttgcccgatgcaaacatacggtgctcccaatccgaataatcattgtaattaacgggaagggaaggcaactcatgtcccctgtagcattcgaataattcctgtacaaaaatattcgcggatataccatcgcagatgatatgatgaaaatctaaaaacaagtaatgttgctgccccggaatgtttaccaggcgaatcttgaacagtggggattgatgcaggtcgaaaggggtaaccaactcctgtaacaattgatccaggttctccggagtggaagttatataatcgaacggcaaagccactgcttcgtgaatcctgtataccggctgttgagggcctttaaatgacatacgtaacacttcatgcctggataccagtgtttctatggctgccttcagcttttcccggttaacaggaccgtctatctttaaaataacaggtatattgtatgcggtagacgtttgatctacttcccatgtatagtacatccgtttttgtgcagcagacaatacatatgtatctgccggtgctgtacgggagatggaatgataaggcgccgctttctccaggttggctatttcagcagcgagcgccgggatggtgggatagcggaagaatacttccaggcccaactccactcctaattcctttttcaccaacatgcatacctcagatgcccttaaagagtccccgccattttcaaagaagtgacctttcccattaaaatgctgatgcttcagaatccgctgccagatatcaaatagcttttgctcgacaggtgtccccgggtgaaacacgtcaaaatcattggctgcatcttccgttaagcgaaataatgcatttgttgtttccctgtacttaccttcgaggtattgcgctatcagcttaaaacgttgcagcttaccactggtagttctgggtatattctttacgggaatcacctggtcaatctcaaatccacacctggtattgatcaatttcctcagctgcatggcggtttgaataaacgaagaaagctcaccccggtgaagcacaaaagcaattacttcgtctctctgcgtatttctgttaaaaaagccaccaacggctaccttgtttagttctatggcatcaatttcctccgctatgcgttcgatgtcgtgcgggtaaaaattctgaccattaataaagatgatatcttttgctcttcccgtgacaaataatgatcccttatcattgaggaagccaaggtcacctgttttcaaccatccatcagcactgaatacttgtccggaagcatgtttgtcattgtagtagccctttgttacattatctccctttatctgtatatggcctattacagcagcatcaaccggatgatcattatcatccgctattctcagtgagcagccgtccaccggtttgccaacatctgcaaaagaaacagcgtcagcagtctcttcactaaacacaaccttatcattgatattaacatgatttctgctaaccattgcagatactacatcgctgtcaagatccgatatggtaactgccacactagcttctgccagtccatacaccggccgcattgcctgtttctgcaacccatatcttttcatgctatctgtaaactctttacagatttctgtagatatgggctcagcgccgttatagataatccgcaggctggagaggttccagtcgtgatgatcatcgggcgtataatgcttcagaaaataccggtagccgaaattaggtgagcaggtaatggtggccctgtgccgggaaagtgcatccagccacagtgcaggcctgcgaacaaacaggctcgttggcatcaggcactgattcattccatgtagtaaaggattaagatgaaagccgatcatacccatatcatgggtcagtggcatccagctcaacgtggaatctgaaaccgaatatcgggcagcattactaatgccctgtatgttggcaataagattttcatgagtgagtacaacgcctttgggatttccggtagagcctgaagaaaactggataaacgcaatgtcctgcgggcttacgattaccggctcagccgccgcacctgctgatagcgcttccgactcattaatgtaacgggtgccgatctcgtcactgtttacaaaaagggagtttgacagggcatatgctgtcatcttttcaaagtgcgccgcagaggagatgaggtgaggcctgttcaatatcttccagacattaaagagcttttgccgatgcatatccgttcctcccgttgccagcggcaccggtatcattcctcctaatatgcaagcccagaaagcaataagaagagatttattatcatcagtttgcaggatcacctcgtcattccggcaaacgccccgtttctgtagcaccagtaagcactgcaatgctttttcatacaaatcttcatacaacaggaaatgttcatcagtatggctttcaataaaggtaataccagcatttcctaatgtactttgtgcctgtataagttgaatgaggtttgttatacgcatatcgcttagttaactcagatctggcttccaaactcagcgggatgctcacgtggaattacaggaaaatcctgtcagtacaatcacgtagcggcatagcataaatttttatcgcatagcttgctctgttcgcagaattattacattccggaaaataagtacgctgacggcaaaatgagtatcaggttgaatttgaatggagcaagacacagctccgctgaaggttgttacaaatcgagggtcaataaaaaaaattgagaaattcgggtttaatatttgcaaaataatgttttaaatgataatttcaaaattattagaagagtcaaaactgcttttctattatttgtataataacccaatgtttactgtgctgtatccatatgccttcctatagcgcatcacacattttgaatcttcaattatcaattaatttctgtttatgcaatccaacgttacaaaacccggtttattaacgaagctccaaacctcatctgtagccagatccttaaaagaaaaaatcctgcttaaaataaaatcacgctaccggataagcgtagatctcggtattatcagcatcaccggtattaacagcataaaaataaagcctgttagcttacataataacgcccggaatatgatatgtgaaaccggcagcattcaggttaagttcagctggtattcccttttaaaaggcaggataaaattgatcgctgtaaaaatatctgattgtaaaattattattaacaaaagagaaactatacctgcaagtacgacagctaagagtacggtagttgccaatccccaggatatgatcagaaacttttacaagcgcatatccacccgggtagatactgcttttgaatcgattcctccgcaggtcaatatggagaacctggaaataattttttcggggcccaaaaatgtacaggtaaaaatcagttcgtttgctttgaacaagcgctattacaacacggcgccagacgcccgtcacctggatggacgcttccagccaaaaggaatatccaggaagctggttgcggaaaaacagctgacaatagatgtaggtaatttcaccatggtggctgatctacaaacagatactccctccaccacagtaaccgccaaacaattaacattgaagcttagccggggtaaagacgaaaacaacgggatctcttatgatcttgaaaccaatacgcatgacctcaccttgcacaatagtaaggtaagtaatcagcaggcatttgcgtgtgacctgggcatgatgctgtatgccaaacccgacttagaaggatttcatatcgaccgtcaatccagttttcatctgaataatctcagattccccttctacctggatcatttctacagggaaaatgacattatcgagttgggagtaaacctggtttcttgtcaaatgggggatatattgaaatcttttcaggacttcagcacacaaagtttatacaggagttcgttttccggcaccctgggcttcctttcccgtctacggtttgagttaaccaactcattcaaaagagaatttgaaatcaaactggataacaaccttcgcattttggatcatggcggcgcagactattcttatttaaaacaaccttttgttcataccgtctatgatggagatatcgctgtaaaatcaattaaccttgacagcagcaattcttttttccttccactggacaagatatcagcagatcttaaaaaggtaattatctgcaccgaagaccctcattactacactcacaaaggaattgactccgaggctatttttcttgctatggcatccaatataaaaagcaggaaattaagccgcggcgccagtaccataaccatgcaggtggtcagaaatcttttcctgtatcatagaaaaaattttcaaagaaaaatagaggaagttatactgacgtggtacctggaagaagtgttttccattggaaaggaccggatactggagatataccttaatatcattgagctgggtccgggtatctatggcgtccaggaagctgcttacttctactttgataaaccagctaatcagctcaccctgaccgaatcgcttgccctggcttatattataccaagaccaaaattcttcctggaagcccttaaaatgaattcaccgaaattaagaaagaacctgacagcacacattctgcacaattcaaaagtgatgcttaaaaaggacatcatctctttagaagaatttgaaaacatacaatacaaaataacatttgcacccggcctgggagagttgaacctgacagaagcggaggctactgtgaccggtagttaacctgaccaaacgatataaatcattaatcagataaggcagccatctgggattcggaaaaaatgttctccgtatgtccatctgcgtaagctggccttgacaaagaaaaataggtatgttgcaggaaccggctgtaaagctcactggacctgagatccttaagtatttcgagacatttgatttcatagtcgccgaataattcccggaatgaaacagtttcgacatcccctcccagatccagaaattttaacttgatttttcctcttgtcaaaaatttcaacctgaataacctattggttcccggctggtatcttttgatggttgtccacatgatctcgtcatccttcataatgtcccatttgaaccagtttctgtggagaaataatatttttccggccgggtcatgttgtaccattgacataccgcagaagccaacggtagactcttccattccacatagtcctacgccatctgcaatcatataataaggagtatgcagcgctttccacgcaaatctgaaggtatctttatctcccaataacatcctgtaatagtcttttttattcaggttaaaatggaggcaaaggttcagctctttccagcatttttctttgtcaatcaatagctgtccgctctcctgctctatcgaaccatcctctccggaatcaataattttccaaatagggttatggcggtctgttgtccagaagtcgggccaaaaaaccgttccatattcctggtattctttactgtcaaacaggaatgcaggatctgagatacaattattatcggcatccaggtataacacttccctgaaatcactttgtagaatggcaaatggcttcatggcgtagctcgtgagtgcagcaagattggttgttgtgtaatcctggcaattcctgcaccttacatccaatccttccaatgccgtgatgacctctgcattcagctctattccggtataccatacttctatcgggagtgtgcagccatttcttctcaacatattgatgttgatccaggcacaggtaaaataactcacgcccccggcgcaaattacaattcctcttcctgaaaaacgggcaggaaaaggttctgtttcagttacgaattttttccattgggtatttaatttcctgatccattgtctattacctgtgcaatggactttcctcacacaatcatccgtaaatgttgactttccttcttttaaagatccggaagtgcgccttttaaaaagttggagaaacttagtcgtgagcataatagtagtgtcgggtttaaacaaattaacaaatccgtggcatcagactaatataggaaataatttgaaaattattttctaaatacaatcaaagggactagaagattcaaatgattgcgcaagagtttgacaagatttttaagcgctcccgtaaacaaccaaatggaatatactcttcagggaataaaaaagtgattatgaaatataaaaaaagaatacgtattttgtaatacctttgagcaaataatatgcaggaacaaaaagggaaatatgaaggcttacagcatgatgaactgggaataaaggttcgctcaaacgacaatccttatctttcagctgatattcaaaacaagatcctgcaaccccgcagattatcttcttattttattgtattaattgaaagcggttccattacatacaatatagacttacaagactttacgcttactgacgggcacctgctttttgcaatgcccaatcaaattttgacgccacccgctaaaacagacaatctcaaatatttcaaattactgtttgatgaaaatacattggccttgttgccacaacaatttccttttttagtcaaccctttaaacgcaccgaccatagctcttgacagtgctgcaaaagaaagagttataaaggtttttggaattttaaatgagatactgtatttagataaatatgaaaccgatactgaaataatattagcttatttgaacttattgctatcagaattaaacagcgcctatttcaaaaataaagaacacggcaatatcttaaatgcaaacctttcaaagtttattgaattcaaattagttgtggaaacatcccttacagagcaaccttctatcaacgcaatagcagaaaaattagctttatctaccaacagtttataccggattgtaaaagaatacgccggcacatcgcccaaagactattttattaaccgcctgatggcggaagctcagagaaaattgcggtattctaatatttccatcaaagaattggcctacgaattgggttttaatgaccccgattatttttcaaggctcttcaaaaaaagcacaggaaaaagcgccagtgaatttttacccaggcaagatttgtcgggagaataaacagatttgtccatccccgctatttttggcctctctacttttgctttataaaattcatacaacatgaaatttgcattagtaacaggagccaacaaaagcattggctttgaagttgcacagcaacttgctcaggaaggaatgtatgtttacctcggcagtcgtaatttagaaaacggcgttgaagccgttggtaaactaaaagcaaagggattaaacaatgcagaagctattcagcttgacattacagacgatgaatcagtaattaaagcccgtaaagaaataggtaaaaaaacaaacgtgttggacatacttattaataatgcgggtatttatggtggttccccacaaacggcacttgattcaacgattgaccagtttaaggcagtttatgacgcaaatatctacggcgcagtgcgggttacgcaggcatttattgatttattgaaagagtcgtcagcaccccgcattgtaaatgtaagttcaagtcagggttcaattaccctccacagcgacccaacatataaatactacgactacaaaggcgctgtatatctttcttccaaatcagccttgaatatgtacacggtggttttagcatacgagtttaaaaattctcctttcaaaataaatgccgtttgccctggatttacaaaaacagattttaatggacatcgtggacccggaacggttaaagacgccggaaaacggatcgtaaaatatgcgctgattgacaatgatggccctacaggaaaatttttcagtgaggaaaataatcctgaaacaggagaaataccctggtagtgggcagctgatctggaatagattttgtgccctggtattccgtatatgagtacacaaaatctcaacatacagatcctggcggcaccttccatattggggctccgcacgaatggcgtgcaggacctggcagctgccctgctggaagccggcctcggccggctgcagcctgaacatccggtgctgcacctggctaccctcaacgggcagtacagtgataaaagagaccctgatacccactgtctcaacccggtgccgctgcgtgatttctctatcgagctgggaaaagccgtcaatttactgctggataaagaccgcttcccgcttatattgggcggcgattgcagcatcctcctgggtatcatgtcaggtctcaaaacccgtggtaaatatgggctgatctttatagatgcacatgccgacttctaccaacccgaaaaatcagtaaccggcgaagtggcggacatggacctggcgattgttaccggtcggggaccggatatacttaccaacatcaacaactcaaagccctatgtgcaggatgaccacgtgattcatatcggccagcgggattgggaggagacaaaaaaatacggctcgcaggatatccgcgaaaccactatcatccgttatgacctggaaaacattgaaaaggacggaatagaacaagttactgctgctgcaatagcaaaccttgatcccggcctggagggctattggatgcattttgataccgacgtgttgtctgatgagttgaaccccgcagtagagtatcgcctgcccggcggccttgattttaagcagtcggaatattttattcaccaacttctacgtaccggcaggatcattggttttgatgtcaccatcttcaacccccgcttcgatactaccggacagatcgcccaaaatatcagcgataccattgtgcgtgccttccgttcctgtaatgataaacacgtgttttgattgtcggtaacactggctatcctttagagaaaagtcgctccagcttcaataaaatgtccttgtgagttgaaatcatctcccgcatccgatgaaatatccgtattatctggatatttacagctatggctctctcactgttcaaaacacaggaaagcatagtcacaccttgctcactaaagcaaaaaggtgcctagcgaagtcccttaaacacttctttagaggacgcaaattgcgtcctccaattctcaaactcttctttgttcatttcaaacataaaatcctcaggaaaccgacttatatttcttcttacagcctctttcaatcttttagtttcaacaccataaagttcataaattaaattagagaaagccttcaaatcttgcgacttgaaggctttcaatcttccagtgatccctatggtacaaaacccgaacctttttgtctttgatttacgaaaattggccgaaatagcctaactgtacattcgtacttttgtaaaatatacagtaatcgcaggcattcggccaacctcattttcctaaaaaaagttctcattaaaataacctttctttatggtaagaaatatattcttaatatgaaaggtatacaccaggattctgttgaaaaaatcgtcggaaaactctttctccttcttttgtttatctgtaatgctgatcctgtcaggggacagttagcagctgattcgctaacagccgcgctaactacacaataccagcaaaacggttttccgggattcagcgtatctattgtaaacagtgatagcattttatacgaacatgcgttcggattcgctgaccttgaaaaaaacattccttacaccactactacggtacaaccgattgcttctatcagcaaactatttattggaatggcagtgatgaaagctatcgaacaaggcctgtttacactggacactgacatcaacagtattttaccttttaaagtacaacatccgtacgcgcctaaaatacccatcacgttaaaacaactcgttacgcacacttcagggataacagataaccctgttgcatacaaaaagacatacttatacaatacccccttgcaggaagacaatcccatctatagtctactgaaatcaaaaggttatggtgcaaaaggccaagacactactttaggcgcatttctccaggattatttaagcgcgtccggcacttattattcaaataataattttgataaagccgcaccaggtaaaagatatgagtactccaatatcggttctgatctggcggcctggctgatagaacttaaatcaggtatttccttcgctcagtacacacaacaatacattctgcagccattgcagatgacacataccacctggtctaccgccaccgcagaccagacaaagctggcaaccttatacaccggcctcaaagtcccttatccaaaatacagttccgttacttatccagatggcgggcttaccacttcttgtcatgagctgagtctttttctgaaagaaaatattgcagggcaggaaggcaaaggaaaaattcttactgctgcctcctacaccaccatgttacaacctgcattttcaactgcttataatccaaagaatatagatccaggagagcctaatattggtgtgttctatgccatgaaaaaaaatggtatcatcgggcatagtggcagcgatggaggagttactgctttccttttctttagccccaccaaaggttatggcatgttattaatcaccaatacagaactggaaggactgaatggtgtgaacaaaaaattgctgacaggatttgaaaagatatggggcactatgagccactacgcaggaaaattgcacctggttaaatgataaatacataggttgtaaagaggttatacaatcgaactcggctaaaaacaaaaacccgcgctatgcgcaggcttgtaagttgtctgtgatccccttgggactcgaacccaagacccatacattaaaagtgtattgctctaccaactgagctaggagatcctttgctgttaagcggttgcaaaaataggaatatttttattcctgccaaatttttattcaaaaatatcccaaaccgggcaccacaaagtattataacacctcccacccaaaaatagttcattacatttctgtaaatgccttgtaataaattgatgttactcacctatttttgtgaagctaaattatacccatgaaaacgtactttcagaataaaacggttgtcatcacaggcggatcgtcaggaattggaaaagcccttgtaacagaattactgggacatggcgctcatgtggctgtttgcggcagaaagcaggctgccctcaatgacctgcaacaggaagtcaataacacccggctgtttactttcgtcgcagatgttagtgtagaggccgaatgtaaagcctttatcgaaagtaccatcagtcaattcggaaaaatagatatccttatcaacaatgcaggcatttccatgcgcgccctgttccgcgatctggatgtaagcgtattgaaatcacttatggatatcaatttctggggaaccgtatactgtaccaaatttgcatatccctcaattcaggctaacaagggaacgattgtgggagtatcttccattgccgggtacaggggcttgcccgcacgtaccggctactccgcttccaagttcgccatgcagggtttcctggaagcgctgcgcaccgaaaatttacatacaggcgttaacgtgatgtgggtatgccccggattcacggcctcgaatatacgtaacaccgcactcaatccacagggacaggcacaaagcgaaaccccgctggacgaaggtaagctgatgagcgcagaagcagtagcagccgctattgccaccgctatcgccaaacgtaaacgtacgctggtactcaccggccagggcaaactcaccgtgctgttaagtaaactcctccccggcttcctggacaaaatggtttataatcactttaaaaaagaacccggttcccctcttcagtaagcaaccattcttttcactgtagccgttaacgttagtgcaaaaaattccgcttaaaatacgatcgcctcggcttttttgtctttatttgcactaagtttagttcacttaacccccaatggcatcttttttggaaggaaagcgcacttttaatttgccattccggataaatgaaaaacggatagacgagtgaggacgggaattgattcgtgggttttgaacactgggatttggatttagattttcgggcatgtccattataactttaacatcagacataggaatgcaggattacctggtaggtgccatcaaagggcagctctggcaatactgcccggaatgtcatgttacggacgtcacacaccatatcagccccttcaatctaccacaggccacttatatctgtaaaagcgcctttgcctatttcccgctcggcacctttcactttgtattaatcaatttattcgataaacgcccggatcatgtgctggtagcagaacataacgggcaatacatcggctgcgcagacaatggcctgctcaccatgattgccggaggtatgccggagaaggtcattaaactgccccttccgccggatgcacccaaaaacacatttaccatcatccagctgctggcatccgccgcccgggagctaagccgcggcaaagccctcggtgaactcggcccgctcacccagcagatccacgtaaaacacaacctgcagccacttgtgggcgacgacttcatagaaggacagatcattcatatcgacagcttcgaaaacgttgtcgtgaacatcacccggcaacagttcgatatgcagtgcaaaaaccggaagttccgcatcttcttccgacgcgatgaagtcatcagccagatcagcgaaacctatgcagacgttcccgaaggcaccaagctcgccctattcaacgctgccggctacctggaaatagccatcaacaaaggaaatgccgccggcctattcggcctgcaaggcttccgccgcgaccagctcacacagccagccgggtaccagcaactgtcatactaccaaactgttagaataatttttcaatgattaaccgtatcgttaaaatggaattcgacccgggaaaagtaaacaccttccgggaactctttgccaaacaacaggaactcatccgccacttccccggatgcctccacctcgaactgtgggaacacgccgcctccggaaatacctggttcaccttcagccagtgggaatctgaaacggcactcgaaaagtaccggcaatcccccctcttccgggaaacctgggccgccaccaaagcgcttttcaatgcaaaacctgccgcctggaccgtccaaactgccgtgagcctgtaaccaacagcgcctgatcattgaattataatgcttttttaatctcccggaaaactcccttccggcgcccggatgcggctagccaaaagggtaacagctaaaaagatatttacaaaaagttaaaactgttcgccagattagcataatttgctgttttttatatttttgtcggaccttaaaacaaccttatgaattttaaaaggaccaacaacatggtcggctgggtcatttgcatcatcgcctgctttgtttacattaaaacgatggaagctacaggcagcttgtgggactgcggcgagtttatttcaagtgcttacaaagtacagattccccatccgcccggagcgccattgttcgtgttgcttggaagattgtttagtatgttcctgaaaccatctcaggccgccctgggcgtaaataccatgacagccctggccagtggtttcactatcctgttcctgttctggaccatcacccacttcgcacgcagactcatggtgaaagccggtgaagagatctcacgtgaaaaaatgatcgctatcatgggcgcaggcgccgtaggcgctttagcatacaccttctccgattcattctggttttccgccgtggaaggtgaagtatatggtatgtcctccttctttaccgccatcgttttctgggccatcctgaaatgggaacatgaagccgatgaaccctatgccgaccgctggatcgtccttatcgggtacctcctcggcctctctatcggtgtccatctgctcaacctcctcaccatccccgctatggtaatggtgtactacttcagacgctttaaagtaaccggctggggaaccttctgggccttcgttatcggttgcggcgtcaccggcctggtacagaaataccttatccaggataccgtaaaggcctccggatatatggacgttttcttcgtaaatagcctcggaatgggatatttctccggatttaccttctatttcgtactcatcatagccttgctggtaatcggttaccagaagccaaagttcggtatctacgcccccttcatcgtaatcgctaccatcatcctggtacccgcgtttaacgaggcaggctccggtgccatcttcttcaaattcctgctggccgctttctttatagccatcccatacctgctgaaagcagtaggcgtgaaaatggatatatccagaacagcacacttcagccggctcaccatctccttcgtgctgttcatgctcgtaggatactctacttatattaccaccatggtacgctctactgccaatccttcagtagatatgtacaacgtagataaccccatctccctggtaggttacctcggtcgtgaacaatacggcgacttcccgctggtatacggccaggtgttcactgcccgcccaacaggttacaaagaaggcggtaacatctacgcacgcggtgcaaaaaaatatgaaatcgccggcaagaaaatggaaccggaatatgacccggctgatatgatgctctttccacgtgtttgggacgccagcaacgatcagggccacgccgattactaccgcacctggctgggcctccagcaaggtgaaagaccaggatttggcgataacctcaaattcttcctgcaataccaggtgaacttcatgtatgcccgctacttcctctggaactttgcaggtaaacaaaacgatacacaaggctacggcaacgtacgtgacggtaactggatctcaggcattccgttcatcgataacttcttatatggcgaccagtccatgataccggacagtctgaaaaataacaaggctcacaacaccctgttcttcctgccatttattctcggggtcatcggtttcttctatcaatataataatcaccgtaaagataccctcatcgtatctctcctgttcttcttcacaggcttcgctatcgtcatctacctcaaccaggccggtaaccagccgcgtgaacgtgactacgcctacgtaggctccttctacgcatttgctatctggatcggtttaggcgtactgtcggtatacagcttcctgaaaaagaggatcaaaagcgccatcacccccgtattggctacagctatctgcctgctcgccgtaccggtattaatggccttccaggaatgggacgaccatgaccgctccactaaatacgtagccagggatgtggccaaagattacctggaatcctgtcagaaaaatgcgatcctgttcaccgtcggagataacgatacctatcccctctggtacgcacaggaagtagaaggcatccgccccgatatcagggtgatcaacctcagcctcctcggggtcgactggtacatcgatcagatgcgcagagccgtaaaccaaagccctgccatcccaatgacctggtctgccgataaatataaaggtgaaaaccgcaactatatccgcttcttcgatccgggaaatattcctgccgacaaatactttaacctgaaagaaatcatgaacttcatgggaagcgatgatgtaaacagtaaagtaaccacgcaggacggcggcgcagaaaacttcctgcctacccgtcagctgtttattccggtcgacaaacaaacgattcttgccaacggcgtagtagcggcgaaagacagtgcgaagatcctgccttccatgcctttcaaaatcaccaaaagctacctgctgaaaaacgacctcgcagtatatgatatcatcgctgccaacgactggaaacggcctatctatttcaccagccctaccgatcttggcctgaatgaatacatgcaaaccgatggtcttacctaccacctggtgcctttgcctaaagctacatctaccgatccgctgggcatggacatcaacgcgaacgtaggcgtgatgtatgataacctgatgcacaaatttgaattcggtggcgctcaaacacgcggtacctacttcgatgagcccaacaggaaaatgatcatgtacctccgtcaggcatttaccaaactgtctgtagccatgacgcaggaaggcgcctctaaagacagcgccctcaacgtgctccgctacatggacaaaaacataatggaaaccaacttcccttatgccatgaccactccgggtaacatgcacaactatacttctattcaaaccatctacgcctactatatggccggtgatgcgaaaagagcagaagaactgtcgaaccaggtgatcaaagactgtgagcagcaactgcgctactacagctcactgccgccaaacagaatgaccaacgacttacaacgcgatggccagaatgcacaacagttcatcacctggttaaaccagatgaaaggcgagtttggccctaatggtaccaaaagaaacaaagacggcgccggcgccatacaagtaaatacggaagattctacaccggtgccaaagccggctgattcagcgaagtaaccgtacttccggatataaaaaagagagcccgtaccaatggtacgggctctcttttttatcaatataattactctgctcttaaactcttaaccgggttggccaaggcagctctgatggccttataccctaccgctatccacgcaattaacacggacaatacaatagccaatacaaaaatgccccagcccatgtctatatgatagtggaaaccaagtaaccacttcttcataaaataatatcccaccggagctgccaccaggaatgcaatacctattaacgtggtaaactccctggaaaacaggtacaatatactttgtacagaagcccccagtactttacggatacctacctctttggttttctgtactaccataaaagaaaccagcccatataatccaagacaggaaataaaaatggccaggaaggcaaataccttgaacaacgctgcagtaatggcttcagccctgtagaagttccctatctggtcatcaaaaaaagtacaatcataaatgtaagtaggatatacggcagtgaatatctgctctacctgctttaacgtagcaggtactttttcaggatccagccggagtgccagcgtgccataatcattattatcagacgaaattacagatggtgaaatctcatctctcagtgaattattattaaaatcgcgtaatacgcccgccaccgggaatttacgggagccgttatcaaccgcaactatcttcccgataatatcctctgcagaacgcaatcccagttttctgaccaccgtttcatttaccagtacttcccttgtgctatcatcggaaaatggataacgtcctgccaccaggcccaaacggaaggtattgaaataaccggtatcggcattgatccgcttcacgctgtaaggctgcctcttagcttcgttattataatagaaatcggtgaaccgtccgaaatgggaagatggctctatagagcataaactgcccgcttctactccaggcagctgcaaaagccgcgatttcaaatgggaatattttagtcttaaagtactatcgctgggcaggtcaagcaacaccaccgcttccttttcaaagcccatgggtttttccctgaaatacttcatttgctttaccaccaccagcgtgcctattaccagcaactgcgctaccacaaactggaacaccactaaagcccggcgtaaggaaataccgtttgctggccggatgctgatcctgctcttaatagcagccaccgggttgaatcccgagagcacaatagcagggtaaaaaccagccaggaaagtaacgatcacgccggataatactaaaaagagtaatatcgacggatggcgcagcgggttcaactccagcgtttttcctaccaggttgctcaggtaaggaatagccagccaggccattatgctgcccaatatgatggcggaagccgtgatcagggcagtttctcccaggaactgttttaataactggagacggttactgcccagtacttttctgataccaatttctttggccctgttaaccgattgtgctgtagccaggttaatgaagttgatacaggccaccattaacaggaacagaccgatgatagccaacgcccatagttctgtggccgacagggagtcgtcttttacggtagcataacgtttgtcgagatgcatttccttcagcggctgaaaagtcaggctgctaaagcctgttgtctgattcacatcttcccggtaattatttttcacaaacgccggcagttgcgcctgcagcttgcctatatcatctttcggggaggtgagcgcaaaacattgtgttccgccactaagcgagcgccagtcttcccgcgtctgacgttcatgatcgtccatcctgagccaggtagcatgagatgctgccatacgtaccggcagatctgtattatatggcaggtctttaaaaacgccggtcacacgcagtggcacgcggtaagaccatagttgtattattttgccaatggcgtttttatagttgccaaaataggcctcagccatactttgcgtaagcgccacggtattcggttcttttaactccgctgcacttccatagagccaggtaaaatcgaatatgtcgaaaagagctggttctacaaaaaagagtcccccgctttctttaaattttttctcttcgccgccgttttcccccggaacatatacctgtgcgccgccgatatattcagcaaccgctactttttcaagggaaggaaaatcccgtcgcatggcagatgccagcggcgccggcaccatactatgcctccacttttcaccggtgctgcggttggtgaaagtggtcactacccggaaaattctttcgcgcttactttgataagtatcataactcatttcgttgcggatcacgaggaagatcagcaggctggcgccgatgcccacggccaaccctacgatattgagcagggagaaagatttctttctccaaagagttctgaatgacaatttgaagtaactattaatcataacaggaagtattgccgctttgcctgcaaaaaccgggacaggaatatatttgtttaattttcaaagagatataaaaaaaagaagcagtgcgaatgttcagtaaagaacagggaatgtccggtatcgaacatccataaaaaaatccggagatcccggccaggccgttatctccggatcaattgtccgtaagaacaataatttattacaggttgcttacaatcgttctccagaatgcagcgctggccttcacttcaggaacattgttatcccagttgtattcgtattccgcagaaaacaaacctttgaacttctgatttttcaatgtttccagcactttcggcatctggcaaacaccgttaccccaaactacatcatgggaatcagcagatttgttgttcagatctttgaaatgcaggcttacaatatgaccatccagctttttgatacattctaccggatcgaggcctgagcgtacccagtgaccaatatccgcacaggcgcccattaatttacttctgcctttgatcgcttccagtaccgtttcagggttccagtaacggctcggtttcgggtgatcatgtatcgccagcttaatctggtactgatcacacagggaagagatcaggtccaggtcttccggcttgggctcagaagtaatgctctggatacccatcctgttggcaaaatcaaacagcatacgccattcggcagccgattccggcactaccacgccaaatgcctgcagcaccttgtgctttttcttaaacaacgcctttacttcttcctgtttggaaggcgacatatggtaatcaaatttaccttctataccaccgccaatcacttgtccgggaaatgcttccacgtactggataccacagctgtccattttatccagcgcctccgccagcgtaaaatgattgaatgtccacgcctgcgctcccagcttccatcccaatgcatctgccctgctctgggcaactgccgattttgcaaataatgcaaccgccaggccacctgccaggatcaacgcatttctcagttttttcatatagctatttttttgatgattgaaagtaattggtttcaatctaaaatgcaagttttaagcgaagaaaaatccgcggaggatcgccttcggcgatttttaaattgtcttactgcctgattacgctgattatactgatcaggatgatttgattatgttttgattataatgaattttataaaggatgaaggaatatataagcggatatcagcttttatctctcctgattattattaatcataaaaaaaatcaaaacataatcaaatcatcctaatcagtataatcagcgtaatcaggcagtaagacaatttaaaaatcgccgaaggcgattctccgcgaaaagtggtaaatttaattcagaagatgagctaagctatgagaggaatacaatttaccaggttcaacccggacgagaacaaaaaaccacctttccagaaattactggacctttttacccaactccttacctacaccagcggagacgtgtcagaagccctgcaatggctcactgagctggacaacgaatataatctcaccaaccaggaatatggtatcggcgattttatacaggagttgaaagataaaggatacatccgcgaaaacgaggaaagcggcgccatagaaattacttccaaagcagaacaaaccatccgtaaaaacgcattggaagaaatcttcggtaaactgaaaaaatcagctaccggcaatcataatgtccgcaaatcaggcatgggcgacgagctcaatgccgaaacacgccccttcgaatttggcgatggcgtggatcagctggatattaccgcctccatccgtaacgcacagatcaatcacggtatagacagtttctctatcagccaggacgacctggaagtaaaagaaaccgacttcaaaacacaaacgtcaaccgccctgatgatcgatatctcccattccatgatcctttacggggaagacaggatcacgcccgcaaaaaaagtggccatggccctggcagaactgatcaccacccgctacccgaaggataccctcgacatcattgtgtttggaaatgatgcctggcagatagaaatcaaagaccttccctatctgcaggtcggcccttttcataccaataccgtagcaggactggaactggccatggacctgctccgccgcaggcgcaacccgaacaaacagatctttatgatcacagatggaaaacccacctgcctgaaaataggatcacagtattataaaaacagctttggcctcgacaggaaaatactcaaccgtaccctcaacctggccgcccaatgcaaaaagctgaaaattcccatcaccacctttatggtagccaccgatccgtggctccagaagttcgtaacagaatttaccgaaaccaacaacggtaaagcattcttttccggcaccgataaactgggacagtttcttttccgtgacttcgaaagcggcaaaagaaagttttattaatagtaaacagcagcatagacaaaaaacggatccccgcatccgccaacagctactgccaatttgtaatgcgtaattattaaagatgaacacaaacataaaaacactaggcgaactcaaaaaaagcggctataaaccagtttccgtaaaagaagaaatcaggcgtaacctgatcagaaaattaaaagaaaaggaaagcactttccccggcatcatcggctatgaagacacggtgatccccgataccgaaagagccctcctgtcaagacataatatcctcttcctcggtttacgcggccaggccaaaacacgcatggcccgccagatgaccgatctcctggatgaatatattcccgtagtggaaggatctgaagtaaatgatgatcccttccacccgctctcccgctacgcaaaagacctgatcgccgaaaaaggcgaccagacgcccatcacgtggcttcacagcagcgcacggtacggcgaaaagctggctacaccagacgtttccgttgccgacctcgtaggcgatatagaccctatcaaagccgctaacctcaaacttagctacgcagatgaaagagtgatccacttcgggatcatcccccggtcaaaccgcggcatcttcgtcatcaacgaactacccgacctccaggcacgtatacaggtatccctgtttaatatcctccaggaaggcgatatacagatcaggggcttcaaagtgagaatgccgctcgatatcctgtttatcttcaccgctaacccggaagactatacgaaccgcggttctattgtaacgccgctgaaagacaggatcgaaagccagatcattacccactacccgaaaacaatagaaaattccctgctcatcacagaacaggaagccgatatccacgaagatcagcaagccaaagtacaaatcgccgatatggtaaaacgccttatcgaacaggtgtcctttgaagcccgctccagcgaatacgttgacaagaaaagcggtgtttccgcccgcttaaccatcgccgcctacgaaaacgcggtgagcgccggcgaacgccgcgccatcatcaacaaggaaaaggaaacacaggtgcgcatcgccgatctgcaggccatcatccctgctatcaccggcaaaatagagttggtatacgaaggcgaacaggaaggcccgctccaggtagcccataacctgctcgacaaagccatccgtaccctcttcgccatctacttccccaacccggattccttcaagaaaaagaaagccggcgcacctgctgaaaatccctaccgcagcgttatccagtggttcgataaaggcaattccgttcagctcctgcaggatatcagcgacaaacaatacgacgctaccctcagcaaagtagacggactgaaagaactcatcaaagcccgcttcccgaaagccaacagcaaagaagccctgctgctcatggaattcgtgctgcacggcctgtcgtcctactcactcatcagcaaaaaagtggtggaaaacgaaacccgcttcagcgacctgctgggcaccatgatgaacttcagcctcggcggcgaaagcggcgagccggaggaggagtaatcgccgcgaattttgtcttggctcaggattacgctgattttactgattacctggatttttacttttggattttataaatgattaagggagatagaagcggatatattcgcttttaactcccctaattattattttaataaaatcaaaaaaatcaaaaaaaatcaaaaaagtaaaaatccagttaatcagtaaaatcagcgtaatcctgagccaagacaaaattcgcgtggaaggcgataaactccacttttttccctattttgtatttttaattgtcattttaacaattccacattccacaaaacgttttattacatgaataactcccgtagaaactttatcaaatccgcctccaccctggtggcaggagcaggattggtgtctgcactgccagccggactgcaggcattcccattgcggacagtagccgccagcgaccggctcaatatcgccgccatcggtattaacggtatgggatgggccgacctcacctccatgctgaaaaaccctgccgcacaatgcgttgccctctgcgacgtagataaaaacgtgctggataaacgggttgccgagctcgcacagaaaggcatcaaggtaaaagcctacagcgattaccgcaagctcctggaagacaaaaatatcgacgccgttgttatcggtacacccgaccactggcactgcctgcaaatgacagacgcctgcgccgccggcaaagatgtatatgtagaaaaacccatgggcaactccatcatagagtgccgctctatggtaggcgcccaacagaaatataaccgcgccgtacaggtgggtcaatggcaacgcagccaaaaacactttcaggacgccatcgagtttgtacactccggcaaactgggcaaagtacgcctggtaaaagcatgggcctatatgggctggatgaagtccatccctgtaaaaccagacggcaccccgcccgaaggtgtggattataaagcctggctggggccggccactacccggccttttaaccccaaccgcttccatttcaacttccgctggtattgggattatgcgggcggcctgatgaccgactggggcgtgcatctcctcgactatgccctgctgggtatgaaatccggcgcaccaaaatccatcatggccgcaggcggtaagttcgcctaccccgatgatgccgccgaaacaccggatacacttaccaccgtttatgaattcgatgactataacatccagtgggaacaagctataggcatcgatggcggcccttacggacgcgatcacggtattgccttcatcggcaacaacggtacactggtgctggaccgcggcggatgggaagtaatccccgaaaaaggaaaaatggaagccgtaccacgtcaaaaatccgtcgataacggcctcgacctccataccaccaatttcgtggaagtagtgaagtccaggaaactcgacgacctccacgcctccgtacaggtgggctccctcgtagccaccaccgcacaaatgggtaatatcgcctatcgcacaggtaaaaaagtatactgggatcagcaaacaggtaaatttaccgacagcgatgccaataaactgttagcagcccaataccataacgggtaccatctgcctaacgttaccgcctgaacgaaaacacatatttaaatatcatctacctaacaaaaataaaaagacacatgcgtacgctactgctatctgcctgtaccctgctcgccgttaccgcaacagcgcaaaacaaagagcagataaaacccgaagccacggaagtatgggagccggtaccaaaagtaattacacccggtactgaaacccttacggcgccatcagatgcgatcatactgtttgatggcaaaaacctcgacagctgggaatcagaaaagggaggacccgcaaaatgggaggtgaaagatgatgctatgacagttgtaaaaggaggtggtgttattaaaacaaaggaacagtttgaagacttccagctgcatatcgaatggcgcacccctgctgaagtaaaaggcgaaagccagggccgcggcaacagcggtgtatttatgcaggaacaatacgaactgcaggtattggataactataacaaccgcacctattccaacgggcaggccggcagcttttacaaacaaaaaattccgctggtaaatgcctgtaaaaaaccaggcgaatggcaaacctatgatgtaatctggaccgctccccgctttaacggcgacggttccctgaaatctcctgcaagagccactgtactgcaaaatggcgtactggtgcagaataatgtggagctggaaggcaaaacagaatatatcggcaaaccaacctatgtaaaacacggtgccaaatccatcgcactgcaggatcatggaaatccggtaagcttcaggaatatctggataagacccctgtaagctatcatccttttatatgttatgcagcggaggaaaatcctccgctgcattttttttaagttaaactgtcctcttcaatattgagcgataaatacactgcgtcgctgatcggattatcataatacgctgcgatcggctgaaatccgagtgaggtatacaaatcaattgcaggacgcatatgcgctaatgtatccagcaggatccgcttgtatccaagctcccggctctctgcaatggcggcactggccagggcctttcctacgccgtgtcctttaaatgcatcctttacgaaaagacgcttcatttctgcggtactgttgtcgaatgaccgcacggccacacatccggccagctgtccatctaccaatgcaaggaacaatgcgccggttggaggcacatacacacccggcaggttcgccagctcatcttcaaattgttgaaaactaagatctacatttagccaattggcatattcgcggaaaagcagcttcacctggttaaggtgcttggaatcttcggcggttactttaataatctctgtcataaccacttctttttaatgtatataaaacgcaacaagccttctgcatgcagaaggcttgttgaccggaaaatgatggcagctccatattttaatagaaaatgccgccgatatctttattatcaattacacacgctgtgtttagatagctatagtaaattattgataaatctcttgccttctgataacctcacctgcctcttgcggggtatgcaatataatcttttgaattgatatttcaacacacttggcattatttctttttcacccctgaagtcagccagcagcgggcatcttcgcttcaaacacacctatacttcccagatacccccgtattccatcagccactgtggcacataatatgccggttgccattacaaaaatctattacagttttaccggaaatgaaaaagccgcggtgtacgcggctttaagaaagagatatgtggaggttccgagcggattcgaaccgctgtacgaggttttgcagacctctgcctagccactcggccacggaaccatcagtttcaaaatgttcgccgtaagtcccccactggcgtacatctcattcattttgtgggattgcaaaagtagtgaatttctaacaaccaccaaatattatttaaaaaatatctgaaaaaatattttgataatatagcagaacaaaggaatattgacactggaaatgttgatttgcgaataataaaaattagtacaatggataaccgtattgcagaatcagaactgatcatcaacaaccgcggagccgtatatcatcttgatgtaagaccggatgaactggcccataccatcatcaccgtaggcgaccctgaccgtgtaggcgcagtaagcaaacactttgataaaatagaaggcaaataccagcaccgtgaatttgtaacacataccggctatatcggcaacaaacgcctctccgtagtttctaccggcattggcaccgataatatcgatatcgtgctcaatgaactggacgcactcgtaaatatagattttgaaacacgccaggtgaaatcaaccctcacctccctgcaaatcatccgcctcggtacttccggcgccctgcaggaaaacataccggtggatagtttcgtggtatcctcgcatggcctgggcctcgacaacctcatgaactattacgtgtttgaaaataccaacgcagaaaagcagctgatggagtcgttccgcggacaggtattcctgcagcccggcggcgccaacccctgcctctttgaagcatctgcaaaattacaggaacatttcacagatggttttcatacaggcatcaccgttacctgccccggtttctacgcaccgcagggccgcgtactccgtggcgccctgtctaatccaaacctgatcgataaactcaccagcttcagctacgagcaccaccacatcactaacttcgaaatggaaacctctgccatctatggcatgggccgcgtactcggacacgaatgcctttccataagcgccatcgttgccaaccgcatccgccaggaattcagtaaagatggcggcgcagcagtggccgccctggtcgaaaaaggactgggcatcgttgccgccatttaacagtgcggattttgtctgaagcactgattacgctgattttactgattttactttttggatttttttggattttcagatttaataataaataagggagataaaagcgaatatatccgctgctatctcccttaatcctttataaaatccaaaagtaaaaatcaaactaatcagtataatcagcgtaatcctgagaaagacaaaatccgcgcatcggttaattttttatctttgtacccatgaacaaaatccacttctataaatatcagggaaccggtaatgactttgtcattatggataaccgggacggacaatacgactggctgacagacgaacaggtgaatgaactatgcgaccgccgcttcggtattggcgcagatggcctgatgctgctcaataaaagcgaggactacgacttcgccatgaaatattacaacgccgatggccgcgaaggaaccatgtgcggtaatggcggcagatgcctcgcggctttcgcccacaaaatgggcgtaggcgacggtaacctctatttcatcgcagtggatggcgaacatcaggctaccatggacggtaacaattgggtaaacctgaaaatgcaggatgtagatgatgtggaacatggccccctctactactacctcaataccggctcaccacattttgtaaaatttgtggaagatgtacaggcagtagatgtgtttaacgaaggccgcggcatccgttacaacgaccgcttcgcagcagaaggtaccaacgtgaactttgtacagaaatttgaaagcgggatatttgtccgcacctacgaaagaggcgtggaagatgaaacctactcctgcggcaccggcgtaaccgccgccgcacttacttttgccggcacagaaacaaaggaatacacagtgccggtacaaactttaggcggacaactggaagtacgctttaccaaaaccggtgaacgcacttttgaaaacatctggctctgtggccccgccacactggtgtttgaaggggaaatccaggtaaggtaatatcacttgttccggagtaaaagattctttacaaatcctccccacaccttaaacaggttataaggaattaagtgagcagggcaggataacaaaataaaagaggaaaaataaacaggattaccggtggctctcttcgaaaatattttcttaagatattttcgaagagatttttcttttaaaccatgaataccagtggtttcttcattcattaatattttgactgtttcatcactggctaatctaagccccctccttcttgcccgtatagtaaattcataatccgatccgtaatgcggaagcaacaatggcctgaaacctcctgtcttcataaagctgccaacagtcataaatagccctcgggtagaaagacaattgatctcttccacacaggttgcctgatcaaaagtcatcttacgccagtctgccaatacgccaaggtcaatcaacttaccggattgcttaccatatgcctgcgataataacaacgtatccggaacacgggtgataagctcaactcctttctgcaaataatcaggttcaaattcaacatcatcattctcaatcagcaccacagcatttttctccgttacatactttttgatccagttatatccctgctgcaggcttcctccccaccaccaatcgccggtacccgtaagaatggtggcatccggcaaataagatctcaccatttcagcggttccatcaaccgatccatcgtcaaccagaataagatgataatgctgataggtttgtttaagcagacagagaataaaggtccgggtgatctctttcctgttatgaacaggcaggataatataaactctcggattcattcactacagaggtttctttaaaaaatagataatattatcgccggcattaaatgcatcaaataagcgggtgatcaggtaattgatcttcaaacgatggaagcctgccaatatcttcataataatacgttgtgaagtagttcgctctgcaaagctctgcgtccaaaataccgatttttctccctgtttgggatacacagccatatgtaaccattggtaatgcagccactctgaattggtgatggtaatcgacttttccagtacaagccccgcctctgcagcatatttcttcattgatttcctggagaaaatatgaagatggtagggaatatgccagtgcgcccactttttgccaaacaccggaataccccagcctttgccgttcggtgtggtaagaatcgctgtgccacccggtttcagtatcttttcgatgcctttaagggataccagcggatcaatgacatgttctattacctggtccatggtaacataatcgaaatagtttggctgataatcatccgcatcaaacagccctacctttacattaaacccgaatttatctcctacccgtttaatgttttcatctgcctctacaccatacacttcacatccacggctttggtgataaccaagggtttcgccaaaaccgcaaccaatatccaatatcctcacattctccggcacccagttataagcggtactccgtaaacctttaaaccaggccataaaccctgctgcttttttatacggctgccattcttccagcgacatatgtgtcctgggatagtagttggaatacaggtcgccaatcatagccggcgtaaagtctgctgccagtgaaagatgatcacagttcctgcattgccacatcgtataacttccaggataaccataccggttgtcaaacatatccttataaaatacatccagtggattgccgcaatatttacaattcatacaagtctctttttgtaatcgcctaatgcgaaaaataaacttttatctttactttttcctgcccagcttcttaaagaaagtagctgccgtactgttgatatcatcagaaacacgccatgccagggttcccaatataaaaatagctgagaaaaagacgcttcttaaaataatatcaataaccggctgagccatatgtggaagccaggcaaccgcccagtaagcggcgattgccactaccagcgccttcaacgtttgaatagtaaacggttgcagtccaaattttttccatataaatacacaacggatcgtgttaaatacaaacattgacaataaggccgcatatcctgatcccagcaggccatagttacgtatcaacaggtagttcagcggaatagacaacgtcaccagcaccattgagctgataaggtcgaaacgccataatctcgaagtactcagcaactggctgttcaccccggtgccaaggtctattatttttgacaccccaagataaaaaaagacatacttaccaacggcatattcgggcggcaacaaccggaaaaacgggtcaatgctcagccatatacccagaaatatatacatagccgctatcagttgtaataaggaagatttccggtaaatttccaggatcttatccatatcttttcctacccatgcttcggccagcacaggaagcgctatggcagaaatactacgctgcggtacctgtatcaaagtggccatgtacatggcaatgctgaggtatgccacattcttgagaccgttagtactggaaatgatcaacggggcaatattgttcgccaacagggtgaaggaagtagccagcaacagcgacaaagaatatgcactcatcggccggaacaattttttcgtcacaaaactcacccggaagttcagatgcagcaggtgatttcgccggaggtaccccagaagtaccaggagaaccactccccagatcaggttaaataaccagaggaattgaacaaaactgagtatcttaaatatataaagtaccaccagcaggctggtggccacacgtactaccagctcttttagaaagttgggcatcaccgtttcatgcctggaccagctgtagttctctatgatggcaaaaaaagaataacaaaacatgaaaggataaaggaggtaaaagtactccaggaacatcggcgcattcttcgaatacttccggaaaatcaggtcctggaaaaccacagtaccaagtacaaacaacaagtatcccgccagagtggctaaaagtacccagctcaacatgtcatttttcttgtcgtccagcctcgaactgtaataagggtagaaacggttcattgtagggcccatacttaatgtgcagaaaggcaccattataaccccaatatccaggaaaaggcgtgttaatgcgaattggtcgtctgtaaaaaaatgcggaaaaaggaacaaagtattgattcctccaatggcaaacccgagatagataagtaccgtagatataatactttgctttttaattactcccatttaaatattgacatgatatgaatataaacttcaggtcacaatattacattaaaagccaacacgattcaacattttaactacctttgcgcccgatgatccagtattttacaaatatagattccaaaactgtagaaatacaccagccggaaaacggcgcctgggtaaatattaccccgccgcttaaacaggccgaatttgaacagttatccgaggaactcgatattcccctggacttcctcacagattccctcgatattgacgaaaaatccaggtttgagctggaagacaatgtaaagctcattgtcctgaaaacgccgaccgaaaacaattcgatcaatgaaagtgaagcctattacattaccattcccatcgtaattatcctgacccaccaccagatcattacggtaaattctttcgacaataccgctatcaaaaagttcctgaatacttttcataaccgctctcccgaaaaaaggaatatgatggtcctgaaaatatttgagaaagtggtgatcaatttccttgattacctgaaggaaattaaccagcgcaggaacatgctggaagctaaactatatgattccaaccggaacgaggaactgctgggtatcatgcgtatccagaaaagcctggtgtactttgtaaccgcgctgcgcagtaatgagctgctgctcatgaaactggaacggactaacttcctgggactgaacgaagatgaaaaagaattcctgcaggatctgatcgtagatacctcccaggccctggaaatggccaacgtatatacgaatatcctcagcagcaccatggatgcctttgccagcatcatctccaataacctcaacgtggtgatgaagcggctcacctccattaccatcatccttacattccccatgctggtggccagtatctatggcatgaacgtggatatcccgtatcagcatacccttcatgccttctatataccggttatcttgtctatcgctatttctgtagtcatcagctggtattttatgaagaagaaatggttttaagcccttttaattaagcatatgcaaacaggatttaacgtaagagtatacggcatcatgatcaacgatcagaagcaggtgctggtgagcgatgaatatatccgtgggggttattataccaaattccccggcggtggcctggaattcggggaaggcaccctggagtgcattgtacgcgaatggcaggaggaactgggccaggatgtaaaagtggtagaacatatttataccaccgacttcttccagatctcagcgttcgacaacgttacgcagatcatctctatttactacctcgtaacgccactgtcgccgtttacggcatccgtaagcaccaccccgttcgactttaccataccggaaggcgtggaagaagtggaacgcgcccgctggatcagctgggacgacttttcatcagcagccgttaccctgcccatcgataaggtggtggccgacctggtaaaagcaaaatattaaaaagagaaaggggctgtttgatcaaacaacccctttctctttatcagtcgttcgtaacaggttcttcaaacggttgctcctttcccatcgccgccgccttcatctgcttagcggtatcatgccccaggtaacgctctattcggtgttctatcaaatagatcagcggcgtgagcactaccgccaccacaaacttatagctgtagttcaccaggcatatagccagtacccgctgccagctccagtcgttacccagcttaaaggcgatatacagtacaataaaactgtctaccagctgcgatacaatggtggaacccgtagccctcagccatacatgcttttcgccggtacgttttttaattttatggaacacggtcacatccacgatctggctcacgaggaaagccgttaagctaccgagtatgatccacatgccctgcccaaaaatactggtgaaggcattctgcatgtcgggaatacccgcatctgcccggctgcctttccaccagccatctgcaggtacgctcatggctacccaaaacataataaacgcataggagatcaaccccaccgcgatataggaaatacggcgcaccgctttcggcccaaaatattcattgacaatatccgtcatcacaaactccagtggccataacaacacccctgccgttaaggtatacgccaatccgctttcgccaaaaagggtgaaagtatgcacgggcaatcccagtaacttctccagggaaaacagcttaccgccaatacattctgcaatcagcgcattggccacaaagaagctggtaaatatcacgaacagtttagtgggcttatcgtttaacagatttctgagcattagtaattaactataagttgaaatataaggatagcaatattgaacaaatataaccagggtggcaatgttttccattgtattttttttaacaataataacacgcccgtcagcacacacaaaacggcattcagcggaaaagcaatgcctacacccaataccagtatgtgattcactacgttatcaaaagaatgatcataagccgtgatgcgcaggatttcactggttatgaagcacagattgcatataaatgcaaattttaagaggaaccggatccagcgcatattgaaatttcggataaattacagttatttttgtttctttaaaactaaatccaaaatatccgatgaagcaaaactggctaaaagccattcttccacatgttgcagcaatagggatcttcctcctgctggcatttgtgtattgcgctcctgtccttgaaggcaaggtggtgaatcagagcgacatgaagaatgtaaaaggaatggcgaaagaggcaaaggactattatgaagcaaccggcgaacgtccgttatggaccaacagtatgttctccggtatgccctcctatgtgatatttacaggtcccggcgccaataaaatagcgtacatgaacagagttgtgacgctgaatacgccggatcccgttaatatgctgtttctggccatgatatccatgtacctgctcctctgtatattggacttcaaatactggatcagggtaatgggcgccattgcatttgctttctgctcctataatgtgatcctcattgatgtaggtcacgttaccaagatgtacgacattgccctgatgcccgcggtactcgcaggcattgtcctcacctaccgtggccgcctgctcaccggcgctgcgttaaccgccctggccacagccatgctggtttataataaccacctgcaaatcatttactacacactgatcatggtgttttgcctggccgtgtgtgcatttatacattttttccgggagaaacaactgctccagttcttcaaagcttcggccttactggccgtggctggtatattggcggtgcttacttctatggacagtctcatgatcctgcgtgaatacaccgactacaccatgcgtggcagcaaatcggaacttacgctggataaagatgatgtaaaccagaagaagtctaccggcctggatatcgattacgcatacgactggagctatggtaaagcagaatcaggaacgctcctgatacccggatacgtgggtaactcctccggccagaagctgaaagtaagctccaactttggccagcaaatgattagccttggcgccgcagaaccacaggtagaacagttcctgagccagcagaaattaccactctattacggcgcccagtcgaaaggcacttccggacccgtatacgtaggcgctatcatctgcttccttttcgtattatcgttactgttagtgaagagctggcataaatggtggctgattgctataacggttatcggcttcatactggcatggggtaaaaacatggcgttcatcaatgatccgctgttttactaccttccgctgtataataaattccgcgcacctgcgcaggcgctggtattgccgtcactcacctttgtggtgctggcctgctggggcttgcaggaaattgccaatggcaagcataccaccaaagaattattgaaaaaactgaaagagtcggcgctgatcaccggcgcatgtatccttggctttattctcatcagctatttcttcgtaggcttcaaatctgccagcgatgaaggcatgctgcaatatttcgcccaaatgatgggtggcgaggaaaacggtaaactgctcatccgcgcgttggagaaagaccgcgccagcctgttgcttacagatgcgttccgctccgtgttcttcatcctcgtggctgcaggtgctatctgggctttcctgctgaataaaatgaagtggcaggtatcagcgatcatcatcaccgcagccgttaccatcgacctgtggcaggtagataaaaactacctcggcagcgacagtttcgtggatgatatgagctatatgcaggacctgcagccatccgctgccgaccttcagatcaaacaggacccggacccatactaccgcgtgttcaatcttactacttctccgtttgatgatgcgtctccttcttacttccacaaaaacatcggtggctacagccccgcgaaattgtgggtttaccaggatctcatctcccaccagattgccaaaaacaatatgcatgtgctgaacatgctcaacacaaaatactttatcgttccggatcagaaaacaggtcagccggtagcacaacgcaaccccgacgcctatggcaacgcatggtttgtacgtgatatcgtatgggcgcccgatgccaatacagaaatgaaaacgctggacgcgctgaacacccgcgactccgcagtgatcgataaacggtttgaaaagcaattgggcagcttcaggccaggcgctgatagcaccgctgccatcaaactcaccaaatacggcctgaataaactggaatatacctcccgtaacagccaggaaggtttcggcgtgttctccgaaatatactaccccgccggatggaacgcatttatcgatggtaaacccaccgatattatccgtaccaactacgcactacgcggactgaaaatacccgccggagagcataaaatagaaatgaaatttgagccaaaaacttacttcaccggcctcaggatcgcaggtatttcttcttcgatcctcttactgctggtagtactgctgtttggctgggagttttttcagcaaacaaaggacgccaaagtaaaaaaataatgtaccggatcacaaataaccgggataaaaaaagaggtgccgctgtaatagcggcacctctttttttatcccggtttcctttagtatctcttcgaaaaaatataccgcaatccaataaacaagtgatgcgcaaaattaggcagatgcccgtagtatttgctcaatatccggtaacgttccttccaggcccgctgctggtgctgcttggaagtgccccccaccctgaacctggccactaccaggtgcgtattacatactttacgcgatgccttcaacgtgcggatcatccagtcgatatccgcgcaaacccggtattgcaaatcgtataacgggctcaaactgcggcggatcacataggcctggtgcgatactaccatgccatgtttcaggctcttccaggtgagctgttccggtacgcggtgtggtgtctgctcagatctcagccctatatcctgcccgttctcatccataaacatggcctctccgtaatacacatccgcatcttcacaggcagcgaacattttctccaccacatctggcgccgccagtacatcatcggcattaaggaacaacaggtagccccctgtagcaagttgcatgcctttattcatcgcatcatacaaaccattgtctttttcagagatcacggtagcaatacgggagcggtatttttcaatcacgctcatcgtattatcgcgtgaagcaccgtccacgatgatgtattcaatatgcgggtatgtttgcgccagcacactctgaatggtattctcaataaattttccggcattaaaacaaaccgtaatgatgcttaataccggtgaagaggctttgttcatgtatctgattattgcgggttcctaaccacggattgaaacaggtgatagtactgcccggctactactttcattccaaaatactgttctgtaaatgttctggccgctttaccaaactgccggcaaatatccgggtggttcagcaaatgcagcgtttttgcagcaaactcctgctggttaccaggtgctaccacatatccggttacgccatcccgcactatttcccggcatccgcctacatcaaaggtaatacaggccgtttcacaactaccggcttctatcagcacattgggcaggttatctgccttggtgggatagaaaaaaatatcgctggcgctgtagcattgcatcattttctccgtttccttcacatagccggtatatacgcattccaggtgcttaaatgttccgggcaactggtccctgcctatcatgagcaggtatactttccggtcgagctgtgcatccagcaggtgtaaaatatgcagcaattctgcaccgcctttaaactcgctgttaaacaaccgctcggatacaaaagtgatcacctgcgcatctgccggaagaccaagtgcctggcgggaagcagttttatcctgcgggcggaaataatctgtgtcaataggattgggaatatgatacagcggtttgttctttgtaagcggactttcagcggtcatgtcatacaaccaccgtgaaggcgaaacaatgtgcaggtcgctgctggcatagagccgctgttttctttttatcaggtaatttccggtaggcaatcccatggcaggcgcacgtttgtgctcttccttgccggccctcccgcttttccaggaagtatcgccaaaggtatgcgctgcgttgcctgtgatggcccacatatcatgcagcgtccatacaataggcgcgatagcagataagcgtggtaataaggtagcatcaaaatatccaccgtgaatattatgcaggctgatcacatcgggccgataagcctgggtatgccgcatgatggcggaagtagaaaaaggaaaatacagatattgcagtccggcccggttacttaatacattgagtcctctttcaataacattccgcacggcacccggacgggtagccgtggcgcggggagaagccgtgtgggtgcctaccaggaaatcattggcggtatgataatactccgccatcccggctgcaatcctttgcgctgctatagcagcaccaccgctgttctcatatttattgataaaaagtactttcaccggctagtatttaaagaactgttgcatttgtttgcggaacacatccggcggccagttgcgtaccaggatgcggggtagcgcatacggattgctccagctgtgcacctgtccgtggtagttggcgcataccatttgtaaacccagcgccttgcaggctttgatgctgtctgcattgtaatagcgtttggtaccgaggaatttcctgccgccaaagggataggaaaaatgtacctgcggggcgcccagtaccccttccaggatttctttggacatccctatctcggtatattgttcttcgtagcccagcatgcccacagccggatggcggtgggtatgacagccaatagtagcataggccgcctggcccattgcttttaattcttcccaggtcattaaccggtgcgaagcgcggccggtagcggttttaccagaccagtcatacagctgctgcatggcggattcaatttccgccggtttacaaaagcgcagcacctgttgcagcgcataatatgtttcacgtatagccgcaagcgtatctgtaatataccgcgccggctgtccattgatggtaatctgtagaacagggggcaggttgccgggggtaagcaatactctctccaggtcatcccaccacaattcgaaggcggtattgatcttagaggtggtaatataaaaaagggcaggcgcctggtgctttgtcagcaaaggcaatgcctccaggtaattgtctgcatagccatcgtcgaacgtcacaaatacggagcgttcggggaaagcttttttattttttacatgataaagaaatcgttcagcatccagtagattatagtcagtggccagatgcgcaaggtgtgagttgaagtgttccggcgtaacagaaaggtcctgtgggtcctgttgcagggtggtaacccggtggtacagtaaaataaccgccggttgctgcactttgttggctacataatgcgcaacagaaaatattttttggctcaggtttcccatcagataatgctacattttataggcgtatacattcaactgcatgtccatagtatcgttcaccgctttattcacaaacggagccgctctttctgtcgccgattcaatgaagtacctgaaaccattccgttgaagggtttcgagtatttctcccaatccctgcggcgctttgctaaaggaatgatattctataaagatgttctttaccacagacaaagcggtgtcgcagtctttgatcacagctacttccgcaccttcgatatccattttaagaaagtcaacgcttcctgcctgttccagtaagcttttgaggcgcaccgttggtactactactttggttccgctcccatttccgaatacactgccgccatcggcattatcgctgtagaaagtaatacctgcttcatccgtccatacggcccggggcactacggtaacgtcagcaaaattgtttttccggagattatcaccaagaacacccgctatgaatggatccgcttcaaaagccgtaatccgggctccggggaaaagcgatttaaaatagatacagcttaaacccacattagcgccacagtcaaagatcacaggggctttattactgctctcaaactggtatacgccggaaaaaaatatctccttatactgaaatacaaaagaaggtccgtctacaatgtttacatggtagtccagaaaatcagcaggcgcctgctcctttatccgctgttgataatgtttgcggtgtaagcgtaaaaactcccggtaatacttattactgataacctgtttaatcttctgcagattttcactgatcaatcccatgtagtcttttttttgctttaatggtgataattaccgggtataccggatcgttaaaatccaattctgcggctgttaactcctctgtcacaattccctgcaatatggcagtgcaggcaagtacatttccagatgacgatacttctatgttctcctctccaaaaacttcaccaaacgccttagcggccgattgggtagtaaatcgccagtaatctccccattgtttcatatcagtggcagacaattgggtaatccctgccagtgttgccagtaacactcctcccggcttcagcaaataataggcgccggcaatggccgacttaaagtcatatataaaattgaaagtttgtgtgcaaataaagcagtcaatacaattttcaggcaaggtagccggggaggttaaatcccccacaatagttacctgtggttcctgcttcatatgcagcacttcatatttacttacctcctgtccaaattgcctggagtatttgctttctgctatttcaagtacacttccggaaatatgcgtcctgttcactttcaggaactgctcaatgtaatagcggtctaccggcgttccacggtcaaaaccaaaagtggtggaaagcggttgcagacttcttaaattagtccacgacaacggcgaaacggtattcctttttaaacgctttattatcttcctgaccagcttaaccatttccagtaatttttttccagaatttagctatccgctgcttaacctttgcttcaaaggtcattccggcattacgccttaagaaagtaccgaattttttttctatcaacaggtaattgcttacaggaatatcttccacaggaatcctttcctggtagatttctgtataggtgtaatcgtattccataaaatggtgtgtggcactggctacattgccatcgtgcctcaccagtgatttcaccggataaagggttaacatatcattcagatatgcggtggccctccagcggatagcccaggaactcacctttccattcttctgctggtgcaacatcctgaaaaacggataccctccccaaaaatcaaactctttcttcagccctcgttcctttatttgcgcaattaccttttctgtatctctttcaaacttattccatgccctcgaccacgtcccccatcccaaacaaccgggatcatgtatcataaaggtagccggcttataatctcccggcatttctatcgggtacagatagccatgaatcgcaatcatcctttcttcgtgctcatacttccggagaccatcgttcatatactgcagaaaataaggggacaccgcgaggtcatcttccaaaacgattactttaccatgtttacggatcacctccgttacaccatctatcactgaagtggccaaccctttattcttctcagcctccagcaccactacttccttgcaccattgcctgctatgcaccacttcacgggcctttttaaccaacgctacctgttccggtgtggcattctcttttgcaccgtcgcaatatacatacaacgtactctcccctgcttccctgttttcactcaggtgttgcaaagtgctcagcgtcagctctggccggttgtatacaaataatacgatgggagcaaattccataatacaaaaaagtactgcgcagcgcagctgttaggttaaaaaagtaaaaatcgtataaaaataacaataaaacaaatgtgtagaagtggctatagtcttcctccgccggcaaaataacgcttccagtacggctctttcagatcgctgatcatgacgccggcactggtagatgcatgaacaaatttatcattctccaggtaaatacctacatgagaaatacgtttatgatggatcctgaaaaataccaggtcgccttcatgcaggtcatgcggttttaatcgtttcacctgtgaaaacaggtcggtggagtttccggaaagccccagctgaaacacggtgttcatcagggtatttacaaatcccgaacaatcgatgccgtctctcgttttcccacccaaccggtagggtgtaccgtaccattcgtcaataaaaccatacagcttctggttcagtacctcttctaccggaacatccagtaactgtgcatatttaaattgccagctctgcgcattttccaggttggcactgcccctggtgatgtttttgctgatgcttacatctttgctgttatagtgagaagtattattgcgggtggtacggctggtagcaataccatctataaattgaatacggttgttgttggcagcagcaggtgtggtagcagtttttttattagcatttcctttctttaatgaagcgcaggaactgagcgataatgcacatatcgataacttcacaagtagatgtccctttactctgatcataagcgctggctaaattttcgctaaaatacaaatatatagcgatttacgaatgtcgattttcgcgagagggatcgtttgtcgccttcggcgacggaaattgtcttactgccggattacgctgattatattgattaaggggatttgatcacgttggatttttaaggataacaattctgtaagcgaatatatccacctatatcttcttatatcttcccaaatcctcataaaatcctcataaaatcaaaaacataatcaaatcagcgtaatcacggttaatcagcgtaatccggcagtaagacaatttttatcgccgaaggcgatcctttcccctaattacattacttttgtcgcttgacgaaacagattagcagatgaatttttcccacttacacgttcatacccaatactctttactggatggggcagccgacatcaaatcgctgtataaaaaagcgatggcttccaatcagcccgcactggcgattacagatcatggtaatatgtttggcgcatttcagtttgtggcagaagcatacaacaataaattaaacccgggtgatccgaaagataaaagactgaaagtaaaacctattgtaggctgcgaattctatgtagtggaaaaccgccacaagagagcttttacaagggaagaaaaagatgtgcgttatcaccaggtgttactggctaaagatgatgaaggttaccgcaaccttatcaaactttgttccctgggctatatggaaggcctgtatggtaagtatccccgtatcgataaagaactcgtattacaatatcacaaagggcttatcgccaccacctgctgcctcggcgcctctgtacccaggatcatcctgcgcaaaggcgaagaagaaggagaaaaagaattccgttggtggctggatattttcggagaagatttctacgtggaattgcaacgccatggcatcccggaacaggaacaggtaaacgtagtactgctccgctttgctgagaagtataatgtaaaggtgatcgcttccaacgactcccactatgtggaccaggccgatgccaacgcacacgatatcctcctttgtatcaataccggtgaaaagaaaagcacccccaccaataaagacttttcagacgatgatagcggtggcggcggaaagaacaggcgttttgctttttataacgaccagttctatttcaaaacaacggaagaaatgagcaaactgtttcatgatcttccgcaggctattgataataccaacgaaattgtagataaagtacagctgctggatcttaaaagagatatcctgctgcccaacttccctattccgaaagaatttattacccaggaccagtacctgcgccatatcaccttcgaaggcgcccgtacccggtatatggaaatgaccgccgatattgaagaacgtatcaactttgaactgcaggtaatcgaaaacatgggttttgccggttacttcctcattgtggccgacttcatcaaggccggtcgtgaactgggcgtatttatcggcccgggccgcggatccgccgccggatcagcagttgcctactgtatcggtatcaccaatatagatcccatcaagtacaacctcctgtttgagcgtttccttaacccggaacgtaagagcatgcccgatattgatacggacttcgatgatgaaggccgtcagaaagttattgactacgtagtacagaaatatggccgtaaccaggtagcgcagatcattacctacggtaccatggccgccaaaatgagtatcaaggacgtggcccgcgtaatggacctccccctggtggaatccaatatcctcgctaaaatggttccggataaacccggcatccagctggatcgtatcttcaacgcccccctcgaaggagaaaagagcctcgccgataaggaaggcctcgccggtgaagatattgagaatgtgaaaaagctgcgcgaactcatcaaaggcaccgacctccaggcagaagtgctccgcgaagcctgcgtactggaaggctccgtacgcaacaccggtatccatgcggcaggtatcatcatcgccccgcaggacctgtacgacctgatccccgtatctaccgcaaaagactccgacctgctggtaacccagttcgaaggaagcattattgaatctgccggcgtaatcaagatggacttcctggggctgaaaacccttaccatcatcaaaggtgcgctggaactgatccgccagaaccatggcatctccatcgaaatagataatatcccgctggacgacgccaaaacatatgacctctaccagaaaggtgaaaccaacgctacgttccagttcgagtcgcccggtatgcagaaatacctgcgtgaactgaaacccgataggttcgatgacctcatcgccatgaacgccctgtaccggccgggcccactggagtacatcccctcctttatccgccgtaaacacggcctggagccggtgcaatacgacatcgccgaaatggaggaatacctcaacgatacctacggtatcacggtataccaggaacaggtgatgttgctgagccagaaactggcaggcttctctaaaggtgatgcggacgtactgcgtaaagcgatgggtaaaaagcagatcgcggtactgaacaaaatgaaagcgcagtttatggaaggttgcgccaaaaatggccacgatccaaaagtctgcgaaaaagtatggaccgactgggaagcatttgcctcgtatgcgttcaacaaatcgcactccacctgctatgcttttgtggcctatcaaacagcctacctgaaagcccactacccttctgaatacatggctgccgtactgaactgcgccagcaatattgaaaagatcaccttcttcatggaagagtccaaacgcatgggcatcgacgtattgccgccggatgtgaatgaatctttcaagggtttcgctgtaaataaacagggccaggtacgcttcggtcttggtggcctgaaaggtgtaggtgaagccgccatcgaaaacctgctggaagaacgtaaaaaggacggtcctttcaaaaatatattcgactttatcaaacgcgttaaccaacgcgccgtcaataaaaaatccctggaagccctggtgatgtcgggcgctttcgacagcttccccgaactgcaccgtgcgcaatatttccacaaaccggaaggcgaacaactcaccggccttgataaaatcgtgaaattcggacagcaggtaacagcgggctcttccaacatgggcagcctcttcggcgccgatgacctcccggatgtagagccaccaaagatcccggcctgcgacgcctggccgctgatcatgaagctcaacaacgaacgggatatcaccggtatctacatttccggccatccactggatgattaccgctttgaaatgaagtattaccacatgaatactgttcaggaactggtggagtatcaaaccgaaatagcccaaccgggtggcaacggcggccgctccagggaacgcaatttccgcctggcagtatatattaccaatgcccaggaaaggatttcccgcaacaaccggcagtttggcgtgatgaccatcgaagattacaccggaaagtttgaatttgccctgtggagcgaagatttcatccgctttgccccttacctgaaaccaggcctttgcctgttcatcaatggcggcttcaaatccaaacggttcaatgacaatgaatatgaattcaaagtaggcagcatccagctcttacaggaagtgaagaaaacacacactaaacaggtgtacctgaacacgatgcctaagttcatcaaaaaggaaacggtagacttcctggtagacaacgtaaaccgctttccgggcaacagtgtgctgcatgtacatctgaccgaccgggacgatcacacccaggcaaaactgcatactttcaaccggaatatcgagatgaatgacgagttggcgggtttcctgcacaaacagccggatattgatgtgtatatagagataatcaataagtaggatgtcaaaaatgcagtaatttgcactcggatcaagatttgatcgtaatataacaaatcataaaaatcaaaacaatcgttaaaataaaaacattttaaaatcaaagaatatggctttagaaatcactgatgcgaactttgaaacggaagttctgaattccgataaattaactgttattgacttctgggcagaatggtgtggcccttgtcgcgctatcggtccggtaatcgaagaattgtctaaagattacgctggtaaagtaaatattggaaaggttaacgtggatcagaacccacagttatctgtaaactacggtatcaccagcatccctgctatccttttcgtaaaaggcggccaggtggtagacaaacaggtaggcgctgtgcctaaatccgtactggataaaaaaatacaggccaatatgtaattttataaaaactgacttttgaaagcgctccggtttgttccggagcgctttttttgcgagtggatcgccttcggcgatgttaaattgtctttctgcctgattacgctgattatactgattacgctgatttgattatgttggattttacttttgagattttttaaaggattttgggagatgtaagcggaggttgtctttttgcctgattatgtttatctttatattgtacctaaagtattgatatccagtttctttctttgttgaaacttgtctaacgaatgtcgtcaaaccccctatagccaattgatacacaatacattaccgatcaagtccacgtcacctccacatcaaaagcagatcaaaagcatgtataaggcatatacaaagcatatgcaaagcggatgtaaagcataggctatcccatcttcacccatctttttaaatatccatctccaaaagaaaaaagtaaaatcagcgcacagcctccgcttacgtctccccaaatcctttataaaatccctaaagtaaaatccaggtaatcagtataatcagcgtaatcaggcagaaagacaacctccgcttacatctccccaaatccttataaaatccccaaaataaaatccagataatcagtataatcagtgtaatcctgctccaagacaatttaacatcgccgaaggcgatccgcaaaacatttttcgcgtatcttcaaagccaaaatctacttttttgcgtcactacttcctcgccctgggtgcctttttttattgcgtcaccgccaatgctcaacgcaaatgcggcactgccgaagcactgcaacagcgggtaaaagaaatcccttcccttcaaaagattatacagaataacgaagataaaatgatgctgggccagcaacggcaacagctgcgtgcgatggtggaagccattccgcaggcggtatccgttcccgtagtgatccacatcgtgctggataacccagcgctggttacagatgcgcagatcgcctcccagatagatgccctgaaccgggattataatgccgctaaccctgatgtaagccaggtacccgccgtatggcaggcgctcatcggcaacagccgcattaatttttgtctcgctcaaagaacgcccgacgatgaacccaccaacggcgttgtaagagtgcaaacagctcccggccaaagcttttctatcagcaacgcggcggcagacgccaagtacaacagcaccggcggctccgatgcctgggatcacagcaaatatcttaatatctgggtcacccgcctttccggtaattacctcggcgtggccgcccctccgggtaccggctaccctgttgaacaggaaggcgtggtggtgcaatacaccgcttttggtactaccggcagcgtaggtagtacctacaacctcggcagaaccgccacgcatgaaatagggcattacttcggtttaaagcatgtttggggagatgataacgggggatgtaccattgatgacggtatcaccgacacaccgctccagggcgataatacctacggatgcccgtcctttccccggctcgacaactgcaccgccacctcaccgggcgtgatgttcatgaactacatggactataccgatgatgcctgcatgcatctctttaccgccgggcaggtagaccgcatgcgctttgtactggaaaatatcaccgccagcctgatgacctccaacggatgcgtaccaccttccatggtaaacaacgatgcctccctggtgagtgtcaacgcgccggatggcaaaatatgcaccaacaatattacacccgtagtaaccctgcgtaaccgcggcgccaacaccctcactgctgtgagaatctggtaccaggtaaacagcggcgcccttacttcttaccagtggacgggcagtttggccagtttgcagcaaaccagcgttacacttccttcttccaatgtagctatcggcagttataacctgaaagcatatacgcaatcacccaacggccagccggatggaaatgttaccaacgatacagctgatatccgcttccggtacgacgcggaagcagccctcccctttgaacagggctttgaaaacgacagcttcccgccaccaggctgggatctctataatcctgaccgcagcttcacctgggaacgcgttcgtaatgtgggcaaaaacagcagcgcttccgcgctcatgcgcaacctgggatataataccaacgaccagacagatgacctcatcacgccggttattgatccgcagggcgcagattccgtattcctctttttcgacgtagccgcagccgtatttaccgaccctgctaccacctccaatgcctgggataccctccaggtaatcgtgaccaacgattgccgccaaaccggccaaatcctttattccaaatggggccccaatcttattacacgcccaacaccggttcaaacagaattcatcccaaccaccaccgaatggcgccgggattctgtaaacctgaccgctgcaagccataaaggaaagttccaggtagccttcagaaacatctcaaactcagagaataacatttatattgataatattaatattgttaccaaatcagtgaatccaatcctccgggaaaaaggggtattggtgaatcctaaccctacagatggcatcgtttgggtaacattcctggaaataccggaagacctggtgcaggtatctatttacaatatacagggacagttcattatgagccgtccggcagcagatatcggcgccggcaaccggatgacctttaatttggtaaatgagccaaatggtgtttattttgtaaaattaatttacaggaacagggccaacaccatcaaattaatgaaagtaagatgacgatgagacaagattatccggctgttcaaacgctccttcagcaacctaacctggacgcagcattgaagggcattgcagaaaagatcctccaacaggaaagaattacacccgcagaagggctgatcttatttgaaaaaggcgatatcggctttttaggtgcgttagccaacctggtaagggagcggatgcacggtgacaagacctacttcaaccgcaacttccatatcgaacctaccaacgtttgcgtattcacctgccacttttgctcctattcccgcctgtataaaaacagggaagacggatgggaactgagtatcgaccagatgatggacatcgttaaaaaatacgataaccaacccgttacagaagtacatattgttggtggcgtacatcctaaaatgcagctcaacttcttcgtggagctgatccagaaaatcagggcacaccgtccggatctgcatatcaaaggatttaccgctgtggaactggattacatgttccgcaaagctaaagtgagcatagaagaagggatgcgcatcctcaatgaagccggcctgcaatccatgcctggcggcggcgccgaaatattcgcaccggaagtacgcgctaaaatatgccacgataaagtagatgccgacggatggcttgccattcacaaagcagcccacaaccgcggcatgcacaccaacgccaccatgctgtacggccacgttgaatcttttgcggaccgcatcgaccacatggaacgcttacgtacactgcaggacgaaaccggtggctttaacaccttcatccccctgaagttccgtaataaaggcaacgatatgtcgcatatcccggaatcttctatcgtggaagacctgagattgtacgctatcgcacgtttgtatatggataactttccccacctgaaagcctattggcctatgctgggaagaaacaccgcacagctgaccctgtctttcggcgtaaatgacctggacggcaccatagatgataccacgaaaatctattctatggccggttcggaagaacaaaacccttccatgaacaccgcccagctcaccatgctcatcaaacaggccggcagaagaccagttgaacgggataccgtgtacaacgaaataagagattacactgatgtggttttttcagatgaagaactgctgaccaaatagtatcgctgttttatgcaattacacctgaaatgtatactgatagccagtttatatatcgctggctgtcaccagaacaacagtagcaccaacaattccgcagccaccgataccaatacggcggccaccacggaaactgccggtgaaacatccaatggcatcgcgtttaaaaaacaaggcgccctggctttcgtttccaaatcaggcgcagataccctgcgaaaaatagatatccagctggcgcaaacagacgaacagcgcgccgacggactgatgttccgcaaatccatgacagacgatcagggcatgcttttcattttccctgacatggaagaacgcgcattctggatgaaaaacacctacatctccctggatattatctacatagatgataagctggaaattgtgtccattcagaaatacgcaacgcccctgtcggaagaaagtcttccatctttcaaaaaagcaaaatacgtcctggaggtaaacggtggattctgcgacaagtatcacattaaatacggcgataaaataacttaccaataaaaagaaagccctggcaaacgccagggctttcttcgcttatataataacctctttttatacactcccttcaggctttgtaacatctaggatatgcagctgcgtttttcccgcaggcacttcccaatctatcacatcaccggtactatatcccagcaaggcagtgcctatgggagaaaggatcgataatttgcccagctgtaaattgctggcagccggcaataccagctgtacattcctgatagccccactgcgctcatccctgaatctgagggtggaatttacctgtaccacatcagcgggtaccttacctttcctgacagtggccctgtcgagctcttctctcagcttgtcggtgcccggtgcgtgatagcacagggttttaaggatttcgtaatcatgcagggacacgataatctgtttctttttcatgataaccgggttttatgtcagtgtttacagatgactgcccatcgtgtcatccgatgaatgataaaactgatttgataagattgttttagaaaatattagcggaatagcactacgcaggtagttatccccccgggtacaacactttatgtactaaaagttgcccgggcttaattgttgaagtcttttgggcaggataggaacggcaacaggaacccgcacgtgcgtttggatgcacgtggtgtattgagtaagtgtaatatgtaaattgccggattcaattaatgaataattgtatccggcaaagataaggcttttatttacaacaagcggtcaattcgctaactctcctgctgtgaagggcttctggcggccattattcagcttacgcacctgctggatatctgcagcggaaactttatcggctttattattccaggcactgcgcaggaaagtgagcagttgtgcaatatctgcatcactgaattcatcactggcgccgatacccggcatatcgccatttatttccggggctttgtacactttcccgtgtacttccaccggaccggtaagaccgtataatacgatagatataaatgcttttttgttaccgtttacccagttgctttcattgagcggcggcgccatcgccgtaatgccctccccgtttttaccatgacaggtttggcatacggtattgaagatcttatatcctctcggtagttctttccgtaacgcttccatctttttcacattggctttgctgtccatgtttttcagcactgtttccagctgacggcgcaatatcagcgtggtatcagggttccaggcaatgacctctttcagcaaggctgcttcccggttggccgcattatttaccagcgctgccgccacataacggttaggggcatacgcttttatcattttatcttccaggcgggtggcagctgctttatccagtttccctaccgcaggcaatatataagccactgccggcgccaggtatgaattatccgacaaggagtccagcgctgttactgttgctttgatgttactgctgtttaatacagatggcaatgccgcgagcgcctgcatttttagtgcaggatctgcctgttgccagatgccgctgatatcatctccggtgagactgtgcaagccttccagcgtccagagggcgtggatctgtgtcagcgggtgtgccgcgtctttcagcatggttctcagttccggcgccatcgcggttaggtgctgatcaatgatgagctgttgcgctttatctctcaaaacaccattatcgttacccagcattttcccgaggaaagcgggcgtaagttcaaatgtaaccggctgtggtttactgccggcaggaatgatgcggtaaatacggccgcagttcagcggcagcgtaaggttacgcatctttatctcgttcttcaggtaatctgtcaggtaggttttatgttgcaggatgccccggtacatatcggcgatatacaaagcgccatccggaccggtacgcaggtccaccggcctgaaacgctcgtcggtgctggccaggaattctttccgctggtatgcttgtacacctttcacgacatagctgctgtctgataaaatattccttttaatcaggttggcagaaggctcggctacaaacgcattaccggcataggtagatggcagcaaggtgccgcggtaaatcaccgggccgcaggcggcggtgaatttcaccaggcggaggctgtcgtccagcgagcctttctggtaaccacggtttacacccggcgttggatgcgcggggtatgtgcggttatcgggtacaattttttgatcaaaaccggcggcattgttctgttgctggttagtgccgcctaatcctggaggaaaataatcgcccagcaggttttccgaattattgttataataaagacggccgtaattatcctgcgtaatgccccattgtccgcggaaatgcgtgggctccttcagccacttatctcccgccttacggtaacgcctatccgattttgcattatagatccagttgtccattgcgcgcagcaacccgttgggctgatgctccacgtttccgccggcagcgtattgatcatctaccagggttcttttgccgggtttgtcgccattgttttctataaaccacaattgcggcggcgtagctaccagcacgccgttttctatcaggcagatagcccttggcagcaccagtgaatcaaggaacacggtgcgtttatccattacgccatcgcggttggtatcttccaggatcacaattttaccgtcgggtttatcttccccggtaccggcagtatcaggcataaagccggtcatctccactacccacatgcgcccgcgctcatcaaaagtcatggctacgggcgccactaccattggttcggcggccaccagttgtacttccaatccttcatcaaattgcatgtgtttgatggctgttttgccatccagtacgggtgaagcagcaaactgctcccgcatggcaatagaatctttttcgtgcttgttcccgttgttctgctgatttccttgtccacaggcaaataaagccagagataacgtggtgattaaacgataatgaatacgctgcattttttactattcgggttacgaaagcgataaaaatacatttctaaatatattttttctgaaaaattatatgagataacagtttactatgtgagcgacggcaaaaaaacttatcttcgtcgcttcattgcatacattttacgatttatttgcatttatggaacgctttcagggcatcataggcatcgtacttattctgggtatcgcctttctattttctaacaacagaagtaagatcaattacaggctggtgttcagcggtattggcttacaggtgttaatcggctttctggtatttaaggtgccccctattacctggttcttccagcgggtaggagatgcaatgggaaagctggaaggatttgcccgtaaaggcgctgcctttgtatatggaggtattggtgtatcgcagcccgatggcaccggcctgaaggactatgccgccggaggttttgtatttgcttttaacgtaacggccaccatcatcctggtgtgtgtgctggtagcggttttatatcattatggcattatgcagcgcgtggttgcggtaattgcccgcgccatgaattatgtaatgcgcgtgagtggtgcggaagcattgagcaatgtggccagcgccttcgtaggacaggtagaagcacaggtgatgatccgtccttatttatcaagcatgaccaaaagcgaaatcctcgcctccatgagtggaagcctggcttgtattgccggcggcatcctcgtggtgtatgtgaatatgggattgcaggctggtttgcatattgcacctttcctgatcaccgccagcctcatggccgctccgggggcactggtgatttcgaaaatcgttttccccgaaacagaggaaagcgtaacaatgggtcgcgttaaaatggaagtaaaaagcaattataccaacgtaatcgacgcgatttcacacggcgccggcgatggttttaaaatagccatgaacgtgatcgccatgctgatcgggtttatcgctttcattgcactgatcgactggggccttattcatatcggtcatatcttcaatcctaattttgatctcagcctcgactggatcttcggaaaagtgtttatgccgatggcctgggcaatgggcgtgccacagggagatgtacaaggcgtagctaccctgctcggacaaaaactcaccattaatgaatttgtggcttttaaaagtctcactgataaaacagtaccggtattaacctccaaagggattgccatcgttacaattgctattgcgggttttgccaatttcagcagcgtaggcatgcagatcggtggtatcggtgagctggcccccgacagaagggctgatctggctaaattggggctgaaagccctgttgtgtggaacgctggcatcttatatgtcggcctctattgcgggaatattgatctaacgcggagtttgtcttactcaggattacgctgattatactgattaactggatttttactttttggattataaaggattaagggagataaaagcgaatatatccgcttttatctcccttaattatatcttaagaaaatcaaaaaaatccaaaagtaaaaatccagttaatcagtataatcagcgtaatcctgagtaagacaaactccgcgcgcgttattccaagcgtttaatgagtcccgcctgtacagccgcccaggcttcaccctgacccgcatcttcccagtaattcttcatttcggaggctgccacaattttatttacagcggcgattgcctggtttctgagtgcgcgcgtaccaataaggttcagcacatccagctgatccaaaggatcttccgggaaatcttcgcttgggcgtgctaccaatgctgccaccagttctgcagcggccaacgcctcttcgcaatccgaaacttccagtgtttcgatgttgttgatgacacgcgctaacgtgtcagacaccaaaccaccgtctttattatcaatcaggtcaaaaatccaatcctgtgatccatcattttcaaaatttctggtgccccatgcgcccatagtgtttacgtttttttatttttttagaataaagaataaaagtaatgaactctctttacaacaaccaaaccaaccggctagttcaaactcctgaaatcaaccggaacgagtttgctcactcccggttcctgcatcgttacgccgtagatcacgtctacagccgccatcgtttgcttgttatgtgttacaataataaattgtgaattatcggaaaacttgcggatcatgttggtaaacttacccacattggcatcatccaatggcgcatctacctcatccaggatacagaacggcgccggcttaatcaggtaaatggcgaacagcaatgcggtggctgtcagtgttttctctccaccggacagctgtgtaatcgccgccggccgcttgccttttggcttcgcgataatttcaataccagtgtccgccaggttttcaggatcactcaggatcatatcgcactggtcttcttccgtaaacagggctttaaatacccggataaagttttccttcacctggttaaaggtatccaggaatttctggttagcggtggactctacctcctggatagtggccagcagggaatctttcgcatttaccaggtccgttttctgctccaggataaactcgtagcgcttcttcatttcctggtaagcttcaatggccgtggggttgatttcccccatgttctccatgcgctttttcagtcgctctgcactgcccgtcagctcatccaccgacagttctgagttgcgttgctcatctataatttcatcgaggttcactttaaactccacgctgagcctttccttcatggaggccagttgcagccgcagttcatttaccttgtccttaatggtattcagctgctgctccagttcctgtttggcgcgctgttttgttctcagcgtggtttccagttcctggaggtggttacggaagttatagtattcctggtctttttcgttgagtgccttttcttcttcttcgcgctggcggaataattccacgagtccgtcgtctgcgtggctcagtttatccacggcagccgcgatgttggccacggcgtcttccaactgcgatttgttactggtgatctgtatgtgcaggtctgccagctgtttacgcttaaattccagttcctgtttaagggcctgtactttactttgctgacgggtatgctgcaggttttggttattaaactgcaccgtagccatattaaactgctgttccgcttcctgggccatcctgtcggcatccgcgatgctgtcctgcagctcggtgaccctttcgttcaggctttccagttcgtctttcacaccggaaatgctttcctggttggtttccagggattgctgcatttcttcgaggcgtttatcgccggcttcaatgaggtggtggaagttttcaatcctgttctgtaagccaaacagctgattgctcagctggtttaccctttcccgcgcagcattgatattattttcattcagctggctgttgtagcctaatacttcgtcgtgtttgctttgcagcgccactttcaggcggcccactattccttcgagatctttgatctctatttccagcttttccaggtttttggcccttcccagctttttaccttcaaataatcctacagaacctccgctaatgttgtatttaccacgatgcatgcggccggatttttccaccagcagcatcctttcgtccgccacctggctgaattccaggcgggtgaggtcttccccgataaatacttttccaaggagatgctgtcccagtccccggtacttctcttcaatttccactacttccagcgcaggaatggtgcctgccggcgccagcagcgggctgtaatcagtccggaactgatcgaggatgaagaaattggcttttccttttttgttgttatcgagcaactggatggcctgtacggcttcatgtacgttgttcactacatagtagctcaggtaaggttccagcaggttttccacgcaggtgcggtattcctctttacagaaaaatatatcactcaggatgggggcgttattgttccagtcgggattctttttgagaaatttgatactctccgggtagccttcgaggctgtcgaccaacgacttgagcaggtcgaactcgttctttttggaatcgagggtacggttttcgtctaccagtttatcacgcaatccttcgatatcggactgggtggcgagtattttacttttggtttcttcctggaaacggaccatgttttccagttccgttttgccgccggtcagtgtttgctgcagggcttccttttctgtttccagctgggcgatctgctgcaggcggctggtcttttcttcctggagctgctgcatgctgcgttgcaggttcattacggaagtatcggcaacggctactttcttttcggcttcaaattgctgacgctgccagcgttgctggtcgttgcgcaaggtttcaagggcctgtttcttctgatggaagcgttctttcttttcctccaccatatcgcggagggtgtccagttcgtcggccatggtttcaaacacttccccttcttcttctacctgtttttcggtgaattcgatagaagaagtaagtccctgcagttgtccttctgcattgctgaggaagtcgctgatatttttttcccgctcgcgcagataagtaagttgctgcgtggcgaggttcttatcgttttctttggtgcggatggtggataccagctcattaaaagatttctgcatggtttgcagttctctttcttttgccacaaaatgcagtttatcctgctccacggccgcttctgcggtgaggatctcggtttccagcgccagtttgcggtcgctttcattttgctgggtatccgacagttccttgaaggttacgttaaagccttccagggcggctttggcaagttctatgctgatttcgcggtattccttttttacttcgtagaagcgttccgccttacgggcctggctttccagtgttttaaggttgttattgatttcaaacaacaggtcctcaatacggttcaggtctccttcagtggcgtctagtttggatttagcttcttttttgcgggttttatatatggagatgcctgccgcctgttccagcatacggcgacggctgttttccttgtctttgatgatatcgtctaccattcccagttcgatgatggcataggaatcggtacttacgcccgtgtccatgaacaggttatggatatctttgaggcggcaggccacatcgttgaggcggtattcactgtcgccgttcttataaaatttgcgtgtaatcgtcaccgtggtgaactcggtgggtagtacgttcttggtgttttcaaaagtgagactaacctccgccataccgcttgcagagcggcttttagaaccattgaacacaagtcctgcctggttatcagaccggaggttactgattttgtgctcgccgattacccagcggatggagtcgataatattacttttgccgcaaccgtttggcccaattaccccagtgatgccctcatcaaactgcaaaacggttttatctgcaaaacttttaaagcctttaatttctagtgtttttaagcgcacgtcgtactccgaggttttttaaggcgtcaaagatataattttacccgaatcaaaaagtaatttaagtgagatgcaataatatacagtaattatttatacacaattaccggtcatttgcccctgtccgcagcacgcaactaaagtctaaaagactggttataaatatagtaaaaagaacaattagaatttaactccctgttagaaaattacgcggatgttgtctttctcaggattacactgattatactgattaacgtgagatatcttctgaaccctgcattaaattaaagtcaaaagtaatatattcatctttaaaggataagaaaaaagataatcagtttaatcagcgtaatcctgagaaagacaaaatccgcttatctttgcgccatcaaaaacccttttacgtttgcgtacagaacagcggatcaataatataaaaagtttcctttacagttatcatttcagcaacggtatgcgtaccaccatcagcgtggtagtgccttcactggtatgcgcttactttggcatgctggacctgggtatcgctatgtcgatgggcgccttgtgtacggccctcagcgatgtacccggcaccattgtacacaagcggaacggccttatcatcagcaccatcctgatctttttttccgcgctgggcaccggcctgctcattccttacgtaatacccatggctatctggatagcggtgtgctgttttatgtttgccatgctgctggtatatggtaaccggggaggtaatattggtaccggctgcctgctggtagtagtgtctattctcggggaaacccagctcacgccgaagcttaccctcctccactcctctatggtgctgctgggcagtatctggtacgcggtgctggccctcatcctctggcagatccgaccctacctcaatgtgcagcaggcactgggcgactgtatcctgcaaaccgcccgctacctcgaggtaagggccaacttctacacgcccggcgtaaatgtcagcgaaaactacaaggccgtactggaccagcaggtgatcgtcaacgaaaaacaggaaaatgtgcgcgaactgctgctgaaaagaagatccgcccaacagggcactaccagtctcaataaaagcatggtactcattttcctggatatggtagatctccaggaacagatcatggcctctcaaaccgactataacgccctgcacgccgattttaaagatctggcgatcctggaaaaattccatgctctcatccttgaattcacccaggagctgaaaaacatcgggatggccgtggcagcgggtcagcgctccctgcccaaaaccaacctgaagtttgagatggaaaaggtaaaacaggccattgccgacattaccatgaagctgcctaccctcaaggaaagaacccgtaccatcccgctgagcaacatcctgcaaaacctgcaggacatggcccagcgcatttataacctgcataggcttacccggctggaaagactgaaagacgaatccatagatccaaaactggagctgtcgaaattcactacccgccagaaatacgattttgaaaccttccgggataacctcactttcaaatcacatatcttccggcacgccatccgcgtgagcctggctaccgtattgggttacgggctgggtattgcccttcacctcgaccgggtatactggatcctgctaaccatcgtggtgatcctgaaaccaggcttcgggcttacaaaatcacgcagcatacaacgtttaatcggtaccgttaccggcgccttatttgccgccggcctgctttaccttacgcacaacgatacggtgatctttatagtcatgctgatctgcatcctgggcgcctacagctttatgagcttccagtataccgtcagcgtattttttgtgacgccgtttatcatcttcctgctgcatttccttcatccttcagacctctacaatgtaacgcagcgggtactggacactttcattggcggaggcatcgctttctttgccaacatgctgctgtggcctacctgggagcataacttcctcccggactacatgaaaaagatgatggaagccaaccggaaatattttgaactggtgatgcgcgcctattccaatgaaaaggtatccattacagatttcaaactggccaggaaagacacctacgtggccgccgccaatatgatgtcggccttccagcgtatgttatcggaacccaaaagcaaacaaaagaacgcgtcagaagtatatcatttcgtggtactgaatcatacactcacctcgcataccgccaccctggcggcctacagcctgcatcacggggtgcagtttccccgcccggaataccgcgaaataacggattatctcctccattatatggaccagctcaccctgctcacagatcccgccaccagcagcagcgcccaaccctccccgcaggtacatgccttcgaccggctggacgcccacctggaaagcctcgtacatctgcgtcaacaggaaatcaatgaaggcaaaggccctacacccacccgcgacgaaatgctggaaaccaaacaggtgcacgaccagcttgtagccatcctctccctcgtaaaagacatgagcaaagcgctgaaagcggagtgacgcggattttgtcttggctcaggattacgctgattttactgattaccctggatttttacttttggattttataaaggattaagggagatagaagcggatatattcgctcttatctcccttaattattataagaaaatctaaaatcaaaaaaaatccaaaagtaaaatccagggtaatcagtaaaatcagcgtaatcctgagccaagacaaaatccgcgttactccgctaaaatggtaaactccgcggttaccggtgtcagcgcagcaagcacgcggtcgaagaaggcggggccttcctgggcgtaccagggcaggaagttctccttgcgctcctgtaacgaaccggcaggaaataatttattcttaatctggcggatctgatctgtttgccaggcgaactttttcttctcggcacgcaggaacttatgttccagtttaccgatcgacttcagcgctttctttctttcagaggcggtagtggcaatcagtgtgacatcaatgctgcgagccttttcttccagggaatcaaacaactgctcgatggccgcatattcatctttcaataccagcgaagcattggtgtgtttcttcacgtaatcgtttacgatatcttccgttcccttgaaaagatcagtggtggtgagtcccagcttattgatccgctgttgggaaagtgcatcggtaagcaacagggagttgcgcagcaataaaacagggaaaggcactttatagtgtgcaaaaagtcctttcaattccagccagtaggcaatttcaccacccccgccaataaaggcaatattgggcaggatggtttcctggaacattccccgtaaaataacattgggactgaaattttcaggatgtgtttccagggctgcttccagcgaagcggcgttgaaagtcaacgacgtgtgtaatactttccactgatcaccgtcctgaacgatgcgctcccgcgacccttcctgtaaataaaaaagatttatttcgcgtggattggcctgcactttataatgttcccccagcttcgccaacgtatcgctgacaatggcatgcgacgcctggttaaacaattcgtcctttataacgggaaggtataaacgttttaatgcggcgttgtccggtatcagtaccaccaggccaaagcggccgaataacgcatgtacaaggtacagtgtggcttcctggatattttcatgttccaggtaggccttttgcaggaggtctgtcagttcgtcgctgtgaggtgcatatcccagcgttttcttcacttcagcgatcagcgtttccagtccttccggcttcatacgccctactgcgccctgctgactggtattccaggtgatggttttcccttccaggtagatgctgcccagctcttcgagatcggcatcttcactgcccatataatataccggtacaaaattatgttgcgggtattgctgtttcaattcatgacacagcttaatggtttgcaggatcttataagcgaagtagaggtagccggtgaaaatattgggctgatgtgcggtgcatactgtaaaggtattaggctgcaacagggcggtgatattatcctgtactgcctttacgggctccagggaagtgtattgctgttccagtgcggctaccagtgcggttcttggtgtatcaaaattttgacgggcggctattgcggcagcaaagtccggatgtacaggagaataggtataaaatggtctgatctgcggacgttctgctaaaaaatctgttaccagctggttaaaataaccagttttcccataaggaatatattcgggcatattgagtttcgaattacaaattaccaattacaaaacgatgcagtgccaacacatcgaaatttttgaatgtacgaagttaggtaattagtcaattggttgatcagattattggttgaccggtcatcattccggtacaccggtttctttggcgcttgttttgacagctatgctgcaaacaacaggcgccttagtgcgctaatgttggaaaatataccattatgaagatagcaatactggcgccgatagcctggcgtacgcctccaaggcattacggcccatgggaacagatggcggctaacgtggcggaaggcctggtagccaaaggaatggatgtaacgctctttgccacggccgactcgctcacttccggtaccctggcggccatttgcgccaaagggtatgaggaagaccgcgaggcagatgccaaagtaaatgagtgtatgcatatcagttacctgatggagcaggccagggatttcgatatcatccataatcacttcgatttcctcccccttacctactccaggctgattaaaacgcctatggtaaccactattcacggattttcctctcctaaaatattaccggtataccagcggtataatgatataggaagatatgtgtctatcagtaactccgaccgccatccgtcgctgaattacgcagccacggtgtataatggtatccgcacggaagattttgcgtttgagcctacgccggacagctacctcttatactatggcaggatccatccggataaaggcacgcatgatgcggtacaaatcgcccttcactcccgccgcaagctgatcatagccggcatcatacaggacgaagcctattttaatgaaaaggtaaagccctatatagatgatgaacagatcatttatatcggcgcggtaggcggggaagaacgcagcctgctgctgggaaaagccaatgcactgctgcatcccatcttttttgatgaaccttttggtttaagcgtagcggaggccatgctgtgcggcacgcccgttatcgcgtacaaccgcggctccatgccagagctgatcaatgaccgtaaaacaggtttccttgtaaataatttacacgaagccgccgcctgtgtggaagatctcacactgatcaaccgccaggattgccatctgcacgcgaaaaataatttcagcgcggaaatcatgacggagaagtatatcgccgtatataaccaattatagatagcctcgctacacgccgtcttccttgatctgcgtcagcagtttttccaggttgacggtggcgaagccggaagcataatccgacaaaccgtaaggaatgatcagttcatcgttgtggataatagagccgcaggagtacagtacattaggtacatatccttcccgttcgtctttattgggcataagcaggggctcacgcaggcggcctatttccttttcaggattttccaggtccagcaggctggcgccaatgcaatacgtacgcatgggacctactccgtgcgtgatcaccagccagccgtcttttgtttcaatgggcgaaccgcagttgcccacctgaacaaattcccacgcatatttaggcacgtgaaggatctggggattttcccagatattgattttatcagagtacataatatacccattgataccatcaatccgggagatcatcgcatatttgccgttgatctttcgggggaaaagcgccaggtttttattctgcgccccttctccgtagagcggcatgatcttgaagttatagaagtcttttgtttgcagcagctttggctggatggtaatgccatcatacgccgtgtaggtagcgtaataggtaatgttcccgttttcgctggtgtattttacaaagcgggcatcttcaatgcccctgctttctgcatctgaataaggaaaaattacgcggtcagacaagtcggtatcaagtgaaaagttcagctcatagtaggagtctgccagccatagtaccctttccagtccttttttaaggagatgatctacctggaaccgttgttgcatttcccggatcacctttttaagggcgaggtattcaaactggtccggcagggagttttgtatttcacgcatcacagaatccggcagccggatggataccgcattctggaagaacgtttgtttatggtacatggagttgcggataatttccgcttcatccacatagttaccgggtgctatcagtgagatttcattgtttttgtcgatgataccggatctgaaggcaatggaagatacgtgtccttcacctactgcgcgaaagctcatgatgacgcgcttttgtccttcttccagcccgctctggtccacatcttccacgagggaagggttgaagaacgcggctgattcaatggagtattcgttggtgaaataagaaccggtgagcaatttacgtttgagcgagagcccttcgtactcgatctgcaaaccgggaaacaaatgtctcagccggtctgcatgtcgttcaaatatcctcgtgatgttcctgtgtcgccgggaaaattctcttagtataggcatgaccgttatatccacctcggggtcgctcattgctgccacctgttgaatgatagacttggcccgggcctccccgttgaaaaaaaacctggctactaccctcttaaggtcaggataaatttttgtactcttccgctctatggacaatcgcatggttatcttgtttgttaaatactgaatccgtcttccaggaccactccttttttaacaacaacaatgccgtcttttaccgtatatttttcaaagtccccatcagctaagtgttttccgccatttatatgtacgccgtttccaatgcggcagtttttatcaatgatggcattactgatcacgcagttctctcctattcccatcaacgggcttccttctgcgcgtgacttttctatttcgtcgagtgtctggtagtaatcgcttcccatgatataggcattgctgatttcgctgcctttaccgatgcgggtacggatacccactactactctttccagtttatctgccataataatacaaccgtcggcgatcattgttttctccatgtggccggaaatttttgtaggcggcagcatgcgggcacgtgaaaagatagtttgggattcatcgaagaggttaaacaaggggatttcatccgtgaggccgatattggcttcaaagaaagactggatgttcccgatatctgtccagtagccttcatattgataactgaaaatccggcgtttgttttcgatggcctgcgggatgagctgcttaccaaaatcggcggcttccggttgtgcattgagcatatcgaacagtacctgccggctgaagatataaatgcccatgctcgccaggtatacgcgtccttctttctgcatttcctcgcttacttcagacgcccatggtggaagaacggcctgggaaggcttttctgtaaaagacacaatagcgccgctttcatcttcctttaaaataccaaaatcagaagcatcctttgcgctcacgggaatagtagcgatagatatttccgcgcccgtgtcgatatgatgtttgatcatctttttaaaatccatctggtacagctggtcaccggacaatatgagtatatattcaaactcaaagttctccatatgatgaaggcattgtcttacggcatcggccgttccctggtaccaggtgggattatcgggggtttgctccgctgccaggatatctacaaaccccttatcaaaattgctgaagtgataagtgtttttaatatgcttgttcagggaggcggaattgaactgcgttaatacaaagatgcggttcagttctgcattcaaacaattggagataggaatatccaccagtctgtatttacctgccaggggcaccgctggttttgagcggcgacgggtaagcggatacaggcgggtgccggcccctcctccgagaataatggatattacatcgttagtcataatgggaattggttttagaaagtcatcactcaattattctaagctatttcatactcttgtacatttccaggtagcgtagtgccgaactgtcccaggaattatcaatgttcatgcctcttaatcgtacttcatccaggtgcctggcatcctggtacaattcgatggcccgttttacggaatagcaaacatccgcaacgctggcctggttaaagcggatgcctacgccatcctggtctccaaagtcaataaccgtgtctttcagtccgccggtgctgcgcactacgggaacggttccataacgcagcgcatacatctgattgaggccgcagggctctaccctggacggcatcagcaggaagtcactgccggcatatatctgatgggataatgattcgtcgtaaccaatgtgcacattgaagccatagcttactactgcacgggtttgttgcagggaccattcaatatgtgggtcaccactccccagtacgaggaaatttacttcccccggcagttcatgcagggatctgccaattatttccggcagcaggtcggcgcctttgtcgcctaccaggcggcctataaaagatatcagcggcagggaggcatccagcccgaagcgttcgcacaggtgctgcttgttcgtttgtttacctgcggtgatagtatccaggtcataattaaggggtaacatccggtcggtagccgggtcccataccacattatcgataccattcaggatgcccaccattttccctctttcctggttgataagcgcttccaggccattggcattataatacagctcttccaggtagcccggggaaacggtagtaacgcgccaggcgcacttgatagccgatgcgaggggattgatagcgccgccccagtccagtataccggacttccataaatcgaaagatggaatgaggtagagtttatcccagccaaattggccctggtactgtgcattgtgaatagtaagtgcagtgggaatacttttcaggcgctcatatttataaccataattgagcaggaacgggattagcccggtatgatgatcatggcaatggatcacatccggctgatgctgccattcgttgatccagtcgagcacggcaatctggaaggccaggaaccgttctgtatcgttgggatagccgtaaacgccgggagtgtcaagtaagccggggatatctacgaggtaaaggtcgaaacccagctcattgctgcgttcctttataacgttaaagtggtaccagttgtgtcccagccacatgccggcctggtgtaccacgtcgaattcgtgggtgtggtaatatttattcctgtaggccggtatcactactttggcaaagttgccaagctggtgctggtatttgggcaacgcccctaccacatcacctagtccacctactttggctaccgggtaacattccgcgctgatgtgtaaaatctccatgctggttagttgaaatccttattaagttaaactggaaaaataagaaaacaaaaacttaaccgtgattttttacgattattatgaatatccccgctggcggggacaggacccgttgtgatagtttatatttgtaacggcgaattgttatgtgtctcacctctaaatgctgaatgctcatggattttggtcgcgttcccacggatatgctgatggacattgattttaagttgcccgcagaacctgtctttaataagaaggtattgaaaggtaaacccgtgaaaaagccgcaggcctggctgggatgcgccaaatgggggcgaaaggaatggatcgggaaaatatatcccaagggcaccaaggaggctaacttcctggaggaatatgtaaaacacttcaacagcatagagctgaatgccacgcattaccagatctacggccccgaaaccatttccaaatgggacgccaaagcacagggaatggattttaagttctgccctaaagtaccgcagtcgatcagtcatttcagtaccttaattaatgccggcgccaaaaccacttccttcctggaaggggtattggcctttggtaaacacctgggacccatctttttacaattgagtgataaatttggcccggccaaacgggaaaacctatacgaatacctcgcctccctgcccaccgacctgcagtttttcgtggaactacgccataaggaatggtttgaagacgaggccgtgcggctggaattgtacgaaaagctcaacgaactcaatgtgggcctcattattaccgataccgccggcagacgcgatgtggcacatatgcacctcaccatcccgaaagtatttatccggtttgtaggcaacagcctgcatccaacggattatacccgcatcgacgactgggccaaccgcatcaaatactggctggacaacggtttgaaggaggtttatttcttcatgcacatgcacgatgaagccacctcgcccgagctggccgtgtacctggtagacaaactggaagccgtttgcgggatagacgtaaaaaagccccgatttgtaaaagaatagcgcttttttttacgaatacattacaagggatgaaaaagacggactgaaatattaatttcgccctctcaaaacaggttttttaccatgatgcgcgacaagctagagcaattagccgggaaactggaaggcacgctttatacagatgatacgatgcggacactttatgccaccgatgcgtcggcataccgtgaaatgccgctggcagtagctattccgcagcatatcgacgatcttaagacactgatcagttttgcgcgtgaaaataaaacatccctcataccacgcactgccggcacttcgctggccggccaggtagtgggcaacgggatcattacagatgtttcccgcactttcaccaaaatactggaatttaataaagaagaaggatgggtacgggtagagccgggcgttatccgtgacgaactgaacatgttcctcaaaccgcacggattttactttggccctgaaacctccaccgccaaccgcgccatgataggtggtatggtgggcaacaactcctgcggctccaactccgtagtatatggcagcacccgcgaacacctgctggaagtaaaagccctcctgagcaacggagaagaagtaacctttggcagcctcgacgcagaaagcttccaccagaaatgcgaaggacccgatacgctcgaaacccgtatctataagcagatacgtaccagtcttagtaactacagctaccaggaggaaatccggaaagaattcccgaaaaaaagcattccccgccgcaataccggctatgcggtagacatgctgctggaaacaaatcccttcaccgccggcacggaagactttaacttctgtaaactcatcgccggttcagaaggtaccctggcatttctcacggaaataaaactgcatgtagacccgcttcctccaaaggaaacaggcctgctctgcatacattttaataatatcgatgaatccctgcgggccaacatcctggtaatggaatacaaacccagcgccagtgaactcattgaccactacatcctggaatgcaccaaggataacatcgaacaaagcaagaaccgtttctttgtgcagggggatcccggcgctatcctggtggtggagttttgccgcaatacccgcgaagaaatcattgaaattacaggccgcctggaagccacgctgcgcgcagcaggactgggatatcatttcccgctgttattcggcgacgacagtaaaaagatctgggcgctccgtaaagcaggtctgggtttactcagcaacctccccggcgatgaaaaggccgtacccgtgattgaagataccgccgttgccgtggaagacctcccggactttatccgcgacttcaacgatatcctggcgcaatacaaattatacgcggtgcactacgcacatgccggcagcggtgaaatccacctccgtccaatcatcaacctgaaaacggaagaaggaaatttactgttccgtaaaatcgcagaagaaatagccaccctcgtaaagaaatataatggctccctcagcggggaacatggcgacggcaggctcagaggcgaatttattaaacagatggtgggcaacaaaaattatgaactgctccgccagatcaaatatacctgggacccggaaaacattttcaatcccaacaaaatcgtagacacgccatccatgaacacgatgctgcgctacgaacccggacaaaaagcaccggaactgaaaaccatttttcatttcccggatcaaaccatgctgcaacatgcagagcagtgcaacggctccggcgattgccgtaaaacgcagctcagcggcggcaccatgtgccccagctacatggctacccgcaatgaaaaggataccacccgcgccagggctaacatcctgcgcgagttcctcaccaacagcaccaaagaaaaccgcttcgaccataaagaaatttatgacgtgctggatctttgcctggcctgtaaaggatgcaagtcagaatgcccatccaacgtggatatggctaagctgaaaatggaattcctgcagcattattacgacgccaacggcgttccgttgcgggccaatatgatcggcaacttcaccaaactaacttcactggcggctattgctcccggcgtttataatgcgatgatcaataactccttcaccggtggcatcatccgtaagttctccggctttgcggccaaacgctcgctgcccggcctgcacagcactaccttacggaaatggttccacgaaaaatggccgaaggaaaaacaaggcgctgccggtaataaaaaagtatatcttttctgtgacgagttcaccaactataacgataccaccatcggtatcaaagccgtacaactcctgcaccgcctgggttacgacgtacaaatgattgaacatcctgaaagcgcccgcgcgtatatgtcgaaaggattactgcgcaaagcacgcgaatatgcagaccgcaatgttcgtatattcagcaacgttattaatgaaaacgtaccactgctcggcatagaaccttctgctatcctcagtttccgcgatgaatacccggatcttgtaagtgaagggctccgcgaacaggcgaaagcactggctaaaaatgtattcctgatagacgaattcattgcagcagaagcagacaaaggtcatatcaccgcccaacagtttactgccaataaacaacatatcaaattgcatggccattgccagcagaaggcgttatcgtctgccctgcacagcaaaaaaatgctttctttaccacaaaattattcagtagaagtaatcccttccggctgctgcggtatggccggttccttcggttacgaaaaagaacactacgacctgagcatgcaaatcggcgaaatggtgttattccccgccgtccgcaatgcggcgcagggcaccattatagccgcaccaggcaccagctgccgccaccaggtgaaagatggcacgggtgtgaaagcgctgcatcctgtggagatattgtacaacagtttggcctaacgcgaattttgtcttggctcaggattacgctgattatactgattacctggatttttacttttggatttttttagatttttttgattttatttaaataataattatgggagataaaagcgaatatatccgcttctatctcccataatcctttataaaatcaaaaaagtaaaaatccaggtaatcagtataatcagcgtaatcctgagccaagacaaaatccgcgttatacgcgtcccacatagagtttcgtttcgtagtggaatttcaccatcccctgctccttgtattttccgaagaggtcttcgaggtcgcgcatcatggggatatgcgacgggtggtcctgttcggggacgtaggaggaggagagtaatcttcctttgagggcggggaaatcgaatagctgggcgttctgaaatactttttcctgcatggtgccgggctgaaaaaagccggctaactgcgacgccccaacgtttctgtgctgcatatctttatagtcggtgccgtattgatggaggagtttttcgtaacctttttcaaacggcaggtcggcctggcgtacattccacatcagtactacctttgtattttcgcggccgatgcggcggaattctgcggcggcggcctgctgatcaaaccaatgaaaagcggtgccggccaccaccaggtctacggaggcatccgggagggtggtatgttctgcgctgccgttaacggcggtgaagttcggataccggttcagcaatctttccgcggcctcccgcatatctttgttgggttccacggcatataccttgttaccattgtcgaggaatggctgcgcagaaatgccggtacccgcaccgatgtcggccacaatagtatggcgtgttaagccggtttcggcttcgagataaggaataatggccacaggataatgtggccggtatttgatatagttatctacgcgggtgctgaagcgctcagtatttttcatcgtaatgaagttagggttattctcctaatccttttggctttttctcttcattaccatgggcttcgaggtcagccagtttctttttaccgtaagatactttcgtgatcagcacatacaaaacgggtacggtaaagattcccaataaggtagcagcaagcatccctcccactacggtaaagccgatattgacacgggaagccgcgccggcgccctgtgccagacacaatggcaacactcccagtatgaatgcgaaggaagtcatcaggattggacgtaaacgcagttttacggcctccagtgtggcgtctaacaatggcatgcccctgtctacacgctctttacagaactctacgatcaggatggcattttttgccgccaaaccgatcagggtgatcaaaccaatctgggagtatacgctattggattgtttcgttaacgacagcgccaggatagacccgaacaacgcgatgggtaccgccagcaatacggagaacggtaccgaccagctctcatacagcgcggtgagcaacaggaacacaaacaggatagacaatccaaagatgagtacactactgttacccgcttcaatttcctgcagggatacgttcgcccattcgaaagagaagttctccggcagcacctgtgcagccacttctttcagcgcattgataccatccccgctactgtaacctggtttggtatcaccattgatttcaacggagcggtacaggttaaagtgattgattaccggggctccggatgctttcttggtggtgatcagtgcgctgagcggcaccatctgccccgtggcattgcggacataataagtgttaagattattgatgctggtacggtaggtagaatctgcctgcagtactacgcggaagctccggctgaatttggtgaagtcgtttacatacaaccctccgaggaaagtttgcaatgcattgaacacatcgctgacggctacaccgagttgtttacatttgtcgcggtccacctccacgttgaattgcggggtgttggcgctgaagaaagcatatgccctcgctatttccggccgctggttggcagccatcaggaactgtcccattacctgcaggaactggttgatatcaggattcgtccgctgctccagcataaaggagaacccaccggtattacctaatccacgcagtgtgggtgaagggatacagatgatattggccccgatgatacgactggtcgccatttgaattcttcccaatacggtccccatattatccccgtgcttgtatcgctcatcccatgggcggaggctcacgaaaaaggtgccggagttgggcttggtggcatttgccacgaagttgatccctgttataccaaaaaagtgcagcacggcactgtctttcagcaggatatcgctgatttgcgctactacttcttttgttcgctgggaagaagatgcttccggcagctccagtgcgatgaacatggcgcccatatcttcctggggaacaaaggtggtgggcgttttcttaaagagatagaatgccgcggcaaacagtacagccataatcaccagtactgccggcgttttacggatgctgaacatcacgcctttaccatagcggttagtaaatctttcaaaccattggttaaatttgaagaagagcttattcagtcctgtcgacttctgcgtaagatgcgcgggcctcaagagaatagccgtgagtgcaggcgttaacgttagtgccaggaatgccgacaacaacaccgagaaggcgatggttaaggcaaactgctggtatagccgtccgcttacaccgggaataaaggccaccggcacaaacaccgctgccaggatgagggcgatggcgattaccggtccctgtacttccgacatcgctttgaacgtggcttcacgcggcgacatcaggttagcatcgatatgatgctgcacggcctccactaccacaatagcatcatccaccacaataccgatggccagtacaaaaccgaacagcgtgagggtattgatggagaagcccagcaactggaaaaatataaaggtacctatcagtgaaatcgggattaccaggatggggataatggtggcccgccagttctgcaggaatacaaataccacgatcaccaccagtatcagggcttctacaaaggtttctattacttcttcgatagaaattttcacgaaagaggtagattcaaacggcaccagccatttcacatcttccgggaaacgttttgacatttcctccattttggccattaccaggtcgtttacgtccagtgcatttgcaccaggcgccaggtaaatagccataccactgccggttttaccatctgcttttgcttcgatggcataggtaaacgagccgaggtcgatcctggctacatcacggagacgaacaaggctaccattctgactggtagctactaccacgttgccaaattcttcggtggtagccaaacggccttttacactcaccgtatattcaaaagcctgcgtactgcgcataggtgcggcgcctacactaccagccggcacctgttggttctgttctgtgatggcccgggcaatatcgccggcggttaatccgagggcggccattttatccgggttcagccagatacgcatactataatcctgggaaaaggcatttacgtcacccacaccggatacacgggccagctcgggtttcaggtaaatgttcaggtagttatcgaggaattcgcgcgagtgttttcctttgggagagttcagcgcgattaccatcaacatatcattggaacgtttcttaacggttacccctacacgacgtacttcatcgggggtgcttggcaacgcgagacttacccggttctgcacatccagggtagcgatatccggattggtgcccagtttaaagctgacggtaatactcatggagccatcgtttgcacttacggattgtatgtacatggcgcctggtgtaccattcacctggttttctatgggggtggtcaccgtttcctctaccgttgtggagttggctcccacgtagttggcccttacatccgttaccggcggtgcaatatccggcagctgtgcaatcgggaggttaaacatacagatgagccctacaatcacaataatgatagcaattacgatcgtagtattctttcgctctataaatgtttttgagatcatactgtgatggtgatttaggatttattgttttgcccctgctcctgctccggcgatattcacggtatctcccggtttcacccgctggatgccgtccaccacgaccctgtcgccggctttcagtccgctggtaaccagctgcatggtatctgtaaccggcccgggaacaatgtccgtagcgccaactacattgtcttttgaaatagtatatacactggtttctgacaagttctggataattgctttagccggaattgccagctgggtggcgggagtgccgtattgcattacgatgacgatgctcatacctgacttcagcatattttccttgttttcaaaaacgagtcgcacccgtacggtaccggtttgcggatccacaatattattgatggttaacactttgcctgcttcgccgtagcgggtgccatcgccaaactggatatagaatttctgatcaccgcctttgccttgctgaatgcgcaggaattccggcaggcgggcctgtggaacatccatatccgcaaacatggggtgttcatttacgatggtgttgatgagggtttgaccggcattgatcacgtctcccacctttatttgtgcgataccgattttgccggttacgggcgcccgcaccacggcatggtttacatcggtaccggcccttgccacggaagcttttgccgcggccacattggcctgggcggttaacatagccgtataagcctgatctaccgtttgtttggagatcgcatcatggtccaggagggatttatatctttcgtagtcgcgttgccgttgtgccaggtcggcttccgcctgttgctgggtagcggctacctgtccgtaggcggcagcatagcggcttctgtcaatatcatacaggggctggccctttgttacattgctgccgtcggccacccggatggcttccaggtaaccggaaacatccggcttcagctgcacaacatcatgggccatgagggtagcagggaatttctccgacacggtatatacggccggtactacttcaacagcgaccaccgttggcttcatcttccccatcatagcagcctgttgctgttgctttttgctgttgccacaggccacacagagtatcattcctgccacataaaaggtccgcttgtaatttattagatacatatgagaaattgattgcgaattacgaatgctgatactttatttgattttgcccatggctttatccagttctgttttgctgatcagggtgtttaacagggcctgcacataatctacctgcgcctgtttcagttcactttctgcggagatcacatcaagactgctggctactccctgttcaaatttgagcacaatacgttcataaatgccctgggtgagtcccatatttgttttctgggtaacgaacctggacttgttattaaggtattgcgtattggcgttggtaacttccagtttaatctgctgggacaggtaactgaggtcgttctctgatttctccaaagtaattttgttctgcctgatctggtgtattctttccgtaccagtaaaaatgggccatgcgagggtaagtccgagagccgaggcgccgaaaccggttttatacaaatccccgaaatctgaggagaaatagttccagccatagttcacaaaaccatttaatgatggcaggaagctcatcttcttacttttcaggttcagttcattcagggcgatctgggtggtttgtatcccgtattctacgcggtcctgtacctggtaatcaacggtatcactgataaacgattccacgttgaggtcctgcacggtttgtgtaagatccagttttgcttcctggggcatgcccatctggaactttaataactgggtcgtataaacgagtaaccggatctgggtttcaatatcggttaccacattattgtaagacacctggatcctgtctacatctactctttctgccacacctacatcatagcgggcccgggtatctttcaaggttttctccagctggtccatattggctttggaaaggcggatactttcttcgttggccagcacggcgtagtaggcttttgtaatagccacgcgggtgtcgatctccgttcttttataggatttctctgccaggccgccatatacttttgcggctttcagcccgaggaagtagtcgctgttgaagatagtctggtttacctgtcctgttacagcagaggcaaaccgggttccaaactgaacggggattcttacaccggaagtcgggttggtcagatcggggatcaaagaggtggccagtttcaggttatctgtaaagctggcattgacatctgcgtggggtaacagcttcccggtggcttccttgatctgttcctgggagaaattgatatccagccgggcatttacgacatcgttctgatgagccaggccgtactgtatgcaattcgccagattaaaagcaaagggtccctgttgcgctgtatctgtttgcccgtaagctcttgttatccctgaaagtaaaacaaaggtgaatagaaaaagacgacaatgcatacgtattactttgaaagtatatgatgattgataaatacttaacaacaaacaggtaaaaaggttctgttgacgagccggctattataaggctccggaaaatgaacaacatgcctaataactgccggctaaaagctattttcgtatctttcggaaaagttattgttaactatgtctatgtctgttataaaagaacccaaaccgtttcatcgtgagtttgagctggatcgattgatgtttttcagtgatgcggtgtttgccgttgccattactttactgatcatcggaataaaactgcctgcccttccgggaaaaatgcctgccaacggttactgggatttttttgagcctactgctattgagtttttaactttcgtagtgagttttgtgtttattggaaacttctgggtacggcatcttcaattatgccggtttctccaaaattacaatgaaggattgattcatcgtcatcttttctttttattttttattgtgacgtttcctttttctacttctgccttgctgcatacgagttcccactttatgcttcctttctttatctacctgtgcaacctggcgggttgcctggcggctttgttctggatcagctattatgtattccagaaaaatccggacctggccgttgccggtcatcacacggaaaaagaactgttataccagcggtttaaatacgggtttctcactatggcaacgggtttcacctgtatagcgatgacttatttcctgtatccggagaatacggcgtaccagcgtatcagttatatgctgatacctgcgctggctttgtttaattatttccgtttaaagataaaaaaacgtaatacgctccgcctggtacacaaaatgggggcaaacaactgaaaaagcggcctatgttagaactagacaaaaaggaagcacagatagtacaacgggcgattcagtcgtggcagcgcgaccggctcatcagcgatgagcaggccggcgagctgcagaaaagctacaaggtggtgaacaccgactggcaaacgcttacgctttatatttttattgcggctatatcctgtgcgctgatggcgtttggatcactggtcctggatgagaagtggatagagattatccggaagaagttttcgctgaccgatagcgtgattgccctggtatttggtgcgctgaccatttttctttgttatgagggctggcggcgcaataaacatcagccgctgttttcgtttaaccgggagcttttctggctgctgccggttcttagtataggcgtgagcgtggtttacctgggcaaaagcgttaactacctggaaggcaattatggcgcgttctggttgctggctacggcctgctacggcgtgttgggcattacgcttcactcccgcctgttatggattgccaccctgctttgcctgatcccggcttatgtaaagctcacttatttccttaccggcgacgcagcttatttcctgggcatgaatcttccctgccgcatggccctgctgggggtgctgctcacgggcgtggcctggatactccgtcaatttaaagtatatgcacccatcaaagacattacgtggagcggaggctggctgctgctgcttatttccggctggctgatctctattttcgggaattgcggtacctgggatgaatggcagcaactgcggcaggttcacctgttgcaatgggtgatcgtttacaccgtgctgtgtgcgggcgtattgctgctgggtctcaagctaaaagacgacctgttgcgcgacctcggtgttgccttcctgttgctggacctgtatacccgctactttgaatatctctgggactttaccaataaaggactcttcttcggcatcctggcgttatccttctggtgggtagggcggctcattgaaagacggatgaaacagggaactgaacgaaaataaaaaaggcctgcggcgcgatacttctttctgaaaaaataaatgcttctttctgaaaaaccagcgccgcaggcgctcttctaggctgctaccacctctcctacggccataccataccggccggtatctttcacactccagtcgtaatttcctgtaatccaggaccggagcaccgacacgtaccgcaacagttcataatcggtttccgctcctttcaggggaaggagtttttccagggtaacaaaaatggctacttcttcattgtgcatccggacagcttcgttaatcgcctcctgcaggctgcattgccgggcgtgttgtaataccagcaccaggttgtgcacgtcgccctgcttcgcttctttcgtacaggaaaacaggtcgtttgcccagcaaacaatattgttgcaggcctggatcatgcgctggatcaggggttgttcgaccacttcccggctgagatacactttttcgatgatttctatggcttcaatatccgccaggagtgcgccggtaaagggccgcatgtgcacataatccgccacggagggaacaataccggcctcccggttttcggcttcccagatgcaggacgtaaaataatcgtccatgctgcggataaaacgaaggcgccaggcggggctgctgatggcgcgcatgcgctcccatatgctgctcagggccgccggcagcgggccaccggtttccggggttactacccggttgtgatgcaggatgtccattaaccccgccatcatgcttttgagatagtcggctttgcggcccatggaggcttcgtcgcactgatcatcaaggataaacagccaggtgttgaaatccgcgatgatgcaaagctcgtgcaaagcggcatcaggaaaggccctggcagccagccaggcgaaccgggctttctcaaagcgccgccaggccagctcagaagtgatcagaccataagcttgtacccaggaaacaatgtgttgctgggcttcatctgcgtgttggttaacgccggaagggaaagggtaactgacagttggcatttggatggttgtcatgtgtctttggatttaatagttaactatggtgggtaataaaaatgacgttggcattaccgggcgggaatcccggaaaagtgtgaaggagcgggcacagggaagcagccgctacttaaagcagtaaataaggcaggtaggtgctatcatcattttaattaaaatgatccggttaacagcaaaattggcatagtaaaataaaagtttaattatacagcgctgatcggcgtacccaggtattgtaataccattggcagtgcacgatgaaaccagatggtaaatgcagccggttcttttttcattaattccagtatctcgccgggagacaggtagcggtaatcacacacttcggatgcttcgggaaatatgttgccgttataggtacccagcaatacatgatcaaattcgtgttcggttaacccgttatcaaaaccggttctgtaagtaaaagaaaaaatctcctgcagatcgcaatcgaaacccatttcttcccgtaaacgccggtgcgcggcagcagcagtatcttcacctggatacgggtggctacaacaggcgttggtccatagtccggcagaatgatatttctccagtgccctgcgctgcaataaaatctcgcctgcatcattgatgataaatacagaaaaagcgcgatgaagtaatcctttctcgtgggcttccatcttctccatcgtcccaatagcctcatcctgttcgttcactaatattacgtccggtgatttcatagactgtcaaagatatttgatttacgcttccggcagataaaaaataggacaaagaatcaaaaaactatgcttaaacaaataataattggttgagtggttaacagcaatactttaacggttacttagataaatataatataaattttccggacttttgcaatattaacaaccacaaaaaaatggcagaagacttacaaatcatcaaaggaaataaagcggagcaatacacttctcttctcccccagataaaaggattactggacggggaaaccgacctggtggccaatatggccaatgtggccgctgcgctgaaagagcagtttggatggctttgggtaggtttttacctggtaaaagaagatgaactggtactcggtccgtttcagggcccggtagcgtgtacccgtatccgtaagaaccggggtgtttgcggcagcagctgggcacaggcccaaacactgattgtacctgatgtggaagcctttcccgggcacattgcctgcagcagcttatcgaaatctgagatcgtggtgccgctgatccgtaacggcgaagtaacggcgatactggatgcagacagtgagcatctttctcattttgatgttactgaccagcaatacctggaagaaattgtggcactgattgtgtgatagcaaagcggattttcgtatcatcgctttattgagagaccattattatgctttttttcaggaaaaaaaataccgaaacaacgccgcctgcagacctgctggcgttcatggctacagatatccactcccacctggtgccgggagtggatgatggcgtacctgacgtggctacgtcgttacattttattgaacagctgcaggcgatggggatccggaaaattatcactaccccgcatattatgatggaccggtacccaaattccgccggtacattaaccaatccatatcaacaggtacaacaggagttgctccggaaaaacagtccccttccttttcactttgctgcagaatactatctggatgaacagtttgtgccgctgatgcagcaacctttgctaaccatctccgggaacagggtgctggtggaaatatcgtttatgtcggctccgccgcaactggcgcaatggctgtttgatatacaggccgccggctatcagcccgtactggcccaccccgagagatatggctactatcacgcaaacataccgcagtacgaacaactgaaacaacagggctgcctgttgcagcttaacctgctgtcgctcaccggttattacggaaaacatgtacagcaggccgccgaaaagctgatggcggctggtttatttgatcttatcggtaccgatcttcatcatgaaaaacacctccgtgccattgccggcatagccaaaaatacgaagctccgcaaggcattggaagcctattcctttggcaacgccgcattataatatcattggatcagcatcaccgtaccggtttgctttctcgcctgttgcttgctatcagtatacaaaagtacccacacataagcggccgccggtaacattttccctttgaaaaggccatcccatgcgccatccgggctattagtactaaatactgtttgtccccagcgggtatatacttccagcttgtagtcagttacatcatcgtgtacttttgcacggaacaggtcattctgaccgtcgccgttgggggagaatgcggtgggaacgaaaacggcgcactggcggatgtttttatcaacatctgcagatcctttcacctcacagtcgtttttatcttttacctgaaaataatacctgcctttgtcaaggtgtccaagtatgctgtccatctgccattcagtgccttccaaacgatacgcatagggctgggtgccaccgtttgcctgtaaaaagatcctgccatcagttgtttcgctgcaactggctgctttcgtggtaacgctcaacagttgcagtttcggtggttctttcaaatctattttttcatacggatcttcacatccctgttcatcctttaccgtcacgcggtaagtaccgggatgcagctgattaaatgcaggtgtgtaactgggttgcgtatcgtcatttaaataataacggtaaggaggaatcccgccgctggttgtgagcgcaattccattttcgttatccccgttacattttgagatgatgatgtttacaacgcttttcagatccgtttctttaatgatcacatctacagtaaccgaagcgccattaagcgcagtaacagtcaacttataagtgccggcagacaagccactgacatgagaggtcgtttgcccgccaggcatccataaataggtgaccggattatgggcactgagcagcttcacggatgcttcgccggtactggcatttttacaggtggtggtagtggttactgatacctgtggcacctcgcggatagtaggagagaaattatccaccaatacagccgcataacttctctctttacatttaaatattgaattaggtccgaaaatgatctgccggtaatctttttcaggcgtaaaaaccggagcgtaacgtttccaggtggtgtgattaaaattaccggattcccagagcagttccggttgttcgccgggattacatccataaatagcgaaagagccattacaaatatctctcgtataaaatgtggtagaagcaaggtctactgaaagcgtatatgttttacctgcttttagcggactgcgaagattttgtccaaaaagttcctgccaatcatttgtaagcactgcgccaatataaaaatctccggctgacgcaggaaaagaaaaaccggcaattcccggttgctgatccggcgattggcttatcaccagccagggcttgggtaaacgtcctgacaccgttacctttccttccaatgagggattatctattacaatatcctgtgcagcagtatcaaaggcggatgttaaaaaaagggaaaggaaagctgccacacaaacaactttccttaacaagctattgcttattaaagaagcgtctgcacgggctttcaataatgcgatatgcactatacaggatatggtcttcatagataatactaatttcaaaaacaggatactgatcacatgtacattctcccggttgagggaataacggttgaaaagtatttatattatccaccatgactaatgtaacgaatacttcattgatatccgtgcagtttttttccagcgtacacagtggtataaggattcagcataaaaacaggattaatcacctaccactgttagtggtggtaccacatcgccctgtgcaataacggtatttctcattataacggcaccctggcctatcagtgcgccattaccaataacagcgcctccgcctatataggcattacctgcaatatgaacatagtcacctatcaccgcgtcgtgatccacaacagccccggcattgatgatggagtgatttccaataatgctgttggcctgcactaccgccttggccagtacaacactgccttcacccaccaccgcattgccggctacataagcagccggatgcactaaagcagtaaaacgatgcgataccttttcagataaatgccgccggacttcgttattaccaattcccaatacaagcggcacctccggaaaaagtgaaggctgatatgcctgtacccgggagctttcacctgttgcctgatccgtgaacattacgggaacggatccgcctgacaacatgaccagatcagccagtacatttgcgtggccaccagcaccataaataagacacgactccattgttaaacagttttatgcatcagttttgattttgcaacaatgtacaccagcaccagcggcaaacataccactaagatatttaccatcaggttagtggcattgccgattacaaaaaaattcaccagcaactgggccgctgcatataaagacgttactaccaggtgtggtatttttctttcattagccagtatctggtaaaaatgcaaacggtgtgctttaaaaatattctggcgtaatgacaaccggtgaatgatcgttaagatagtatccaccccatatacagaaaggaacaagagatacttccagtcgccggtagtaaatatcagtttcagcaacatggtaacgatccagaaggcaatggtaacgcttcctacatcgccggcgaaacatgctgctttttttctgaaattaaagaacagaaacacaacacatgccaatgccggtaaccagataagatcttcactgataaaagcctgttgccggatatttacatactgcatcgccgccagtactaccaggctgtataagccggtgataccattgatgccgtccataaagttataggcattaataatacctataacaaggatatacaacaggatcaccataaaaatatttacgttggcgaatacctgcaggtagtaaagcatcatggttacggcggccacctggaatatcatccggacgcggttaggaaggctgtagatatcatccaggaaactaacggtaccaataatcagcatacccagtacgggcagccagtattcatcaaagtgccaaaccagcgctgccagggcggcaacaacaaagatgattccaccaccccggatagtaagggtggtatgggaactgcgttcgttgggtttgtcgataatgttataatgcgcggctattttaaaatatactttaatagtaagaaagaaaaccagcgctaaaacaaggtagatcatacaacaaatcgtattttttctgcaaccggcgatggcctccagttaagcgaagatttcgccctggcgtcatcaaaagtcagcgttgctgttattttttttaatttatccgtattaataggaaatttgtctcccattacatctccggctagagccagcagttttgccagcggaagcggaattgtcagcggagcttttttacccaggccttcggctattttatattccagctccctgaaggaaggatgccggctatcagtcagattatagatacctcccctttgcgcaactgcaggtataaccattgccacatcgtatgcccataccatgcttttgcgggcatctgccttaccgatgctcaggtaccgaccggtacggatgccatttatcattgcctgaaggttgccgggaggagtgggtccggctatcagcggcagccgtaatatgcccagtttaacattgttaacggccgcccattcctgcaggtattcttctgccataattttactctttgcatacggactggtgccgtccaacggatcatcctcgctgataagcactccttcttctttcccataaactgccaccgtactgataaaaataaaggaccggggaactttaccttcctgttgcagcgactgacacaagtttactgttccacgataatttacctggaagaagctttccttttcctcttccgtttttggcacgctatgggccttccctgcacaatgaattacacaatcaacatcaggcaggccggtaatcagttcctttgaaaaatcggcggtcagatgcccgccgtttgctacagcaggtcctcttcccacagtggtaatgaggtgctgcgaagaaagaacctcgtatatcacctttccaagaaaaccggatgccccggtcaatagaatatcagttttcactcattgtcagttttacatacttatccaaaatgatgtcctgtgcataattattaactgccagggctcttgcattcttacctttctgtgtaagctgtgctacatcagtaacggataatccattgaaaaaatcaagcagggccgctgattcagacacatcaaaagtccaccctacattgtgttcatttatcatgagtgaaatctcgctgttggcattgccaataaacaatatgggcttgcctgcagccagaatgttatatgacttcgacggtactcccaatcctgccattccttcctgtaaagacacgataccgacatcagttgcgttcagaaactcctgctgtttgctcctggagaaagaatccagcatagatacgttactcaattgatgctttgctataaactgcagcatttcctttttcaccgcgccttcgcctataaatataaaatgcagcaacggattccggatatctttgatgacatgacataattccattaacccctgtaccctgcccaggttaccggcaaactggaaaatgattttatcggcaacacccagtttcctgatgacagggttttcatctttcgctgttggagcaatagataccgtatccgcccaattctccacaatctttatatcaggttgctttttgtacccctgcaatttggattcaaacaccgctttcatatccctgccgagcacaaaaagtaccgccatattactataagccttgttaaaaactgatttcaacaaacgatatggcaagcttcccggcttcattatttttgccgccaccaggttctccggaaacacgtcatgtacaatggtaaagcacttcagggatttccatctgcacacccatgttaccagtggcactacgggagcgggattggttacgatcagcacgttgtcacctctaccggcttttctccataatttatacgttaactggatacttagcaatgccatccgcaacgcacgttgcaacaatttatctttattcagcccgggcgttttcacccgcgtaattgttatgttagcgttaagtgcttccgtggctaccaggtttgatttctgataggccgccggcccgcatataacatgtacttccgtatccctggcaaaatgctcgctgatctttgtcatgatatacgcagtggaagtttcttccgggaaaaacaactcagtaactacccataatttccgtttgtcttttttcattagtcgtttattttccagacagtccttctcacataatccacataagaaataatgattctgactactttatcggaaacatttggcatggaatagtcgcttacctccctgaagttcctgcgatcaccccgttcctggtattcaagctgttgaagaccctgcaatatcctttccggattcagtcctaccatcataacagacgcctcttccatagcttccggtctttcgtgcgcttcgcgcaggttcagcgcggggaaattaaggatggaagattcttcagagatagtgccgctatccgacaataccgctttggcctgcatttgtaaggagatataatcactgagaccgtatggtttcatgagttttaccagggggttaaacgtcactccttttgcctctatcattttgcgggtacgcgggtgcgcgcttacaatcaccggcacattaaatacttctgcaatgctgttcagggaagttaccaggtggttaaagttgcgttccgaattgatattctcctcgcggtgtgcagacaccacgaaatattggcccggctgcagcttcagctcctccaggatggtagcggcttttatcttcggcatgtagtgatgcagcacctcatacatcggactgcctgttttaatgatacggtctgccggcagcccttcccttagtaaatattccctggcaatatctgaataggttaaattgatatcactgatatgatccactattttccggtttgtttcctcgggtacccgctggtcgaagcaccggttacctgcttccatgtggaagatcgggatctttctcttttttgcgggtatagcgcataaacaactgttcgtatctcccagtacgaggaaggcgtctggttgtatggtttccagtagaggatcgattttaatcaggatctgcccgatggtttcggtggctgtttttccggcggcttccaggaaatgatccggcttccgcaaaccaagatcttcaaagaaaatctggttcagttcatagtcgtagttctgaccggtatgcactaaaatatgctcaattgctgccgattcatccagcttcgccaatacccttgataagcgtatgatctcaggtctggtgcctactaccgttaatacttttaatttcttcgtaaccgtgctcataaaaattatatgattaattagttgctataccgtttcaaaataagtatcggggtcctgttgatcaaagaattcattgatccagaatactgtgtacagttcttctgtaccggtatttttaatattgtgtgtataccaaacgggcatatctacataggaaggcgtatctccatccagttcgaaatccagcacttcatctgtattatatttcctcagctggataagcgccttccctttaatcaccaggaaacgttctattttcctggtatgaaagtgattccccctggtgattcccgggtgtgtggtagagaaagacacctgccctcctacttcgaggcggatcatttccacaaatacaccacggttatctgcgtgttttttgagggggaaaggaaaatagtttttatggtctatataactacggaatgtattaaacagctggatggtgaattggtccttcatttcggggaaaacaccttgttccaggtataactccctgaaggtattcagttttgccaggatttcagacacatatatttcactggtgggcgctacttcatatacgccgtcgttgttgccggtttccactgcatggatgatggccgtagccagttcatctacataaatcagtttcagaaaaccatcctgatctattttgggtatttgattattacagagctgatggcagaaggtagccaccacggaattataaaacggtttcccaaatggcccgaatacattggggattaccatcccggtaaatttggctccgctggtagcagcccattgctgtaataattcgcggccggctttctttgattttccataaagattatcccgttcttcctgagtggaagaagaaaagatgacatgcggtttattgcctgttttctttaatgcatttaccagttgctgtgcgagacccagattggtatcatggatcacctgctgatccggatgccggttcaggccggcgagatgaacgataacgtcacattgccctgcccagttttccagggcttcggcggtatcaaagaaggatctgtcgaacggcaccaatgtaaatgtttcctttaacagcgaacacctgttaaacaaataagatcctacaaatccattctgtccggtaataccaatttttttcatttataaactacttgatttatgataatagttatgcggtctgtttacaacctggcatgctgccaatcgaaccactgatcttccgggaatgaccacctgtcggcggccgattcctccagggtcagatcgctgtaaaccatcagcactgatccgggtataagtgccttgataccattggcatatccggcgggcacactcaatactaccggctcatcttcatttaatatcacatggtctgccttcagtccgggagagggtttgtcccaatcgtctattttcacccatgccagtacaaaagctccttttaccacgtaaaaatatttctgctccacccggtgaccctgccatgcacgcacaacagagacatcatgatgtaacatttggtaaaatctttttacgtccggaaaagagaaatcattgacaaatttcagcgttcccctgtgatcagtgaaggatgctccttttatgagtgttacttctttcattcaatgttattgtttcctgtttattgctaatgtacaaactgaaggtccgtttttttactaacggagttgatgattaagttccgggtctgactggaatccaataccctcctgttggcggaggatattttaacaccggagaaattcagcttcaggttcttttcatatacacccatggcatcaagggctctttttgagttgctgttccagtgtggattaataaccgagatgttcccgccaagattaccgccgttgccaggctgcagccgataggcaactacccttagccctccggcggaataattatcattatggttttgcacggttacatctaccaggttgttacccccgccatataagcgggtaatgttcatcaggataccatagctttcatttttttccgttaccgcatctgtgatacggatgcgcttcagtacattttttgcattgttaggctctacgtcgataccgcacataggagattggccgtttgtataccccgcatagggcgatatcagctgaagaccgtccacactcaccacagaaatgccgtttctccggttattcctgcaataggcgccggaaatcaggatgtcccggctttccctgcccagtttcatatcttccccgatataaataccatctccccagcaatcgtatacctttgggtttttgatagtaatattattgccggaataaatgccaattcctgcaccccattgaccgcctgttccgagatgctgcttccggtcgccatagatcaccggatttacgatggtaacattactcacatcacgcatccttaatatcgcatacgacccagcggtggttggcttcaacataattttcgccccactctcaaaagtaatatgcttattgctgccaatgatcaggcccttatcatttaccaataccggaaaaccagggaagatgattacatcatgcgtatcaatggccttttgtattacatccgtataatcgacagaaccatctttcacatagcccggtggcaaagcatcttttatattaaacgcggcggattgatccggtgtacctgatgcagtacccacactatatattgctgtttcccggcaatggctatcaacggcggaatttacatccggagatgcaaaaaccagactaaaggcaaccagcggatataatggcaagtggatcattcctttgctttttaatattgaacgttcgtgtttctctcctatgatgctatattggccacggcttccttgctgttcatcagttccgccttcacgagcggttgtttcgccaacagcttcttcatagcctccacatccagttgttccgcgttatgggaatgataatcatctacagtggctacattcacttctccttcagagaaatactggctgtagttcaggttcctgttatcagcaggaatacggtagaaatctcccatatcctctgccttcaccatttcttcgcgggtgcaaagggtttcatataatttttcaccatgacgggtacctattatttttatttcgttatccgcatggcataattcttttaaagcggctgccaggtcgccaatagtaccagccggcgctttatttacaaagagatcgccctggttaccgttttcaaaagcaaacaacaccaggtccactgcttcttccagtgacatgaggaaacgggtcatattcggatctgtgatcgttaaactttcaccgtttctgatctgtttaagaaacaaaggaataacagagcccctggaccccattacgttaccgtagcgggtaagacataccctggtagcgttttcgggaatattgcgggaagctgcaatggctaccttttccatcagggcctttgaaatgcccatggcattaatgggataagcagccttatctgtactgagacaaattatcttcgatacattattggctactgccgcatcgatggcgttctgcgttccaaacacgtttgttttggtggcttctatcggaaaaaactcgcaggaaggcacctgtttcagcgctgccgcatgaaatacgtagtcaacgccacgcatggccttttcgatgctgttataatcccgcacatcgccgatataaaacttgagcttcccgtttttcaactggttgcgcatatcgtcctgtttcttctcatcccggctaaaaatccggatctccctgaaatgatccgtatgaagaaacttattcagaacagcgtttccgaatgaacctgttccacctgtgatcagtaataccttatctttaaacatatcagttcttatagtttaatgaatacatttttaaaatcaaatagggtgtcaggtaaactacctttgacataaattccagtgttttcctgttcttaataaaatatttctctgtaaaatcaatcagcgagctgccggccttacaaaatttataactgaaccttacgcccggcttcagcgtttgcaattccggtttaatagcgttgttattattaaagagcgtccagagctgcgccttggactttatctgtacccttgcccgcagcgccgcattggcgcctctcagccgcaccctggtaagagatgcaggaatagccagcaacggaaacaatctggccatcatgatccacaaataccagtcctgtccgtgtctcataacatttgaaaatctgcatgcggggttctctttcaggtattttgcccggatcatcacacaaggagtggcaatgggcgtagaaagtaaacccctcttaaatacttcgccgctgaagtcagaaatgtctaccagtttataatcggcttcactgccatcatagaatgatgtatagctggtatgcgaccatactgcgttctccgcaatcatggcattaagctgcacttccagtttctccggcatccaaagatcatctgaatccaggaatgcgatatattctccctctgccatttctatgcccaggttcctggcgctggcagggcctgcattctttgtttttatgtatttgatcttagtttcatactgcatcaaaaagtaggtatcatcttccggtgatccatcattaatgaccagtatttcataatgcggataagtttgggccaatacactgtcaatcgcctgagccagccagtcaacattcgtataaaacggaatgattacacttattttcgcctgattcaccatactattcaactgctgttttatgtttgattaatttagccggcgcgccccccacaatgctattgccgggaacgggttttgttacgatagcgccggcggcaatcactacattatctcctatttcataaacattcgacaggatcatggcattcagtcccacccatacatttttcccgatcaccagtttcttcccctccggtttacttctgggatccaatccatgatcatgagattggatgataacgccttccgataataaagtacctgctcctatatgtatgtccccgctaaaatcgatcctgcaattccggccaatcaccacatgatcatccagcctgatttttcctgcaggtatttctgaggagaagatgacattcatacctattgttacattgtttcccagggaaatattgccgggatttctgtatttgaatcccctgagaatagtaactccttttccaacgctgcccaggttcttttgtaccagggcgccacccagcttatctttgaactgctcaacacagcgggaggccaccagcattaccagtcctcccacgccacttatcctgttattccaaaaaccgctaagccttgccattactaatcatttttacttcgtccaaaacaatatccaggtgggatttgctattctcttccagatatctttttatggtagcggtgccgtttaccgccacctgtgcgtgttttttataattattaaaaaagggcaacatcttcgcatacagatctgcgccgtttttaggctgtatttcataacagttctcctggtctttcatcacgtacgaaatactccctacaaacgtggtaatgataggcgtaccaaagatcatcgcttcatagagtaccctcggaaatccttcatgatgcgtgggcagcaggaatacatctgcctgcaggtaaaagtcccggatacggtctttatcatataccgggccatgcaggattaccttgtcagccagcacgctgccttgcagcatttgctttacggcctccatatcggctccttcccctgccacgtccactacaaaattggtgatgccgctttcaagcagtttatcgaacgcttctatcagctcgtaaatacctttgtcgcgctccacccttcctataaacagaaaacgcagtaccggctttgcttcataagtcctgtccgttacgatatccccggccccaaaccccatcatgggtttgatggtatatgactggtcgcagaacggctttgtattgttggtaaaccgcggagacacggtagctataaaagccgcacgtttaaataaaaaagtggatggccagctgctgatccccttctctcctctcacatacaagccaaaaggttttcttagtatcactgctgcaaatcccagtaaaaagaaactgttgggataaaacagataaaggaaatcattgctcattaaccgttttaaaccggtggtataagccactacataagacagtaccttacttttcctgatctttaatgccgttaactgtatttgcgtttctttcagattgtaattggccatagcgtcattcccgttgaaaggacgcttataatgaaagttctctatctggaaaacatgattcagttcattcagaaattttcctgtttccttatagatatatagccccttactatcttcaaacatcgcattactattgataactaatatcttcatggaatatcaattttgttgttgtcctttgacgcttataggtcatgaacctgataatggccagcaaaataatgggccataaaatattacggaacgcagagaaataggatgctcttggataataaatcgcgaacgacatggagatcacataagcgatcacataattaatatcctgtgaataaagcatcttctgctgaaatcttgtatgtatatatccgaaaaacaacatgaatgccaccactcccagcacgccaaacgacaggtaaatatcccctatcaggttggttcctaccccccaggtggcatcatcgccgatggtaagtttattgataatccttcctgaagacatctcgtcttccgtcatcccaagcaccgacaatacaacaggttgtaaaccaggcacgatccctactacctgggtgatcatggttttgccgtagttgatgccgttcttgtcggcataatccaccgctacatacaggttcctgttgttcatcgtcaggtccattcccaaatcaaaaatggagttgaatttcatattgctcgaaccccgctcaagaaatcccccgatggagttgctgtcgttaaaaccggatgttctggttacgcgggcggaagaaataaacagcatgaggaacatgccaagagaagctccgagcaggaatacttttagcttcactttttttacgtacacggcatacagcgttaccaggatcaggaatacctgcaacgcaggtcccctgtcgccgataaaaaagaacaacaatatgaacaggaacataaatcctaaaaaaaccttatcgaactgcccaacgaatttccagaaggtcatcttttcggaagacctgtaatagccggtataacaaaccactgttactgttagtgcgaccagtgactgaaacccgatgaggaaataattggaactggaggtgccggagttgaagataccggagaagaagtcgcgccccacaaaagccagaaacaaaccaaaaaaggcatatgtgagcagcttcagaatcccggtaaaccgggcaaactgcattgggcggtagttcgcttcaaacgtataatctgattttattctcagcatggccgcgccaagtgtataggcgcttgatcccagcatagcgagcgcggtagatttagagatcaggttctcgttaaaatcgtaattaaatacagggaaataatacttatctacaggaaataaaaagaccgggtacacaaaattcacaaaaaagtagctgatcaggaacagcacatgaaaattgaaataatttccattagaccgtttccggatcacccaaagcgatgaaaccaggaatacgacgaatgtaagcacgcaatagttgtatgaatacacaccgggtgcaaacatgtatataacaattgataccagtaacaggatgatttcaacaatcatttattacaatctttatgattatccaaataaatacctatagccattgctgttatttttttgttttgtatatcgtcaatacctgtttaccctcctttacaatatcggacaccctgaaaacacggagcagcacaaagtaagtagccgcaaacaccggtgttaaaagcaacaacagcggtcctttcagatttatgtagttaaacagcaggccccaggcgagtgtattaaaagcagctatcacaatgatctttgccactactatcagctcatacgcggaaacacttccaagtattttacgggaatagtagaagttgatcaggtaactgatagctgatgtaataacaaaacccacgagcatgatatgcaggtccctgtaaaatactcctatcacaaggctgacgcagagtatcgcctttttaacaagttcaagatgcagtatggtcctggttctgttaaataccttgaaaatattccggttcatggtttcctggagaaaaaagaaggagcccagtgtcagcatctggatgaaataagtagagtctgaccatttagcgccaaacaggaatacaattatttcctttgaaaaaaggaaggtaactgatgttattaatcccatgagcacggtaaacaacagaataattttattataggcacgggaaaactgttccttatcattttgtaattgtgataaagaagaaaacagggctccctgtatggttaagtttaacacgttaccgggaacatcctgtaatttttttgcctggtaatataatccgacctgcataattgaaaaatactttcctattattatctggtaaatattatcaaaggcagtgttgagaatagatgccagcgtggtatttacgccataagcatataaatccttaaacgacgccctgctaaaaatccatttgcgtaccggtccttcatagtaccataacagtatggtcaggaagagggaagaaaggatctggattaacaccatagcccatacaccggcccctttccatgctgcaataatacctatgaccgaagccagtgcaatggcaacaaaattgaaaactgatttccttttgaaggaaagctctttaaccagttttgcgttctgtaccatttgaaacgcattaataaccagtacagtgctcagtaccattaatatgcgtttcaatgacggatctttataaaaagcagcaatggttcctgcaaacaggatcagcaataagcaaagcgctatgcttacaacaagattaaagatgaataccgttgaaaaatctgtttcactggcatcactttttcttaccagcgcgccgcttaatccgctttccgtgagcacatttgcgatcacgataaagaacatcacaatacccacctgcccgaattcataaggggataatatcctggacataatgatgttggtaatcaacatcactcctacgtaagcaacttgtccgaacattgaccaaaaagtacctgtaagtactttatatctaagtgctgtcattaaaaaagaatacggtacgtagtttttacttaaaatatggaaaggatttctgttggtgtaccgcatcaccggcacactccgggagaagtggcggtgatggtttcaataaagacatggtatcaacagaatgaatcaggaagcgcaaaaactgataatcttcctggttctcctattactcaaaaatatggttatacaataatattatacttcttcttactgacggctgtcccagtaccagttacaagccagtttcagtccatcgcgcacagaaaattccggacggtatccaagaactgttcctgccttgtttatagaagccagcgaatgaggaatatccccgttcctgttacctccgtgtttaaactccgcctggctgatagccgggtcaaaagcagacaggttatcttttaaaatctgtgccagctccagtaaagtggttctttcgccaaatgctacattaaacacttctgatattgctttaccagcggtatatgattcgcctatcccttcgtaataccgtgccagatcctgtttcaatgccgcagatggtttagcggccgccagcaggttcgcctgtatcacgttatctatgtaagtaaaatcccttgaataggaaccatcgccattgataacgatctgctccccgttgatcagggacgaaacaaacttgggtatcactgcggcataggccccgttggggtcttgtcttctgccgaatacattgaagtaccgcaaacctattgtttcaataccatagatatcggagaaattttttgcaaataactcatctacatattttgtgatggcatagggcgacagtgcatttccaattttatgttccacttttggtaaatcaggatgatcaccataagtagaggaactggcggcatataccacccgtttaacacccgcttcctttgctgcatggagcacttttacaaaaccaccgatatttacgtctgtggtagtcatgggatcaatgatagaacggggtacagagcccagggctgcctggtgaaaaacgaattcacaaccttccgctgcttttacgcaggtttcataatcgcggatatcgccctccaggagtgtaaaaccgggctgttgctgtgcaggttccaggttagtctttttcccggtagcaaagttgtccaaacagatcacggtgttgttctgcgccagtagctggtcaatcagattggacccgataaagcctgctccccctgttactaatattttactattactgatcatctcgtaaatactatcttttctgctttaatgataaaattcctgcctgatgaatacaatgtatgtacaatggcggcaggcaattgccgaaccgccattgacggttattacaatctggcatcaatgctgtttacattcaatacccctttcacatcatagatcactttattttccttacagagcttacccagatccagtgttttgaaatcgtcgtgggatacagcaaggatcaccgcatcaaattgttgtaaatttttcagttctgtaacagactcccatccgtattcatgtgccacttctgccgggtttgcccacggatcgtaaatggtgatattggtatcgtagcctttaagtgtatgcaggatatcaaccacttttgtgttgcgaacatccgggcagttttccttgaaggtaataccgagtacaaggatgttggaatttctgacagcgatgtctttctttaccatcagttttaccacttcatgcgccacatattctcccattccgtcgttcaggcgacggccagccaggataatttccggatggtaacctacttcctgtgccttttgcgccagatagtaaggatccacaccgatacagtggccgcctaccaatccgggcttgaagttcaggaagttccatttggtaccggcagctttcagtacatcgtcggtatcgatgcctaaacggttaaatatttttgcaagttcatttacaaatgcgatgttgatatcgcgctgtgcattttcgattaccttggctgcttccgctactttaatacaggtagctttatgcgtaccggcagtgataacggagttatatagctggtctaccttatctgctatttcaggggttgagcctgaagtaactttctttattttagcaaccgtatgttctttatctccgggattgatacgttcaggtgagtatcctgcaaaaaagtcaacgttgaatttaagtccggataccttttccagcaccggaacacattcatcttccgttacccctggatatacggtggactcatacactacgatatctcctttcttcagcaccttacccacagtttcacttgctttatacaagggggtgagatccggtctgttatatttatctaccggggtgggtactgtaatgatataataattgcagctgcggatatcctccagggtactggaacagtaaagtccggccggagcattgttgtctgcagtaagtacatttttcagatctgctgaggtaacttccagtgttctgtctgttccttcgttgagttcctttacccggctgctgttgatatcgaagcctatagttttgtacttctttgaaaattcaaccgccagcggtaatcctacgtaacctagtcctattagggctatcctggcatcctttacggatggagcattattgttcatatccaatttaattactgtttatgtccttgtttattagcttcgtgaaatagattttcctattcttttaaagatgccttttttgttttcttcctcatatccgtagccatagccatacccgtatccatagccataaccataggtgctgccgcttttaacgtcattgataatgagattaagtttaggcatttttctatgaagatataattccctgctgatctggagctgatctttgaaagtatagccctgccggaccaggtagagggtggcatctgcccatttggccagcaactgggcatcagttaccatacctatcggggcggtatcaacaacaatatagtcaaagttttctttcagctccctgaaaagcgattctgttttatccagcagcattaattctgcgggatttgggggaatcgggccggaaggtataacataaaggccttcatgtaaccctgatggctggataataacatccatcagtgattttccgatagcataagtgctgaatcctgcctggttactgagtcccagcatggtggatattttgggttttctcagatccatttccatcaggaccacttttttgccggagagggccagcatagttgccaggttggtggcaacaaaggacttgccttcgccactcatactggaggtaagcaggatcactttgtcgttggcgccggacaatacaaactgcaggttagtgcgtaacgcccggaactgttctgccagcggggttcttgtattgttactgatcacagcttcgtgtttatcactgtgtccgatctctgataagataggcaccggtgtattattggtaatatctcccctggagcggatacgcctgctgagcatttctttcaggtataatatcaaggcaggaagaccggcgcctaatattaaacccagcgcaaatataaggagctttttcggtgaaaacggcagggcgtcgctctttgcggggtctactacctgggcaatggccaggttggatgcctttgaaatagccgattcctcgcgtttcttcagcagaaacaggtacagttcctgcttcagcgcctgttgcctggagtaatccaggaatactctttcctttgccggcacctggcggatctgctggttggcggcatctgcgttcctcttcagctcccggatacttacctccacattacgtttaaaggacgacaggttgctgctcagatctgtccgcaatccgcttaattgctgatctatattacggatcatcgggtttgattcggtactcgacagcaacatccgctccctttccagctgcaggttgttatatttttctaccagtgaggcaaaagtaggatcttccattaccagggcagaaggtacaatacgtttattgttcttgtcgtcctgcacatactggttcagggattctattatattcaggcgtacctgctgatctatcagttgcttggcaaaatcattggtattggagaataataatttggattgttccgtcagatctgccagttcattcgtttgtttaaattcctggatatctttctccaccccgcttagttcgcggcttaccaccgacaggcggttatccacaaaagcaatcgtactgtctactatcctgtttttgtcttccacgctgttgtgcaggtatacgtcaatcagtttatccaggatcttttctcctttaccgggaacggagctggtaatactgagatctactgtacttacctgcttattggccacactcacatttaataccttctggtaatcggccactgttttgtctaccgaacggattttaaccaggtatgcatcttcattcagcggtacagacgccattcttgttacctgtaagattccttcccgggtatgtaaagtatcgttccatttcagtttccttgcctggccatcttcccttgtgatccggaaagcggtttcagattctgggatcagcgaataatttacttctttgttaagcgtatcccggagtgtgatccaatgaaatgcaaagggaacattattgaattgttcgcttttctttacccttccttccacataatattcaacattcagctgcatatcctttaccacccgttccatcaggctgcgggatttgaggatttcagcttcattatccacattacttttgctgtcaaatatttccagttgctccaggatttctcctcccgggatgctgggccccttctgatcgtctcttacgagaatcttcgcacttattttataagttggtgtggcatatctcaggtacaggtaggcgccgaacacacaaaccagggtactgatgagaaaccagtaccaatagtgccacacccaatccacaatttgcctcagttcgaaaccgttttcctttggctcctctgaaggcataaacccattgggaggcattttcccgttcccgttagtataaaatgtttctctcattttctaaaaattaaccctggtcgcaattactatcaacaaggaaagtacagatgctaaaattgaaatacgttttacctgtgccatatctgtggaggctgatttagccttgtttggttccacatatacaatatctccctggtgcagaaacaggtagggagaagtaaatagcttactgtcattgagattaaaacgtataaactctttcttcccgttggtttccctgatcagcaacacattttccctcttgccataaatggtcagatcgccggctatacctattgcatccatgatcgttaccttttcattgggcattacataggacgatggcctggctacttcccccagtacggttactttaaaatttgcgaagcgtacatttactaccggatctttatagtaggtgcttactttacctgttatttcattccttacactgtctgttgttttatcctttgccaggatcctgcctaccagtggcaacgtaatatatccatccttatctactacatatccgcttactcccggacctgcattggaaagccctgcagcgcttccggttcctaccaccggccactgtgcggtgttctgctggttaagcaatgtggaggcagccgggtccagtgtttgaatagttacctgcaaaatatcatctgtctggatgaggggcatggaataagccgccatatctaccagttgtcgctttacagaatccggaacatccctgaagtaggtaatatttttaggtccggaacaggaactcacacaaaagctaaatacactcaataacaatacagccagagctggaacacgtcgggctgaatgtttaccctgatagattatactcattttaagacagactaattaaaaatatgttttggtattattccctgatgaatcaggtagttatttttcccttatctaattcttcgtaagcagagtttttactgatgaactctggtaccagcgccttcatccttgcaacagtgggcgtcaggtagtgctctttggctgtagctatcaactgattgatctgctcatttacctctgtaaaatcagatgcccttactttggcgatcatgatcttttcgtggtaagtaggcaatgtattttctgcattgttcaatagttcctcgtagagtttttccccgggacgtaagccggtgtatacgatctggatatcctttccgggctccttacctgtcatacagatcattttccgggccagttctgcaatcttcatgggcttgcccatatcaaatacaaatatttccccgccttgtcccattgctcccgcttccagcaccagttgacatgcctctggtatggtcatgaaataccgggtgatatcgggatgcgtaaccgtcagcggcccgcctttttccagttgttgtttaaatcgtggaattacagatccattggaaccaagtacattaccaaaacgcgtagtgataaaacgtgttggtggcgtgccgtacaccgggcccagtttctggtatttttcgttcaggtgattattaaaggattgggagaagatttccgcaattcttttggaagctcccattacattagtagggttcaccgccttatcggtagataccattacaaatttctctgcaccatactctactgataactccgccacaatttttgttcccagtacattgttcatcactgccacggatggatttttttccatcattggaacatgtttatatgctgctgcgtgatacacaatggaaggagcgtaaatttcaaacagttgttgcatacgcaccttatcacatacatctccgatgaatgggatgatgggtacgctcactgctttttctgacatttccagctccagctcatggagcggggattccgccttatcgcacaacacaatcacagagggttcataactcaccagttgtcttactatctcactgccaatagaaccggcagcccccgttaccaaaatgcttttacctttcagctctttgctgagctgttgatttttgatgctgataacagatctatcaagcagatcttcaatgttgatgtctttcaattgaatactgttattgttagaaccttctgtccactgactcacgggaataattttttgcactcttatgttcaatgcaatacattcttctacgagttcattcagatgcgctgcatccaggtgatcatcaggaatgagcaacaacgaaattttgccctcttttaccatcttaaagagttgtcccttacgggaagcatacactggcagcccttcaattgatttgccagcatgggcattggtatcggccagaaacgccgttatcctcacatccgattcagggttgtcgctgatggctttgcgcagcataagactggtatgcccggtataataaatagcggcgcgcgtccggctttggctcctgaaattgttgtagtacttaaacgtccactttaccagcaggcgataagataataaacagaaggagctgataaagaaattaatcaggattactgaaatgggaaagaggttctgttgctgatccatcacatgactatagccaatggtgaaaaggatgaggcaactcacaatattcaatcctgctatgcggccaatatccgtgaggcttgtaaatcttacaataccgcgataagtacgcaaaaataaggagaggaaaaggtttacacctaaaacaagcattccgatttttcccagaggaaatgctgcatataactcagcatcaaagttcagcctgagaagaaatgctaaattgattgcgatgacagagcaccccaggtctaatagcaagattagccacgacggggtaatccatgatgaattacgcaccataggttcaataataagatatggttattaaatataagctcgcctgttcaactaaggtcgcgcaagtttcaaggttttcatagaggcgcttagttaaaatacaggacggagaattaaacgattacgatctttctttcggttttcaaagttagcgcaagataagtactaaaagtgaaaagttctgttatgaaaaagtaaactgttgaaaaaaatttccagctgctactcttctgaaagatcaacaacacacgcattccccgaccactctaacaaagcggttatgacaaccattttttcctatggattatttgctcaaacactgatcagttggcacataacggcaaataactccgtcggttaaacgaaaaatgcggatcagccaatcatgctgtccattttgcatactattaaagagatttctcccgtgatgctacattggtggtgatgcacctggatcttttgctgtaacgacgtgttctgatgccgctctaaagtgttaagtagatgaaacatggtctttctttttttctggttaacgcagctactaaaaaatatggctataaatactatggttaaaaaatcactgcgctatcgattcttgcaacgcacgcaattgaacaaacaccataccaacttcgggggatctatttaatttcccggcctaaagttagtgaagtatttattatactgcttcaattattgaaaaataacgaaaatattctgtagataattttagcattcccatccagaagatttcactacagaaacggcctcaccggttactggtgaggccgtttccacaaagtgtaacgtacttgtgtatacgtaaaagatattatgctgttgtaataaatacgaccaggcttttcgctccatgcgcgcccagtaccagcgattgctcgatatcagcggttttggaaggacccgcaataaataccccgaaacccgtttgcggagcgcctatcttttcataagcttcatgcatagtaggaagtagcttatccgcaggcagtacaattgccaggtgctgacatataaacggcagcacccttaccggtatttccgcctctgtaagccatatggcgccattctccgctaccccccactgaccgggcacaaccgccatatccacatcctccagcaaatgcggatcttcgtgtatccatgcacgttgttcactgcctaccatgataatacgttgcagatgcggataatgctccgccagtaatgccggtatctcactttcatcttttatctcaaacaaactgccgcctaatccttccagtactttgcggtaagcttccagcgtaccgggcatattgccggataacccttccagggaaggtaatacggatgcctccggctgattttgcttaacggcggctaatatctggtccctgctgctcatgactttttatttttttcataccactgggagaatgattgcgccggcggcgcaggcatctccctttgtttataccaggggtttaaacggttattcaccataccggggaatgcacgcattacccatcgtcccattttgcccgctgtccggtaaacacggggagtggataatacaccgctcatagccttcatactggctgtttttgcggccgtagtatacccctcttttaccaatacctgccgccacttatacaattgctgatgaatatctattttcacggggcatacattagagcaggagccgcacagcgttgatgcaaagggcaggtcggcataatccttcatatccaggttaggcgccaggatagcgccaataggccctgctacagcggtatgataactatgcccgccactgcggcgatatacggggcaggtattcatgcaggcgccacagcggatacatttcaatgaattgcggaagtcttccctgcccaactgcctggaacggccattatccaccagtacaatatgcagctcctggccaggccggggctttctgaaatgactggaataggtggtaatgggctgcccggtggcgctgcgcgccagtaaacgcaggaatacgcccaggtgcttacgttgcgggattattttttcgatgcccatacaggcaatatgcacatcggccaggtgtgcgcccatatcggcgttgccttcgttggtgcacaccaccatttcaccggtttccgctaccgcgaagttcacaccggtgatagccgctttggcctgcaggaactccctgcgcaggtgttgcctggcggcagcggtgagaaactgcgggtcggcattcccggcgggcgttcccaggtgttcgtggaacagctctcctatctcttctttctttttatggatacagggcagtacaatatgactgggcggctctttggcgagttgcacaatccgttcgcccagatcggtatcaataacatcgatgccattggcgatgagatggggattcaggtggcattcttccgtgagcatggacttacttttcacgaggtggtgtaccccatgtttctttaatatgtctgtcacgatccggttatgctctgctgcatccgcggcccagtgaacggtggcgccattttgtatggcctgttgttcaaactgtacgagataatcatgcaggttgcccagggcgttcagcttaatgcgggaagcggcttcccgcagctgttcccattcggggatggtccaggccatcttatcccttttggcgcgtacccaccagagggtttggtcgtgccagtcgacccgcggctcattctcgttgaacttatctgccagcgtggcgtgatcagctgtttgcctgttcatggatattctgattgagaatttctgcaatatgcatcacttttacgcctgcatgctgccggcgtaagataccttccatgtgcatgaggcaactcacatccgttccggtgatcacctctgcgccatgtttaacgtgatcggctacacgatctttacccatttttacggatactgcttcttcggtcacacagaaagtgccgccaaagccgcagcactcatcctgcctgtcgagcggtaccagctccactccttccaccatacgcagcagcttttccggtttggagaaaggcgccgccaccagttcactcatctgggcaagggcgaggccgcgctgcccgtggcagctctggtgcagtcctaccttacaggggaaacgtgccggcaggttttccactttgagtacatccgtcaggaattcggtgagttcgtagatccgttcacggatatgtgtagcagctgtttctgctgccggatcgtgcagatgatctttgatatgtaacacacaactgccggaggggcctacaatgtagtcgtagtcagcaaaattttttatgaacaggctattgcactggtgtgtaagatgttcgtatcctgagttggccattggctggccacagcaggtttgcccctgcgggtattccacttcacaacccagcttctgcagcagttgcagggtggcaatacctacctgcgggtagaactggtcaatataacatggtataaataatcctactttcacgggtgaagtaatttaaatgatcattgctgacctgcaaatttagcgggcaacttgacagtaatcctacctcttttttaccggttactggcttatttttcactgatacaaattaaagcagtgtttggagagtggcaacccggtctgtcctgttgcgcgccttcggcgcggtgcggaggttgtcttactcaggattacgctgattttgctgatttatttgattttactttttggatttataaatgattatgggagatataagcggatattttcgctcatatctcccataatctttaaaatcatttaaaaatccaaaaagtaaaatcaaataaatcagcaaaatcagcgtaatcctgagtaagacaacctcctagtcgttcataatctgttcttcctgtttctttttgaggtaccactggaccacgcggatttcagcgaaggtggcggcatcgccaaccctttccttaatggggcctgcggcggtagcgcctaattcgccaatatggcggaggataaggcgcatggtgccttctgtaacaaagcggttgatgtccatttcgccggcttccacgcattgggccaggtggctttcaatggtgctgacagcgagttggcgtgtggtggcgatgtcggggatagatttaccggcgaggtacagttccagggtgccgcgacggctgctgcccttttccactttgcctttggcggctttttcctttgcggcggcggcaggtgctgcggcggcagcagcatctgcatctctgagtttggtgtagtctttaaggccggtggtaaaatccaggtccgcgtaagatacttcccaaacgtgacgcagcttgttccagcaatcggcttcaagggccatgagctggaggagatattttttcgactttgctttcttcacatcagcaatgtgcgcctgcaaaggctggatgaggtcttcataaatgctttgggtaaagtagccgatggctttatttacgcgttgcttcagctgttccatttcgcctgtttgcacggcggtgtccagcagttgatgcagctgtgtcacaaacctggccgctacttcctgctgctgttctactttggcagacatggcgcggctgagtttaatggcggcatcgaagtcggggatctttttatcctggatccatacggcgtggctgcggatggtggcctgcatacggtaccagtcgaacagctgcagcagggacgtggcctggaacttcttcttttccatttccagcagcactaccagttcattggcttcgttttccttttctgcgaattcaatcacctggcggtctgttctgatgctgccgtgcccgatgcgggaatgcagtaccagtccgtccagcgaagtacagcggctcagcgccacgtatacctgtccgggtgcaaaggcgtatcctgcgtcgatgatggcgcgttcaaaggtaagtccctggcttttgtggatggtgatggcccatgccagccgtatcgggaactgggtgaagctgccgatctcttcttcctcgatgctgttctcgtcctggttataggaatagcggatgttgcgccaggtttcctttcccagtttaagctcttcatgggagcctgccagcaccagtacaatttcttcgtcgttaatttcctttacggtggcaattttgccgttgtaatagcggcgtggctgtgccaggtcgtttttgaggaacattacctgcgcgcctattttcagttgcagcagtaattccgtgggcaatgccttatcgctgaaatccccttctatctttccttcaaagcgatatacttttccgggcatatctgccaggcgcctggcattgatttcatcggccttccggttatgggtggtgagtacgatgtattcttcatcctgtcccgtaaaattcggctgataatgttcattgagcagctgcaggtcttcgtgcagcacttcattattgcggatcctgttcagcacatcaataaaatgctgttcattctgccggtaaattttcttcagttcgatatacagtggcggcgcctgttctattactttggccgcaaagaaaaaggtgctgttgtaatattccgagagcatccgccattccgcgtcgggcactaccggcgggagctggtacagatctccgataaacaatacctgcacaccgccaaaaggcagcagtggtttattgcggaaatggcggaggatcacatcgatagcatcgagcatatcgcagcgcaccatgcttacctcatcgatgatgaggagttccatttcctgcagcaatacttttttatcgttggtaaaacgaatattgcggaacaggccgtgtttatctgtactgctgatttcatccattccaaatcctcttttagtgccggggataaagggtccgaagggcaactgaaaaaaggagtgcatggtaacaccaccggcgttgatagcggctactcctgtaggcgctactactaccgtgtttttacgcgtatgttctttgatgtatttcaggaacgtagttttccctgtaccggctttaccggtaaggaagatatggcggtgtgtgtggtttatgaaatctgccgccaggtgaaagatagtatttgtattatccggttggggcatttgctgttaaattgaaagggcgaatatacagaaaaagcggcgaaaatagcggagatattgcgtgtaaccaaatgtaaagtatcttcgttttactttctgccaacaaaaaaattttctcatatgaacgatctgaaaattgctaccgcgcaatttgaaaacaggagcaatgataaagcgtataacctgggggttatccgggagttatcgcggcaggctgccgctgatggtgcagatgcagtggcctttcacgagtgttcagtgacaggatatacctttgccaggagtttgtcgcgggagctgatgctggagctggcggaaataatccctgatggcccgtctatcaaggtattacaggatattgccgctgaaaataatattgccgtgctggcgggattatttgagaaagatgcggacgataacctgttcaaagcctatgtatgtgtagataaaaacgggctggtggcgaagtaccgcaagctgcatccgtttatcaatccgcatttacaaccgggaaatgaatatgtaatttttgacctgaggggatggaaatgcagcatattgatttgttacgataataatattacagagaatgtacgcgcaacggccctgctgggtgcagaaatcattttcatgccgcatgtaactatgtgtacgccatctacgcggcccggcgcgggtttcgtggatccggcactgtgggaaaaacgccgggaagatcctacttcgctgcgattggaatttgacggcatgaagggccgttcctggctgatgaagtggctgccggcgcgtgcgtatgataatgcggtgtatgctgttttctccaatcctatcggtatggacgacgaccagttgaaaaacggctgctctatgatcattgatccgtttggtgatgtgatagcagaatgccggaaactggacaatgatgtagtaacggctacgcttacacgaaataagctgaccgaggccggtgggtaccggtatcgactggcacgccgtcctgatttgtatggagaagtgattgcggcggcgcatacgccggtgcaaaaagtagtatggctccaggaaaaaccgtgaaggcgcgatggataagcgttccggagcgacggttcccggacttgataatttaaactaaattatcatacaaataaaaaaacacgattggttgcgggttttggctgaccggccataaataaaagcggcaaatccggctgaccggttatctttgcaactcatttacaccgtttacaaagctttaagataacccgttttttagcttcttgtataagagaaccgttcccttgtggagcggttttttatttcccggaggtggggattgccgggcgccttcggcgcttttaaattgtcttggagcaggattaaacttattacgctgatttcactgatttgattattccggcgagaaagggactgttattggatatacatggctatagcagggatattacgtggcgatgggataggaaatacggtgggaatggggatgacatggagtaaaggcggagttcacgtggaggtgacgtggacttgatcaggaactgtactggcagtaagggttttggcgattttttgtttgccggttatcgcgggtaccacgtgcatgatatcggcggccgaattgcggcggttcgccaatatagccccgtcttcggaggtaattatttgtaaaacgtgcaacagggcgccattgccccggaggtgattatcgagtattgtgccgttgaaaggcttatggaggtcgatggtgacggtactggtacggctgctgatgatgcgccgttgtagaaagctgatgcggacagcgatggcggtgagatggaggtgtgtggcactcccctggggaagcagctcctgtgcgggtatatcccagcttcctgcgggcgttaactgcggctgccggcaaaaaaattgtgacaccggggtgtacctgttgaagcgaaacccttcgagatcctgcaggcggttattaccggccttgatcagtgctttattgaggcggtttacgcaggtattgtccggtatcatatccaacagcggactgatggcatgccggatcagccttcccttttggctggccatgccaaactcccgggcagaccgcctggtagcgctggtttgccgcactgtttgcgccattgcgcggataaaataattgccatttctccggtaacctacctggttttccagcttaccggtaaaaaggacgatacctgtttgttttgccattgtttaatacacctgttttcttaaaaattgtttccttaaaaatacgaaaacaggctggctggcaggacaccggaaagagagtgaacaaaatgaacaggcaaggggctgttcattcctgttttatgcgtaaaagtttatgcataaaaaaaaccgccctggcaaagccagcgcggtttataaagaactattataaaataaattatgccagtcttacgttaacagcattcgggccttttctaccttcttccacgtcaaaaactacgcggtcattttcgccgatgctttctttgataccagatacgtgaacaaaaatttcttgtcctgaaccttcgattttaatgaatccaaaacctttagcttcattaaaaaattttactacacctgtttgcattatatttaatatttaattgtgaacgtgttctcgccattattattacagcaggcggctacctgggcaactagaagaaagactgtaagaaaaagctgaatgtgagaggtgatctaccaacagaattgcaatacattatccttaagaagcaatacgaagataggtgttttccagaatacaaccctaattttttttcaactttttcttcgccaccatggcctcctggctcataattccgtattaaaatatattttcgcattctatatgaaacatcctgacgcatggcgaattaaagccatattaaccgggtctgccggcaacctcgtagaatggtacgattggtacatttacgccacgttttccctttattttgcgccggtcttttttccgaagggcagttatacggcacagctgcttaatacggcggccatatttgcggtgggtttcctgatgcggcctatcggcggctggatgtttggccgcattgccgacaaacaggggcgtaaagcctctatgacgctgtcggtgctcctgatgtcgcttggttccctgctgattgcatttaccccttcctataacaacattggcctggcggcgcccgcactgctgctgatagcgcgcctgttacagggcctcagcgtaggcggtgaatacggcacttccgctacttatctcagtgaagttgccacaaaggacctgcggggcttttattccagtttccagtatgtaacgctcataggcgggcaactggtagcgcttggcgtgcagatgttgctgcaaaaggtattccttacacctgagcagctgcatgaatggggatggcgtattccgtttgtgatcggggccgcgctggcattttttgcgctgtacctgcgccggcatatgcaggaatcaacttctttcgaaaaaataaaagcaacaaaagataaaggctccctgaagctgctgtttaaaaagcacccgcgggcagtgatgacggtggtaggcttaacgatgggcggtaccctggccttctatacttataccacttatatgcagaagttcctggtaaacaccgtacatcttacaatagaacacgccactaccctcacctttttcctcatgcttattttcgcggttttgcaaccgcttttcggctggatttcagacatctatgggcggaagcctttactgatcggctttggagtgttagggacgctgtttaccgttcctattctcacggggattagccatgcggcctccgagtggacggccttcttgcttattttaatggcgctgctgatcgtaagcgggtatacttctatcaacgccgtggtaaaagcggaaatgttccccgcagaggtgcgggcattaggtgttggatttccctatgccattacggtggcgctgtttggcggcacggcagaacctattgcgttgtactttaaaaagattgggtatgaaccgctgtactattggtatgtaaccatctgcatctttatttcgctgctggtatacgccacttcgcgggatactaaaaagacgtctttgcttgatagggatgcgtgatctccctgacggtgccatcggcgttaccgataatcagccggctggcgtagtggagaaataaaccattttccactacgccgggaatattattcagctgtgtatgcagcgcggccgcattgtgtattttctggtaatgacaatcgaggatataattaccgttatctgttacaaagcggttattatcctttaaacgcaatacgggatgggctcccagcgctgccagttgtttgaaggtaagctcccatccaaaggtggccacttctaccggtaaaggaaatttgcccaggtgcttcacgaattttttttcgtctatcaccaccagcatttctttggaagctgctgcaataattttttcccgcagcaatgcgccgcctcctcctttgatcagttgcaactgggcatcggcttcatctgccccatctatatcaatatctatcttttcaattttttcaaaatccaccagggggatctgctgttcaacagccagctgctctgactgtgcagaggtagctactgcctttatttcaaggccggccctaactaactcgcctatacgcagaattgtataatatgcggtgctcccggtacccaaaccaacggtcataccaggcttaatatactcagcggctttttcgcctgctgctttctttccgatatctgtttgcatggaacaaatataactattagctgttagctaacgatatcttgcgggagaaaatgcagcaatatccatactggtattggcgttattggccagttccgccaacagcttgcccgtagcggggcccaggctgaggcccatcatagcatgacctgtacccatgagcagatttgtatgagagggcgcgtaaccgatatagggcaggccatccggtgaacaggggcggcaaccgctccatacctgatttttgttaggtatttgtatagggagatttgtgaaataacagttcacggaatccacgatccccgccacacggttcatatttacctggtcgttcaccggcgctacttccatagtgccgccataacgcaaacgattacccattggcgttagtgctacccttgcctcgcaaaggatggccggaatatttaagtttacggatggcgcctccagggtaacggaatatcccttgccgggcatcatgggcagccgttcgcctgccagatgtgctacagcagggctccaggagccggttgccaatacaaacacatctgcggcatgtgtttcctgcccggttattacggctgttactttattaccattggttttgatctttgttacttcgcgctgcggcaggaactgtacctgtttttgttccaggtattgtttcagttgctgcatcaggtcgttgggatagagatggctgtcgcaacgataatgtacgccgcccagcacatccagctgcacctgtggctccagcgcctgcagagcggctttatccagcactacagcgtccagtcccatggtattggcctgcgctgcaaggtgcgcttcttcttccgcaacagccgctgttttataatacatgataatgcctttccgttccagtccgaagttaaacccgggctgctgcgccagcgatgtgtacagcgagcggctgagtaaattaatatcccgcagcggctgcgcggaggcttctacatgctttgccgtagcgcttttcatgaatttaaggccccagctgaccagttgtttgttcagcgaaggtttcacgtaaaaagggcttttgctgctaaacatccaccggattccctgtgaaataatgcctggtgctgccagtggtacaaaatggctgggtacaatcatgcccatatttccataggagcagttgttactgaaatctcctttatcgagtacagttacatcccaaccgctttcgttcaggtaataagcggtacaaagaccaataattccaccaccgatgacgattgctttcatgttttaataagttagatcacctggaatccgtgtacatacgggtcgtcgtcatccagtataatagtgttatagccggttaccattgcccagccttcgatgcccggtacaatagcgggtttgccgccgatggtggtttctgcttcaatggtgccggtgaattgtgagccgatgatgctttcatggataaagcggtcgcctgctttcagttttcctttggcgtgccactgtgccatccttgcggatgtgccggtgccacagggtgagcggtcgatggctttatcgccgtaaaacaccgcattgcgcgcggttgcctccgggctaatggtggcgccggtccagagaatatggcttaatcctttgatgtgctcattttccggatgcacaaaggaatagttttcgtttagtcttttccgtagttcccggctccaggataccagttgatccgcggtatgattttccagtcctttgaagttttcctgcggatctactattgcgtagaagttaccgccataggccacatctactttcagcatgccgagatcggggcacattacttccaggttttctgcagcgagaaaagattttacgttggtgagctttactgatttcactttctttccttcctgtacgtagctgaccagtaccagtcctgctggtgtttccagtcgcagctggccggggactttcgggatgatcaggccctgttcaatggcgatggtaacggtaccgatggtaccatggccgcacatgggcaggcagccgctggtttcaatatataatacgcctgtatcgtttgcttcatcagtgggtggatacaggatactgccgctcatcatatcatggccacggggctcaaacatgagccctttacggatccagtcgaactcctgcaggaaatgcaggcgtttttccatcatgttgttacccttcaacaccgggccgccgccggcaaccagtcgaaccgggttgccgcaggtatgcgcatctatacaaaaaaatgttttggtcgacataagcatttaatattttaacgactaacggtgtcctttgtcagctgaccatctatttttctccagatacctaagggattctcatctttcagggcatccggaagcagctgctgcggccagtcctggaaacacagcggtcgtgcaaaacgaatgatcgccgatgcgcccacagaggtacttcgtatatccgtggtagcagggaacgggccaccgtgatgcatggcgtaaccgggttccacgccggtaggcacattatttaaaataacgcggcctactttctggcacagggtttccacggcttcttcatatgctaacaagtccgtaggcgtagccattacagtaccggttagctgaccgtgtaaatgtaataacaactttgtcagctccgtagcatctttacatactaccagtaatgacgcggggccaaacacttcctgttgcagttcttcattggttataaaatcctgcgccgctacgcggtagagcgccggagagcctttggtagcgtctttttccggcttgccggcgtacagggtttgtactcctttgcggcgcgacagctggtccctgttttcataatagtgataacagataccgggattgagcatggttccggcgttgatggaagccaactccttttgcaatgccaccacgaattgttccgtggcatcgccggccagtgctaccaggagaccggggttggtgcagaactgccctgtgcccagcgtgatagattgcgcatactgttgtgctgtttgttgcgcggattccgccagtttgccgggtaacagcagtacggggttaatgctgcccatttccgcgtacacggggataggctctgctctttggttcactgcatcaaagatagcggtgcctgccttgaaggagccggtgaagccgatggctttaatgccgggatgttttacgagttgttgtcccagcaatgcgcccgggccattcaggctggaaaatacgccatcgggcataccgcaggattgggctgctttctgtatagcgaaagccaccagttcgttggtgcctaaatgagattcatgggctttgacaataacggggttaccggcagccagtgcggatgcggtatcgcctccggcagtagagaatgccagcgggaaattgctggcaggaaatacgagtacggggcccaatggcaccagcatttttcggatatccgcccgcggtagcggggtacgttccggttgggccggatcgatgatggcttccacccaggagccttcacgcagcactgctgcgaagaggcggagctggttcactgtgcgcatacgttcaccggtgatgcgggccagcgggagtccggattccgctacggccctttccagcagcggatcgccgatggccagtatttccgttgcgatggcttcgaggaatacggcccgttgttccggggaagtttggcggtatgttttaaaagccgtagcggctttttctactgccaggtttacttcttctgttgttgctgttgcgaacatttccggcagggcggcattgctaacgggatcgtatgcacgaagtgtatccgttcccgtagcagccgccgtgaagccgataatatttttgcctgttatcatgcagggagttttaaataatccggtagttgcgggcgtacagccagtgctgttgctattacgttttccgcgtaggccaggtcggcgccctgtggtatgagtcgtggtgcgcgtacattcgtagtgccgatacccgtagcagtggctgccagtttaatatattgcaccagtttaggatcgatgtccagttccagcagtggcataaaccagcggtagatggccagtgcttccgcgatgcggccggctttcacgaggcgatagatagcaactgtttcgcgggggaaggcatctaccaatccagctacccaaccattggaacccagtaccaggcattccagcgccagcgtatccacgccgcagaggatactgaaacgatcgccaaagcggttgatcatgcgggttacgttggtagtatcgcgggtagattctttcacggcccggatgttgggcgctttcgacaattcttcaaacatatccagtgtgacgaggatcttataatccaccgggttattgtagatcataattggcaaagaagtgctgcctgcaatagcgaggaagtaggccactgtttcgcggtcatctgccttgtagcgcatgggaggcaggagcatcagtcctgctgcaccggcttcctctgcggctttcgcgcaggcgatacctgcagcagtagtttgctctgcaatattcatcactaccggtactttaccagccagaaaagccactgcgtgttttacgagcgcatacttttcttcgttcagtaaactactggcttctcccagcgagccgccgaggataataccattaacgcctgcatcgatctgtgcctgcaggtttttgtcgaacatctcataatcaatatgatcatccgcagtaaaaggggtgagcagtgcgggaaatacgccttgccagttaattgctgccattttttcctatcttttttatgtcaacaaaaatagccgtggaggcccgatagcacgctgctgtaattaatcaatactacgcagattttaaccgaaaaaactcatcttctaccgaaatttaaaaaatatccgcatattatcaactcacctattttttggaaatctagcttaagtccgctaatttttgccctgaataaaccgtaaaacattgaaagtacctatcatactggcgcttgcggcgcttttccccggtatgggactgaaagcgcaggattcaacggccatcaaagctattaacccggcagattttgcacggcacatcagcgtacttgcatccgacgcctttgagggccgcaagccctttacccgcggggaagacagctccattcaatacctggcggcacagtttaagcagctggggttaaagcccggtaatggcaacagctatttccaggaagtaccgatggtgtctatcagttccaagcccgccggcaacctggtaataaaaggtgccggaggtgaagtatcgctgcaatacctcgaagactttgtggccgccacccgccgcgtgcaggagcaggtaaccattcccaccagcgaacttgtatttgccggctatggtattgtagcgccggaatataactggaatgactataaagggctggatgtaaaaggaaagacggtgattgtaatgatcaacgaccccggctttgccgacagcacgctgtttaaaggccgcatcatgacctactacggtcgctggacctataaatttgaagaggcatcgaggcaaggcgctgccggcgtgatcatcatccatgaaaccgccgccgccagctatccctggaaggtagtgcgcagcggctggtcaaactccaagctgcacctgcaaaccgccaacaacaatatgcatcgtaccgcgctggaaggatggatcacactggatgctgcaaagaagatcttccagctggccggcctagcacctgatattatgcagcaggccaggacaaaaggtttcaagccggtagacctccacctgcaaacatctctcgttatcaataatagtattaaaaaatctacctcgcataatgtgctggccgtattgccgggcgccaaacgcccgcaggaatgcgtcgtatattcggcccactgggatcattttggtataggcgagcccgttaaaggcgactctatctacaacggcgccgtagataatgccaccggcaccgcaggactgctggaactggccacagccttcaccaggctgccacagcgcccggcacgctccctcctgttcctttccgttaccggcgaagaacaagggctgctgggatcggaatactacgcggcgcatccagtgttcccgatggagaagaccgtagcagatatcaatcttgatgtactcaatacgtttggccgtacccgcgacatcacggtgataggtttcggtcaatcggaactggacgaatacgcgctgcgcgccgcccaaaaacaaggccgcatcaccatgcccgaagccaatcctgaaggtggctggtttttccgctccgaccatttcaacttcgccaaaaagggcgtgccgggattgtatatcggtccgggcaacgatgccataggccatgaaaccggctgggggaaagaacagacagctgcgtataaccgcttacgttaccactcccctaccgatgaatttaatgccgccacctggaacatggacggcatggtagaagatatccgcctcttatttgacgtaggctaccacctcagcaatgaaagcagtttccctgcatggaagaaaggttcagagtttaaagcatacagaaaataactacagacatggttttattcggattgataatgataggactcatcctgttcctgtactttcaaaatatgtacggccgcaggaaagggaagaaaacggcggtacctgaagggtaccagtcgttgttagaagaacatgtacgctactaccagcagctgcaaccagcagaaaaaacgcgctttgaaggcatgctgcaacgcttcctcaaaagaaccagcatagaaggcgtaggcaccgaagtggaaccgctggaccgcgtgctggtagccgccagcgccatcatccccatcttcggattcaaagactgggaatatttcaatcttaccaacgtaatcctctaccccgacaccttcgacgaaacttaccagtatgaaggcaatcgccgtaacatcctcggcatggtaggcagcggcacactgaatggacaaatgatcctttcccgctccgcgctgcgggaaggcttctccaatgtaaccgataaaaacaataccgctattcatgaatttgtgcacctcctggataaaactgatggcgtcattgacggcttcccgagtaaactactggatcacagctatagcattccgtggatgaaactggtgcatcaaacgatccaggagatttcagaagggcatacggatatcaacccttatgccgcgatgaatgaagcggagttttttgcagtgatatcggagtacttttttgaacggccggatttgctggcggagaagcacccggagttgtatgggatgctggtaaggatattcaggcaggatcctgtggggaaggggtgagggaatataagaaaagccgcagcaaaatatctgcggctttctgtctccttatatttcaattaattcaattaaattgaagtccaaaatcttatctaattgatattgctcatctattgatgggataaaatattctttatccaataaatctcttatgtcttttaacttattatcattaaaaatgaatatatttctttgatcgactttataacgtgttccatcttccttcatagttgaaatcccattcctattacaatatgcagctactatcaatttttcaaaaatactttcaaaatcagctttattattattgaacaaataacttgaatcattccaaataataaatctcctctctggctctgtttcaaaatttaacaacaagtcataaagtgcatccaatcttggacctaattggtagcctactggcaggcttaaattcacctgataaataaaagtctctaaactattaatagcattcccatatagtggaacaacctcgttagcaccctttcgaaccaaatattgagtatagtttgtcataaaccaaattaacctatcttggtcagtttcaaataaaataaagtcattagcataactgttattcattaataaatcatgccacttagaaactggctcattcacatttattttaagttgtttaatgctcatattattggttaatgataatcttgtatactatgaataaatatttcatcctcagtggattggaaaactatacgaagtgcccctctaccttttccactccctttaacatcaatcgcattaaatcctttcaaattccctgttaaaacatgttgatttcctccggccttcccatggcgaattaactccagcgcttcctcaacactttttcttgctgaaggtcccaatttatccaaaacttttgttgcatcaccagactcgactattactcttcctatcttagaaaatttcatagccttaatagttcccagaacatttctaatcttccataaattcctgccaaggttaactcctcccacatcgacataatcaggaggcattccagcaacatatctagtagccaaatcggaagttatataacctgcccggttaacaacatgtccccctctctgccgctggcctccaaaatattcttccatgggacttcttgacggtcctgctttatacccaatcccaaaggtcaatccatatccatagtcatcccaaccagtagtaacttttgttggtgtaacgtctattccatttaatcttactacatcagtattagtattaaattcattccaaactttgggtaaatcgctcacatgcactgtgtcgtcaccaaatggatcactcaatccaattggattgttaagaacatggctataagggctgtaatcttcaaagagatctacttttgggtcaatctgccaccatcggcctgtttgtggatctagattccgataaaacgcatcgtattgattcaaatctaagtctgttgtatgttctattccattaaactcgttccgatttttggtataattcgtccccttcaacgcattagaactaatccccgccatcgttaacccaaacggataataatgcgtctcctccaacaacggtccactcgcctgagccactactacattatcaaagaacacctcctgcgggctttcattactcgtgtaaacatacagaaacccacttttctccatcaccattttgtcctgggccaatgtctgcaattgatccggctctgcttttacctgcttaactccactatttccgtctactaatttaaactgatcatcgaacaaaacaaaattaaggtatgctttaggcctgtctgtgtttggctgatcaggttccttttccttcaggttctggtaatcattgttataaaaactgctattaaacggcgtagcctgttgcgaggaagcaacaccgtgagtagcatctgaagaagcggcgccaccaaatacctgtaccaggtcagccagcatactttcagcaggtgccggtgagttattcttatcctgcggtcctgtggatttatagaaagcttttgcgccaatctggatcgtatcacctgccatgaccttcagtacaagagaagggcctatttttttaccaccgctggttgctgtcaatttcgacacggaggcattagtgcctgcactctcatctgatgggtatcccgccggcttagcagaacgggtgttatcaatattactgaacaaagccgtttctgttgcagctgcggaggtttccatggtggcggcatacatggagaaatctgattgctcagtcaataccattcgtatatttcccagatggtcctttacgaagtaatcgtatttaaaggctggcaattggcccgattgaaaaacagtacgcacacgtccttcctcatgacttaaaaactgcaaggtatcattctgataaacaaacccgttaatatagtctgtcgtagttgtttttgcaggagtaagcgtattatctataactatctttcttagtttattaccggtagcatcatactgatatttaataatgcctttactggtaatggctatactatctggcagattgaggtgattatagcgaattgcgactatatttttattggcgtctttagtaagattaccattggcatcatacgcatagtctgctgtttcattgttattgatctctttaaaatcgcccagctggctttgcgtgttattttttcggtctgttacaaatgataatttgttactagtagcaagataaccatattttaagctgtcaatggtttgcactactgcgccatttaaccctttctggttcatgtataagatattaccgttggcatcgtatgataacccgcttacagaaaagtttgccaaattatcagtccagttggaactaccggtattctgttgcgtaaaatccgctacggtcaggcgattagccttatcgtaactgtatccatagccgcgcgcaataccattattgcggcttttccatttcgatccggcaatgtttccattgaattgaggcgtggtaaaaccgtaatcataattaagctcctgcccaaaccagtttgttgtgcttcccactgccgggataaaatccttgttaattcccctcagccagccacggatattatagtcgtaattcaaagtttccagctgagtactggcaccagtaatccctaaacgcttcttctttaactgacccagttcatcatactcatttacggctactgtcctttcaagatttacatcattattcagtcgcttctttatgttaagcaggcgaccgccggcgtcgtatgccaacatggttaatacctcagtttgaggaatagtgccactacgctggtttctgtgacgaagataggtactcagtaatttcccgttaaaatcataaagattagtgctcacatcctgccctccgctgacattgtccgatatcgtttggatcaaccgtccattgtcgttgtaatagttggtggtggtcaaccattgatcggtatccaacacttttactttagtacctgtaaccagtccttttatcatagtgctggcaacggcaggtagtgcttccgcatttaagttgctaccggcttgtggtttggtgatatctgtactggcgtaattttccttatcagcaaacccgtaactctcgtaaaaggtataagtcagcggtgttagggcactgatgggtatattagacagcggattggtaaccgtaatattggcattaccattagtagccgccgcattgatttcagcgatcacttctgttcctgttccggtgtcaaaaccatctgttagtgtaatactattagtagctacgtaagaagtgcttccattatgggatgccagtaccaggtccgctgttccaggaaagttatacgacaggctctgcgtattgctgattgctgcgttcatagttccctgcaatgtgagccggtcggtagcaacgttgtaaagagcggtcatcgttggccggttcagcccatcataaaaagtaaccagccagcttttgcccttcatattgccatcgcgcgagaaagccaacctgtcgcgtacatcataaaccatttctgtggagtcggcgccgggcactttttttacgaccatgcggttgcgcccatcataacggtacataaaacagagctcggctgcaatagcagggctgatcatccagttgctgataatggcttccaccgctttgggtggaattacaaaacgcaggtttcccagatcgtcatatgcataataagtacaaagccagcccatgtggccagtgccgggatttgtacccaattgtacttttttaagaatgaccttcccttccttatccttgtattcaactagctgattattggcctcatcgattgatacatttttatacagctggccagcggcatatatacgccctgctacactggtaggaatagtagctccggcaataaaatcccagatacgcactgaatctgcaagggcgtttatcaggtattgattctggactggatgattccctcccctttccactgttgatgggtcattctttgcccagctattacctggcgcataggtttttaaaaccctgtttaaaggcgatgcttcataatcaatacgactataatacacactttccccactggcaccaggcacctgtgtttgatagaaactcttctgcgcgttaaatggatctgttttaaacttaccatctttcacgttttgtggaacataaggaagatatttagtttgttctcttccaaattgatcataaactataggagatacaatgtcgttacctccgaagctcatggcttttgacaccgtttgtaacggtctgccaagtccatccacataggcggttgtttgccttacctccgcaactgagcgattggcggatgctacataggcagtgtcggtggttggcaatgccggttcccaggtgcggacgtaattgattaccgggttagtataagcggaaggcaaaggaacaggtactgctgtcggcaattgtgttccgccgggtgtttgagcctgtacgttgactgcgattataagcagcaatacacaagcagttatttttaaaatacgggacgacagataaaacatatagttactttaggtatctgcaattagtttagttaattcgtttgcttgtattggtaatcaaactgcttcaatatctttccgttttggtcttttatgagcttaagtcttccaaaaccatcgtattcataaaagactgttttaccagaaggatctgtttcagatgtcatcccttttaagaggctataggtatatgtagtcaccattgcacctgggagtttggttctcaaattggcgagttcggtacgtaactgaacatcatcagttggattatctaggatagtttgattaatgtattgtttcactgtatcatactccgctccaattaccctggcgactggatatatccctccgtatccccacaagtaagtttccttaacatcatttgttttttgttgctctatcaggtttcccctgacatcatatttattaaatgaaatacgctctgtatatcgcgtatcttttgtgacagcccctgtcagattcctggatgcaataaaatcagttatcggcacactgttttctaaactgtaaaccttatccttctgaggtaaatctgaacgaaatgagaagtaataggaagataacaaccgttgattggtgccatctgaattcgccttataactactcatctctatttccggtgcatacacatgcctttgctgtaatagcttaacgccggcagtagtagcatctgtagctgtcaggttcccatagtcagatgctctcagaatattcgtaataatcatttctcctttgctgtcgctcttctttgtttgcttcagtaaagtggtagcagtatcgtagtcatattgttcttttacaatatttacattgccattatcatcatatgtttttaccacaacgctatctagtgtactatatccagatgtatagtaaaaagtggtatgtctgaaatactcctgtaactggtattcatggtgaccattgctccaaaatggataagaactaccaggaagcaagtacctggatgcaaaaaatgcttctccataggcttttctattacgctttaagtccgaataacttcgcttctcctctgataccagggatattcctgttccttgaactttatacacagattttccaaataatcttccataggtccaactattacccgtaaatggtggataaggtatgaacttataattttctccacccggggaatcatcaatattattatcaaagtaggtaatcgtgcatccattggtagcaccagttgtaagattgcgttgggtttcctttactgtaccatatccaattacgccacccatcatatccagaattggataaagactactggaagagattactttctcctgttcactggagtagccatcgttttgaccggataaatcagtatagaggaaatcagcatacttctcaaaataataatttccattccacggaggctttacaccattactatattcatactccctcatcattttgtttcctgatgcagaatcaatatcggtaacgcttttaagtcttattccaccagctgcaacattgtctactgttgtaatatattccgtatgacaattaaaaggggcaatcctcatattacaaaaaatatctgccgcgcttcccgggtaagtctggccgttatttttagggtatatatagtaggttcctttattcaatgttaggcttttcgtacacgtggggtatggatactgcgaatagctatcacaaaataatgagttattacgataggtgtaaatgaggttgttagtggcactatctcttatttcgatgtagtaatacggtggaaaattactatacctggaatcaagcgaagtgacaacttctacaatagaactattaacagaaacatgaaattcacgaggtgccaaagcatccggatcattgggaataagaggggcaaactgtactcctgtaaaattagtattaatgttaccatcacatacttcaacaggctctgttgttgctacagattcattgaagtgaggctcgtacacaaaggcggtactccccccggtgggatattgaatatttgtaagaacagcctggacagcataattaaaatccggcctttttagaagtgttaaatccctttgatacccctgaaatgcatcaaagcttctgcccggaataacgtcaccaattgctttataactcttcccattggcaaatccccaggtgtctccaccggacatcagtcgtgaaggtaaccctatcgaatgctcatagtcgaaaagataaggcggtaaagaactaccatttgcatcggtttctttaacgctacgtaacattaatctcagctcctcttttgccgcggctcccggcacttcagcatctttatacaaaaaggtgttatacaagtactggtattcaaaattatatgactttatcttgttattttttatattataaagaacaatgctgtctaaacatttcccttgctgcatatctttacgatccgtagttccgtagaattggagatagccgccattgaactttataaactttatccgctgtgattcaatctgatttttaaagttggtcctacttttatacggtgtaagtcttggtgcgagattaccggctaattgtttggtggaatgaatgtcactagaacccgaagtccaataataggtatccgcagtttcatatacaaaactgatagtgtcttttttactggcacttataatattagtcaaatgccaattgaatatataactttcagatacatggataaaatcatcaggcggctgaggactggaattaccatctatataagtatatggtgtagttacagataattcaggtttcaagaactggtattgagtaccattttcatccacaagattaaaaccgacaatcgcatccgccacagtaatacctgtatatgaatttctaaagctaccctgaattattggagttatcagattactggaataaggaatagggtaaacatttttctggtgatcaaaaacaaacttaccgttcataccagatacattataactgaaaagatccggctgtgcatccaactttcccaaactataaaggttcaccctatcatattccatatagggattgtctggaacaaatgttattgggtaccgggcccagaatccatcattggaattatcgtccacttgtcctcccatcatagttctgttgatcacaccaccagcatttaacgaccatcctattcctacctctgaaccaacatcattgaccctgatccctcctgaactatacgacagagaaaccggtaaggacaactcgcccgacttaatttcaaataaaggaatactgattggggcggttccggtgaaactacctagcggccagtttccatatcgttgtatggctgctacattgggggaaggcagtactacattttttgtattaagataattattctgggcactcagaaataacgggagcatagaaagaaagactaaaaaacatcttactttttgatagaaataactggacatattgtataatcttggttgatgtgcctattgaacggtatttcactgtttaaataagctaagtataggttttaagaatttttcgtcgttaaatatgatatgcgggcttaaaaattataccccagcctcacctttaccgggtccgtccgcggcacatgctggttatacaaaaagtcaaacaacaccatcatattgcctttcagcttactattgatcttgtacttcttactgatcccaatcaacccgctctgcgtccacttctgccctactccttccggtacccctgcgtaatccggttgataattctgctcatagccgccattcaggaaaaaggtgcctttgagtttccagtcgatgaaggagcggatgcccataccctgaccggagaaatgaatgttatcaaagccggtacccatgcccagtttgtaagaaagaccaagaccggcgcttccatttttatggaatttataggctgcttgtccggcgagatcgccggtagtagggaagaatttattgctgcgctgaaactggatgttgctgccaaactccaatcgctgcaggaagctttttgttttcatttcctttggcttgaaatcgggcatctccgcagcgttgtcaagatctgggaacttgcttttcagttcgtcgaatttgctgcgggcttctgccatctgctgacttacggcggcactggcattggggccgctgcctaagcgctgctggatcagctgttctacctggttgcgggtttgcagtccttcaaggttgggagctgatgcactccccccttgtatattaaacaggctggcgagttgggaatgtttttgcatgaagtcattgaaagcggggatcttcttaatcacttccattgctttttgttccgctttctttttatctttaaaaacttctttatactcctttagttgctgcgcataatagtaggcttctttgttcatcttctgcagatctttggtgaagccagtatactgacttaactgttccttcagcagttgtttacgttcacggatatacgctttaatctgctctgcctgggccagtttgtctttcaggttatcgactgactttaacgagccattcaatttatcggtaacacccttggacttttccagtaaacctttggaatcttttagaaaggacaatgaattgctaaggctatcaagataaggaccgccggattgggttaaggcaccggaataccttcccagcttgcctttcatacgggatttcaggcttccgagggaatcgatggaatgtgcaaaaagattattggctttcagggaatcaatgcggcccagccggcgtttcagcttttcctcctgtttcataaaccggctcagggctttttcgctgcgctgggtgatctgccgctccattttatctgacttttgttttacctgcgacaggtacttacccggaatggcattggctttctgcagcaggctgtcctgcgcctgtgcggtgcacaggcagacgaacaatagtaaggtcagttgataaatagttttcatggcaaatccgggggttatttggtggcgatcttctgtttaagcacttctacttctttagaaagagtagccagctgcttattcatctctataatatacaacatttgctcctctactttctgcaataactgcttattcatctctcctacatccactccgtctttttctatttcactggcagatggaataccaggaagatgttgattctttacaacaaactgctctacttcagacagggttggcaatttgtaatctgcgtgaaaaacaaaatccggccagttagcataggatttcaccactactcttgtaaagatgccgctgccgtttacggccagcttatagcctttggtatctgcggttcctatggctacgctgccattggcttttaccaacatgaggtttacgccggcactgttaacagccaggacattactggttgtaagcttcgcccctgttttacttctgctgtcaagtattattccgccataggcaatatcagaagccggaagtacatcctccacatcagctataagataaagacccaacgaacgacctgggatataaccccgtccgttgataacaggaatataattccccgcgctaccagtgccattcataaaactcagtgcgccatcggccgcagaaacatcagtttgtgtaaatctggcaaatacagttccaggcgaaccatcaacatgcagcctggcagacggtgaggtttctccaatcccaacaaatccattatttgcaatcctcatcgcttcaaattcaccaccactgcctcttacaaaaaacttcatagcggacatcctcccagaggaatcagttctctctacttccagttttcccaggttagaaccagccatattaaacttaagcgcacctaccacgcctaaaacgtcggagggatgggtcagttttatgtttgataaacccgcggagtaaatttccagcttttctgtgggagaagtggtgccaatacctgcattaccggtggcttccagtttattctgggcgtagctgctcaacgccacaaaagaaagaagcagggaacaagaatatttcataaataaaggataaaataataaaaccaacttatcaggtatacaactatgacttactatcagggtaaacagttacattcttactgggttgaacactacagttaattctgacgcaaaatagtaaaaatcagttaaatccgggtcaaaagtaattaacttattattaaccgggtcatcccacattcgtgggattttgtcttgtactatccggggcccggaaggaagaaatattgaccggtacagccataaaaaaaccgctcctacttgcgcaggaacggttctatatctcaaacaaaaaactacagcgttttcaccctgatattcctgaacctcacaattgatccatgtcccaggaaaccgatatgaccggtttccctgttcaggccgggatgcttcttatgatccagtgtaccgtttttacgggcgtctgcaatgtcgccgtcgaggataacggtgccattcagtattattttgatgtgcgtgccatcaacaatggcttcttccgtattccactctccaacaggtttcaggaagccacgtttggcaggaattacaccgtatacggagccatgatattgatatacctgcaggtctttatagatgtctgcttcgttatcgaggatctgtaattccataccttcgtaggcggcatcgccttccagtggtgcgcggatacccaggccattgttagcgcctggtgtcaactggaattcgaaacggaaagagaagtttttgtattcatctttcgtatagaggttaccgtgaccaccattggttggatagatcaccaggttaccgttatcgattacatagtctttggtgttgcctgtccattcatgcatgttggtgccatcgaacagcaatttgtagccggctttcttctcttcatcgctcagcacataaggcttcggacggggaatttcacggatgtacaggtcgcggtacgccacataggtaccatgcgcctgcagctcaatctgctcttccgggaagatcggcaatccgcggttccagtagttttccaggatggtattatcagtaacaagttctccgttgagatatactgttacgcgatcgccctgcatgaggatgcggaaatgattccattcgccgatagcgttgtctgctaatttaagaggcttgctttcatgctgctgattattgtataaaccgccggatcctacctgtgcgcccacatcggtgcgggaggtgtcccatatctgtacctgcggggaaccacggagataaataccggcatcgccctgtgaggtgatcttccagtctaccagcatctcaaagtcgccatacttcttttcggtacagaggttatcaccgctgccgctaaacaccagcaggccgtcttttgcggaccagcctttgcgtatgttgtcgtttgctttgtcctgcgctttgctgagtgttttggcatccattttaccgcgtgctattgggttctctacgagccctttccagccggtaaggtctttaccgttgaagagcggaacaaatccttcaccagcgggcatttcagcgaggtatttgcggatcgactgccgttgataatcggcatcggggccgttcagcaccttggctgttttctctaacagggaacgcacgatggcgccattgtagcttttatctgccagcgcgatgttcattacggcattggcagccgcctgttgtaccggtgcattgtcgaggtagttgccggcaaatagtaacgcaggcagtgttttgcagcgctcaacaccttccagcaccttctgctgtattaccgttgagggcgacagctccatggcgttgcggaacatcagcagctgctgatcggcaggcaaagcggagcggcgggtaagcgctatgtagccggtaagtgcttcatcacgataggtagcatcttcacgcgcaatttttaagagcgcagggatagcggccatatctttccaggaagacaatgcctttactgcggcttttttcgtagcagcgtcaccgttattaaaggagttaactaccggtaccagtgcatctttttcgccgatacctgccaacacaggaaggtagcgggattgctgaccggcaggcgcctgcttcatttgtgcaagcacatcgctgctggtggcgccggcgctgatgagcgcagcctgtatgctggcgatatccgtttcactggcggtgttattgagtaaggtaaatagttccggaagatttgcctttgtggccacatccttcaatgcggcaatggccgcactgcgggtaccggcatctgtgctggcggtgaggggcagtacatcatttacacggctgtctgctttacgtgcagccagtaccgttagtaaggctgtttgcgctgcagctggcatggtggccagggaggcgccggattgtgcggctacttcgtcgccgggcataatcaggagcgcctgttttacggcttccacggtagcggcatcgccggttttcatggtttgcagcagggagggtaaggcagcggcgccgccggtttggccggccgctttgatagctgccagtttcacgccttcatctttgctacccagtaatttctggagcgcaggtaaagcagcggctactttattatctcccaacatacctattaccgcggctttattggcattatcggcacccggcagtttctttagccataaggcgttgccggcaaggccgtattgacccacaaatttcagtgcagcatcacggtatgctgcattcttatcatcagcagcggccatcagcagcggcatattcttttcaccacggatggcggtgagtagttttaatgcagctgtgcgggtatgcacctgcgcatctgtttttgtttgcttcagcaggttctctgctattttcgcggcggctgttttatcggtgatattattagcgtagtacaggtaagacgccgttgcgtcggttacatcataggagtaaccgctgttggcagcggcggtagccaatacaggagcagaagccggcgaaccgatctgcgccagcgcatacagcgctactttggcgagtttcttatcggcactggtggccagtggtgcaatagctgttgcagctgcagtataacggccatcccccaacgcttctgtaagggtgatacggttatcgcctgaagcggtgctgagcgcctgcaacagtgcctgttgcgcggcgggtgtgttaacctttaccaatgcgcgggcagcaggatcgcacaaacggttgtctgtgaggtacgactgcaacgtgccggtggcgttatcatctgccagggtttccagctgggtgatcaggaaaaacttattttccggctccgctgttttggccaatgctttgcaaagcgcagcagaagcctgtttgcgggctgcttcttttccgggttgcgtaacataataagcatatccggccagcgcgtattccaactgcgtattattaccttttccgggtgctgccagcatgccggcaatggtagtaagcccttcttcccccagcgccgcaatcgactccatattggtgttaaactgcgttttattgggggctggcatcaacgccagcacatcggctattttagtatgaaacgcacgctgatctgatggcccctgtgcggaaaccaggctactccagccaaccagtaatgcaacgagtaagtattgtatctttttcataattcgtttacttgattgtttagatagtccacggtccgcgcattggctgatagatcagcgcattggcgcctgcatcctctataaattcctgtttcaccgggtcgaatttcagcgagcggttcaggcgcagggcaatcttacccatgttcacgagggtagcggaacgatgaccattttcctcgttcagcgcaaacttccggcggttctttacagcatccacaaaatctgtttgctgtggggcggggtcagggaatgcagccagtttcttttccaggtcctggatatctgagcggaaacccgggtagagttttcctttgggtccttctatataagcggccttttcatcggcgccatcgccatcgaggatgatctggcagccatctgcataggtgtaggtaattcttctccaggtgcccactgcatcaggatgctgttgtggcgcatctacttccacacttaccgggctggtgtcatctttacccaggaaatactggataggatccaggtaatgctgacccatatctcccaaaccacctccatcataatcccagtaaccacggaaggtttggtgcacccggtgggggttatacggccggtaaggcgccggccccagccacatatcataatccagttctttcggtaccggcatggcttccaggttggttttacccacccaatagaatttccagtcgaaacccgtatgcttgctcacggtaactttcagcggccagccaagcaggccactgtctaccagttttttaatcggcttcactgtggtgcccattccataaaaacggtcttcaaagcggaaccaggtattcaggcggaagatccttccatgttgctgtactgcttccacgaggcgtttgccttcgccgatggtggctgtcatcggtttttcacaccagatgtctttaccggcgcgtgcagcgtctgcggcaatgataccatgccagtgcggcggcgtagccacgtgtacaatatctacctccggcagggtgatcacttcgcggtagtcgctaaaggtttttacgcctttacttttatctcccagctggtccattgccagtttcaggtgactgcggtctacatcgcagagcgccactacccgggtgccggcgtaaccaaagtggccgcgtcccatgccaccggtgcctataacggctttggtcagctggtcgctgggcgccaggtaaccgcggcccagcacatgcctgggcacaattgtaaatgcagcaagcgctcccagggaatttttgagaaatgcccgccttgaatcgctgttttgtttcgccataattcagtttaattgaatgcctggatttgttttgattgatagtattagttcactgtatgatgatatattcactgtattgtcacatcgtggttgtatgaatggtaagatataatctaacaagatgatatgcaagtacagtaacgaaaatttgataaacggtaaaaaattaatacccggtgttctgcgtcatttccgggttagataacatttccttttccggtattggccacaggtaatcccggtcggtatacgaacggtcctgcaccttgacggccacacctgtttcgggattggtagcgccaaatacctgtccgttcattacctgcttaacaatgccccatctccggatatcaaaataccgctgtccttcaaatgccagctccgcctgccgttcccggcgcaccagctgccgcagcatggctgcactattgtagcgctgctggtcaaccaccggcatgccagcccgggtacgaacatcattcagatattgtatgatcagtggatcctgccagttgcccagctcaatcacggcttctgcataggataacaatatctcactgtaacggatgtacataaaatcgagggagccactcctgccctgccggtcgcgcggatcaaggtatttccggatccagtagccggtggcagtagatttctgcacacctattttatcggtgttgttggtagcattatcaaaaggagaaaggatataattggcatcgaggtacgactgaccgggatacaggacagacacagccaaccggggatcacggttatttttatagttgggatctttacggtatatcgccatggaatcagggcccagctccgccggggttttaccctgttttgtttcaaagttatctactacctgcgccgtgggcgacacgtaggtttctcccccgatgccataaggcgcaaaggtggtccaggcgttgtcgcaaccattggccttgaaaaaaatacgctctttgtttaattcaccggtgtaactgaacaattccgcataactgttcacgcctgctttttcactgcggtgtaatttataaaccccggtgccgatgatcttggccgccgcatccctggccacatcatagtgatggaaaaacaatgccagtcgcacgatcagcgcattacaagcccctgcggaaatacgccatgtttcatcgctgtcgtattctttcggtaagttctccgcacacacttttaactcgctcaggataaattcatatactttttccgccggatctcttttcaggcgattttccagcggggtaacggactttgttacaatgggaatgtcaccaaaaaacagcatgatctccatatgataaaaggcacgtaatgcacgggcttcatacttcatacgggtgcgcaactgctcgtccataaaacatttatccacgttttcaagaaaacggcaggcacggcgtacatctatataatcatcccgccagatccattcggccacatcccaggtagggttttgcaatccgcgggtgtaaatatcgtagttacctctgaagtcgccgcggcaaacggcttcgtcgctcaggcccgaccagaacattacattcctgccgctggaacctgccggcaccccggcataaatagagcccagcgcattataggcatgactctccgttttccaccactccaggtcagtaacaccggaggggttatcgtgggtgagaaattttttgcagcccggtgaacacagtaataccaggcccagtatcatcgttatgttgaatttcattttcattgcgaaaaagttgaatggttatagttgaatacttacccctgcagtatacattttcataatgccatacgtccattggttgccctggctttcagggtctaccagtttcatggaagtgaatacaaacggattttgtgcattcaggtataccctggcaccgttaacgcctatacgttttaacgtagtgctgctgaaattataacccagctggatatatttcatcctgatgtaggcgccgttctggatccagaaatcggacgacagcttattgatatccggtgtagtggttaagcggggaaagcgggcattggtacgctcaggcgtccaatagttgtctgcataatattgtgtaggaacacctccgtcaaaagacatatccaatggataggccagcatacctgacagcaccgcatcgcttttactcacaccctgcaacagcatttccagttcccattttttataggtgatgcggaagttggcaaagaagtcggcgcgcggtgtaggattaccgatcactgtttggtcgttgccatcaatgatattatccccgttctgatccaggtagcggatatctcctggttttgcattagcgatcactggtaccagcggcgtgccatccggtttaaaatccgcggcctgcaacaaaccatttgttttataaccatataaactcttcagtgcatatccttccttgtcaatgttcctgccactgatataagggccgcccaataccgtcaggaaggtgtttttattataagaaacgccagggcgtacagagagggtgacatctttaccaatacgaccattataattcagcgacagctccactcctttgttccgcaatttgcctgcgttgatgggaggagtgcccataccgcctacataagataccggtggcttgagaataataccattggtagttttgttgtagaagtcgaacgtaagctccagtttactctgcagcaaagccaggtccagtcccagatccaacatgtccactgtttcccaggtaatatccgggttaccgaaaattgattccacgccatctgtggcgctgatcatattctggtactggtaaaggtctatattctcattacccagccggccgtaagatgcacggagcttcatgctgctaataacagatacgggcgccataaaggactccttatgtacattccagcccaacgctacggaaggaaatgtaccgtatttatgacccggaccaaaacgtgatgaaccatctgtacgaatggctccttccagcaggtatttatctttataagaataatttacttttccataaaacgataacagggaatttatatcccagaatttactattgttctcttcctgtgaatagccacccatcagataaaagtgatgatctttcaggtcataggtatagtcggccgttacgcctgcgtaatagtacgtagtcctatccatagcggcagtccgctgcacaccccatgtttgcaccagtttaccggtataataatcaaagaagtaataattgtcacgggaagtgcgggtcacgtcgctgttcaaccggaagctgaattgtccgcggagattcaggccaggcaatacttcccatttaggctgcaggttaatactggattgaccgtactcattggcagattgaccgccatgttctgcgtaggccaccgggtttacaatatccacgtagcggccatacatgaccggtgcgccatcttttgccgggtatttgggaagaatagtaggcggtacccggaaaatatcttccaatatcctgtttccattactcccattgggacggttagggtaaaaagtatttcgtttgatggccagcatgtccatgtataccaggaactttttggtaagggtaatggaggtattggcgcggatattatacttattggagtggttgaggggaatcatcccttgctggttctgatagttggccgttaaggcaaaacgtgcgaggctgttaccgccgctcactcccaccgagtgactggtaataggcgccgcgcggttcaggatttccttctgccagtcggtgttaggatattttaccgggtcgtcgccggctgctgtatgttgaatatcttcttccgaatagaatggcgcgttgccggcgttcacctgtgcttcgttaaacatgcgcatatattgcggcgcttccaccagcgccggcatggaggagggcgactgcacaccataatagccatcgtaggtaacggctacccttccggctacgccgcgtttggtagttaccagtataacaccgttggcggcgcgggcgccgtacacagcggcagcggcggcatccttcaggatggtaacgctttccacggtaacgggatcaatatagttcatgtccatcggcacgccatccaccattaccaatggattggaggcgttcgtcgtgctgatgccacggatctttattatagcagcatcgccaccgggcagaccggaactttgcgttacctgcaaaccggtaacgcctccctgcaatgcctgtgataatgcggtaatgggcttgccattggtttgctgtgcaatatttacagagctgatggagctggcaatatgtttccgttgctgttctgaaaggcccaccactactacttcatcgagggcagctacgttttctttcagggaaatattcagtgcattgtggctccggataatggtatattcctgcgcgaggtaccccatttgcgtaaaaacaagcaccgcattttttttagcgcggaaggtgaagtagccatcagcgtcggtagtggtaccaagactgttattgtcttttacccggatagttactcccggtagcgcctgcggaggttcatgcgtatcgtatacccgtccgcgtatgagataggtactgtcttccaacagcgagatggtggacaggcgttgctccggcttacctttttccttcgggatgatggctacctggttgcgcatgatgcggtagctgagacctgtatttaacagggctttgtccagtacttcgttgatctttttgtcctgcagatcaagcgtcagcggttgttccctgtttaccagttcatctttataaaagatacgccagcggctttgcgactggatctggttaaacagctggggtaaggttccctggtgtagtttgatgttgaggtgttcgtcctgcgacttgccggtagcagaaaccccaaggatagcgatgaacagtaaaattacagtcagtttcattgttctcaggagtttaatggcaaaaacattgcctggcggtacccgccattgtgcatagatttttttcataacttcactacagtttttttagttaaacaaaaagacaagcccgtccccgcttcggcggggctgtgcaaccggaagatgtcccaccatcttccggcttttttttggtgatatgtatggtaattagtctttctctttcagtacgatgcgctgtccctggcgctcatagcgcagcgagttggtagcgcatatcacgtcaagtacgttttcaagatgatcttccaggtcaaggtcgccggaacaggtttccagtccgggttgtgttgatgcaaggtccagctgtatattatagtaacgcgttaattttttcaggatttctttcagcggtgtgctgtaaaacagcaggcgcccgtctttccaggcggtataggtagctacgttcacggtgcttacctgcaggttttcgctctccatgcctaccgtagccatttcgttgggttgcagctgacgggaatgttgcccgaagcggcgctgtgaaggcaggtggaggcgcacacttcccgatgccagtaccaggctttgctggtggtcgtccggataagcgctgatattaaaggaggtgccgagcacttctgtttctatacgtgaagcatatacgaaaaatggcgatccggcattgggggctacctcaaaaaaggcttccccttccaggtatacttcccgttttttccggtgaaaggtagcgggataaacaaggcgggagccggcattcagcagcacgatggtgccatcttccagctggaggcgggcgcggcggccgtaaggtaccaacagcgtattgtatggagctgtggacgacagggtactatccgcgttgatggttacgccttgacccccatacaccagtgatgcgttttttccttttactacgatcgcgggttgcttcccaaggatcaggcgggtatcggtggcgcgttccaggtgttgctgctgagcaaactgtaccagtgagtgcggagcctggggccagaacaaccaggtggccacggacaacaacagcaagacggcagcggcgattttgaggaacaggtatctgtgcacaaatggtttggctgctaatcccgcggcgatatcctgccacagcagggctttatcggccgggtcccacgtttctgtggcggcgtttgtgatcatgcgttgcacggcatctgccatttgctgttgcacgggatcatcgctttgtgcaggcggctcatggtcattaccaagcaggtcttccagtttcaggtgtttcttatcaggcatctttcggcatctttgctatatagagcaacaaacaaacaggatatagactccggaacgaaacttttttttattcagggatgctcccgggaaatccaggacattaagaggatcattaacggcagcaccggtaccttttccatgttggcacgcagttgccggaacgctctgtaggcgagagtgcggcaggttggtacacttattttcatgattcccgccacttcttcgtacgacaagctgcagttgaatttgaggaaaaggacttctttctgccgggcgggtaattcgttgagttcacgggccagcagccggagcaattcctgctgctgttccgctgcaatcagcagctgttctgcatccggctcatagaagatcgagaaatagtcttccggattggcagtatgcagcatagtggcattcttttttacggcctggtggattttcctgcggaatgaccggagcaggtaaaaccggatgttcacgtcatgcgccaggttattcctgtagtgataaagactggtaaaaagctcctggatacagtcttttatcgtgctggtatcttttatatatctcaggccataccggaaaagcatatccgcatacatttcatacaactccctgtaggcttgttgatcccccaggatgacattgttccacaaaatattatcagctgcaattaggcggtctttcaaacagtaaatatttagaagtggttgatgcccctaatataaaggaaaaagcagaaagctgaaagcaataaacaaaaagctactggcacaggcaccggagcggatattttttccggagatgaatatgctccgggaacttacctgctttggtcattgcgccaatagcttctttttattttatgcttttgctgaacggggggtgcttatgcttcctggaaggcatgccataagctggctgcgccgatcagtgctgcggcttcgccgagggtagctataactaccgggatggtgatctgttgtttttccagttctttttttagttggggaagaaacagttctgccgcattggcgatatttccgccgatcactacaatttcaggttgttcttctttaataaaggtggtaagaaaagtaccgaggtttaccgcaaactcattgaacagctgcggtatcctatcgtcaacgcctatacgtgctaccagcgcttttacatctgctattgcttcgccgcttatttcttcatagcgttttacaaaccagcgcgtagagagatagtcttccgccataccctctttaaagggagcgcaccagcgattggcatcgttggctgctccgtcgcgataaatggcagaacccagtcctgtacccagtgtaaggccaattacctgttggtgattcctgccggcgccgctgaatacttcgccctgcaggaagcagccggcatcattgataaagcggatttgctggggggaaattccgaggcgcgttgccagtaattcctttacattcaggttgtataaagcgtcatatttgtgttgccctttcatgaggctgatcccccgctcatagtcgaacgggcctggcatcccgatgccgatgtgccgtacatctgcagaagcgtgggcgaaaacctcactgataacagccgcccagccatcgatgatatctgctacttcgccctgtgagttaatacgtgtacggttccatgaactttctatgatggatcttgtgccaagatctacgagtgctgcggtaatgtgagagccgccgatatctattcctaacgccgtggaatttgtcataaattcaataatagaatgttttgctaaatcgttaaagctatacaaatataaaaaactatttggttgacatgcttggaaaaatcgttttagcagagtgaataatggttaaactcctcccaatatagggcgtttttccaaaaatcaaaaaaaacggacaaattttcaacggatatcaaaaaaaactgcccggcattatctgaaacagtttgcaaaaatgatccggaacaacttatctgaaaatccgtgctaaagaaactatcgtttgcccggaattattttgacagatgaaaaataatcatcacttttacatcgtaattcattcttcaatggaatctgatcattgctccggcaacaacatcctgatatcttatatcgctacgaacttcaacacttcgcccccacttttctgaaacatacctgcatggcccaaaccctgatctgacaagtccgtcagccgtatcgccatgccgttaaattcatcttacacaaatacataccttaacaacaaccctgcaaatggaaaacacatttctcagatgggctttgcttatcggcctgcccattctttgccttgtattgtacaaagtaattcttcgtatatgctttggcgtagtcattgtaccggaagaccgtattggtctggttactaaaaaatttgtactgatcggtaaacaggaactgccggaaggccgcatcctcgccaccaacggcgaagctggcttccaggcgcaaacacttgctcccggcgtatacttctggaaatggatctggcagtacagcgttaccttccagccatttaccatcatccctaccggtaaaataggactggtactggctaaagacggttcagaactggaaacaggtgctatcctggcccgcaaggttccctgcgactccttccaggacgcagtggcctttctccagaatggtggccgcaaaggccggcaaactgctattatcacgcccggatcgtaccgtatcaataccttcctgtttgaagtggaaatcacggacatgctgtccatccccgataatgcggtaggaattgtgactaccctcgaaggacaagccattgaaaccggctccattgcgggtaaaaccatcgacaaacacaacaacttccaggatgtggatgccttcctcgaaaaaggcggttacaaaggcttgcaggaacaggtgatcctggccggctcctactttattaacccctggtttgccaaactggaaatggttcgcatgacggaaatcgcgatcggccatgtaggcgtggtcatttccttcgtgggtaatgatggcgtggatctcagcggcgcagaattcaaacacggtaatattgtggccaaaggtaccaaaggcgtatgggcagaaccactgggacccggtaagtatcctgttaatccctatatcatgaaagtagaattggtacctaccaccaacctggtgctgaactgggccaccgccagaagtgaagcccaccagctggataagaacctctctaccatcaccgtgaggagccgcgacggttttacttttaacctcgacgtagcacagatcatccacatccctactaccgaagcccccaaagtaattgcccgctttggtaatatgagcaacctggtcacacaggtgctggaacccactatcggtaactacttccgtaactccgcccagggatcagacgtgatcagtttcctcaccagtcgtaaggaacggcaaacctccgcgaaggagcatatcggccaggtactggaccagtataatgtgttcggggtagataccctcattggtgacattgtgccaccggaaacactgatgaaaacactgaccgaccgtaaaattgcggaagaacagaaaatcacctacgacacagaacgactggcacaggaaacccgccagacgctggaaaaagaaaccgccattgcagaaatgcagaaggaaattgtaaaagccgaccagggtgtttggattgcggaaagacatgcagacgcctccgtgaaaaaagcgaccggcgatgccaacagtgtgcggttgcaagccaacgcggaaagcgaccggatgaaattactggccggcggtgaagcagaaaaagtacgcctgctggcaaaagcagaagcggaacgtactgaatggattgcaaaagcggatgcagaaaaaattgccctcactggtaaggcagaagcagaaaagatcctggctattggtcagtccagcgcagaatcctataaactggcggtagaagcaatgggtggcaacaactttacccaactgaaagtaatggaagccatcggcacgcagcagatccgtatcatgccggatgtactcatcaacggtggagacagcgccaacggcccgatcagcggactgctcggactcagactgctggaagatgtggcaaagaaaaacgaagccggtaaacaggcagaatagtcactgccgcaagcataacaacaaggggagggccgtgatgccttcccttgttgttaaataaagcttccctggacagggttaccaaaaggatagcgttatccttcacgatagcagcgcattgcgtatctttatacccgtttatacccggaaaaagaaaatttgaacgtatgcgaaaagaaaattcctctaatgccatcaacggaaagcagctgcgcggcgactgcggcacagcatataccctgtcgttgatcggcggacgctggaaacccagcatactgtggcgattgctggatggtaaactacgctataacgaactgaaaaagtcgatcaccggcatttcggaaagagtgctggtgttgcagttaagggaactggaaaacgaccacctcgttaagcggatcgtgtacccggaagtgcccccgcgggtggaatacgaactcaccccgctgggatggagtatggaaagtatgttgcagcatatctccgactggggaaacatgcaccgggaagatgccatagcgcgccaggcgtccaaagaaaagaccgtagcggctatggccgataaaggttaaaccgtaagtccggcgtcttccagcgcaccggaagccagtgcggtccagtcggcatcatgtatatccttcgccaggatggttgtgagccggttctgcaccaggttagccagcggcatcggcgtatgcgatttccgcgccgtttgcaataccaggtccatatctttcaaccctaattccgcactgaaagaaggattaccggtaaatttacggtccaggatcatggctccataattcctgaagatgggacccgaaaataaagtagtcgtgagcatttcatatgcctccctgggatctaccccgtttttctccgccagcgcaaaagcttctgccatcagttccaacgccccggcaatcataaaattacccatcagcttcagcacattggcgctgcccgcgtcttctccgagatcaaaaatattgcgggcaaatcctgcctccaataaaggacggatcctttctttagccttagccggaccggaaattaccgaattacccgctttcgcggtcgccgcctccggacgcgcaaataccggcgcccctacaaataacaccccgtgctttgcatgacccgccgacaactccctggaaatatccggtgataccgtactcatagacacatggataccaccttcaccaagggcctgcaccagcgcatcggtagctattgcttccagcgccttgtcgtccgctaccaggctcagtacaattcctcctttaacggcggtttcctccgggccgcccaccagtatagcgcccagctgctccagcggcaacgccttctccctcgtacggttataaattcttaaagtgtatcctgccttcagcaggttctctgcaatgggatagcctaaatggccagtgccgataaatccaatggtttccataatacttcagttaatgacttcctgattcaaatctatcaattcaaaacgattaataggaacatatttggatattgctttgttagtaaagaaatttctgaagtactcattttcgcttatttaacgtattttaatacctgcactttataaaccgccaccgctatgagaacaatccatcaatggctggacgagtacggcagcagccaccgtaaccataccaacaaactgattcactggatttgtgtacccgctattttttttagtatcgtcggatttttatacgcgatcccattgcccattggtggcgtacgttcctacatttcggtagcgcatgtggtattgctgttactgatcatttactatttgcgcctctctccttccctggcggctggcatgttgctgataggggtgatctgcttatggctatggcgccttatagcggccactcagctggtgatctggcaggtggcgctgtttatttttgtagcagcctggatcgggcagtttatcggccataaaatagaaggcgcaaaaccttctttcttcaaggacctgcaatttctgctcatcgggccggcatggctgctgagtttcatctataaaaaagtgggcatccgcctgtaaatgcctcatgtggcagccgacaaataaagccgtaatacataactcatctcgtataagataaataaaataaccagcgccccgtgaaaggtccggttactgatcctgatggccagcaggcagaggacaatgtgcgtgatattacggatcgggtattctatcccgaaatgatgaaagtaatcgtgtccttttatcagcgtatctattacatctgcaataaacgaaaacgccagcaccccaaagaaccactttcgtcgtgagtaaaagtagtcctggtatcctttataatctttcagatcgtcggggtacaatagtgcacagagcaggaaaaaggtggtaataaaggagatgataaagatatattccgggaaagtccatttcttcagtgcatgcaacggcatttcccaccaccagaaatgcaccagcatcacaaagatgtaggctacccatgaaaggtgtatccagtaaggcttttcccggttgggatgctggatgaatttggcagtgcctttgagcagatgtgcaatgctgaggctcaggataaatcctatcaccattcttacatggccgaatgtttccatagcggggtatttctatgaatttaattcattgcccctgaaaaaacaaaagccccgattaaaatcggggcttatttacctaaacctacaactgttacactgttattgcaacaatattttatcttgaaaaactgtttccgttagtgcatagcagacggatcgagtttcgcagctttcttagcttttaccatgagtacaaacggtacgcaaatgaggaatatcaggcccaggtacaggaacacatccatataagataatatggcggcctgtttcgtaacactaaaatcaagtaatttataacctgtattcagtgcctggtgcgggtccattcccttcgcgccaaaactttgctgtaagccgtttacccggttaatcacatcagggttgttggtatccagttttgataccaggtcgctccggtgcagcatattctggcgggccataaaggtagtgatcaaagccaccccaaatgaacctcccagctgacgcatcataccagtaaaagctgctccctggccaatctgctgccctttcaaaccagacagtgacaacgtggtgataggaataaagagtaatcccatacctataccgcgaacgatcagcatccagaagaaggcatctgagccggtatctgccggtgtgataattttatatccccagaaacagaaaacaaagaagaggaacataccacttgccaccatgtattgttgtggaatacctttctccagcattttacctatcagcggcatcattactgcggtagtcaatgctgcgggaatcatcagcatacccgactgggtagcggtccatcccagcgaaccctgtgtgtacagcgggataataaaggtagatccatataatccaaagcccatgatgaaagagagaatggtacctgcccggaggttcccgtttttgagcaccctcagctccacgatagggttcttataggtaagctcacgccatacaaagaagaacagggccaatgcacttgtaacggtgagggccgtaatagtggagtcattgaaccagtcgtcttcctgcccacgttccagcacaaactgcaaacttcctaccatcaccgccaggagccctataccgaggaaatctatctccgacatcgctcttttcgctccgtacttcgggctgcgcacaaactgcaaagtaagcagggtagcgattacaccgataggaatgttgatgtaaaagatataaggccaggaatagttatcggtaataaaaccgcctaacggagggcctaatgttgggccgatgattacacccaacccgtaaatggcctgggcgataccgcgtttttcaggcggataactttctgtgataatcgtttgagaagttaccagcaaagcacctccacccaaaccctgtatgaagcggaatatgatcagctcccacatggcagttgcgttaccgcagaggaaagaggaaacggtgaatataataatagacgccgcgaagtagttacgacgaccaaattgctgtgataaccagctggtcatcggtactatgattacgttaccgatagcgtatgcagtgatgacccatccgatttcactgagcgtagcgcccatgttaccacgcatgtcattcaacgccacatttacgatagtggtatccactatctccagcaaagcgcagaatatagcggtgatcgtaatgatcaccctgcgtgagccgtattctatcaatgattcttgttgcatgcagcaattatattttgaatgagaacaaccctacccggagttaataattaatgacgaacatgacctttctgttgaggatctgttgttagagctaatcgattacgcctgcctgttaattattgcatggttcccactaattattaactccggatacgttgctattcatgtatatgattagttgagatgcacgtctaccagcacgttcatacccgggcgcaactgttttaccagttcatcgttagggttatcgaactcgatttttaccggtaagcgctgcactacttttacgaagttaccagaggcattatccgcaggcagcagggcgaatttagagccggttgccggagaaaaggaagttacttttgcttccagtcctttttcaggataagcatcgatatgcacggtcactttctgacccagtttcattttatccagctgtgtttccttgaagttggccactacccatggagtagtgctcagtaccacgctgaataaagactggcccgccgtaacaaactgtccaggttgtacgaagatttttgataatacgccatcttccggagcgaggattacggaataagacaggttcagctttgcatcttccacatctgtttcacgttgtttgatacctgcattggctacgttgatctgcttggaggtagcgccgctctgggagctaaccacgtttgtctggcggctggcggcggctttttgcctggccagtacatcgagctgacgttcagcagtttgcttggcagcagaggcctgttcaaattcctgttgggtgatcgaatgatctttgatcaggttggcgtagcggtcgtaatcctggctggctctccagaggtttacttttgctgcttcgatctgtgcatcaatggttcctacctgcgcctgtgcggtactgataccggcttcagcagcggcggtggtagcctgtgcggcgcccaggttagcctgtgcggcatagagggcgttttcagcctgctgtactttaatggccaggtcgcggtcgtccaggatcactaacgtatctcctttcttcactacctggttatctttcacccttacttctttcacataaccggatacacggggtataaccgggctcacattggcatcgatctgcgcgttatcagtttcttcatgatgctgaccatgaacatacttggtgataccgaatgcgccgccacccagcaccagcactgccagcactatgacgaaccctttgcttttctttttaggggcggttgtttcctgcatgtttatattgttagtaggttttgtttgagtttgcgtttccacggctttgatatttattggtttgttggtattatttattgttggattccagtatacctgcagactgtaacagtttgttatatgctacaagtgcatctgccttcgcgtacgcatagttgagatgcgcctgcagatttgcaacgtcggcatcgagcaggtctgttgtggtagccaggttgttatcatgcttgttcttcgtaatccggtaattttcttccgactgttctatcgctttgatataagtatccatcttcttgtggctcaggaggtagttttcgtaagattgatatacgtccaggtgaataccatccacgagcttcgcctcattggcctgcacttctgccagttgcgcctttgcattacttacttttgatcctgttttccagagggaagaaagattgtatttcagtcctacgcctgcatttaccgcattggtaatggtgattacattaggaatgtaagctgccacatatccgccggttactgcgagtgacgggaaataatctgctttcgctcctttgattcctgcattggcggctttttcacgtgcgctgagagaagctgcatctttacggttctggtaagccagttgttcaaactctgccactccgcggccatctactttatcatctactttaaatacggtgctgtctacctggatcacggtgttatccggaaggcccagcatgatatccatattcagattcgcaattttcaggttgttttcagcgtccatcagtgccagctggtaattggattgctgtagctccgcttttaaaagatcgttacgggcaaggagaccattcttttccttgttggaaaactccttcactctttcatccgactgccggatgttttcctgtaccagtgctactgcggcttttgccttataaagattgctgtaggcggcaatggtattctgaattacatcttcacggtctttgtccacatccagccgtgcagcttctgccaggtaacgggcagattctttaccgctttgtatcaatccaccggaaaagatgggaagggatacactggcgataccataagctgccgaattcactttggggctttcacttttggcgccaccattactatcatctcccagcttaagtttcatgtcgatgttaggctgtgcaagcctcaaataagaaccggaaacacttacgtccggtaactggcgttcatgggcttctttcagtgaggcagtagcctgatctactttagcgtgactcacctttaattgtttgctgttttgtatactcagcgatatggcttcatttaacgaaagcggttttacgctctgttgtgcggatgctgtctgaaagaaaaaagtcagcagtattcccgatgcaagcgcatataatcgtgtgtatatgcttttagaattcatgtgttaggattgctttgaacaatttttttaaatgtgtacctactctgtttttcaaatactccctgtattcatcgtcattcaaatccttcgcctcagggtttgttctcaatatatgtttggcaggtattacctgatgaatagtcccgaataaagaagtcatcagcatttccacgtctacatctttataaaagatgcctgcttcctgggcatttgtaacgatggggcgcatcagaccgagcatttctcctttcagttgccagataagatccctgatcgggctttgctggctgttcaactgttcacggctcataatgcactggaagtattgctccccgagcattttgttgacgaaccggtcaatcagactgtttatcttctccagtggctccatcgtatcgttctccaacaattcattgatgaacttccgggaagtctccattctatatttgaaaatagattccagcaatttgtcctttgaaccgaaataataggagatcatggcgatattcacatctgcctcctgggctatatcccttaccgatgtgccatgaaagccctgatcggcaaatagccgctccgcaaccgttaaaattgagagctgtttttcactatactcttccatgttccttttttaaatttgacttcacaaagttaaacaaacgtttaatttaaacaagcgtttatttaactctttgtttaaattttgattatttacaactatatatgcatgattatcaataaaatcacttgaaattttaagctgtttttaatatttattaataatctattaataaaagcggtgaaaatcttatcaatggtgaggtttttatagtaaaattttttaatttaagagatgtagtcacactatcctgttttaccatataaaaacaaatcacatgcgtcctgtttcctcttttccgggaactgttttactggccggccttattgccggtaccctggacattctttctgcgtttgtacatttttttattgttacccacggtcagccggtcaccaggatactggtatacatcagcagcggtgtatttggtaaagcggcctttagcggggagccggccatgatgtggtggggattactgtttcactatcttattgcgctcgcctggtcgtttgtttttttcctcatttatccgaagataccgggactgcgtaagcacccggtggcaacagggctcgtttacgggttactggtgtggtgcgtgatgaacctggtggtattgccgttaagccaggtaccgcatggaccactgcgtttagtcaactccgttattaatattctcatattgatggtcatgatcggattaccactttccttcatggcgcgcaagtattatacacgctgaaagcggagggaaatttccctccgcttttgattttaatattttacgccgggaaattccttttgcgcctgcaggaactcttcctcccaactggcgggccagccgaaagcaatggtggcctgcggtttcaggtttacacctgcagcgccgctccagaaatgtatgaactctccccagttcatatcgcgcgtatagccattaccgttacggggaaaattggcggccagtatggtaaagaaattgtttaatactttggcgccgccatactgatggtaaaccgggtaaaaccagtttttaaaccattgtgtacccggccgtggaaaattatctgtattcttcatctgcgtatcaaaccatcgctgcgcttccgcatcccagcccaatgcgcggtatacatcatattgatagatctccatccacttgctgtctttccatatcgggaaggcaggcgacccatgcactcctttggcggcgccctccacaatatgccccacctcatgcacagcggcatccaggttccagccggtattactcacccaatcaccttcatgccccacatcaatcacgttgcggtagtcgtgactaccatcgaaataggtagacgggtgcccgccgccatatttgccggtatgcaacagcacaaacaggcggttatccttaccaaaggcgccataagttttagtagtgtagttccataccttcgttaacaacgtgtccggccaggtaatgctttcaggcgtttctttgtcgtaatacaccgtcaccgacgagttgctgaatacccggcgcatcacctgcgcatgctcaaaccaatgctctttccaggtaagcggcggcatagcggtagtatccttcaccacgggcgccatccatcctgcattttttgcagcaaaagtggcaagggtaaaaagactgcaaccagctaataatacattacataaatatctcttcatacagggattttataaaaaatgctaaatcgattttctgatatcaaaaaagtagtatcttaatggtgaaaatagccaacaggaatcgaatcaattttaaaaaatccctaacggattgtaaacaaaacttaaaagcatcgggagcggacgtcgttatcaagtgaagaacaggaaaagtcaaccaaaagtaataaagcgaagcatgaggcattctatcaagctgtatatcctgacagctgttatctgtattatcgcgttggctattgtacagtttttcctgatatataatacctatcagttgctggacagccgttttaactacgtggaaaaaggaaggatcggcgaagcctataacctggccatcgccaatgataagctgttcccgggaggacagccgctgctggacagtatcattgtgccgcagtacccttacctggaacaactgtataacaccaaccgccacggcttcgacaccgccgcacaacacctcgtgaaccgcatcatccgggaactggtaaagcatgagaacaccgacagcatgctgaaagccatcaaggccaacgacgggatcaaagattccctcctgtttgctttatgcattcaccggctggatatcaagttcaaagacagccagtatgtaaacgtatacaaccgctttaaaaagtacccgctcatcccggccgacaggcaaaaggaaatgggactctttatttgcggcaacctgccgaagctcaatgagaacagcgcggcatcttcgctggtggccaattcgcccctgccctattcttattccctgtcgttctcattttacgcagatccctataaccgccgcaccctggtgctccggcaaatgaaatataccatcctccccggcctgcttaccctgctggcggtgatcacattgtttgccatcacactcttcaaatggatccggcaaaagcatctgtcagatatgaaatccgatttcatcaataacattacgcacgagtttaacacgcccatcaccgctatcatcgttgccaataaaaatatccagaatgaaaaaacgctggataacaaacaaagcgttaccgcgctgtccgaaatcatccaccgccaggcagaacgcctgaaactactggtagaaaaagtgatcaatattgccgccacggagaaactggcgctcaaaaccaccaccaccgacctcaatgaactgatcagcgggatactggcagtgtatagtcttaataccatgaaacagcctgtccgcttccattttcacaacagcggccaaccggtagtgattgaagcagacacctttcattttaccaccctgctgcaaaatatcctggataatgccgtgaagtacaacgaccaggcagagaaggtcattaccattaccacgctgcaggaaaaagaatccatcgcactgatcatacaagacaatggtatcggcatgaacgctgctaccctccgccatatcttcgaaaaattctaccggcatcagcctaacctgtccaggcccaccaaaggcctggggctgggcctttattatgtaaaacaatgcgtggatgcgcatggctggacgattaaggtgagcagtgaacccggtactggcagtactttcgtaattaacataccttcaaaaatataacgctatgaaacatcacattctgctggtagaagatgaaacggacctcggtaacgttgtaaagcaatacctggagctgatggactttaccgtcgactggcaacaaagcgggcgatcggcgttggaggcgtttaccgctactcctactgcctggcatattattctgatagacatcaaccttcccgaaatggacgggttcgaactggcgcaggaactggtgaaaatacaacccagcgttccgttcctcttcctcaccgcgcgtggtgaaaagaaggaccgcctgtacggcctgaagatcggagcagacgattacattgtaaaaccatttgatgtggatgaactggtgctccgcataaaaaatatcctgaaaagaaaccagatcgtaaacagcatcgccaccagcaatgccattgaacttgggggcatgcgctttcataaagactccctgaagctcattggtaatggcaaggaaactattctcaccccgctggaaagcgacctgctgctgcacttctatcacaacagcaataaggtaatccgccgcgaagatatcctgcacgaggtatggggagcaaatgattattttgtaggaagaagtttagatgtgtttgtatcccgcttccgcaaatacttccaggggaatgaaaatatcagtatccggaatatttatgggattgggttcatgttcagtcttacttaataaaaaagggcgggcgctacatcgcttaagggcccgcccctgcacatctcttacaagatgttgtgcctgtttatcaaccgtatcttcatcatttcagtaatatcgtgcaagggaaaaacatatacaggtgggcattgccgctataggtgtttttcatagtgatacatagttaacagggataacggaaaaaagttcagcgggtgcagcgaattttgtctttctcaggattacgctgattttactgattacctggatttttacttttggatttataaaggattaagggagatagaagcggatatcgcttttatctcccttaattatcttaatcaaataaaatccaaaagtaaaaatccaggtaatcagtaaaatcagcgtaatcctgagaaagacaaaatccgcttatttcagtgaattgatccacgtagcaattttcgtggcatctgcctgcggcacctgcgggaacggaggcattggcgtagcatagccaggccagttctccgcctgcggatttttaatcagcgacagtatcttggcaacagaataatttctttttgctacatcacggaaaccaggtcccacctgctttttatcaggattgtggcaggaagaacaggtgtacttgttcagcaatggcttgatctgctcgtaggtcagcgtctttgcaggagctggtttggctgctgtggaagctgcttttgcatctgccaccttggtagccgtagtagctggtttggcagcagagtttttagtgctcagtgcggcaactgccagctttgcaccatcaggaatgttattcagggtgtagtacacgtcaggatgtaccagtgaataggaattttcctgggtacggataccattcagcgacagcttatggatgtagtactggcgcagcccgtcgatcacgaggcgaaccttcataccatcgggagatacctgcacacctttgatggtcagcttttctgagttaacagtaggactgccatataccgggtgatatttatagataaagctttctgcattgtaagaagcgatatcttctgcatactttttatctaccggtaaagtgaaagtaatttcaaaaccgtcaggcatggcgcttaccgttctcatttcaaacggtactttgttgttccataccaggcgttgcaggccctggttggcatcaccggcagaaccccatccacggttggtttcacctacaaagagggaaccgtctttaccccaggcgaggcgcagtacgcccgactggaagccgcttctgaaatcccaggcagcgccctggtattcaccttttactttctccaggaatacacgtacaattttgctctgtccctgatcgccgatcagcacttgtttggcaaacggaccaaaagcaccttcggggatggtggtgagctgtgcattggaaatacctaaaataccgtgtggcagccaaacagcgggcacttgtacttcagggaaatatttcttcatatcaaacagcgttacaaacttttcgttctctacgttttcaggcttgatagcacgaccgtttgcatccctgcggaaacgcggatctactttgctgtacagttcttccgtggtgagttttaccggggaatttggcagattggtccagcgtaagcctgcgggatgtccaacaaaacttcccttcttcacgtgggttaacccacccgatcccatccagtcgccctggttttctgtgtagaacagttctccatcgatcataccaagtccgcatggagagcggaaaccggtcgcaaatggttccattttaccgtcttctgtaatatgcatcatccagcctctccagggtaccttgctttcaccacgccaccattcttcatcgccaaaggcaacgttgccggaaacaaagaaggagccgtctgtgcccagaaccggaccaaagctgtactcatgatagtgaccggataaaggccaggagtatacggtttcaaacaggtccattttaccgtccatgttggtatcggtcattttggtgagttcaccgcgttgtgcgcagtagagggaaccgtttttgtaagccagtcccagtacttcatgcagcccggaagctactttcctgaagtagggtgttttgctggtgggattctctactataaatatatcgccgcggcgggtagctacacccaggtcgccattgggaagggtgcataaaccacccacttccagcagggtgccttcgggtgagctgatacgcgcgatgcggaaaaagtcctcttccttcggggactcctgtgcttttacaggcgtgatggccgttgtcatcaggaacatgcctgcggctattcctgctgtaattcttttataattcagtttcataatagtcattagtgttgctgcttagaagataaccgcataacctgttttcgcctgtaccggcactatcagctccgcgcggccgttctggttgcggataataggattcgctttggcatcatccatcttcacataataagatttgtcgccgatcacatataatccgggagacacctgctcaatactatcgccttcggctatacgcagatacaggtcggatgcaggttgcttcaccgtaacggtacggtgaataccctggttttccgggagcacgctgatatcgtcggttaccgcagtaccatagatattgtagcggaaagtaggtttgccgctttcatcgagtgaatagccggttggacggaagccggtaccggcggtatcagagctccaggcagtttctttggtggccagtttaccaatggccagcgcaggttgattggtaattacctgcacagtacccagcggacgggaagaaccatcgccgcggtcgtgccacataggcgtggtgttcaggaattcgccgcgccacacctggaagggtaagccattgtccatatcgtaggtgtaatgcactttagcaggactgcccacagatacggcgtgtaccacgcgtttaccaccaggtacatccatgaaactgcgcaacacggtgttttcgttggctgttaccaggataggatcagtaggatcatccaccggtacgttggcatcgctgatcacaaattcgcggataccggcttcgctcacggataaagtgatggacggttttgcccagtcggtatttttgacatacagcacttccaccgggtaactgccgggttgtaattcaatgctgccgtggccatcccagccccgtggtgtgacaacaggctggttatttaccttcaatacgccgccgccgccggaggtatgcaggttaaagttgtatttaccagcggttttaatggcgatggtagtggtgtaacgcaccaggaagtcgttgtccggcaaacctgcaatgttggaggtcagcagcgcggaagttccggtagttaagggtttcagggtagcaaagtcgggttctttatcaaagcctcccttgtacacgctgtattttatgccttccagtgttggtctgggagcgctgtagttattgatcacgatgttcctgaaagctacggtgccgtggtctccctggatacggagcgggccggaagccacttcattattttgtacggcgccgcgggtaggtccggaaagcactacgttttcctggatagttacgccgttcagttccagcttcaggataatggcatcggcggttttattgccggcggcatcaaagcggggcgcctggaatgaaattttcatgtgctgccataagccgggcgcgcggcttacattctggcggggagcatgaccgtcgtagccttgctgtccttccggtttgctgtcgttccagcgttcgtagatccctccgttgtcggaagcgcggggagctgaagtgccccagctgtcgagcagctggatttcatatcttccctgtaaataaatacctgaattggagcctttggacatcatatagtccagttcgagatccaggtcgccatgttgcagtgtactgaaaaggtcctgtccatgtgcattcttttcaggcaggtttaccaggatgcctgtacctgcagttgtttgcagcaggttgttctgttgcaggtctgctttaacgccaccggctatacgccagttggctgcgggctgctgaaatgcagataaatctgttaatggcaatttgttctgtgccatcatctgttgacaactgccaatacttaaaatcaataccaaagttctccggtcgtacacacgtaactgtttcaactttggacggaacttgttccatctaagcatagatctggattttttttaaaaagtttacattgattgctaaatgcatttagctctatagctaatacatcattattttctatataggcaaccccaattgttaatgaaatttaaattctcaactatcgctaaacgtgggactggactaattttgatcacgggtgccaaaatagaaattaattacaagaaagtagtcagtgggagcaaaaaaattacaccagcggtaaaaaacctggcggattttgtctttctcaggattacgctgattttactgatttttactttttggattttttttgatttaattattaggggagatataagcggattttgtctttctcaggattacgctgattttactgattttacttttagattttataaaggattaagggagataaaagcgaatttgtccgcttatatctcccctaattattaaatctaaaaatccaaaagtaaaaatcagtaaaatcagcgtaatcctgagaaagacaaaatccgcgacaatctacaataccaatccgaaagccgccagtttttttacggtgctttcataatctgtatggcaaacgccgttgataccaagacccgcagctacatcgatgaacatggagcggtcttccacatacaccacttccgcaggtttaacctgtgcaatatcgagtgctatcttatagatatctgcatcgggtttgcggaaatgtacaaagcaggaagaaatgtaaaagtcaacaaaacggctgatattaaaatgatggatccggtgttcattcagctccctgccttcattattaacgatagcaattttcagtttgtatttttctttcagctgtgggatcagctccagcatctccgggtacggcgccgactgggcaaacataaactcgcggaaatcctggcggctaaaggatctgtcttcataaaacactacgcggctcaggtattcgtccagcgtgagtttaccttcttcgtaagtatcaaaggtaaggtgatgccgttcttccgtttccaatgcatccagcccaaaagtttgtatagccagtttacgcgcggccctgtcccatccgttagttaataatacgccgcctatgtcgaggaacagcgtcgtaatctttacatggttgtccatctgcagaaaaatttattgctacgctaatgtaaggatttgtgcggaggttgtcttactcaggattaaacttattacattgattacgctgatttgatcactttggattttaaaagatttggggagacgcggattttgtctttctcgctgattacgctgattttactgatttttacttttagattttataaaggattttaaataattggggagatataagcgaaaatatccgcttttatctccccaaatcttttaaatcaaaaagtgatcaaatcagcgtaatcaatgtaataagtttaatcctgagtaagacaacctattcttctatctccccaaatcttttaaaatccaaaatgatcaaatcagcgtaatcaatgtaataagtttaatcctgagtaagacaatctccgcttctatcttcccaaaatcttctaaaatccaaagtgatcaaatcagcgtaatcaatgtaataagtttaatcctgagtaagacaacctccgcgctgcgttatttcttctttttaacttttctttctgttatatacccgttaaaactgatcggcgacctgtcgctgctggttacctggagcgatgcatagccttcgccggaaatgctcaggttcatcgattgtactgatctgtgatctttgggcttaatggtaatattccagccatcctttttgccgggagtggcgttatagtcgaaagatttggttttgaaatccagtggcgacctggtggcgccatagtccaccgatgtataggcacggccaaaataaggcaggtagctaattacggagtcggccgctactattacgttgtactccgatgtaagattacgcatgcggccactcatgggcagagcattctgcgctacaaaaacgtaattctgcgagtcaatcagggatttgatcttagctactttatccgctttttgctgcgcttttgtttcctgtgcaaaaaggccggtagatataacggctcccatcagcaggagcaccattgtttttaatacaaagaaccttttcatatggtaagtttttacgtaagagggaatgctaatatcgtaccataacagtaaggaacttcgttttgttcatcgccattgcgatacaaattgagcgtaaaacattacttttaagggccaatgattaaacccggaaacatgcccaacccatatgtctcgttactgaaaaccgcctggaaatatgcccggaaagagcgtaagaaatacctcctggtctatttccttttcctgatggccaatgtgatcttttccctgaacccggtgctgttcggctggtttatcgggagcatacaacgcgacagcgcccatctgccccggtatacaatgatctttggcgcctcctacttcggacttaaattcctggaatggtgcttccatggccccgcccgcgtaatggagcgccacctggcatttaacctgagccggaacttcctgcaggaacgctatcaccaggccctccatcttcccgtaaaatggcaccaggataaccatagcggcgccgtgatcaaccgtatcaggaaagcatacgaagccctgaaagagttctttgaacgcggctttatgtacctccacgcgatctgtaaactgctgttttccatgatcgccatgctgtatttttctcccctctatggaagtatcggcattgcgctgggcgtgctatgtatatggattgtgctgcggttcgaccgcccctttatcagaacactcaatgaaataaatgaaggcgaacacgtagtatctgccacgctgttcgacagcctttccaatatcatgaccgttattaccctgcggctggaaaagagcatggaaaacggtttactggcaaagataaaacgcatatggccacccttccggaaaaacacggtgatcaacgaatggaaatggtttgtagcagaaatgatgatttcacttatttactgtgttattgctataggttatgttttccagcattgggtaccgggagaaatattctatgtagcgggactcgtcaccttgctgggctatgtaaaccagttcaccagcgtgttccaggatgttgcctggcaatataccgacgtagtgcaatacaataccgcggtggataccgccggcaatatcagcgacgcctatacgcagcatcaccgggcagatgctgcaccggaactgccggccgactggcagcagatcaccatcagctccctgagcttttcgcacacggctacctatgaggataacgcagcgccgcaacgcctacacgacctccacatcctggtggagaaagggaaaaagatcgctttaattggggaaagcggcagtggaaaaagtacgctgctggctattttgcgcggactctatgaacccgaacccggcgtgatgatacaggtaaacggagccgcattaccgttggctaccgtgaatgaaagcgtcaccctgttcccgcaggaacccgaaatctttgaaaataccatcgaatataatattacgctcggcctgccctttcagccggatgaaatcatggctgtgtgcagcagcgcccacttttcggaagtagtggaaatgctgccacagggactggcttccgatatccgtgaaaaaggcgtgaacctttccggcggacaaaaacaacggctggcgcttgcccgtggtatcctcgcagcgcgcaacagccaggtgatcctcctggatgaacctaccagcagcgtagatcccaaaaccgaggccatgatctacgaaaaaatgttccaggcattctccgacaaagctattatttcagccatgcatagactccacctgctcccgcagttcgattatatctatgtgctggaccagggccgcattgtgtctgaaggtactttccattacctgcgcgccaacagcgccgctttccaggagctttggagacaccaggaaaacaaataactttttttgctaatattgcagtatcattacagtcacgctttcatcctatgtaatggttctctccctgctgatattacactatgaaaacgctatgcaaaaaatttcactgtacgacctgaaacgtaagctaagaaacagtcaggagccagatgaaatgatcaccctcctcggatataacctttcgtttttttcacgggaggaacggtcgcaactactatgcgatttactggaataccaggaaatattttttgaggcagcagaactgctgattgaagaaggcggggccgacatccattataaaaaggaaggtattattccaatcattttctgtgcagtaggcgccaataagccgcaggctgtacaatacctgctgaaaaaaggcgcctcccttcacatcagcaacgccgattacctgtttgccattgcctatatcttcaaacatcaccggctggcggccatcacggacatactgctgatcctcatcgagcacaacatccacttcaattttgtactggccagtatggatacccctttgctgctggctacccggcataataataaccgggaggtagtacagtttttattgtcggaagaagtgaataaatacgtgtatgacgaagatggctttaccgctatccattatgttccgtttgccaaagcccctcacctgtataaagatatgatcacctgtatggcggatatccaggtgaaaacgaagtttgccaccagcatggagcccgtctttgaatgcgtgatcaaagtgagtgaacaccatacttttgaagagtttatttatgaagccctgaacgctttcctggaaaacaggcaccgcatgtacgatgatatctttgaaaaatactattaccgccttcaccttatagcagaacatatttccactatccgcgccaacgccggcgataacgtatgacgcattttaattttgcaacaaagttgcaatatcttatttttgtcttcttacatgattattaaataccaccatatgcaaacatacgatgtgatcattgccgggggcagctatgcggggttgtcggccgccatggccctgggccgcgcacgccggcaggtactgatagtagacagcggcaaaccctgtaaccggcaaacgccgcactcccacaactttctcacccaggacggcgctacacccgccgccatagcggctgcggccaaagcccaggtattgcaatacccaagcgtacgtttccaggaaggaacaataaccggcgccactcccaccacggaaggctttacagttaccaccgctgcaggcgaacagtttgcagctaaaagacttctgtttgctaccggcgtaaaagatgaaatgcccgctatcaaaggatttgcagaatgctgggggatttccgcactgcattgcccctattgccatggctatgaaataaaagacacccccaccggtatcctggccaatggcgacggcgcttttgaatacgctaaaatgatccgcaactggaccaatcagctgactatattcaccaatggcccatccacactcaccgcggaacaactcggaaaactgcagaaacaccgtatcgcggtcgatgaaaaagaaatcacggaaatcaaacaggcaggcgggcaaataagtgaactcctttttaaagatggcagcacccaggcgctgaacgctttatatcacaaacctgccttccggcaacactgcaacgttccagaagcactgggctgcgaacttacgccggaagggtatcttgtagtgaacgaattccaggccagcacggtaacaggcgtatacgcagccggcgatgccactaatcctttcaggagcgttgccatatcagtagcagcaggaaccctggccggcgcgatgatcagccgggaactcattatcagtgaatttgaataaaacagaccagtgtgtgagcagtcatttgtacatgtggaaataattctatattttagaacaagtgattattttccattacctaaattaaccagaatgctcacaacacttactgtcttagccgccctattcttcctggcccacgtttatctcctgtttacctcatttggaaaaaaaggatttcaaaaacaaaaatatctatggtcgcatattaccctgtggattacaggaggcctggcctgcgttattgccgtcctttttgccggtaaaaatgtttccggcgtaatcgatgtatttgatacccccggcaaagcgtccctgcttatcctgatagcactggtgttgtcggccacagcgcacagcatcgtgaaactgctggtgctgccaaaataccaacgcgccgtataataacggaacagattatacgaaaatcccccggcggaacagccaggggatttttatataaatcatacctgcacgaccatttatgttcatttaacggtccgttttgttacataaaatgttaaaggtggaaaattttctttcgccatcaacaatattcattatatttatacctgttgatcctggtttcttataaccgccggcgctgactggctaccgcaacacctgcaatactccgcaggttctgacagatgatcaccatcaaaagaaaaaattgcgcgttgaaatcatcttcataattaattattttattagcacgaaaagagagacacatttttatgaataagaaagatatctggagatataaatctttggagcagttggagaataagagttgggcaccggccacagatcaagattcgggaatagttcagaaatgtcttgccttagttaaagtaccagtagtaaaattagccgcaagcgaattgcggatcttaatcggacaatcctttaatccttcctacctggttcctttagcgctggagatattacaaaacgatgtactggtaaccgccggtatgtatcccggcgacctgctgaaagctgtactcgacgttcctgctgctttctgggaagaacatcccgatcttcacaaaaacctgctcgacctgatgcaggaacgaagcgaagaaattgaaacagaaatagacttacctgaattctggcgtaacaacctggtcatgtaaccatggctgttttcacattcgctattcatcaaaattgaacaacgaaagctgtcctgacggaggaagtttctcctggttcatcggcgcatcattgaaattagacagggtaatgcctaacaggcggattcgcttatcttccggataagtagctgccagcaattgctttgccgtgtctacaatgatatcgtaatctcctaccggaaacggaaaggactgattccgcgtgatctgtttaaaatcactgtattttattttcagggtaatagtgcggcctttcaggttatagcgctgcaaccggtcgtatacggttttcccgatcttctccagctctgcttccatatcggcgatcaaggtaagatcataggggaacgtatcctctgcgccaagcgatttggtttcccggtgcggctgcacctcgcggtcatctatgccccgcacaatccggtagtaaaagctgcccaccttgccaaaatgggttttcagatcctgctccgacaatttcttcagatcagccccggtaaagagtcccatccttttcatcttatctgccgtcactttgcctactccgtgaaatttctctaccaccagcgtttccataaacgattcaatagacgatggcccgataaacgtaagcccgtcaggcttgttgaggtccgacgctattttagccacaaacttattgacagacacgcccgccgatgcagtcagctgtaactcatcccggatggcctgcttgatcagtttggcaatttcaatggcagaaccgataccctgcttgtcttccgttacatccaggtaagcttcatcaagcgataaaggctcaatcagatcggtataccgggaaaatatttcccggatatgccgcgaagcctccttgtaagcatcaaaccgggggcggacaaaaatcaactcaggacataactgcaacgctcttttggaaggcatcgcggaacgtacgccaaatttgcgcgcctcgtagctggcagtggctactactccaccccggccttccggcgaaccgcccaccgcaatggctttgccacggtagatggggttatcgcgctgctctacagatgcgtaaaacgcatccatatcaatatgaataatttttcgttgtatgctgtttgaacggttctccatttctacatcccggaagcaaacataaagatattcagtatttagctattcaggctcacaaaatgattttttttacgccttcactgctaaaacataatccctaccttcacaccttaaacttttcaccgtgtccggctacgatcaggaaatttcgcacgaacataaaaaatttgaaaatatcatctgggagggcaaaaccatctcgggcagggagttctacgattgccatttttataaatgcagtttgaaggaatgcgtttttgaagaatgtacttttgataaatgcacctttgaagaatgcgatttatcattgatacaattcaaacaaacttctttcaacaaagtgatcctgcaacataccaaagccattggtattgcctggcataatgcccgcaactcacttaccgtagagtttcaccacagccgcctgagctactgcagtttttcgggtaagaacctgaaaaaaggaatcttccttcactgccaggctgacgaagccgatttttccggctgcaatttatcgcaggcggatttccgcggcaccgatctggcgggagcccgcttttccgacacagacctcacccaggctaactttgtgggcgcacaacggtatgccattgatgtacacaccaataaaattagaaaggcgaagttcagtttgccggatgcgttgtcgctgctggatgggttgggtgtggagatcgtggaataagcggaggttgtcttactcaggattaaacttatttcactgattacgctgatttgatcactttggatttttaaaagattttgggagataaaagcgggttttgtcttactcaggattaaacttatttcactgattacgctgatttgatcactttggatttttatatgattttgggagataaaagcggatattttcgctgatgtctccccaatcatttaaaatcctttataaaatctaaaagtaaaaatcagtaaaatcagcgtaatcagcgagaaagacaaaatccgcgtctccgcttttatctccccaaatcatataaaaatccaaagtgatcaaatcagcgtaatcaatgaaataagtttaatcctgagtaagacaaaactcgcttttatctccccaaatcatataaaaatccaaagtgatcaaatcagcgtaatcagtgaaataagtttaatcctgagtaagacaacctccgctgccaaatattgttataaaaatggattttcttactttgagaagaaaaccggctgcgttatgatcaggaagaaagaaggctttcagggccagcggatgatcgtgataccgcgtaatatcctgagcaggaaatgtgcccgggaagcggtgctcacacccttgcacctcaccgatatcggttattatccgaaagcattgttccaccaccgcaaaagagcgcagggggcggagcagcacatcctgatttattgcgtggagggtaaaggcagtatcacgctgaaaaaagaggtatatactatccaggcgggcgattgcttcctgctgccccgcaaatgggcgcatgaatacagcgcagatgagagtgatccctggaccatctactgggcgcatttccagggtaccagcgcagatgggatcgtacaatcggcggtcagggaatggaatggcaaccgggtattccttccccattccccggaacggatccagctgtttgaacagatctatcaccaactgcagcggggttaccgcgatgaaaacctggtgtggtccaacatgaatttctggtcgttcctgtcgtcctgcatttacccggatttcacacagcccggaaagcccgcccagcaacacgatgccattgaccagtgcatcgattatatgaataaacacctcgatcagatgcttaccctgcaacagatggcacaggcggtaaacctctcccaatcgcacttctcctatctctttaaaaccaatacgggcttctctcccatcgaatacttcaaccagctgaaggtccaaaaggcttgccagtacctgctcttcacccaatcacgtatcaaggaaatagccgccctgcttggcatggaagatccttattacttttcccggatgtttaccaaggtgatgggtgtatcacccaatcagtacagggaaaggaagttctgaccgtaagataatccatcataatcagcatatcatctagccactattcgatggtcccggcttatttttacggacgtcaatgaaaaaaacaatgttccatttctccacgttgaggattacagtgagcctcaccataacagtgggggcaggcctgctgtttgccgcctgccataccgataaaaaagtagacttcagtaccgaggtaaaaccagtgcttaacaagcattgtatcagttgccacggaggagtaaaacaaaatggcggattcagtgtgctgttccgggaagaagcccttggcattaccaaatccggaaagcccgccatcattcccggtcatcccgaaaaaagcgaatttatccgccgccttacctgcaaagatccaaaagaacggatgccgcagaaaggagaaccactcaccaacgccgaaatagatatcctcacccgctgggtgaaacagggcgcggaatggggagaacactgggcgtatatatctcccaaaaatgttccggtacctgatattactattaccaacggcaacgaaatagaccacttcatacaggaaaaactgaaacaggaaggattgaagccctccccggaagcagataaaatgaccctgctccgccgcgtaagcctcgatcttaccggtctgccgccaacacctgaaatggcacagcagtttgccgccagcaccgacgaacacgcctatgaaaaaatagtggacagcctcctgcaatcgccacactacggtgaacgctgggcagccatgtggctcgacctcgcccgctactccgatactaaaggttacgaaagggacgacagccggaaaatatggcggtaccgcgactgggtgattgacgcatttaacagcgatatgccgtacgacagcttcaccatcgaacaactggccggcgacctgctccccgatcctacccgcgaccagctcatcgctacggcatttaaccgcaataccatgaccaacgacgagggcggtacccaggatgaagaattccgcaccgccgccgtaatggaccgcgtaagcaccaccatggatgtattccagggcgttaccatcgcctgcgtgcaatgccacagccacccttacgaccccttccgctttgaagactattataaactgatggccttccttaataatacccgtgatgaagatacccacatggaacatcctaaacttcgtttgtacgacagcgttagtacggcagaagtaaaaaaggtaagcgactgggtagcgcaaaacggtaccacccaacaggcaaaagatatacaggagttcctgaaagtactggaaccaaaagtacacgcccacgttgccgataactatatcaacggcgccctgctggataccaaatacatgggcatccggaataacggcagctgccgccttcccaaacagaacctggaaggcaaaacacaactgctcatgaactactggaccggcagcaaaggcggctccgtagaattcagactcgacagcttaaatggccgcaccattatcaaacatacactggcccccaccaacgggcggctcgccatcagtatgccactgccaccggtaacaggcacacatgatctttacctcattttccgcaacccttccctcaaccccgcagatgcggtgtgcagcgtggaatggttcgcctaccgcgacgacattcccggtaaaggaaaaccaggttatgatcagatcaacaacacctggttaacactcattaaccaaaacccagacgacgtaccggtgatgatagaaaatccgccggtaatggcacgcgtcaccaacgtgtttgaacgcggcaactggatggtaaaagggaaagcagttacaccggatgtaccacactccctgaacccattccccgcaaaagcgccacgcaaccggctgggtttcgccatgtggctcaccgatacaaaaaatcccctcacggcccgcgtaatggtgaaccgtttatgggaacagatctttggcaccggcatcgtggaaaccatagaagactttggcacacagggtttcaccccgtcgcatcccgaactgctcgattacctggcctaccagtttatgcacaaatacaaatggcatgtaaaaccaatgctgcgcgaaatcgtattatctgccgcttataaacaatcctctgccagcacaccggaactgcaggaaaaagatccggctaaccgcctgctcgccaggggcccgcatttcaggcttacagcagaagaagtaagagaccaggcactcaccgtgagcggcctcctcaaccgtcagctacacggccccagcatcatgccatatcaacccgataacatatggcaatccgtttggagcggcgcctactggaaaactgccgacgacggcaaccagtaccgccgggcagtatatgttttccaaaaacgtaccagcccctatccgtccatgctctccttcgacggcagcagccgcgaagtatgcctgcaacggcgcatccgcaccaacacgccactacaggcactggttaccctcaacgacccggtatatgtggaaaccgccgcctcactggccaggcatatgctgaaaaatggcggcaacgacgccactgcgggtatccgttggggttatcagaccgctatgtacaaaccattgcctgaaaataaactgaaagtattgcaaacactgtataaacaggcactcgcggaatacaaacaaaaacccgcggaagctgacaaactgttgcaacacaaagataatacaccacaaaaagcggaactggcagcactcaccgtagtagccaacgctattatgaacctggatgaattcctgactaaatcctgatccggtatgactaagcatgcacgactgataaaggaagcaaacgatcaaacactgcggtatttcacccgccgccacttcctcacggactgtgtgaaaggcctgggcgcagccgccttcagctctttcctggccagctgcggcagcagcaccaaaaccttgctggacctcgcgggcaacccaatggcgccccgtgtaccacagtttcccgcacgggcaaaaagcgtgatctacctccacatggcaggggcaccctcccagctggaactgttcgactataaaccggccctgcaaaaattacataatcaactgtgtcctccatccctgctggaaggtaaaaagtttgccttcatccgcggcgttcctaaaatgctgggaccacaggccgtcttctcccaacacggggaatcacgcgcctgggtatccgatcacctgccacatttcgctaccatggcagatgatgtgagctttttgaaagccgtgcaaacagaccagttcaaccacggccccgctcaactgctcatgcaaaccggcagcgcgcggctgggacggcccagcatcggctcatgggtgacttacggcctcggttccgaaaacgataacctccccggctttgtagtacttacctccggcggtaaaacacccgacgccggcaaaagcgtatggggcagcggtttccttccctccgtataccagggcgtacaatgccgcaccaagggcgaacccgtactgtacctcaccgatccggaaggcatgagccgcgacctgcgcaaggaatctatcaatgccatcaacgaaatcaacaaacaggaatacaccacctttggcgacccggaaaccctgtcgcgcatctcacagtacgagctcgcctataaaatgcagatctccgtaccggaagtaatgaacatcaacaaggaaccggattatattcatgaaatgtatggcacacagccaggcaaggaatcatttgccaacaactgcctcctggcccgcaagctcgtggagaaaggcgtacggtttgtacagctgtacgactggggctgggatagtcatggtacagatgaaaacctggccatcgactacggcttccgtaataaatgccgcgaaattgaccgtcccattaccgcactgctgcaagacctgaaacaacgcggcttgctggatgaaaccctggtagtatggggtggcgaatttggcagaacacctatgcaggaaaacagggacggcaaagacatgcccttccttggccgcgatcaccacgtagaagccttcaccatgtggatggcgggcgccggtatcaaaaaaggattttcctacggagaaaccgatgaaataggctacgccgccgtgaaaggaaaagtagccatcaacgatattcatgccaccatcctgcaacagctgggcttcgatcatgaaaagctcacctaccagttccagggccggccattccgccttacagacaccggcggaaaagtaattacacccatactaagctaaaccgtacatgaacagtaacaggagaaattttatcaaacaatcagccatactgggttccgcattatgtatcccttccctgccggcatttgccacaggaacagccgccgccgcaaaagacggataccgccttattgtactggccaccaactggggctacaacggcagcatcaacgacttttgcgcacaggcaaaaaaggcaggatacgacggactcgaaatatggtggcccaacgaaactgccgcccaacaggaactatttgccgcagtggaacaacacggactggaagtaggttatttatgcgcgggttacgatggcgactatacgaaacacgcacagcagtttgaaaccatgctgaaagcagccaccggcaataataaaatcaaaccgctgtatatcaactgccactccggaagagattatttttcctttgaacaaaacagtgcattaatagatatgaccaaccggatatctaaacaaacaggcattccggtataccatgaaacacaccgctcacgcatgttgtttgccgcacatattgccggtaaattcatcgatgcaaaacccgacctgcgccttaccctcgatatttcacactggtgcaatgtacacgaaaccttattgcaggaccaacaggctacagtagccaaagcattggcacgcgcaggccatatacacgcccgcatcgggcatccggaaggaccgcaggtgaacgatccccgcgcgccggaatgggccgccgcggtgaaagcacatttcagctggtgggatcagatcgtgcaacggcaccaggccgccgggaaaccgcttaccttcctcacggagtttggtccggccgattacctgcctaccctgccctatacccggcagccggtagccgatcaatgggatattaatgtatttatgatgaaccagctaaaacaacgttacagcaaaccatgagattattgatcagtagcggcagctggagtatgtttattggacgttcgcatcctttactggtacacctgcctatcggcattttaattattgcatttatattaacactgctggcgcgcagggaaaagtggcggcatgtacaaacagccctgccggcagtattgctggcggctgccttgtcggccatactcagctgcatcaccggctacctcctgtctctcgatggagggtacgaagaaacactactgcaaacgcataaatatctcggtataggcgtagccgttatcagcaccgggttgtacctgctggaaagaaacaaacaccgctttccccgcctgcaactgcctgctgccctgctgatggtattgctgctgggcgccgccgggcattacggcggtagtcttacccacggcgatgattacctcacccaggccatgcccgccccgttacagcggatcaccggcatgaacaaaacagtgactaacgctgccacctatacgaatattggcgatgcccgtttgtatgaagacctggtgcggccggtactcaccaaccgttgctatggctgtcataatgaacagaagctgaaaggcggtctgcggctggaatccattgccctcatccgtaaaggcggagagcacggaccagtgctaaaggacagtctcccggaagaaagcgaattattcaaacggctgatactccctgaagaagacgaacaccggatgccgccaaaaggcaaaccgtccgtaacgccgcaggagctggaactgttgcactggtggatagcggaaggcgctcctgcgggcaaaacagtaaaagagctggaaaaaacgtcccggatcatggcggtgctggaaggaatgcaacccgctaccccactggataaacaggaatttgttccggaagaaaataccggtgctgccagtgaacaaaagatggctgccctggaagcattaaaagtaaaagtaatgccggtgggcgctggcagtcattacctcactgtagacgccatcaatgccgccggcttcagcaaccgtgatatgcagttgttactgggcttaaaggagcaactgatctggctggacctttccggtacggccattaccgacagcgcattggccgtgctcggtcagctgaagaagctcacccgcctggatctgaggaatactgccattaaaggtaatggcttaaaagagctgggcaactgcagggaattgcggtatctgaatctcgccgggacggcggtaaatgcagaaggattattatcgctgcagcaaaataaaaaactgcaacagttatatgtataccaggcaggctttacacctgcggcactccggcagctgcagcaagctttacccaaactgaaactggataccggtggttaccgtttacaacaactggcttctgacacagtcatctatcataaaatcagcgggtaaattatcgtgcaggcatacgcgttattcgtactcctgcgcggcctgtgccagtcgcaatgcaatttttttagccagggatttgggggacagtacctttatatgttccccgaatcccaggatttcccgctccagttcaaagttcagcaccacgtcgatactcacgatggtggcctgttcatcttcctttaatatttcctgcgaatgatgcagcggctttgtaagcacataaggtgcatgcttgttatcaatttgcagcactactttatgtgcaggatctttttccgttttggtaacgccaatgaggttatcataatattcatcaaagggcattccgtcccaggccataaattgctctttcggtaattcctgtatgctgatgatcctgtccagcgcgagggtaaccagctgcggggtgcgtttattccgcgtgataaggaaccagcggttacggtattctttcagcaggtagggataacagacaaactcctgcgctttgctggctttaaaagatttatattctaccaggagggctttcttatgcaggattgcctggtaaagcgggttgatatgcgataagcccagcagccgatgattattttccagctggatgcagttgagatgtgcatcggtagatttatacaggttgttttccagccgggcaatcatgtcgctcatatcatcgaaataactgaagccgttaaactgtttcagcaccgctactatttctttcattttatctacatctgcattgttaatgggcgcattggtaatgctataggccgcatcactgtaagcataatacttacggtccttcacaataataggcgcattataacccagtttatcgctgcgcatcagctgaatatccgcctgtatggtgcgtttactcaccccgctgctgatgccttcaagatcatacaacacctccgctactttttcaatgagatcttccagcgtccatttacgatagcggttacgcaggcactcatcaatggccttgtaccggatcaacgccagtttattgatggacatactaataatttgtacaaagaaacaaaaatactgcgcattatacctgcgtagtattttttctttttagaaagaatgaaatataaaccacagataaccagatgtttaaaataatttttaaagaaatatttaagtacgcaggtatgctgcgcagatacatgcgcatctttgtgtcatcggaagcggtcaaataaatgttacttcacgaacctaaagcacatttataattaacgcagaagatgggaaagcagtagttcaatggttgaacaccggtcgctagttttaaaattaccagagggtcaattgaaacttacttccagactccaatccggagttgctggttcgaatccagcctgctttacgaatcgaggtcaattgttgcttacttcatttttggataaacagcaacaaaattatctgattattaaataccattacaatgaacactttattaagaacaggattaacacaacaggcgatttacattccgcaaacagtggtggaggaaaacacctcacagatcacccctgcatctggcctgctggtggccaatctcgctaaactgggattcggcgtaacggaagatctgctccatgcactgaaccatacctcaccggcttaccaggctacgatcctggaaacattccgggaagtgatgggcgtgaacaccaactggaccccgctgataaaaaactggcaggtgcctaccaatgaatcattcgttgatcacctggtcacttatttcactaatatatttaacggtcctggtactacactccaatgcggccatatcattcctcccaatacttttccgctggaaagatataacggctgtccttactgcggtacaccgtttgaaaccggcgaactggaaaacatgggccagggaagcaagatccgtgtgctgaaacgctgggatgaccagctggcggccaaatacctggaggatctgctgacctccaaaaccgcactggatgctacccaggtggaaagcctgaaggcattgatgcataccttcccgctgcctgcagtgaaaatcgggatgaaagaaaccgtaatagccgtaatagatgtgctgatcgaaaaagatgaagcggaacaggcagggaaactgtttactacgccaacggatatactccgttacctgtggtacaaacatacagggttcctccagctgatcaaacccggtgtgatcattaaacggaaaaccaaaaaccagcggcaggtccgcccggatatttaccctacgatacaaacggcatcaacggctgcggccctgaaactgaaatacagccgtcagcagggactgatagccgcgcgctggctgaacaacctggaaatggacataactaccatgtgcgaaaccatgcacccgcaacgcgggatgtgggtacgcttcatccgtgccctgcgcctggcggagttcagcaaacgtgaagggtttggtaaactgcgtgaactgatggaccggttctaccgccaggattataccatgtggcaggaacgggtgaactactaccgtttgcgctatgatgaagctaccacgctgcagctgctgaaacaacgtccgggtctttttgcccgctcgctgtttgccaacatgctgtggttcggaccggaagcggtaaccgccgcctttgcggaaattacggataaagtgccggcccggctgttgctgaccttacagatgtacgcagggtattattttgataaatccaccacccgtgcggtaaaaccactgggaggtattgggaaaagcatccctgccaaccggcagctgaacatctatgaagacgagcagttgcaggaaatgcaacaggccgtaacagacctttgcatcctggccatgaagaaacgctttgccgcagtggccaccactgctcaaagcatctacattgcaccggagctgtataaaataccgctggctatcggcgaccgcagcgaacaggtacaagacctgccaggcgcgttaatgggtacccggtttaaagtggaaagcgataaaatcatcctgttcatgcaatggggtaaaggattagccgcccagcacctggatatggacctgagctgccgtattgcctacgaaaacaaccgtacagatacctgctccttccaatatctgaaaacaaccgggtgtatccatagcggggatatccgctccattccggaaaaagtgggtacagcggaatacattgaaatagacattcctgcattggccaaggccggcgcacagtatgttactttcacctgcaatgcctacagccagggcgccatcgccgtgaacctggtactgggatggatgaacagcaaacacccgatgaaggtatccgcgaaaggggtagcctacgacccatcctgcgtggatcatatggtgcgcgttacgggcggattaaccaaaggactcgtattcggcgtgctggacgtggccgcacgggaaatcatctggctggaaatggctttcgatggccagatgatacaggacctcagcaccgccaatgtacaggctatcctgaaaaaactggacagcaaactaagcattggccagctgttagccgccaaagcggaagcccagcaattacaactgaccagcgacacaaacgccgacgaagtgtataccatgcaatgggccctgaataccgccgccgtgacacaattgctcatcgattaatttgttttccccctataaaacaacagcagccgggccagccccgtgctgctgtccgttatatgttttaacacactttttgcatacccccacgtcaattttctgaaaatcgtcctatattcattccattgtcatacatggatagaaagattttactactactgctactggttacgcctgctgtagggtatgcccagcaggaaagcacggcagactcaacagccaccatctcagcgcccaaaggtttttttgataacatcaagtattacctccagcataccaacgtagaaaagaaaaagaagaaggtagatctcagcttcatcggcggccccgtatacacccccgaaaccagcttcggattggccgtaatgatggccgcacaatataaaacagatagaaccgactccctgctgcccgtttccaacgccgccgtgtacgcctccggcgccctcaccggcttttatggaatcggcatcagcaacaccactatatttccacacgaccggttccggctcgcattaaaggcctccttcagctcccggcccaataaatactggggcatcggctatgaagccggcagccgcaaagatgactatacggaatacgtgcagctcacagaaaaactccaggccgacttcagcatcaacgtgaacggaaacctgttcgtgggcctctgcacacaaatccagaacgtacaaaccaaaaaactggatactgccggcggcaaacccctgatggttcccggaaaggtactcggcatcggggccggcccgtttattgtatacgacacccgcgactttattcccaatgcctacaaaggcatgtatatacggttgggataccgtttcttcccctcgttcatgggcaataaagccgtattttcgcaactggatctgcagttcgactggtacaaacaactatggaaaggcgccgtactggccaccgatctgtatgcagaagaacgcagtggcgatgttccctggagcctgctcggtgaagccggtggctccagccgtctccggggctattatgaaggccggttccgcgacaaaaactacgtggccgcacaggtggaactccgccagaagatctacaaccgcagcggtctggccctatgggtaggtggcggcaacgtgtttccccgcttcaatgagtttgaattccgccagtcactggtcagctatggcatcggttaccggtgggagtttaaaaaaagagtcaatatccggctggattatggcagaggaaaagatcagcagggtttttactttggcattaacgaggttttctagggagaagacagcttttctgtctaaacaccatcgcttcaccggcctcaaatcctttacagcagaaggttcccggatcaagtccacgtcacctccacatcacttccgtgtttcctccatgaataaggcatgcgccaggtatgtcctaagccactgcgaagcaggtttgcccccatggctacctggtaagaagcttacttattcccctccatctgtttaataatattattcacctccgtttcggtggcgcgtaatttttgctggcaaaattcaataagaatagccgcccgttttaccttttctgccagcagatctaccgaaacagcttcattctctatttcttcagcgatcagctgcaattcattataggcagcttcatatgtcagttcctggctcatgtacagtatttttttcagtaatagttgcttccagcgatgcatcctgcaacagcaccgtgatatgacttcccggctggagggaggttgcatcgggaagaatgtgcccgtcctggtatacaatggcaaagccgcgtttcaggatactggcaggactcatcagtttgaacagggagtcgtaatgcgctacctgcccccttttgctttgaataaataacctgctgaacgaacggaaacgacctaccatattgctaaggtcattcagccggttggaaacaatgatccgcggtttggataacaccgcgttggatacagtcattagctcccggtggcggttcagcaatatcgacttcgaagtatgcagcaccacgttattacgcgcatgcaacgcttctttatgattggccagcagtgtgcgcgactggttaatgatggcattgttgagataagataatgcctggaaatgcgcggaaaacaactgctgcgaacggatgataatattctgttgcatattgaccaccgcttcttcaaacaaccggttgtgcgcaatgatcagctccgccgctttggtaggcgttttggtggcggtatgcgccatcatatccgtgatggtttcatttttctgatgccctatcccggtgatcacggggatagggaactttgccaccgccctgcccaggataaaagtatcgaagatcaggaagtcggtttgcgcaccgcccccacggataattaccacggcatcgtatggcaccccgcgctggtagatgtctatcagccgctgttgcaccagctccgcttttgtttccccctgtactacggtgaaatagttgtcgattttaaaggtatacccgaaatggttatgttccagcgtgtgccggaaatcctggtacccggcggagttgccggatgtaatcaccgccagccgctggatcacagcaggcaacggcaactggttgttgcgggtaatgtagcggtcgcccgacttacggatataatcggcgcattcagtggtaagccgcaacagggtttgttgcttctgctgctccagcaatcctaccgtaaaactggtatctatatccagcagcgtaatctgcaatccatgcacctggtggtatcctacagatacctttaccaatacatgaatatcattcttaaactgctgcccggtaacaatttcaaattcctttacccggatagcgccatttccccaggcaaccgccgaaactttggccacaataccacccgcatgttcttctttttccaccaggtcgaaataatgatatcccttttgctggtagtaagaatgattggtgatatctgccactacccaataagtttgctccgcaaacacctgttgaagcgcctgctggattttcccggtaagaacggataactttatggatggagaatcggtcatgctaataggtaaagataagtaaaacgtttattatgaaccctctcatggaataccgggggaaatgtatatattgctgtccattgaattatgaaaagaatgccggatcaaccaaaaccgtaacaaacacttaataacagacttattccgatttatatatttttgcgccatgagagaaaatgagcagataaaagggctttttgaaagggtctgctatgacaacagtatccaggcgtacaatgaattatacatagcattatgtgcccggctgatacacttttctgcatccattgtttcatcattccatctggcagaagaaattgtgtcggatgtatttctttcattgtggcaaaagcggaatgatttgtcgcacgtacaaaacccggtggtatacctgtatgtaagcactaaaaatctttccctgaacacgctccgccaacagaaaagacatcagcatcattcactggatgcattgaatacagacatgctggccattgcccccgatgcagagaacggaatggtatccgccgaagtatctcaaaaaatagaaagagccatccgcagcctgccgtcccgctgccagctgattttccgcttaataaaacaagaccgcctcagctaccgcgaagtagcagagctactgaatatttccactaagacggtagacgcacaactcaccatcgccgttaaaaaaatatcccaggccatccgcttcgacctgtccgacgaaaccgcccaaacctacctccggctggactcataattttttttttgatttcctttagggaactttcactgtttagtttgtccttcttatagatgcaggaacaaaattgcctcctacactaaaacaggcgcctttttgttcttcactgacactatggatcaggaaaaactttatgcgttgctggcccgcgaaatggccggcgaattaactgaaaaagaagctgctgcattggaacaattgctgcagcaatacccggatgccagctacatccgggaagtgtttgcgcaaaactgggcaccggcaggtaaagtatacacaccaatgcaggtgcagctgcagctggaaaaacaccagcaacgcctgcaaaacctgcccgacactacgccctatgaggaaacgcccgcagggggacgcagatggttgctgtacagcggcatcgcagcaggacttctcctgctcttcgccctgggcggatattggcggtacacacaaaaagcaaaactgccaccggctttatcacagctggtgaccgacaaacgcatgcgctcacaggtgctgttacccgatggtagcagggtatggctcaatgccggcagtaaactggactatccccaacaattcgccgcacatcagccacgggaagttaccctggaaggagaagcctttttcatggtaaccgccgatgcggaacgccccttccgcgttcatacaaaagcctttaatgtgagggtactcggtacttcctttaatgtaagggcctatccgcaggaagacagtgcagtagcatcgctcgtgcaaggctccgtggaagtggtgctgaatgatgcttccagccaggtagtatcgctgaagcccaacgaaaaattaacagtgccagtacacccggcaacagccgtaacaacagaaaacaccaccacagtaaatatccctgtcgtcgtatataaaacaaaactcaccacattaagagatagcatcattccggaaacggcctgggtacaaaataaactggcctttaaacatatgcagctcgacaaagtagtatatatgctggagcagtggtatggggtggaaatcaactttagtgacaaccgtaaaaaacaactctactttactggtgttttcgaatcagaaagcctggaagaagtattgaatgccctggaaacaaccctatcgttttcatggcataaagatgcagaaggcaaaatatggattgactaacatttctttcacctgtaaaaaaatcaaactgacagtctgaacaacgagtaattactaatttatcaaggaccgcttaaaaccgaaaaaaaacgggaaatgttcgcaccattccccgtgtaaatatcggttaacagctttgtattgggtaaactttccatcaacaaattaattaaccaacaaaacaaatgtatgaaaaaaagtacagtggacaattggcttccgcccggccggaggttgtataaactgttaatttttatgaagctttctatgctgcttgtcaccgttgcctgtttacacgtaagcgcaaaggtacattctcaatccaccataacagtgaagctcacgcaggtgcagttggataaagccctcaccctgctggagaagaacagccattacaggtttgtttataacgatgataatcttccgttaaaccataaaatatccatcgatgcaaaagattggtctatcgacaaagtattgaacgaaatcctcaacaatacctcccttcacttccggaaaatgtccgacaaactgatcgtgattgccccggaggcggtggtgagtaaagacaacctggtaaaaggacacgtagtgaatcctaccggcgaggtattgccaggcgtaagcgtaaggcttaaaaacacgtccataggcactgttacggatgtaaaaggcgactttgaattaaaggtacctgaaaatgccatcctcgtgcttacctacgtaggctttgatcagcaggaagtgtcactcagcggccgcgaaacccttaccatcaccatggaaccttcaaaaaattctatggaagaagtgattgtggtaggttatggtacgcagaaaaagctgaatgtaaccggcgccatcgaccagatctccggtaaacaactggctgcccgtcccattgccaatgtgatgcagggcttgcagggcctcagtcccgggctgaatatcagctaccccggcggccggcccggacaaacgcctactatcaacatcaggggtgtggccagtatcgcttcttctaacggtaatattgctccgcttatcgtgatcgatggtattgccgcagtaatggacgacctgttacgcatcaaccccgcagatatcgcgtccatctccgttctgcgcgatgccgcttctgccgccatttacggcgcacgcgcggcctacggcgttattctcatcaccaccaaacaaggtaccaccggcggcaaacaaaccgtcagctatagtaactacttcgccatgtcgcgccgcaccattatgccggacgctatcaccgatccctatatttactcacgcgtattggaaacagctaccgataatacgccgtgggactatgtaaattattcagacgagtattataaatgggcaaaagaaagatccgaaaacccttccctgcctgatacccgcgttgatccgagcgatcctaccaaatgggcgtacatgggcagcaacaactggaatgattacttcttcagtaaaaataatttttcccagtatcacgctatttccctcagcggaagcgcagaaacagcgaagaaattacccatcagctacctgctctctgccgactataccaaagaaaacggattgaataaactggcaaaagacgactggggacgttacggattacgtggaaagatcagcctcaaacctatcaaatggttacaggtagataataatatgaacatctaccagacaaaagccgacgcgccagcctataatattacggacgtatactacctgcaacccacccaggtagccgtaaatccggacggcacctgggccaacaccgccgcaggaaatttagctgccaaactggtagacggagggcgcaacacccaaacccgttttggtttccaggatatcatccgcggcgtggcttctttccttaacaatgaactcaccatcaccggcgacgccagcatcaaaagagaactctggaaataccacatcgaccagaaaaaatataagatcggctacggaccagacgatgtccgccaggaaggtggtaacggcgcagtgacggagaataacggaactatcagtcatgatgtaatagacctctttgccaattaccacaaaaccctcggtaaagtacacaacatcactttactggccggttataaccaggaaagttatgagtggcagctgatcaatgcatccaagcaaaacctgatctcttcttccctcccctacatcgcgcttaccagtggtgatccggcggtgggtacggaatattattcgtatgctatccgtagttttttcgggagaattaattacacttttaaagaccgctacatcatagaagcaaatggccggtacgatgggtcttcccgcttcccttccagcaaccgctggggaatgttcccttctgtatctgcggcctggatcgccagcgaagagagctttatgcggaatacgctgccagtaatttccaccctcaaattcaggggatcctacggaagtttgggtaatcagagcgtagcttattttggctatctccaaaccctgggcaccaaaaaatcagactacctgatcggtggcaatgctggtcaaactgtggttaccggcgcaccatcactgcaggtagatccggccaactacacctgggaaaaagtaaccaccaccaacgtgggtaccgacatgggctttgtgcagaataaattccaggccagcttcgactactttatccgtaacaccaccggcatgttggccgcagggcaggaattacccgccgtactgggtacccgcgctccaaaccaaaacgtggccgatttgtccacccgcggatgggaactgagcctcggctaccgcaacgactttaacgtggcttccaaaccactgggcttcggaataaaagttattttatcagatgataaaacaaaaatcacccgttttaagaacgaccagcaactgtttggctccaggtattgggaaggtcaaacctatggcgaaatatggggacttaccaacgatggctattttaaaaataaagatgagatcaataaactggatcaatctgccatcatcccctggggcgccctcgaaatcgtagaaggatggcctaagtacaaagacctggacggtaacggcaaaattgaacagggcatttctgtcaaagatcccaaagacctgaaagtgatcggtaataccagcccgcattaccgctttggcgtaaacctcgacatgaactggaatggcatcgatctttcggttttcctccagggcatcgggaaaatggactactacccgcatcactatttattctggggcccgtaccaacagccatacgccagcatttacccctggaacctcgactactaccgggctaccgccgacaacgaagctacccgcgcacagcatagcgaatcctatatcaaagcaggattggcagatgccaataccaattcgtacttcccggtgttacaatcgtggctcgcagataacaatgataaaaaagggctggatattccgcaatccaaatacatgctgaatgcagcatacctgcgtatcaagaatgtcaccctgggttacaccctgcctgcatcactcaccaggcgttatcacatcaatcgtttacgcatctacgtaacgggtgaaaacatctttgaattctcctccatcaaaaaatacctggatccggaatccattattgatggctatggatgggcatatccttaccagcgcaaatatgcagtaggattaaatcttgacctgtaaaaccggaacgttaaacattgtaacatgaaaaaatttacgagctatataattatcggggtaatggtgatcagcgcttcctgtaaaaaggatttcctcgatcgctatccgcaggatgctatttctcctgaactgttctttaaaaccgaggaagacctctccctctatgtgaacggacttcttaaccaggcaggcaccgatgaatacctcggggaccagaacagcgacaacgccgctactactgctgctgtggaaataaaaaatatcatgatcggttcacccagctctcaaaccattaccagcggctgggagtggaacaggctccgtgacgtgaattacttcctcgacaattacaacaaggccgctgttacccaggacatcaaagatcattatgccgggctggccaggtattaccgcgcccggttttactttaataaaatcgcccgctattctgatgttccctggtatggcaggacattgaatcccggcgatgctgacctgctcaaagcccgcgatccccgcaccatggtggtagacagtatgatggccgacctcgtgtttgccactacacatatccgcgccagcgtacctgccggcacacccggactgtgggccgctaaaatgctctacgcccgtattgccctgtttgaaggtacctaccgtaaatatcacccggaactgaacctcgcaggcaccgccgcacgcttcctcgacagcgcacgggtacaggcacaggatattatcaactccggcaactttaccatttacaacaccggtaaacccgaccaggattatgccgccctgttttccagccaggatctcctgcttaacaaggaagtaatcctcaccaatatttacgatttgaacaaaggacgtggcggcaatatcaacgggaacgttttcggggattatgaacaatccgtttcccgcgacctggtacaaacctacctgatgaaagatggtaaacgcttcaccgatatccctggttatgataagctaacctttgtagccgaattccagaaccgcgacccgcgtatgcgccaaacccttgcaggaccgggcttcgcccgcgtcagcgataccaggccgtatattcagcggctgaataaaaacttcaccggctaccaccagttgaagggatatattaacagcaacgacaatgtgattgccaatagcgtggactttcccgtgtaccgctacgccgaagccctgcttacccttgcagaagccaaagcggaactgaatacgctcacacaaaccgacctcgatcagtcggtaaacctgctgcgcgcccgcgctggtatgcctgcactgaacctggccgccagcaatgcagcccccgatcccgtacaggccgcaaaatacccggatgtaaccggcgccatgaaaggtgtgctgctggaaatacgccgcgaaaaaaggatcgagttcgccatggaaggttaccgctatgacgaccttatgagatggcatgccggtaaactgctggagaaaatcccggaaggcatgtacttccccggcttaggtaaatttgatcttaccggcgatggcgtggaagatattatcctgatagataaaggcacagatattcctgcagaagataaaaaagaaaagaattccctcggtatcacgctggtttactataaagccggcagcatcggggaaaacgtaaccgtatacctgaaaaatggcgttgcaggcggcacgctggcaacggaaaccaacctgcgcaagttcacggagcccaagtattactaccgcccggtaccctatacgcaggtagcgctgaatcttgcactgaaacagattttcgactggcaataaacatgaatatgaacagaagagatatcctcaaacacaccgggctcatggcagccggcaccctgctgggaccggccgcggtaaaggcggcggcaagcggcaaatgtacaccggtactcaccgtggcgcatataacggatgtgcatatacgtgaagacctcaacgcacccgcaagatttaaaaaatgcctggaggaaataaaaaccaaaaaggtggacttctttctcaatggcggcgactctatcttcgacgcctcctacgataccgtaaaaagggaaagggttacacaactctggcagatctgggatgaatgcatcagcactctgaaatcatatgatctctacagctgtatcggcaatcatgatacctggtggaaggcgccctccaaagacgacagcatgtatggcaaagactatgtagtaaagcggctcaacattccgcaccgctattacagcttcacccgcaaaggatggcacttcattatcctggatggcaacaatgaaaaaatatcactggacgaagaacagtaccagtggctggagcaggacctgcaaaagctgcctgccggaacgcccacgctgctgatgtcgcactacccgatccttggaattacccccatcctggtaggtggcggccactccgatcatcagcggttgaaagcgctctttttcaaacaccgcgataaagtaaaggtatgcctcagcgggcataatcatctttccgacaacgcagtgtacaatggcgtacgctattgctgcaatggcgccatgagcgggttttggtgggaaaaaggcgataaggaatctgccggcgaaggttattactttgaaacgcctcccggttacgctatcctgaaattatatgcagatggtgaagtggaaaatgaatatttcccacatacctgaccaggttaaataagtgtatgcctgtttacaatctttgtaaacaggcatatttttttagcggaactgcgccagctccccggcatcgaacacccattccggtgtcagcagttttcctgtaaatccggccgggtaccagggcgtggcgccacccggatttttcaatacatggatgttctgcgcaggcatgtaactctgcgccagcaggaaaattctttcaccggcggcattttccgccacatccattacaatcaccgcatgaccaggggaaccacctttaataaacacattcccaggcagtattttacgtgtatcctttaccggtagtagttccttgctgagtgataaggtaccagcccaggagaatacggtttcgaggtagttgctgaaacaggccggcccgctgcatgccgcagcctttcttactttcaccaggcggttttgttttaatacaaaccggtcgccttgcatccagctattgtaatccatcagcgtgccatcggtggcatgaaaagcaatctttcccaactgtttggtgtgatacaggtattccgcgtacaggcggatcacggcatccgcgcattgctgcaggtctttgttgccggtagaaatatccagtacggcatactgtgcctgttgattaccctttaaatgcccgttataaagatatactttgttatcctgcttcaggggcatggaccgcagccaggcgccaaaactgccggccggttgcggcacgcgtgtaaatcccgccggaagcggcagaccgcctacagacgcaggaggcattgctccatttgaaaacagcagattaaggatagttgccgctggtacggacaatgcgcttgccaacggccaggcatatacgaaagtggcgggtaaagtaaggatgactatcagtaatgtggtaaaactccgggcgctgatcataacaatgaatttcaggaaagatgccggtacctgatttttccataaaattattttctcagcgccggcgtgagtatccggtggatagtaggtgtttttaattctttcccgataaataccagtgtggaagatggagtggcagtaccccactctcctgccggttgtatgtgcaggtacttcccggtagattgtaccagcattttttcaggcgtgtcctttacccggatataccctttgatacggtatagctggtccgggtaagcattgaaatgaaaatccagtacaaataccagcatgttcagatcaaaggcttccggcgattcaaacaataccgtgttcactttatgcggatgcttcaccggcgcaacagccgaaacagcggcgcctaccggcttctccgggaattgcaattccttcagggcaacagacccatcttctgaagtggtgataaacgccagcgggttcatttgctccagctgttgggaaagataaatcagttgcggtagcgccagctgctttattttattgatgatgattacgtctgcacaggaaagttgtttaccggcttccggcacctgttgcaatctttcaaaaatattttccgcatccaccacacaaacggtgctcgcaagcgcgtaatgccgctgcacgtcgggcatgtggaacataccaatgatgttgcctgcatcggcaataccggtggtttcaataaatacatgatccggccgctcttctttttgcaggatgtttcccaacacctccagcagatcgttatccaatgagcagcaaatgcagccgctggtgagttcatacagctggtctattttttcggtgatcaggccggcgtctatattcacctttccaaactcattttcgatcacaatattattatgcccaatgaactgccgcaataaactgttcagcacagtggttttgcccgctccgaggaacccggtcaatatatacaccttgatacgctcatccctatccatatctctgcttataaaaaattaaaaaataaatacctaacacaatcaatgggaggcttaataactgtcccatatccagcaggcggccggcttcaaaagccacctggttttctttcataaattcgatcaggaagcgggcgctgaatacacccgtcagcagccagccaaacagtttaccaggctccgggcgattccggtacaaaaaccacagccatccaaaaatgagcagatatgccagcgcctcgtacagttgggcaggatgccgcggtatatcatctaccctggtaaataccacggcccatggcagcgtggccggcgtaccgataatttcggaattaaagaagttgccagtcctgataaacgcgcctgccagcggcactaccagcgccaggtgatccagcagccacataagcggcacccggaaacggtaactgaaaagtatggaagccaatacaatcccgatggccgcgccgtgactggccagtccctggtagcccgtaaaagtaaactggccacccgaaaaggtaaatggcaggatgatctcccaaagatgttcccggtagtatgcccagtcgtagaacaaacaatggccgaggcgcgcccccaccaacgtaccggtgatgatatataccagcagccggttcagcatttcgggcgactgccgttcccgccggaatacatacagcaatatcatatacgaggccacaaaagccagcataaagcccaaactgtagtaccgcagcgcaaaaccgccgatacggaaaatttcaggggaaacaccccagcgtaaaaagagcatcaggatcaggttcgttatgtcctgcaaacataataaaacaaatataacaaataaaataatttgcaacaatgttgcatatcaaaatacccatctcagcaaatctcgacttgaaattttacctttgcccacatgtcgctatttattacatcattgaattcgggaagcaacggaaactgttattacatcgggaacgacagtgaagccgtgctggtagacgcagggatttcgtgcagggaaaccgaaaaacggatggcccgcctgggacttaccatgagcaaggtaaaagcgatatttatttcacacgaacacatcgaccatatccggggcgtaactgtgctggcaaaaaagtaccgcctgccggtatatattaccaacatgacaatgatacatggcggcctcaccctggaagaacagctggtgatgtcgtttaacccttacgaaccggtacagattggtaccctgtcggtaaccgctttccctaaacatcacgacgcttccgagccccatagttttattgtagccggcaacgcggtaaccatcgggatctttaccgatatcggcgctccctgcgagcatgtgatccgccattttcaacaatgtcatgccgctttcctggaagcgaactacgacgaagagatgctggacaaaggcagatatccttattacctgaaaaagcgtatccggggcgggaaaggacatttatccaataaacaggccctggaaatatttactacctaccggccaccttttatgagtcatctcctgctggcccatctttccagggataataacagtcctgcgctggtacaggaactttttgaccagcacgctaacggcacgcagatcgtggtagcttcccgttttgaggaaacggccgtgtaccacatttccgtccgcaatacctgcgaagttctgccacagaatgattaaacgcttctacacttctttttttactttataaaagcactttaccgcttctcccttgccagtagcatcattccactgccggccggtactggtatgctttatggtggatacctggtacatctaaaaaaaattaccatggaaactatcacaccaactgccactaacgaggtattgaacgacctgattgccatcaacaacgatcgcattgcaggttatgaaaaagcgctgaaggaactggaagaaggtaatgccgatctgagacctctttttaccgatatgattgcggaaagtcaccagctcagaaatgcactcggtaatgaagtacaggccaacggcggaacaatggactccggtaccacagccagcggcaaactttatcgtgcctggatggatgtaaaagcagtattcaccggccatgaccgtaaaacagtgctctccaactgcgaagccggggaagacgctgcacaacgggcctataaagatgcgatagaacatgaaacgctgcccgcttacatcaaggaactcctgacacaacaaaaagcagagctgagacgctcgcacgaccagataaaagcattacgggaccaggctaagtaagacaactagtatatcatcaacctgcagcaggggacgtatccctgctgcttttttttgggaagaaaaataacggtgaatcattatcttgcaggcaaacaatgccgctatggatcatgtattgcccgcctggtatgaccggctcatgaaaaaataccccgtagtaacccgggcagagtggcagttgctggataacattgccaccgtaaagcacataaaaaaaggagacgtcttcctgagatacggcaaagtagcccgctactccgcctttgttatatccggcatgttcaaattcgctatcctggatgaagaaggaaatgagaagatcgtaaaattcggctttgcagatgattttctcgccaactgtgaaagctataatagaaaagcgccttccgctatcagcattattgccgtggaagacgccgtaattttgagaataaatatcaaaaagctgcagcccctgtacgacctgcacatgaacctgctgcatgtaaacctgcagctgtaccaggaactgctggaacagcagtccgaacaccagtacatcctttctttaaaaagtccgctgcagcgttaccggttcctgctggaacggcgccccgccatcatacaaaaagtatcactcaccaatattgcacggtacctgtatatcagccgggaagcgctgagcagggcacggttgttcctcctggaccggacccgtaatttttgtgactgagatcacggccgcccaatttttcccgtaatagttttgtatcaaaaaagatatgaaacaaagcatgatcttattgcacggacttttcggcggacttagtaactgggaaggcgttgttacacattttcagccgcattacgatatacacatcccacctcttccgatttacagtgcgcataccggcgaccagctgggatacctcgtcgattttcttgatcaatacatccgggaggccgggctccaaaacgtaatcctggtgggcaattcattaggagggcatgtagccatcctatacacacaccgctttcctgaacgggtagccaggttaatcctcacgggcagctccggtttgtatgaaaataccagcatgggtagttatcctaagcggggcaattatgcatatataaaagaacgggtggcctacactttttacgatcctgcagttgctaccgatgcattggtggcagaagtatttcaaactactactgatgcacagaaatgcatctgcattgtaaggatggcgaaatctgccaaccgtaattatgtagcggcgatactaccggaaattcctgtgcaaacattattgatctggggaacggaagataaaattactccgccggaagtagccctggaattcagacgttacctgccgcatgccaccctggtgatgatagacaggtgtggtcatgcgcccatgatggagcgaccggcggagtttaataaaatactgggaacgtttcttactaaaggttaatgcttacgtaataataatttgcggtaggccagccagcccaatgcacctgccagcaggaaaggccataactgtataaagaaaagcaggatgttgcggaaaatttcagcgccattgcgcagggccaccaacagctctgtgccaaagccggcgcggattacacggtccggattgatgaccacttgctcatcggttacctgtggctggaacaattgcaccgtgaaagtagaataagccacatcatcgaggattacgaggttatccatctgccggtcgatggcagcagcggctttctggtctttgtactccaccacatccagcgtggttcctttctttgcaggtgtaaccttactgagctgcgcttcctgtgtttcctggcgctcattcttcaacgcattggccaggtacttcagggtcatatcctggtctttcaccacgcggtgatcaataaaccctgcggtggcagtgagtgaatacactactgagtcgaggtgttccactggtaccttcagtgtgaggttggcagtgggcgtgtacagctgaacactcttcaccgagtcggtggaataaggcacgctgaaatgttgtacggattcattctgcaggttgctttccactacaattccgcccaggcgcgttaccagttgctccatacgggaggtagcctggaacacgtcactgacgcggcaccgcacatcggcggactttactcttttgcgggaagcggaattcaattttgtgatgtcgttggagaaagacgtagaatcagcagtagctgcatagtctctcatttctttgttcatacctccctggcaggcacacagagccagcaggggtatacccaggtaatagagtgaaaagcgcataacaggagaatttaacctttatacaacagacgcagaaaaggtaacctttcagaaatgttaaagtggttgtgacggattacatgataacctgatttagtatctttaggtaagatataaaataccatgcccgtacttcctcagaaatatcagaccaggaaagcagcaattactgctgactttattgctgcggtgaatgaacacatcgaccaggtgatggatggccgcatagaccagatgtatcatatcaaggattttgcgcgccagttgtatattcacccggtgcatctcagcaatactattaagttacacaccggtcatgcaccgtgctacttttttgaaatgagattaatggaagaagccaggaagatgctacagaatccatcgctcacggtgacggaaattgccaccaagctaacattcgacaactccaattttactaaatttttcaaacggtttgaaggcgttacgccgtcccaatatcggctgcagcatgcggctgcctcagaggtagcgttgcaggtaaatgggctttaagaagtaataattattcaggggcttgttatcgaacaggtcgccatcgtcaaaataaaacccgttagtgaactctgttttggagttgagttgtattttaccggtgttgtgctctactataaaatacacggggatgatcacatgatacttaccacttttcccggtaaatttattccatttaatatccagttcttccagcctgaaaaggcgtggtttcaggtttccggctacattggtggagcaatccagcttggtgatcacaccatgatccacttctgctttcaatgaaaaagcgaggctggtagcacctcccttcatgggcacgagggctgaatccataaaccggcttagctgctgataagtgtcgttgaaagaaggggtttgggctttggagctgataccggaaaaaagaatacctatgtggaggaaaatgatatagaaacagttaaatctcataatatcagtttttcatctggaataacgttcacgcctatcctgtttttactgcatagttaagttacgatttcttccggctaaaaagatcgcaggcgtagaaaaaattcaatataattgaaaggcacgaggttgcatatggcaggtaaatattatttaagagctgttgcctttctcccggcggagctgaaggagaaagacaacaacagagatgtttacacactggccggctgcggtattgccgccttcagctttttacggtgcaggtaatgcgcgatccctatctccaggcagggtatggcgaggatgagcaggaaagtgatcaatacacctttttgtaatcctttcaggaaatgatctacctggataagggcaatattgataaacaggcccccgttgatgatggcagtaatttttgtttccataagatccgcactgacgccctcttcgagtcctattttttccgagagcattttgcggatgtattttttcatggtgtaggcaatgcccgcacctttggtggtgcgcagcataaaggcagccagtttgccctgtacgccttctttggcggcttgctgctccagcgtagtgccgtatacgttatagatcagggtgccggcggtgtcaatcagctggttggtggtgagctttgatagatcagcggggctcccgtccggattgcggaacagggattgtatggctgcggatgcctgttcatcaaatactgccggtacatgctttgaatatacgccggcatgcatttttacatctttacgaagactattaaaaaagccccatttaaaagcaaagaaccctgccagcagcggcagcacaaaaaaccagcaataagcaataatgcggagcgctttattggaacgtggcaccagtataaatttccgcagtacaatcaccagtactacagcgataataaaggcagtgaggccggccaaaaaggctccccacataaattttccggggttggtaaattctccgatgaggttaaagtagttaacaacagatttcatggggttaatttttatcagaatttaatagtcttccctgtacggaccgactcgcgggcagctgccaggatgcgcaccaccattacattattggctggtgcatacaatccgtctgccggcatggttactttaccattcagcacgtctatcaggtagttgaacggatcctcatacactggtatatccgttgccgttatacggcgcgtgatggcgggcgaccgttcactattgcgttgaataagggtattcttatcggcggcaatgagatagcctttgtcgccatacacttccatatccttccggctgaagctccagttccacgacgcctggatggtacactgcgtatcgccatagtccaccaggatagtggcatcatcttccactttgggatacacctgtggtttaaagtgacgcgccaccgcggtaacggatacgggcaaacgatttttcatgagatgggtcatgaggttggcgccgtaacagccgaagtccatgagtgccccgccgccgttcagcaccgggtcggtgagccagtttaggaattccgggccgcagccaatttctttaggtccctggtggccgtcatttaccgtcacctttctcactttgccggcgtagctgctatcttccagcaactggaaggttttggctacggacggataccagctcgtttcataatcggtgagcagctgtaccttgtaccggcgggccagcgagtccatatacaccgcgtcggccacagtagtagccaacggtttttccaccataatatgaatatgccggggtgcggcggcctccaccacttcccggtgggccttgatggagccaaatgccagcactgcagcgggtttcaccgcatccagcattttaccgagatccgtataaaagatattttcaggaagatgatattgcctggccctcaatttagcgacggccgtatcaggctcatagatgccagcaatctggatgtcccctttgtcagggcgaccaagaataaaagccgcatgcccatgtgatacaccggcaacggctacacgcagtggctgggctatgatgcagccaaacacatgcatcagcaggaaagtaaaaataacagaacgcatccctaaatctaggaaatatgtgcagcttttaataatagaatagataaacggtcaatgaccatcaaaaattacaggctcactgctattttaatgactaccttttttaccggtataggcgtgcttaccttgatgttgggcatgtgcaggtccgtaggaaagaaaatggcaaacatgcccttttccaaccgggagaaaaacatcggatgctctgcaaacaactggtagtccgcagtttcatcatatgctttggaaggcgcctgttcacgcaggaagtcgtggccaatcagttcagaacctgacaccatatactggatatcgatgtacttcttatgcgcttccatttgctccgtggaagcgtctacggtatcatattcattgacaatagcgaagatattgcttccatcgatttcgtacttccccttttccaggccggccaggtctgtttgtgccaggtactcaaaagccttgataaatttaactcccaggcgatagtaaagatgggcattctgcagtgtatccagtatcatgttttgtaaaaaggtgttaataaggcggcaagatacttttttttctatataccaaaccttccggcgctcatctacttctttaacaggtgaggctgaacagctttctcccagatggcgtatccctttttattcatgtgcagcatatcattgagaaacagctcctcgcgcgacttccccgttttgtcgagcatcagcgaaaagatatcgacgtatacgatatgtttttctttggagatgtaatctttgatcagtgcattcgactgcttcactttctccacgtacttcacccgggaaggactgggtttcatagaaatatacaacagcggtgtttccggcagtttacttctgatagttgtatacagcactttaaatctttgcagcagggaatctgcggtggctttctcatccactatatcattttctcctacgtagatcactacctggcggggatgatagggaaagataatatcgttggcaaaataggtgatgtcgttggtaatggcgccgcccactcccctgttcagcactacatagctgctgaaattcctttccaggtcgtcccatttcctgatggaagaactgcccacaaacaggatcggatgttccggaggcgcatacatcttatcaaattccttgatggtattaacatccttcgcaaaacgcatgggtgattgggcaaacagggatccggttacgtggagcaatgtaaaactcaacaggaacaaatatcttttcataacgatttaatttttcagcgagctttaagataaacgaaaaatatttaatttagaacaaactattacatgaatacccatcctgtcaacttagccgtacgttttctgctggaaattttaatgctggtgatattgggttactggggctggcgcctggttaacggatggtggtcttatgtactggtggtggcgtttccgctcactgctgcagtgctgtggggcgtattccgcatccccaacgatccaaaggcagcgccggtagctattcccggtgtagcgcgactgctacttgaacttttcctgttcggattggcggcgtgggcattacactcattgggttatctgcgcgaaagcattgcactggcagtagtggtgattatacactacgccgtatcctgggacaggacctgggtgatgctgcaaaacaaaccctacaacgggtttgctggcaagaagatcatgggaataaaaccttagatataccaaacggtttcgggcgctacgcttatattcaccgctgcgccttttttcaggccggcatccgtggttttgatggtcaccacttcatttcccagtgccacttcggcttcaaagaaactgccatagtaggcgatatcacggatcttgccgggcacagcatctttttttgcacgaacaattctgaagtcctccgggcggataaagatgcttttaccattcagtgtaatgccgggcaatccgtccagcacagcggctttccccggggaaaggagattatattttccaaataacccggctacatattcattcaccggctggttatagatttgttgcggagatccctgctgtacaatttccccgtctttcatcaccagtatttcatctgcccagggcaggatatccatcggatcgtgggaaatcagcatcacggtgataccgagcttatcgcctatatcactgatcacttttttcaggatgcttttatggatcatgtccaggttggaatagggctcatccagcaaaaacagcctgggagaagaaatgaggagtcttgccatggcaatgcgttgcttttcaccacccgacaactgatctgtttttcttttgagcagatgtgaaatccggcagatgtcgtagatctctgcggcttcttcatcggtgagcttattggcataggacagaatttcttccacccggtaattatttctcagttcaaaatgctgggaaagataggccgtgccgggatgccctggaatcaatacttccagcgctcctttcacacgtttgccttcaaacatcaccgtaccggcatctgcctgggccatgccgcccacaattttcatcagggtgcttttaccggagccggtttcgcccgcgatcactattttctgaaatgcgtgttgtgtgaagctgacattctttaaaatataagcgccgtgcagttccttgctgatgtttgagacttcgagaaaattcattcgcgcaaattaataaaaatagcggagtttgtctttctcaggattacgctgattttgctgattagctggatttttacttttggatttataaaggattacgggagatacaagcgaatatatccgcttgtatctcccgtaaatattatta

SEQ ID NO: 6 - DNA, 506048 bp, Chitinophaga pinensis
  source 1..506048: mol_type = genomic DNA
tttacacaataacttctggtgcgtaaacacttacaacttccctttttttcaactgcaaattgtggataaaaccatccttaaagcctaaaatgaaaaagctgcctcatttatttatgagacagcttctttttgttttaaacgagaacgattaacttttacttaatagcatatatgcggtaaactatctattgccttttattttatcttttgacgatttagcggcgcaaaacgatcggggttttctgaaataatttcaggtagccattcacatattgtgattatgttagcattttagtaaaaaaggatgcttatctttattggtatgttacggacacttctttttgcggttatttttatgtcaggtatgagggtaaatgcacagatagactcctctttcggggctataaatggcatggaaccggctttcagacaccgtcaacaggtaggtgatactgccaatatccataagaaatggtttgttacaaagtatgccggcctttctaccggcttcataggatttaaaggaggtagcagttccttcctgtcggtacctttggcattgcaggttaaccgccagttaaccaataacctgtacgccttcggcggggtatcggtaacgccttacgttttccgttataacagcgtgccttatcagcctgcggttaacaagaaccagagctggatacaaacgaataactttgccgcctggtctgatgccaaaattggggtaatgtatattagcaacgacaaaacattctccatttccggtagcgttggcgtaagcagaggcagctacaatggtaattctcccttttattcccccatgtactctcctgtgcggggccatagccaatggtaattaagttatcgctggaatcgcgcgatgccctgactttatatcttatataatactgatagttcatttcttacaggaatatttttgtatgttcgttccctcaatattcctactatgaaatgtttgtttgctatacccgtattcatgttactgggtattcttgcctttgggcaaattaaaattgtgtcacaaagcccggttttgggagaagatgaatctgtcggtattcaaagggtattacttatgaacaatggtaatacattttatcttggcctgagtaagaagtcgttgacagtgagggtatacagtcctaaattcacggtaaaagccaccaaacaattacatccccaccttggtaagggcagcagttttaaagtcaaaggactgtatgatatgaatggagatgtggtagtgctggtgagcgctgtagataagcaccaggtagtgttacaacggctggtaattgacggtaaaaccggggcgttaaaagacgagggtacgattggggaactggaaaaagtttcctatttcaaactcgctggtatcgcatttgctgatgtgccggaaccggattttttttccgagaaaatgcctgaaggaaacgggtacgctgtaatagccatgaacagttttcagcccgacaggaataaacgtgtggttgttgctatctatggaccagacaataaagagctgagtcatgctttttataaatcacccgaagagaagtataagtatattgaatacctgggtatggcccctcttgagaagaataaactgggcgtattagcgtatggttataataccaggtcttcgggtggcaaggaatgtgaattgatatttggtacgctcaccacaggcgatagcttactggtaatagataaacttggcacttcgaaaaagcctgcttcttcttcggtagcaagatataatccggtatcaaaaagaatgatgctactggaagtagttgcaaaaaacgactattcagccacggtggtagacccctttggaaagacggcttcagccaggctaccggttggtaaaaacaaggatggtgccccacagaacctttttgtaaatgaggatggttcattctctgcggtatatgaaaagcttactgtctggaccgataaatattccactaagtattcctccggttatgatatggaagattataccgtgagcgtgctggcaaatgatggggaagaaatacaacattatagagtgccaagacgtcatttacgcgcagagatgttaaggactcctatgttttacaatgcatataacgccttcgaaatgtcgtataaacagccttctccgctggaagcatttaactacctgagtgcagggggtactaattacctgttcctgaatgatgatgcagataatattgaaagggtacaggcaggaaaagatccccgtaaagtaaaatcactggacgattgtgatgcgttttgctataaactgagtggtgataaggaaatccctgcagtggattatttttttgctaaaccatctgagaaaagggatcatgaccagggattgtttaaggcgtatgattataatgcggagagtaagacctatgtagttgtaaaagcggaacaacggggccgggatttgaactggaagttggtttggatgaagccataaataataaagaggtggccaaaagtaatggagaccacctctttatcgtttgcgtcaacagatcagcaacaacctgctctctccgggtttttccgttggagcacggtgaatacagggaggcacctggctttcaggatgatcaaccgccagcctccataggtgaccaagccctaagcttattggccgtgcatcaggcgtagcctggtaatgcagatcaaagaaatggtcgcttaagaatgattcaaaaccttccgctgctccatgatatagttttttgagttcatcacgtattgcgggaataagtaccttctttttgccttgtgaatttggtaatatttcactcgactcaccatagtaagtgcataaaaaggtatcggttggtataggagagcgatctacatgaaaagaataaacatcggttgggaaaaaagggaaggtatcatcccggtcgtagtagctgatcacattaaggatgggcgatgcgccgtgagctttcaatacctccaggtcatgtaaaagaatttcacgggcaagttgcccttgttcactcagctgaagttcatgaagttcctcttgttcaatggtcgtaatatttccgcttagcgctaccttttttacaatctcagaaaaatcacctgttagttgacggggccagcaaatcgcattcatttctccactgaatggcgtagcaacaaggtcctgaaaattcgtgacacggtgaatttgatgctcagcaggagataaatctgtcatgatagttaatataaagcagccggtcaagccagctttgatgaagataacaacaaaaagctaacctccagccatgtacaataggggtggaatttacaaaaaagaaagagcctgctcattgagcgggctttttatgtatgcccggtagcagtaagttttcgaaccaaaacaagcgtaataaccatccgccctggtgccttcgtctgacaggcaggagctttctgctaacaaacacaatgtcaagatattatttacaaagtttacacttctatttacaatacagattccttaggctgaagtaaatcaaagtatttttgttgcaccaacttgaaaggatacgaaaaataaaaaggaatgccttaaacggatctgatttatcagaagatagatttatgttaattaaacctaaaaaatatgaaaaaagctatttatgcgctgatcttaccgctggtggtggtaggcggactagtatttgccaatcgcgaaatcaaaaatgaaaaatcagccccaaagccactttctgctgctgaaatgaaagccgaattgaaaaaatgggaagctacccccgagggtataaggttcaaaaaatggaaagcgtctcctgaaggtcaaaaagtgcttgccggtgcggctaaaataaagaagcaaacaagtgcttctaccaatatggaagctgttgtaacctctctttctcttccgccaggctcacgattaggtttcggagtgatggtcaggattaatggtgacgattatattcttagttttgggctggaaaacgctaatgaatttcagcaaatgcatagcctgaaggttaacgacaaaataattataagaagccattttgtatcgtacgcgcccaagtattcatatccaattgtatcgggcgactatgtagaacaagatggtagaataatttataaacgtgcccctcgcaaaggtggctgctgagtaaagttatgatggaaagatctttacggaatttaaaggtaagagaggtattcttcagcatcccaaaggaacaaaactgattcgaacaaaaaaggcctcaagtctaatgacttaaagccttttttaatttcgtgcccagaactggattcgaaccagcacatccttgcgaacgctgcgacctgaacacagtgcgtctaccaatttcgccatctgggcatcgcttgtccccgtaaaagggattgcaaaagtaaacacttttttaaactaaccaaattttttttcaggacataaaaaaacggcgcctataacaggcgccgttcgtcaatatataaagatttataccgctacattaaactcacgcaaggtgtcgttcaggctggtcttcaggtctgtagaggctttgcgctgaccaatgatcagtgcgcaggatacctggtattcgccggcagggaatttcttggtgtaagttcccggaattaccacgctgcgggcaggtacacggcctttgtattctatcggctcgctgccgcttacatcaatgatcttggtagattgcgtcagcaccacattggcgcccaataccgcttctttttctacaataacgccttctaccacaatgcaacgggagccgataaagcaaccatcttcaatgattacagggctggcctgtaacggttccagtacgccgccaataccaacgccaccgctcaggtgcacgtgtttgccgatttgtgcgcaggagcctactgttgcccaggtatctaccatcgttccttcatctacaaaagcgccgatgttaacataggaaggcatcaggatacagcccttggcaatgaatgcgccataacgcgctactgcatggggaactactcttacgccgagttctttatagttcgactttaatctcattttatcatagaactcaaacggaggcacctccattgtttccattggctgaatggagaaatacagtaaaatagcctgtttcacccactcattcacctgccagccgtttgctgttggcgtcgcaactctcagatgtcctttgtctaccgcttctatcaccgccttaactgcatctgtgtactgtgtctcctgtaagaggctgcgatcagcccaggcagccagtatttgttgttgtaaatccatttttcttattttcctgcaaacataatacgtagaaaataaaattacgaattacaaagaggtatttccggaaatcttatcagatatacgtaattcgccatccgtaatccgtaattttgccttttgtggaagaaagaactttatgaaaataggattcgacgctaaacgtgcattccagaacgacactggtcttgggaattatagtcgtaccctgatatcatctctggtaaaggattttccggaagatgaatattacctgtttgcccccaggcaaacaggtatgtacgatctcagtgccctgccggatcttaaagtagtggtgccggaaaacccgttgtaccgctggtttaagtcggcctggcgcagccgttttgtggtaaaggacctgttgcgttaccagatcggtatttaccacggcctcagtcatgaactgccttttggtattcataaaagcggtatcaggtcggtagttaccatgcatgatcttatttttgaaagataccccgagcagtataatcctattgatgtcatcacttatcgccgtaaggcccgttacgcctgccagcaggcaaacagggtagtggccatcagcgagcagacaaagcaggacctgatcacttactaccacacgccggcaagtaaaattgatgtggtataccaaagctgcgatccctcttttgccatcacataccctgatgatgatatcgccgcaatgggcgccaggtaccgtttgccgtcccagtatttcctgtacgtggggtcaattattgaacggaaaaacctgttaggcatcgtaacggccatgaatacactaaaaggaacactggattttccattggtggtattgggcaatggcagtggctataaaaagaaagtaaaagcatacctggaagccaacgggctcacacaacaggtgattttcctcaatgaacaggtacggcttaaaaacagtgagttgcccctcctgtaccagggcgcggtagcgcttatctatccgtctttctttgaaggattcggcattcccatactggaagccctctggagccgtacaccggtaattacctcccacgggtcctgttttgcagaaacagcgggagatgcagccctgtacgtagatccacgggagcctggctccatagctgacgcgatgaggcaaatcatgggaaatccttccctggtaaggcaaatgcaggaaaaaggatggcagcatgcacagcgttttaccccggaaaagtgcgctgccgccatgatgaaagtatataaacaattaaataaggaaatataaaatgtttgaagatgatatcagtgcagccatgccggtgctgcgtaccggcggacttatcctttatcctacagacaccatctggggtatcggctgcgatgccaccgatgaaaaggccgtgcagaaaatttataccctgaaaaaaaggagcgaaagcaaaagcctggtagtattgctggccgatgtgaaagacctgctgcattatgtggcaaatccacgccccgatatggccgacatcattgccggctttacccgccctaccactgttatttatgaaggcgcactcggcctggcccccaacgtgatcagcgaagatggtagcatcgccatccgcattgtaaaagatcctttttgccgccacctgatcaaaagattgcgcaaaccactggtgtctacctccgccaatgtcagcggggaaccctcgccggccagcttccgcgacgtgtccgccagcatccggagtggcgtggattatgtggtgaactaccggcaaaacgatgaaacccccagcgccgcatccaggataatcaggataaacaaagatggttcaatcgtgataatccgggattaaaatcgtttatttattacatttgcgccctggtttcagagaaaggaataaaaattaacaggaatatttaaatatgatcagcagcaagccgttggacataccctgctccctgcaggaaagaaaagtgctggaaaagatagcattggccgcccaggaactgggcgttcccgcctatctgatcgggggctttgtgcgggataaactgttgggaaggaaaacaaaagatatggacattgtttgcgttggcgatggcatcgcactcgcacacaaagtcgcagcaaatttaggtgacaacattcccgttaacttcttcaaaacctatggtaccgcccaggttaaactgaatgacctggaaattgaattcgttggcgcccgcaaagaaagctaccgcgaagaatcccgcaaccccgaagtgtctgccggaaccctgcaggatgaccagaaccgccgcgatttcaccatcaacgcaatggccatcagcctccgggatattgactatggctccctgctcgacccattcgacggcctcgtggacctcgataagaaaatcatccggacgcccctggcgcccgctcaaactttcagcgatgatcccctgcgcatgatgcgtggcatccggtttgcttcccagctgcagtttaccatcgaagaaagcacctttaccgccatacaggaaaatgctgaacggatcaggatcatttcccaggaaaggatctccgatgagttcaataaaataatgctctcaacaaaaccctcggtaggactggacctcttatatcaatccggcctgctcaaaattattttcccccaaatgatagatatggtgggagtagagatgtacgagggaaaagggcacaaagataatttttatcataccttgcaggtagtagacaatatatcggaaaatacacgggatctttggcttcggtgggccgcattgctacacgatatcgggaaacccgccaccaaaaaatttgaacccggtcatggctggacttttcacggtcacgatgcggtaggtggtaaaatggttccccgtatcttcagcaggatgaaactgccgatgagcgaaaaaatgagattggtaaagaaattggtagaactacacctgcgtcccatcagtctcacaaaagagaacataacagactcggctatccggagattactcttcgatgccggagacgatatagaaggactgatgatgctgtgcgaagcggatattacctcaaaaaataaaaccaaggttaagcgctacctcgaaaattttgaattggtccgcagacgcttaaaagaagtggaagagagcgaccggatccgcaactggcaacctcctataaccggggagatgattatggaaacatttgggctgaaacctggcaggatcgtaggcgatctgaaaagcgccatcagggaagctatcctggatggcgaaatcccaaatacttacgaggcagcatacgcttttttattggaaaaagccggcgcattgaatctaagcccggttaaataaaattggtaattttacaataccataataaatacactagcattcaggatccaccgctcattgcggagtgtttaatcattaaataacttataacctttttgtcatgccggttttgaaattcagagtttactgggaagaagatgaaagtgtctacagggacattgccattaagccgaatcagacgtttttattatttcaccaagcaattttgcaggcattcgaatttgattcaaaacacaaagccacctttttccgcagcaatgataactggcaacgtggccgggaaatcatcctggaagcagataatcaaccccgtaaagcagaacccctgctcatggcggacaccatgattgctgccgcagtgaaagatcctaatcagaaatttatctatctctacgatttcgccaaaaactggtcgttcctcgtagaactcatcggcgtttccaaagatgaaaacagcaaaatggtttaccctgcctgcgttcgcaaagaaggcctggcccccagtcaatatggcaccaaaggcctggtaggtgataaactcgtggaaatggaagaaaaatatgacctcaataaagaaggtatggacgccgacggcttcggcgaagaaggggaagaaagcgacgccttaggcggcgatagcacagaagaatttggcggagaagaagaaaataacttttaaatagaactgtcagtcattttagggatctgtttattttttgcagagattacccgtttcatccacttagttgaaatggcccgtctcccggaaaaaataaacagatccctaaatatttagcgcaatacttatgcaaaaaaccgtcatcattatcgcaggtcccaccgcttctggcaaaacagcgttgtctgttcaaatggcacaactgtttaatacagcagtgatctctgcagattccaggcaatgctaccgcgaaatcagcatcggtacagcaaagccctccgcggaagagctgtcggcggttccccactactttatcaattcccacagcatccgggaagacgtaaacgcaggcgtttatgagaaactggccctgggctacgcccgcgaaatctttgagaaaaacgacgtagccataatgtgcggcggcaccggtctttatatcagggccttcgcggaaggaatcgacgatatgcctgtcattgccccgggcatccgcactcacctcaatgaacagtatgcacaacacggcctcgcctggctgcagcaacaattgcaggaacgcgatcccggcttctatgccgccgccgaaacccagaacccgcaacgcctcatccgcgcgctggaagtgctcgacgccaccggccaatctatcacctccttccgcagcgctacccggtccccccgcgatttccgggtaattaaaataggcatcaccctgcccaaagaacaactccaccacaatatccaccaccgcgtagatacaatggtacacgccggcctggtggaagaagtccgctccgttttaccttaccgcgaacacaatgccctccgcaccgtaggataccaggaaatattcagcttcctcgacggccacatctccctcgatcaggccatcgacgatgttaaaacacatacccgccaatacgcaaaacggcaactcacctggttcaggaaggacccggcattcacctggtttgatccgcgcaataccgcagatatcatgaactacgtgcagcaacaaggctagtacgcatgctccgcgcaggattttgccaccagttgtaacgccgcggtatacatctcccggaaaataattacggacaaccactgtactgaaaccgaacatttgcgataaatataaaatatataaatctcttgtatttaaaagcctggtaacatggcattttcttggcggcaccgtgtctgcacagctcacgaaaacagttgcttatgtttaaaaattacctgaaaacggcctggcgccacctgctgaaaaacaggcgttttacgatcctcaatctcattggcctgtctaccggtctcgcctgtacgttgctgatttgtttgtgggtatacgatgaactcagcattgatcacttccataaaaacgaccaccaccttttccaggtaatggaaaatcagccacacgaaaaaggcattaccacctccaacggaacacccgcactgctggcggatgcgttgaaagcaaatatgcctgaagtggaaaatgctaccgtgagcacaccgccatcctggttccctaaaatagcgctgaccaccggcaacaaaagcacgaaatccgccggcatatttgcaggtcaggattatctccaggtattctcctatccattgctgcagggaaacagccggcaggtactacaggacaaaaacagcatcgtcatctcttcaaagcttgcacaaacactgtttggtacaaccgatgcactgggtaaaaccatcacctggcaggtagaccggttcaaaaaagtcagcactgtttcaggcgtgttagatgagctccccaccaatacttccactcaattcgattgcctgctgccattcgatgcattccgggaaatcatgaacatcacggcgctggacccgcagggaccgttcaatacctttcttgttatgaaagaaggcgccgatatccccgcgtttaatgcaaagctgagcagcttcatgactggtcttaccaagggtagcactacaccccgtaacctgttcctgcagcgctacagcgatcattacctgcatggcaattatgaaaacggtgtggctgccggtggcaggattagctacgtgaaattattctccctcatcgcactttttatcctggtaattgcctgcattaactttgtaaacctctccaccgcacaggcttccggcagaatgaaagagatggggatccgcaaaacaataggcgccaaccgcctggcgctggtactgcaatacctcggtgaatccatgctgatgactattctcgcgctgggcatcgcattactactggtggcactgctgctgccggaattcaatcgtatcaccggcaaagcattgtctttctcgctaagtggcccaatggtgggtatcattatcggtgtcgcgctgctgacgggcatcctggcgggtggctacccggcgttgtatttgtccggatttaatcctctgcctgtgctaaaaggaaaagtgccgggatcaccggggcaattgatggcacgcaaaggcctggtggtattccagtttacactctcagttttatttatggtgggcgtaattacagtataccggcaaatagcttatgtgcaggataaaaatcctggttacgacaaagacaacgtggtatacttcgatgtagaaggaaaagtgccggaacatatacctgaattcctgtcagcgttgaaaagaataccaggcgtggtgaatgcctctgctatggtagggaatgtgctgggcgcgccttccacagggtgcacctggaagggcaggggcaccacggaaactattatgtgccgtccgtttatggtgaactatgatatgatagaaaccttgggcatcgaaatggcagctggaaggtccttttcccgcgactacggtgcagatgattccaggatcatttttaatgaagctgctatcaaggcaatgggaattgataatcctgtaggcaaagtgatagaatttaacgggatgaaaacggagatagcaggcgtagtgaagaactttcattttcaatctatgcacgaagttatcagcccgttgtttttccggctggattctctgaacagcacggtaatggtaaaagtaaaagccgggcaaacaaaagcagtgttggatgcactggctgccttctaccagcactataaccccgggtttgcgttcgattataagtttctcgatgaagattaccaggcgcaatatacagcggagaaaagagtggctgccttatcaaaatattttactgcactggctatcctgatatcctgtcttggcctgtttggactggccacttttaccgccgaaagcaggcgtaaggaaatcagcatccgcaaagtattgggcgctaccgctacccatgtaatgatgatgttgtcgggggaattcctgcggtccgtactaattgccgtgctgattggtttgccgctggcatggtattgcatggaccggtggttgcatagctttgcttatcacatcgaggtgggagccggcgtgtcgctgctggtagggattacgattgttggaatcactttactcacagtgagcttccaggcgatccgggcagcgttggaaaacccggtgaagaatctgaaggcggagtaatagacgatacataaaaaaaagccgtggtgaattacaccacggctttttttatgtatcgtaaaatgaggttgcttaaaatttaaatcctactgtcagtacaatgttgcttctggtaaaatccagtgttgccgccgcaggactcagctgtgcgtcgtacaccgtataaggctggtacctgtctttgccctgggtgtagctgtaggtagcatctgcataaagacctttattgcggaagccaataccaccgctgtacactttccgggaagcgtttacgcctgcgttgtatttatcatcgctgtatggattgccataggaagcaaaacccgcccttaccgcgtatatcgccataaatttaacctcggcgcctacacgaatattggaagtagatttatacaccgcgctgatgttatcgttcaggtttttttccccggccctgtcgtcactcatcctgaatttaccggaaggggtattcacgaattcgtaatcagctgtaataaagccctgggggctttgtggttcctgcaggttaccaaaaaagtaagatgcgcccgctgctgcgcgtaaaggcgcagtatagttgtagtcgtattctacaggataaccttctgtttgatcaaaggaagtagaaccctgttcaccacgaccatcttctatatctgagtacagttccgaactgtagctgtcatgaagggaataccaggtaggggtagcgaaagtaccacccagtctgaaatgatcggacactttatacaggataccaattttaccgccaacgcctaagccggtacgtttcaggtccttgtaataatcgaagtagccaaagtcgttgcctttgttactgctggcgtcatcttctgaccaggcgagtgattctttataattaatgctcggcaggtttaagctggcgccgatatacaggcgatcgccgtagttaccgccgatagcaaaagtgtattcattcaaaccaccttctgttttcagggtacctctttgctggatgccttctgtaagaccgcctatttgcctggaaggagaggccagtgtcataggctctttgttaccgccggtaggctggtaatcagccagtaacccggtactgaatcccagatctgtgcccagtgcctgtgtagaggtactgccatcgaatatatcatctacaaaacgatcggaataagaagacaaggtattgtgacctgcaatggcaatttcgttgttgtaattggccagtcgttccatacccagtgaaaaggtaatgttgttccaggtactgctgccgctattcttattggtagccataatgagcccgatggatggcaactggaaattgctgcggtttcctttattatcaagctggctgttgcccaggtaattggaggtattttgagagatgcctacgccacctgaaatatgaaattcgccggtcttaaaaatggcaatacctgccgggttaatatgagcagatgaataatcgcctccaaggcccacacctgcaccgcccagcgcctgggtcctggctgtaccgtgaggctgcaggggggagtaaagtaatgcgtcgttggaactctggcccatggctgttacagatataaacaagccacctaaaagaggataaagtcttttaatcataatctgtattcttaaaatgagatttgcttgcaggttaatttaacggttactaacgcatgccgcgataagtataacgtgctgaactggcaaaacgtgtgcgagataaaaaataagcgtaggtttttaggctacgcttatcttgtaaatgattttatttattaacggcctcctctggatggacggctgtagccaccaccaccgccgccaccggaattaccaccacctacgcgaccaccgccggaactaggaggagtgtaacttggagccggagtaggagcaggtctgctgtactctgttctttgcggacgggaataaccgccgccattgttgctgctgccgctgttgttctggtaagaaggcctggttacaggtctttcagaactggactgctggaatacacggcgtggtctttcaccattggatgtaccgccattggcaggctggaaagtaccggttctggaaggacgggtgtaaccgccgccgcctgtgccgccactgttggtataatctgccctgcgaactctttcgttaccgcctcttacggaaccataggagttggaaggacgtgtggtataatgtccgtaataaccgccaccaccgtagtaaccaccgtggccatagtagccgccgtagtatgggtagtagtaagaaggccagtagctgcctacgtatggataaccccatccgccatagaagccggtgctccaggggctgtagtaaccacccattccccagccgaatccaagacccaaaccaaaggaaggaccataaaagctgctgtatgggctgtaacctaaaccaaagccgctaccgtatcccataccaaagccactgctcatgtaaaggttggaggctgcattgtaaccatcccagtaatcaccggaatagttgctgccactgccaaatctgttcaggcgacgttgatagtcaccctggtcatcgtcctggtaagttacataggtaccgccatcatcctgcgttccttcaacatagttggcatcgttttcatcctggcggctgttgccgttcgaaccgttgctggaggcataggtacgctgctgctgacgcggagaatagtatacatcatccggagtctgagccgttttataggtactggaacacgctcccagtgcgagcgatgcggccagtccaatgtataatataggcttcatttgaaatatgttttaagcgtgattcgtgtagtaaatttacttcttttaaacggaattaacaggaagaaagttacaataacacagactatgttatattattttatgataagtgtttgcaacgttatgtttttcatctatgtttgtggaattttcttcttaatataaatggacaaaaactaagccaatccagcctttggcacccggcggatgggtttaattttgtctcgacaaattgaaccggaactagcttaaaaataacggtatataaataaggtaaaatttttatgagtaaagagataacggcccgctcggaagactattcaaagtggtataacgacctggtattgaaaggcggactggcagattattctgcagtaaaaggatgtatggtcatcaaaccatacggatttgctttgtgggaagccatgcgcgacgtactggaccgcaaattcaaagaaaccggtcaccagaatgcctatttcccgctgttcatccccaaaagctttttaagtaaagaagctgcgcacgtggaaggattcgccaaagaatgcgccgtggtaacccactaccgcctcaaaaacgatcccaacggcggcggcgtaatcgtagatcccgatgccaaactggcggaagaactgatcgttcgccccacttctgaaactattatctggaatacttataaagactggatacagtcgtaccgcgacttacccctcctgatcaaccagtgggcaaacgttgtgcgctgggaaatgcgtacccgcctgtttctccgtaccacggagttcctctggcaggaaggccataccgcccacgccactgcacaggaagccatcgaggaaacagaacagatgctgaatatctatgctgatttcgcagaaaactatatggccgtgcctgttgtgcgcggactgaaatcccccagcgaaagatttgcaggcgccgtggaaacctactgcgtggaagccatgatgcaggatggtaaagccttacaggccggtacctctcacttcctgggacaaaattttgccaaagcattcgacgtacagttctctaataaagaaaataaactggaacatgtgtgggccacctcctggggcgtgtctacccgcctgatcggcgcactcatcatggtgcacagcgatgatgaaggccttgtaatgccgccaaaaattgcacctgtacaggtagtgattgtgcccatttacaaaggacctgatcagaaagcaggactcgatgaaaaagtaaatgtcatcgttaaggaactgagaagcgccggtatcagcgtgaaatacgatgattcggataacaaccgcccgggctggaagtttgccgaatacgaaatgaaaggcgtaccggttcgtatagccattggcgcgagagatctcgaaaacaatgtggccgaagtaacccgccgcgacaccagggaaaaaatgagcttgtcgctcgatggtttaccaacccgcatcacggaattgctcgacgaaatacaactcaacctgttcaacaaagcaaaagcttaccgcgatagtcatatcacccgtgtagatacttttgaagaatttgagaaagtgctggacgaaaaaggcggcttcgtatctgctcactgggatggtaccgccgaaacagaagaacagatcaaagatcgcacaaaagctacgatacgctgtattccgctcaacaacccgcaggaagccggcaagtgtatcctgaccgggaagccatctaaagaaagggtgcttttcgcaagagcgtactaggaaagaagtttcatattaagtattacggggccggatttttgcgggtgttttccggaaaaatccgtaactcgtaatacttacaggtaatactcctgcaataaaccattaaactccgatgcccttgagccgttttataatgttatgggggttggtcttcttttgcactgttacaacaaccctcgcgcaggggctgatgatccgtaactataatgtaaaggacggactggccaacgctactgtttatgctgctacgcaggataaagacggtttcatatggtttgcaactcctaccggcgtcagtaaatttgatggtaaaagattccgcaactacgccaaaaaagacggtctcacagacaacgaggtagtgaaactcgccgccgactccaggggaagggtatggtttttcaccctcaacggaaaaccttcgttctataagaaatcagtgattcataacgaagaaaatgattcctccctcatttttaacagccgtagtcactatatgcagtatgcatttgaaggcaaaggcggttatatctggttcctcaacagcaacaacaggattgttcaatacaacggtaaagaaataatctatgataaactgggcgcctcgggatcagacctgtacttcctgatgcggaacgacagtatcttccacccgctgcaggcctcctttcacctcgaaagcctgcgcgaccccagtaattccaagcaagagatttataacgcatcgccgtacccgctggatgattccgcgtttcacaaccgtataaacggaagcgccattgtaattatccggaacacgctttactcctacaccgcaaaggatgccgtgtgtttttttaacggcgcagaatggggtattaaagatgatatcagccacatatgtattgataacgataacctgtggattggcacccagcgcgccttgtattacctgaaagattattttaaaggagaacggcagatcacccggctgctggataatcacttcattacctccctgctgaaggatagggacggcaacatctggatcaccacttttggagacggcgtgtataacatcccctacaaaaacttttacttcagctatctcgataataccaacggactttattcacattccattttcagcatcagcaaagataagaaaagcgacctgctgctgatcgggcagaatgccggcgttctcaatacaatggatgcggaaaacagtatccggcaatacacagtggataccacttccggccgtaacagcgtactttccattaccccgtataccaacgataatgtactcattggcaccgataacggcttgtacaagtttaataccctgtcccggaaaacaacactgttaaaatccgtgagaatgctgaaagatgtggatgtgtcgccttccgggaagataaggattgctgcaaaaaaccaggtagtagcactggatgattatgccatcagcgacctcgatatgctggttacttcgctggcaagcatcaacgactccgcttattacgttggaaccaacgcaggcctgtttttttgtacagacggcaggcggcaactgttgccagccggtgcagataccctgcggaaggtaagtatcaaggatcttaaatggattgatggctccctctggattggtaccagcgaccaggggatttacgtgatgcaaaatgataacgtcatcaaacacctgtccaccgccaacaacctggccagcgatatctgtcagcagctttactacgatggcgtgggccggctgtatgtggccaccaaccgcggagtgtccgtgattgatgtaaaaacgcagacgattacacgtaatatcacctccagcgacggcctgatgtcggacgatatccgcggcgtatatgccgataatgataccctcttcattgctacctccaatggcctgtgttcctttaatgcggatcatatcccggtggatacggtgccgccggtgatttacctgaataatatccgctatggcgacagcaccttcctcgcctccaatagctttgtacacctgtatcagcgcaaagcctcatttgaagcggaattcggtaccatcgtttttgacctgccggagctggtggaataccagtataatttttccggagataccaccagcggctgggtaaccaccatgtctaacatcattccgttccccgacctgcagccagggaattacacccttatgataagggcaagaaaatataagagcgactggtcaaagccggtgagcatagatgtgaacatactacccaggtggtaccagcaatggtgggcaagaggcatcctcctgctggctggtttgctggtggtgctgatcggtttacggtatatcatcaggcggattaaacaggcggaaaagcgtaaaacagagtacaaccggcgcattgcggagttggaagccaaggcgctgacgaaccagatgaacccacattttatttttaattcgctgaactccgttcaacaccttatattggagaaggaagagaaacaagcgctgaatttcctggcagactttgctacgctcatgaggcagatgctcaacaactccaggaaatcgtatatatcactggaagaagaaatcgctttcctgacccgttacctggagttggaaaagatccggtttgcacattcctttacctatcactttatcatggaggatgctttgaaggagtataccatctacatcccacccatgattattcagccgatagtggaaaatgccattaaacacggattggcgcccaaaaatatcagcggttacctggaaatccgcctggaaatggtggacgacctgttatattgttcggtagatgatgacggaataggttgggataagtcaaatagcattaaaagttcaaggctcattaaacacgagtctactgcacttagcgtgattaaagagcggttgcagattataaaatcttttaatggaagtgttggaaagttagaaattattgataaatttaaatctggtttcggcaataaggaaggtaccttagttgaaatactgattcccattgttaagatgttatgagtaatataaaagctgccattgtagacgatgaagtccgcaacattcatattttacgcaatatactcgagaactactgcaaagatgtgacagttgtcggtgaggcgcagaatatcaatgaggcggcagaaatgataaaaaataaccccattgatgttctgtttcttgacattgagatgccaccacacaatggatttcagctactggaaatgtttccggtactgaattttgaagttatttttatcaccgctttccaggaatatgcactgcaggcaattaaatttgctgcgctggattacctgttgaaaccaatcaaggtcagtgaagtggaagatgcacttgaaaaagtgaagaaaagcaagaaggggcgactcaacgagctggcatccatactgaaagactacgtaaagaacaacgataacgccttctcaaagatcgttataccggtgaacgacgggtataatgtaatcgatctgaaggatattatttattgtgaagcctttgacagctatactaaaattcagctgatcaacaacgtatctcacctgatctccaaatcattgaaggaatatgaggaaatgctgtccgataaaggtttttaccgggtgcataagtccttcctcattaatattcatcacatcgtgaaaatcatcaaagggctgggaacagccgtggtgatgagcgatcagaagaatattcctatctcttcccgtaaaaaggacgagttctttacccagctgaaaggggtaattaatctctgatattattaatttactttaattattaaagccggtgagccatcgcttaaccggcttttttatgcgttgcctaagccaattctcctgtttacggattaccccgccaacttatcagatacttattttattttcctaataggttttcatagaatgactgattgcacggtctgcttttccaggcgaggcgtgtatgacttaaaaagaaaaagtcccgctccggcttgccggaaacgggactttttcttaagacctaaaacccaattactttaaggggatcagaggttttcggcctcagtgccggtagcaatattatagtaataaatatttccgcctctttcaggatagaaacctatcagcttgaggttcttttgcttttccactatctggctgagttcatccacggaggtgacctgcgtgttgccggctttcaggatcacaaagcccggggccatagtggtctgttttttcaggataccgttgccgatatcgtttacaattaccccaccattcacacccaaacgggcggcctggtctttatcaagttcggagaggtctgcacccaaacgatccagggcagttacctttaccaggtctgtattgcctttcaggttcttcatcaccacattgttcacggtaacttctttaccgtcacgcagatagcttaaactgattttatcgcctggtttgtagcgtgccacctgttcgctcaactgcgaagtggtaggaatttttacgccattcacagcggtgatcacatcaccggtacggaggcctgcggccgcagcagagctgttgggcaatacatctgttacctgtacgccgtttacatcccttttaataccggcatcctttaactgctcatcgctcatattggcaatgagagaggaaggcgcatatcttacgccaaggtacgcccgctgtacattaccatatttcaggatatcgttcaccacttttttgatgaggtttaccgggatagcgtaagagtagccggcataagagcctgttggagaggcaatcgcagagttgatacctaccagttcgccggcggtatttaccaatgcgccaccactattaccctggttcacagcagcatctgtttgaataaaggattcaatagcgctgttcactttgccaccgcttctgttgataccgatagagcgtgatttggcgcttacaatacccgcagtcaccgtagcatccaggttcagcggataacctaccgccagtacccattgtcctatttctacattgtcggagttgccatacagcagataaggaaggtctttcgcatcaattttaataacggccaggtcggtgctggggtccgtgcctatcatctttgctttgaatactttgttttcgttgctgagggaaacgctgatttcatcggcgtctgcaactacgtggttattggttacaatgtaaccgtctgcagagatcagtacgccggaaccggatgccatctggcctggaacatagtacctgcggccatctccgccaccgttaaattcatctccaaaaaaatcatctccgaaaaggtcctgcaggatactgcgtcttctttgcaggttattaccattggttacctgcctggggttgatctttgttttgatatgcactacacccggcactgctgccttggccgcggtggtgaagtcggaaggtggggtggcattcgcattcccttccgtacccggcatgtagcgggcatagtttacgggaatttcagtaccattctggaaaacaatcggctgcttcggctgaatatatttgccatacacaaatatggaggcagctgccgttacagcactgataagaacagtcgtaacaatttgcttgaatttcatattatagtgtgtttgcgtgatagttaataataacgccgggatatgatcaatttacatgcccttactacaaatttaattcgccctgtgaatcaaacgcaacaggggtgattcactttaacacatttttatatcaatcgttaaacacggcttaataccgtactgacaggaatgacagcccgcctgtcaagataacaagtaattgcgacaaattgttagggcggcgccttcggcgcctttaaattgtcttggagcaggattacgctgattatgttgattacgctgattttcccacgtcttgttgtttttatatttcggggagataaaaagagaccacattttatcttttctaatcttcccattaccatcacaacaaaaggtggaaaaatcttcataacaaaaggtgggaaaatcagcgtaatcaacataattagcgtaatcctgctccaagacaatttccgcggcaagcgccgaaggcgtgcgccgcgctacaactccagcaggaacttcagcgtatctatcccgtctgcataatcagcaagcgacggctgctgggcataaccgaacggcgtgaactgttgtcctaccaggcactgcagggcgtcttcaccggaaagctcctgttgcagctgcgccatatctacataataactatagtgtaaaacgctgatgggtgaaaacaggccggtgttttcctgcagcaggatactgccattagtcatataaggactgctattcagcagcagcagggccaggttatagtcgtagttgtttttgtatttgtgatggtcagccaggtggctgtatttctccagtgctttgagcaggggggcaaagtcgtagttcagtggcacataaatcttagtaacattccgacatccaaggccgaagtacagcatcacatcatcggccagggcaagcagttcctccggggtttccttaccggtaaggatggcggcggatgtgcggttgtggcggataatgtgcgggtatttggcaaaatagtagtggaagtaccgggctgagttgttgctgccggtggcaatataagcgtcgcagtttttcagcatgtcctgtatttccgtttgactggcctggtccggataccattcaccgatcttttccaggatatgtttcatcaggatctcatctttacccgaaagtttcattttaacccggtgtccgctgatgaacccgcaaagccagtcgtggaagcctaccagcgggatattcccggcagaaacgattccaacagttttaggggtgcgtgcctccgcagctttgggatatccctgcaaccactgctgtaaaggggcaggggagaggaaataacgggagatattatccagcgcattgtcgataaaggaggggataaaccaaccattggcaatatatgcacgctcttttactgcttccaattccgggcttttatccgccagatactgccccaggcgcaccaatgcggcttctttttctgctatgttcatgaaactatataaataatgacctaattaaaccgggaaaattttatttttgtcacacaaaattaatggcttactacttaaccaaaaagtttacactatggcaattaagataacagacgaatgtataaactgtggcgcctgcgaaccggaatgccccaataatgcgatatacgagggtggtgttgaatgggcgctagccgacggtaccaccgtaaaaggctcctatacattaatggatggtagtgtactggatgctgaccagcgaaatgcgcctatcagtgtagatacctactatattgtgcccaacaaatgtacagaatgccagggatttcatgaagaaccgcaatgtgcggcggtttgcccggtagattgctgcgttcctgacgaaatgtaccaggaaaccgtcgatgaactgatggataagaaggcaaaactgcacatttaagatattctccaggaagcttaataaccgttcccgcgctggctggaacggtttttttatgtaatttgaacagccaccgcccacaggcgctgcggctcttgacaattaacaaataacctttaactttacccgcttatagtaaaatctcttatgaagaagaatatagctttggtcgccggtggatattccggagaatatgtgatatccgtacaaagtgccgtaactattgaaaataacctggatagcagtaagtataatgtatacaagattattatcaccaaagagagctggagccataccggcgccgatggccaggtgactgaagtggataaaaatgatttttccttaaccatcaacggaaagaagatcgtttttgattccgtatttattggtattcatggtacaccgggagaagatggccgcctgcagggatatttcgaaatgctcggtattccttttaccagctgtggcatggttacctccgcactcacattcaacaaaagctattgcaataaggtagtagatgcactgaacatcgtaaaggtgtccaaatcagtacatattttccgtcatcagccctataatacagcagaaatactgcagcaactgcgtttacccgtgttcgtgaaaccggcagaaggcggcagcagcattggtatgtcgaaggtgaaaaccgctgaagaactgcagccagctatcgataaggcctttaatgaagattcccagatcctgatcgaagagtttatcaaaggccgggaacttaccatgggattgtaccgtgcaaacggcgctattaccgtgctgcccatcacagaagtagtgagcagcaaggagttcttcgactacgaagccaaatacaccccgggcgtttccaacgaaattacccctgcacccataacggacgatatcgcccgccaggtacaggaaaccgctactgttatttacaataaactgaattgtaaaggcattgtgcgggtggactttatctatgaagaaggtaccgggaaattatatttcctggagataaatacaatgcccgggcagtctgaaaacagcctggttccccagcaggtaagggctgcaggaaaaacgctgacagaattttatggcctgcttttggaagaaagcctgaagtaaggattatcacacttaatataattatcgtgttcgactttattaccaaacgctcttttttatttaatctgctggcggttattgtagtgttttttgccctggccctgttgtttttctccatgctgggcttcattaccaaacacggacaacagcaaaccgtaccggatgtgcatgggaaaaatataaaagaagctgttgcgttgctggaaaaagccggctttgaagctgatgtaagggattctatttatattgattctattcctccactggcagtgtatgcgcaaacgcccgacaagggagcacaggtaaaggtgggcaggactatttacctgaccgtaaataaaacagtggcgcccatggtgaaaatgccggacctcgaaggacttaccttccgcagcgccgaaatgatgctgaaaagcatgcgcctcaacgtaggagacaccatttataaacccgattttgccaccaacaccgtattacagcaactgctgaatggcaggaaggtaaagcccggcaccgaagtagcggaaggcagcaatatcaccctgatccttagcagcggaaccggcagcgtggaaaacccggtgcccaacttcgtaggacttacctacgcagaagcccgcgaaatgctcagcgccagcaatcttaattcaggtaccgtgatcattgatcccagcgtatccgatacagcaaatgcctacgtgatcaaacaggtgcctacccgcaaaaatgagatcggcgattttaatatggtaagggccggtgaaagcgtggacttctggttatcagctaccaaaccggtaaccgacagtaccgccgcccctaaaccagttgaagaggataattgaaaatgatgtaatttgattttaaatacttaataacatgcaaaacattacggcagaagaactgaaacaacgcatagacaacggtgaagaactttatatattagatgtaagagaaccacatgaacgcgcagagttcaacattggcggtacgcatattcctttgggctttgtacagcagatgcaggtggacgaaattgaggactggaaagacaaggagatcatcgtgtattgccgcagcggtaaccgcagcggacaggcttgtatgttactcgactccatgggctttaccaacaccaaaaacctggtaggtggtatgctgaaatggacagagctgtataaataacatttagtgccttctgcgcctgctttgcccggtttgtaccggaaatgtaagcgcagaaggattccctccatcaggctttctgctctacaatagcagtagcttctatctccaccaggtaacggggatcaatcagtttacttacttctaccatggtggtagctggtttgatgcttttaaagaactccccgtgtgcccttccatactcttcccacctggagatatctgttacaaacatccgggtacgtaccacatcatgcagcgtggcgccggcattgattaaggcggattctatttttgccagggcaaatttcgtttgctcataggcgttaccttccgctaccactttgtcgttatccgatgccacggtgccggatacttcaattacattgcccacccttactgcccgggagtaacctacttttccttcccagagtgccccggaggaataattggtgcgtttcatagctgttttttagaaagatgaggagatatgcaaatctacaacatcttctttagtgtgtggccgcggtgttggtcccggaggtatctgccgggggcggcgcgttcctgaatttcaccacctttcccagcaaatcaaaccagaagggcgctcccagcgatatggccagtgcggtaatgcaccagccggcgaagaccagccagccgttttgctgaaaaggatgcgtgtaaccgcagcgcagggtaatatggccgccggtactgtcggttacacaggcccgtttgatgccaagcacgtttgccgcatcgccggcatcgctgcgcagcatgccatacacgcccagcagggaagtatcgctgacgagtatacgaacagaagtatcggcccggaaaaaggcgctgtccttatgcagtacgtttttacgtataagcgtatcagtgatggccgtataacccggcgcccggctggatgccagctgcaccagctgtgatcttacatttttgtctttcatgaggatccgcgcaatagcaatggaatccacgttgaacaacgccgcaatggccatacccatacatagcagccaggtttgcgtttgcttccggtaccagccgctggcgcgggtcatggtttcattaaaccatgtttccatattaatccggaaagctgccatattgtgccccgcatcttcaaataattgtaacaggtgctccctggtacccggtaccagctgcaggtaattgtgcgtcagcgccgctttgatagccagggcatctgttgccttgtgctcgggcacactactgcgtaacaggtgcaccattgcctgggaaaagatctgcggactgatataagcagggcgcgaagtggcgctgttctcgcccaggttccggatagaaggcgtgctgtaaaactttttaaggaaaggacttttccggaaaggctcgaagaaataaaccacactccatcccagttcataaaaccagttgaagaaagtaaacttcccaaaccagcccaggtctttactgtgatcatcgtcctccagcatccggcgtaagcctttcgttaacagccgcgccctggaattgaagatcctggcaaccagctcctgcaccaccgaggccagcaaactgtatagcagataaatgaaaataaggccgagggccacatctatggccaggttactaaacataaggataggtattaagttgacatatttacataaaagtaaatatttataccaaagataaaaggacactacgcaatgtatttgcaaactctccgttatgttttttaacaaattgctgtgtcagccgcagcatggaaacaatatatctttgccaatattttagtgtatatgaaattgaaacatttagccttgtgtttgggaatggccgctaccgtcagcgcttccgcccaaattaaatacagggataccgagaagaagccgactttaattccttacgacagcagcattgcctttcagcatcttacaccggatattgcccagctgacgctggtaggacaggagatcactttcctgaaactgaatcccaggcgttcggtgagaaataaggaagataccctgctggacaatcttaaaatgaaagccgtagtggaagtgccttataaaagtgtactcaaaggcggacatttttatacgccctataaggcgatagaaaataagacattccggatcgttgactacgaccggagaaacctggaaggtacttccacacttattttcacgctgcgtgatgaggagcggaaactattgcttttccaggtgccggaagacaacctttctaacacaccggttattattaacggcaactacgaatggttgaagcggcagtatgtaggaagaaaattacatctccggaaagaaaataaaaagacggaaaatgttctggacgataacaaggaaattacgctcaccaacgaggacatttattcctgcacagacattgccgttatttttgccggtaaacagaaatatggtcagcccttcctgatcgttaaaaacagcgagaaccaggaattggctatcggggtgggaaaaagaagtgaatacaccaccggaccgctgattgaagaatttgcattttagtcttaacgggaaagcagctataccaaatgctttcccgttatttattttgtatcgccggattcaaaaaagcaacagctgccaccaacccaggtatctttgctgttgaatcctacgcctatcattttacccttgctgatccgggccaggttatgcaccagcatcggccgcgcagcgccatcctgccagatatagatcatgcgtatttcgcagatagccggacccgtaggcgtttctatggcaggtgcatatttcaccttatgttgtaatatccagttctcaggatctttgatccggtcaatatcttccgcagtcacatctatcaatactccctgccctgcaaaagaaaaaagcggctttagtacataattttccaggtcggcaggcaccaccggtaattcatgcaggaaccagcttttgggaacatactcgctgtgaataaaaggcatgatatacttactgatgcggtaaaaccagttggggtgcgtgatccactccacatccaattcctggaaaagattgacatgagcgccaatactgtcggcctggcgttgcaggtcgtcgaaaataatccggttataaatacggcgtacacgggtttttataccatctttcaggtaaaataattgcttgccttcctgtatgagggccgttaagcaaatggtggggatatccaggtttttcccggtgctgtaaaaatcaatgcgggttttctgttcttccggcttcacttccagcagtatcacttcttccggcgcataaggcccgatgatcatttcacgcaacagctggtaataggctgcttcatccagtccgttgaaaaaattactgaaggtatccggtatgttgaaatgcgttttaaaacggcgggccatcacttcctggaaagccatcatggtggggaatccctgcaattcaatgagctgtggcgccaatgaaccatctgcagctttgcaaacggcaaaatcaatgacaataaaatgcggatgctcattttcattgggcaccttcagtgaaggtggaatagcgtcgcgggtaatggttttaaaatcggggcgcagcagcacatccactatttcttcgcaggcctgaaccagtttattacgaagggctgccggcacaaatacaggagtttcagccacccggaaagcaggcgctacaccggtatctgccgcaatacctgctaaaaaagcctggtattgcgctggtgtgaattgttgattatatgcctttcttactgcagggatcataagtttttaattagaagaacgagtgctcgttatcattatgcgccgctacctgcaccagccgttcaatggccgccagcctgtcggacagccggccataaatagcgtagtcgaggaacgcggtaataaagcgatcgtgcgtaagcataatcctgttgggatcagtgagctgacggatcatgctgttgtatttttccaggccgtgatgcttcactacctgttttttcttttcttcctggaggaggtacatgtgcataccggcagcatcggcttccggatggaactgggtaccaatgaagtgttcattgaaccgaatggccatggtagcacgttccagcggaacatgcggccgttctttttccagtgcaatcacatatccgcccattgcctggagattttcataatccagttcaatcacctgccagtcgcggctatccacaatgtaaaaaggatcggggagtgcgctgaatactttttcctgcatgcctgcagcggttttatgcacggggaatacgccgaatgcagacgatttgcgtttgcatacatttcccagtttataatagcggcacatgagctggtaagagtggcagataaaaaagacgggctttttttcttcgtgggtacggttccattccaggaggctttctaccagggagaagtaagcggtttcccagtcgctgccttcactggccacggggctgccggggccgcccgtggaaatatatatatcataggaagtatcaggaacctgtatttgctgccttacttcaaactcatcaaattgcaggtccagtgcatgcatgctggcgtatttcaccaatatttcacggatacagcgcatcccttcgttgggaacaccctcatacatgtccagcacagccaccttccagctatttttaattggatgcatgccacaaaattacgcgaaatttattttatgggaatgtactaacagccctggaggaattgaccctggataaaatccgttactgccacaaggtcattggtatccgcatatacctgcaattgcttatctgcaccggtgccggtttccagtaaccgggtagtagcgctgataatatcgcggctgccgagttcatctactacgtcgtcaataaagtcgagcagttccgagataagcgcgcgggtatttatttccatctctttaccaaaatcaatcaggtagccatcgatcccatagcgggaagctctccatttattttcattgatcagggagcggttatagataatgaaattgagattctgcatccgcagcttatagatctttgcacataccgcctggaaaagcccggctatcatgatggtatcatcgagggtgagcggcacatcacaaacgcggaattccacggtgttaaagaagggatgtacccttaaatcccaccatacctttttggcgttatcaatacaattggttttcaccagcagcttgatataattatcatattcttctatgctggcgaaataatcgggaataccggtgcggggaaatttatcaaaaacctttgtgcggaatgatttgaagccggtgttacgtccttcccagaaaggggagttggtgctcaatgcaaaaatatgcgggaggaaataccggacagagttagcgatatgaagggccatctccctgttttccattcctacgtgcacatgcaaaccaaagatgaggttggagcgggcggcgtcctgcatttcattcactatttcaaaatagcggggatgatcagtgatgagttgtttttcccatttgctgaaagggtgggtaccggaagcgcctatgctgaatcccaggtcgccggctatttgtgcaatggtgcggcgcaggtaagctacatctttccgcgcttcatgtatgtccgcacaaatctgtgtgcccacttccactacggcctggtgaaattctgcttttacctggtcgttgatcactttatgcgcctgttctactattttttgttcatgtgatctcagttcccgggtaacggggtccattaccatatactcttcctcgatccccagcgtgaacgccttaaacatgttgttagcttttagcttttagctgcggcgtatagccagcagcggtaattaaagcgattcatttcagtgtagtgctttccgcaaatcgaaagactaaaaagcatgaacgctgtctgcaaatgtagggcagtaaaacggtttcacttttctttttgttgttttttagcagggctttttttagcggccacctttttctccttttcgggtgcgcttttctttgctttgggagctgttggtttctttttctcaaccgtcgttgctgcctttgcttttgcccggccaggttgcacaaatttgccccaggtaagattgtcttttcctggtttctgtgcaatggccctttcaatggcatacctggcgctggtttccactacccattcaaaatgttcggcgccaatggagtgaatatcggcgtccggtgccgggttgcagaaatcaatggcataagggacatcactgcgcaccgctatttccacggtattgaaatcgtatcccaggtgctggtgcagggtaagcacctgctccgtgatccgggccgcgagttccgggccgggttcataatctgcctggtaacgcaggtgcggtgcatgttttggattgtatggcataatccgtacttctttaccgcctatacaaaagcagcggtaatactggctgaagtcgatctcttcctgcagcatcatcaccagctgtccggtttcgctgtgtttatggaagaaatcgtccttatcctctacgcggtatacgtttttccacccgccaccggcatagggtttcatgtacgcagggaaactgacgtattcaaaaatactgttccagtcgaacgggtagatcaggttacggaacgacttatcggtagtatcatccggcagtttattagaaggcagtaacacggtgcgtggcacatttacgccgatcttttctgccagggcgttattgaaaaacttatcgtcggcactccaccagaaagggttattgatcaccgcagtgccggcagcagcggcatttttcaggaacgaccggtaaaagggcacatcctgcgaaatacggtccaagataactgcatagcccggatcagcgccctgcatcactttgtcgatggtcacaaattcggcaaagatgccgggagggttaatacggtttacacggtctacaaatgcctggggaaaagtgttttcctgcccgaatagaatcccgatttttttcatggtacttacttgataagtgaaacataatgcggcagcatttcccgccataccggccagtcgtgggtggtttgcgggcggatatccagccagtgggctatttttttgccggctaatatgccggacaacaattcgttttgcggccgggttacatccctgtcggccacgcccaatacaatacccatgcgccagaggtcttcatgctggttttccggcacataatcggccggattattatagtatacgttgtcgtcgtaatgtccgtccatgcggaatttaatatcaaagatcccgctgaggctgaataaataagaaacccggtccggatgccggaaggcaaagttggcagcgtgataaccgccgaagctgcagccggcaaccactatccgctgatgtcctgtttccgtaacaatgcggggtaatatttcttccatgagtagcttgtcgtaacaggtatgattatacgctctttgttccggggaaatatttttattataccagctgagtgcatcaatactatcggggcaatacactttaattcttccttcttcaataaaccagcggagggcttcaatcaggccaaagtccttgctttcataataacgtcccatagaggtaggaaacaggagcaaagggtagccgctgtcgccatataccaacatctcaaattcctttcccaggttgggagaatgccattttaaatagttttcggtcacgggaaagtgtttagataaatttaaagaagattattggtttattggtaaattgttccggtgcaaatacgtcaacattatatcgattctgtgtacctggcgcgcagtgtgcagctggatacctgcttcaccggtacatctccccatatacttttactggtaaatgatggccaggaactttcccggttattaccggagctgccagccactgtgctggtggcaggcatttatgcggacgccgaccggaaagcggtttacggcaccgccggtgtgccggattacctggggcagggccagctggccggaagctatacccgctttatcatagaagaattgctgccattcctgcaacagcagtatccggatatgcggattgtaaaacgcgcctttgcaggcttctccctgggaggcttatctgcattggatattgtatggcgccacccggacatcttccagctggccggcgttttttcgggttcattatggtggcgtagtaaagcgctgggacctgactaccaggatgataccgatcgaattatgcaccaactgatccgtgctggtagctatcatccggggcaacagtttttctttgagtgtggtactgccgatgaaacggccgacaggaataacaacggggtgattgatagtatggatgatacccgggacctgataaaggagttattacagaagggctacaaaccggacaaggatattttttacctggagattccaggtggccggcatgatatggccacctggaaaactgctatggatctcttcttacaattacctttcttttattaataattaacggcaatgcctacattaaaagaggcgcctttccctttggaataaaacccgggctgcataaaccactgagcgcgtgcggggaaatagtcttcgttgaaaagattatcaatacccagcgtaagcagggtacggggagctactttatagctggcattgaaatttaccaggttgtaggcagacacctttccttcgttgccattgtaaacacctttggcatttttctcaaagcggttgcggccatttacgcccatgtactgcagtcttacttccagggttggcagggggcgataggcgatgctgccggttacttttggaggagcaattcttcggccgttcaggtatacattatagctgccgcctgttttagcggtatcggctttcccttccaggtagctgtagctggcgctgatatcgaggttatgcagtacctggtactgaagcgatgcttcaaaaccgtatatgcgttcgggtgttctgcttacattgaacaggtcggtgttgggatcaaagatcatatctgcacccagcttggaagtgctgatgaacccgctcagttcaaagcggagctttttatattcacttacaaagcccagttcatagttattcaccaatactgcttctgtattgatctttttaatatcgtttactttagcatcgcgcagcgccaaacctatgtcagatacggagaacccctgtgagaaactaaagtagggcatgaatgccggcagcctgttgtaacggatgcctgcgttaaataaagtagctgtataatccaggtcgccgccttttaccgcaatgctcggcgcactcgtggtgccgttggcgttagtaagctgaagggtggtataatcatccacacttacccggaccctttccacgcgcacacccgctttcaggatcagattctgccagagcgaccattgtgtttccgcaaagggggcatagttcagcatgttcatctccggaacccataccctgccatctaccagcggctgcgaggtcacattgttcaacaggtcagcgccataggaaagcgtaccgttaaaggcggatttgttcgacaacggggagttaaacatcaaccgcaatccttttttcttgtcgatggtatgcgattgtccgtcgccgccttcaaagcggccaaacgatacataaaagatatcatcccttgattcataataggcatctgccgtgagggaagtcccgccaatcaggctgtcggcctggtacaggaggtggagggtttgatttcctctcggcccggtggctacgccggtgggcgtacccaatacaccggaggcagggatgcctttggcgatgtcgccgttcacgaggttatagtgggagttctgctggctgcggtagtagttgtacatcagctgtatacgctgacggctgtttacctggtagccaactttcgcaaaggcgttgtagctgtctgtttcgcccaggctgtagttggggcctaccagcttgcctttggcgtctttgaattcgccggtttgctctgccacaccgctcacgatgtagtcgaactttttatatttcccttgcaatacctggtttaaacggccacccacactatttttgatgctggtgagcgaaccggtggcattgatcattgttttaccggacagaattttatcttctttaggcgtaacagtgatatagttgatcagcccgccggtagcaccattgccgtaaatggcggtggcgcctttcagtacatccaccctttccaggacggatgggtcaatagagcgcatatctacttccccgttacggagcggggtggattgcggaacgccgtcgatcataatgagtacggagcggccgcggagggattgaccaacgttgctgttggtttgtgtgccgggcgccaggccgggtacttcccgggcgaggatatccgttacatctgtattaacagtcatgtcgttttccagtgttttccgggtgatcaccgtcaccgaggaaggaacattatccagtgttaccggcttgcggctggcagaaactacaatttcgcccagtgctctcggttcgccgagggtatcttttttatggttggtggtattttgctgttgtgccatcaaaggtgcggtaaatccgcagccggagagtaacaggaggcataattttttgtgtagcatgtggtgtatggcagtagtgttgccgtttaaaatgtacagatttgcgtattggccgaatttattacgggggcgaaattaggtaaaaggcgggcgattgatttacgcaatcgggaaaattttggggatggttttaagcttcctggagaaagaataatcatctggaaagacaaaaggctaaataagagagggctgaccatccggccagccctctctttataaattaatcattgctttcttagaagctgtaacgaagaccaagttgtcctctccagcgtgcagtgaagttgttgatatagtatggtttttcatcgccaaaaccattgatttctcttcttctgtcatactggaaaactgctgcacctgaggtagcatcatattttctgaaggtgagtggagtagaagcgttgttggcgataaagtaagttctgccccaatcctggttcagcaggttgcctacgttcaggatgtcgaaagtgatttccactttatgacctttgtaaatgggcagtacctgtgccactttaaagtcgaagatattttcgaacggcgtgcggcttgcatttttctttgcattttcaccacggtgtttgctcaggtagctgtcgttgctgatcaggcgttccaggtcggctctttgttcatcgggtgtgcgggtataggtcacattacctttagaatctttctgagagatcaggtcgaagctcattgtagcaacttctgtagcctttggaatgtagatcaggtcgttgttaccgctggagttcaggtcatcaccggtaggatcaaccgtgttgaaataaacccatgagtaaggaataccggattgaccgttatagaacagggttacggtagtacggaacttatcttctttaccatatttaaaggttttggaagctactgccagtacgcggctgcccatgctgtagttagagcgggccatttccaggttattcaaaccgttgatgtttggtccgaaacgccagttggagccggcagtagaagaggtaccatcatttactgagtaggagtctccgtaagaataacccactttcaggaacagaccattgcttgtttgtttggtcagttcaccggagatgttataggtataaccttcgctggtatttttcagcaggaggatctggttaccccagttagtggttttctttttccaggtaggtcttttaacaccaccacctaaagaaacgctgtcgccggtaggaacaacgttcaggttttcccagatggcattgttaagcgttttggtaaagttaccttctatagtagcactcattccccatggcagtcttctttctacagccaggttggttttaaacatctgtgggaatttgaaatccttgtctgacaggttaatgttggaagggctgcttcctacgttagcacccatcgccgacaggttggcggcagaatactgtccgtaaaaaggactgttaccgtcgtagttgaaacggaaactatttggtaaaccggaaccgctcaaacttacgttggtatatacgttaccggtattgccgtactggttggaaatccatacaaacggtacacgtcctgtaaaaatacccacaccaccacggatggtagtcagtccatcgttagttacatcccagttaaaaccaatacgcggagcaatcaatggtcttgattttggaatggtggtagtggaatagcctgcaaagttcgggtctttagaaaatgctacgttatccggaggggtggttgggaagataggaatgtctattcttacgccataagtcagggtgaagtttttcctgatgttccactcatcctgtgcataaataccgatctgtgctgctttaaagccaataccatcccggagggtagaatcagcggtgttgtagttgatctggtattgtcttggtttcaggttattgataaatccgctgatggaatcataagtgtaagaaccgaaagcaccctggataaaggtatttttgatcttatagatttcagcattggcgcctattgtaatggtatgtttacctttatacatggtcaggttgtctgtgatagtccagatactctgatccaatgcattggcagtagaagaaaactcactgcccaggttgatagtacgcccgttatcattaatggtaacagttgggaaaggttgaccgagagaagttcttctgtcttttacattattataaccgaccctcagttcattactcagcctgttagagaagttggagttcaactcaatcacactggaattacttttagaagggaatttataatagttatttgcaaaagcagcagagctattggtccggctgtagatcaaatcacttgcattcaggtaattatgacgtacagtcagtttatgaacggagttgatgttccagtcgatacgtccaaagagggtggtagctggtttatcacgttcctggtctgtatagcttcccaggtctactttatatttattggaaacaaagtcgtagatgcttttcagttcatcggtggttacgttggaagctccggtggcagggttataatctatcgggttattcctgacagatctctccgcgtttacaaagaagaacaatttgtttttgataatcggtccgccgagtgatgcgccgaatattttattggtgaaactgccgtagtctgcacgggtagaatccggggctttacctacgagggattgaccctggtagaagaagtaagcggcaccatgaaaatcgtttgttccgcttttggtaatagcattgataccaccacctgtgaaaccgctttgtttaacgtcgtaaggattcagtacaatttgtagctgatcaatagtttctatggagatagggttggctcctgcctggccaccattggtaccggaagcagataagccgaatacgtcgttggttacagcgccgtcaaccgcgaattggttgtacttgttgctctgcccgccaaaagagatacccataggtgacccatctttaccattggtagatacagatgcctgtgggctcagtcttacgaaatcctgtacgcttctgttaaccgtaggcaggttatcgagttgggtacgggaaacgttcagtgcggtaccgccattacctttagcaatcgccctgctggctgtaatgcttacttctttcaggctggtagagccttcagaaagcgtaacatttaacttcagcggttctccgagtttaaggaaaatgtcgttgtaagtttcagtgccatagctgataaatgaaacttccaccttgtaaggtccgccaacacgaacgttagggatggtaaattcaccactgccgcgggtagtggtgccataaattgttccagtaggtgtgtgggtggcttttacagtggccccaatcaggccctggccttttgaatcggttacaacaccggtgatgctgctggtagttacctgcgcataggttacaaacacggtgagcaacaatgaaaatgtaaagagtagttttttaaaccccataaagcaaagaagttgttgtttcagacgcaaagttgaacaattttcccgtgaaaattttaacgcggaattaacaaattgttaagtacactgtggatatctcaagcggcacaataaaatttgaatgacatctagctataaccggcttaataaatagtttttccaagaatttccctgaaaattacgatttctcaaatatgagataataataatgagagaaatctgccaccacagtgaaccttataaggtttcaggtgtataattccgttatcaaattgacaatcattattatatgttaaaattcagctgtataattaacatcttcccaatacttttcgggtagaatcacacttacttcccccggcaacttttcataagtatatgtcgtaactttgcgcaattcaacattactgacccggagggaataatatatgttagatacaatagaagcagcaatagaagatataaaaaacggtaagctggtgatcgtggtagatgacgaggaccgtgaaaatgaaggtgattttatcacggcagcacgcaatgtaactcctgaaatcatcaactttatgagcacccacggccgtgggctcatctgcgcaccgctggtggaagagcgttgcgaggaactgggactggacctcatggtccgcgataataccgccctgcaccaaacccctttcaccgtttcggtagacttgctcgggcacggttgcactaccggcatctccgcacacgacagggccaaaacagtgcaggcgctgattgaccccactaccaaacccgaacatttgggtaaacctggccatatatttccactaaaagccaaaagcggcggcgttttacgccgttccggccacacggaagccaccatcgacctggcccgactcgcaggatttgagcctgccggcgtactggtggaaattatgaatgaagacggctccatggcccgcctgccggaactccgcgaaatagccaccaaattcaaccttaaactcatttccataaaagacctgatcgcctacctcctcagcacagaaacgctgatcgaagaaggcgtgaaagtacaaatgcccaccaaatacggcaactttgaactcatcgcctttaaacaaattaactccggtgaaattcacatggcactgaaaaaaggcgactggaaaaaagatgaaccggtactggtaagggtccactcgtcctgcgtgacaggggatatcctccattcactgcgttgcgactgtggcgaacaactgcacgccgctatgcaaatggtggaaaaagaagggaaaggccttatattatatatgaaccaggaaggaagaggtatcgggctcatgaacaaactgaaagcctataagctgcaggaagaaggcatggacaccgtagaagctaacctggaactgggctttaaaatggatgaacgcgactatggcgtaggcgcacagatcctccgccatctcggtatctgcaaactccgtcttattaccaacaacccgcgtaaacgcgccggtttaagtggttatggcctggaagttgttgaaaatgtacccatagaaattcatccaaacccacacaacgagaattatcttaaaaccaaacgcgataaattagggcatgatatcctcaggggataagtgacggtcaccattgagaacgcgtatagtaaggaatgaatccattcctgcaaagtaaaccacacaggggagtaatactgtttaacagcaggttgctccctttgttgttttattcaatgttggtagtatctgctttaacccgggaagaatcttcctgttcctgtttcagcatcgccgcgcggcggagggaatccagcaacggcgtgcgcctgcgccgcctgtcgttaaacaactcgctgaagcggttgtattccctgatataggaaatacccaccccggatttcgtacggttgttgaggttatatacatcataatccgttttactgaaggcgttgatacggaaacggccatccggcgtaaggaggtactcaatgcggaagtcgccggcaaaacggttggtattggcggaagtagccgttttaccccaatcgtaatccccaccggcatataaacggaaacggttattaaacaaattgctcgtaatacctgcgctcacctggttacggtctacggacgagttgtcctgtggcccgcccacattgtacgcgcggtaattcacattcaccccgatgccacttcctttcagcagcacacccgtaatattgttgagaatggcctgcgcctgggccgataacgcctgtcccacgctgtttttcccggtaatgcccacgttggcagcggcggtagtagtagcgtcatccggcaggaactggttggaaaacagcaacccccacacctggaacaatgccttgttctggtcattgttaatctctttcaggtgcgcggctacaccactttcataagccaggctgccgacttccggcaattcaatggagtacgtaatatccggcttcagcagggcgccacgcagattgatccgcacatccactttttcggtgcgcgtggccagcttatctgtgctcacattggtaccctgacctaccaggttatacaagcttacctttggcagggaatatttcgccataatgtttaccctggcttccgacggatcgccgttccaggtaatggtactgttcttttctatgtcgaacttccagctggtgagccgctggaaattgaagttgtaggaaccgttattgatttcgtagttgccaaacatggtgaagtcgccttctgtattcaccgtgatctgcaggttaccggtaccgttggcggaaataatatcgccggtggtggcgtccaggataacatcgatctgcgcatcagggttggcggcaatgtccagcttgacggtcagtttggtattgtcttttttcttcttcttttcaacaatctcggtgccatagcttttgaacgtgatgtagtcgtatttcccgatatccttgctgtcggacatagggagatagaagtgggtgcctttaatcgggcgggccaggatgtgcatctgcatatcattcagcggccctgagaaatatacctttccgtcggccagcacatctccgtaaaacaggtcgttatcggaagcgctggtattcaggaacaggaatccgcggccggtgacatcaaagtcgaaattgagcttgtcgaaatggtcatgactgatatacccgctggcagtgcctttggtattgtatttatctaccagcgtaaagttgccgaattcaatcaggttgtcatctatgttcacattcagcttcggaatgcggtagtgagtgcccaggtaatctacggtaacacccacggtatcgagggtgagcgcgccttttacagatggcacgcgcgtggtgccgcttacatttaaagtaccggttaccgcaccggtgagattggatacatagcccgcgaggtatttattcaacaggctgatagacgtgccgttgagcttcacgctggcatcaatcccattgttggacgccgttaatcctactttaccacgggccaggaaagcttttccttcgttatccgattgtatgttaaaggtggcgtcaccggtaaggtgatgataggtgccatctatgtttaaaataccgatggaatcattgtcgatgcgcagttcccttgttctcagcgctgtattgatatccaggttctgcgtgggatctgcaatattaatagtgccgtccgtaattccctccaccctggtggaaatcagctgggcaggaattacatcagccaggttcagatttttgagggtaacgatgaatttggattcatcaggattaaactcattggtttctacggtaatgctttggtcgttgcgggttacccgcaggttttttaccgtcaggaaatgtttgctccagtatatttcattgccgggggtaacattccattgccgttcatttacggtgaaggcgctgttgaggaaattgatcttcaacccgtccgatacggtaatgatccgggcgtagaagccatccagggaggaagtgtcttccgcagccaggtccacttttacaaaagaggtgtcatgccctgaactggccagtatcaccgggttttcgaggatcacatttttaccggataatactttgccgatgctcgcactgatgttaaccttattaaagttaccatctcccttaatctgtaattcctgtacatgatatcccaggtagccggcttcgggtacctggatgttcaacgccaggttgccgccattcatggtattgagggcgccggttacggtcgcatggtcaaaccccgaaaactggttggtaaagccactcagcagtttatccacttcaccgagattaatggcgtaggtgaagttctgattgatgaccgcattttgcggcgcgctgaaatagctgggataatatttatacagcagcaggtgaaaagcatccggcagctggaggaaactgtactgtccttttacaaagccgtcgatttcactgccggtaaattcaagcagcttttggttatccaccatatgcgacgatacatacagggaatcaaattcgaggcggcggttgtccttaaacgcagatacatcgtacatccgcgcggtaccatcgaagttatcgatgttgctgcccacaaagttcagctccagtttggcctgcagggtaacggaatcttctgtgatatgcagcgctttcagatctgctttacggatttctgaattgaatttgaattccggcagggcggcattaaaatcaatggtcccggcaaagtccatgtccaggttaggatcagtggccgtgagcgcaccattaaaaaatttgcggctcatttccccctttgttttgatattccggtaattgtatcccagcagggatatttcctggatatctgcatccacggtagctttcagcgttttaaaattgaaacccgcgccgtctactttggcatcgagggagatggtagaaaggttagcgttattaaaaagggtgccgatatcaaagttggtagcttttaaactcccggagtaaacagggacatcgcggctggttttaaagttcagatcggagtttaccttaccaaggttggtctggaactggccataggccacaaagtcgttgatgaacccggtatagcttccctggaagcggatggaagacagcttgtcgatgcgcacggtgctcacaatgtcctttacaatgggcatgatctgcatcacgtcattaccggtggtgatgagttcttctgtatgaaaatcaataaatgtttcaaagatatccggcagtccgcgcatttccaggctccctttaagacgggtggtgctacctgcggtcagatctatttcagatgctttcaggttgctcaccgggcccctggctttgccgctcagcgtaatttcctttttccaggaggaaaggggcggtgcaaaaaaggcgatatcatctgacgatagtttgcaatttttaaaccgggcctgcataaacacatcattgatataatcactcatatcactgatgtcgctgtattgcatggtgtaatagtcgccgatatgactgcggttggtttccaggtcgagctgtgaaaattccatttccacgggcgacattttaaaccggctggttaattttttcacctcaaagccgctgcgttctttggtgctcagggtaagatccccgatcacactgtcttttaccagactggtattgctgagggagagattgatgtcattgaagcggatatgattgggtgcaaaatagccgggttcaattttcgtgctgtcgtcggggttatccaccccgaagatgccgtctttgatattgagttctttcaccaccagcttccagttggcattattccagcgcagctgctgcagttgccctgtatctggtaccgggtggtccggactgggtttccgccggcgccgcaggggagaggcggcataactgctgataatgaagtctggattggtaagcgtcaattcctgtatatcgatgttatgtttctggaggtccaggttcttcgcatcgagataaatgcgtttggcagatgcccgcatatcttcacccacccaggcatccacctggttgagccggatgtttttaagatcaatttttttcaggtcaagggagatgccgccggagggttgactactggtatcggttttggatgagccaaatgcttcttcgaggaaatgatagttccagacggaatctttgcgggtacgcaacaggtttacctgggcgttttccaacccgatgaatttgatcacgggcttgtcctggaaaaagaaccagtcggtaatgcgcacctgcagcttgcctgcatacaacagcgtgtctctgtgctgatcttcaatgagcgcaccttccagctgcatgctgttgaacagccggaaagtcacgtggtctatttccacgcgcgttttaagctgctgcgacaagcggctggtcacttcatgcacgaggaagttctgcactacggggatgtttaccagtattccgatcagaatgacaaggcctaacaaacacagtaacacgacagataatattttccgtacttttttcaggcggcaaagtttatccggcaaaaataattaatagttggcagccaatgccatttagcaaataaataagatgtatttccggtttaagtatgctgatggacgatttcgtatataggtgccagtgagtatgtgcaggtccgttatacgtccggaaaatcctctggtgataagtttatcacgaaattgtcggacctgtctttttattgtgatgttatattcgtatttaataatagtattttgtctttaaaagacaggtgcttaaatgggtctctcttgtttatatctgattgtcaataatttacaagaagatataagcgttttctgtcgcgtgaaaatctccgtcacggtagtgtcactaattctttccggcctattaggaaaactttaacatttctaaatttccttccagaacaatgaagtacaagtgagcaatcgatgaacaaagtagcatttcagtgaacaaaacattttagcaaccggaattattcaagccaaactatagcataccagcaacagttgtaattcacccgtttcaataacagtaacaaggattaattcaccagtgaacaaatttcagtgagcattcagtcaaccagtctgataattccagaataattcaataaaccagaatctatgcacaaaaagttgctactactagcgctaatgggattcctatgcctgcacgcatgggcccaggagcgaaaaatttcaggtactgttacagatgataaaggagcggcattgcccggcgtatctgtaaaagaagtaggtaccaataatggggcagccacaagccccgacggccagtttacgcttaccctgaaaggcaattccaacaaactttccatttcatttataggttttgaaacgcaaacagtggtgttgtcggggaaagcatctattactgtttccctgaagccggatgctaaaagtctgaaagacgtggtggttatcggctaccaggaagtacggcgtaaaaccgtatcagcggcggtttccagcgtgaaaggcaaggatatcgaaaacctgccttctcccagcttcgaccagctcctgcaaggccgcgcggccgggttgaacgtacaaaacttcaccggtgaaccaggtgtaagaggctctttcgtggtaaggggaaatacctccatcagccgcgatgccagcgccgcccgcaccctcagctccccgctgttcgtgatcgacgacatccccgtttcactggacgatgccgccgcatttgacaacaccggtaccaactacatcgccgggctgaatcccaacgacattgaatcgatagatatcctgaaagacgcatccgctgccgccatttatggctcccgcggcgccaacggcgtggtgattgtgaaaaccaaacgcggtaaacagggcaaaccacaggtgaacttttccacctacgccggtatgatccagaaaccaaagtttgaaaccgtatatggcggcgcagaagaaagatggttcaaaatggactacctgcagaagtatcttactgatcagcagaaagtgaatggtattcccatgatgctgacagatagcctgaaccctgccttcagcggagcggtcgactggcaggacctcttctaccagaatggtattatccagaactacgacctgtctatctccggcgcttcagaaaataccaactaccgcgtgagtggtaactactacgatgaagatggaaccatccgtggtaccggctttaaacggtacactatttcagccgccatgggcgtaaaaatgtcgtcccgcctgaatgtggcctccctgttccgtttgagccgcggcgacagatcccgcggtcgcggcgtgttccccggagaaaatgtgatcccgttaatagatggccagtatctttcttccctgttcaatatctcggatatcgaccgtaagaactttaccggcgacctggaatccggtcgtgataaaaatatcaatgatgatatcaccgccagtcttaccgtgaactacgatatctctaaaaagctgcgctttgcttccatcgggtctatccagtccagcatcaatacccgcgatattttccgtcccggagagttgaacaccgccggtttatcttacgcacaaagtggtaagtcgcgttttgaaaatgccaacctcgacaacaccctgagctatacttctgatatcatcaataaagatcatcatctgaacgtgctgctgggtaacactatcaacaatatcaggaatgaatttaccggtattggcagcggcgcgctgagtaatgataacgtgaaagtggtacagggctacaacctcagctacctgatgtacagggatgcatatggcaacctcgtttcaggttccgattaccagtcttccggtatgctgtcctttttctcccgtgtgaattataactataaagaaaaatacctgttgtcatttgcctatcgtgctgatgcttcttcccgttttggccgtaacagcagatggggttacttcccctctgtatcaggtggctggaatatttccgacgaaccatttatggccccgcttaaaaagtgggtggaatatttcaagatccgcggaagctatggtgtaaccggaagtttaccaaaacaatattacctccagtataataattacagcatcaaccagggtacctacggcggatctaccggcggcacctacaacggcgtgaatgccgtaacgcctaacttctcagatggtgtggcacaggacggactcacctgggaacaggccatccagtccaacattggtgtggatgcaagcttctttgccggcagattaaatgtaactgccgacgcatttaacaggggtacttccaagctgctgtttaacctgctgctgccttccactgcggggtatgataaagtaaataccaacgcggtagatgtacgcaacaccggcgtggaattcacggtgcagggccgtatcacaccgcccaccagcaaattccagtggagttctaccctgatattatctttcatcaaaaaccagattgttaaattacccaatggtaaccgtgacctgatggtaccggataacaataccggtatgacgtatgtgctcactaagggccgcgctatcaacgagttttacctgatgaagagcaaaggcgtatatgccagcgaaaaagatattccgtttaacccttacaccggtgaaaagctcacctactggaatggcaaccataccgtgcaggcgggcgactttatctgggaagaccagaacggcgactacgacgtgtgggactggaatgacaaggtgcgcagcggtaatcccaacccggcatgtaccggcggtttcaccaacgtattttcttacggcccctggagcatgcaggtgtatatgacgtttacccttaaacgtgatatctacaataaatacatgtccgacaggctcaccggcttaaccaacagctatgctactattgcgggcatagatccttcttcgatcaacagctggcataaagaaggcgataacacccaatattcagaagtaattccttacagccagcagtattactaccagttccttccattttcgtcagcctttgtagaaaatggttcttacctgcgtatcaaatacctgaacctggcttaccagttcagtcctaagttcctggaacgtgcaaagctgagcaaactccagatctatggtgtggtagacaatgtaaagatgttccagaaatcaagcgttccggatgcggaagcagtggatgaaaaaggtacttacaccggtggcggctaccccataccacgtaagttcaccctcggtgtaaatgttggtttttaattttaaaaaagaagaagatatgaattgtctgaaaaatatattcacggtaatagctgcaggactgctgttgtcgcctttcgtgtcctgtaagaagctgctggatcaggagccgatcaattctccctataattccgttttctggaaaaaccagcgggatgcagaacagggtgtggccggcggctatgcgttattgcgcagggcattaactaccaatacggactgggaccagaacatgtcgcattttgcatatggctccttacccgcgtatgaatttaacgactacgacgtgtatgatgtgaggttcctggtgaaaggtggagatgggatgaatacggccgatttcctgggatcttacctggataaatatcacgactggtctccctactataaagtgatcacacaagcgaatattatgttgcataatattcccaatatccccgatgcacagtttacggatcagcctacccgtacccgtaaccgtttcgtcggagaagcttacttccttcgcgcgttcagttatttctatatggtgcgcctttggggcgatgtgccgctggtaacgaagtatgatcctaatcctgtgggagcagaaaatattccgagaaccaatgagaagatcatcctggatacttgtatagctgatctgaagaaagctatcagcctgttgccgtgggaatacaaaaacggcactgaaagagcggtaagagctaacaggggcgccgcatttggcttactggcccatgcatacatgtggagaaacttcctgaacaaaggacaggtagtatccgatgtaaccaatgcgattgccgccatcgattcggttgagcaaagcggtcaataccagttactcgccgccgaaatgtatccaaagatcttccacggaaaatcaatggaaggcatattcgaaatcaatatgcaggtagcggatggagaacagcaggtagaaaaaggattttattatagcattctgaaaacaccttttatcagtaataaagatggaaaggtagacgcgccgaatattgacctgatcaatttactgtatgatgaagccggtaccgatgtgcgccgtcattattacttcaccaacctggatgcgtttgggcagtacgatgtgatgatctgcaagtttgcaggccctaaccgggaaaacattaactaccgtaatccgggcaactttacagatggtgctgtagatgccaacatcatcctgatgcggtatgcagatctgctgttgttacgtgcagaagcccgtgccgaccagggcaatgtaggcgccgccttgcaggatatcaacagggtaagggcacgctcgcatgcggaacctattttagcagaagatgtggccgacattaaagaagaagcattcctggaacgctcccgtgaattatatgcagaaggacaacgttggtacgacctggttcgcaccggcatgctcatgaatggtaatgtgaacgctgctccaggtttcccgcaggaccgctttgatgccggtggctggaaatggccggtaggacgctcgctgttcctcaataacagcgtgcttatacaaaatacatactggctgggtaaagtgaaatagcatcttgaaattttaaacgtactgacatgaacaaactaaaaatatttaccacaaaagcaggatggggcatcttaatgatcaccctgttgttcgctgcctgtaagaaagatgatcatttcctgggaggcagtcctaccaacgatcacaccgatcttactacctacgattacctgaaagcaaatcctaatttcgatacgctgatcctgctgatcgacaaggccggtttaaaagaaaccatcaacagcgatattacttttgttgcgcctacagattattctatcaaacaattcctggcggtgaggaccaagctgttgcagattgagctgaacgatgaaaacgttaagtatacgattgatagcctgaaaacgcctgaactgcgcgactccctgctggcctatgcttttgcaggtaaaattgtacgtgcagatctttcactggaatcacaggtatataaaaataaagtgaacgaagacttcgctttcaagcttactaaaaccgacgcatttggcaatattttttccgggggtgtgcggtatatggcgcttacaaaagtgattaatggtctcgatccggatccccgtccggatgactatccggaggaagacagggatatgcagtataccttgcaaacaaccggtatcattaccaaaacaggtgtattgcatgtactgcaaaacaaccacgtgttttattggaaatagtcatcaccactaaacttaaaagtatgttgtataaatataaagggataaaattccttacatccgttgttctgctgggactattgatcgccggatgtaaaaaaattgaggaaggctttctgagcgaaggactctacgtaccggacacccccataaaagtgcagcggggtaacgctttccagaaaacaagcgccatccttgcagatggtaccacccagcccatgaccgtgaagctgcttgacatcaggagggcagataacaaaaaacatgcggatgaattttataaagaataccctgtttacgtatatacggcagcggtagatcccgcgaaagacaccaccattgaactggtgaacaaaaagcgtgaactgaaaaagatgcagccttatgtattcctgaccagtggccagtttgtgtttaacggtgctaccgacagcttaccgctggatgttacctacgaatatgatgtggaagtatccaacgtggcaggctccaaagtgtataagaatatcggtacgctcactacggttgatccgccattggtgactgaaacaacggccaactgtaacttcttcccggatgatgcttctcccaccgtgccaatgggcgcaccggtaatgacgattaccagggtgagtgaaagcggcgcctctgttattctgaaaattacggataaagatggcaaacctttcaatcctaaaaagggagagatcattaagcgtggcgaccgtcctatttttgaaaactacgccaggttccatcccattgagtatacagataccgccatgatctgcaactttgagattgcaccattcccattgagccgctattccaatggcggtaccaactggaactacctgatgtactatcgtattccttctgcctttgtatcggtagataaaaatgtatccagcaaaataggcagcgtaaacccgctgtttgctttccgcctgatgaaagcgggaacctatgttgtggagctgaggatgcctaaaacggtaaaggtaacgccataagaagttggtaaaacataaataaaaacggggttgtattcaacgtaatacaaccccgtttttttgttattttcgccaatcaggtgtatctttagagcatgtataaaacattgacgtacaatatctttctttgcgacgttcgtctaaacagaacgctgaaaccctgtgcaagaagctgatccccaatagcttaccgatcaagtccacgtcacctccacgtcaacaccgtgttaactccatctcaaaggcatgttcaaagtattccctaagtatgtccaaagcaatggcgaagtatgcactatggctgtttatgtttttgtgacaccaaactcctggaggaaccggtgcagcgttgtcatatcttcctggagatgtaacgcagaaactaccgcccggttgattaccgggctatgtggctgcggatatgcaaagctggaaatgatcacgtccctttcctgcaggtattgtaccaatgcttcaccgggtggaagaataaacatgggcaggccatgcggattatgcacagcggtgttggcggtaagatgaagaagaaaggcgatgttttgctgtaacgaccggtgcattttgacaatcagttcaccggattgcagccacgcatgggcataggccggcatcataggcgtgctggcggaaaacacgggcagttttttgatggccatgatatcggctgcatgaccggcaacaacgccgccgggaatactgtaggcctttgccagtgaggcggtgagcaggtatcttacaaaaggtgtttgcggcagaaaatggatggcgccctgcctggcagggcctaatataccgatgccgtgggaatcatctgccagcactaacactttgcgctgcaattcctgcaaccagtgaaaagaatgaatagtgccggtaagcgggttcaccgtatccgtgatgatcacaaagtgatgatccgggtgagtgtttactttttcagtggtttgagtaatccattcgtcgcggctcatagccggcaactccggttgctgctgccacagcgaaggatgcgcatccggtgcatacaggggctgcttgttactgacagcgtattgtgcagcggcttgcgatgcctggtacccggaagaaaaaacaacggccgactgctgctgcaaatgaacagccagggcatgttctatttcttcgtatatggataaacgtaagtttgccgacctggaagaaggaaacagggcgccatacctttcaatcccctgtataagcaggtgtttgaaggctggcagctgatgcagccccaggtaggcaaaccccgaaaagaacaggcagctgcggccgtcctgtgtcactgttctgccgggcgtgtgatccgtatacaacatagccgttaatctttcttagtacataagataaactggaaatcggtagaagttacctgcatgtcgaaataatcttctgtaagccgggtaacggtaaccaggttctccaccttacggtcgccgttcttcgcggtaacagagatcatggcgccattgctgaggataaagtacttacccgtatccgacctgcctgcaatagtggccacgaaaacgttgttatcgaggaattgataataagcatcccggtagtaaccttttttaaggtcctgcgcctgtatgtattgtgtgttgctgatgggcgactccggtggaatttttacatcgtatacccgccactttttattcatcagcagttcattgttctttttaccctggcaggcggtgatcacagatagcaccgcgataacggtaagtagatgacgtattttcatggatggtcagttccctgttttttctttattgaaggctgccgatccgcctttggggatggacaggctttcccaattacttttcaggatcattttcccgatgtatacgatttgtcccacgtggtagggcacatgagccagttgccggttaatggcatctatcacaatgtgaggctcattacggataaacacggtcctgtccaggtctgtttcctgcaggctgcggatagccaggagcatacagttccagccttcgtcccaaagctggaggatttcttccggggaaagatcgctttcttcaaattccccgtcgcggttacggccgggcttctctccgtcggtggtgaggaagtcggtccagcgtgataacatattgccatgcaggtgttttataatcatggcaatgctgttcggctctccctccggttgccagttcagctgcgctttgttgagccgcaacatggttttaaggcccagctcccggtgtatttcaagccgttttagtacactttgtaaatagatagactgaatagacatgtcaatgtttttaagttaatatcctgctgcgctgtcgtcgccacgtttatccccggaagcttccaggtagcggctttcaggcgcccgtttaataatttctgtacggccaatgccgccgcgttttactactttatagcccatcccttccagcgcctggatggtggtgtcgggaaaatcgttctccacggcaatttcatccggcagccattggtgatggaatttaggtttgttgatagcttctgatggggtaagcccgaattccagtgtattcatcagcgtttgaaaaacggaggtgatgatagtcgcgccgccgggtgtacccaatgaatatagcacttcgttcttttgtaaaacgagggtaggcgtcatggagctgagcatgcgtttggccggtgcaatggcgttggcttcggtgcctaccagtccgtacatattgggcacgccgggttttacgctgaagtcgtccatttcattgttgagtagaaagcctgctttacctaccactgttctgctgccgaagtggccgttgagcgtggtggttaccgctactgcattgccatcggcatcgatgatgctgaggtgcgtggtttcctcgctttccggcagcacgcccgctttggtttgttcactggaacctgctttaccgggtgtaaagtcctgcatgcgggcggccaggtattttttatcagtaagttgtgagatgggtactttcacaaaatcggggtcgccgagaaactgggcgcggtcggcatacgcgcgcctttccgcttccaccatcagttgaaccgcctgcggcgactggaatccccattgcgagatgggatagttttccaccatgcccatcagctgttgcaggcaaatgccgccgctggaaggcaggggcatggttacaatcgtatagcctttatagttaaaagctaccgctgtcctttcctttgctttatagcttttaagatcctgcagcgtcatgataccattgccgcgtttcatttctgccacgatgctggcggcggtttctccctggtaaaatcctgcggctcctttatttcgtataagcgtgagcgtatgtgccagttctttttgtatcaatgtgtcgccggccttccagggttgttcttttacaaaggcggttttgctggtattcagtctttcgaaatcagccctggcgttgttcaggccactggcttctgcttcagtgatcacaaaccctttctctgccaggcggatagccggatctatgagttttgcaaaaggcagcctggcgtacttcatcgcggcaaataacccggcaacggtgccaggcacgcctgcggccagctggccatcaagactcagctgggtaaccgggttgccaagagaatcgaggtacatatcccggtgcgcttttgccggggctgtttccctgtaatcaatggcgatattccggccacttttgaggtgacctaccaggaaccctcctccgccaagattgccggcgcccgggtataccacggccagcgccagctgcgtggctatggccgcatccaccgcgttgccgccctgttgcagtacgatggcgcctacacggctggccagcggatgcgcagatactactgctccatgcagcactttgatatctttttctacactataatcgtaaggatgtagttcatctgttgtttgctgggcacaggcggtatgtaaagtgcataccgtcatccccagcatgataaggaaacgcatgggtatctgtttggatcgaaattaaggatatgcggggaattataggaaatttaataatttaagcagtgttaataattatcacccgaaaacaattcctaacttacagtatccaataatagcaggctttctatgcgcagatttatactaatgaccgttgttatgctgggcgttctttttgcaaatgcccaggtgccaacccctgatcagtttctcggttatcccctgggaacacagtttacgccacattataaagtggtagactatttcaaacaggtagccgctacagcgaagaatgtaaagctggaacagtatggcactacctatgaaggcaggccgctggtgctggcaattgttgcttctcctgaaaatgccggccggcttgaggagatccggcagcacagcctggacatgtccaacgcgaaaggcaacagcgccggcaatcagccggtgattgtctggttaagctataacgtgcacggtaatgaggcggtttccacggaagcatcgatgaaggccctgtacgaactggtgaataacgcgaatgcacaaacgcagcagtggctgaagaataccgtggtggtaattgacccctgcctgaaccccgacggacgcgaaagatatgtgaacttctataacaacacccgcggcgctacacccaatgtaaaccgttggtcgagggagcacaatgaaccctggccaggcggaagggccaatcattattactttgatctgaaccgcgactgggcctggcaaacacaaaaggaatcgcagcagcgggtggcgaagtacaaccagtggatgccacagctgcacgtggattttcatgagcaggaaatagaagcgccttattattttgcgcctgcagcagaaccttttcatgacgctataacgccctggcagcgccagttgcaggtgctcattggtaaaaacaatgcgaagtactttgatcagcagggctggttgtatttcacaaaggaacgtttcgatctgttctatcccagctatggcgatacctatcccatgtacaacggcgccattggcatgacgtacgagcaggggggcagcggaagggcaggcgtggcagtactgaaaaaagacggcgatacgcttacactgaccgaccgtattgcacatcatttcaccaccagcatgtctaccatagaagtggcgtcccaacaggcagacaagattatccaggagtatacccaatactttgaagcggcgcagaaagcgccacagggcgggtataaatcatatgtggtgaaggccggcggcaacaccgaaaagcttaatacgctggcagaactgctgcgtaaaaataatatcgcattcggctttggcgccaacaccggcagcgccagcggcttcaattactttatcggcaaaacagaaacgtttaccatcgataaagaagacctggtgatcaatgcctatcagccacattccaatatgctgcgggtattgtttgaaccggtctctcatttaacagattccattacctacgatattactgcatgggcgttgccgtatgcttacgggttaacttcctatgcggtgaagctgccgttaacaccagcggcagacgcgccggcggcacgtaacaacacgccgttgtcgatacagcaaccctatgcttacctggctaaatggaacagcgtgcgcgatgtgaaattcctgtcggcgttattgcaaaacgatattaaagtacggtttacagaaacaccgtttactgccggcggtaaggatttccccgcaggtacgcttattattacccgttcgggcaatactgccaaaggagatcagttcgaccggttcatcaccatgcaggccaatcattttaagatttcactggaagcagtggctactgggttcgtagataaaggaatggactttggctcagacaagatccggtttatccgcaagccggaagtaaccctgctggcaggaagaggcatctcttcactgggcatgggagagatatggcatttctttgagcagcagctggatttccctgtaacggtagtggatgaacgaaatgtggatgatattaactgggaccggacagatgtgctgattttagcagatggggattataagatgtttgaagataaagcggctaccgacaaactgaaagaatgggtgaataacgggggaaaactgattgcactggaaagtgcggcggtacaggtagcgggcgccgactggggcattaaactgaaaaaggaagaagagaaagataaagacgccaaagaaaaagccgcagcagcgcatccgtatgatgccgtgaaaccttatgccaacagggagcgggaaagcattaaacagtttatacccggcgccatttataaagtgcagctggataccacgcatccgctggcctttggctaccctgctttgtattatacattgaagcaggatgcgcatttgtatgagtttattgaaagcagcggctggaatgtgggcgtgttaaagaaagacagctacctcaccggctttgtgggcgcatctacccggcagcagttgaaagacgggctgctgtttggtgtgaaagaaataggtaacggatcagtgattattcttgcagataatcccttgttcagaagtttctgggaaaatggcaagctgttgtttagcaatgcagttttcctggtaggacaatagttttacaggttcctttttatattacatcccagggtatgggaagtgtttacgctgacaggtttgccagccagcatttcgttgatggcattttgtaagaggcgtgtttttacagcgtctgcattacccggactgtcgtcaattccgcccttataagcgagcaggctgtttttgtcaaacaggaagcattcgggtgtatgattggcgtcgaaggcattggccagtatcgcatttttatctatcacataataccaggtgaaatgctgcgaggtggcatactgcttcatggcggcaaaggattcattgccggtacgcgcagcttcgttggagttcaccataatgatgccgatccggttttttgaagcatacacgcagatgttacgcagccgttcctggttgcgcagcatgtacgggcattgattacttccaaagatgaccagcaatccgttggcgccttttgctgcgcccaatgaaatctcttttccggaaatatcggtacaggcaatttctgactttggtaaaggagatcccggttccaggggaacttcccggtttggttgaaaggaagaaagtaaaatagtacagcaggataaataaaaggtggcctttatcatagcgtatggttttcaggtcctgattaaatatagtaaaatgctacaggatattcctgtcttttttcaaagacaaataatcgtttaagatataataaaaaagaataagataaaaatatttgtcagggaataaaagaagaagttgacgaggtttgttatgcgggcagggaagttttttttgtttcttttcttgcgtcgctgatggttctgatgctggcattcagttcaaaccccacgaggaggataaaggagttgaagaacacccacagcatgagtacgagaatggtgccgatagatccgtaaatcttattatagttgccaaaattattcacaaaccaggagaaccctatggtcaccaggatcatgcatatagtggctacggcggcgccggcggtaatgaatttccagcgggtggtggtagcggcgccaatgcggtacagcaccgcattcaccgaataaaaaagcataatgatcagtacccaccgggcgatatcgatcacgttccgtaataaggtgctgtggatgccgatgatgttaaacagccagcggagcgtagcgccttgagcaatgatgagggcaacggtaatgagcagcaggaaaaccagtatggcggtgagttgcagtgctatcagcctgttttgccaccattttcttttccggaagccggcgccctgtattttactgaaggaacgaagaatacccattacgccgttggaggaatagaagaatcccatcaggaaggcgatagagagcaatccgttgcggtgtgtgtagaggaagtcgtggatcattccccgcacaatcatataggtgttgtagttgggtgtcaggtcttccgccaggtcgtagagggtgggctctatgttttgcaccgggatgtatggtaccagtgtgaacaggaagatgaaaaatggtggaatggccaggaggaagttaaaggaaatggccctggcgcggtcccccagtccccggcttttggtttcctgtccgaagtgtttcagtacgtcgtatagtgggatgccttcaaacccgggaaggatcagtgttttagtccttgccaccagccggcggtagggttttgaacggaagatgatgttttcgggtctgaaggccaaatttgttatttatttagaatcctcttttattcagttctgcctggtattttcttgcgtttatcaggtgctcggcataggtggctgcgaaagcatgatagccggagaagtcggctctggcacaaaaataaaggtaatctgtttcaggagtattcaatacggcatttaaagttttttccgagggcgtgcaaatgggtcccgggggcaggccggcataacggtaagtgttatacggcgaatcgaagagggtatgattttcccggatccttttcagcccgaagtcctgcagtgcgaacttcacggtaggatctgcctggaggcgcatgcctttccggtagcggttgaggtatacgctggcaaccattggcttttcatcgtttttattggtttcttcttccacgatggaaccaagaatggttacttcattggcggtgaggcccagtttagcggctttttcttttctttccgccgtccagaattcttccctttctttttccagttttttaaatacggcttctgcgccggtattccagtagaattcgaatgtattggggatgatggcgcacatgacggtgttggtatccaggccaaactggcggaggtataccgggtcatttatcagggagcgcattacattggaatctgcttccaggttgttggagatcttcctgacgaaatcgtttttggtgcgtagtttattgatcacgagtaccaccggtgtttgttttccggagcggagcatgcgggcaatgtcgaagttgctcatgccgcgggtaattttatagcgtcctgcttttacgcggttgggatagtcgagtttttccgccacccagttaaaactgttgcggttgcggataatgccctgttcttccagtccgtcgagtaccgctgagtaggtgctgttggtgcgcacataaaagtatttgctgtcgccaaatggtttggtattggggccaaatacgcggtaggaggtatataccagtgcaccggccgccaaacagccggcaatgaccagtatccgtcttatccagactgattttgcgctggattgtttgcttttcttcgccatagatcgtgttggaagttacaagtgggcaaaggcgtgatcagccaggtttttcaatatacgccgccggttgccattaaaaaaaacctcgcttttaacggcgaggtttcaaatattattatgctgatagtgttaattacttgttgggagcaggagccggtgccggagcaggggtgccttgtaacggagttgatggtgccggaggcgcaattggctggccagcggatgctttttctactgcacttggtgcaacctgctgcactttgctgcctttaccaataaagaaaggagcagtgaggcacaagatggcaatcagtgccgccagtatccaggtacctttttccaatacgtcagttgtctgacgcaccccaatcacctgattaccaacaccaccgaggctgccggagagtccgccaccttttgggttctggatcagcacgaagaagcccaacaacacacaggctaatatgatcaggataccaaaaattatcaacatagaaattactgtttatttttatctgtttttgactttaagtctaatatcttttgcgcaaaataagcgtttttgtcgggattaagcaaacttaatttttgatatatcttaatcgcgttgccatactgctgctggcgtacccagatttcggccagggtttctgaaacgatatcattgttgaatacaatggagtccatcgccattttttccacggtttcagaaacttccggttcttcctcttcttcgtacatccggtgtaactgctggtgataccagtctttgctggttttcccggcaaaattgtctttcatttgccgtaaccaggaagtaaaactcttcatttctgccgctccttgttcgtttaaatcatctgcttcatcgggatttttaagtctcttgtaagcaaaataatcatctgtgtataaaggttgaaagatcagttccgtttcttcttcggccgctgccatcgggaatatcttaatagggccggaggaagttgattcttcttcatccgcggcctctgcatgatcctgcccgttggtagccgccggcattactaccggtggtgggagtatttccgcggtggcggtatgactggcgttacccggttcaaaatccgcgacggcgatgggcgcctccggttcttccattacctccgggagtgcatcttccggaataatggcagctacgcggttttctacaacctgtaacacctcttctgctgtaatcagctgataagcatagtgatgctgatctgaatacaggagcgctttttttagggcggggtgatgaaggttgccggtttcctggtatactttttttgccagcaggaggcgggctgcggaaaaatacgggtgatccgctaccagttgctccattgccgcttcattcaccaactccagggagggttgtagaaacacatgtgctataatcctgtttgccgtcataggttgctaatgtaataaattaatgattacacactaccagtttgcaaaagccctgttaaagatatcatctgtgataccgggaataatattgctttccagcagattgttttccacggagctgggcaattgcgtggccgggaactctgctgaacgggaaaaggattgggtgaagccttttttatcgcctatccttttaatgaaagtaacgtttacagtaacattgagcctggaagtagccgcctggtccacattggttaccgccgcattggaaaaggagtagccggtaatagtggctttgaactcgtaatcggcgcggggttctgtttcattcacctgtgtaagacgggtttgtgaagtaatcttatcacgcagtttcattgtcagcttctggctcagggtcgggttattgatgggcgccctgttttcgatgaagcgtacattcacggtggtggctccctgttcgatactggcgccggtggtagagtacttcacgctacaacctgccaatattgccattacgccgatggctataaatactttgatattgctgatcattgtggtgctaggattaagattcgtttattcggcgatattatattctttgagtttgcggtaaagcgttctttcggaaataccgaggtccagcgcggcatccttacgtttgcctttgtgttttttcagcgctttcacaatgagttccttctctttgtcggcaatagatagtgtttcttctacttcttcgtgatgatcaattttattatccgacaggataatgggctgttgcgctggtcccaggccggcgcctggaggcgtattcatttctgcagcgccgggataagtgtgcagcacatgattatcaggatgatattcagctgcatgtggcatattcggattttgcaggatgtcgaagaacattttctttacttctgttacatctttcttcatatcgaagaaaagtttgtacaggatatccctctcactgttaaaatcgctgttctgctgtggcgccgccaacatgggcaggcggttcacttccggctgatcggggaggaatcttttcagatcattggcagttaccagtttatctgaagacagaacggaaatttgttctgcaatatttttcagctcgcggatattacctctccacgggtagtttaccaggatattacgggcttcttcatccagttgtatcgaaggtgttttatatttttcggagaagtcgaccgagaattttctgaacagcaaaggaatatcttctttacggtcgcggagcgcaggcacccggatggggactgtgttgagcctgtagtaaagatcctcgcggaatttgccctgttgggtacgttccagcaaatcgcggttggtagcggctactacccgtacatctgttttctgtactttggaggaacctacgcggatatattcaccggtttccagtacacggagcagccttgcctgtgttcccatgggcatttcgccaatttcatcgaggaaaatagtaccgccgttaacggtttcaaagtaacctttacggctgtcgaccgcgccggtaaacgatcctttctcgtggccgaaaagctcggagtcgatcgtaccttcggggatagcgccgcagttaacggcaataaacggattatgtttacgtgcgctcagggcatgaatgatctgtgaaaaaacctctttaccaacaccactttcaccgttaatgagtaccgtgagatcggtattggctacctgaacagccacctgcaatgcgtaattgagcgcaggactactaccaataatgccaaacctgttttttatagcctgtatgtccataagcggttattcgtatgtttgatggtttaaaatagcttcagcttccgtttttaaaatgggaagatgattattgacgatatcccacagaatcctgtaattgatcccatcatagtcatgaacaataatgttccttgttgcttttattttttgcacctcactgatattcagatcgggctttatttttagcgcacaaataacggcttcacctattatttgtaattccctttcaatagcgctggtcaatagcctggaagacacgaacgagtcgaaatctgttgcatctttagtaaatatctgtatggcattgatagaatcaatcacatcatacatatatttttctattgatttatccttcataaaccagggtcttatctttattaattgctttaatgaagtatgggttccgaagataatcctgcgcaacaagatccaccttaatcttcaggatgctttcaagtgagcttttcaggtcaaaaaaattgtcagcgtactgatcgccgggaatttctttttccttgaaagagtataataaatccacatcacttccagagtgcatggtattcctggctgcagagcctatcagaaagagatattttacatgatgtttattacaagtatcttttatctcttccaggtgacgggaaataatcggatttatcatactatcaattatttattgctaaactacagctttcccgatcaaagtacctgatgtgcagctttccactttaaccatcacgtaatcgccttttttaaagttttcctttggaaacacgattaccttgttctgatcgttgcggccaaacagctgctcatcggagcgtttggaagtgccttctaccaatactttgaacgttttgcctacttctttcagcatgttttcctgcgaaatatcgcggtgcagcgccaccacttcggccagtctccttttctttacttcttccggaatatcatctgtataccggcgttctgccagtgtacccggacgttcggagtagaagtacatataagacaggtcgtagcgggcatagcgcatcaggctgagcgtatcctggtgatcttcttcagtttccgtgcagaagccggtgatcacgtcggtagacaggccgcagtcggggatcagttcacggatgcggtctacctttttgatataccattcgcgggtatacgtacggttcatgagctgtaagatgcgtgaactgccgctttgtacgggcaggtgaatataattgcagatgttatcgtacttcagcatggtgaatagtacttcatctgtaatgtctttcggatgggaagtgctgaaacgtacgcgcagcaaaggattgatgagcgctactctttccagcagcatggcgaaggtaatggtttcgctgccgtcgttgctggtccagtagtaggagtcaacattctggcccaggagcgttacttcgcggtagccattggcgaaaagctcttcagcttccttcacaatggaataggcgtcgcggctgcgttcacggccacgggtaaacggcaccacgcagaaggaacacatattattacagccccgcataatggacacaaaagaagtaaccccgttgttatccagtcgtaccgggctgatatccccataggtttcctcgcggctcagcaacacattcaccgacttctgaccggttcctgcttctgcaatcagcgccgggagactgcggtaagcatccgggcctactaccaggtctaccagtttctcttcttccagcagtttacctttgatgcgttcggccatgcagcctaaaacacccaccagcatgccgggagtttgctgttttatttttttgaattcagtaagacgtttacgtacggtttgttccgctttttcacggatagagcaggtattgagcaatatgaggctggcttcttccgcgttgcgggtagggccatagccttcctcgcccaggatggaggcaacaatttcactgtcgttgaaattcattgcacaaccataactttcaatgtaaaattttttagtatatgtttgggtgccagtcgttgcaggagcaaaagcttctccctggcgactttcatcatgcactttggtatccagatcaagcatcctgacaaaaattttggaaggcaaaaataggtaataaaaataacaaaatgacagaatggcagaaaatagtatttccggatgattaatgtgcttttgcagatgtgttttcagctacacctggtatataaaaggacattaatgatccggaaacagataatatggtttagaagcgctaacgccctgccggcttgaagttacgcggtttttaacttcagctttgtggctatccagctgtttttcagcggctgcagccagctggtatccagttcctgcctggtaagtacggtattgttcaggtagatggtattttcatcgatataacctttctccagtgcatagccaacctgggccataggcaataactccactttatcttttacgatgaagccgagcaggaggcggtcgaacatattaacgctgtactgttgctctatacttttgataatgcgaacggaactatctgtgctgcagccacttacggcggtctgcgattcatctgccatcaatacgatcacctggttcagcaccacctgtccccagccttttacgggagcgccgtgggcgttccactgggcggtgaactgatgcagctgctcgttaatttccagtatctcctgttcattgaatggtctgttgctctggtatatccaaaccctggaggcgggagaaaagcctgaagggaagatgttgctggtattcataacacaaatttaggtaaatggattcatttcatgctctctgcgatcagttctgctatatccagcacctttacggattcttccttgccggcgtcttttacgccatcggtaagcatggtcatacaaaaaggacaattggaggcgatcacggccgccccggtagctacggcctcacgtccgcgttcaaagttaatgcgggtggcgcctttttcctcttccttgaacatttgtgcgccgccggcgccgcagcaaaggccattgcttttgcagcgtttcatttccacgagttcggcgtccagggtttccaataccttgcggggcgcttcatatatattattggcgcggcccaggtagcaggaatcatgataagttatttttttgcctttgaaggtgccgccttcctgcatctttatttttcctacgtcgatcagcgactggaggaaggtggtatgatgtattacttcgtagttacctcccagtgcgggatattcatttttcagcgtattaaaacaatgcgggcaggcagtaacgatcttctttacttcatacatattcagcaactggatattattctgcgccatcatctggaaaataaactcgttacctgctcttcttgccggatccccggtgcagctttcttcttttcccaaaatggcaaaacggacgcccactttttcaaggatggtagcaaatgcccgggttattttctgggcacgctgatcaaaactccctgcacatcccacccagaacagtacttccggggtttctccgtttgcggcatattctgccattgtcttaatatgcattcttgttattttaaattaataccgaaaatgattgcatgcaatcaaatgaaaagccgaaaagtcatgcaactgtctaaaatttgggtgtatcctttaaattccgacacttgcttactattattactgtttatatctttaagacgaattgaatataaagataaaaaacagaaccgcacaaattttaaatctaactgaattgtacgccagcctgaatgataaggagctatggatcaaggtagtggaaggcgataaggatgcattgtcttttatttatacacagcatttccccgcactgttcaactatggaatgaagattcatcccgatgaaaccatcgtgaaggattgtatacacgatctttttgtgacactctggttcagccgggagcgtttatccattactgataccattcgtttttacctgctggccagtcttaaaaggaatatcatccgcagcctgaagcccctgtatgttcccagtatgtttgatcattcgatggataaagctgatttcagcaccaacccggaacagatcatcatggggcgggagtcggagagggagcagcagcagaaactggtaaaagtgatcaaccagttgccacgccggcagcaggaggtattgcacctgcgttatttccagggcctggatacaaaggaagccgccgcgctgatgtcgctcagcgtgaatgccacgtatgtgctgctgtcgcaggcattgcgctttctcaaaaagcacagcgacaaactggttaccctctttttattatggccattttaatgagtgtttaacagacaattgaaaggcggcaaaaaaaaataaaaaaaagtggcgccggaacgctaagattttaacaccggtttactttacactataagtattgaagatgagattcagggaattcactatttcagattttttgcaggaaccttctttccggagctgggtgctggataacaatgccaccgccaccgctttctgggaggaatggatgggcaataatccggataagcgtgaaaccgtaatgcaggccaggcaatggctgcaggtaataggttccccttcctgggtacctgatgctgccgcagaagcggatacctggaaccgtattgaacaaaccatcgacaaaacagaaaaatcaggcaaaccgggcatttttgccctgcagccggtaatgaataccattaaaaacaggagatggctgccttatgcagctgtattggccggtattgcagttttatatgccgctgcttttttcctgttctccggcggggaagtacatcaggctacccaaatgggagaactgaaaaccatcctgctgcccgacagctccgagatccggctgaacgtgaattcttccgtgagatatgcggagaaatggaatgcaaaggatgcccgcgaagtatggattgagggagaagcattttttacggtaacgcataaacacaataaccagcgttttgtagtgcatacgcgcgacatggacgtacaggtaacaggcaccgcttttaatgttaacacccggcgggtgcaaacacaggtagtactgaacaacggcgtggtgaaactggcgctgcgtccccgcggaagcgatacggcagcatctatcatcatgaagcccggcgacatgatcacttactcagccaccaccaatgagctgaccaataaaaaagtagacccggaagtatattcttcctggcaaagtaaaaagctattatttacagatacgcccattacagaagtcattaaatccctgcaggataacctgggcatcactattgagctccaggaagaaagcctcggcaggcaaacatttacaggaacagtacctacagataatgtagaagtatttttcagaacattatccagatcgttacaggtaaccgttacaaaaacgggcgcccggacatacaggatcaaccaacaatagtatttgaactgacataataaacaatgccctgcccgccgtatccgggaaggggaaacttatgcaccgatgaaattataatcagccataataacgaggtaacaattattcaaccaacctaatctattgctatgatagaattttacgccaggcgtgttggcggaagcatggctatggccctgctgatacagctttgtgtgtcgccggctacagcggcgcctttgcaccgtcaacatgatgtattgtatgccactgcccgcccggttacacagcagcagccacttcccctgaaggaagttattgcgatactggaagaccggtataagatacgtatcaactatacgggcaacaccatcaaagacctgaaagcaacggttccttcgccaaaaacagcatcggttaaaatgcaggcttacctgcaacgcctgatgcagccactaaacctggaggtagaagaagccggcgcggataattatatcatcttccggaaagatgcgcctgctccgcctgcttccgcaccgaagcaacaggcgccggttgcgaccccggcagcagctgtagtaaccaccgcccctgcaccggtgcaggaggtacccgtgcatccgccggtgaaaggacaggtaacgcaggaagacggtgtgcccatccccggcgtcactatcgtggtgaaaggtacccgcaatggcgtacaaaccaacgcagatggccgctttgaactgagagacgttcccgataacgctgtactggtttttagctacatcggctttaaaacacaggaaataaaagcaggaaaacgtacttccatttccgttaccctgctcaccgatatgcagtcgctgaaagatgtggtggtaaacggttatcagaatatcaagaaagataatttcaccggatcggctattactattacgggagaagagctaaaacgattcaacccccagaatatcctggccagtatccaatctttcgacccttcttttaaactcgtagagaataatttctccggttccaaccccaatgcgctgcccaacatcaatgtaagaggcactaccgcattgcctaccggcaaaaccacggaactcacccgcaaccagatcaacagcacacccaacctgccgttgtttgtaattgatggttacccggttccggtgcagtcggtatacgaccttgatcccaacaggatcgcggcagtaaccctgctgaaagatgcagcagccaccgcggtttacggctcccgtgccgccaacggcgtactcgtgatcactacccgccctccgaaagaaggcaagttgtcgctcacctatggctatgaactgaatgttaccacaccagacctcacggcatataacctgctcaacggcgaacagaaactggaatatgagcgactgtcgggagtatacgaaaatgcattaggacaagggcaggacgaactgcagatgcagtactacgccaaacggaggaatgtactggcgggtgtaaatacctactggctgtcgcagccacttgccaccgattttggtcataaacattccgtgacgctggaaggcggatcacagtcgctcaaatatattatcgacggccgttaccaaaccaatgcaggagcgatgaaaggctcgggacgcgaccgttacagtctcgctaccaacctgcaatacaacctgaaagataataaggtactgttccgcaaccagtttaccatctcgcaggtaaacggccgtgaatcgccttacggggagttttccacctatgcgcgcatgaatccttatttccctaaaaccgattctaccggcaagctgctgcgggaactggataaatggaatgtgccggattacgcaaccaatggcatgaagctcaacaccgtgctgaaccccatgtatgaagctacccttgccagcttcaacaaatcagaatacctggagtttaccgacgccttttctgctgaatataatatcaccaatactttaagactccgcggagacttcagcttaaccaaacgccgctctaccgccgatcagttcatttctccctatagcaacgacttttttgataaaaccggcgacgacctgaaagaccgtggcagctatactttcggcgttcgtgatgagatacagtacaatggtaacctggtattgaattacaacaaaggaataggcgatcacttcttcaacacttcgctcgggttgaatatgcaggacgctaaaagttccctgaaaacctttaaggcgcaagggtttaccaacgaccagtttaccgatatcacctttgccagaacctacgaaaaagataaagcgcctaccggcgaaacttatgaagagagactggccggcgcttttggaagcatcaactactcttatcaaaaccgcctgctgatggatgccacgctgcgggttgacggatcttccaaattcggggtagatgcacgcatggcgccgttctggtcgtacggccttggatggaacctgcacaacgaaaagtttttgcgtaacacgattgtgtcgcagctgaaactgagagccaccaccggtttaacaggtgaagtatctttccctgcctatttgtccaatactacttatgagtattataccggcgactggtactctaccggcgtaggagcgcattttaaagcgtatggcaactccaacctgaaatggcagcgcacacaaaactacgacctgggtgcagaactcggcctgttccacgaccggttgtatgtagcgccccgctattattataaacgcaccaaggatctgctggcagatatcaatgtagcgccttccaccggtttttaccagtataaagagaacctgggagaaatggtgaataaaggatatgagtttaacatccgtgggaatgtataccgtaaccgcgatatgtctgtaaatctctgggccaacatggtgcataataccaacgtcatcaccaaaatatccaatgcgctcaaagcctataacgatgatatcgacaagcaacagaatgaaaaagatgaattgaaatctttatcgctgctacgttataaagaaggccaatccatgaataccatttacgcggtacggtcgctgggtattgatcctgaaaacggtaaggaaattttcctgaaccaggatggctccaaaacttatatctatgatgtgaaaaatacggtgccggtaggggatcaaacacccaagctggaaggcttctttggcggcaacgtggtgtataagagctggatgctggaagtgagcttctataccaagtttggcggcgactactacaaccagacgttgctggaccgtgtggaaaatgcagatcccagatttaacgtagactcccgcgtgctaactgaccggtggaagcaaccgggagatgttactttctacaaagacattgcggatcagtcgctgaccagggcttcttcccggtttgtacaaaaagaaaacaggctggaatttaaatcgctgtatctctcttacgaagcgcctgcagcattctacaaccgtttgaagatgagaagcctccggctttccctcaatatgaatgatatcggctactggtctaccgtagcggcagaaagaggtattgactacccgtttgccaggagcttcactttctcacttcaaacaaggttctaaaatcattatatatgaagaagtatttagtcctcattttattactctccacttcctgcagcaaatggctggatattaaaccgatttcggaagtatccggtgatgagctgttcaaaagcgaagatggctttaaagatgctgtgaatggcctttacagcctgtgtttgaatgaagatatttatggcaaggagctgatgggtggtttgccggatgtactggcgcagaactatgcgatccctgttctcgacggggcgggttaccggcaggcatccctgtataactataaagataaaagcctgatcgacaggaaaggcaggatctggcaaagactgtatgaagtgattgccaacagcaatttaattcttgctaaagtagatcagcaaaaaagtatcctgtcgggtgttaactacggcctgataaagggagaatcgctggccatgcgggcctggtgccattttgatgcgctccgcctttttgctccttcctttgccagcatgccggccgccagaggcgtgccttatgcaacagagttttccaagaacgctgccgcgatgcaaaccgtaactgcgctgctggattctgtgatcaaagatctcactgcagcaaaagaaatactgcgtggagtagaccctattttaaatgcgggttataaagtaggatatatgatcgcggattccagtaccgaagccaatggggaaatgtttgcgcagcagcgccggcaccgtttaaattattatgcggtatgcggcgaactggccagggtatatctctataaaaaagacccggtacacgcattacagaatgccctggaaatcattaatgccaataaatttccgtggacccggcaggaagatttcatgaatggcaatgatgcaaagaaagacaggatcctgtataaggaactgatcttcggcttttatatgcctaaccggaaagatgccatgaatgacctgttccggaaaggcaccggggaaggattatttatttccagtacagaaggtaaaaacatctatgaagtagcaggcgtaggcggggaggatttccgctttaaacagtggttcagcgaacaatccgttaacagcactacttatctgcaactggaaaaatacaagcgcacagatgacaatcttcattacctgatggggcctgcgttacggctcagtgaaatttattacatcgccgcggaatgcacttttgctactgatccggataaggcatgggcatatttcaatgaagtacggttacaccgcggtatcgggccatatagcggcccggcagataccaacagtttttatgccgaactgctgaaagaagcgcgcaaggaattgtatggggaaggacagctattctacatgtacaaacgcctgaacaggtcgatagtgggattaggcggtaagccggtgccaccctccgatggcgtgtttgtactgccgcttcctgatgatgaaatcgcatacggtaaccgataaaatatcacacatgaaaaagataatagcgacaggcatgttcagctggatactgctgatggcatgcaaaaagcaggatgatctggtgttccgtgagaacaataatgtttattttgattttacagattatataaagaataccaggatagacagcttcttttattcctttgcgctttttcctgaaaaatcgatagatacgcttttactgccggtaaggatttcgggggaacgggcatcgtacgacaggtggttcaaagcacaggtaatagctgagggtactactgccctcgtgggattacattacaaaatgctggactcggcctataagatcccggcagattcaggcaggacttttttgccgctgatcatttccggcagcgatccgctgttgctcgatacctctgtggtgattaaactgaagcttatggcttccagtgcatttggcaatgacttcccttcctacgacacggctaaggttactttttcaaaccggctggaacagccgctgtggtgggtggtatgggaaagcgaccttggtgtttattcccgtgtgaagcatgaactgtttatccgtacatccggtaccactgaattacagctggataattccgactggcagtctactcccaaaacattgttttacctgcggcagttccgcgcgtttatgatggatcctattgcccgtgcggccgactataaggataagggatatgctatcgggcaggaaccggacggtacttattatttctacaataccggtaatcttaataaaaaatacccgctggaacacagtactgcagacggcaggtattatttccatgatgaaaacgggaacaggattgtaccacaataaccaaaaatctatacgcatgaaacatgtatttctatatatcattggcatcctggtattatttaccgcctgctataaagacaaaggcaattacgattatcacccaatcccggagccggtgatcacaaagctggataccgcttacatggcggttgtaggggatagctttatcatatcgccgaaagtggtgctggcctccggcaatacaaagtaccagggattgtggaagatatccgttccgggccagatggggacgcaggattataccggccaggagctgcgcattgtatttggtttgggcgcatcgcgttaccccgcagtatacattgtgtacgatagcattaccggcatgaagtactattataaatttgtgatcaatggtaccgctacttttacacgtggtacggtggtgttgagtgatgatgtaacgtcttccaaaatatcttttattaaagaagatgggacagtacaagccgacgtatataccaatattaatcacgatacccttcctggcggcgcattgcagctaaccatgatgaagaatgttaattatggcaatctcattaccggctactgggctacttttaaaacaggcggcgtttatattgatcccaataaccttggaaagataagaaccctggcgaagaatttttattctgatccgggtccgctggaggtatctacttttatcccttcgagtcttggtgtacccgtgggcatcatcaataaacaattataccgcggcgctacagaaacagctccttttgccacctattacggctttatgggcatcccgctttccggtacctatagcctgtcgccgtctattattgccagtgatcctgataaccgcgggtattttgtgggttttgaagaaacgaagcggaagatggtgcggatggattggggcaattatcttgataccaattacattgtaaaagattccgcttttacaccgaagaacctgaagatggatatgttgcacctgggtcgtttttcagataacgtatgttatgcgttctgcgacagtgcgggccagatcagggaactgcgttttggcgtggagttcagaacaggcagcgatcctgtttttcatgcgctggaaaaaaggaagccggtgattgcggataagatcagtgcggccacgctttgggcagagtcgccggtgggtgtattttattttacccaggcagataaggtgtaccggtataacccgttgaataaagatgtaaaggaaatggcttcttcattcggcgggcaaacgatcactatgctgaagttgctggaaaatggcaaccagctgctggtgggagtaagaggcagtattttttacctgaatgtaggcacggggcataatggtgaaaccacaaagagggtggatggtattccgggagcgccgaaagatgtgattgtgagagcgaattaatttgcataaaaaaaggaaggtttaaaaccttcctttttttatgcaaattattccccggtccatttatcccggtcgtccatactgaatttccaaggggccatattattttcgatattgctgaacatgccggtccattctgccggggcgctggattcttccattaccaggtggcggcgcagctggaggataatatccagggggttgatgctcacgggacattcctgtacgcaggcgttgcaggtggtgcaggcgcgcagttcttcttctaaaatataatcgcgtaagagggctttgttatcatctttaaaggtgccgccattggctttgatgttgtggcctacttcttccaggcggtcgcgggtatccatcatgattttgcggggcgacagcagtttaccggtgatattggccgggcaggcagccgtgcagcggccgcattctgtgcaactataggcatccagcaaatttttccaggtaaggtccattacatctttggcgccgaacttaggcatggtatcggaggcgggcgcgttggcagccaactccggttgcagcatcagctgtacttcatgctgtacggagggcatgttttccatttcaccttttggttccaggctggcgtaatatgcgttggggaatgccaggataatatgcaggtgcttggagtaaggaagatagttcaggaaagcgagtacgccggcaatgtgcagccaccagcagctgcgttccagtacttccagcgagccctcagacatgccgctgagcaggggcgcaaacatccctgaaatccagaagttgccggtagccacataatgtgaggcgcctttggcctgtaaagcctgatctgcagcgttcatagtaaggaacagcagcatcagcacaatttccgtgatcaggatatagttggcatctgagcgcggccaccctttgagttcgcgggccataaagcgtttcagcttcaatatattcctgcgtatgaggaagatggcgcagccggcaatcaccagcacagccagtatttcaaataaaccgatcagcaccgggtaaaccgggcctaatacgggaacgaataaacgatgtgtgcccaggataccatccaggatgatttccaggatttcaatgttgatgatcaggaatccggcatatacgaagaagtggagtacagctaccagcgggttacggaacatttttttctgaccaaaagccagcaacagcaggtttttccagcgttgatccggatggtcgctcaggtctttatcacgtcccagtagtatgtttttccttatccggattgctttttgggcaaaaagatataccgctgttccgaacaggatcacaaataataattcttgtacaattcgcattagctcagatttgactccctaatttatgtcttttttagctatcagccgttaggggttaaggtttagtgtatttgatttttttgctaagtgctaactgctaatggctaattgcttatttttgcaaccatggaaagcaggaacatcattctaacgcaggatatcattcaaaagaaaattgagcgtatcgcatatgaaatctatgagcataacagcgatggcacggatatcatattagcgggtatctgggaccgtggcgtgatcatagcccataagctggctgctatcctcggacagatatcccccctgaacatccatattattgaattacgcctggataagcagcatcccggtgaagtagtggtatctgaagaaattgacttcaataacaaagtgatagtggtggtggatgatgtggccaactccggccgcaccatgctgtacgccctgaaaccattgctgaaatatctccccaaaaagatccagacggccgtgctggtagaccgtaagcataagtcctttcctttatccgttgacttcgtaggatattcactggctaccaccctgcaggacatggtgctggtggaaatgaacggcgaagagatcatctccgcttatttcgaataaggcgttaaaaataaaccgcgtgtaatttcatattcccctttgagttgatttcaaaggtgggggcgggaaacttcagcatattcaatacctggaatattactttaacacccttttttcgtgtgggtattttcgtgaaatccacatcaggggaaagataaaactgccgtacacgctgtagttgactgtaatcgtgaccgatgccgcgttcgtctgtccaggtgttatcgcggccacccatcataccctgtgagccatatcccacggcaatattcagccatttggggagccggctttctttccggaaggagtagaggtttactgacagccagtaggtttgaccgttataatctttcagggttctttcccagaaggtggtgccaaagagttgatctgccttgtgctgtagtaccgggtcatcgtaatgttgcggatgtgctgagaacttcagctggatgcgttgttcattccaggccagttcctggctgatgagcagggcggagccgatggcattggcgcccatatcaccccaggaaaatccccattcagccgagtagccatccagtgcctccacaacggactggtaagcaaatccgctcaggcccccgatccagatctgtttttttcgtggaagccccgaccagcgccacatttcgcggctatatttaccgatgaagtaagcgctgaaaatatgcccggctttatccacctggttccattctcccatatcattaaaaaaatggaatcccgacctggggtagcctttgtaccaggcggtattgagtgctgccagccccgcgccgtaaagggctgcggtggtgccgctcaggatccatacgcgtgatgggatggtggtatcaggaatagtggaaaaaggcacctttttttgtgccatgctgctgaaaaacggcagtaacaggatcaggataagcagtggctttttcatgcgggtagctaaacaataccgggaatgctgaaagggggaaattccggaggagtcctttctttcaacattcccggcttttatcatcttttcagatgacgggctttatttcagtttcagatcctgaataatgccatttattttctgattcagttcagcggtcactttgtcgtagtctcctgcactggccagtggtgcgtttacgctgaagtagaacttgatttttggttcggtaccggagggacgggcagatattttgctgccatcttccaatacaaactgcagtacattggatttcgggagatccagcgctttggtgtcgccggttttaatatccctgatctgttgcagctggtagtcgtacagcgttgcaaccggtgatccgttgatggtaaccggtggattttcgcggtatccgcgcatcatttcggcgatttcttccgcgcctctcattccctttttggtaatagaaatcaaactttccatgtaatagccatagcgtacatagatgtcgatcagctgttcaaacagggatttgccgtgactgcgggcataggccgccatttcacagatcatggctacagaggcgatggcatctttatcgcgcacattctgaccaatcatatagccataggactcttcacctccgcagatgaagttttcctccggctctttacggcggatcaggtcagcgatccatttgaagccggtgagtacgttatagcaggtaatattgtttttggcagcgaatacatcgatcaggtcggatgttactactgttttggcaatatagtcgtttgctttggcgagtcctttgcttttgcggctttccacgatgtagttaaacagcagtacgccggtttggttaccgttaagcaggatccattctcctttgaggtctttcacggcaatgcctacacgatcggcatcggggtcggtacccaggagaatatcggcatcgagttctttggcttttttgaggccgaggctcatggcttcggattcttccgggttagggtacactacggtggggaaattcccatccggcgtggcctgttcctgtacaatggttacattggtaaagccgtattgttccagcagctggggcacctgggtgatgccggtaccgtgaataggtgtgtatactattttaaggtcgtgctgttgtttgttgatatcgggattgatggacaggctgagcagttccttgcggtaagcttcgtctatttcctggccgatgagggtgatattggcttcaccaccggtccattttacctcatccggggaggcgatgttctctacttcacggatcacgttgttatcgtggggcggcaccagctgtgcgccgtcgttccagtaggctttgtagccgttgtattcctttgggttgtgggaggcggtgagtaccacaccaccctggcaacgcaggtgacggatggtaaaagacagttccggtgtgggacgcaggctttcaaaaagaaataccttaatgtcgttggcggcaaaaacgttggcaacggtttctgcgaaaaagcgggcattgttgcggctgtcgtgtgcaatggctaccttaatttcgccggtgaaggtttttttgaggtaattggcgaagccctgggtggccattccaagagtatatttattcatgcggttggtgccaacgcccatgatgcccctgaggccaccggtaccaaattcgaggttacggtaaaaggcgtcgttgaggtcatcagggtttccttcctgcattttcttcagtgtggcaacggtttcagcgtcgtaattaccgttgagccattgcgctactttgttttgaatatttatatccatggtcttttttttgtgagccgtaaatgctaaaatggattgtaaagtaaaaataaaaaaatgaatgttggaaattacggatttcaaaatacattgaaaatcccttgtattggttaattttgcggccatgaggcggtatgaagatacttataaacaaaaaggattacgtaaacagttagtcgatagtatccgtcagaaaggtattacagatgaaaacgtactggcagctattggcaatattcccaggcattttttcctggatacggcttttgagagtatagcctacgacgaccgggccttccctatcggggaggggcaaaccatttcacagccgtatacggtagcctatcaaacgcagctactggaggtaaaaccttatgaaaaagtactggagatagggactggcagcgcctaccaggcctgcgtactggccgagctgaaagccaatgtatacacgatagaacggcaacggaagctgtttgaccaggtgaaaagttttcctttcaaagcccaatatcgcaatcttcgtttcttttacggggatggttatgagggattatcgacctatgcgccctttgataaggtgctggtaacggcagctgctccgcatatccctgaaaaattactgcaacagatgaagatcggcggcaaaatggtgattcccgtaggcggacaggatgtacaacgtatgctgcggatcaccaggatcagcgaaacggagactgaacaggagctgttcgacaacttctcttttgttcccatgctggccggaaaaaaataatgcaggggtgatgatacccctgcactgatatgatcctgcctgattttattaaagccgtccggcgccctccctgggcttttcttcttcctgtttttcttcttcttcctgtggtttctttttcttaaacaggttcgggtccattttgccaaagcggtaacgcacattcagccggatgaagcgggtagcccttttacggtcgtagtcctggatgaaggtatttgtttcgtaatgtgagctgaactgctgtgtattcaacagatccgagatattgagggccactaccagcgatttgttcagcaattccttgcggattcccaaatcaatgccattcatggccttgaaggttccctggggctgaatgcggggagagcggaaatgaccgccgagttccacactaaacttaccgggtaaacgaaattgtgtatttccatttaacccgtagctgaagttttcgttattgacggcgatgctggtaagcttgctgtactccacattcaggttggcccatactttccaccatttggtaagattcaggctgtaagaaacattaccgcccatattctgctgggtggccaggttcatgggtttggtagtggtaacgccggaaatagtgtccagtgtgctgatacggtcgatattatcgtttgtttgcgcgaaatacgtactggtgctcaggtaattattggacgacgggtagtataccgagtagctgacctcaaacttatgcgacagtgcaggctgcagctccgggttaccggtacggatattctgcgggtcggagttgttgatatagggcagcaactgatcaaagttgggccggtctatccgggtggaatagttgaataccaggctttggttctggttcttcggcatattatatttcaggaatacacttggaaacaggttaaagaagcggttattcaccgtggtatcttttgtaaacgagtatcctttgagctgcgattgttctgcgcgcacgcctatctggtaaccgaggttgccgatggcattggcgaagttgagatagcctgcataaatgtcttcttcataatcatatttattcgacagggtagggctgatcacataatccttgtcgtcccagtcgaacagcgtagccacgtaattattgtcgatatgccgcatagtagctttcacgcctgcttccagcttacctttctttccaagtggggaagtgtagtctgattgcaggttccagaagcggttaccattttttcctttattgctttgtttgtcggcgttgggaagtgtatctactgaggcaatgtgatattgggtattgtagttactgccgctgctgctgttattaccgctgtagctgatgtaagccgtgagttcctggttgggcttttcaaaggtgtgtttataactgagattggtatttttattattgctgcggttgtagctgttattggcgcgctctccgttacgcagggattccattttctggtccatgtagttcaggaggatattatcttcattttggctgtggccaaagttaagtccctgcgacagtgtgaaggtattgtgatcatccatgaagtaatcgaatccgaagcggccgccgttattggtgttcctgttttcatttttactgttctgggagaagaaccaggtattgctgctgtctgctaccaggttttggcggaagcttttcccgctgccgtttacctgttcgtagcgaccgttgtagttgccgaagaaattgaaccgtttcatgcgcaggcttgcattggcgcttccgaagccttccccgcgggtggcgccgcctacgttgaacataacgttatagccgattgctttatcttttttcagtacgatgttgataataccgccgctgccgttggcttcaaatttcgcagagggattgttgatgacttccacgtggtcgatgctttccgcgggaatcatttgcagggctgttttagcatccccgaaaggagagggtttaccatccacataaatagtaacacttttaccacggagcgtaatgttatcatcgatatccacatccacgctgggaatgttttttagtatatccgttcccgttcctccttctgcgttaatcatgttaccggcatcaaatacctgccggtctatttgcatggagaacgctggtttttctgctttgatttccaccgcattcagcactttaccggccgattgcaggcgaagtgtgccggccagtgtattttttcctgctgttacccgcactgccttttccagtttttcgtatcccataaaggtgatgcggacaacatagatgccgggtgtgacattattgagtgaaaatgtgccggcgggtgtggtgtaagcgccggtaaccatggaagaatcggcttgatttagcagtaccacagaagcgtattcaatgggtttcccggtaacaatatctactacctttcctgttaccttcaggctggcagaaatgggcgtttgtgcgttagcgttatacgacacaacaaacagcacgaccatgagtgaaaaaagatttcgcatgcgtggacttagcaactttaataatgatacaacaacagcgtaaaagtaataggcgtatgtgtaaacattcacgaaatatgatgagtggtagctaaaaaaacatggccggcagagtgctgtaacactactaaccggcctgtggtttgcattcaccttctttaatatgtttttagaaactctgcatgggatcgcccatctgcgtatcgtttccggagtcttttcttttctttttaaacagcgatgcatcaaacttaccgaagcggtagctgaagttgagtttcagtatcctggattcacgtttgcggatataatcctgtgcaaactccggtgatgcctggttcagttcatactgacgggtattgaaaatatcggataagctgagtgttaaagaagctgctttatttttcaggaaatcttttttcactgccaggtctactgtgctgaagcctttgatggtgccttgtgcggagctggggatctggttaaatccgccgcctccgccaccacggccgcctccgccaccaccgccggatgagggcagcgcaatggtgggcgcctggtaagtggcatttacctgcaccgtgaagttggccggtaattttgtttcagagtttattttggcaaaccagctaaagccgttattatcatagttctggccattggcgtttaccttcatatctgtttgatagaagttcacgttactggtgagatcccatcctttcaggatttgattcttcatggtcagctcagcaccataggaattgctcctgttggcattgatgtattgtgtgagcagcgtatccgcaccgatgggcgtgctgatggtggaaatcatgtcgttggtattcctgaaatacacgctgccgaggaagttgctgttagcccagttttttacatatgaaaattcaaagctgttggtatattccggtttcaggttgggattaccttcccgctgattctgcggatcgctgtaatcgcggtaaggaatcagctggaagaaattgggcctgtttacacggcgggaataattcagctgcagttcctgatcgttctttaatttttcggagaggaagaggctgggaaataatcctggtaccgctttggtgggtttatacttagtgccttcattttcgcctgcgtacacatattgttccacacgtaagcctacctggtagccgaagttgccgatggtgttggcgaagttggcgtaaccggcatagatctcttcgttgtatttataattgttggagagctgcggattgttgataaactcgccggtagtggtatccctgtcgtatacgttgtatagactggtataatcgcgtaaagtagctttggcgcctacttccagcttaccgttctttccgatgggattggtgtaatctgtttggaaagtaacaaaagtggttttaccgttggtggtgttattttgcagcaatgcctgtccgagcggtgatccatcggcgttttgcgcctgtgtgagatagtcgccgttgcggttgtttttgctgttgttataattgatatcagcggtccattctttattcggttgtgcaaaggtatgtttgaaactcagtgcagtggtgtagttgcggaagctgaagttattattgttcaggcggtcgctgatcccggttaccacgtgattcttgtcggagaaggtgcttcgcaggtcttcgttgtttttaaaatcgccggctacaatattttgtgagatagagatggtgttcctgttatcgagcatatagtccagtccgaaccgtccgaattgaaaggttggtttgctggtgctgttgctgttctggaagaggaagttggtgtctgccttttgaccgttgctgtagttgctgcggctggtagtaccatctgcccagttctgattggcattgatattatagttggcgaacacattgaatttgccttgccggatattaatattgccaccgccgttatatttgttaccggtaccaatacctgcgttcaccgcgccattgaagccggctttgcggtttttcttcagtacaatattcagtatgccggacataccttccgcatcatattttgcagaggggttggtaacaagttcaatactttctatagcatctgcgggtatctgatcgagggtaagtgtagaaggtttaccatctacaaagatgttgggagaagcattacgcacggtaacatttccatcgaggtctacattcacggaaggtacgcttttgagtacatcctgtgctgttccgccaacggaggtgaggttcctgtctacattaaatatttttttatcgatacccatggcgaaggcacttttttgcccggtaacttccacgctttgcagtgtttttacattctgttgcattttgatattgccgagatcctgttctgtagcctgcggggtgatgattacttttttctgcatgctggtgtagcccatgaagttgacgcgcagtatcatggggccgaatggcaggctttcgaggctgaagtcgccattgggtttggtgagcatacctgtcaccagtgaggaatctttctgccttaataaagtaacagaagcatattctattggtttccctgtttttgcatccaccagtttgccataaagatggccaatctggggcatgttaggtcttccctgttgtccctgtccttgtccttgtccctgccgcggggctgtggctccaggcgcctgtgcaaaggtgtgcgcctgcaacaaaagtataccagcaagaactgcgtagcattttttcatccttatcgttttttatccggactttcttctcagataaggacaaatgtatcggggtacaggtatgaatggtttaagattgtgatgagtggaattattatgcgcaggaaatcgcaaatataagcgctaagaggtcttaacagtagttaacagagctgtgtttcagcggattaccaaagggtgatgaccatacaaattaacccggtaatcagtccgctgatagcgccgaggagtttgaaactttttagttccctgctgaggaggttatgtgtaatggtttccagttgtgctgcagagatacctgcaattttctgtgatatcattttttccaggttcaggtcctgttccacgttatcgaggtattggcggatcagcacgggaaagagggtgtccagttctgctaccaggtgggtttttatctggttaacaatactatcgccaatgaacatggacagtacgggcattgctttggggagccgttcccgcaggaagctgtccaggtgcgcttctaccagtggaataatttttttgatcttttccggatctgtcatttttgttttgatatcctcaaaggaaaactgttgcgctaccagtgtcccgatgctgttggcgaggtgtgtttgtcgttttggaaacaatccctgcagggtgataaagccgattttaacgggtttatacgggcggaaaagcagggtaagcgccaggctattgagtaaccaaccgatgacagcagcgatgaggggaaggaaaaagatcattgaatgaattgattttcagctattacaaatgtaaaaaattgggagtcaataagtaaatgatttttttgtgcagataaaagagaggtgacggaatggataggagaggcgatatttacaaataaaaaaaggcttctttttacagaagcctttttcgttttttgggtgattgaagggtttcgaaccctcgaccctcagaaccacaatctgatgctctaaccaactgagctacaaccaccgttttatctttagtttcgtattatttcgttgttgggagtgcaaagataagtgaaactatttttaaattccaaatacttcagaaaaaaaattttcaagggattatatattgatcatattctgcagatgaaacccaatattacaatcgttttcatttgttaaaaaggggcggtcttaacattaacaagcggcactattggaacttacagaaaaggtgtatctttgcgcactttcccattccattcccatttttataagtgattaataatcagtaggatgttattttacggcatcaaagaaatccctgatttcaggcgatttagtgcccttagtccggataagttaaccaagacaggaaatatttaacaaaatcccttttactactgactaaaaacaaaacaagtatttaatatttaactgtatatacatatggatcagcttaaactgaagttgcaggagtactatcagcgttaccagcaaatggaccaacgggtgaagcctggaaaggaggagcctggttttgaggacgtgctggacatggaaaacgatattctttcacaatttggattgcctacatcccggcgttttgtgcagatactgcatgatttcgtgcatcatggtcatgtgagtgaccagttactggattatgtgagtaaaaaactacgtacggccgcacgtaagtatctgttggcgcctgttatgtcggacattgatttactggaaagcgcccgcgaacaaaaacgcagcgcatatgatgtgttgcccgaactgggctacccggcacacgaatacgccttattcctcatcggagagcttttttaccgccgcaatatggctgccggtgatatcctcgatgaattgaaaaagatgcagcattttgatagctggaacgacctgatgctgctgagtaaaatacataatcatactacccacgaactgtacaccaaactgaagaaacatgaactgcgctttattgatgagttcattcagtttacccgccgccaggaaccgtccaggctggtgaataaacgtgctacgccgttggaagatggttatacgcccaactataaaaccattaccaaagtacaggtagaagatatcatctttgatgaacaaactacgccaagcctgtttggtaaaataaagagtggcaggggatacgcccgcatcactatcagcctggaattttcagagctgaaccagatccttatgagcagtgatgaactgggtgttgaaatcagcaatcatattaaaaagcgcctggccaatccggctgcagagaaaccaacggtaatagatatacgtgccgaattcggcgatgtgctgaaactggataactgctacctggaagtgtataaaccccagcacagggaaggcaataaatgggtagaagataaagaccacttctacttcgtggataaaattcttactaaaaaagaatttgaaaagagaaccaaagaagcagaagtaaaacgtaaaatacaggaatgcctggaactgatcggcggctcttatgtatattaccagcgccttcgccgtttaggcatcaccgacgaggaagccaaactgcgcgcaggtttacaggacgagctgttgttcaagttatcgtacttccttaacaaggtaaaagaataacgcgtaagcggaggttgtctttctcaggattacactgattatattgatttagtggatttgaccactttggattttaaatgatttggggagatataagcggatatttttgcttatgtctccccaaatcttatttaatcctttataaaatccaaaaggtaaaatcaaagtaatccatgtaatcagtgtaatcctgagaaagacaaactccgcgaaagacaaactccgcggaattatttatgtttacgtaaaaaagagatggaagaacttactctcggcgttggctcccgggtacagcacgcacattttggtcccggtgttattgttgctgttaaatatgcccagtaccgtgttacgtttatggatcatggtattaagatgattgataaaacggatccattgtttgaagtgctggtggcggaaaatgcgaccgcggaagtggaaaccacttcagatgtggaaacatcgctgctgaagatcctacgcctctggggcggtattgcggaagtggtgccactgggcgaccgctggaagggcggcaacctcattcttcagcctggtgatactaccctgaaagcaaaggagttgcccatcgataccttcttccataaaatagtgatgctgcgcgaccgcctccgtgtactggagcaaaacattaacagccacaaagtactcaccgacgaagagaaggtgaacatgcagcaatatattacccgtatctatgggtcgcttaccacttttaatgttttgttcagggataaggaacattggtttaccggcgaaaaaagcggcaacgattagtgggagtctatatgatagatctgctccagttcccagcggtaagcctctgggagatgattgataaagatattttttccatcaaacgggaacttctcatcgtaaccttttacgggatataagatcaccggtgtacctgccggggtatagttgtgactggccacaaaatccggttgctgatactccggcagtattttttttacccgcttgtacgccaggtttcccaatacccgctgcatgcgcctggaagcccttttggagggccggttcagccggccgtacatataattcaatgcaccccgcaccggccatttctgctcctttaatgcgcctttaatatcggtaaagggattcacggtattgaagtcgtgggttgtttgcaaagagaagggcgtttccggcacccagtcgcgggcattcactacccgcaatccccacccatcgcggcaaataaaatcgaagtcgtatgcgtaatacaggttgcctggtttgggcgctgcactggcatatgttttaaaaacaatatccttcggcaggccgatagtatattgaaaataagaacgcattaaaaaagaaatggcgcctccctggctatgtccgaagatgataaattcgtgtatgccttgctggtagtattcgttgatcttctgttttatttccggtcccatagcagctactgccagcatccacccggcatgtacatatgctttgggatcttccgccactttataggggacggccgtgctgtcgtttaattgcacagtgccctgtgccggtatcatgccggcatagaaattttccagccaggaaggcgctgtgccattggtgccacggattacgatgatgccaacattgtcttttcttttccacagatcccagcggtttaccaatcctgattcgggagcacggtataccagctcacaatcagcaggcggggtactttttattttggtccacggcgtatccctggtgcgttccgccagcttcagcaactcactgtattcagcggcattgaaattgggcaacaggcgctgggcaaaacaattacttcttacggaaaataaaattagaaaagagaacagcgaaatacgaaaccccatagaaaataacaaattataaatgaccaatgacagacgaacagtaacaaaagtgctgcactttaagataaaataaaacaattgaaatgctttcattgttctaaatccgtttaactttccgacctaaattactttaaatatggcaaagagaattgagcacgatttcctgggagaaaaagaaataccgcaggatgtgtactatggtattcaaacccttcgtgcaatagaaaactttcatattaccggtattcccctcaaagtggaacccatgtttgtacaggcgctgggttatgtgaagaaaggcgctgccatggccaaccgcgacctcggcgtacttgataaaaacattgctgaatacatcatcaaagcatccgaccgcgtaattgccggtgaatttaacgaccagttcctcagcgatctgatacaaggcggtgcaggtacttcggtaaacatgaatgccaacgaggtaattgccaatgtagcgcttgaaatgatgggcaaagaaaaaggacagtatgaattctgtcatcccaataatcatgtgaactgctcacagtctaccaacgacgcctatcctactgcattccgtattgcgctgatcaacaagcttaccggctataaattaaccctgggtgaactgggcgatgctttccaggcgaaaggagaggagtttaagaacgtgctgaaaatgggacgcacccagttgcaggatgcggtgcccatgagtatgggcgatgagttcaaagcttttgccacgaatatcaacgaggagttgtcgagggtggaagacagcaagcgtctcatctctgaaatcaatatgggcgccactgccattggcaccggtgtaaatgctcccaagggatattcggagctggtgaccaaacacctggccgctatcaccggcctggacctggtgctggccgccgacctcattgaagccaccgtggacaccggcgcctatgtacagttatccggtgtgctgaaacgtaccgcggtaaagatctccaaaatatgtaacgacctccggctgctttcttccggcccacggacagggctgaacgaaattaacctgccacccatgcagccgggctcgtctatcatgccgggaaaagtaaaccccgtaataccggaagtggtgaaccaaactgctttctatgtaattggcgccgatctcatggtaacaatggccgcagaagcagggcagctgcagctgaacgtaatggaacctaccatcgctttcgcgctgttcaccgccattacttatatgaacaacgcctgcagggcgctgaaagacaaatgcgtggtgggcatcaccgcgaatgcagaccgcaccagagatatggtcatgcaaagcattgggattgtcacccaactcaaccccatcatcgggtacgaaaaatgctcagcgatcgcaagggaagcactggaaacgggcaagtcggtgcacgacctcgccgtaaaagaaaagaagtgggtgacccaggagaagtgggacgaaattttcactttcgataaccttatcaggccgcggtttataaacgcgtaggttgtctttcccactgattacgctgattatactgatttagggatttgaacactttggattttaaatgatttggggagatataaacggatataggttttaaatgatttggggagatatgagcgaatgtatccgcttatatctccccaaatcatttaaaatccaaagtgttcaaatccctaaatcagtataatcagcgtaatcagtgggaaagacaacctacgcgctagaactcctgttcaagacggccaacgctgccgtcttcgcctataccttccacgactaaacgaaaacgtttggtgtagtcattgttgtagaattcgaccctggcggtgtgcgttagggtgtctattgctacgttcgggttccagtaaagggtgaggcgtttatccggtaaggcgtgtacttcttttttcacggagtaatccggtgaatagaattgtttcacgatctggtaaccggcttttttatacagtttaaagccacggatgctggggtcatttttcggtgaattgtcgccgccttttttggtgtataccgcgatagcgccattggcgccgccgaagccacccataaatggaggacggaatactttaatgagcgcgatatcctggatagagagggtgctcagcatgctcacatccgactgcatttcattaaggtataatcccggtgcaccgccgcgccaggaaagggtgggattattataatcgcctgtaatctgcaagcctgctactttggattgcaggtactggaatacgttgagtgcaatcggtgtttctttggttaagtcgaaggagtaaccgtcgccaccggagaacataccagatgcataacgtttttcagtagtttcttccggcttcacttttttcgcatttacgtttacttcctgcaggtataccgttttattattgatagagcggtttactttgttgccttctgctgcattggcgaggaattgtttcagtgcgttattatccaccgccggtggtacgcgcagcgggtaaggaattttaatttgtgtaggacgttcaaagaagtggttatcgaatttcacatttacatccacgcctttttttacgaggtcgttgccctggtagtaaatgtaagcggtatcggggaataccatgttggccatttcaaactgtcctttatcgttgatgggagtagaagcaaacatggaggagctgtctatcggcaggcggatgatcatatccagcttaccggtaggcatggggcggccgttgagcatggtggcaacgcctttcatgagcaagccctgttcgtaagggaatcttacttcagggaattcgttattgacgatcttttcccagctgaaacgtctccatccgttggtcatcattaccaggtccaggcctttcagggtggagtcggcgtcattgcggaaataccacgatgggttgtagatataacctttgatgtcggaggtgagcaggaaagtagagatgatgttattggaatttttatctaccggtaccgcgtctgcatctgtgatagctacagagatatttgtttgcatggtatcgggtagtctcagttcaatggcattttttgttcttggttccttgtgggtatctgcatccagtacatctatctgcatcaggtcatttttgcggacgaaggcaagccgttctgcgagcggcatgcctgatttggcaaaaagggtaatttgaataatgcctgacggcagatgatcggcggggataaatccgctgatgcggccttctcctatgtccaggttggctttgtacaccagttggctgcccatctgggcgatgatcacaaggtcattcacggaggtatcggctacgttgccgggtacggcctggtaaaagatgcggctgcctttattgaatactttcagggaggcgccggccgctactgctgcgggcagggccactgttttggtttggcctttattgttttttacggttgcctggaagatgtcctgtgcattggcgggggtgatctcgaaagatcccatgccatcgtgcagggttttgatcactgcgctgttggcgcctttagcgtcttttacagcgccggatacttctaccgggtaaccattgttatcgatggctttaaacgctactacgttcggctggcctgcgatgaggtttccgccttcggggaaaaactgtacggcaaagtcgggtgtggtggcgctatctgcttccggtgatgttttctttgaaggatcaaagatttctatggtccgggtataactgaatgcaggatcgaagttgagcatccaggcggtataagcccttagctggtatacgcctgctttttgtgtttcgggcaggtcgaagttaccgggtgcgccggcgttacccacggcgaacagtttcttttgcacgatgttattgtttttatccagcagctccacatacaggttggtggcggtggtggcgggcatgccctgcagggtgagataggctttgaaccagatggtttcaccggctgcgtagtagtccttatcaagatgcagatatactttttcggccgggtaacggctgccgaaggtttgtaatgcctttataatgcggtcggaccagtcagttgggcgcgtttgtatagccagtgcactcattacgccgcttaacattacggctggtattatccatttcagatgttgtcgctttttcttcaggttcgattgcatgcaatatagtttgagcgggtataatatatgtcaaaaatataaactttggaagattaatcagtaagattacggcaggtttgttattattgcgtgttcaacctacggttttaacaagattttaatgagttcaggaaagaaacgtttagtgatagctggtggcggtgctgccggttttttttgtgcggtgaatgcggcccgcctatgtccgcagctggaagtggtgttgctggaaaaaacaggcaagctgttgtcgaaggtaaaagtgagtggcggcggacggtgtaatgttacccacaatgcccctgatattacgtatatggctaaacgctatccccgtggccagaactttgtaaaaaagtcgttttcccggttctttgttcccgataccatctcctggtttggggaaagaggcgtactgctgaaggcggaagacgatggcaggatgttcccggtaacagataactcccaaacgatcatcgactgcctcctgcgcgaggccgacaaataccatcttaacatccgtaccaatacagaagttacctcttttaaaaaaggcagcaacgggcgctggcagctggaactgcagcaaggtcctgcgctcaccgccgattatttatgcatcgctgcgggaggctatgcgcaggcaggtaagtttgcctggctggaacaaacaggtcacagcattgtgccaccggcgccgtccctgtttacctttaacatgcccggtaatcctatcaccggcctgatgggagtagctacccatgcacaggtgaaagtggccggtaccaaactgctggagcagggtcccttgctgatcactcattggggaatgagcggcccggccatattgcggttgtcggcctggggcgcccgggaactgcagcagctgcaatatacttttaccgccatcgttaactggattccggattacaacgaaaataccctgcgggaacactggcaggacctgcgttttgaatcagggaagcaaaaaatatataataaaaatccttttggtttaccacagcgtttatggcagttcctgctgcaacagacaggaattacggaagagatgagatgggcggacatccccgcgaaagaccagaaccgtttaatgaaattgctggtaggcatggagttcccggtgaaaggtaaaaccacttttaaagaagaatttgttacctgcggcggtattacgctcagtgaaatagagccggctaccatggaaagccggctggtacccaacctgttcttcgccggcgaagtaatggacgtggatggcatcaccggcggcttcaacttccaacatgcctggacgagcggctttgtggccgctagtgcgatagcccagcgcgaaggttgtctttctcactgattacgctgattatactgattaccttgattttatttttggattttataaaggatttaaaagattttattttttggggagatataaagcgaatatatccgcttatatctccccaaatcatttaaaatccaaagtgatcaaatccccaaatcagtataatcagcgtaatcagtgagaaagacaaccttcgcattataatttgaggtagtgcacccccggttcgtactctttttccagcgccagcagcaggtggtcgaagtcttccggttgccgcaggaaatctactttggtggtgtctaccaccagtgtgcgtacgggatgttgcttgatgtattgcatgtacatgtcgtgtacattcagcaggtattcgtcggggatttgctgctcgtaggagcggttgcggtgacggatattttcctgcagtttggtaaccggtgcgttcaggaaaataagcagttcgggctgtaccagctgggggttgatgatgtcaaaaagtttctggtaaagggagtattcttcttccggtaaattgatcttggcaaacagcaggcttttgatgaagaggtaatcagaaatgatcacatcgctgaaaaggtcctgcgactgcaacatttccttgagttgtttataccgttccgccataaagaataactccagcgggaaggcgtattgttgcgggcgttcataaaaaagagggagaaaaggattgtctgcaaactcttccaatatcagttttgcagagaaatgggtagcgagcatgttggccagcgtagttttgccggcgccaatatttccttctaccgtaataaatctatagtgcatgaaaacgggtttaaaattaatcctggtaacggtttgcagctaatgtatccggacagctggctgccagctcccgtacggttttatgcaacacagggtgcatataatccggaatgatttccatcaaaggcgccagcacaaaccgccggagatgcatccgcggatgcggtaccttcagatccggcagcgaatgaatgctgtcgttgtaaaagatcaggtcgatatcaataaccctcgacccccatttctcctggcggatacggccgatctttctttctatttctaacagtgtatgcaataacgttagtgcatccaatgatgtgcggatctccactccctggttcaggtagtcgggttgatccacggctccccagggagcggtttggtataaggccgaggtttgtaccacctctccggctgtttcagcaatcaattgtaccgccttttgcaggttcccggtacgatcacctaaattgccacctataagtaatattgctgtattcatgtatatttcaggactcaaaagtagccatattccttatttttgaaaaaatgtatctttccatctcagtttcatcttaacaaaaaagtatgcgtttctttaaagttttcctggccgcattccttgcattcgtagcattcacggcaatatgcttctttatattgctgatcatgataggaagggccgttacccctgaaaaggtaacaatttcccccaatggcgtactggtactcgaaacagggcagtcgtacaacgaacagaatataattaacccactcggcagactgatgaacgacgacgccgcagttacccccggattgtatcagaccgtaagactgatagaacacgctgctgacgatgacaacatcaaaggcatttacctgaaagtaaacggtaaccctaatggctttgccagcacagaggaattccgcaatgcgctcctccgtttccggaagtcaaagaaatttgtgtacgcctacggagaggtaatggaccagaacgcctactacctggccagtgctgccgataaagtatacctgaaccctaaaggtggagttgattttaccggctttgccagccaggtgatgttcctgaaaggaaccctggatagactggaaatcaaaccggaaattttttactgcggcaaatttaaaagcgctaccgagccactgcgcgaaacacagatgacagatgccaaccgcatacaaaccacccagttcctgggagaactgtatggcaccttcctgaaaggaataggctctgcgcgcaacatcgacacggccactttacatggctatgcaaatgaaaacctcatccagcaacccgcagatgcgctgaagtataagctggtagatggtttgaagtatgacgatgaagtagtagcggaactgaaaagcaaaacaggcgttaaacagggcgacgaggtaaacctggtgacgctaaaaaaatataacagtggcaccgacctttcttccggtggcggagatggacagttggcgctgatctacgcagagggcgatatcataggcggggaatcagaccgcgataaaaccattgcaagcgacgactatatccgtgaaatccgtaaagcccgcgaagataaagatgtaaaggcaatcgtgttccgggtgaactccggtggcggcagtgcgctggcatctgaagtaatctggcgggaactgtcgctggcaaagaaagtgaaaccggtggtggtatccatgggcgactatgcagcatccggtggttactatatttcctgcatggctgacagcatttttgcagaacccaatactttaaccggttctatcggcgtattcggcgtgatgtttaatatgcaggacttcttcaaaaataaagtgggcgttaccttcgatggcgttaaaaccgcaccttatgcggatcttggttccgttggccgtccgctcaccgaagcggagagacgctttatacagaacggcgttgacagcacctatgcctctttcaaatcacgcgtggtagccggcaggaagctgagccccgctatcgtggacagcatcgcccaggggcatgtatggagtggtttacaggcaaaggaactcggactggtagaccgcatcggtggtatcaacgaagcgctggcctgtgccgcgcggctggccaaactgccggactaccgcctgagagagttcccggaagagaaaaacccgttgaacaaattcttcaaaaccttcgccggcaacgtgcgcatgcagctggtgaagcaggaactcggcgccaactacgacatttaccagcaggtgaaggacgtacaacagttgcatggcgatgttcaggcgagaatgccgtttaagtacagtttctagcgaattttgtcttagctcaggattacgctgattttgctgattagctggattttactttgggattttataaaggattaagggagatagaagcggatattcgctcttatctcccttaattattatttaagaaaatctaaaaaatcaaaaaaaaatccaaaagtaaaaatccagctaatcagcaaaatcagcgtaatcctgagccaagacaaaatccccgcccctgcattttttactaaaagctggaaaaacgtcgtagttttaccgccggtttttaaatagcagaatcagatgaatggagcgaagtacagtcagttgagggccatgctggccattacaaaaggaagtttaagaggtattttccgtagtccttccgccgtagtgttcagtttggggttcccgctggtatttatcctggtgtttgggtttattggtaaaagtactgtttccgttaaagtgggggtggaccgccggactgatattaccagcaggtattaccaggaattgtcgcatgccgggacgctgaaactggttaccgatcagcctgaagcggaaatggaggatgatctgaagaaaggccgtttggtggctattctgaacattgtgcccaaagcgggagttaaccatgtaactgcttacgatattaatatccggacctctacggcttccgatgccgcgaagaaagtaaccctgttatcggtgctgaaaagcatcgccggcaaactggatgatgaaacctataaacgccctacggtagccacttttacacaaacagaggtgccgggtcgtgaatttaagaccatcgactttattttaccgggacagctgggctttgccctgatgagtgccgccgtttttggtacggccttcctgttttataatatgcgtcaaacgctggtactcaagcgttttttcgccacgcccatcaaacgcacctatattgtactggcagaagcgctgagccggatgatcttccagctcatcagctctgtggtgatcattgcgcttgggcatttcgcctttggctttacgctggtacatggttttgccaccttcctggaaatgcttgtattgtcggtattcgggctactggtattcatgggttttggttttgtggtgagcagcctggcaaaaaatgagagcactattccgcccctggccaatatcgttaccctgccacagttcctgctggcgggtacctttttcccgatagattcctttcctggctggctgcagccaatctgtaagatcatgccgctgacctacctgatagacgcgctgagaaaagtggcctttgaagggctgcatctctggcatgtgggctgggatatcgcgatccttactttatggggtgttgtcgtatatgcggtagccgtgaaagtattcaagtgggaataaggcgatttcgttagctttgtgggacctaaatccagtcacatgcaagcctttttcattatcctgggtgcgttcattgtccttgtgctggggcttttcattttcagtttattcctctcatctgccattaaggtggagcgttcgctggtaataccggctgcgccgggagctattttcccgctgatgaacgtagtgcgtaactgggagctatggtcgccctggaaagaacaggatcccaacgttaaaattacttacggggaaaaggaaagtggtgtgggcgccggttacagctgggaaagccgcaaccggaatgtaggtaaaggacatatgacgatcacggagtccaaacctgatcagcaggtggccacccacatcgattttatgggcatgggcgctaccaaaggctatttccggctggacccggtaaatggcggcaccctggttacctggggaatggtgtgcgatatggggcaacatcctatccggaaagtgatggggctgatgatggacaaatgggtaggaaaggattttgagaaaggactggagaacatgaaacggctccttaaaggataatatattttttctatgcggtttattaagttgttactgatcagcgtgatcattttaggcatggtgattttcgggttgtcgctggcatttccttctacggcagtggtggagcgtacaggtgttatccgggcgcctattgatactgtttatgcacatatcagtaacctgaaagcctgggatgcctggaatccctggacccgccccgatactaccgctaccctggtatactccgatccgccttccggccccggcgcctggtacagctgggacggacaactcaacagcggtaagctaacggtgctggacagtgatccggccaaaggaatacattacctgctggatattaaaagtgtgcgtcctgtaaaaggaggcatagaactgaagcctacggcagatggcaaagccactgcgatcttctggcatatggaaattaagctgggcatgctgccgtggtggaagctgaggggatttgtggccgacagggtatacggccctgctatgaacgatgggttgacaaagctgagccggatctgtgaaggaaaatagtatggagttattttaccattgatccaatagttttgtttacgatggtttttatgatttaaattgttatcgtatctcaacaacttcttacagaaaaaactaaaaaaaatgaaacatttctttttggcaaccttatttctggcctttaccagcctcgtttttgctcaggagaaggcacgtaaaagcccccacgttacagtagaagccaacggtattaaagtagtgtacggccagccttccaagaaaggccgtgaaatttttggcaaactggaaccatttggtaaagtatggcgtacaggcgctgatgaagccacccagatcactttcagcaaagacgtatcttttggcggcaaaccggtaaaagcaggtacttacactttgttctctattcctgatcctaacacctggaccgttatcctgaatggtaaactgggccaatggggtgcttatgattacgacaagaataaaggcgaagacgtagtatccgtgaaagtaccacgcgaaaaactgtctacaccagcagaaaaactcacgttcactttacccggtaacgccgtggtatttgagtgggatgacactaaagtatccgtaccggttaaataacacgaccgggaaaaatatcaggggcacagacaccgcgtctgtgccctttttttatgataaggtggctaccagttcccggatactgccatacacttcatccagctgttcgttggtgatgcagtaaggcggcagtatataaagagtattccccagcgggcgcagcatcactctttttgcccggaagaagcggtgcagttcatcggccaacgcattcgtgtaaccatcggcgttagcggttactatttcaaacgccaggatagtgcccagcaatcttggattttttatgaccgtgtaagtaaacaattctttcagaaagacagtatgcttttcgtgtatgcgttcccggttagccgcgcaggctgggtcggtgaagaggtcgagactggccagtgcagctgtacaggccagcgggttggccgtgaaagaatgcccgtggaataatgtttttagcttatcattggaaagaaaggcttcatacaccgccgcagtgctggtagttacaccgagcgccatggtgccgccggtgagtcctttagaaagacaaacaatatccggtggtgtttgcaggtattccatagcaaaatttttcccggttctgccgaagccggtcatcacttcatctgcaatcagcaggatattttgggaggagcaaaactgcaggagctgttcaaaggcggcagcgtcatacatcaccatgccaccggagccctggagcagcggttcaaacacaaaggcagcaatatcttccggttgcagtgcaataatgttgtttataatttgggagatgttttccgcagtgggcacttctatgaactgaacatcaaacaggcggtcatcaaaaacgcgggtgaacacacttctgccgctcacgctcatggcgccgaaggtatcgccgtgataggcgttgtggaaggccagtattttatgtttcggcgtgcctttgttatcccagtactggatggccattttcagggctacttctatggccgtagagccattgtcggaataaaaaacgcggcgttggttggcgggaagaagcggtaataaccgttccgcaagatgaacggccgggggatgggtgtacccggcgaaaatacagtgttccagttgcagcgcctgtgctgccagttgctgcgcaatgtgcgggtgtgcgtgaccgtgaatattcacccaccagctggaggtagcgtctatatagctgttattattttcgtcgaaaagtaaagcgccttcgccgcgtacaatgcctatgggcgcaggtgcagtttgcatttgggtgtaaggatgccagatcacgtccagatcacgggccgacaaagaagatgtttgcataattgctggctgttggtgcaggcgcgaaggtactataaaagcgggttatgttttcctgtgccgttccagtatctccagcagatccgctgctgcatagggtttgggcagcatatgttttacatgcaggcgggccagccgttcggttacttccggcattatgtctgccgttaacacaatgataaaagcatccggctgcaggtgccggatgtgcggaatggtttcataaccattcatctccggcatatgcaggtcaaggataataccatcgaaagattgttcctgtattttctgtagtgccagtctgccattgctggctgtttcaatctgcgcaccggagtttttcagctgtaattgcaggatgcggatattaatggcattgtcttctactaccagcagcttcatattttccagatggccttcctgttgtttatttttctggggcacaggaccgggtgcagtttcaggtattgtaaaactgatatcaaaacggaaggtagtgccttcattttttttgctttccagtatgatgctgctgttgtggagcgccaccagtttttgagtgatggcgagtccaagccctgtaccgccgtgatggcggttggtagccgaatcttcctgtacaaaagtatcaaatacttttgcctgcatttccggaacaatgcccacaccggtatcctttacggcaaaggaaagcgtacagtcgccggcggaagtgtttgcccggcgtacttccagggtaaccgatcctgcactggtaaatttgatggcgttgtgcaacaggttattgagtacctgggataatcttacgggatctcctttcagtgttcccggtaaatgatcaaaccgggaaatgagttcaatacccttgctggtagccagtggctggcagttacgtacgatacccgttagcagcgcctccggatcaaatggaatattttccagttcaatttttccagcctccattttgctgaagtcgaggatatcattgatcagtccgagcaaatgatgggcggagaactccaggttatgcatcagttccgcctgttcgggtgcgggattttcccccaggataccggcgatgccgatgatggcattgaggggcgtacggatttcgtggctcattacagacaggaaatcacttctcgactgggcggctttctgtgcattatcccgggcagcagtaagcgccagttctgtatctttcttatcagtaatatccatgataatgcccctgaaatgcgtgagctggccctggctgttaaataccgccctgccgatggtgcgcatccaggtatgtttccctttagcggaaatgtgccgtaattccaggtcgaacggggttttatgggtaatcagcgcttccctggcagcaacgaaaacaggctggtcgtccgggtgataaaatgcaacggacgaatgaaaagtaagcgggaagtcgtgcggcacctccctcaattcatacacttcgcgggtccagtaggtttcgccggtggctacattgaattcccatccacccattttgcccatctgctggcagatgcccagcagctggttactgcggcgtagttcagactgtgcctggaggtagctgttgttctttttttctatttcagagatattacggatcatcagcaggatgcgccggggtgcgggcaacttatctttaatcagccgtactttcagctggtaccagttttgaggaccctgcctgatatcaggatacacgtattcctggttttctccggtttccagcagtttgtcgaccagccggttaaaagtgccggcatgctcgccaagggcttctgagatggttttgccgatgacctcttcccggggccggaataacaggttgtcgttgctgcaccataccccggtaaagaccttctgctcgttcatctcaaataaaatatcatccagggtaagcatcagcgaatcccactcgtattttaaccgggtaaaagcggattgcagctgcctggtttccttttccctggtaccgtgaaaatgcagatgccccaatatttgcagtagtggttggaggaaagttactgcatctgccgaatagccgtccatgcagcctgcgagccctattacggccagcacctgctgctggtatgttaccggcagcccgataaatgcagtggtagcatcccctgccggcaggatcagcggttgcccgttgccggccacttcctgcagggcaggcgtgaagttccagccgtgttccggcgcatgattgatgatagtaatggtatgcagttgggaaggtgcatcgcttttcttcaattcccccacaaaaccgtaagagctgcctgtcaggtccattagttgtcctaacagttgctggacggcattaaccgggtgttcctgcaaactgtagtctgcgggaatactgccaatgatatccagtaatttttgttgacgcagcgctgcagtagccagcatgagcgatgttggttttaatattcggtgttaaaaagaggccagattatgaaaccggtgtagttatattgttatcgtcaggattataccgggggaataaatttagggaattaaccggagaaacgaacaaggaattattattataagctgagggaacggttttcgacgattccctcagctcggagaggattgttattttgccatgccgccgtttttaaacagggcataagcagtttgatagttggcaatactgtttttgagaagtgcgctgtccattgccgtggcccgttgttcattgcgctctttgttccagctgaagcattgcgctttttgctgcgggctgaggatcagcagtttacccggctccaggtaacccagtttttgataggtacttaccatggcacggggctggtatcccggttccagtacgttttcgccgtaaaacttactgttataagaccagtgcagcatgcccaggagggtagggtaaatatctatctgggagcacatggcactgatttcctgtggcgctacgcccggaacattgtacaggatacagggaatatgatatttactgatctctatttcatttttaccggcgctgctggcgcagtggtcagccacaaaaatgatcacggtatttttaaaccagggcttggtgcggatctttttcaggaactgcccgatggcgtagtcggtatactttaccgcgccttcacggctgctgccggaagggatgtctattttgccggaaggataggtgaaaggccggtggttggaggtggtcatcacgaaatcgtagaacggcttgccggccgcatatttctgatcggcgcttttaatcgctgcggcataaatgtcctcgtcgcatacgccccaggcattttcgaactgtacggcgctgtcgggaatatttgtgcgggtggtggtgatatgatcatccaccagtttatgacggagccggtcggtaatatcatagccgttgttcccaaagtacttgttcatgttatcgaagtagccgtcgccgccataaaagaaggtgctttcataaccctgctgctcaaataactggcctacggaaaagagttgttcattctttttccggcgaacaatactttgcccgggagtgggtggcacggcgagtgtaagcgcttccatccctcttaccgtacgggtgccggtcgcatacatattggtaaagagaataccttctttggcaatactgtccagcacaggcgtaatatgaccggtgttaccaaagcggtccatgaaatcggcgctgaagctttcaatggtgaccatgatcacattaggtgcaacacgtgtacccgtatccgttatactcctgtaaatattgttaccggcagtcaggtaatggctgtcgggcgattgcagcaaggtgcgcatccggctgaaggcggtgttatcatcttccagcaaataatatttatcgtaagccagttcattattcaggtaggcggaaataaatgaatacacacctgctttggataactcctgtgcataccggtttttgcttttttcggcccaggtgttattgatgaagaaaatgtgcaggagcattagccccgccagcccggcaaagatgagcagccgtttcccgaaaggtgtgtgcgattggaaactgttgcggaaaatacccctgcgggccagcacccaggtgatgagggcggtgaataataatacgccgccaatcagcaatggtaaagggtacgactggttaatattactgattacttcataggtataaatgaggtagtctactgcaataaaatcaaagcgcccggagtattcgccccagaaggttaattctgcaaaaaaggaaaatacaaggattaccaacgccaggaaaaagccggtgtaagtgaatatccggttaaacagcgtgttattgagccgttgcggcagcagcagcaggtaaagggcataaccaatggtaaaaaacaaagctaccccggtatcatatatcagccctttgccataaatggctggtaaatgggataagcgcagcccggattgagggaaagcccataccagcaatacagttctaacgaggaacgacaggatcaggagtacggcgccaaagcccaggagcaccgcgtacctgtttttgatgaatttcatagtgtacagaaaattaaagaccgcgaagttacactcttcctcataaatttaactataaattaactttcaatgacatattgatgattcttccatctacaggcccccatagttgggcaaattccggatgcgtaatggtgccggtatataagggtgtgttcttgccttgccttgcgtcaaaaatgttctccccgttgagtaccagggtaacgtgttcccccaactgccgggaaaccatcgcagcccagaaccagtagtcgggtgttttttgattgcgatcgtcgaactgatggcctatccggctgttttcaatgccgaagcgccatttgccttcgatgctgtaggccagtgtaccggcaaatttgtcctgtggcgcaaacgcgacattggtatgggcagcatcgttgtaacgggacaccgtgtggttgtatcccaggtacagttccaggtgatccagttcaaagcggaggtaggtatctgtaccaacactgtttacagcgtaaggcatattctgcagcaggtacattccctggctgccgggttgcagcaccggcaggataggatctttgatatgtgtgtaatagagcgcctggttcagggtcatgtctaccttacctaaactggtatggtagttcccgtcaaagttaataccctggctgctttccgactttatacccgcgctgagcggcagcaggtagcggtagccaatggtttgggtctgcgtggtgaaaacagccggtgatttataacccgtgcctgcactcaggcggatgaacaggtcatctagtggtttgtatacaaacgccagcctcggtaaaatgtaccatccgaattcattgtgatggtctgcgcgcagcccggcttctgccatcaactggtccgtgatccggaaaccatcctgtataaaggcgcctgccgtgttatactggtagttgccgagtaatgtgctatcgcctttggcgcggtggtatatttcgccggtattattgatgccggctacccagttgtgccggccgcttgttttatggtaggccgcttctgcataagtgctggtttgatttccgagcagcgtaaaagtttccacgttgttttgcaggtggaagaagctgcctgctccttttattgttaaagtgccgccgccgaggtttttccgggtgaattgcagctctgcgctgtgtctttcgctgttattggtttctgtatactggtggatgccggccggggcatgatccagtacctgcatatcgccgccttcgcgtttttcgatggtaccggtatagccggccaccaatgtggtttgcggattgaggtaccagaagaagcgggggtggagtaggtattgacgcaggcgcggcacatcgctgaagccgtctttatttacgtcgctggcgttttgtgtggtaacgccggcaaagagggtgataccggttttgccgtatttttccgcatagtaagcgttcacgttggtttctttcagcgtactacgattaaccagtaccgttagttcgggtttactgccgggcgttttggcaatgaagttgatgatcccggcaatagcgccgccgccatagagagtggaaacagatccttttataatttctacctgtttaagatctaatggcggaatggacagtacaccgaaattgccgctcaatccttcgtacaccggcacaccgtcacgcagcagctgggtgtatttaccgtccagtccctgcatgcggatggcattgttaccactcactgcagaggtattctgaatatggattacagacaggtcgccgaggatactggccacgttacccggttttatgccgctttcttccatcatatcttctcttcccagtacttctactttcatgggcaggtcttcaatacggcggttatcccgggtagaagaaatcactacttcttccaggtcggatactttgctgatggtggtatctttcaccggttgctgtgtggtgtctttaacgggaacgggtacacgattttgtgcggttacaatgcctgttgcgctcaataaaatgatagccagtattacatgtttcatatgctcctttgtactgcaaagaaaaacatggaatctggagcaaatctgaacggtgggttataggcttacacggaaagtatgctgaccatttgcataataataggtaagatggaaatgataggagtctgccatttttttaacaatggcaagtcccagtccgttggaattagagtagccgttgttgtgttttttgaagcgctggaacaacacgttggcgggtatttcaggcagatggctggtgttggcaatagtgaacgcctcgggtgttaactgaatagtgatgctgccttgcgggtaattatatttgatggcattcccgagcaggttgctgaccagtatatcggtgagtgcgggatgcagcggccatggtgcggtagcggttatttctttatgaatgtgcagatctttctctttgataagttcttcaaaaagcagcaggtatttttcaacaacggtgcaaaggtccggctgttctgtgagcgggtattgctggttttctattttggccagcagcaacaggttgtgattgaggcgcgacaggcgttgcagctcatcatagctggtgaggatgctgtttagttgtatttcagagagggtatcgtcctgcagcaataattccagtttgctttgggcgatagcaaggggtgtttgcatttcatgggctgcatcttccgttaactcttttatactggtgtaatcgttgtgaatacggctggtcatggcgctgagggcggtattcagccggttaaattcatgggtggcagctggttcaaaaacggtggcgtccagtttgttcagttgcagcttttgtattttgtcgagcgaccggtaaaacggtttccagatgcttctactgataagccagttggagagcaatgcaaacaggagtaaaccaccaaaagccgccagcattacatgaatgatgttttttaccaggtcatctttttctatcagtgatttacggagtaccagttcataatttttgttatgcaaactgattacctgcgatagttgccggaagggcgcgtaggtattttccggttcctggtaaatgtttacgcctttcaggtgatgtgttggctgcgctgcgtcgttcgtaggatgcaggttaaattccggtgttttgatactaaaaaccgggttgttcacactggcggtatcaagataccgcatccactggagtttgtcattcaccagttcctcatctgtttcatattttatttcctgattgaattctgtgtacaggtaaaaagcgcctgcagtaaacaccgggagcatgatcagtaaaaagtatagggttgtttttgtcagcagtttcatgtgcgcaatcttttaagggatgttatccgaagcggtaaccggttccgtatactgttttgatgtaatcttcgccgcctgcttccagcatttttttccggagatttttaatatgggtataaataaaatcataggagccggcctggtcatattcatcgccccaaagatgtcctgccagggcggatttggtgactacccggtgttgattggcaataaaatacagcagtagctggtattctttcccggtgagggtaagggatttatgatgaaccagcactgttttggaggcgggttttatggtgatttcctggaagttgacggtggtattgccgtcaaagtttttccggcgtaagatggcatttacccgtgcattgagttctgagagatgaaatggcttggtgagatagtcatctgcaccgagttcaaggccgttaagtttatcttccaaagagtctttggcagaaatgataatgatgccggctttggactccagcagtttcagttcctttaccacgtccaggccgctgccttttggcaggccgatgtctgccactatgcagtcgtagtcaaattcattgaccttatcaatggcctgtggaaaatctgctgccagttcacagatgtatccctggtgttccaggtattcctgtatactggccctgagagccggttcatcttctataatcagcactttcataggctaaaagtaggtataattcctaaaggaattctgtagcagcattctgcaatcccatacgggtttttcatcattttttggcaggaatgaaaactatgtactcctgtatttcgtaaatacaataccgatatcaaaccattcattcaggcattcttatgagtacttattttaaaatggtggcagataggctattactgaaaaagttgccggaagcagccatcacacaacgaaaggtttcagatgatgacacgagggagttgtgtgccctgatggaccatattcccaatgcgaaatcagtggcagcaatgtaccgtcagatgatgagaacgggccggctcacagagcgttataccagcggggatcctggcaggaggtggctcgaagtggagcaaattgtgctgaaccggaacgagagaaagaaagaaaacaaacgccggctcatatggatgatggtggttttcatcacggtgggtattgcttcctatttcggaggcgtttatttgctcgcaaaaggaaagcacctggctgtccaggtatggggataaaatatatattttatacacttataatatggctgaataaaaacgtcccggcagtacattactgccgggacgtttttattcagcccatttccggtattattttctttcaggcatctttacactcaatggcttttcattgcgcaacatgctggcggcttcgccggttagccagagataatgatctgaaggcttcccatctaagttgataaacggcgtggtgctgcttacgggaggctgatcgcttcctttaaatatggcagtggcttcatttacttcatcaaacatggccacatacagcatgctggcgccggcagttaaggcggtagaaatttgttgccagtaaaaacgtccgccctggcggggaatagagcctacgggttttatatcgtccgggaattcataacgactgaggttgtgccagctaaagccgggatatacgcagggcacatattccaggtggttggcgcggcaccaggccaggtcgtcgatgaggttatcgcggtagcggtccatatcattgtgaagcagcggggaataccgttgtaccgtccagggcagtaccaggtcggcttgtttgatgatggtatgcaggtaaggatcagggaggcagtcggcgttcaaagtgcgccaggcggtgggtacgcccagcataatggcacagccgccatacacggggtcatttttcaggaaatcgatgagcctttcgaggccaatattacggagattatacgggcggtcaggaaagccaattccccagatggctactaccggtttgccgttttgctgcaaataagttttggcgccgggctggttggttactttcagctgatccaccaggtacttccagtcttcaataatagcggaacaatcctcccctgtggcacttaacccggaaaggtcatacatcacggcgatagcccttttatatttcgaagctgctgcgaaggcatttttcaggacaacggaagagacgctgtcgcggcgtttggcattattaaaaaagcgttgcatgaaaacgccgtcaaccccatattgctgcatccacttgaagtgaatgtctacggtgcttttgtcgtaagaactgaagaaacgtgcgggctggccgttggcgagcttaaaaggcgtggcgtatgttttttcatattcgcttacatccggccacatgtctattccgctgcgggtttcatcgccataggaaaagcgccgggcgccggagccgtcaccttcggcccggaaccatccctggtagccggccatcaccaatccatgataagttgggtactgtgattccctgctgtgtttcaattgtgcctgagcgggtatgctcagcaggaggaggaaagctagtaagatacgcttcatatatatactgtttgttattaacgtggaacctgcttttaaaaagaggagaacccggcttgcccggattctccaaaggttttgcattcaccttagttgtgtatcccggtgatattccccggaataagatgcaagtaaagcgggaaggactaacaggagcgttaacaaagcattaattgcgggcattaatggcctatttaccggattaatttccggaaacggcaaattgacgaaggggaatcgcggtatttagcagtatcttttatttttcgtacgaacagcatggcggaataatatttatctttctgtatacgcaacccaatgttttatgcccgtaaaaacaaacagattactattccgcgctgttactgtatggctgttgatgatttttgcaaatgatgcaagcaatgcccgggatatttgcggtggaatggccacgcgcgaatgccgcagcacttcagataccaaccgcagcaagcctgcctttgcagcgttggtgctgtatgaaggcggcggccaccatgtggcgttttcaaaagcggccagggtatggctggacagcctcgcagcgaagaaacaatttacccttacctatatcaacaacactgatgcgattaatgatgactatttaaagcagttccggctttttatccagctagactatccgccttatggatggaagcctgcagctgcagcggcatttgagcgatatattcaagagggccgcggcggctggatcgggttacatcacgccaccctgctaggtgaattcgacggctttcctatgtgggattggttttcggcatttatgggcggcatccggttcacgaactatattcctgagtttgccaacgggaaggtaatcgtggaagataaaaagcacccggtgatgaagggcattacatctccctttattattaataaagaagaatggtatacctacaataaaagcccccgcccgcaggtgcatgtgctggccagtgtggatgaaagctcctatgtacctgcttctgacaggaagatgggcgatcatccggtggtatggaccaatgaacattataaagccaggaatatctatattttcatggggcatggccccgggttgctggataacccggcatacctgcaattgttacagaacgctattttctgggcagccggtaaataacaggatgtggaagttttagtaactttagctgctgcgtaggaagagcctttctttgggtgagttataagaaaaaataaaccatataaaatggagaaaaaatttcttatcagcggtatgctgtattgtttgctcctgctgccgttgcttttaaacgcacagccacttcccatcggtgcggctgcaccggattttacgctgccggccacagacgggaaaaactattcattgtcttctttttccagggcgaaggtactggcagtggtttttacctgtaatcattgtcctactgcgcaggcgtatgaagacaggataaaacaactcacctccgactatgccggcaaaggtgtggagctggtggcgattatgcctaacaacgcggaggggttgcggtatgatgagctgggatacacggatcttggggattctttcgatgatatgaaacagcgcgcaaaagacaagcagttcaactttccttatttgtatgatggtgacagcgaaatagtttcacgggcctatggtcctattgctacgccgcacattttcatttttgataaagacaggaagctgcgttaccagggaaggattgatgatatggagaatcctgcaaagaagccagggtcgatggatgcacggaatgctattgatgccttgttgcagcagcgggaggtgccggtagcggtcaccaaagtatttggttgttctgtgaagtggaaagataaaagtggcagcgtggaaaaagcaacgcaggcctgggcgaaagaaccggtgaacctggatacggtgtcggtggacggtattaaggagctgctgaaaaatacttcttccaatctgcggcttattaatatctgggctacgtggtgtgtgccttgcgtggcggagttcccggagtttattatcctggccaaaacgtttagtgagcgtgattttgagtttgtaagtgttagtgcagatgaaccggagaagaaagataaggtattacagtttttacagaagaagcattcttccgggaaaaattatcttttcagcgggaaaagtaaatatgaattgattgaagctgttgaccccaaatggcagggcgcattgccgtatactattttagtggagcccggtggaaagatcgtatatgcgcaacagggagaaattgatcctgtggcgcttcgaaagttaatttttcataaccgcatgatcggccccatgtttaaatagatcggtgtccggccattttgtggcgggatcgttcactgccttccacagcaatccatccaggtcgttaaagaagctgctgtcggtacgcgtgttgcaaagcatcacccagttgaatcctttttgtgcgcgtattacttcgctggcagtgccgggcagggagccggagtgccaccagttgtgataaggatttacagcccatcccagggcgtaaccggggttggcttccgagccggtagtcatagcagtgacagactttgcagtgagtatgtccggaggtaatgcgaagccatctacatgaacgagcaggcgtgcaaggtcggcagcgctggctatccatcctccgtgcgcatccatgcgggtaatgttatagatgtatggttgttcgccatgctggccgtagtatactacctcatttggtttccgctctgccagggtattgccgcctgtttgcatggctgtgatgccacagggtagcagcactgctttttttacatacgcttcatacggcataccggatactttttcaattatacggccgaggatacagtacccgaaattggaataggcgtatactgttccgggaatattgtccagtggctgatgatcaatagtccacgaaatcagctgggcggcgctcatgtccggatggctgaacatgggatcggtaccgttgttggtccagccgccggaggtatgttcaagcaactgccgtaccgtgatctttttcaggtcttcccggtagggcggtgtgccgtaagccgtgcccaataaagcattggggccaaatacatggtcgttcagcgacagcttttttgcttctgccaattttaatatagccgtggccgttatacattttgatacgctggcaatgcggaacaggtgttgggaatttacggggatatgttgtgtggtatctgcataaccgtagttgccggtatataccagtttgcctttgtaagttactgcaaccgccattcccggcacgtggtagcgctccatgaaagcatgtacggtgctgtctatctgcgggaggggttgtgcggcagcggtattcactgccagcaggcataacagcagtatacgggtatatctcataaaattaaggtacaaaaatatttccttccaggtaagtcttgcaggtaccgcctatcaatacgcgttcgccggcatccacgcagtagagctttcctgttctgggggatacctgcagggcgatcatttctttcttatccagctgccggctccagaaggggatgagcgagcaatgtgcagagccggtaacggggtcttcaaagatactggcctgtggcgtgaagaagcgtgatacaaagtccacctgctttccttttgccgtaacaataatgccgccggggtcgaggttgatctggtcgaggatggccttatccggatgcaggttgcgtacaatttcttcgtcgtgatacacgaggatataatcccttgctttcagcacttccatggggtatgcgcccattcctttgagtatttccggaggaagggatgcgggtactgcgggccttgacgggaagttgagggtgagcagatcgttgtgtttggaaacggtaagcggtccgctttgcgtatgaaaagtgagttggtgcatatcccatccgaggtgattgaacagcacatgtgcgctggccagtgtggcatgtccgcagaggtccatttctatttcgggcgtgaaccaccggagctcgtagtggccctgttgaccggtgggaataaagaatgcggtttcgggcagaaaattttcggccgcaattttctgcaaggtatctgttggcagccatgcttccaggagacatactgctgcggggtttccgccgaacagttcattggtgaaagcatctacctggtaaatgggtatatgcggcatggaaatcagttttggtgttgtaccgtaaaggtattgcttttttgagcgtgtatcttccgggggagggtgaatgcccagaagagcagtcctgtggcgctgatagcggcgccgagtatgcatacggctatccatccggcgaaggcatatatagtagtggcggcaatgcttcccacgccgctgccgatggaataaaaaagcatgtagcccgctaccatgcggttgcgtgattccggtctgatgttgtacagcatactttggttggtaacgtgcaccgcctggatggccaggtccaacaggatgataccggcaataagtgctgtcagcgaataggtggcaaagccgagcgggagccatgaaaccagcagtaacaacaaggcggcgccggtggtgcgctggccgtagccacggtctgccagtttacctgcacgggcggctcctaatgcacctgccaccccgattaaaccaaacatgccaatcgcggtagccggaaaggaatacggtggcgcactaagtggtaataccagcgacgaccacaacacgctgaaggctgcgaagatgaagaaggcaagaatagcgcgtaccctaagaatgggttcttcgaggaataaccggaatacagacagcagcaattgcgggtagctggtattggctttctgcgggtcgtgaacgggcaatacgcggtaaaggacaccggcggtgagaagcattaatgcagcggaaaaaaagtataccgagcgccagccggcgatgtctgtaagtgcgccggaaacggtgcgggtgagcaggatacccagtactacgccgctggtcactaaacccaccatgcgccctctttccgccggggcggccagtgtggcggcataggccaccagcgtttgcgtaaccaccgccaggaatcctacggctgcaatgccgcccaggaaaggcagtttggccggcgaccacgctacggtaagcaatgcagccactgccagtagcagttgggttacaatcagtttgcggcggttaaacagatcgcccaacggtaatagtaggagaagcccgagcgcataccctgtttgcgtaatggtaacaatgatgcccagtgagcgtgacggaatatgaagatcgtttcccattgtgttcagcaagggctgtgcataataaacattggcaacggcgaggccgcaggccaccgcaaatagcagcgcggtaaaccgggtgaatttttccatgagtgaattatgtgttttgtactgtagggtacaaaatagatcataaaaaaggggatacgctgttccctggttaaccgagtatttttaattgtgtttctatcagttcggagagggcttcgttatccgggtaaatccgccgggtaataccaagtccattccagttattgaggagcaggcgggccagcagtgggggcggcagtttggagtgcagggtgcctttttgttttccgcgcagcagtgcatccaggaataatgcttccagtccctgcaggtgagtggcggcccttttcatcatagggttttccacgttggaaagctctgctactgcgttgccaaagatgcaacctttctggtgcctggttttggtgctttgcgctaccctgcggaaaaactcccggatgtaatccaccggatctacggcggcgtccagttctcttctgaactgtgcaatcgcctgatcactatgttgggccagcgccttttcatacagctcttttttaccccctttaaaagccaagtaaaagctgcccttacctatgcccatagcagcgagcaggtcttccgtggaagtagcctcatatccctggcgccagaagatttcagccgctttgctgagcacttccccgtcgtcaaatattttcggtctgcctgacatatctctctcttttacatctcaaagatatattctttaccaaatagtacaaaatttttccggcataaaaaaacctgcggaatacgcaggttaatcttttgtgtggaaaatataccggctagtgatgcggagtttgtgggtgaagcagttgaaacaattctctttgcagatcatcattatgaagattgtttaactgctccgttgaaatttcgtaaaaggcagttttcttgcctaatacgcctatcacaaacgtgtgtccggcctgcaccggttctgcggtctgggggtgtttttttgatagtgttaccactacatctttgaattttgacatgtagtgaatataacaaaaattccggattttgggtaaaatcacggatcagctcacccttaccccgtgcagtaatttttccatcgcgttttgtaaagaccctgccctggtgacttctcccgaattcacaaaaaagatctcatcggcattttcaatggtattcaaccggtgcgcaatgattacccgcgtggtattttccggcagcttttccaggatttctcccagcaactgttcggtaacggtgtcaatattggcggtggcctcatccaggataaggagatcgggtttacgcaatactgcccgcataaaagcaatcagttgtttttgtcccaggctcacaccatctccgccggaaagcacttttgtttccagcccgttttcaaaaatggccagcagtttttccaggttagcttccctgatcacttctgtaagctgttcgttggaaaaatctttatatgccgggttgccgtataggatgttttctttcacggtgccggtaaacaggaaaggttcctgcaaaatgaaacctattttccgggaacgttcatcggcatcataactgcggatatcccttccattcagtaataccatcccctgcgtaggatcatacaaacgcgcaatgagtgatgccgtggtggttttgccgccgccggttggtcctactaacgcataggttttccctttctccagcgacaggctgatgttatgtaatatttccctgccttcggggtaaccaaaatgtacattccggaactccagtaatgctgacgagtcgctgtaatccttgccggcattcactgtaacaagatccgtttccagtccgagtatttcggagatccggtcccagccagccatcgccacctggaagttggcccacaatgtagccagttgccgtaatgggttatagaaataagtggcatacgccaggtaactaacgagcaggcctatactaaattctccctgggtgatcaggtagataccaccggttaataccagcaattgtgcaatactggcgcacatggcataaaaagggaggaacacattgttggcaagcccggtgccaattgcgctctggtagtttttttcattggcatcctggaagcgttggcggaaataatcgcggcggttaaaggctacaattactttgaagttgctgagactttcctgaatttctgcactcatattacccaccgttttcaggttggctgcattttttctttttacccagggagataatacccttgtaaagaggagtatcagcaaaccgggcgccagtgcggcaatgccgatcttgtaattgatgatcagcaggaagataccggcgccgatcatagtagaaatgttaccaataaactgcatcagcgattgtgaaaaaaactggttgagtttatccgtatcattatttacgcgggagataaggtctcctgctttattctggttaaagaaggctacgggcagttgctgtatcttactaaaaatagcattccggagggtaaataaggtacgctgaccaacaccgcccatgagctttgtctggaagtaactggtgaacagcgccatcaggtaaatgcccagcaggatgcctgaaaagatcagtacgccgtggtattgcttatgctgcacatagtgatcgatggtataaccgattaagaagggcccgagcaggttgagtatagaattcagcaggatggcggttaaagccactgccaggtttcttctttcgtgggaaatcagcttcagcaaattcctgaatgcggagtagttggatatcttctgctctttctccgtaaacttattaagattgtaattcatagttgctggtgctttgttgggaattaaagatctgcacgtactcggggctggtatggagaagttcttcatgtccgccggtggcgataatttcaccctgcatgagcaggatgatctgatcgtaatgcgttactgaagaaattttctgtgttacagacaggagtgtgatacccgggtattccacctgtacgtttgccaggatctttttttctgtattggtatctacacgggcggtgaaatcatccagcagcaggatcttcgggttaatggccagcgcgcgcgccagcatgatacgttgtttttgtccgccggaaagactggcacctctttctgaaacaatggtatccagtttttcggggagcgcttcggtaaattccttcagttcggcggtgtgcaatgccttttccatggctgcttccgtaacggtttcgttgaatgcaatattttcccggacgctcatattaaaaatgatactgtcctggaatacaaagcccacctggctgtgaaaggattcgctgttataatctgctaccgggcgcccatctaccagcaccgtgccggaggtaggtttgattaaccctgtgagcaggtaaagcagctgcgttttacctgcagcagtaggcccgatgatggctacttttgatccggcttttatggagaaggaaatatctttgagcactggtttctgaccgtagttaacgttcacctgctgaaattcaatatctcccttaacaggcgccgtcagagaacctgcgggcataatgtcgggcatattgatcacggcgctgatcctttgataggaggcagtggcctgtgcaataatattgctcataaaaccgatgaccagtatcggaaagatcagaagggcgagataactgctgaacgccgcaaaatcgcccaggctcatactgccggtgataacgaaatgcccgcccagcgccaggatgatcaggttggcaatgccggcggtaaacgtaatcaccgggatcagtcctgcgaaaagttttatgatggataacccgaagtccatcgctttaccgttggcgtccaggaatttctggtattccagttgctgcgagttgatcacgcggatcagcgctgcgccgagtatactttcgttgatcactttattcagccagtccattacttcccggctcttgatgaacagggatctcactttacgcagtaccaggaaaaaggtaatgcctattaccggcagcgtggcaatcacagccaatgccagttcccagttgatggtcagcagcaggatgctggcgcctataataataaataaggaagataccagtgaaacgatggcctgggaaacaaacagcttgatggaatccacatcggcaatcaggttggtgagaagccgcgaggggttggcttgttccacccatgcgtaactctgaccggatattttatccgatattttagtgcgcaggttacgcgccactttttcagatacataggtttgtatgatgttctgcagataggtaaacaccaggatgatgatgaccgccaccataaattttatgaccagcgtattcagctggaaggtgccatgttcgtagctgtcgatgccgtttccgataattttgggcaaccacaggttgaggccattgctcaccagtgtaaacaggatcagcaggctaaccatacccatatatggttgcaggagactgaatacaccggcttctttctttttactaccctcttcttgtttcatttttaactggtatgtttagcaggacgcggcttttaaaggtttccacatgaggacggatccgctccgcaaatattgtataaatatctcaacaagatattgtttttttagcggtttagggaacgcattccggtgagatatccggagaaggagtagaggtggagaaggaaagaagaaccagcgcaggtccctgcccgttgggagatgcgctggcttttgatttaaatagtgacagccgccttctttttttcgtagatggcgctggccagccaataaaattcatccataaacctggctgctgatttgagcgtatgctcgctggtaaggtcgtgtgtatcattgaatgcgccgtacacttccggcaccagcagttttaccggtagtgcgtaagcgcctacgctgaggatcacctgttgcagttgtgtagctgcgttgatgccgcccagttttcctgcactcactgtaacaataccgatggctttcctggaaaattcgctgtaaaaataatccagggcgtttttgagtacgccggaaaagctgccgtggtattccggtgtaacaaatatcagggcgtctgcggcgtgcaggcgctggctcagttcttttactacctgcggcagctggggatgtacgcctacccgttcttccagcatgggcagcgggttttcggccaggtctatgagatcggtttccaatcccttgccctctaattgcttttgcaggtaatgggcaattttctgtgattgcctgccctgccggatgcttccgattaatatggctattctcattgttttttattttttgtgaagacatgcagctacctgtactgaaagtgatgtttcagcagtaaccggttattgcattgtttggttgttaccagccggagggcccagccggctggtatatgggagcgcagtatgccgctttttcatacctgtgtttgcgcaccgcacaggtataaaacccgcggaagtctatgcccgcgttgcgtatccaactagtcgttttctttatggaacaaagatagtatctttgcttaataaaccaaataaacactttgtttattatgaataataactttgccgataatgagcgggcggtatggatactgaaaacacaagggccacaacccctgtgtaagttggcagaggagctgaaagtaacgatggagggcgcgcggtttcagttgctcaaactggcaaatgagggattggtgcaggccaccacggaagccaaaggcaggggcagacctaaacagatctggtcgctcacggaggcgggcaatgcgcgtttccccgaccggcaccaggacctggcattgcggctcctgtgtaatatgaataaaacactccccaccagtatgatggacgaagtgctcgacgccacagcccaaagcaccctcgaaaaataccaggaagagctgaaaggcatcaccagcctggaaagccgtgtaagcatattagcggatatccgtaaccgtgaaggatacatggccgaatatatcaacgaaggaaacagttatctcctcgtggaaaatcattgtcccattcaggccgcggccagctgctgcagccgcttctgccagtcggaacacgagatgtttacacggatactgggaaagcatgcgaaagtggagcggctggaacatatactgggagggcagcggagatgtgtatacaggatcacggggaaatgatgctgatctttactatattttccccctatctataaataaatcagcttttatcggtatttttataccgataaatcatcgtttatattgccaggagggtgtttccagggatgatagaggagtattcaaacaaggagcatattttactgcaaaagttcgctggtggagaacaatccgctttccaattcatttttaaccagcattacaaagcattatgttattttgcctttaccattgttgcggacgcacaggaggcggaagacctcgtgcaggaaaccttttcgaagctctgggataaacgcggcgatttcaaatctgccgccaatataaaagcctttctttttattgccaccaaaaatgcctgcctcaattttttgaaaagcagggagcggcttaatgtaaaggaaaaggaattttcttatttacaggaagaacaggtcaccacagaaatagccggatttgatccggtacttacggaaacggaaatcattcagcagttgtaccgggaaatagaacatctgcccacccaatgccggcggatttttaagatgagctatctcgaaggaagaaagaatgaagaaatagctacctccctgcaaatctcctacaatacggtgagggcgcagaagctccgggcgcttaaacttatcaggagcagtctcattaaaaagaacatactgcccttactgggcatctatattacccttctcaaatattattataattattactgatcctgttagcccgtaaaattttttcagatttatttaatcgaaagtagttttttattgtttctatagtaaaagaggtgagttggaaatagatcaaaacagtgaaacaaatccattattgcagcggatagcctggctgataggccgttatcagcagggtatactgacagccgccgaagccgaagagctgcggacctggtgtgatgcctccgcggagaaccgtcttttttttgaacagatgaccgacccggatatactccgtgataaattgttgcaatacgagaaatttgatgttactgccggctggaacactttcagtgcaaagcatttcccggtaaaagataatgtgccggtacgcccgttgtatcgctggtggaccgctgctgcggctgttttgctgttattgggtgcaggcttatattttcttcgcccttctgccccgcctgccccggtaacggccctttccaccacgtctattatgccgggtaccagcaaagccacgttaacactggcagatggttcggtaataccgctggatagcaacggtaaccgcgtgatcacacaacagggcgcccttattcacctgaataatggtcagctgcaatacaacgcgcaggattattctgcacaaactacgctgaacacactggctacgccaagaggcggacaattccgcctcacgctgccggatggtaccagggtatggctgaatgcagcttcctcaattactttccccactgcattccagcaggggaaaagggaagtggagataaaaggagaagtttattttgaagtggctgccatggcgaaaatgccttttcaggtaaaagtgggccaccaaaccaacatagaagtattaggcaccagttttaatatcaacgcctatacagatgaaccaggcatcaaaacgacccttatacaaggagccgtaaaagtaaatgcaggcaacaattccagggtattattacccggtcagcaggcattggtaaaaagtcctggaaatatcgatatcgtagcgcatgcagatatggctgcgatactggcctggaaaaaggaagaatttaatttccgcgatgcagacatccccaccgtgatgcgtcagctggccagatggtatgatgtaacaattgtttatgcaggtaatatccctgcccgccggttccaaggggaaattcaacgtaatctgccactgtcggatgttttggaaggactgcaaagtaccggtatccatttccgcctgcagggacgcagcattatcgtggaaccgtaatgggtttattttttagctattgtcaactgaacatttatgcaccaccaacttcagagattgtaatgccgctatacggataaaaaaaccggaggtgattggacccacccccggcgaatatgtccggatgatagtagcactaagcttgtacatacttgaatactgattatccatcctaacaaatgcaaatctatgcaattgaattattatggtaaagtcctttctatgcctggactttccccaaccaaaattgcacttactatgagattaacgattgttctcatgattgtggcgacattgaaagtatctgcgggtgcctttggtcaaacagtgtctgtatcggtgaaaaacgcgccgatggaagaggtgtttacctccgtaaaacagcaaaccggctacctgttcttttacgaccgggacttgctgcgcaccgtgaaaccggttaccatcaaggcggaaaacaccaggctggcagacttccttaccgaaatctttaaaggccagccactggattacacaatcaaagacaaaacaattttcatcaaaaagaaagcgctgcccgcaggcagcaacaacatcagcaccgcaccggaagccactcagcaaccggtgacgggtgtggtgaaagatgccgcaggtaacctgcttatcggggtaaccatcaaggtgaaaggctctaatattggtaccatcacggatgaaaacggacatttctctctcgcagcaggtcccggcgatgaactggtgctaacctacgtcggctacgaaccatatactgttcgtatcgggaactatggcccattacagctgttccttcgccaacgcgccagcagcctggacgaaactgtagtgattggctacggcaccaccagcaaacgcaataacaccggatcggtatccagcctaaaggcggaagacattgcctcacagccggtaatggacccgctggccgccatgcagggccggatggccggtatgttgatatcatcttctaatgggttacccggatccagctttaaagtagtgataagaggacaaagttctgttggccgcccaaacgatccgctgtacatcattgatggtgtacccttttattctgatccgctgaaccagtttacttctgccaacggtaatcaaagcccgctggctaccatcaatccttcagatattgaacgtatcgacgtgttgaaagatgcagatgctaccgctatctacggttccaggggtgccaacggtgtagtgctcatcaccaccaaaagaggtaaatcaggtaaaacacaggctaacttcaacgtatacacgggcgcaaataaagtagtgaataccgtgaaaatgcttaatacgcccgaatacattgccatgcgtaaggaagccttcaaaaacgataataaaccatacgacgaagatgttgcaccagacctgaccctttgggatcagcaacataccaccgactggcaaaagttcatgatcgggggcactggtcatactacggaagcacagggttcagtgtcagggggcaatgaacaaacacagtttatattaagcggtacgtatcacaaggaatcaacggtaatgcctggaagcctcggctaccagcgcggtgcaggccacttcaatttaaatcacagcagcgccgatggtaagtttaacatcagcacttctgtgaactattccgccaataaagataattcgctggcaagtgatcttaccactttctttaacatgtcgccaaattacccgctgtatgactccgccggtaaatattattggttttcaacagctcaaaatccacaggcatacctgttgcgccgttctgaagtaaatactaataacctcgtggccaacagcaccatcaggtatactatcctgcctggactgaatctgaaaaccagcctcggatataataaatccaatatgaagcaggtgcaggtatatccggatgctacctttaatccgcttacttccaccgggagtatgtcgtacttcggtaatgccgatgtcggatcttacatcatagaaccacagatagattataacaaaaccatcgcaaaaggcgatctgcaggtaatggtgggcggtacctggcaacaaaccattaaacagggacagtccgtaaaagcaaccggcttttccagtgatgcactgctggaagaccagcaggcggccggtctcgtcctccctaatccatcgcaatactccttttaccgctacacatccgttttcggaaggatcaattataactgggacggaaaatacctggtgaatgccacttatcgccgtgatggctccacccgcttcggccccggcaaccgttttggtaatttcggcgctataggcgctgcctggatatttaccaaagaaggttttatgaaagatgtgagcttcctcagctttggtaaacttcgtgcaagcatcggccttacaggtaatgataacataggtgactacaagtatctcgacagctggacttccaatccctatccttatgatggcgtacccggactcgcaccttcccggttacctaatccattatataaatgggaggaaaaccgtaaaaaagaaataggactggagctgggattcctgaaagacaggatactgtttaacaccaactattatcataacatttccggtaatcaactggtggagaatcagcttaccccgcaggtgggattcccctctatcactgccaactttccagcaactgtgcttaacagcggatgggaatttgaagtgaatactattaatattcagcgacctggctttacctggaaatcatcgttaaacctgacggtaagtaaaaacgaattgaaatcgttcccgggcattgaaggctctgcttacaaagacttgtacgtagttggacagtcactgaccattgtaagaggatacaagtttgtgggtattgatcccgaaacaggcctggcacagttcttcagtaatagcggcaccaccaccgatccggcggaatttgacgactacgtaacactgggtaaaacgatgcctgcatattacggtgggttacaaaacagctttacttataaaggcattagtcttgatttcctgctgcagtttgtaaaacaggaaggcccgcaaattggctatggatacagtagtccggccatcggcacatttgccaaccaggacctgcgcgcactcgaccggtggaaaaataaaggcgacaacgcaaatgtgcccggcgctactacctccgcaggaacggctaactacaggaactacagcctctctaccgccagttggggcgatgcttcttatatccgcctgaaaaatgtttcggtgagatatgacctgtcgaaatataccaaacgttggaaagttaataatatcagtgtttatgcactggcgcaaaacctgctcacctttaccaactataaaggtcttgaccctgaaacacagggtatggtaatgccgccattgaaagcatataccatcggctttcagtttgctttataaagaatattcctgttttgcagatcataaaaagatttaccatgaaacgaattcatatatttttaatcggcgtcctccttttcagcagcagctcctgcagcaagtatgtggatacgccgttaccaaagaatgagctggtatccggactggtgtttacagatgataaaactgctacggccgctgttaccggtttatatggcaccatgtactcgttcaactaccagtttgcaaatgtgctcatcaactacctgactgctatgcaggcagatgatatggcttatttttccagcttcgccaactacgatgtttttaaagaaaacaggttactgcccagcagccagtatgtacaaagtatgtttgcggatctttacagttatatctaccagacaaatgcctgcgtggaagggctttccacagcaaccgcattaacgccttctgtgaagagccaattaatgggagagtccctgttcatgcgtgcattctgttatttttacctggtaaatatgtatggagatgtacccctgatcaccggcaccgattacaaagcaaatggtgtgaaaccacgcgcaccacgtgcagacgtgtataatgctatcatcacggatcttaaagcggcagtggaattaatgggagatgattatcctacggggcagcatatacgcccggataaatctgtagccaacgctttactggcaagggtttacctgtataatcaaaattgggcgctggcagaaaccaccgcatcactggttatcggcaatggccattattcactggtaacagatctgaataaagtattcctggctaacagcgatgaagctatctggcagctgcagcccctcaatgtactgggtggccgcaatacctgggaaggatttacttccacaccagctattaaccctaccacgggcgcctttggtaccgcggtattcaggttggatactaccaacctgattaaaaaatacgaaccgaatgatctgcggcttacgaaatggattgcctctaacaagaccactgcaggcgttactgtttactttccctataaatacaaagtaagaaccagcaccagcggcattaccgaatactccatggtaatgcgtcttgcagaacaatacctcatccgtgcggaagcccgcatccagcaaggaaaactggatgatggccgcgccgacctggatgctatccgtcaacgcgccggtttgcccggtttgtccgcttccctcacacaacccgccctgctgctggcagtggagcaggaacgaaaagtggaattgtttgcagagtggggtcaccgttggtttgacctgaaacgtaccaaaaggtcggatgcggtgctgggaccgattaaaggcgccaactggcagtctaccgataccctgtacccgattccttctgatgccatcagaaccaatgttaaccttacccagaacgaagggtacaaataaccattgccgatatgaagaaattaaccatcctacttttactggctgccatggcagccggtaaaatatatgcacaacaacgggtagtgatcaccccggaatatccggaacgtggtcagaccgttacggtcacttacgatcccgctgcgccgggagctggcattccggttaccgctgcgccggtcaccctcgtgttttcctattccaacttttacaaccttgcatggcgcatgaatatgcagcgtaccgggaataaatggaccacctcttttgtactggccgactacaccaccttcgctaccttttacctggaaagcggcgatgctgtggataagccggcaaaagaccggcactacgaagtagcggtgtataaaaacaaagtgcccgtaaaagacatggcgctgtacaaagcttacagtcttagtgcgcaaatgggcaagtctcctctactggccgataaacaggccgcgctttataaagaagaactgaaacgttacccggacaactacgaagcaaaactgcgcctgcttacctacgaaatgaacaaggccaccaacgccaaagaaaaagaaaagttcaaggcacaggcacaccaggtgattgcagacaaatttaacagcgcgcccacaactcccggcaacatgaataaggtaaccatgggctacctgatcatcggcgaaaactcccggctggactctatccggcgcgtagtgatggaacgctacccggaatccgcactgggccgggatatcatgaccggcatcgtggcgaaaggaaaagacacagcccggcagatcaccttctttgaaaacgaactgaaaaaggaaaccccggaaaacagggaatctttcacagaaatgcacgatgtcctgtttcaatattatgctgtaagaaaagacagtaacaaagcattatatcatgcccgttttatgaccaccgaaaaggaaaatccttacaaggtgatcacctggcaacagattgcgcaaacactgctggataataacctctcgctggataccgcacgccggtatgcacaactggcgttagacagcgtacgcagctacccggtaggcgtgatccgtcatttcccggaaacgggatacatctatccgtatgcagacgatagtacgcgtaatgcggtgtataataaagccagccggcatctggcatctgtactgggtctcatcgatatgaaacagggacgcctggcagcagcagacaaacacatggaacaagccgtggattattatgcagataaagaaacactcgacaacgcggaaacatattaccagcaaaccaataataccgctcaactgaaccagctgcaggagttccggaaaaaaatactgatagaaaaagtaaagaaacaacggatcaaccgtcccgccccgccactcagctcctttgtggatatgaaaggtcagccggtatcagccgcttcactgaaaggcaagatcatactgatcgacttttgggccacctggtgtgtaccctgcatgcaggaaatgccctacctgcagaaattgtacgatcaatataaacaacaccccgatgtggtttttatgattgccaacagcggcgcccgcaacaccctgggcgacgcgcagggctggagcggtaataaaaaatattccttcccggtgtattataataccgacccggccacaggagataagttcaagtttaacatcattcctgcttcctatctcatcaacaaagaaggaaacatcattttcgccaacatcggctttgaaggaccggaagtggaagaaaaactgaaacagcagctggagatcctgttaaacgactaaatacttaaacgggtaccattaaatacttaagtagtcaccataaccagccggaaagattcccggaaatttgtcttatcaaaaaaaataaaacaaaatggcaacaaaaaacaaaatagccctggttactggtggcagtcgcggattaggtaagaatatgtctttacaactcgctaaaagcgggcacgatatcatccttacttacagaagcaaccaggcggaggccgacaaggtagtagcagaaatccaggctatcgggcaaaaagccatcgcctaccagctggataccggcgacacaaaatcgttcgatggattcctggcaacagttgcggcgcacctgcaggaaaacaccggcgaaggcaaattcgatttcctggtaaacaatgcgggcatcgacagaagctccctcatccccgatactacggaagaagattttgatgagctgtatcaggtgcacttaaagggcgtatacttcctcacacagaaagcattgccttttattaataacaatggtcgtatcattaatttgtcgaccggcctggcgcggtttgccacacccggatatgccgcctacgcttccatgaaaggcgccatagaagtgtttaccaggtacctggctaaagaagtgggtgcgcgcggcattactgccaatgtagtagctcccggcattattgaaacagattttacaaaatccgtttttgaacatgcaccacaggcaattaaacatattgctgcccaaacagcccttggacgcaccggcgtaccggacgatattggcggcgtggtagcgttcctgtgtaccgaagaagcccgctggatcacggcgcaacgtattgaagcttcgggaggcatgttcctgtaatagagtaaaacaaattatgcagcacggcgggtttcctgccgtgctttttttatatcgggcgattaaaataggtttatttttggctgttgccacttaataaaccatgaccgtaatcggacacctgctgtattgaaaccgggcatccggtagtcgtgtattgatgttaaagtgctgattatcatgtctcctgatttccggcatccaattagaacgccctgcatattatgtttaagaattacttcagcattgcactcaggaacctttggagaaacaaaggtttttcagccatcactatattcgggctggctattggcatgaccacctgtttacttatcactttgttcgtaacagatgagctgagctacgaccggttcaataaaaaagccgacaggatctatcgtatcaatgctgatttctttgtaaacggcaatgcctttaaagaaagattcagccccagccagctgggcccggtgctgctgcaggaatatcccaacgtggaaaactatgtacgatttatccgccagggaagtatcctggtaaaaaaagggaacaccaccctggtagaaaaaaatgcctgctttgcagattccaccctgttcgatgtattcagcttgcagataatcagcggcgaccctaaaaccgcgctcacccaacctaataccatggtcatctccgaacggatggcactcaaatactttaatagcaccgatgtagtgggtaaaacactgcaaacagataatgtggccacttaccagatcagcggtgtaataaaagatgtgccggatcagtcgcacctgcacttcgattttgtgcgcgccatgtccgaattacccgaaagccgggaaaacggcggatggatgtcagacaactacgccacctatgtattaatgcgggaaggcgccaccggcgcgcaactgcaaagctatgtggatgccgttaccaaaaaatatatggaggggccgctgaagaaaatgaccggcagtacctttgcagatctccaaaaatcaggggggcattttggatataacctgctgccgctcgcaagcattcatttatattccccgctggccgatgaagcagaaccttccggcaatattcaatatgtgtacatcttcattgcggtggcgatcatcattctgctgattgcctgcgttaacttcatgaacctctccaccgcccgctcagccgggcgcgccaaagaagtaggggtgcggaaggtgctgggttcccaacggtcttccctgattttccagttccttacggagtctacgctgaccagcttctttgccctgatactggcagtggcattcgccattttactgctcccgtatctcaaccagctgtcaggaaaaaacattacgctggaggcggggtattttttatggctgctgcctttcctgctggtaactgctggtgtgatcgggttgctggctggcagttatcccgcctttttcctgtcgggctttgagcctatcaaagtgctgaaaggccggttgaacagcggtttcaggaacggatggttgcggaacagcctcgtggttttccagtttgcttctgctatcctgttgattgtaggcacgctggtgatcaacagtcagctgaattatatacggaataaaaagcttggttatgaccgcgaacaggtgctcatcctgggcaatacccagtcgttgtggacacatgcccgcaactttaaaaatgaagtgctgaacataccaggtgtggaatcgggtaccatgaccggctctttgcctaccgatataagacagaacaccaatatctattcaaaagatgccgcccgcagcaccgggcaggtaaccggcgtaccggaatggtatgtggatgcggattacatccacacaatgggcatgcaaatggccagtggccggaatttctcgccagacatgccttccgatacttttgctgtattgctcaatgaaacggcagcccggttatttgatttcagggatctgaatgaaaagtatctctatgccgatggagacaggccgctgaaagtaataggagtggtaaaagatttcaatgccggtagcttaaggaataaaataccgccaatggtgttccggctacgggaaaatttccagtcaatggcattccgcatccagaccagtaatatccagggactcattgcaaagataaaaaccgcttacgaagcgcagccgggtatgggtgggcagccattcgtctattcttttcttgatgacgattttaaccgcctctatattgcagaacagcgtacaggcaggatcttcatttcctttgccatattggccgtattaattgcgtccctgggagtattcgggctgatcacttatgcagcggaacaacgtacccgggaaataggcatccgcaaggtgctgggcgcgtcagtaacgggtattgtggccatgctgtcgaaagacttcctgaaactggtattggtggctgttgttattgccagtccgcttgcctggtatgtgatgagccggtggctgcagaattttgcctaccaggtaaaaatgagctggacaacctttgtattggccgcgtttattgcgatcgccatcaccattttaactgttagctaccgggctatcagggctgctacggccaacccggtgaacagcctcaaagcagaataatcagttggccagcggaagttccaggtaaaaggagcttccgccttcgcggttgttttcaaaccagatctgtccctcctgcgcggtggtatattccttacagaggaataaccccagtccaatccctttttcattatctgttccgaaagtggaacgtactttcagggagaaaatatccggttgcctggacaggtcaatacccacaccgctgtctctcacttcaattaagcatttattgccggccctgctggttttgatgaagatggttccaccggaaggggtgaacttggcggcattgccaagcaggttacgcacaatcagctgcagcatattgatgtcggccatcacttttatagacgcgtctatattggtatccaggctgatcttttttttggataccgccattttgttgattttaagaatgggatgtatggccgatgccacgtctacaggagtaagatttacattgagcccgtccatttgcgttttagaccatacaaggatattatatagcatctcctgtgtgctgttgaccacgtacagcagttccgtttctatctgggttttattttcggggtccagttctatttcccgcatcagctggaggtacgattgtatcgctgccaatgggttacgaaggtcgtgcgagatcagcgaaaagagtttgctcttttccgtgttcatgatttcaagtgcgcgcgttttttcttctccctgctgcttttctttgttatacgcatttttcaggtaaaccgttcctacgaaaattacgcacacgcagataatataggtaggggtcatatctgcaaaaatgtctttcctcgttttataaaccgcatctaccaccgccgggtgataatattcccacatgatcagcccgagtacggtgagcaggttcagcgccagccaccagtaatattgtttccgggaggaaatcagcatgaccaggaagaacgccagggtaaaggacaacagggaggcgccctgtattcccccgctgtagaaatagttaatagcgaagctcacgttaataacgatcgcggcaatggctatactgatatttaccttcttccggtatctcgacaaaaaataaataaaggagaatgcaggcaccagtaaagcaaagatgagcgaggtaaccgtaaggccggtaatataattatatggtacgttaatggcaataataaagagggaaatagcacatatcgcattgaatatgcggttttccagcgagaaccgtctggggtctcctatcaggaagtgtgagaattgtttcaatcgttgggatatcgttatggttccgggtgttgacatgttactaatttaagcaaaaacaactgctgttggcagtgaaaatgccgggctcaggataatcatattattgtaatgtcacaattttttcgcggttttctttatactacctgattaattttaaaaaaaatgcagcgtggccaaagaaaatctgaccgccatcaaaagcaatatccgcgccattatctgtaagcgaagataatattgtcccaaacgcgaaggggtatacgtaaagaccatccgtttccgttacattttgctaaatgcattttacaaaagcgggaaagctaaaataattatcattaattttcggccgcgggagagatgatgaggtattcacccacttttaatatgcgcgaaaaatgatgagtgatggagacttattacagcttataaaaagagatgatacagctgcttttgaatctatctatgataaatattggcaggccctttatttaaaggcttgtcagcgtgtggataaagatgaggcgaaagacatggtgcaggaggtgatgattacgttatggagaagaaggaacgatatccgggtaacgcaggagggagacctgggccggtacctgttcaccgccatccggtaccgcgtgatcagccattatgcctttagtgccgcagaaattaaaaaggcggatttttttgatactttcgacgattacattgcgaccgatacattagaaaccaaagaactaaaagccaaaatcgaaaccgagatcggcaggttgcctgcccgcatgcagcagatcttccgcctgagcagggaggatgattacaccatcgccgatattgcaaaaacacttaatatttcagaacaaaccgtaaagaatcagctgacagatgccttaaaacgcctccgtacttcattgaaagcctcttccaccggcgactggacactggtattaatctacctcttctcccagttacatcagcaacagtagtccgccggataaagtttttcccggcgtgcaggattggcccgatgatctaaccttttccctttgttaccggcaggctccccgcaggggagaggcggtactgtgtcatccattgcccggggcgcatcattcatgcagacgacggggcgttcccggaatggctgtccccgggaaggccatatcattggtggtaaagggctatctcccggagatgatccgctgccaggcatccttttcccggagggaaaatattttttaaaccggactagtaccggatattattttttcagataagtaataaaatcgcgcgctttggaagtcagtaaaatcagacagctttttaaaaagtatatgctggggcatagctccggaccggaaaaccaactcatagaacaatggtaccagtcgttcgatgcagcagctttaccagaaatggatgaggcggagcaacagcatataaaacgcgaaatgtggctaaatatccagccgcaaattgaagtcgctaaaacgttttatcttacccgtggctggaaaagagctgcagcggctgtattgctgctggcaggcgccggggcggcctggtacctgctgcatccacacccgcgggctacctggaccacctacgctacccgcaccggtgaaagaaaaaccattcacctcaacgacggatcaatagtgatgttaaacgccggctccacgatccggatacccgacaacctctccaaagaaagaaaactcgacctggttgacggggaagccttctttgatgtgaaaacaaatcccggcgtaccgttcattgtagaaagcggtccgctccagaccaccgtactgggaacgtctttcaacatcgccgcctataaagaaatacacaccctcagcataggagtggtatccggcaaagtaagcatctctggaaaagcctcacccgcacacatcctcgggcaaaaccaggaactggtgtacaaccggaacaacgggcagataaaagtttcaccggtagacgaacaactgcccggatggaaggatggcaaactcgttttcaatgatgttactttccacgacatggtgatactgatggaaaaaaatttcggcatcaccatcaccaccacacaggaacatgtaagaaccaccagatataccacggaattgccaacagatatggcgcccgaaaaagcagcacaggtgctggcggcgatccatcatctgaaagtacgcacgatcaatcagcacaccgttatttacgaataataaacaatgtatcaccaaagctaatcgcttaaaacaactacgtattaatgccacgtaaatggaaccttttgttaatgctaacaattaatgcctaaccacgtatgaagaaaattgtaaaaaatttcagaaaacgaatgcttgcagtcgttttggccctgacgtgtgtcccagccatactgccggtatacgccggccagggacaaatcctgcaggaaaccagcgtcaccattgcattgaaaggaggtagcctggaatctgccatcagggacctgcaccgccatacaaaaattaattttgcctacgacaggcaactgctcagcggctacaaagtagaagggtactcgttttccaacgagcgactggactacgttctcgaaaaattactgcaacacaaatccctcggatatgcagaagtaaatgatattgtagtcatcagtaaactcactgcccccaaagcggccatgacccgccaggaagtagtggtgtccggtgtgatcaaagatgaaaacggtaaaccacttcccggcgtaagcgtagctgtaaggggcgtaagcaccatgaccaccaccgacgccaacggacgttacaagatcatcgtaaacgctgctaccgatgtactggcattcagcttcattggttatgaaacggcagaaatagtagccggcagtcaaactaccatcaacgtacaactgaaagtagccagcaaatcactcggcgaagtagccgtagtgggtttcggtacccagcgtaaagtaagcctggtaggcgcccagtccactatccgcccggcggaatttaaacagccggcatcagacatctcttccatgctggcaggccgcatcgccggcgtaataggcgtgcagcgtaccggcgaacccggtaaaggcagcgccgatatctggatccgcggtatctccaccttcggaggcggtaataaagcaacgcccctcatcctcgtggatggtgtggaaagatcgattaacaacatttcaccggaagacattgagtcctttaccatccttaaagatgccgccggtaccgccgtatatggcgtgcgcggcgccaatggtgttattctcctgaaaacaaaaacagggaaagtaggtaaaccacagatctacttcgattataatgaaggcgtaaactcctttaccaaacgaccggaaatgctcgatggtgttacttatatgaacctcgccaacgaagcctctaccacccgcaaccacaacccggtgttctccgaagaaactatcgaaaaaacaaaaagtaacgtggacccgctgttatacccgaacgtaaactggatggatgctgtattcaataaatacggtcatacccgcagcgctaacctcaacgccagcggcggtgtggaaaatgcacagtactacgtatcactcggctactataacgaaagcggcttcctgaaaacagacgacctggagaagtacaattcttccttaaaatataaccgctataactttacgtctaacctgaacctgaaagttacaaagtccaccaagctcgatgtaggcctgcagggatacttctccaacggtaactaccccggcattaacacccacgatattttccagagcgcgatggacgcctctccggtggtgtatcctgtaatgtaccctggtggcttcgttcccggtcgctcggccaacggcggcttcaggaatccttatgccgaccttacccgcagaggctatcgcaacgaattcaggaaccagctgtactctaatatccgggctacgcaagacctgaaatccattacggaagggttgtcggccaccgcgatgtttgccttcgatgtatttaaccagaactatattacccgctccaaacgcgaggacacctggttcccggatatgaacaatccgtacaagccggatggtacgcttaacctgttgaaaacattcaccggtaatcaatacctcggcttcgataaaaacgatggcgaccggcagaccacccgccagttttatacagaggccgccatcaactacgaccgtggttttggtaaacaccgcgtaaccggtttggggctgttttataccagcgataaaaccaataccctcgccggcgactttatcaactccatcccggaaagatacctcggcctggcaggtaaagcagcctattcttacgacgaccgttactttatggaattcaatttcggctacaacggctcggaattgtttgcaccggaaaaccgctacggatttttccccgccatcggcttagcctgggtaccttccaatgaacgtttttttgaaccatttaaaaacgccatctccttcctgaagttccgctactccaacggtaataccggtctcggtagcgcagaagaacgtttcctgtatatcaccaaactgaatgataacgatcacggctatacgtttggaaaaggttttaacggcggcagtggtatcagcatcacccgttatgcatcggatgtgcgctggtctgtttccaacaaacaggacctgggtatagaactgcgtacactgaacgaccgtctccttgtaaatgtggatgtgttcaaggaacaccgtaccggtatcttcctgcaacgcgcttccaacgtggatttcatgggattggacaatcagcagtacggtaacctcggcgccgtggaaaacaaaggcttggacgccaacctggaatacaatgcgcgtatcgggaatgtagaagtatcggtgcgaggtaacattacctggaaccaggataaagtattggaagatgaccgcccgccgcagctgtacccatggatggaacaccgcggcaataatatcctggcgcggtatggttatatcgcagaaggcttgttcattgaccaggcagacatcgacaaaagcgccgttccgggttcccgctcacaggtgaaaccgggcgacatcaaatacaaggatcttaacggagacggtaagatcaactcctccgatgaaacaaagatcggccgcggcgacgtacccgcaatggtgtatggcttcgggttaaatcttgcctacaaaggatttaatattggtttcctgttccagggaatctccgatgccgatcgtatgctgcagggcagcgccatcattccgttcaatggcggtggtggagaaagcaacgcctatagcattgctaccgacaggtggacccctgaaaacccacgacaggatgcgttttatccacgccttgcctatggcgaagcagagaatgtaaacaacacacagccaagcagctggtgggtaaaagatgtgagcttcatccgcctgaaatctgcgcagatcgcctacaacctgcccgccagtttgctgcagcgcataggcgtccggaattcatctgtttacttacagggtatcaacctgcttactttcagcaagttcaaattgtgggatcctgaattaaataccgacaacggttctacttatccaaatgtgagaaccatttcgctgggagtaaacctgaaattttaatcacgtaagcaactgatcatgaaaaagctattatatattttactgggcatcgtgttattgacgtcgtgcaaaaaatacctggaccaggtgccggacgaccggctaaccatcgaggaaactttccgtacctgggctaccgcacagaaattcctgaacaacgtgtatgtccgcataccggatgaattcggacaacgcaaccccggcgattacaacaaccgcggcttatggaccggtgggtgcgatgaagcagattatgtgtggggatttgtacaatccaacagcgtaaacatcggcagctgggacgccaaatccggttttgtgggcgactactggaccaatttttaccggggtatccgcgcagccagcgtatttattgataacgccgacaaaataacagatctctcaccggatctcatcacccaatacaaagcagaggcccgggcactgcgcgccatgtactatttttacctgatgcgtatatacggtcccgttgtactcatgggtgaaaagccggtagaagtggatgccagtctccagatgccgcgcaactcctttgatgagtgcgtagcctatgtaacctccgaactggaaacagctgcggccaacttaccggtaatacccaacaacgatcaggactacggccggatcagtaaaggcattgcactggccttccgcgccaatgcactgatgtacagcgccagcccgttgtttaatggcaacaccgatatggcggccctgaaaaacacggatggcaaacagctgatcagccagtcgtacgatgccaataaatggaaactggcagcagacgcctataaatctttcctcgatcagtttgtgccttctacctacagtttatttaggaagaataatgcaaagggagaatttgatccttatctttcctgcagggatgtattcctgaccgactggaacccggaagtgatttttgcccgtcctgccaattcgctgaattcccgtcagtacgaaatgacgccgttccacagcggcgcgccttccagcgatgtacggggaagcggcggcttaggcgctacccagaatatggtagacgcattttttatgaagaatggcagaagcattgatgacccgttatcgcagtatgtaaaaacaggctattcagattttaccggtcctaacgaaacggcgcccagtaatatctataaccaatgggtaaaccgcgagccccgtttttatgtaaacatcacttatgatggaagcacctggctcaataaatcttttgggaatatcgtcacccgcatctacaatcacggtaactccggtaaagccacaggcaataacgattacagtcctaccggctatattgtacgcaaggcgcagggcctcggcaaatgggatgtaggtggccgtacgctgatgctcatccgcctggcggagatctatctcagctacgcagaatgtgtgaatgaagccaatcccgccagcccggaagcactgaaatatgtgaacctcatcagggaaagggcagggattccgcaatacggatcggcagaattgccggcacccgccgggcaagccgccatccgtgaagcgatccgcaaagaacgccgcgtggaactggcttttgaaaataaccgtttctttgatgtacgccgctggaaaatagcagaacaaacagaaaacggtcctgtctatggtttgaacatcggatctgatatgcccgacttcctgcaggtagtgccttttgaaacccgcgtatttgaaagaaaacattacctgttcccactgccggcagatgatgtggataatgataaacaactggtgcaaaatccaggctggtaagtatatttaaagaaccaccggaagccggactgtagtaccggctcccggttttaacccgatcatatgtataaaataacctgtttactttttgcagtattgctgctgcacagcaactgctccaaaagcaacgcaaaagaagatcctgttacgccgggaccaacgcccacggtatcttttactaccaaagatgcggctactgcctacgccagttttaaccagtatttctacagtacggccgacaagctctattacagcaataccgaaaagaaaggcatcggcgccatctgggtccaggccatttactgggacatggccatgaacgtatacacacgcacaaaagatccggccgatcttcaacgcatcaccgatatcttccagggtggttataaccgctatgataaatacaactggaacaataccaaggaatggtttatttatgatgatatcatgtggtgggttatttcactcgcccgtgccagccaggttaccagcaacaaggcatatctcgacctctccgtttcgggtttcaaaagggtatgggatggatcttatgatccggataaaggtggcatgttctgggactttaaccatagcggtaaaaacgcctgtattaacttccccacggtgatcgccgccatgaccctgtataagatcaccggcgaagccgcttatcttcaaaaagcaaaagacgtgtacaactggggcataaataatctctatgatcccgctaccggcagggtggcagataataatgtaaatggtaacaaaggctggtccgattacacctacaaccagggcacgttcattggagcagccgtgatgttgtacaaagaaaccggtaccgcgacttatcttgatcaggcgaagctcgccgctacctatacgcagaaaaccatgagcgatgtaaatggtattatgcccgccgaaggcgactggaacgaacagggcatattaaaggccatcttcggacaatatgtgatgacgctgatcaacgatgccggtcaaacgcagttcctgccctggatccagaaaaatatcaacgccgcctgggggaaccgcgacgttacccgtgggttaacctaccgcaactataaagtgccttgtgtaaccggcgtgctgcaatcctatgaggccagcagcgcagtatacatgatgcagatatgccctccggcaaattaatggcaacgcatcgttttcaggaggtaaaacgctatttttgcgctttaatcaatatacctcatgaaaacgatgttgttttttacgctgacttgtttgttcgcctgttttgctacccctctttttgcccaggaacaggaatttatcttcaatacctggtcgttaaacaaagatgatagccggtatatttttgcagatacggcactggtacgtatgagcccggataccaaacaagccgccatcgacacgctgctggccggcgatgatattactacggtggaggtattgcccggcaaaatgctcacactcaaaggtctcacccttccctgggtacagattaaatacaaaaaagatggtgtggaaaaacaaggctacgtgtgggaggggctgatctcttttcctcctatgcgcagaggcgacatgaaatttgtatttgcctacgaccgccgagtggatacactgatcggcaatgaaaaacatccgcagtatattgtgaaattaaaagccgtacaagcccgtaaaatccttgctgccaccacattccggataatggatgatgaatccgccggtttttcctacgcgaaggtaatggccggtctcggtcttaccaacgtgcaaaatatcgtatctgttggctttggtggagcagcctgtggtgtctccacaaactattattatttcgcctggatgaaggatggacggatcgccgcactgccggaaagaatggatgtgggtgatgccggtgtatattatcatgaggagtctttcattttccccggcgagaaaaacggtctaccagatatcatcatcctgaaaatgcatgaagaagaagaaacagataagctggataagaacggggaaccggttatgtcagtaaaagaagagcttaccaaatacagctgggatggcgtaaacggcaccttcaaaaaactggggaagtagaagaccgccggtgataacatgatttgtgtttctttgtatcttacatagatgttagctgtaatggtaaaatgggtactgaaaacaacaggcgtactgctcctcctgtatgcagcggtttgtgtccttgtgtatttcatccaggagcgcttgctttttttcccggagagattaccgcctgcgtatgttttccagttccctgagcccttcgaagaacgcactattaccactgctgatggcacacagttaaacgggctgctatttaaatcccgtggcgacaaaggccttatcttttatctccatggtaacgccggctcccttaggtcgtggggagaagccgccagggtatatacacacctcggttatgatgtatttatgtttgattaccgcggttacgggaaaagtagcggtaagatccacagtgaacagcagttttatgctgatgcgcaaactgcctatgacagcgtaaaaacagtttacccggaaagtacgattgttattctcggttattccatgggcacaggtaccgccgcacgcctcgcagcagacaatcatcccaggcaactcatcctgcaggcgccctacttcagcatgaaagatatggccaggtactattatcccatgttgccttcatttttattgaagtatacatttcctacttacaggaatatacaacgtgttaccgttcccgttaccatctttcatggtgataacgacgaagtgatttactacggctcttccgaaaaactgaaagcatattttaaaccgggagatacactgatcacactgaaagggcagcggcataatggtatgacggataaccccgaataccaggagcggctgaaggggatattggaataactcatgcgcttatcacctttactcccttcttcttacaatacttcaatgcggccggatcgccatccgtaataattgcatctaccaactccagtcctgcaaaattcaggtaggaggttttccctatttttcctgcatcgcataacaggtacgtatagtcactttgtgtagccagtgcagtggcaatggctgcttctttttcgctgtgtgcaaacaatccctgtgccgagaggccatctacaccaataaatgccttgcctgctttataccgttgaatatgctctgtggccattgtaccatgtatagcctgccgggccgcatcgtattcaccgccgataatgttgagggatactgcggaatgttgcaactcaaatatcaccgggagggagttggtgattactttaatctttttgttttttataaactggcataagcggaaaacagtgctgccgcaatccatgaaaataatatcgccgtcgttgatttccgctgctgcttttctgcagatcttatcttttgctgcttggttggctgctgctttgttcacaaattcaaagggggaatcctgcccggtcaccgggatagcgccgccgtgggtacggtacagcagcccgtcgtccgacaactgattgagatcccgccggatggtgatttctgaaatacccaatgtctgcgccagttcgccggtggctacttctcctttcgcatgcagcagcgccagtattttttgttttcttagctggaaattcattttaaataattaacttgatcaaaaataatcaaaaacgatcataatcgatcatttaatatgaaaacaattaatattctggaaacagccatcctgtcggacaactggtacacgctcaagaaaatcacctatgaaatgaccggcagcgatggggcagtagtgaagcaagaacgggaggcgtatgatcgcggcaacggagctactatattgctgtataataaggaacatggcaccgtagtactaacgcggcaattccgcatgcctacctatatcaatggcaatgaaacggggttgctgatagaatgctgtgccggtttgctggatgaagataatgcggaagaatgcatccgccgggaaacgatggaggaaaccggttactaggtaaccgcggtggagaaggtatttgaagcgtatatgtcgccgggctctgttaccgagatcctgtatttttttgtggccgcatacacgaaagagctgaaagttcacgaaggcggaggactggaagccgaacaggaaaatatagaagtgctggaactgccatttacgcaggcaatggacatgatccgcaccggggaaatcagggatgggaaaacaatcatgctgctgcaatatgcggcgcttcatcacctgtgtggctaaacgaaaaagcaatgcaggtatcagttatccgccaataccactttgttttcatctttcatcagtaaggcctggttctttttgccccattgatccatggcctttatcaatggtaaagtgcttagtcctacttctgtcaggtaatattctactttcaacgggataccggcatatactttcttgtacagtatgccaagatcttccagctccttcaggtgcatggtgattacgcgcatactggcgccatctacttccatctcgcggtgaatttcacttggccgcctgatatcatcatgaatacactcaatgatccaggctttccatttaccgcccaataccttcatgaaaatgctgatgccacagtgcagctccgggatttttttctcgtacatggtgattcatttgcaggaaagataaacattttacactatttcataaaagcgcatcgtcgtaatgcaacaggggagtataccgaaaaatttttccatgggtgaaacttttttcggttattgtccgtcaccgccatagtcaagacatttgaggtctaaaaaatgagacgatgacaacaaataaaagtgttgctgtaattggattaggccctatgggatttgtattggcgcgcaccctgctggataatggttaccgcgtaaccgtatggaaccgcagcacagaaaaagcatcgccgctggtaacggatggcgctgtattggcagcagatcctgccgcagcggtattggcaagcccggtgatcattacctgcctcaataattacgaaaccacccgcagcattctttccacgccggaagcagcagcggcgctgaatggccgtcttctgctggaactcactaccggcaccccgcaggatgcaagaacagcagcaacctgggcgcagtcccttggtgcgcactacctggatggcgcactgctggccacaccccggcagataggaaaaccggatacgcctatttttttatccgggcaacaggccgcttttgaaaaaggagaagccgtgttaaaagtactgggtggcaacctgatgtatatgggagccgccaccggcgccgccgctgcgtgggatcttgccattctttccagcctgttcggtttgatcaccggctttctgcaaggcgccaggatttttgaatcagaaaagctggatgtaaacgcattaggcgatatgatcaataacatagcaccggtactcggggaaatggtgcggcacgaaggcgctgtgatcagcaccaacaatttttcccaaccggaaagcagcctcaaaacctgcgcggtatctatgactttaatgatgaaacaggccgctgaatccggcattcccggcgatgtgcccgccttcatcctcaaccttatgaataaaggcatcaaggccggttatggagaagagcaggtgggagcattgataaaagccatgcggtaaggaggaggttagtgtttagtccgccggactaaacactaattatccgtatctttataagcactcaaattgttaccgcatgaacatggaaagttatctcccctcagctattctctctccatatgtcagcgcttatctgatcatcgaaagcaaagacggcatggagaaccgcgtaatgccggatactgctgtggtgatgtctttccggtttggtggtaaagtaataaccggggaatccggtgaggcaaccgacctgccggcaacagcgctggcaggtttgcgcagaacttcccggttgttacactatgcgcccggcaccggcaatgtgctggtgaagtttagagaaggtggcgccgcggcctttttcaaaacacccctgcatgaattgttcgatacccatgaatcgctcgatcaactggtacagcgccataaaataagggaagtggaagaacggttgtacgaggcaaaaaacaacctgcagcggatcgcgattgtggagcaattcctgatggcggcactcagcagccggcaaccggatttactcatccgccatgccgtacaacaaattaaaacagccgccggcgatgtgaagatcaaatcactggcagcagacctgtacatcagtcaggatgcatttgaaaaacgattcaggcgaagcgtaggaactacgcccaagcaattctccgccatcgtaagattacggcacctgctcgatcactttccggaagccggcagcctcacagaagcagcctatgatgccggctattacgaccaggcgcattttataaaagacttccgggctttcaccggtcaaacaccacaggcatttttgcagcaaacctcctggtggtaatcttatacggccattggttctgttttctttttcattaatgcctcaaattcaccctggtagtcttctccccatttatccatcgcatccaccaccggcaataacgactcgccgaaattggtgagatagtactctactttcggcggcagctcatgataaataacccttttgatgatgccatggaattccagttcccgcaactgcagatccaacacccgccggctggcggaaggcatcgctctttgcagttcactgggtcttcttacccctttgttgatcaggtataccatataggatttccatttaccacctatgatttccatgatgatcgccatcccgcacgcaaaactttttggaatctttttttcatacataaccggtcacttttctgatacggacaaatttatccctaatagccggactccaggcatacggataaaattttccgtataggaacataatgtccgttattgttctgttcacccgatctgcgtcactttgcagcattgatcatcaaaataaaaataacatgaccagcacaatgaataattacaatggaaagacagcggtagtcaccggcggtacacatggtatgggattggcagtggttaaaatgctgatcgcaggcggtgcagaagtattgctcaccgggaaaaatccaaagaacctggaagccgccaaagaagagttgggtaacagcgtacacatcatagcttccgatacatcatccatgagcgacattgaaaccctgcgcaacaccgtggctgccaccctggggcaaatcgatttcctgtttataaatgccggcttctcgttgctggaacccttcgacaaagtaaaggaggccacttacgataaaacctttgccatcaataccaaaggagcctatttcaccgtacagcagctatcgccgttaataaaagattatggcgccattgtattcactacgtccatcgccaacaactccggctatgcatgcatgagcgtgtacgccggtgcaaaagcggcgctggcctcctttgtaaaaggttttgcggctgaactgctgcccaggagcatccgcgtaaatgccgtgagtccgggttttattcatacacccacaatgggcgtgtccggcgcatcgaaggaagaattgctggccttcgaaaaaatcggggaggaggtaacgccgttgaaacgcaatggtaatacggatgaagtggcgaaggccgtattgttcctggccttcgatgctacatttactactggtgaggaactaaccgtggatggaggtctttctaaaaatctcaccccacccgatctttcacactaattcaaaagggttgactataaaatttatagtcagcctttctcaaaatctcctgtctcaaaaaaatattttaaaatgagcaatcgctcacttatctttgtgcggcatgagatacagagacgaaaataaaatacaggccatccgcgagtccgctattgagatggtggtgaaagatggactcgagaattttggcatcaaccggctggcaaaagcagcgggtgtatctccggcaactatttatatttattataaagataaagaagacctgctgaccagtatcagtacagaagaagcactgaaaatgacgcgggctaccctgaaagattttaacccggaaatgggctttgaggaagggctgtggatccaatggaaaaacagggccgctttttcactggataaccaccaatctgtcaatttctttgaacagctgcggaattctatgtataaagaaaaaatgctggaaacgatctcacatgaattccatagcgcaatggggagctatgtacataatgctgtaaagcgtggagagatcaaagaaatgcccctcgaagtatactggtctgttgcttttgcgcccttatactcactgataaaattccataacgaaggacgaagtctcgatggccgcaagtttaagttttcagagaagatcatgaaagaaacattcgactgtgtgataaaaggaataatgaaatagcctttttttttatcaaattaataaatgaacgctcgctcacaaaaacaaattagtcatgcaacacgttctcattttcaaaacaaacattgccactgtgcaagcccgctccaaagtagcgtcgttactggatcagcagtcctttattgaaaaatggacagtagacatggaagacgtagattgcgtgctgagagtagtaactgccgaaccggtgccggatcgcattattgcattaatcaatgccagcgagtacgaatgtgcagagctggaagactaacaaatacataagctcaaaatctccctgatgaaacaagcatccaccgcattttcgggtcaccagaaaatgatagtagccctgttggcactcacacaattcacggtcatcctcgattttatggttatgtcgccactcggtgatatgcttatgaaatcgatgaacataaagcctaaccagttcggactcatcgtatcggcctatgctttcagcgccggtatctccggcctgctcaccgccggctttgccgatcgcttcgaccgtaaaaaactgctgatatttttttatgcgggctttatcctcggcacattatgctgcggcctggccaacacgtattacacgatggtggcggcccgtatcgtaaccggtttatttggcggcgtaatagggtctatttccctggcaatcgtcaccgatctttttgatatctcacaacgcggccgcgtgatggggtttgtgcaaatggcatttggcgccagccaggtactcggtatccctatcgggttatacctcgccaacgcatggggatgggaagcgccctttttcctcgtggccggtgtagccgctatcgtgatgctgctgatcatctttcagctgcaaccggtcattgcacacctggccgtgcaacgcgataaaagcgcattcacgcacctgtggcataccgtgagaagccgcgattaccgcatcggttttaccgccaccgcactcatgtctgtaggcggatttatgatgatgcccttcggtagtgcatttgccgtgaataacctgcacgttacgcatgaacagttaccgttgttgttcatggtgaccggtgttggttccctgttcatcatgccggtgctgggaaagttaagtgataaaaaagacaggtttacgctctttaccattgcttccatttatgcactggtgatcatcattatttatacgcacttaacaccgcatccgctctggatcatcatgtgcctgaacgtactgatgatggcaggtatcatgggccgtatgatcccattcaccgccttaactaccggtatccccgacctgtcggaccgtggagcctttatgagcgtaaactcgtccctgcaacaaattgccggcggaatagcggcggtcattgcaggtatgatcgtatcccagaaagataaattcagtccgctggaacactacgatacactcggatgggtcattgtaggcttaacgctgccctgtatttacctggtacaccgcgtaagcgtaattgtaaaaagaaaactggccaaaggcgcggtggtgaataccaccagtgtagcggcggaagtgtaatatttttttggggagccgggctaaccggctccccaaaaaaatatttagtaagataaggtacgcgcactgcctgtttgggttgattcagcgaaacttttatcttagatttgaattatgaaacaaatatccattctcgttcccaaaggcgccgttgcgctcagtagtattgaaggtccctttgtactgtttaccaaagccaacgacttcctcgaaagcgttggaaaggatccgttgtttaacgtgcagctggtgggactctccaaagaagcacacgaatacgaccggttttttaaagtgacaccggacgtaatgatcacagaaaaacataaagcagacctgatcattattcccgcagtaaacggggagcgtgaagtggtcatagatcagaataaggatttctatccctggattgtacagcagcatcagcatggatcagaagtggcgagcctttgtgtaggcgcctttttactggcatccacaggcttgctcaatggaaagcgttgctccacgcactggctggcagccaatgaattcaggaacatgttccccgatgtggaactggtgtctgaaaagatcattacagatgaaaagggtatttattccagcggtggcgccaactccttctggaacctgctgatttacctgatagaaaagtatacagacagggacatggccattcttgcgtccaagtattttgaaattgaaatagaccgcaccaaccaggcgacctttactatttttaaaggtcagcgtgaacaccaggatgaatcagtaaaacaggcgcaggaatttattgagcagaactggcaggaaaaaatcacggtagaacagttgtcatccatgtttgccgtaggccgcagaagcctggaaagaagatttaagaaagcaaccagcaacaccgtatcagaatatattcaacgggtgaaggtagaagtggccaaaaaaagctttgaaagcagccgtaaaaatatcaatgaaattatgtgggaagtgggttattcggatacaaaggcgtttagaacaatctttaagaaaacaaccggcttatcgccactcgagtatagaaacaaatacaataaaggtgcaactgctaagtaaccctttatttttccggggagaagaacttatgccatctgccttccaatacccgtttcagcatggtgcataattcctggaaagtattgggcttggtcaggaataattttgcacccagccgcatggcatcttccatatcttccttcatatcagaagtactcagtatgatgatattcgttaactgatgctgaaggatctttttcagttctaccaggcattcgcgcccgttcatcagcggcatgttgaaatcaaggaaaatgtaatcaggagccggaattttattttcctggaacatcgctattgcctgtattccactatcgcatacatgtgtttctatgaccggagagatattgtgaatggcttcctggaaaaaaattctatcatcggcatcatcatcaataatcattatttgttgtggtctcgtcatggctaaaattttaagcattaaggtcttcacgttcgtttggatcttcggcgggaaatatgaagataaacaaaaatgcaaaagcgttcaaatttaagattttaccatacatacggtcgcgctccttttgtggcatccggtggcgcaaatattgtaagagagatggtatcaccctaaaagcaccttctcatgaaaaaatatttgttgtcacttttaatgttgcccgcaacttatcagctgtgtgcacaagacagtgcccgcctgccgccaccccatgccacaaaatcatatatgaattatagccaggtagttggctggggtcctggtgaaacacccgttgcaccagcgggttttcatgtgtctttatatgcggatgacctggtaaatccacgctggatgtatgcgctcccaaacggcgatgtgctggtggcggaatcaaacagtaatttcccgctggtgattaaaataggggcggtgtttgtaggcgcccagaagtcaaagagtatgcggcacagtgcagatcgcattaccctgctgcgggatgctaaccacgacggtataccggagttccgcagcacctttctttccaatctgaatcagccctttggcatgctgctgataggcaaccatttttatgtggccaataccaatgcgttagtccgctatccttacaaaaccggcgatacggtgatcaccgcggcgccggagaaaataacagacctgcctgtcggcaaaaaaaatcagcactggacgcgaaatatcattgctaataaagatcaatccaaaatttatatcgctattggctcagccaccgatcatgcggagaaaggtattgaaaatgaacaatcgagggcagccatcgtggaaatcaatcccgatggtaccggtcgccgcatttacgccgcaggtttaagaaaccccgttggcatggactgggcccccggtacttctaccttatgggtggctgttaatgaaagggataaattaggcaacgacctggtacccgattacatgacaggcgtaaaagaaggcggcttctacggatggccctggaagtattacggtcagcataccgatacacgcgtgaaagatcccgcgccaccggaagcaaacaataccattatccccgatgtacaattaggccctcataccgcctccctgggtctggtattttaccggggagatgaatttccggaaagataccaccagggtgcattcatcgcccagcatggctcctggaaccgcaagcctatttctggttacaaagtattgtttatcccttttgctaatgggaaacccgccggtaaaccaacagattttctcaccggatttgtgaaagattccaccacggcagatgtaagaggccggccggtaggactccttgtattgaaaaacggcgcaatgctggtaacagacgataaaaccaaccgcatctggaaggtggtatacggacaataatgaaatgtttaacttgcacggcatgaaaatattccaacaggcattacagctacagcaaagaagaaggggatttcacattatcaccacggaaatcgtacaggcatttccgcaactctccgaaataaaaacgggaatgctgcaggtattcatccagcatacctcggcgtcgcttacgctgaatgaaaatgcagatcccaccgtgcggaaagatttcgaaatgtatttcaataaaaccgtccctgaaaacgatccggaatacctgcacgatgatgaaggatccgacgatatgccggcgcacctgaaagccgcgttgttaggcagttctgttatgatccccatccgcaacggccggcttgcagtaggtacctggcagggcatatacctgtgtgaacaccgcaatcacggtggtccgcggaacctgctgcttaccgcatggggagaataacaatcagctcaacgcatcgtgaaaaataatacccagcgtgtgccggttcccgttatgcaccgggcttacgccatgtttcatgttcacacggtaatatcccttgctgccttttacaggccggaaattagtggtaaaaatcagcatatccccccgctgcggccgcagcacattggctttggattgcgccctggggatctgttccgttaatacaaactcgcccccggtataatcctcttccggctcattcaggaatactaccagctgcattggaaaataaatatcgccgtacaggtcctggtgcagggtgttaaatccatcctgcccatatttaaggatcaggatggtgggtttcgtttgtccgttaacgtgacaatgcgcttttaatgcagcatgtgtatcgggataccgctgcgcaatgtgcaatacttccatccatttgttggctaccggcgcaataaacgggtacactgtttcccggatagtggtgaccagctccggcaggggatactgaaaatatttatattcccctttcccaaaacggtaacgctccatcacaattgttttccggtaggtgtcgtcggcctggtaatcattgatcagcgcatcacattccgctttgcccagtacacctttcagtaacgtatagccgcggtcgttcaattgggtggctgcctgttgccagtcgtgcgccagcagccgctgtttaatatctttcatctggtattttttttatggagatacaaaaataactgcccgggccaccacggaaaacccggttcttgcggtgttggggtaatggtattattcaacggaataatagtattttcatagtttattattgcctgaaatatgcagtgcatgaattaaatagtaacgttgcaaatatcaaaatgaacaaatgaaatgttgaagctggccatcatcagcgatattcacgcaaacctgcctgcgttgatatccgtattggaagacatagaacagtttggtgcccaccaggtatactgcctgggtgatctcacggatgcggcgccgtggcacaatgaagtaatagacctgatccggcaaaagaacatcccggtaattatgggcaatcatgatgaacgcatcgcctttgaccaccctgtatacccgcttagtaaacacacgccggaagagcaaacagccaggctacaggccatcgactatacaaaagataccattaggccgcaacacgcagccttcctcgcagaactgccaccccatatacagatggatgttgccggcgtaaaagtattactggtacatggcagcacccggagcaacgatgagtacctctaccaggatcatgatgaaaatgacctgttgggaatgatggaagaatatcatgcagatataatggtgaccgggcatacgcatctctcttatatacgcccgctgaaagcggcgggaaaaatggtgatcaacaccggatcagtaggcaggtcgaaagaaaaagaccgcctggcggcctatctgcaactaacggttaccggcagtaaaattacaccggccatccggaagataccttacccggtggaagaaaccatagccggcatccggaacagtcccattcccgatttttacgcacattttttagcaggtaacgataacgcttagtgcgtatctttatccgtaaattaacgggtatggaaactgctcaccgggattacagcaccatcagtcctactgccaaatcattgttgctgctgaaaggcgttaccgctattccttacgcaaaggaagctgcacaactcatgctggcgccgctgccctatcaaatgaatacggatagtaaggatctttcattctggctaagagtggtgcatttcgaagaccgttactggagtatcaatcaattactggatgaattgccggtgaaaaatgtccttgaattatcttccgggttttctttccgtggactggaaactgtgaaacaaccggggtatcactatattgatacggacctgccggaagtaatagcactaaagaagaaatttgttgcggcgttggagaaacaaccaccggccggtgtgctggaagtattaccgttaaacgcattggatgaagcgcagtttatggaaacagtgaaccgtttcccggagggtccgctggtaatagtgaacgaaggattgctgatgtaccttgatgatactgaaaaggaaaaactatgtaatattatccgccgcgtgttgcaacaacgtggaggatactggatcaccgcagatatttatgtgaagcgggatgccgccaccaacgaaataaaacgggatgaacagtggaaagcattttatgcccagcatcagattcatgaaaaaatgttcgacagctttgaagccgctgaaatatttttccggaagatgggattcgaaatagagaaggtggctgcccgtgatcatgcgcgccttaccgggctgccacacgtgatggaaaacgctacagaagagcagctgcataaaatgagggcggcgggaaggatcagggctacctggcgactgaaaccggtggagtagcatctgccattactaccaggtctttcaatatcgtatacagttgttcaatatttaccggtttactcaagaatccatctgcgccggaagcaattatttcttcctttacttcactgtaggcattgccggataccagtatgaaagggatctgccgcaactggcggtcggccctgaactgcgacaacatttccacaccgctgatatgcggcatgatcatgtccattagtatagcatccggttgatgcagccgggctttggcaaggccctgcggaccggagtcggccactattacttctatgcccatgcgtttgagcgccagtgaaaatgcgaggtggttcaggtggtcatcgtctaccaccaacacttttaagccttttaaaatagaatagtccatcatttgatggatagcagcaggtggagtggtaatttccaccggcatgcgcagggtgaaaatgctgcccccgccatcaggattatctgttaccgtaagatcacctcccatcatgcgggccatatgccgggcaatgggtagtcccagcccgctggattctgtatgctgccctggttcagtcacatacggatcaaaaatgtgctccttccggtcggcgctaatgcccaccccctgatcagttacggaaactaccagctggttgtttttcatgccggcccttactgtaatgattgaccggaaagtagtgaacttgatagcgttgctgagaaggtttacaataatggtgcgaagcttcgacttatctgccaggatatactccggcaggttgtcgttcagtgaaatattgatatgcacggatcttcttttggccaggtattcatacgtatcacataagtgctgcacccagtcgctgaagtgaaacggtgatttgctgatctcatcttttccttcctcaattttcgaccatcccagtgcattgctcattaccagctgcatatcctggcaggcaaaatgtacggcttccaggtgggcaatgcctacctgtaccgtccttttcccctggtcggccgtttcaatataattttgcaggatgctgtttaccacattcaatggcgaccggatttcgtgggtggtttcacgcacgtagatgcgcatggcctgattggctttgtccagctggtttaccaacgatttcagctgtttattctggaacctgctttccttggcaaaataatacagggcggtgccgttcagaaaagtagcagaaatgatcaccagccagtgtaagtataattcggtgtccttattaagcggaagcgaagcaatcacggggtacctgaaattaagcagtaccagtatcattaccactgcactggcaacaagagctattatctgggaccagggcttttcgaataccaggaatacacaaaaagcaaggaagggggcaaacaggtaaatctgggaagcaggtcccagcaacacgccaaaaaaccagatggaaacactgtgtaacaagaacatcaactgtttcccgtaaaccggtttgctgtaacgggtaatcagcagcgtggaaagaaaaagggcgctttccagcagggcagggtaaaaaataatgccgtagcccgtcatataatataacaggcatccaagcgtaaatgccagcaggctggcgcttaccgccagggaattgacaatctttataatccgttcctttgcttcattttcctccgcattgcggccatttatcctggtcagggtaaggttgtttttcataaaatccaggttttcatgttaaggggttgcaggtctttcttttcccaatgcattcaaggtagaagaatgcagattatcaagtgtaaattctttgttaacaacatatattttttggtagcggtttaaagttaccgtgtgaagatttgaacaattaacgcacatttttttgtcagttataaacactactttcatattgaaattatcatgtacatgagtatacgtttgttttacctggtcatctggctgtttatcataccggtggcgggcaaaggcgctatcatcattgaagggcagctgtccggaaatccgcacagcctcattaccctgtatggctatgccgattatatcagtaaggcgcccgtggaaatactgaaggtacatacaaatggtgccggaaatttccgggtaaccgtatcggattcctgcggaccattggtaaaactgctcgtggaaaacaggtcactgtcctttttcacgctgccgggcggcgcctatattattcaggatacgatgggccaactcaccgtaaccgatgctgccggcactcccgtgaaccaactcctgcatagcatggaacaagagctcctgaaaaactggtatcccttatttgtagataccaccggccgtttccggctaaccctaccggcagatactgtttttcaacgcttccacgaaatagtatcaaaatatacgaacgataccacatcaacagcttacccgctgctgcgctatgatgcggcgatctattacctggcatttgtgcaacagctgcgggataccacaggcttgatggatcattttgagaatgattatttcaataacgcgcccattcaggaaaaaaatcccttttatacgaagctgttggaagatgatttgtttgtaagaatgatgttttttgcccaacaacgatataaaggaagtgcaggtaacctcatcgacaaggtaacccacgaagccgcttattttaaatcgccacagctgcagcaactggcgctggcagcagggtgtaaccaggcctaccgggtcaatcgtgagccggggcagaaagatgaactgtcccgccgcatccgcgccaccatcctggatagccttacccatccagggatcaggacgatgattgcccacgtcattacagaaaatacccgcgcccgcgtcgggaataaatttccgctgctgacactgaaaaatggaaaaaatgaaaccgtaaattttgcagatataaaatctgatcttatcctggtcgacttctgggccacctggtgctggggctgcgtggaaggaatgaaaaactttccctcctggatcagtcagtgcaacggccagctaaccatcgtttccatttccgttgacgataacctccagcaaatgaaagcattcctggataaacgcgaaaagctccccggcgtattatcgctgtacaacggccgtaccggtggctatcttgataaattgcagatcagcggctaccccacctatattcttcttaataaaaaccgcgaaataattgccatgccaggctacacctctgcggtggctgagcagctaaaaagcatcatgaaataaaaatcaaaaaaaatcgaatcaaaaaaatcagcatcatcagtgtaatcctgagaaagacaacctcccccgcaatccggaaaaataaatctcccgaaaaattcccgatatcgaaaatcctttgaaagatatacacctacttttacagcagatttaaatacctataagtacgctgtatgctgaatacctggataccatgctgcaggattcgctacggaataaccttgccttatgtcgtttcaataaagctgtttaaaatgtgatggcggaagaattacggcaccaaagcagcatattgatatcacttttatgcagaaaaatatgaatgcaaattcaaagaaaacggccgggaaaaaagcaaagtcccggtcgctgttctatcgcatctccgcctggctgcatctgtggctgggcattgcttcgggtatcgtggtagtcatcgtgtgcgtaaccggatgcatctacgtgttcaacgaggaaatcaccggctggatggaaccggaagcaaatgttccggtacaatcgcagccactcatcgctccttcaaagatcctggaagtagccgcgaaagaatatcccggcaaaactgtaggctacgtgctgtataaagaaggcaaagccgtagaagccaatatcggcgcaaggagaggcggttccaccctgaagctgaacccctataccggcgcggtaatcaataaagtaaaccgtaaagaaggggaactgaactttttcagatgggtactcaacggacaccgtttcctctggctgccggttaagatcggccgccctatcgtcaactacagcactttgatctgcgtaatcaccctgatcagcggcctggtgttatggtggccgaaaagatggaataaaagtacccgtaaccagagctttaaaataaaatggggcgccagcttcaaacgcatcaactacgacctgcacaatgtactgggcttttacgcactgctggtactttttgctatatgcgttaccggtatggtatacggactggaatggtggagcaaaggcctctactgggctacctccggtggaaaaacattgccggaattccgggaactgaaatcagattccctgcaggcgggcaaaaaacaggatattaacctcggccagaaaatggatattgcctggaaaacagcgataggcaaacacccggaggcatccggtttttacatggccttcccggatacttccaaagccaccgcgtctattaccgttattgtatatcctgaaaaaggacagtattataataaccagcgctacgtatttgatcagcatacactggaaccgcttaccgggaataaattatatgagcaatcctttgcagaagccgaatttggcgctaaactcaggcgcatgaactacgatatccacgtaggcagcatcctggggttaccgggcaagttcatggcattcttcgccagcctgatcggcgctacactacctatcacggggtttattatctggtggggtaaaggccggaaaaagaaaacgccggcgccggtgaaaagaaaggcgcaaacagcagcagtataaaataactatttcccaattacatagattcagagaagaaagggcgtcattcagttgatgtcctttttttatcgggtgtacatacaccggctttcttttaaatgtacagaattaaaggaataatgtacaagtgaataaagagattatcggtataaatttgcgcttataaaacaacggaccatgaaagcaattgttttaaatagtgcaggaagcgtagataacttagtactcacagacttgccggtgccggtaccgggagaggccgaagtactggtaaaagtaaaggccatcagcattaacccggtggatgttaaaacccgtgccggcaaaggcaggtacaacctcctgaaagaggaaaacccgctgatccttggctgggatatttccggcgtggtagtcgcttccaactcaccgttgttcaaagaaaacgatgaagtattcggaatggtcaacttccctggtcacggccgcgcatacgcggagtatgtagccgcgccggccgcgcacctggcgttgaagccggcaaatatctctcacgatgaagcggctgcagccaccctggcggcgctcaccgcctggcaggcgctgatagatcatgccagcataaggcccgggcataaagtgctgatccatgcagcggcaggcggcgtaggtcactatgcagtgcagctggccaaacatctcggcgcgtatgtcatcggtacttcttcggccgctaacagggaggtgatcctcggattgggagcggatgagcatatcgattatcacacccagcccttaatagatcatgtatcagatgtcgatttcgttcttgacaccatcggcggcgataccattgatcagtcgctcgaagtaatgaagcgcggcgctactattatcagcattccttccggtttccgggaagcggtaaccgccaaggcggaagcaaaaggcctcaccggcttcttcatcctggtggcttccaacggggcagaaatggctagtatcgctgctttgatggaacagggcctgctcaggtccatcgtctccaaaactttctctttggaggaaatgaagcaggcgcatctccagatagaaaccggcagaacagtaggtaaaattatcgtacgggtttaaccgttagtaacgattccataataacagcagcgcagtttaaacaggcggtagcccggccgccggcgctgctgattttttttagagagatgtaaagaaatatttctatcttgttacccataatcaagcacaaatgcaccgtatttattcaagcacacctccgccagctgttgttgttttgtccgcaaaataaccagcactactacggcttctagctattcctgttacaggaatcagtttgtcatttatttgcactaagtctgtttattgacctggttattttcgtgtacccatattctcccttttttattacacaaccgaaaataatgaccaggtatatattaatggtttttgccggcgcatgcagcttcggcatcctttctacttttgtaaaattagcctaccgcgaaggctatacagccgcggaaatatccgttacacaggcctgcacaggcatgatcgttttgtggatcctgtatctccttacccggcggcaacgccaccgggtaaagcccggcgattgggcctggctgctgttgacaggcggcggtattggccttaccagtttcgtatattatgtgtcggtagcctatataccggcatcggtagctatcgtaatcctgatgcaatttacctggataggtttgctgatggaagcattgctgtttaaaaagataccttccttattacagctcatcaccaccatactgatcctggtgggcacctggctgggcagtgggttggccggtggcagcctttccggcttgtctgtaaaaggactgttgtatgccggcgcatctgcttttttatacgccgtgtatatcattgccaacagccgcgtaggcaaatcgctggataccggtaagaaaagtgcggtcatcattactggctccacgctatgtattttcctggtaaacgcaccgcaactgttggccagtacccacttcgatacgggtctgctgaaatgggcgctgttcctgtcgctttttggaaccattattccgccgttgctgtttgccaaaggaatccccaaggtaggggcagggatcagcgcggtgatcatgaccgccgagttgccggtggccattgtgtgctcgcatttcatcctgctggaacctgtgaacggccttcaatgggcaggagttgcgctcatgttgttatcaatgctgctgctgaatgcgcgttatttccgcaaatagaagaggagaccgggcatcttgcccggttctttttttactggtagaagatcgctgaaagcactattaccaggccatagtctttaaactccccgcgcattacctgcaacgattttcccatgtgcttttccactgccttaacagagatgcccaaacgcagcgcgatttctttattggacaaatgatcccggcggctcagcaggaatatttcccggctgcgctccgttaatttatccagcgccagcgcaaaccgctgttccagtaatttcagatcgtacgtattatctgtttcggcggtagtagttacgggaagttgttggtggtgctgctcatgcagcagcgaattccgcagttcattcaggatcctgttgcgcagtgcgccatgcaggtatgctttggcgtttttaatgccggtaagggtagcgcgttttttatacagggagataaaaatttcctggatcatatcttccagcagatgaggcgccgggaatttcttgtatgcatgttgatacagttctgctgcatggcgctggtataagacttcaaaagccttattatcattgttcgccagtagtgccagtaaagcttcatcctgtaatgcaatatattccgtcatgcttaccacttaagccggatcacatgattgccggctgcccttaaaaagcataagatataaaaaaaaggatgcaccacataaaacgccccgaaaaaataaatttctaccagggggtagggtagcctttcactgctgtgtctatactgcagacaaccaaaataatgagtgatcaacaactgataggattactggaaaaatacctgcagggcaggggtactgaagaggaacggaatgccctggaagcctggtatgaaacataccagtccgcaaaagcgcctggcagcgatccgcagcccgatctgctgcagatgtaccacgacattaccggcaggctgaaacaggaaggggaatgggtggagccgccacgcgcaaaaatccacccgctcaaacaacggggatggcgcatcgccgcagccatactgttcctggtggccggcgccggcatctggacgctgcttccccgcgctaacaggcagctgtcggcagatacaaaagacggcatccgcaaaaaaatacaactggaagatggcacgcaggtatggctcaatgtaagcagtcaccttacctatccggccaacatcggcaacagcagcagggaagtatacctgaaaggagaggccttttttgaagtaaagccaaaggaaacacaccccttcaccattcatacgtcgggcgtggacgtgcaggtactgggcacccgctttaacgtaaaagcctaccaaaccgatgaaagcatggaaaccacgctggtagacggccgcgtggcagtaagccttagcgggcatccggataaaaagctggtactggcgcccggtgaaaaactcaccatcaggaagaaggataaaacgacgccggtaacaaatggccgtatcctcgactgggacagcgtactggccattgtagaaacaataacgccaaatgtgaccagcaaaaaggtaagcgaactggtatggatggacgaccgcctggaattcaaagacaaatccttcccggaactggccatcttaatgagccgctggtacaaccgtaaaattatcttaacagataccttcccggcagactaccgcttcaaaggcacgttcaagaaagaatccgttacagaagcgctcaaagcattacaggtcactgccgattttaatttcactataaagggagataccatctttatacatcattaatcaaccagatcataaaacaaacagtaacacgatgaaaaaaatattcccggttcccaccgaacctgtataaccactccttccgcccataaaaaaagggaagtgcggcaacacttcccctaaagccaaacatggtacgaaacaacgtaatccgtgcgggatgcccgttgtttctaatgtctaacgttcaatttcaaatgtatgaaaaaaaagctgtgttcaaaaacagccctttccaactattcagtgagaaaaatattcttgtgtatgaagctttgtctcatccttattactgcttcaattttacaggtgcgcgccgaagtgtattcgcaaagcaaattcacgctcaacagccggcaaattgccctgcataagctgctggagtgggtggaaacgaaaagtgactaccggtttctgtacaactacaaaacttttccgaaagatgaaaaggtagatgtcaacttcaaagaagccaccctgccggagatcctggataaagtgctggcgaaaaatttacggtataaaatgctggaaggcggactggtagccatctcggaaagtacggccgatatcacggtaaccggtaaggtaacggctgaaaatggccccgagctgcccggcgtaagcatccagctgaaagggaccagtcgtggtaccaccaccgatgttgacggcaactttaaaataaccgtcccggaaaacggcgtcctcatcatctcctacctgggatttgaaacaagggaaatcgccgtgaaaggcaacgcgcagctggccgtcataacactgaaatcttccgatgcaggtttgaatgaagtagtggtactgggatacggacaaaaacaaacacggcaaagcatcaccggcgctgtgtccagcatacaaacaaaagaactgaaacaaagcccggtagccaacctctcgaacgcactggccggaagattacccggcctcatcacggcgcagcactccggccgccccggcagcgacgactcacagctgtttatccgcggtatcagcaccaccggcgccaccaacccgctcgtggtaatagatggcctgccccgcggagatgccaatatcggtcagctggaccccaacgaaatagaatccgtttctatcctgaaagacgcttcctctactgcattatacggtatacagggcgccaacggtatcgtgctggtgaccaccaaacgcggtaaagacggcccgcccaacatccaggtgaacatgcagtatgccttgcagcagcctaccaattttccccgcttcctcgattcttaccaatccggcctgctggaaaatgaagccgccaaaaatgatggcatgccggcggtattcaccgaccaggaactggaatattataaaacaggactgaaaccttatgactatccaaataccgactggtacaaggaaatcatccgggactattccccgcagaaaacagtgaacatcaatatcggcggcggttccaaattcgttaaatattttgtatcgggttcttacctgcgccaggagccggtatacaaccacgccaatgaaaatatctacggcatcaaatacaaatacgaccgctttaatttccgctccaacgtggatatcaccctcgataaaaataccgacctgcaggtagacctggcctcccgcctggaaaaccgtaccagtccttctgcggaccgtggcaacaatgaatttttctgggtactgctgtcgcagatgaccaatcgccttacacccgtgtttaaccccgatggctctatcgcctccggcaccatgcgggaagatttttacaacctgtatggcgtgcttacccgtaacggttatatcgatgcctattggcatagtaccaacggcagcgtggcactcacccgcaagctggactttatcacacccggactgaaagtaaaaggactctttactttcgagaactatggcgatatcaactttgcactggaccaggactttgattcttatcgttacaaatcagtgcccggtgcagaaggtacgtatacccagcaccgtaaggccaccagtttacaacgctccggttattccagcggcgaaagatattactactatgatctgaaagtgatgtacgaccgcgattttggtaaacactccctcggaggcttactcctgttcaaccgcaattaccgctcccagtcgggtaacctcccacgggtatacgaaggctttgtaggcaggattgcttacaactacgccacccgctactaccttgaattcaatgccggttacaatggctccgagaactttcctcccggtaaacggtacggatttttcccggcgctttctgccgcctgggtgctgagtaatgaacagttcatgagtggccagtcgctgttcagctacctgaaaatgcgtttctcacacggttacgtgggtaacgaccaggtaggcggcgaccgctggttatatgtatctgattacgcccgcggcgatggctttacttttggcagcgtgggcaccggcgccggcggctattatgaaaacagggtgggcaacaccgccattacctgggagaaagcagcgaaaacaaacctcggtattgaaacaggatttctgaaagataaagtgaagttttcggtagatatttttaatgaactgcgtaaagatatccttacctacgccggcaccatccctgcttatctcggtatcaccgcatcactgaaccgtaatatgggccgtatccgcaataaaggtgtggaagcagaactgaatgtaaattccaacatcggcgcagtaggcgtcttttcaaaattgaattaccagtatgtaaaaaataaaatactggagatggacgaacccaaactggcatatccttaccagagcgcagtaggccatcctatcgggtacgatctcggctatgtggccgaaggactgttccgcaaccaggatgaaatcaataaaagcccgcagcaaactttttcaccactcatccccggcgacatcaaatacaccgacatcaataaagatggcgtgatcaatgaagccgacaggatcatgctgcccatgatgaatgtacccaccagttatttcggggccaccttcggcatcgactataaaggcctggatgtaagtgtgctgttccagggcgcaggcggcggacgccagatctactcttcgcagctcaccggcaacttccgcgaaagctaccggcccatgcacctgaacaggtggacgccggaaaacgccgacaaagccacctatcctgttttacacttatcggaaagtaatatggccaataactcggtcagttctacttactggatcaggaacaccgactatgttaaattaaagaatgctgagatagggtaccggctgccggcgcacctcctgaaaaaggtgaaaattaaaagcgcacgcatctatgtgaatggtatgaacctcatcagctgggataatgtgaaagaactggggatagatccggaatccaataccggcggccgctggggctggcagccttatccgattatgcgcgtgtataatgccggtatcaccatcaatctttaatcacctgtgataaattaaaatcatgaatacgttcttcgttaaaacagggatagcagcagtactgatcatgtgtgttactgcctgcggtaagaattacctggacaggaagcccagtgatctgatcactgaaaaagaagtgttttcaaatattgaaaacgccgaaaagtttgtgaatactatctaccaaagcttacccaatatttttaagcccgggtcggcatggccgctcagcagtgccaccgacgaaaccaaccaggccagcgataattccgcttcttatcccgatgccggcaatttcaacaccggctccatgagccctgccaacttcccgatgcagagctcctgggccgactattatggcaagatccgttcgtgtaataagttccttgcgcagtacgacctcgtgccccaggatcctaactatccgcaacggcgcagccgccttaaaggagaagtgctcaccctgcgcgccttctactattttgaactgatgcgcgcctggggaggcgtaccactgctgctgtcggagaaaaatccgttcgatgatccaacaggcatttactacaaacgcaacagcatcgatgaagtaactgccagcatcctcaacgacctgcaggaagccggcactttgttgccggtggcttacaacgatcgcccttccaactggggccgtgcctccaaaatgattgcactggcgctggaaggccgcgtacggctgttttacgccagcccgctctacaatgcaggcaacaataccgcccgctggcaggctgccgcaaccgcctgcaaggccgcactggacactgctatcgccaacggctacacgctgtacgacacctacggcgatatcttcacccaatacttcaaccgtgaagtgatctggagccgccccgcacccggcgctttcggcgatggtggtattgaccgggaaatgaatccccgcagcgccaacggctacggcaacattacaccgctgcaggaactggtagatgattacgaaatgaaaaccaccggcctttccattaaagatcccgcttccggctacagcgcgcaacgtccttacgatgggagggatccccgcttttatgcgaccatcctgtatcccggctgctcctggaaaggaaaggtgctggatccgaacggggccgatgcaccgcgctccggccagattgccaccaactactggccacggaaatatctcctcccttcggtcgacctgtttgcaggcaccggtggcagcgatcgcaaatgggtactcatcagaaccgcggaactttatctcaactacgcggaagcacaaaatgaagccgcaggccccgcaacagaagtatacgatgccctcaatgcaatccgcaccagggccggtatgccgggtatcaacggtggaaccaaagaaacgttgcgcgaaaagatccgccatgaaagaagaatagaactggcattggaagatcatcgcttctgggatgtgcgccgctggaaaaccgctgaacaggtagataataaagaagtacacggcgtagccgttagcggcaccggcaatgtttcctaccgctatccggtaatagaaaaaagggtgttcgatccgggtaaaaattactggcttcccattccgcaaagtgaaatggataaggtaagcagccagaatcctgagtttacgcagaataaaggctggtaaagcgttctacatctccctaaatttaaaaaaatgaaaacgataatataccgcttactggcagtatggctgttgtttacagccgctgcctgtaacaaagacaacgatttcgaacacgataacaacgcaccggtggtggtggataaatttacaccggaaaccggcgccgccggcacggaagtgctgatctatggaaccaatttcagtaaagataccaatggggtgaccgttacggtgaatggcaaaaaagcccttgtcaccggcattatcagcgatcatatcctggtagtaatcccggaaaaagctggcagcggtaaagtagtcgtaaccattaacggcaaagcaggcaccgctcccaaagacttccagtatttatcttcctataaagtaaccaccctggcaggcaacggcgcggcaggctactccgatggcaaaggcacaaacgccgcttttaattttgataaacgctgcggcctcgatgtagacgataacggaaacgtatatgtagccgatgcaggcaacttacgcgtgagaaaaattgcacccgatggcgccgtcaccacactcgccggcagcggcacctccggctatgtggaaggcaaaggccccgccgcacagttctatcttccctttgatattgtaaccgataacagcgggaatgtattcgtatccgatccttccgcatggaccatccgcaaaatcacacccgatggtaccacctcccgcatttgctggggcgaagcctggggaattggcatcgataaacgcaacggcaccctgtactacgccaacaacggcagccctggcagcatttatcaggtaacgcctgatggcagcagcgttacacccatcatcaccgggctaaacagacccgccgatgtagcggtagatgacaaaggaaatttatttgtaacagagaatggaaactccgtgatcaaaaagtttgctgcaggtaactgggcgcccactatcatcgccggcgcggaaaatcaaaccggcctggtaaatggtaccggtaccgctgcacgttttgaaaatccctggagtattatcgtggacaaagccaacaacctgttcgtagccggtaacggcagtgccgacggatcttctgttaacagcaaccaatgcatccgcttcatcactgccaacgcctgggaagtaagcacctatataggcggcagcaccgcaggatttgcggatggcgccggcgcagcagcgctgtttaatgcgcctaccggcgtggcggttgacaaagacggcgtagtgtatgtgctcgaccgcaacaataaccgtatccgcaaagtaacggcagaataagtagcagtggcggcccggagacgggtcgccacttttctcagataattaaatgttcagtaatgttcaaacaagtcctgttttatatagccctatggctgttgcccgcaactgccatgtcgcaaacaccaaaagatttcaaatggaacgtattgcctgtaaaagggttgctgctcagcgtaccagctccccaggatgtgccgctgctgtgccgctttatcaaggaagccctgaaggcggaaggggtaaacacgctggcgttacggattgaatatgcataccagtttaaatcgcatcccgaactcgccgagcgcaacgcgatttcggaaacagacctcaaacagattgtagccgcctgcaaggaagccggtatccgctttatccctaccatgaacctgctggcccaccagtcggaacaaacagaaatgggaccgttgctgaaaaattacccgcagctcgacgaatcaccggactataatccgccggtgccctggaaaaacggcggtatgttcgacttctacagcaaaagcctatgcccgctgcaccccgacctgttcaagatcattttccccctgatggatgaactcatcgatgtatgcggcgccgatgcgcttcacgtgggacttgatgaggtgtggatcctgggctatgataagtgcccccgctgcgggggccgcgacaaagccgaactgtttgcaggctatgtaaacgccttgcatcagcatctcaaagaaaaaaattgccagctgtggatgtggagcgaccgcctgatagacggaaaagaaaccaacctgctcggatggcaggccagtatgaacaataccgccagggctatagacctgatcccgaaagatatcatgatctgcgactggaaatatgaagatgcaccgcccaccccggcttactttgccatcaaaggatttcatgtattgccttccgcctgcggaaaaaaagacgtggcgctggcacaactggaacaggtatatgccgcccggaaaaatgcgctgcgggcagatttttcctatacgttatctgaacggatgcccggcgtattcgaaaccatgtgggtaaatacaaaagaatttattgatgcctactacaaccgaaaaggtgtgcgcaaaccaacacaggataatgcagatacctttaaagcattgtttgcagagatccggaaaaaagaaaagatgtagcatactgctattttacgcaatcgtttgtgctggaaaagccgggtgaaatcgcctaacattatcctccgttcaacagcacaagccatgaaaagaagatccgtttttattgccatcttattgctatcccggctggcgttatctgcccaggtatattacgccggcaaaacgcccgccgtggcagtggtgcaacccgctgccaatacactggggaataatatactggaagtaaaaataaacgtgttgaagaaccacctgcaacaggtaacgtttacggataagctgcgtgctaaagcattctcttttccgcaatatagtttgtttgaattaaaattgaaagatggaaccgtattaaccgccgctgatttccaggtaagcacaaaagacgccggtaacatcactgcttcaccaaccgcagtacggttgatagcgcgcctgcccggtaagcagctcacctttacattggtaaatactgtaaagaatattcagttgatctggcggatcacgttgcacaacgactgtaacttcattcagcagcatttccatatcaccgatccttcgtcggctgtggacgatctgttactggtaaatgttccatcggcctatcagccgcagctttcaggcactgtggacggttcgccggttatagccggcaacagtttctttgcgctggaacacccgatggcacagggacgtgtaacagacaaaggtattcaaagcagcgtggcggcatctgccacgctgcgctccggcaacgggtttgacgtgagcacggcctggggcgttaccccggaaacacagctccgtcgcggtttcctttactacctggaaaaagtgcgcgcggtaccttatcgtccttttccacattacaactcctggtacgatgcaggttacgacggccgggaaattaccgaagccaacgcaatggaccgtatccgcatgtttggcgacagcctcgtcgtaaaacgcaaagcaaagatcagcgctttcctttgggacagcggctgggatgattacaataaactctggtatttcagcaggcacctgcccaacgggtttaagaatatggaagcactggcggctaaatatcgtgctgccatgggcgtatgggtgtctccctggggcggctacgaccaggaaaagatcagtcgccttgccagcattaaaacgctcggccttccctttacgcccaatgaaaatggccttagcctggcggataaaaattacttcggctactttaaaaaactaaccaccggttttgtgaaagaccagggtgtggtgagctttaaattcgacggcgtaggcgcaggcaacggcgccagcggggcaggagagaagtacgctaaagatgtggaagcatttttacgcgtcatcaccgatctgcgcaaaataaaacccgacctcttctttaatttaacggtaggcacctggccttctccttactggctcaattatggcgacgccatctggcgcgccggcggcgatatggatgtactgggcgccggcaccaaaaggcagcaatggatcaactaccgcgatgcggaagtatataaaaatgtagtacaacgcgcaaaattatatccgctcaacgctatgatgtatcacggcgtggtaatcaataatgaaaatggcgtgggcgcaggttttaccaacgacgacaaaggcattgcggaagatatctgggagttttttggcaccggcaccggcatgcaggaactgtatatcaatccgcacctgatgagcagcaacagctggaatgtattggccaaagccatgcgctggtccgaaaagcaccgggatgtattatccgatgcacactggatgggcggtgaccccggcaaacaggaagtgtatggctttgccgcatggaaccaacaggaaggcattttaacatggaggaacccatctcccggaacaaaaagaattactttcaatctaaaagaagtactggaattgccggttggctatcataccaggtttgctgttttgaatgttacagaagatgtaaaagaagaagagatggatagtgagaaaacgattatacttgaactggcgccattccaggtgaaggtgctggagctgaagccggagaagtgattccaggttatttatggcgggcggtttttatgacagcgtttaattctgcgagaaataaatcagcttcctttttatttctgatagacatggaaaggctatcgttgcttaaacgttgcgtggacgtatcctcaaccggcctgacagccttgccggagcttgctgcaaactgaatgattttatctaatttttgttggatattcttcgtcatatgtcgaaattatggttttttattgaataatcagttgtttaaatgaaacatataatacctataaagatcctttgtagatctttggtaatcaaattgttccggtttaggtttgaaaaacggaaatcccagattgtctttttcaactgtattattccttaataatcttacataccaatctactccaattgttataataacgtcgcagagatactttttattggtttgaaacatcctgtgatacaaatatgcacgtatatcattagatccatccacgccaatggtcgatgaattatttttccgcagaaagcttaaggcaaacaataagaccgtcgagaacattttgccgatatttgagtgattaaccttaatctcgtcgttaatttttccttcttcatttaaaggaccaaaggccaggttgaaaacatttggcaataacggatcggtcagaggtctgatttctatttttagtaaaatcaattttccgttctttagtctggaatagaattttatatccgttaaatcagtggcaacttctatcggctcaaatgtatcttcaaagtttattctgatcattagtcaaacgtatagattttttagaaggagaataacattaattgtacactacaaagacataaatagtaatataggtttaacatatttttttaaaaaaaaaaggcgtttcacactcaatgaaacgccctctccacctcatttaaacgggtccgcatacttcggctccgttaccagcgactgatcagtcagtgttttaagaaaagcaataatatcatttttgtctttcgcggaaaacaccaagcccccgctttgtattcccgaaaactgtatcccgatatttggattttgtttgatcccggtagaatagtgttctatcgcatcttcgagtgtggcaaagcggccatcgtgcatgtacggggcagtcagctccacattccgcaggcttggaattttaaaggtaccctgatcggcgggtttgtgggtgatctcaccaatacctttgtcggtgtagttactttccagcccgttgttggagccaaacccggtatttaccccggtattgtccacaatgaggtaggacgagttttttcccaccccggcggtggagaagtcgctatgacattcggtgcagaaatccgcctgcatcagccgcatgccatttttttctgaggcgctgaagttgctgaattgcgtggctactccctgatcatacctggaattgaaggatacaatgctccgcaggaactgcgatattgctttggctattttatcggaggtaaccacttcgcttccgaaagcagctttaaatagtgccgggtagtaacttatccctgttaatttcgtttcaagagcagcgagggaaggtattcccatttctatatgatccaggacaggcatcagcgtttgcgtttcaatatctttggcccgcatgtcccagaacatggtggccgaccggaagaagcggagattcaccaccggcatgctgttacgccgggttaaattcccttcaaatccttcggatgtggctacgccgtcggtaaaggctttgtcctggtggtgacaggaaccacacgaccgggtattattcaccgacaacgacttgtcataaaataataccctgcccagggtagctcctgtattggtaataggattgccaacaggcgtattgtccagggtaggattggcattcataaatgcctgcatgtaaggaggcatattgttgcgggtgcccacatagtcataaagtgtaccgggcaggttaggagcgtcaggatcatttccgccaggctccgggttcggctcattgggtatgggagcggggttggcgccgttgttttcctttttacaggaaaccgaatttaaaataacaagggctgtcccggctatcaggcagatgagatttcttttgctgatggttttcgtcatggtacagatatttgggctaatacactttaattcatttttacccttacctggaaccattaaaaaattattatttgaaacagatagggggatttgaaagctgaagtgtattaccagggaacgatcacttcaatcacggtaaccggttttgtattgaacgcacatattggcaaggcagatgacctgtacaggcagatagaaacatactttcaaatgtattttgaaggattgcaccgctatgccttcactatactaaaagataatgatgaggccaaagatgcagtacaggtggttttcctgaagttatgggagaaaaggacaacaatagacgggcagcagtcggtgaaatcctatttgtatacggccatctaccattattgtcttaatataaaaagacataaaaaaataaaagatcattacgcaacaaccaacaatcatcctgccggcgaattcaggaatgccctggtcagcaaggaaacgcagcaacggatcatggcatgcatcggaaaattaccgccacaatgtaagctgatcttcaccaaaagcaggtttgaaggaaagaagtatgcagatattgcggcagaaatggacctttctgtaaaaaccgtagaagtccagataggaaaggctttacggatccttcgagaggaactgtcggacatcacgatcgctgtatttattttacttttattacaaccataatgagcaacggggagctgttatacgggttattagggaaatacttttccggggaagcctccccggaagaggcgatggccgtggatgactggatcacgcaacacccggatcaccgcaaattatacaacgaagcagcagcagcctgggacgcagccgggaacaacccgcatcaccagctgccggataaagcgctcctgctgcatgaaatcaaacaaaaggcagtggggtataaaccgcaaaggaacgcttggcgtatggcagcagtcatattggtgctgataggcgccgcgaccctttactttatatggcggccatcacctgcagttgctcctttggtgatcaggcaaaccaccaccggcatttaccacgataccctgccggaccactccctggcagtagtgaacagccattcggctatcaagtataccccgggcctcgcagataaaacaaggttcattcagttaaccggggaagcctggttcaatgtaacttctgatcccttaaaaccgtttatagtatcagtgggggacctgcgcattaaagtattaggcactgcctttaatgtccgtgaactggcagccgtgattgaagtagcggttaccagcggcgctgtactggtcagcaagggagataccgctataatagtaaaagcagcacagcagctggagtacaacaccatctcccaacgtttcagcatcaaaggcgcctttaatcccaataaaacgggatacgccaccaggatctttaattttgaaaatgcgtcgttgaaagaaattatcactcaactggaaaaggcatacaacattaaagtgatcctggaagataaacgcctggagaactgcaccatgagcagtgcctttgagaataaaccgatacaatacgtatttgaagtgatttcagttacgttgaatgtacaatgtagatttgagcatgacaggatatatatcagtgggacaggatgtaattagtctgctatcgaaattttttatagcggcagggttaaccctcttaacagccaccgtttttgctcaggaagccaccgtgaagttacaggaagaagtaaccattcccgttgcagatatgcgcctggatgccttgctgaccctcgtcagcaaacagcaaggcatccggttttccgtgaacacaaggaagtttccaacctccaggaccgtgcatgtaaaaaaaggaacgcaatctttgttaaggttgctcacagagctgcgtgaacataccggtattgattaccgtgtgctgggaggtcatattatttttgtagatgcaccaccgcttattgttacaaaaaaagctcctgtagtgataaaacgggaacgcgtaataccacctgcccgttttgtcatcatccctgtttccccggtgactaccaaacaggcaggtgttatatttcccgcgccggacaccgtaaaaaagaataccggctatttctggccactgataactgcaccacctgccggcgctaaaagaagcgaatcggcattcgcattaaaaccctatgccgccgcagggatggtagcagacgaatctttttatgtaaatccaaccatccatgtaggagtaccattcctttacctcgtcggttcctggagcactaacttttctttctctatgctccggtatggcgcaggtacttctatacgtttatcagacaactggcgtttacatctgcagggtactacaggaaggatggaagcgaactacgactcgctggcattcctgcaaaaaacagtgaaagcacagctacataagttatccctggcaggggaaaaacaaataggcgatcattggcggcttcagtttggggtggcgctgaatagcctgcaaacaacctattacacagaaggaaaaccacgtgccctgggaaagcaggagagtgaggcactcgctaatgtaaagtactttaaaccaccttataccatcagcaataatttctctccggatgcaagccgcagtaataaattatggatcggtttccaggcaggcatcttctacagtttcttaagatgattgcattaaacataaaaaagaagccggctccatgtaagaagccggcttccttcctcaattacctaacaccgctttcaacttttgatccaattcatccccgccacttccaacaagtttgaataatactttcccgtccttatccagcagtattttagtgggaaacccggtgataccatacgccattgccaaatctgccgatgccttttcgtagttgttaagtacctgtatccagccgatgccatcatcactgatggcttttaaccatgccttttttgcatcttccaggttgttggctttttcatctgcaacgcccactatttctaatcctttatttttatactttgcgtatacttccttcaggtgcgggtgactcgcccggcagggaccacaccagcttccccagaaatcaagtaatacatatttccctttaagggaggataacgtaaacggctgaccgtaattatcttttttggtgaagttaatagccgtggcgccctcgctggtagctttggcgccggatatccgggagcccaggtacctgcctaaataagtacttttataagtatcgcttaacttgttgtaagcctgctcataggctactgcatcgtagtcgccctgcaaccttaccagcaacataacgcttacgaaagacttgggatgctttgccacaaactgtttacgcataaccgtgagctgttcattggcggcggccatttctgttgtcatggctttcctggcggtgctgtcttccggtttgcgcatggcggccgacttcttcctcagctcccatacttttgataccagcggcatttctctttgccggagcgcattcagttcttcattggctttgtcgcccttcactactgctttgtaaagttcggtggcatcaccggtaatggttacatccgtattttccgtgagaaggatttccaggttaggcgcgggcataaacataccgcctttcaccatttcaaattttgaagcagggtggcgcgacaaaaaagtacccactaccggctcctgtacctgccctgaaaagatgaactggtcgccattgcgggcaattaccgtatctgccatatgcccgctggcggttacatacgacaggctcagacgatagtcgtcctggcctttgatatgggcagttatcttgtatttcttttgtgcggttgccgggagaaaagcggccagcagcatgctgccggccattatcaatgtgtttttattcatggttggtgtatgatgtttagaaactggacattggaacagaggccgcctgttttgcaggaacggctttggtgccttttgccaggctctcctttattttcttttctgcgtcttcactgtagccggtgaaacgctccataatttttccttcggtatccaccaggtacatagtagggatgccggaaaactggaattgttccatagtcttatccttgttatcactcagcaattgttcccacggcatagcttcctctttcattgccttttcccaggcatttttatcagtgtcgatggaaatgcttactacctcaaagccttttgccttgtaactttcatacagctcttttacctttgggatggcctgcctgcaagggccgcaccagcttgcccagaagtcaaccaacaggtatttacccttgtatttttccagtccggccagcgacccattggcatcagggtactttacagatggcataggctgccctgctttcaaacgcatggcctgtgctttgttggtgataatcgtttccttcagcagctttgcttctgttaaccacggataacgcgctatcagcacttccagcattttcatggcattgtcgtattgtgcacctgcctgtgtgcccgccataccacggatggcatataccatcaccgggcggtcggcatacgctttggtaagcacctcttcgcggattttataatcctcgcccatcgggttatatttctgatggtccctcatataggcgtaccagttagtatcagtggctttcttggcataatactccatgttgtattcatctatcatcctgcggtaattcagctcgttgttcagctcgcggaggttcacaaagttattgtcgtaagatcctgctacataattgtagtgcggaatcttcaccttatacctggcagtatcataccctctcatatgtaccgttatatcggcatcgctccagaaggtggcacggtcccagttcatcgcattgataatataaatgccctggtggtcctgtttaattttaaaagaaaaggaattgtctttgcctacttcacaggaatctactaccacaggttttcctttgaagttatctttcgacaaaaatactttattgaccgcctgtttgggatcggtaaattcaacggtgccttttaccgtaaccgatttaactaacttgttctgttgcgcctgtaatgctgcgggtatggccagcaccgctacacaaatcttgaaaattgctttcttcatcattgtttgtttaatttattattttaatattttatttactgtaatctgcattctgcgccaggtcaggattgatgaaaaattccctggaaggcagcggcatcaaagcatgcgttatgggttgcccgaacgattgcagccagctatccattttaccaaaacggcgcatatcactccaccttaaacgttcgccaatgaactctctgcggcgttcctgttctatcatcgcaaggaatgcggccgggctgctgaaatcgctgctgctgacagtgctggctttacgggccgtacgcagctggttatacatgcttacatctgttacgccttcccgtgcattggcttctgctacaatcagtaatgcttcgctataacggcaaaccacatacgaaggcgtaatttctgcaggaaacttggtgagaaagtatacagagtctatgatagcggcgcctttggtacgcaggaaacaagttctgcgcacatctgccggctcataggatttaacaaggttactgtcggcccaggtgttgccggaaccggacatattcacgccgttgtaagtaccgggaccaaataccgcaggcagtccgtaaaaggtactggtgctggtttcattgatcttatacacggcttctgcactgttcacctgcgatttgaaaatatcggtatagctagattggaggctgaacttcccggagctgatcaccgctgttgcctggaccagcgcttcatcattacgcccctggttcaggtataacctcgacaggagcagctgcgctgcctgtttggacccggctgccgggctggtgtagtctgccagcagcgtaacagctgctttcaggtctgcttcaatcagctggttgactgctgtgagcgggctgcgcgccggccggcttttgggatcttccccgccttttatgatagcagcgtcaccaaagcattcagagagcagcatataggagaaggcacgtaacaggtacgcttctcccagcgcagcactgatggtactgtcgccaggaaacccgttggcatattgaattaccatgttggcattggcaatacactggtaaggctgccggtacgctacaggcaacgaattatcattgggcgcgatgttattgttgtcgtatgtggggaaggtgagcgattgaaagtcgtcgctcataatatcctggaacgcataataaagataaaaggaaccgttgttggtgagcgccagcttggcgccgttgatcaccagcggcaggttgtttttactgagttgtgaaaagccgatcttcgtatcgggcgccacctcgtccagttgcttactgcaggcagaaaaactgatggcggctatagcggtaaaatataataaaatatgttttttcatgtgatgccagattagaatgaaagatctatacctacaacggctgcgcgcggattgggcaggttggaacttacaataccgttattagcggctgcttcaggatcaaacccaatatatttcgtgatggtaaatacattttgggcagatgcgtagatgcgtgcccgtgagatctttaccttgcttaaaactaccgttggaatgttatagctcagggaaatattgcgcaaacgcacataagatgcattgtagataaattgtgtggaaggacgatagttccagtcggccgtttgtccggcgccatgtggccctgtaatggcccttggcacatccgtgatatcgcccttttgcttccagcgcttattgatgatatcaaatttgttaggcattacaccgtaaaaatcggggctgtagttgcgtaatgtttgctcatagaaatcatataccttgttacccaccacatagttgaacagcgcatctattgtaaagtttttgtaagacagggtaatgttggtgccaccggtaaatgtgggcagcgccacgggtacggtgatcatatcattgttatcccatttgccatccttgttctgatccttatacaacatatcacctgtttgaggatccacccccagcgactcatacacctgcacggagcccagcgattgccccactttggcttttgtcataggcccgccaaatacataggcgccataagtagtaagggagtctttcaatgacagcaactggttcctgttgatattcatattggtttccactttccacgaaaacgctgccccggcacggctgctgagcgccagttccaggtcagcgccatagttacggatactgcctatgttatccgggatgctgctggcgccgtaaatccaggagatatcattgttgctcattaaaccatcggtggttttattgtaataatcagctgccaatgtgagcctgttgcccagcagcgatacatctataccggcatctatctgtttggttcgctcccagcggatattcggattgcctataacggtggtcagcatcaacgccggattgtttacgtaagaagtagcgttaagcagattctgcgcatcaaaatatcccagcggacggatattgccactgatgccatagctgctgcggattttcagctggttcaccaacctgctgccggaaaggaaattttcacgcgctatatcccatcctgccgataccgcaggaaaccagctataccggttacccgcatttagtttggaagaaccatcgcggcggatggaggcattgaggaggtatttgccttcccaatcgagccccgtgcgcagaaagtaggcgtcagatacttctttgttactgctattattactgccaatggcaaatgcgctgccataagcgctgccagcgcctccgccggtaataccatctattttaggaaaaccattcagctcatagccaaagtaattaagctggttgttataaaacgtgtaacccagggtggcattgattcccaaacggcttacctttttcgtataggtgaaatagttatcgaaattataagagaaattatccacgccggtgtttttcaatacgcccttgttaaaagcccccaggtagccggtaggaggatagaacactgtgttcagatcattgaacttagtggcattgaaagaggagcggaacgacaggtcctgcaataatttaatatctgcagataaacctcccaggtatacattgttcctgtctttgttgttgttgtccatcattacacccagcggatgctgctgctgaccaacataataacccagcgagccatctgggttcagtaccggatccgccggggtgtctggccgtgcattgaatgcggccaccaacgggttattgaaattcttcctgactgattgcgtaatgttgatgttgccatttatctttaaccagttgtttacctgctgggttacgtccaggcggcctgtatatctttcaaaattgccggtaccaatggtggcttcttctgcataacggcccagtgacatataataattattcctgtcgccgccaccactcatactggcctggatattattcaccggcgcatttttatttttaacccggtctatccagtcggtgctgcgatccgccatttgcaggccattcacctggctttgcagggtttgtttttcgttggtcagctggctgatcttgccgggcgtgaggttgccgggatccgatagcaacgtattgatatcgccaatacggttattgcgggcatccaggaaagcggaactgtattcttccgtattcagcatatgccgggaagtaggcacattgttcactcccgtgtacatattgatgctgaaagcaggcttactgttcatcctgcccttcttggtggtaacaatgatcacaccggtagagcccctggcgccataaatggccgctgatgctgcatctttcaatacctcaatggattcaatatcctgcggattaatattgttgatagagatggtacttccctctacgatcaaaccatctattacaatcagcggattggtgctggccgcattcaccgactgcgccccgcggatgaggatattgggtgtgccacccggacttccgtctttagacgcaacaaatacgcccgctacacggccggtcagcgctttcccgaaatcgctggcaatgtttttttcaggagataaagcatcgcttttgacggtggaaatagcgttggttactttgcctctttgctgggtgccgtaacccactaccacggcatccgtgagattaatagccctgattttcaaccataccggcgaagcctggataatactggcagcaacaattacattttcaaaacctacagaggagatctgcagttgcgcattggcgggaacattcagttcaaattcccctttttcattggtggtggcgcctttagacgaaccaattacttttacggtggcgccgggaaccggttggcgggaaaccgcatccttcacggttccttttagtacctgctgtgcatataccgacgccccggacatgcacaacaacaggaataaaaatgactttctcatacaaatggttggttgatttttgcgatatacggactgtctcagaaaaatgaaaatccaagatacttatcctgttttcagctgcaccggataatggacataccgggtgcggaacagtacattccctctttttacatggatgaaacattttccccgccacaaaagcacgaatcaccggaaagtgccggcagcaggtactttccggtaataataaagtaccaacaggcatataacagggacgaaaaaaataaatatcgttttatgccaaaaccgttatttcaaatgctatcttcaatgttgtaagtgtatatgcaacacattaaaccataccgttattttgttcacctggccgtttgcatggccgtgatactgctgtatagttttccgcagctgaaaggaggctggccctatcccattgccatgaaatggacattggtacggctggtgctgtacggatgcattaatttccacctgttttacctgctggttttcggtttacttccccgcccggtacaatataaacagcactggaaagtgatcatttatgtccttgcagcgatctttatttttgctgttattaagtacatggtaggttatttctttttccccgaccaggtattgctccgcgggatcccttttattggccgccccaaaatatatatgaccttcgtcgagtacgcaccggaaaccatcaaaacaggaatgggagtagccctgctggcctacggttaccggttgttgttgcaatggcgcaataccgcacccggcgaccggttgctcgctaccgccgccacacaagccgccatccgttatgagcgtatgcaggatggatccaggcagctgctgcactatctccagcaactcacaccggtactggaaaatgaacaaacccgcgaaaaagaaggaaccaaagcgatcctgctgttgtctgatttgctgagatatatgctgtatgataaagcgctggaaaaagataaagtgagttttaagaaagaactgctcaactatgaacgctacctggatttgcgcaggatctgtcatccccatcagccgctgaccctccgcatcaccggggagcccggcggtatgatcgaggcattacggctgcagaacaccacagaaaaatacctgcagcaactgggtgatacgccgggcggaattatgatagcactgcatatagttgaacaatcggtggcgctgtctgtatcgccggtgctcacagccgttcacatctcccaacataaaataaaattgtacccggaatatgcatagtacccgcaaaaatatacaggagctgttgctcttattgctggtatggatgctggcggtatatggtgttaatgtgctattggcgaggccgctcacaccagagaaattacaccatttaaacatcaaatccggcctgttcgggttgtttaacttcctgccgttttatatttatgtacgctggatagttcctgcctttctacaaaaaacaaattggataaaactgttgctgtctgtagtaccggtcatcctgggaagcattgcattgaaatattttatcgcggatcattttttcagacaggaaatactttatgcaggttaccggtatgtgaatatgcaaaaagtacagctgtatatttccgcaggggattatttcctcagtaacctgtggagcggcgctatgattgtgttagccgctttctcgtaccggttttttattttgtggttacaggaagataaacgcagggccattttacagcaacagcagctgcaggcagaatcaggttttctgaagatgcagctcaactcgcactttttaatcaacagcctgaacagcatctattccctggcgctgatgaactcaccggaagtagtaagcgcccataaaacgcttacccacctgctggcctatatggtagaacagccttcagatattgcttaccgcgctgctataacggaagaaatacgctatttgcaggacttcgtaacactccagcgcatacgcacgggttgcaacgaaggcgttattttttctttgccggaacaattgcccggcaaggaaatagcaccgctgctgctggtgcctttcgtggaaaatgcttttaaacacggcgtgagtaatcgcccggaaaagccggtcaccattaccatgatgtgtaatgaacagcgactggtattccgcgtacacaactatatatccggccagcaacgggataaaaccggtggcataggactggacaatgtaaggaaacgtttacaactgatctatcctggccggcatcacctggaaattcaggatttgaaagaagaatatttcagtaacttaacgatcaactggtaataatatggcggtaaagtgtatagtagtagatgatgagccattggccgcacaggtgttggtagccttcatcaacaaaacgccggacctgcagctactgaaaacatttcacaatccgcaggaagcactggcatttgtaaaaaatgagccggtagacctggtattcctggatatacaaatgcaggaactcagcggcatagaatttatgcagctcgcaccccgcggtatacaggtagtaattgtttctgcctacgatgagtatgcagtagaaggcttcgaccgcgaagcagtggactatctcctgaaacccgtatcgtttgagcgtttcgcgcggaccgtacaacgggtgctcgcgaaaaatgcgcccgctatatcgcagcctgcaggcaccgattatatatttgtgcgcaccgataaacgcattgtacgggtggatgtaaaagatatcctttttgtagaagcgctccgcaactacgtagccatacaaactaacaagcaaaagatcctgacgttacaaaacctccgcagctttgaagacatcctggcgcccttccgctttttccgggtgcataaatcgtttatcatctccctggataaaatagacagcatagaacggcaacggatattcacaggagaacatcatgtgccgattggagatgcttacctgaaacagtttatggaagcgattaatatgcagcggtaacactatctcatttaataaaaacggcccgccaaccggcaggccatctttaaattgaaccccggacccggactactcaggcgccagtgggtacttcttttctaatcctctccgcctcatgaatcgccatcaccgtttttatgattgcatctggtgtaactgaaatactatctatgcccagctgaacaaggaacctggtgaagtccggaaagtcggacggtccctgcccgcagatccctacctttacattctgttgcttagccaccttgatcaggtgcgcaatcagccgttgcactgcggggttacgctcgttataaaggttggccaccagggaagaatccctgtcgagaccaagtgtgagctgtgtcagatcattggatccgatcgagaatccgtctatgtatgcagaaaattcttcggccatcataatgttggaaggcagttccgccatcaggtatacttccagtccatgctcgccgcggcgcagcccgaattcctccatcgtagccagcaccagctgaagctcttccacggtccggcagaaagggatcatcaccaccacattctttaatcccatcgtttcccttactttaaggatcgctttacactccagctcaaaggctggtttgtattcaggggaatagtagcgggaagcgcctctccagcctatcatcgggttttcttccgtaggctcaaagtatttaccgcctaataaattgaagtattcattactcttaaaatcagagaaacggacaattactttttccgggtaaaaagccgcggcaatttttcctacaccatacgccagtttatcaacgaagtaatctgtttcgctggcatgtccctggatgagttgcgcaatcttcgcagacagctcagggtcattcagttccttgtgcttcagcaatgccatcgggtgcgccttgatgtagttgttgatgataaattcttcgcgggccagtcccacgcctttgttaggcaggtgtgtaaactggaacgccatggcgggagagcctacattcagcatcagcggtgtgcggatggaaggcagggtgctcaggtccagtttatcttcccggaacggcaggatcccttcgtatacaataccatcgctgccttctgcgcaactcacggtgatgtcctgcccggcgtttaatttttcggtagcatcgccgcagccaacaatggcagggatacccatttcacgggctactatcgcagcatgacaggtacgtccgcctttattggtaacaatcgcagaagccattttcatgatgggttcccagtcgggatcagtcatgtcggtaaccagtacgtcgcccggtttgaattcactgcccgtaataaggcggttatcgagggagaagaggatgtttactttgccggcggcaattttatcacccaccgcgatgcctttcagcaattgtcggggatgcgtgccgttatggttgatcgcataagtggtgatgaggttatgatctttgcgtgaatgaatggtttccggccttgcctgcacaatgtataaatcattggtaagcccgtctaccgcccattccacatccatcgggcaccagcggccttttttctcagaataataggtttcaatacaacgcacccaggtagccagctgcatgatctgggcatcgcttaaacaaaaatgttgctgctgctttttttctaccgggatgatctttgttctttcatcactgctttcgccatacaccattttcttatcctttacacccagtttcttttcaatgatagggatgtagccatccttcatgcatggtttgaatacaataaattcatccggcgatacggcgccctgtactaccatttctcccaatccaaaagaaccgttgatcactaccacttctttgaatccggattctgtgtcgagcgaaaaagcgaccccggaggcgccaagatcggcccgcaccattttttgcacacatacggataagcctatactaaaatggtcatagccgaagttctggcgatagctgatggcgcgatcagtaaacagggaggcaaaacagtttcttaccgaatcaatcagggctgcggggcctcttacgttgagaaaggtttcctgctgaccggcaaaggaggcatcaggaaggtcttccgcggtggcagacgagcgcacggctacatcggtttgttcctgcccgtattgctgcgataaagcataatacgcagcaatgatttcctcgcttagttcatgcggaaaccgggtgctgctgatggcctgccgtatcttctgaccggccctgcgcagggtgatgatgtcgctgtagtctaccgtggctacctgctcggcaataaattgttcgagcccgctttgcttcataaattcatagtatgctttggtagtgatagcaaacccggaaggaactgctacgcctgcttctgaaagattggcaatcatctcgcccagcgaagcagatttaccgcccactaaggcaatagcatccatgcccaccgcgtggagcggcagtacaatactctctctcatgtaaaaatgagtttagtgaataataatgaggaaggacatttttttgtcttccaaacgtggttagatttctatgacaccaaattagatcatgcagaaatggaatagcggcaacccggataaaagcgaaaacaaaactaaaaaaaggggatgtcaccgattttttttcatcaaatcagtagcagtatcattatttttgatgaaaaatcggcccatgaattttatacctgaccagattgatatgtgtataatggacatattgcaggaggacgccaggaccacgaataaagagattgctgcgaggttgggtaagtcggttacttctatttttgaaagagtgaagcgccttgaagcagaggggtatattttacgctatatcgctgtactgaataaaaataaactgggcaaaaatctcgtagcctggaccagcatcaccctcaaagagcacggccaggacaagtttccggagtttgaacaaaagatcaataccttccccgaagtaatggagtgctataaaatgaacgggcagttcgactacctcctcaaagtactcatcgcagatatggaagcctatgaagtatttaattttaccaaactatccaaactggataatatctacaagatccgcagcctgtttgttttagcagaaacaaaacaggaagtggaactcaacctcaaaacaggactgcaaacaaaactgcaacagaaaaataaataattttaaaaagtaggggagaaggtttttttttccggattatcgtaatttcaggaaaagttaacccatatggcaaaacaaaccgggatgctccagttcaccggtaggctcggtaacattatcggctacaaacgaaacggctcctacttcctccgcactatgccggaaacagtccggcaaacttctgctacccgaaaggcagcacaccattttggcatcgccagcaggaaaggtaaactgatccggcaggccattactccgcacctggacatcaattccgatggatcactggtgaaccgcctgaacaaaacacttattccggcagggaaaaatcacctgcatgctgtcaaaggattccggtttaaccggcattgcggcctggaatacttcttcccggatcaaccggttatccaggacaacatcgtgaaaatacctgcacaggtaataccgcaacaggaagctttcacccacctggtggtaaaagccattgcggtacggctctgttttacggaacgctgcattgagaagatgtataccgccactgctatcattgatctgaaccagcccttcaatggcgcggaactggaaacaacccttccggggaaaggatcactgctggtaatactacaggtacaaccttacaacggtacctatgcaatacagaacaaacgctgcatggcggcggatatcatagcggtaacggcacccgcagccataaagcgaaagaccatcacaacaacaactgatcaccgcatcaagtccaccttttctgcacgcatctggcgggtcctaagcgacccctcgccccatcctccgccattgcttagcgatgtcaccggccattcaccaccgggaattgtgaaatccgcaacttagtacacccaaaaggtaccaaggtaatctcttcttcttcccctgtttccataccataggtaatgctatacggaatggggccggtcatctcattgtataacttccaggaaggaatcctttttgcggttgttttaagggagatgggtacctgcccgggactccacggccagccagtcttactgccatgttgctctacccggtaacgcgctgccagctgatcatccggagtggctatcagtgcgtagttccatggggtagtaggccgcacttccaggtaaccggcgccatagtccaggggatccttatcgttttttaccgccctcacttcctcgcctatctgcagcgcataggtaaccgggccgcgttctactgataatgaattttcaaaccagtgttgctggtagatatgcatcggcaacaacagttctactacatcaccttgctgccaggttctttccaccttcactacctggttgcctgcagcttcctgccatactttaccattgatctttataaccccttttttacaccacgcaggtatccgcaggtgaaaagggaagtttacttttttgggtgtattaacggtaaaagtaaccgcttcttcaaacgggtaattagtgacttcctttaccgtaacaggcgtttgaccggccacatttatcttcacttcgctgggggcatacaccaatgctgccacgccactgtcggcggtagcataccagaggttttgtgcaaacttaggccagccctggtgcatattggaggtgcagcagggataaccggacaacaacccgtaacaaagatccgtaccgctgtggtttacatcaaagttgcggatatgccgtgtagccatcacctggttggcctgctggaaatactgccggctcataaagtcttcggtaatctgcgaaggcaatacattaaacgcgatcttctccagctgatcggcataccttacatcgccgcttatctccaggatactttcaagcgaaaacatcatctctacagcgctgcataactccgatccctgcgtgggattattgccatgcagggcttcatcaccaccataaaggccattcgccatcccattgaaggtacggaggtcatcaaaccctttggccgtggcctgcgggtataacgtgtcgggctgctgctggaaatagatcatgggctcttttatgccctgggccaggtttacgccatgaatactccctgtggtcgataacaggttggtatgcataaaggcgccggcatagtcgaaggtttgcttgtggatcagggctgcaaggtccagcaggaacgcatctcccgtaatattatataaccagtacaccaccatcaggttatcacccgcgcggtacttcgcccagaaggtccagtggtccagcggcttttgcggcaactctttcaactggtaccggaagtagttggtcatgagtgtaatgatccgcggatcagcggtagcatcataatattgcttcaacactttcagcattaccatcttgggccaccaatcgcggctgttatccctttgaatccccggttcagcgggatagtctttagccggaccaaaatagccgtcgggttgctggcttttgatagaccattccacccagggctttacctttgcaatcagcgcttcatctttcaggagatacgccagcggcagcaatccgtcgatccagtaagggccgcgttcccactggtcgccatccccgcccagccatccgttccgctggttcatgaccagcgggtacaatttatccagctgaccggtagcgccattcttttgctgcaccagcacggtacgcagccatccctgtggcgtaatagcgcccaaaggaagcagggagtaaggtttaggatggagcggcgcccggttgccataatactgtggtgcaggcgctgtattcttttttccctgcgccgctgcctgtaaagtaagacccagcaatatcgaggaagcaatagcaaagtatttcataaatgagtggtgacgtggcataatgaaacgccaatatatctttatttcacaaggcgagttatcccggttgcctcattctttctataaaacgtatcataacacctactcataatgtatctggcagttgttacagaaaaaactccgccggttggttttacccaggtaggctttgatgagcgggatctcacaacgcggacaaatctttttcgtatgtgcgagccagtgcttcttcagcacaaaagctttcttccattcaagaaagtcgtagctgtattgtactgcctcctttaccagctccttcttctttttcaacggcagctttcccaccaaactttgcggatgcacgcggatacggaacaacacttcatttttgataatattccctacgccggcaaaaatatcctggtttagcagggcatcacaaaccagggcatcaggtatctttttaagtttagccattgcctttgatgcatcccagctttcattcagcacatcggcgctccagtcgtatacttcatccaatggctcctctatgatccggatggaagaggtataaaaattcagttcccctttggcaaactgcaggtgcaaacgggcaggcatatccttggtttcattgatccggtaagtgccaaacatcaggaagtgaatgcggactgcaaagcccggaaaacagatcaggaaatgtttgccccagcttttaaaagcgatgatctttttccctgtcatccggctgaaatcaattgttttggagttgccggaggccataagcaccttcttcccggtaaagcgggctgcctcttctttcaatataactatggaaggtccttctggcataaaattgatgtaaatttatctaccgttaaccgtactaaattatgtgccgtatatgtcgcagttaagtttttttgatgacaacgaaagcctgcgcttcccggagaacctgctggaatattacccgcatttcctggagacagggcccgcactggcactgatgaatgagttgatagccaccgcgccatggaaacaaaccacgctcaccatcaaagataaagtactgcttaccccgcggcttaccgcctggtatggcgatgcacagaaaagttaccggctgtcggaaaaacaactgcacccatttccctggacacctgcgctgagtgcgttacgggaaaaggtagaagcctttacccatatgcacttcaacagcgtattgctgaattattaccgcgatggaaatgattcggtagcctggcacagcgataatgaaaaggaactgggacaacatcccaatattgcttccctgagcctgggacaggccaggagctttgatttcaggagtaagaaagatcatcagcagaagtattcacttaaattgggcaacggttccctgttaattatgaaaggggacctgcagcatcattgggaacacagaatcccgaaatcagcccggcccctgcaaccaagaataaacctcaccttccggattatttattagttggtattattacacagttgaggaataatgtcacacccgtttatggcatcttgttacaaatgcctactttcgcagtacgttaaacacctgttttatgaatctatacacggcagtagcattaccgttattccttttgaccctgcatccccgggatgtacacagcaaagacaaagctaacacggaattttcggctccaaagccccagtcacggatctctatcggcaagggtattgatcttattgtaaaaggactcggactgaacatcgataacgtccgttttattaaagcgcccaaagccaccgattattttaagaaggccaacgataaagcatcgtatgcaccttcgctcattattgcggctgtcaacggactggagtcgctgcgcgacgtaaacccggaatcaccggctacccgcgaacagtttgccctggcgctgtatgaagcgatccagtcaaccgggcagtatcccgtgaatatgatgtttatcaacatcaaagatgaaaagtcttttgtaagcggaggtatgaatgccgtgcaaacattgatcaagtttaatgtagtggcactggaaaatggcaactaccgtccaaaggcatatatcaccaaaacagaagcttccggaatggtgaagaaggccgctgcatttattcaatcgcataaaagcgctgcagcagaacataacggaaaagaaacggcaagctttacttccacaccggtgaacgataaagtgaacagcatcgttatcaccgcggaaaaccagcctacatccggctattcggttaaagtaaccagcattgtttttacagaagcaggcgaagcagagatccattataaactcacagccccggcttccggcagcatcaacctgcaggtaatcacctcaccaacagcagaaacatttgtacctgccgggtataaagtagtattgaaacaagactgataaaatatcgctataaaaaaagcgggcatttcatatctgagatgcccgcttttttatgatattttttttattcagatgctgtccttgcctatcacggtccagtcgttattgccatgtcccttctcaatccaccggtccatttcagcggcaatagccggcaacaccgccagtttaacatcgcttttctttgccgcatctataaacagctgcgtgtctttccgcgccatgctcagttcccaggaaggactgttatagttaccggaagtcatacgctgtaagcgtgcgggcaacgccgctccggggttccatgaatcaaataacgtacttacatcgcccaaaggaatgttcagtgctttggcaagcgacagggtatcagcaagaccggcagtgagccccaccaggaagctgtttccgatgagtttcatggccgcagctttaccggccgtatcgccgaaattgatcaccttccccgtcattttggagagtgcaggctcccatgtgctgatcactgcctgatcgccggaaaccagcatgtaaccggtgccgtccagcgcatttgccggacccataaataccggtgcatgcaggtaagtaaaaccgcgttccttccattcttttgttctggcagctgcgccttcggcagaagtggtggtatgatcaatgatcaccgctcccggtttaagtgcagtggctgctgccgccaatacttcatttacagtatgatcatcttttaaggtaagatgaatgcggtctgcgccttgcaccgcagcggttacctccggaaatactttggcgccgtatgcttccagcgctgtcgctttcgacgcggtacggttccatacctgtacctgttcacccttgccgatcaatgcccttacgaaatttgaccccaggaggcccatgcctaagaatgctatcataaccttttttttccgaaggtagcaaaaagttaaaaagtgttacctgcatatacggccggtttacgtccgctccacggcgccgcggcttccagctgtgctgccagccggagcagcaacgcatcgttacctgtttgggccgaaaaggtaatgccaacaggcaggccattatctcccatacccaatggtaagctgatggccggcacaccggcaatattgaatacctgcccaaagggagcaacggcacaaacttcctgcacccagctatgccagtcgatgtccgcggcattgccgttcatgctgccggctaacggcgcctgtatagcggtggaaggggtgatcataatatcgtactcttcgtagaagttacctgctgcccgtgatacggtattgctgtattctaccgccctgatgaggtctgcggcagacaatgcctgacctgcctgatagccgctcagcgtgctggtttccagcgtttgcggggagatgttgcgttgcatggcatgcgatacctgtgtgatgccgtaaaacgtataggcgccccagatagtcttgatgcaatcgagaagctgcgtcgcttccaggtcaaagcgttgctcttccacccggtggcccagcgaggcgcatagcgctgctgcggcttttacggcattcactataaccgggtcaacgcttccgggcagccatggctgcaggttgaaagcgatgttcaatacaggcaggggctgtgttaacgcagctacatacgaggctgccggcggtgtgtagtagaattcgccgggcgcggggccggcagtggcgtccagggcagcagcggaatcgcgcacactgcgcgtgagcacatgctgcaccgccaacccgaaaaaggattgtccccggtccggccctacgggattgagattacggctgggctttagtcctaccagcccgttaaatgcagccggtatgcggatagatcccgccaggtccgtagcgtgcgccatgggaaccatacccgccgccaccgcagccgcggagccaccggatgatccaccgggggaatagtccgtatgccagggattgcgggtaatgcccgatgccagcgatgccgtgtcggtagacccgccaaattcaggtgtggtggtacgacccatgatgagcaagccggcggccttgtaccgctttaccagttcggtatcatgcggcgccctcatacctttggcaatgcggctccccatttcgtaatactggcctgcttcaaaggctgccaggtctttcagtaaaaaggggacgcccgcaaatgggccgctacccgtattttccggtaaatgtgctgcccggtcggggtaaacttccaccacggcatttaataccgggttcaactgttgaatggcggccagcgcgcattccgccacctctttccggctcacctgtttttctttaatcagcgctgccaatcctgtggcatcatagccggcgtattcagataaatgcatatttcctgttttttgttatagcaaaattatacccggtagatgggttgttttaggtatgattttgccattattaggtatatttgcacttatgaaagagaatctgcattatccgtttgaaatcatttataaggagctggaagtaggtgaagagaagcggcggacgagcaatttttttgagctcatttatatcatggaaggtacggggcaagagaccatcaatcagcaaacatttaattacgtgccgggacgcctgctgctcatcacccctgaagacctgaccacctttcatatcactacgcccacgaagatgttgttgatctgctttaatgatatctacatcaggtcggccgctttttccggcaatgagcgggagcgggaagcgtggattaaacggctggaatttatcctgcaacacgccaaccacgaacccggttgtgtcctgccaagccagccacataaaatgctggcaaaaacaatggtggaaacgctggtaaccgaataccagcactgtgatctgtacagcaaggaattgattcagcagatggtgaacagtcttatcattctcgtggcccggtccattgcgcaaaggctccccgataaatttaccccggtagccgataaaaaaacgctcgacatcttccaatatatccacgagcatatctatgagccggaacaactaaaggtgagcgccatctgccagtattttaatatctcccccaattatctcggtaaattctttaaaaaacaggccgacgaaacgctgcagcaatatatccagcattataaaataaaaatggtggaaacacgcttactccacagcgatatgcggatcaatgaaattgtaaatgaattagggtttacagatgaaagccatttaaacaggctttttaaaagatataaagggatgagtgcttccatgtaccggaaaacaatgtggaatgcggatatcagcgcgtttacaaaaaacaaaacaatagtgacggaccagcagcgtggcgcttaatttttcagatcttcctgaaggatcgcttctttcaatacttcttcgtgtgcatctgcccattctcccaaaatttttattactggaatgagggatgcgcccagcttagtaaggctatactccaccttcggcggggcctgtgcaaacactaccttcgacaccaggccatgcttttccatttcgttgagctggatgttcaatacccggcgtgtagcatccggaatcttccgctgtagctcactcgggcgcttatgcccttcatggatgaaatacagcaggcgcactttccatttaccgtagagcacttcccccacgaggtcgagaccgcaattcagtgtaatgggtagtttttttacatacatggttcaaaagtactttattgttcttaaacgggctatagggataaattccactctatgcgaatcgtttttccgttattgtccggcatagatgattgacggaattttgctgaaaataataataacagatggaaccaagattaagttttgacaacgaactatccggtaaaacagccctggttacaggcggtacaaagggagcaggaaaagccattgcagcacgactggccaatgccggtgcaaaagtgatcatcactgccagaacgaagccggcagacacgaacccggcatttcattttataggcgctgatctgagcactcctgcaggcattacgagcgtagcaaacgaaataaaggaaaactacggcggcgtaaacatcctggttaataacatgggcggttctgaaacccctggtggcggctttgaggtattaacggatcatcattgggatgccaccctccaggccaacctgctggcgccggtgcggctggacagagcgctgttgccttacatgctggcacaaggcactggtgtaattattcatattgcttccatacaaggcactatgccgctgtatgattccacgctgccctacgcagccgccaaggctgcattgattaattacagcaagggcttgtccaacgaagtggcgccgaaaggagtgagggtactcactgtatcgcccggctttatccaaaccaccgccgccgacaaaatgattcaggaaatggccgaccgtgccggcagcagctttaacgatgccttgcagcaactcatgcagttcctgggcggcattcccatggggcgccccgccaaaccgcaagaagttgcggaccttgtcggcttcctcgtttccccgcgtgcaggatatttaaccggcacacaatacatcatcgatggcggcaccatccccaccacataaataaaaaatgggaagatgaaaatgccaccatttccatcttcccaaataaaaaataaaaaatccaacccaacccaccccaatcaaatcaaaatcaaatcaaaaatcaaaatcaaatcaaatcaaatcaaaatcaaaccaccacaccaaatcaaaaaacctaatcagcaaaatcagcgtaatcagcgggaaagacaacctccgctgcattaagtccgcgccttgtcggcccccccgctctccgcacccgcattacccgtttgcagcaggagtacaaaaggcgccgcccgcggtgcattccccacctggatgaagtattcactccgcccgatcagctccggcgttatccgcgcttcgggctgccccacaggggagactttcagcaggataacccgcggaggcagtttcacccgcaggttgccggataccggtacgttgcacactaccatgtaaacgctgtcggatccgtttttgcggatataatagccccagtcctgtttgtcaaaaccggcatagccgccgccataaacagcggcgccgtttactttcatccagttgccgatttcctgcatacgctgcgtttcttcagggcggaaggtgccatctgctttggggccgaaattgatgacgaagttgccgccaagagatgtggattttaccagcatttcaatcagctcgtccgaagatttaatatgccctgtccatttggcgcagtatccccactggttctcggggatggtcatcacaccttcccagtcgttgccatggatgtccgcatatttttcgggcagcttgcgttcccatccctgttcgtaatcgcccatgaggcggctgttggaatcaaaatgccttgcgcctttttcgtcggcgcggaggcggctgccaatgatcagcccgggatgcagttgctggaggtattgttccagctcatcggagaaggcgccgtcatttttccaggagtcgtcccaggtgccatcaaaccagaaaccttttacggtgggatatttcaccagcagttccttcagctggtttttcacaaatactttgaagcgactgtaggcaaggctgtcggccggcgttttgagcgaggcgtgccagtcggggtggttccaatcgatgatagaaaaatagagatatacgtcgattccttttttattataggcatctaccattgggccgatgatatcttttttataaggcgaggcggctaccgtatagcgggtatacttactgggccacaggcaaaaaccatcgtggtgtttggtggtgatgatcatataggctgcgcccatatcctttgcatattgcgcccattgttccgggtgatagtttacgggattaaactgtttgtataagttgtcatagtcgcagcgcggcatttctttccaggagcggatccactctgcggcgccgttgtatgttttcccgttccattcgccaccgggaatggcatacaggccccagtggatgaattgtcccaggcgaagggatcgccagcgggccatatcggcatcggttctgttgccggtgcggtgggcgccgtgttgcagggtgatggtgtctttaataggattgctttgtgcgctgctgtgcagttgtgcgaggagcagtgcggcagcgatacagtattttttcatgttgctcttttaatgggtccaggtaatggtgtccgtgtatactttaccgttagatacgccggaagcggtgagggtgttcacacctgtcttcagcgtaaggttatcaaaaataaagtctttactattggcgcctgtgcgaccggtaacaggcgctccgttgttcagtgtgagcgttaccttttccaggttgctgaacacttctgcgtgtacccgttcgggttgtcgcacatggttccgtcgctctgcaatgtagatcatgggagcggggttccagttggctttgtaccagtagaaggcgtcctttttctgtttgcggtcgtaggtgatgagtcctttcaggttgcgtgcatttacacccccgcggttccacatgggcactgcaaattcaaacatattccataaataggaggccgcaatataaggatgcttttctatcactgcccattgttgcacgtgtgtggcagtttgataggtttccggaaaaaactgcccgcttaccggatcaaagttggtactgagactatcggtatgctgatcaatatttccatctgcgccgtattctgtgagcatcagtttatagtcggggtagtttttctccaggccggatacccatttttcaatgtcgccgatcctgccttcataccagccaaagtagcggttcatgccttgtatgtcggcggccaggttggccgggcgggtcatttcaccataaccgcttaccgcaacggtatacctgcggggatcttctgttttggcaaggtcgttcaactgccgggtgagtacggccacatgctcgtcgggtgttttggaatacacttcattgtgcatgccccacacgtaaatggaaggatgattgaagttttgccggatcagctccgtcagttgctgcctggcattttcactttccttgccggagaagttatttacaaaagggatctctgcccagatcacaaaacccatgctgtcgcattgcgaatacaggtattcagactgctggtagtgcgcaaagcggatcgtggtagcgcctatttcccggatcaggttcaagtctgctttatgctgcgcattggtgagcgcattgccgcagtcctgccattcctggtgacgggtaacgccgtgcattgcataaggctgtccgttcaggaagcagcccttgccggcggttacttcaaagcggcgtaagcccagcggctgtgtaaccgcatcggtaatgcgcccgttgataagaatggaagtggtgagggaatagagatacggatcttttaacccgttccacaaatgcggccttatcaccggtagctcctggcggatgatattaatgccctgcgggctcaggtttgtctctttaaccgtaacggctacacgttttccgtgctggtcgcggatctctgtttgtagctgtacgttagtatgatgtggttgtttgttctcaatttttgcagtaacacccactatcgcttttttatcgctcacgttatcctgggtaatatagatgccgggagaagcgtagtcggtagtggtgatgttgatgtcattggtgatcagcaaatttaccggccggtaaattcccccgaaaataccaaacaggaaattgttgatgggcagtacatcttcccgtgccgtgttgttggcttttactacaatagtattctctgcttcatagtttaccgaatgggtgatttcaaagcagaaggcagcgtaagagcctttgtgctcgccaatgaagcggttgttcacatatagttgcgctaccgagcctacgccttcgaatcgcaggaataatctttttcctttcagggcggcggctaccgggaaagttttctgataacacgcttcacctgcataaaaattctttccttcctgcatgtctttgttgttccaggtatgcggaatggtaatcgcttcccacgtggtatcagtgctggcatttaatggtcctttcctgaaagtccagccatcattgaagggaattacttttcttccttcctgcgcgtacccctgtaaaaacaggagtacgtggaggaaagtgatgatacaatatttagtcatgtgccggattatttcgtatagcctgtgttctgtgtcagcacggcgtctttgttcacatcaatttcagattgcgggatgggcaggtgaatgttatagtcgctgatggtaggcgctactttagggttgtatttcttcacgcgttccaccagtttctttgttcttaccagggtaagcctgcggagttcttctgcggtgagttcgcgggctctttcatcgaggagatagtcgaggtttacttcgccggccagtacttctttggcgtgggcgcggctgcggattacgttgatgctggcggcggcatcgccggggcggccctgttgcagctgcgcttctgcgagcaggaggtaggtttccccgaggcgcatctggatgcggtctttgtacgactgtgctccctgcagatcctgcggctggaactcataccacttggtggtatgggcatagatattctgtatggtatcaaacccgctcacaattaccggctgaccatatttcggggaagccggatcgttataatagtagttgcgacggatgttgtacggggaattacgcatatcgtctttatcgtacagttcataagtccaccagttggtaggcctgatcctgccgataccacggcctcccagcgaatcacagatcttcatgccggctacgtttacatagaaaggcccccactcgcgccggcgctgatcaaagtcggatccgccgccggttacattgtagttctgctctattacccagatggcttctgtattgccctgactgcggcgcatgttgccataggtgaacatgtcggcaaacggatcgccgggttgcaatgctttggcgccgtagcgtgcggtgatgagcgtaaagaatttactgtcgatgatccttttggcagcagcttctgcatccgcgggtttgttggcgcgcagcaacgcttctgtaagtaattgagctgccgcaaatttattgatcctgccctgtttgatcacatgcgcagggtctggcaggttggcttctgcaaaagtaagatccgcgatgatctggttgatcacatcagcttcttttgcccgcgtgtaatccgtgcgtggcacggttacaggggcaacgatcagtggcacatctccaaaaagtatggaaagatggttgtaagcataagcacggaaaaaactggcttctgccttgtaaaatttcctttgttcatcggtgagctgtgcggaagggttatccgatgccgcaatgatcacgttggcgctgttgatcagcttatatccccagttccagatcgagcttaatgaaccggtttgtgaattgaggttctggtaattttcatacggcgcctgcacggtgttgggctgaccggtaatagccatatcagtgcccacgtaaaaggtggcaagtaatccctgcgtgttgccgtaatcgttacgcataatgctcagcataccggtgctggcggcttcaaagcccagctggtccaccagcgtgttatccggtgcataactggatttcagctcctcgtcaagaaagcttttgccgcaggaagatacggttagcagcgacatccccgccagcacaaatctgtatatatatttagcgtgtttcattgtttatctctttaaaattataaactgatatttacacccatgatcaccgtggtattcaacggatagaagtccgagctttgctgccctgcaccttgtccgttgttcaaacgggtagggttggacgtaacggaagatggcgaggtttccggatcatagccctgccatttggtaaacgtgccaagatttcttccgctgacatataccgtgaggttggaaatcttataccgctgcaaagtgctcttatcgaaattgtagctgagcgttacgtcttttatacggataaaggatgcatcctgcgcatatttataccctttcggattggtgtaaaacaacgccgggttggtattgatcttgttttcagaggtccagtagggaatttctgcgggcaggttaataatccctgcctggtccctgttatcgaggatgttgttggcacgaagggaaccatgcacatcctggatgaaaatgttcaggatgaaatttttgtaggtaaaggtgttggtaagtcctgcaatatattttggtaattgtgtaccaagataggagcggtctgccgcatcaatctttccgctgttatctatgtcagcaaatttgatataccctggtttggcgcccggatctattttggcgtcttctccttcctgccagataccggtcatagtgtaatcatagatccccagcatgggtttaccgataaacaggttattcccgatatcatctttattatcgccgtaaagggctaccactttatttttattaaaagagatattaaagccggtattccagctaaagtcgcccgactggatattgcggctgttcagcatcacttccagtcctttattggcggtttctccgatgttatcgtatacagaagtataaccattgatggacggaattttcctgctgagcaacaggtcggaggtacgggtgctgtatccctcgatactgccgctgaggcgattgttccagagggcaaaatcgatacctacgtttaatcccgcggtggtttcccatttcaggcggctgttgcccagtgtatccgggatcacgccaatggaagtaacgccgtcataaatatagttgacggtgctgagcctcgacagcgtacggtaggcgcctatcgcctggttgcccgacttgccataggacgcccgtaacttcagctgggagatcaccggtgctgccgccatgaacttttcgttgtggatattccatcctgcagccacggaagggaataccgcgtatttattactggcgccaaaccccgagtagccatcgcggcggatagtggcggtgagcaggtagcggctgtcgtagttgtagttggcgcggaacatctgcgacaacagcgtgctcgcgctgtagccggtggtagtttgctgtacctgtgcagccttcatgttattgaagtccaggttatcattgataaaggtattggcatccagttgtgaaaagaactgttcatcctgctgcgcgctataaagtgcggtaaagtccagtgcgtgcttattccgtgtgatggcataggagagcaggttttccacgatccattgtttactttccgtattgtctacgctggcacttcctttcagatcgcccattttccggccggtgtaatcgcccgtgcgggaaggccggaatgcataagacgcattaactcggtattttagtcctttcaggaaggtgggggctacttctgcataaccgctggcagtcatgtttttgccgcggtttattcccgggttgtacaggttgatcagcggattcagatacagtgtttgcggcgcaatgggatatacttcatagtcgccggctgcattgtataatgagccatatggactaagggcgttggcctcatacatcgtcactttgccgccgtcctcgttattatttacaaggaacaggtttacgcctgttttcagccaggaggttacattggcatcgaggttggcccggatgctggaacggttgtactggaagcctttcaggttcccctgttctttcaggtaagtaccggagatatagtatttcacatgatcggtaccaccggaaatgcttagttcatggctgtggatataaccctgttgggcgatttctttgagccagtctgtttccggtgcgccgttggcataattcgtttgttctgttaggtaaggcagatccggcgcatcggggcggcctgcctggatattgtaccagtgatttttggtgcggtattcttccccgttcatttgttttacggtattgctctggtattccggtccggcgtagccattgtaggaaatcaccggcttgcccgttttacctttcttggtggtgatcatgatgacgccgttagcgcccctggcgccgtagatggcagaggcagatacatctttcagaatgtcaacagactccacatcattgggattgatgtcgttgtaactgccgctgaatggaatgccatccagtacaatgagcggtgcattgctggcgttgatggacttaagcccgcgcaggtaaaaagcaggcgagctgcctggcttgctgctgttactgataatgttcacgccgggagtggtgccctggatggattgcaatacattggtgaccggcaggtttttcaaccgttcctttggcacggaggataccgaaccagtgacatcacttcttttttgcgtaccgtatcccaccaccactacttcgttttgttgttctacagaagctttcagcacaatattaaaaatgccgctgccggttacgcttatttcctgcgggatcataccgaggtaggagaattgcagcaccagcggtccctctgtagtgatatgaagggaataactgccatcggcgccggtacttacgccctgcgtggcgccttttacccttactgatacaccgggtaagggattgcccgcttcgtcggttactttacctttcacatctgtggccggagcggcgctggtattgttttcatggccaccggcagatttgggtgaaatgaaaatggatttattttcaatcacgtatttcagtggctgatctttcagcatgaggtcgaggaattcccggatggatacattttccaccttcatggttaccgggttggctttgtccagcacgtctttgctggccactacggtgtagccggactggacacggatcacggagaatattttttccacgcgcacatttttccctgaccaggtgatcagctgcgcgtatcccgtagcgcttacattcagaaaaacgacggtaagtaataaaaacgtcagtttcataactaacagcattttggttggaaaccagttccgggtatgcgcttttcctgattttggcgcataggggaaccggttacaaagagcatttttttgcatagctttgtaatgattaggcttgtaaatagatagatgtacggaattactcaattgttttgcatagctgtaatcttgttgccgggggtgggtcgaatcacctccggttttttattacgctaacttcattggctgatcgctgaaattttgttcactgttttcctataactgtttctgttttgatgattagcttatttattttcctataattaaagtcctgttttcgaggcggaagtgtacgcctgattccttcaggaagttcagtacacttgaaagatttacatcactaccaatttcccctacaaaagtgatatcgggaggagtcgtttcatatactacttcaatgtcgtaccagcgcgcaatcatactgataacggtggtgagctttttatcctggaaattcaggatatcatttttccaggcaatgatggcgagggtatctgcctggttattgagggcggtagcgccggattttttattgatctccagttgctgaccgggcttcagtaaactcgtttgctgctgcacatgtaccctcacagcgccttccaggagggtagtgctgatattattttcgtcggggtatgcatggatattgaaatgagtgcccagcacccggacgctggtttcgttattgagttgtacaatgaagggttgatctttattcgcggttacttcaaagtaggcttcccccgtaagggttacgctgcgggtgttgccggtaaaggcggtggggtagctgatagcgctggctgcgttgagccatacgttggtgccatcgggaaggcgcagcctgaatttgcggccacggggcgtggtcatggtattctgacttacttcgccggtgccggcggcatcataggagagctggccgttgctgagtattacgcgtgtgccctgttgtgtggttacggtgccgttgcccaggctgtccagtactacttcgctgccgtcggccagcgtgagcactgcgccgtttttgccgggttttacatcggcggtggcaactatgggaacggtgcttttacgggatgtccgctgccaggtaaagtagccggcggcgactaccagtaaagcaacagcggctgccgcagcataacgcatgattaccgggcgcctgcttcttacaggtggatcctgttgcaggatactgttcacctgttgttcatacaaagcaggattataggccggatcggcgggagccgccgcatgcagttcactgatcatgacagtccactcctcttcatccgtgccggtacgaagtgcggcaaacaattcttcctcttccgccgcagtggcagaaccgttgtagtaacgctccaataaaaacctgtagtactcttttgcttccacggtacaaacccttcttttgctgatagacgctgaaatattgttactgtactatgcgtcttaaaaaaaattaaaaaaacttcgacaggagtataatcaacaggataggaagtcgtgtgccggtatgtttttccaggtattcccggatgaatctgcgggctgttaccagctggtttttgaccgtattttcagagatgtccagggcatcggctatttctttgcgcgatttgccttcctgggtattcatcataaagacttccctgcgggaggcaggtaatttttctatggcatgccggatcagtacctgtaattcttttgcataaatatctgcaggtacgtctgcattatccggcatatcatcggcgatatcatcctgccggtgcttttcacgggcatgttttctaagcgcggaaagggagtagttggccgccagggtatacatccacccacccggattttcgatgctttccagggtatgacgcaccatccaaactttaaggaatacttcctgtaatacttcctccgatgccatgccggacctgagcaacttctttacagaccccgccagtactgcattatagcggtggtataataaacggaaagctgcttcatctccacctgcaattctcgaaaaaagtatcctgtcctcagataaactcacagcgtgatccggattttgtggcaaaatgataagctatggtcaatattatactatttaggggtttcctgcaagcgctttctttgctgcctacctattttcttccccggaaatcataaatttacagcatgagtcaacatccgcgttttacagaaatggcctccgcggctatccatgcagcccaatccgatatggccgaacatgcccacctggtaccggttttcgctaccgctacctttacattcgataatgcacaacagggcatggaccgttttaaaggtaccgcccccggctatatttattcccggtttggcaatcccactgtaacagtagcagaaaagctgatcgccgccctggaagcttttggcgttactacggcagatggtgagcccctgcaattgaaagcattgctgcacgccagcggacaatccgctatggccagcatgttcctgtcaaatgtagtagcgggaaataccatactcacgcattactcgctctatggaggcacacacgagttcttattcgacttcctcccgcaattcggtgtaaaagcgctcattgccgatctgcatgacacagccgccgtagctgccctgctgcagcaggacccgtctataaaaatgatccatattgaatcgcccgccaatccatccatgcgctgtgtggatattgcagccatctgcaaaatagccggcacgcacggcgtaaaagtaagtgtggataatacctttgctacgccttatcttcagcagccattccggtatggggccgactttgtttttcattccaccaccaaattcctgaacggtcatggtaccgctattggcggtgtgctcatcggaaaagatattcccctgatgcaaacgaaagtcaataaaacagcgaaattgctcggtggctgcgccaatccgttcgatacctttttactgatccagggcatcaaaacactggaactgcgcatgaagcaacattgcagcaatgcgcaaacggtcgcggaatttctgcatgcgcatcctgccgtagcgcaggtcaattataacgggcttccttcccatccggattatgcgctgtcggccaaacaaatgcgtcatcccggtgcggtgatgagctttgaactgaaagatggatttgacgccgccgtacgttttattgaccggctgcagatgtgtttgcgcgctgtatcattgggtgccgtggatacattggtatctcacccggcatctatgacgcattcaggaatgaaaaaagaggaccgtgagaaagcggggatttctgatggtttgatccgaattagtgttgggctggaaagtgtaggggatattgtagcggatctgaagcaggcattggaagggtaataatttttttattaaaatttatagcaagagaagacagaagttggagccttttttttgtaaatttgtgaatgccccgacaatcaaaatatcacatagggatcgaagtcgataaactgaccaacagtatcttaaatactatttccggagacagttttgagaccgttgtgaatccacttgcaaaggaggatttaaaaggggtatcattaaagaatggatggaaattcgattggaaaaaggagtttaaaatgaccgatagagaagtttataaacttactatcgaaggaaatagtcacatattacaaggattagcaagtttgagcgattataccgatcatttttatctccatcttattgaaagtgcgccttttaatttaggaagtgcaaagttatacgaaggtgtgccgggtaacctatttgcttttgcctgtcaattatctatagaccgtggatacgaaggatttatatctttcacatccaaaacaaaactcatttcgcattacgaaaaaacgttgggtgcggtgcatattggtaatcataaaatgattatctttccagacgcagctttaaagctggttattaaatattttaacaataaataacatgggatacattaaagaaccaaagggtattaattttgtcgtggatcctaggcctgttacagaaaatgataagaaattgatcagtgaagtaatttctcattataaggcaacaggaaagaagaaacgggttgtatcaggcaagcctgcgagcaaacaaaaggatagtaaaaagctattccattaggagttttttgtcatctacaccgccagcaccagcgacaacaaatacaccaaccctacagacaccaaccccattaccacggtacccgtgctatacacccgcagcatatcttttatctccaatccggagaatttagagatcacccagaagtaagcgtcattggtgtgtgaaatcatcatggaccctgcacccattgccagcacacaaaggatgcggccattagccgaatccagtcccattaccggcagcagcggttgcacaatggcggccgcggcaatcacggctacggtagacgacccctgcgcggttttcaggagcgccgtgatgaggaaaggaagaaataatcccagcgcagcgatggactggttctgcgcaatatggctgccaatatctgcttttgcgaggatggcgccaaaggcgccgccaccgccaataatcaccagtatgcctgctgctttttcagcgccttcctgcaggatagcgcccatattatttttcagttgggataacgccagcaggatacctgcgctgatcgccacttcaggaataccaagaatagagatcgcctttagcgccggggaaggatgtgttaattccaggccgctcagggaacggatggcaatgagcagtaccggaacagcgataggcagcacagacattagcacagaaggaccacggggcgtttcggtagcaatgtcttcttcattactaacgccaacggctatccgccggccggcgaataccgaccataaataacctgccgccgataccgggatggcaatgagtaatccaaacagcattaccctgcccgtttccgcctgtatagtgccggtggcggcagtgataccggggtgcggcggcatcaggcaatgaacggcatacaggccggtggccagtgaagatgccatcacaatcatcggaatccccgaacgtttggccagcgctttatttaatccgcttaatactataaatcccgagtcgcagaaaataggcatgcccaccaggtagccgatgatattcatcgccagtgcagagcggccggtgccggtacggcgtaacacatagttggccagcacagtagtgctgccggtatgttccaggatcaaacccagcgtagtgccgagcacaatgagcaatcccagtgagccaataatattacccatgccgcttttaatactgccgaggatatccgttacgggcaactgtaaaatcacgccggtgagaacactggccagcagcaatgcaaaaaaagcatgcacccggaagcgcgccgtgagcaatacaatgagcgcaatacccgccagcaatcccagcatgctttgtatcaaaggaatggtattcatatctctccaagataaaaagaattacgcaataccccgtataggtgttaccgtggcagcaccagcgggttataacattaacgcatatatgtttttgtaaatattacagattattaatgcaacagcttgataataactattttacctacctttgcaccttaatacagcggatatgaaaagaatgttattgacctcacgttattgcctgctggcaatagtgaccattgttttaatggcttcgtgtgcatcttcccggaaaagcagcagccagcatgcctatatgaacaagcagtatgaagagctgaaaaacacgttgaatgatgcggaagtaagtatcatcaaagacagcctgaaagtgatcttccccaacaacgtactgttttcatcgtcttccgaccaggtgaacgaaagcgtaaagcctaccttcaaacattttgcagaagtactaaacaaatacaataaaacaaagatcctgatcaccggtcatacggataataccggcgcggcggaatacaaccgtgatttgtctgaacgccgtgcaacaggcgccaaacaattactcaatagttttgaagtgagcaacgaccgtatgtttacctggggattgtctgaccgtgatcctgttgccaccaacgatacagaagccggaaaggcaagaaacaggagagtggagtttgtaattttgtatgatgtaaagaattgatttttttataaagatagtcagccgctccgtcgcccggagcggctttttttttgatatgatttcctggataaattttgtattattaaggaatcaatgaaacccaaatctcccgtcatgaatactcgtcgtgattttatacagaaaattgccgcctccgctatggtactgcccctgatgccgcttgccggttgggcaaaagatctccaacactatgatggcccggtattacgtgtagccattatgggattgggcagctatggcaaccgggtggcagaagccatgcaggcatgcgtaaaggcaaaactggtaggcgtggtcagcggcacccccgctaaaataaaagactggcagagctggttctccatccccgacaagaattgttataattacgaaaatttcgaccgcataaaagataacaaagacatcgacgcggtatatatcaccacacccaatgcactgcatcacgaccaggccatccgcctggctgcagcaggtaaacatgtgatctgcgaaaagccaatggcgctgaatgccaaacagggtcaggaaatgatcgccgcctgtaaaaaagcaaacgtaaagctgctggtgggatatcgcatgcattttgaagccaaaacactggaagttatccgcatgcgtaaaaacggcgacttcggaaaaatcatgttcttccaggggcaatgcggtttccgtattggcgaccccacgcagtggcgccttaataaagaactggccggcggcggttccttaatggatataggcatctatgctatcaacggctcccgctatatgactggcgaagaccctatatgggtaacagcccaggaaaccaaaaccgacccggtgaaatttaaagaaggcgtggacgaaaccatccagttccagctgggcttccccagtggcgccgtggcgtcgtgcctgtctacttacaacatgaactacctcgaccgcttttacctcaccggcgaaaaaggatttgcagagatgcagccttccaccggctacggccccatccgcgggcgcaccaataaaggagaacttacccagccacacgttacccatcaaaccgtgcaaatggaagaaatggcagggatcatcctggaaggaaaacaaccggtggtagctgtggatggagaagaggccctgaaagacctgaaaattattgacgccatctatcacgccgttaaaaccggacagaaagtagaccttaaactgtcataaccccaaacgatctgccgaggaaatatcccgcgtgatagtgaaaaacagcaggatcatctattagtggtccgggcgcagcaattcgcatctgatcaattcgtttctttatgctaaaatcatcagctatgaaaaaacgattactgtcagtattgttgctggtttgccttgctgccgcggccagcgcacaaggactgcattacggcatcaaggcagacctgaacatgtttaaactggatggggcaggcattaaatcaaattatacactgggcggaagattaggcgtatacgccgaatatgattttacaaaaaaatgggggctgcaaccggaactcctgttctcgcaggtgggacccaaacgtgacgatgatttcggtgcaaaatatatttctgccggcaacgacaacgccaataaaagcattaaactcagctatattaccctgcccctgttattgcgttacaacgtgaataagttaattactatcaacgccggaccgcaatacagctacctgttttatgccaatgaaaacctccttaactacaaccgtaatgcttttaaacgcagtgatctgggagtggctgccggcgccacattgaacttcgacatactgcacgtatacgcacgctatgtactcggccttacgaatgtaaatgacattgatgaccgctaccagtggaaaacacgccaggtacaaatcggcattggcgtgaatattaagtaaacagccttacgcctttactacggtatcgtatatacgttgtaactggtgtatatgtctttgcgtatgaatattgatgaactgtatccactccagccgggtaaaaggtccgaagccaggcacttcaaagtcggtgcattcttctgtaaggttaacggtattggcggcagtggttaatttatgccaggcggcagcggtatcttccagtacagcttctttcggcatataaccttcttccggtacaatcatgtccggcgacttcattttaatatcgaagttcaggaacagtgattttacggcgggtattttttcatccggttgacggtcggtaggtaccgcctcgccatacaagatgccgcagtcgccggctttgcaaatatgcgatgccacctgcgcggctgtccagctgccttcaaaaggtaccttgttcagttgttcgtcatcaaaggacgtaagcagttgttgcagggtatcgccggtgttggttacttcgcggagcagttcttgtctcatgattttctttttcacaaacttaggtggatatatcggtatataacgggtgtgaaaacgacaatcaggcgggcaaaaaaggacaataaacagctgcagttatttcactacctgcagctgttccctgcattatattttttggaatgaaaatattatttcctggaagatcccagttttctttcagcagattctactgtttgggcaatcagttttgcgatagtcataggtccaacgccacccggtaccggcgtgtaggcggccacccggtttgctaatggccccagttctatatcgccgatgccgcctttgtgataaccggcatctattacaacggcatcatcttttatccattccgcttttataaattcaggtttacccactgcgcctactataatgtctgcctgttggataagctcccgtaaattattggtccgcgaatgacaaatagttaccgtggcattttcattcagcagcatcatagctaccggtttgccgaggataggactccggcccactactactgcatgcttaccggcaacaggtacctggtaatgcttcagcaactccataattcccgcaggggtggcactgccataagcgggttcgttcatcgacatacggccaaagcccaggcaggtaaccccatctacatctttatcgatatgtattttatcgaaacacgcccgctcatcgatctgtgacggaaccgggtgctgcaacaggatgccgcagatctggtcgtcgttattcagctttttgatggtatccagcaattccttggtagtggtttctttgggcaggtgtacttttacagaggtcatgcccacccgctcacacgcattccctttcattttcacatatacttccgaagaaggatcatcgcccaccaggatggtagccagaacaggcaccacgcccgttttttcaatgatgcgctgcaccctgatctttaattctgcttccatttgtttggataaagcttttccgtcgagtagtattgttgttgctgtcatattttggtgtttatttccgtgtgttgagccagatgtatgtagaagacagcaaagatactaaccacctgcgacataattttttttcgtaagacacattcctgttacctttttttccgtctttataaacataacggtcttttaaagggctgttattgattcacgtatgaaaataaaactcttttctatcctccttgtagctacagggtatctccttccgcttaacagttccgggtttacagcgcctcccagggaggtggacatttgcgtgtacggcggcacctctgcaggtgtaatagctgcttatacagcaaagcagttgcataaaacagtactgctcgtatcaccggacaaacacctgggcggccttacctccggcggtttgggatataccgacatcggtaataagtatgctatcaccgggttatcgcgcgacttctaccgccggatcggcaaccactacggaaaactggaacagtggatctttgaaccccatgtggcggaagctactttccagcagtatatcgatgccgccaaagtggaagtgctgtacggatacaccatcagcaacgcagtaaagaaaaacgggtatgttacggaaataaccgtgaacggacccgcggaacaggtggttaaagccaaaatgttcatcgattgctcctatgaaggcgatctgatggccaaagctggcatctcttataccgttggccgggaatccaatgcacaataccacgaaacctacaacggcgttcagctcctcgacaaacaccagttccccgacggcattgatccgtacaagatccccggcaaacccgaaagcggcctgctgtggggcattagtcccgattcgctggccgcccatggcgagggcgacaaaaaggtacaggcctataatttcaggatctgcctgagcaaccgcccggaaaaccgtattccgattaccaaaccggaagattatgatccgtcccgttatgagctgctgatacgcctcctgaatgctaccaaacctgaagccctgaagcccaacctcaagatagatctcatgcccaacgggaaaacggatatcaataattacggcgctttttccacggatatgatcgggatgaactataactacccggaggccgatccggctacccggaaaaagatcatccgcgatcatgagctttataccaaaggactgttatattttataggacacgatgaacggatcgcttcccatctccgggaacaaatgttacaatgggggtacccgaaagatgagtatacggataacggccattggtcgccccagctgtatatacgcgaggccaggcgcatgatcggcggatatgtgatgacacaggccaattgtgaaggccgggaaaaagtaacggatgccgttggtatggcggcctacaatatggattcccataattgtcagcgtattgtagtaaatggtatggtaaaaaatgagggagatgtacagattggcggtcttggcccttacccggtttcttacaggtccatcacacctaaaccggaggacgcgaaaaatgtactggtgccggtttgtttatcagcgtcgcacattgcctatggctccatccgcatggaaccggtatttatggtactggggcaatctgctgccaccgcagcggcggtagccatcgatcagcgcagctccatacaggacgcagacgtaaaaaagatccaaaccatgctgcgtaccaacccgctggtggataacagcccggcggaaatactggtggacgacaatgatgagcaacacgtaaccattaccggcgaatggaaaaaggtgatccatggctgctatggcccttccatgctcacagacgacagcaagggagctgtgcgcaaatcggtacgtttttcaccggctatcgggaaaacgggtaaatatgaggtatttacctatgtgccgcgcctacccggattggatggaaatgcacgggtaaaggtatacgatggccgtacggtaaaggaagtggaaattgcagcggcaagtataaaagtagagggacaaaccagcggcgaatgggtgagcctgggtagttaccagctgaaagccggaaccggcgcctatgtggaaatagacaaccacaaaacggacgggataatagctgcggatgcagtattatttatcccgagataattattttggaaaaaatagaacaggaaggattcggtttacattttttatcgtctttataattacaggtagttccgcgaaatgattattttgtaataaattccatgaccttccttgccgaaagatagtccacataatgaaaaagagctgttgctgcgtgtggcagcgggggatcagcccgccttccagcggttatttgaccggtactgggggaagatgtatgccaacaccctgcaatttgttaagtcgcctgccgtggcagaagacctgacacaggaaatttttataaaaatatggatgaaccgggaacgcctgctggcagtacagcgtttcgatgccttcctgtatacgatggcaaaaaacctgatcctggatgagttcaggaaaagggtattgcccacggtgcaggaagaaggacaccatgtgtacatggcatcggaccagccgtctgcccaggataaactggaactgaaggattttgaaggccagttgcatgctgccattaaccagctgccggcgcaaatgcaactggccttccgcctgagccgcttccagggattgtcgcacgatgaaatagcccggcagatgaatatttccagggtcacttccaaaaattatattgcacggtccattgccgccatccggaagtatatgggtgggagagcggagcatgttacatgagcatggaaacaggtgataacgttgccggttaaacgaagtgaaatattttccggtaacagaaggattcccgttcgttcttttttcgtctttattatacaacccttcatgagagtgttgtgcttgcatccggttttatgttacacgatgagttaaaagatttattggagaaatacctggacaaccggattacaccggaagaaaccaggcgcctgcaggtattgatgcaggctgaacgtaacgggccggcaatggaagaaatgattgaagccatactggcggaagacaggtatgcggctaacgctcatcctgatctgcaacaggcttttaacaaggtaatggaaactgctgccttgcggcaggcgctgacgcggagagatgatgacgcggaaacaggcaacgatgcgcaaccaccaataaaggaggaagataaccgctatcacatctcccggaaaagtatccgcactttttataaaacaatggccgcggcagcagcagtagcatttatactggcagcgggttacacctggcgctattattacgcaagcccggcaccgttggtatcaagtaaaacagcttcgcccataccggcaggtaataaagctgagctgatcctggcagatggcagcaccattgtactggatgatgcaggaacaggaacagtaggcaaacagggaaacacccgtatcattaaactggacagtggccggctcgcctatcgtggcatgagcagcagcagtggcgccgcccccgaatataataccatccgcacgcctaaaggaggacagtaccaggtagtactgcccgatggcagccaggtatggctgaacgccgcctcttcactgaaattccctgtagtgtttacaggcagcaacagaacagtactcctcaccggggaagcgtattttgaaatcgcacaaaatgtggcaaagccttttgtggttcaaacatccggtatacaggtgaaagtactgggcactcactttaacgtaatggcttacaccgacgaagcacgtgtaaaaacaaccctgctggaaggcgctgtcagcgtaacacaaggcgctgctaccgcaatgatgaaacctggtcagcaggcaagcatcgctgaaaaagaaaaccagtttttaattacccgcccggaaatagaagaggtaatggcctggaaagaaggacagttcaaattccgcaaaacagatatcaccgttatcatgcgacagatagcccggtggtatgatgtggacatcgaatacaagggcgatctttccggtattcagctgtatggcagcatgacccgcaaggaaagtgtaacacagctcctggagctgctggaacaaaccggaagggtgcatttcaccatcaatggaagccgtatcaccgtaatgcccgccactatgaagtaaatcaggagagtactccacgtatgaattatttaaactcaaccagaagatagtatggaactgtttaccattgtccactcccacgggagcaggagccgtatgccggctaaacaacgaacatggcgggtatttaaatttaccgcctggctgctgctggcagcctcacttaccgccagcgctcaaaccgtaaagctctccgtgagtaaaatgccgctggataaagtatttgatcttatcagcaagcaaaccggctaccagtttatctgcgatgaaaaactgctggaagatgcgccgccgctcagcgtgaatatcgccaacaaatcgctggaagaagccctgaagatctgcctgaaagatcttccgcttacctacacgattaaatacggcaccgtcgttatcaaaaaaaacacaccgcccggcggaacgctttccccacaggacggcagctcaccggcaaaaaccattaccggcatcgttacggatagcgccggtgtaggcttacctggcgtaacagtaggcatcaaaggcactacaaaaggcgtgctcacagatgaaaacggaaagttttcactgcccaatgtaacagaccaggacgtactgagtatttccagcatcgggtatctcacaaaacaacaacctgttaagggggagaagttttttcgtataccgctgtccgttacccccgcagcattaacggaagtggtggtagtaggatatagtacccagaaaaaaataaacctcacgggagccgtagccacggtgtccggcgaggtgctggccgcgcggccggtaggacaaaccgccgcagggttgcaaggtaccatgcccggcgttactatcacgcaaggcaacggtaaacccggtggcgatggcggtacggtgcgcgtgcgcggctggggtaccctgaaaaaccccgatccgctggtgctcatcgatggcgtggaaggctctatcaacaacatcgatcctaatgtgatcgcctccgtcagtgtgttgaaagatgcggcatcggcagctatatatggttcgcgtgcggccaacggcgtaatactcgtaaccaccaagagaggcaaaagcaataagctgtccattaactacaacaactacgttggctggcagaaacctaccaatctgcctgcactcaccaacgcgctggattatatgctgctggcgaatgaagcgtataaaaattcgggccgctctccgttgtactccgatgcactgctggaaaaataccggcggcagggaaacggcagctccgattcactgcccaataccgactggcagaaggccgtgttaaccggttccggttttcaacagagccatttcctgacagtgaacggtggtaccgataaagtaaagatgctggtgtccttggggtattttgatcagaaaggattgatggataacaacgaatttaaacgccttaccatccgcagtaataccgatatcattttttcgaagaagttaaacatgcagtttgacctgcagtatatcagcccggtaaccaccgagccggcaacaggcgccgatgtgatctttgcctatatgaataatatttcccccaaccagctggctgtaaacgccaacggtacccgcggggaaggatgggtaggcattaacccggcggcagccgccagcgaagggggcctgaaccgcgtaagcgcgccctggggcagtcttaacacgtccattaactaccagccggtagaatggcttactgcttcctttaatatcgcccccaaatacgtgcaaacctatacgaacaagtttaataaagtagtgcaaacgtatcatcctgatggcactcccagctataagtttccaccggtaagcaccctggacgtttccagtcagcggcagttttataacaacatgcgcggtaccctcacgttccagaaaaaatacggcgtacacgacctgaaagtattgggcggtgtggaacaaaacagctaccgccaggacagattcaccgcgtaccgcgacaactacgttttacccgactatcccatactgaatgccggagcggctaccaatatgaataacggcggcgccggcgaagagtgggcgctgcgttcctttttcggcaggatcaactataactacaaagaaaagtacctgcttgaagtcaatacccgctacgacggatcttcccgttttgcagaaggccgcaaatggggggtattcccttccgcctcagccggatggcgtatttcagaagaagcatttatggcatcgctcaaaccggtggtgaatgaattaaagctccgcgcatcgtggggccggctgggtaaccagaacataggaacctacccgtctgccaccgtagtgaacctcagctcctatacaatgggcggacaaatcataggcgccgccgccctggattctctcgcgaacaaaaatatcacctgggaaagtaccgagatgagcgatataggatttgatgtaaccttgttttcccatctctccataacaggagattattatgtcagcaaaacaaaagatatcctgctgttgctcaatataccactgatcacggggctgacagcaccttaccagaacgcaggaaaagtaagcaacaaaggctgggagcttggcatcaactatgatggcaggatccgcgactttaaatacaacatcggtgtgaacgtatccgatgtgaaaaataaagtagtggatatgcacggtattaaccaatcggctgtaaccgtgagcagggaaggttacccggtgaactcaattttcgggttagaggcagagggatttttccagaatgccgatgatgtagccaaacatgccacacaattcggtaccgttgcgccaggcgatatcaaatataaagatcagaatggcgatggcatcatcaatgaaagtgataaggtaattattggcaacaccattccccgctatacttatggcgttagtttaaacgcatcgtggaaaggctttgacctcagcgcatttctgcagggcgtaggtaaagtagacggcctgatttacggcgccggtatcatgcctttttatgtaagctctgtaggcggtaccgcgcaggaacgcttcaaagattactggacgcccgagcataaagatgccgcctttccgcggctggtatttggcggcaccaacaaccagcagatctccagtttctggatgaagagcgccgcttatctgcgcctgaaaaacttacaactgggatatacgctgccggccaacctggtgaaatccatgcggatcaacagcctgcgggtgtttgtaaatggttccaacctgtttacgtccagtaagttctggccgggctatgatgtggaaacagctgtgggcgtggccgacaactatgccattgtaaaggtctacagttttggtgttaatgtaaatttctaaaaaccgaaatcatgaggaagcgttttacctgttggatgattgtggctgttaccctgctggggatacaggcctgtaataaagattacctggataaagatcctttaaccggcccttccgacgccgcttatttcaataaccaggacgaactgctgctggcagtgaacggactgtataaagggctgaataagcctatggacaaagcctccgacccggcccagctggatgggtttccctcagtgctcctgtttgatgccatcagtgatattggctatgagcggaacaacagcgacctgcaaaaaatagggctgggtaaccacgatgccaacaatacctttacacaaggcatctggacggattactacaaggtgataggacggtgtaattatatactggataatgcggaaagagtacgggccgtgactgatcccttgctgtaccagcgcagtatgggcgaaacccgttttgtaagggcatttatgtaccaacagctgctgtcgatgtttggcggggtgccgttggtaacgcataccctttcattggaaaactcgcaggtgccacgcagcgagaaagcagccatacttaaattcgtgttcgatgagctggacagtgcggcagcattactgccggttacctatccggctaccgataatggccgtgctaccaaaggcgcagcgctcactataaaagcaagggcggcgctgtataacgaacaatggaaaactgctgctgatgccgccaaagcagtgatggatctaaacgtgtacaagctggatgacagctacccgcggttatttagctatgatggaaaaaattcgccggaagtgatcctgtccctgcagtatcagttgccggttatcaactgggtaggaccgtacccgctcctgtgcaggaatgccggcggtgcttccaataaaattccttcacagtcgctggtcgacagctatgagtgtaccgacggactaaccattgatcaatcaccgttgttcaacccgcagaagccttttgaacaccgcgatccgcggcttggcttcacgattgcactcccgggatccatcttttttaattaccagtttgaaacgcataaggacagtctcacgtgctggaactataataccaacccggctacccggatcgtaaaccaggatgccgttaacgcttacgcttctttcagtggttattgctggcgtaagtatgtggatttgaaagataaagacaacacgcgccagtcgaccatgagcgtgatcctcgcacggtatgcggaaatactgctcatgtatgcggaggcaaaaatagaagccaatgagctggatgccaccgtataccaggcgattaacgcggtaaggaaacggccgggagtaaacatgccggacattcccgccggcagcacacaggaagcgcttcgttctgcagtaaggaaagagcggatgcacgaattgtcgatggaaggattccgtttgtttgatatccgccgctggaagattgccgataaagtgatgaaagggccattttatggccgtgtgccgagaggctggcttgctgccgccccgaagatagatgccaatgggatcgccgattacagtgcagtgcccaataaaagcgaaatgagggtgatagaagtgcgcacctttaatgctgcacgggattacctgtggccgatcccttatatagaaacacaaacagatccgttgatcgtacaaaatcccggttattaattccgggagataaatatctggtcacccatgctgctgcccgttgtgtttacagcgggcagcttagtttttaagatctttcggaagcaggccgaatttcttccggaaggcagctgtgaagtgctggggatatttatagcccatcctgtcggccacctcgtttacatacattttttcctccagcagcaatcgcctggcttcctgcattttcaatcctgagatgtagccaaatacggtggtgttaaacagggctttaaagccgtttttcagcttcatctggttaataccggcagtgcgggccagttccagtatggaaagtggttgctcatagtgctgatcgatgtagtatttaatgctgtgaagccgctctgtatcgccgggtgttaatcctgcgggagcgggcgatggctggtccagttgcagcacctgcatcaggaataattccgtggctttggtttccaggtaggtagcctttagcgcgccgctgtatgggctatgttgcatatcgttgatgacgctgtgcatggccggcagcatttgtgcggtaaattccggcgcaggtatattaaaagtgttgtaccggcggaaacgttccataaaacggctttcttccgtgaaaatatgatcaaagaaatcatccgtaacgatcagttcaaagaaggagcgtattttattattggtgggaggaatgaacagatcgtgcgactccggtgattcgcggtataccacgaactgtttttcgcggatggcgtgtgtgctggcggcgccggcatcctgtatcctgaagtgtgatacaatggcctttttgtccggatgaaaagacatcactttggcgtcgtggttgatgtagcttccccagcgtagatctacgccgttaaaagtgatctcttccagttgaatgcgaaacccggaggcatctccaatactcagctgtttttcctgcacgggaggtttatctgcgctatgggttacctggcatctgcggatcataatacttctttttgcgttgatgagagttccttctgcgttatcagccggaatttacgggcggtaactttgggtctgctaaattaaatcattaaaatggaaaacacaccgtaccgcaccgtgtttggtgcaacaggaaaaataggcagggcattgctcggtttcttatcagaggcgcagctgcccactattgcagtaacccgcgacctgggcagggctgaaagcctgccttttgtagaatgggtggccgcggatatgagccggccggaaacgcttcctgccaccatgaaaaacagtgtggcggtttttctggtatctggcatgggggccagcttcatagcggaacaacacaatgtaatcaccgcggcgaaggctgccggggtgaaaagctttgtaaaattatcctctgcggcagccggtaaaagctggcctgcacacattgcgccatcggccatcgggcagtcgcacaggcaagtggaagacttgctgaaagcctccggcctggactggaccatcctgcagccgactggttttatgcagaactggctgggcgagttttcaaaacgggtaaaagaagagcgcagtatttatgaagctaccggcgatggcgggcgggcatacatcgacctgcgggatattgcggaagtggcatttaccgtgctcaaagacccggcaaaacatgccgggcaaacgtatatcctcaccggcgacgaagtccttaattactggcagctcgccgatatcataggaacggtgatccatcagaaagtgacctatgtgccgctcaccctggaggaagcccgggaacggatggaaaagacgggcatgccgcagtggaccattcaaaccctgataacgtatgctgaagtacagcggaatggcgacgccacttatgtgagcaatgatgtgcagcaggtgttgggcaagccggcgcgtaccgccgccgcttttatagcagactatatagaatggttcaaataaatgcccgttaaaggataccgtttacattttttatccccattccccggaaggcattccttccggggaatgtatttcgtgtaaaaatgacaattaatataaaataacaattgaacagtggtttgtttcccgtaaacccttatccatcaaatcttctataataattaaaaaaaatccggaaaaaaaataacgggtcaatagttattaattgtatattagacaattaataattctcacgttccgaaggaacagaaggccgtaggtaaagagaggtttcacgtttatgttaattttccacttatgaatagtgtgcatcttcaacaatatgcagacgatattcttttaaatttgctgaaagaggatagcaaggaagcctttgatgtgatctatatgcgttattgggaacggctgtacttttatctggtaaaggcaatcaaggataccgcggaggcggaagatatcctgcaggaagtatttgtgtccctgtggaaacgccgcagtaacctgcacaatgtagaatcactgtatacctatcttcattcctgtgtacgatatggcggcttccggtacatccgccaggaaatcaaaagaaaccacttccgtaaatcctggggcatactcttcgcggaggccgacgacctttttgaacggcaactggccgccaatgagctttccctgctggtaaaccgtgaaatagataagctgcccctgaaaatgcgggaagtatttctcctcagcagaacagaagatctctctcataaagaaattgcacataagctgaatatctccgataaaacagtaaagaaacagatcagcaatgcattgaaatacctgcacctcaaactgaatgtataattttttcaacttttttttaagtcatctactaccatcccttctttttatacacttctatattaaccacgtgttccatacaaagaaaaacagccgttatgaatgaaactgactttaacacgctgctggaactttacctggaagggaaatgcacgccggaacaaaaagagtggatggagcagtggttcgaccgcctttcagaagaaggaagcggggaggagttgcctgcagataaagaattggtaatgcagcggctgaaagaacgcatcgacagacaaatcaaaagacaaaatttttttaagctcccggtattgctgcgtgtagccgcttctgttattgttattttatcattgggcacatgggcatacctgcattatcacaacacaggcaccgttgcagcacagtatgttacaagatccaccgccagggggcaacagctgaaaataccgcttccggatgggtcaatagtaacattgaatgcaggctccggtatccgttacccggaaaacttccgggagaacagaacggtaacgctgctggaaggagaagcttgttttgacgtaacaactgatcctatgcatccctttactgtttcaagtgcaggcgtacaaacagaagtactgggcaccgcattcaatgtacaggcatacaaagcattgggagaggtaacagttacggttatacgtggtaaggtagcagtggaaacatcttcgcaggaagcgcctttgatggtgctgccggatgaacaggctatcatccatactgccaacgggtcaccacagaaaaggaaagtggacgcggcggccaccaccgggtggctcacagggaaattaatcttccgtaatgaaactttgcagcacgtggccatcctgctggagaatatttatgatgtcaaaatagtttttaaagatgaagctacgaagggaatacgttttacagcaaatttcagttccaccgattcattggaaaaaattcttttcgctattgctaaagccaacaaacttaactggtcagcccggaataaagtagtacaattctaaatcttttcttaaccaaaattctcactcgttatgaagcaattcatttggtgtcatctctatgccatccggaaaacgatgcgcaccggctgtagcatattcctgctcatttcactgggcacacaacttttgtttgcaggcgccttaacagggcaaacagccagggagataaaaatagatgtgcagctggagaaccgctccctgcatgatatcctgacagagatagaaaagaaaagcgggctttcatttgtgtataatgataaactggtagcggaatacaggcagttgtccgtatctgcaaacaggcaaccgctctctgttgtactggacaaagtactgaagaatacgaagcttagttacctgcagaaagataacctgatcattatcgtggaaaaagaaactccgcaccaggaaatcatcaatgatatacccattcagcaaataacgatacagggaaaggtaaccgatgataagaatgaggcactgcccggtgtaagcgtgaaagtgaagaacgggcaaacaggcacttctacagatgtggacggaaaataccgcatcgctgtggaccccggcgccgtactggtgttttcctatgtgggctaccaggatgaagaagcgcaggtgggcaacaggactttgataaatgtagttatgcagggatcgatagcaagtctccgcgaagccgtggttattggttatggcacacagcgcaggggcgatgtaaccagcgccatcgccaccgtgaaggcggccaacttcgtgaaaggcccggtactggatgcgggacagctgttgcagggaaaagtagcaggtttaaccatcgctacacccagcggcaaccccactgatgggtcacaaatattactgcgcggtaacaccaccttattcggcgctaacgccaatcccctcgttatcgttgatggtatccccggcgatctgaaaacagtagcgcctgaagatattgaatcggtggatgtgctgaaagatggttcctctgcagccatctatggcgtaagaggatccaatggcgttatcatcatcaccacaaaaagagccaaaggcaccatcgctaacgccgtggactacagcggctatgctaccacgcaaatgatttccaaaaaactggatatgctcacggcacaggattaccgcgaccagattaaagccggcaccaggctggcttcatgggatgcaggcggctctaccgactggctgaaagaagccacccgtacgccgttttcacaggtacataacctcaccatccgcggcggaaacgctaccaccaactaccttgcatccgccaactaccgcgcgttacagggtatctttaaaaagagtgataacaatactttctccggcaggatcgatgtaaaccacagtatgctggatgataaactgaaactgaatatcggcatcctgaaccaaaccaataattacaaccgtaataataatggtgataacagcttcaacggatggatttaccgccaaacagtcatcaggaatcctaccgaaccggtgcgtaaagaaaacggcgacttctatgaacaaaccggcaactttgattatgaaaatccaatggccttattatatgaaagcgacggggaagccaagaatgtaaattcgcgcatgaatgctacgcttacctaccgccccattaataatttgaagctgtcggccttattctcctacgcgcgttttaactccaacaaaggttatgcagaaacgaagaagcatatctccaatatcaaaagcggcgtgaatggctttgcatcggtggcttcggatttatctatcgatcgccttacagaatggacggccgagtattcccggtcattcaatgcgcatcactttacattattaggcggatatggctaccaggagaatgagtcttccggtaactatgccgataaccaggatttcccgactgatctttttgggtataataatattggtttgggagaaggcatcaagaaccagctggcgaatatcagcagttataaaagagaaacaaacctgatcagtttttttggacgactgaactatagctacgaagaccgttacctgctgatggccagcctgagaagggaaggagccagccagttgtttggtgctaagaacccctggggtaatttctgggcagcatccggtggctggagaatttcaaatgaaaactttatgaaacagcaacggctgtttgacgacctgaaactgcgtgttggatatggtattaccggtaacccgccattggatgggtttttaagccagccattaattggctatggcgactatgtatataccaacggcaaatggtcgcgcatcctggtgccttctaccaatgcgaatccgtttatccgctgggaagagaaagcagaagctaatataggattagactttagtatgctgaaaggccgcatcagcggtaatgtggatgtatataaccggcggatcaaaggattgctgtataattatgaagtacccagtccgcctaatctttaccgcaccactactgcgaacgtaggtaaaatggaaaacaaaggcattgaggtaatgctaaactttatcccggtgaaagcaaaggactttacgtggaatacaagcgtcaacttttctaccaatagcaataaattaatcagcctctccaacgaattataccagaccactacgccttacttcaccactggtgcggcggggattcccatccagacatttaccaacattgtaaccatcggcaaaggtatcggcgatttttacggatataaagtgattgatgtggatgataacggtaaatggatatacgaaggaagagacggtaaaccggtcgcctatgataattttgcccatgcttttgaggacaaaaaagtaatcggtaatggtttgccgaaatattatgccggctggaataataatttctcctacaaacaatttgatctcagtatcactatgcgcggcgctttcgggtaccagatcattaattcgcaaaggatgtatatggagaatccatctatacaaaattataatatcctgaaatcggcttatgatcctgtttttggaaagaaagtactgaatgtaaatgcactggaattcaacagctattatgtggaaaacggcgatttctggaagatagataacattacattgggctacactttgtcacaggtgaaaagcaagtatctcaaaggtgcgcgtttctatgtttcctcgctgaatactttcgttatcacaaagtacaagggcctggaccctgaagtaaacaggttgggactgaaccccggtatggacgaccgcgacaaatacccgtctacccgttcctttaccgttggtgtgaacctgaatttctaatcttccaaaaacacgcatatgaaaatgcttcgtaaaataaatctgctgatggttattgttttactgtcggcgtgcaccaagttaaaagataagccatacaccaccatcatctccacggagttcaatcctactaaagatgatattgccgcgctggtgggcgcaggatactcgcaatggcggtttatattgctggactggaatggcctttggcgggcacaggaagtaactggcgatcagctggtgattccaaagcgcccgtggggatggtttgatgacggggtataccagcgtttgcacaagcacacctggactaccgatgacgatgtggtaaaccaaacctggtcccggacctacgcaggtatcaccaactgcaacaggatcatctaccagattgaatccggcctgatacccatcacagatgaaaaagaagccaccctcgcggaactgaaggtgctccgcgcgtcgtactatgccattctttgcgatttttacgggaatgttcccgtggtaacacagtttgatctgcctgcaggatttctgcctcaacaaagcacgcgtaaggaagtgtatgacttcattgtaaaagacctcaccgataatattcccttgctgagcaaggataacacggtggctacctacggcaagttcaacaaatgggcggcctttacgctgctggctaaaatgtacctgaacgcaggtgtgtataccggtacaccgcagtgggaaaaatgtatcagtgcctgcgacagcgttatgaattcaggcgccgggtatatcctggaaccggcacagaaaaatgtgtttgtaacagagaaccagagttcaaaagaaataatactcgcaattccgatggatgaggattataccaataactggaatgcctttgacctgcacatgcaaacattgcagcaggaaaaccagtcgacctataacctgaagaatacgccatggggtggtatctgcgctattccgcaattcatcagcacctttgatgttgcggatgcccgctatcagaataactggatcaagggccagcagtacaccgccggcggccagatgctgtttgtggcgcagggcgattttgccgggaagccgctgagctttgtgaatgaattaccgggattggaaaagggagagtcggtgcatggtttccgtttaggaaagtttgaaataaagatgggcgccaccaaccggttgagtaacgactatccgctgttccgctacgcagaagtgttgatgatgaaagcggaaagcttgctccgtacgggtaaggccgacgaggcagcagccattgttacccaggtaaggcaacgtgattttgtgggtaatcccgcgaaggcagtggtgactggtgcgcagctgaaaggcggcagttcttaccaatatggtatgaaagacgccgtgaataatcagttcagcaatgaaggcggggcggatctttcattcggccggtttttggatgagctgggctgggagtttgaccaggaaggtcatcgccgcacagatatgatccggtttggcgcatttacgaaaaagtcgtggttgtcgcatgccgctaccaataacattaaccgtacgctattcccgatacccagaacggagatacagaagaataataatctgaaacagaatccggggtattgaggtctattttggttgtataaagatcgcggggatgattagtcatccccgttttttttgacagcaactaataatcgctccttcaaaataaaatttccacaaacgttaggatactatcataaattattttagtttcaatcttgttattttgcttaaacgtgtaagcagaatttaatggtccacggagaaacgatgaaaaacgacacatttaaccagcagagccatagttgattttattgtaaagtgcagcagcggtaccgcttaccggctgtttaaaattttgaacccacatgaaaaaaagtaacaaccggcgtttctttctgaaaaacattgctgttgcctacctgggcgctactactattcctgccatagcgctggcggcaaaggaagaaacgcctccgccgggagaaaaaaaggcgcccggtggccgtcgttttaatgaaacgtacagcggaaagtataataaccgtatagcctttcctgttggaggaataggtgccggcatgttttgcctggaaggtaccggcgctatttcacatatgtcggtacaccataatcccgaaatgttttatgaaccggccatgtttgccgccattagtataaagggcattccagatggagcgagggtacttgaagggagtgtgcccgactggaaaaaattcgggcagcgcgatgccgggttaggcggcaccagcggcgccacctgggggttgccacgtttcaacgaatccacttttaacgcacgcttcccgtttgcggatatccgtctccgtgataacgcattgccgcttcaggtagccataaaaggctggagtccttttacgccaggcgatgaagatcatgccagcatgccttttggcgctctggaataccagtttaccaacaccggcgcgaaaccggaagaatatatcttttcctatcatgcccgcaattttatgcggcagggggatacaggcaatagtgtaaaggccatgccgcaagggtttgttttatcgcaggaggcagttccggatgcacccgaaaagaaaggccaattcgccatctttactacggagccgtctactattgtggatcattgctggttccggggcggttggttcgatcccttaacaatgtcatggaataccgtaaaagcaggcgaaacacgtaacacagcacctgtagagaaagacgcacccggaggatctttgtatgtgcctttccgtttgcaacccggtgagaaaaaagtgatccgtttgatgatgacctggtatgtaccggattcaaaacttcatattggtgatagtccgggtggcggcactcccgctaccggcaaatattaccggccctggtacagcagcaggtttaaagatgtggcagaagcagccgattactggtccggccactatgatgaactgtacaggcaaacatctctttttacaaataccttttataaaagcactttaccgcccgaagtgctggaagcagtagccgccaacctcaccatcctgaaatccgctaccgtgatgcggcagtatgatggccgcttctggtgctgggaaggctcgggcgacagctggggaagttgccacggcacgtgcacgcatgtatggaattatgcacaggcagtaccacacctgtttccagcattggaaagaagtttacgccataccgagtttcatgaaaatcaaaatacggatggacaccagggcttccgtgcaaatatccccatttcgccattggtgcataacttccattcagctgccgatggccagctgggaggaattatgaaaatgtaccgcgactggcgtatcagcggggataacgactggctgaggaaaatgttcccgctggtgaaagtgagcatggattattgtatccgcacctgggatccgaaaagaaaaggtattgtggaagagccgcatcataatacttatgacattgaattctggggccctaccggcatgtgtacgagtttctatctgggggcactcacggcgttcactgcaatgggcgcctttcttggcgaagatgttagcgcctacaaaacgctttatgcaaaaggaaagcaatacctggaaacggagttatacaacggcgaatattttatacagcaaataaaatggaccgacctgcaggcgcccgatccggtaaaagcgcagtcgtttagcacccagtactcgccggaagcattggccctgctgaaaaaggaaggacccaaatatcaatatggtacaggatgcctctcagatggcgtgctgggttcctggattgcacgcgtatgcggcctgccagaacccgttgatcctgccaaaacaaaaaaccacttactggccgtacataaatacaatcttaaaaaagacctgcaacaacatgaaaacccgcaacgctctacttatgcactggggcatgaaggcggactgctgctatgctcctggccaaagggcggcatgttgtcgctgccgtttgtgtacagcaatgaagtatggaccggcatcgaataccaggtggcttcccacctgatgttccagggtgaagtggaaaagggacttgatattgtacgtgcctgccgtcaacgttatgatggtaccgtcaggaatcctttcaatgaatatgaatgcgggcactggtacgcccgggcaatgtcgagctacggcttactgcagggactcaccggcgtacggtacgacgcggtagataaagccatccatatcgattcaaagatcggcgacttcagcagcttcctggccaccgacaaaggttttggcactgtgagctggaagaaaggtgtaccttccttaactgtggcctatggtactattccggccatacacgcgatagttgggggaaaaacgatcccgctgcaacaatccgccgtttaaataataacagatgaacatttaccgctgcctggtttttagtataatcgttgccgttagcactgcatctgcgcagcaaccagcgtcggaaccgcaatggatcagacctgataatgccgccagtccaccggtgtgggggatacgcaatggcattgtaatcgggctgtggccagctgcgatagaaggcgcgcggcccggcaatgatggcggcccccggggactgctgcgcatcgggtatgaatggaaaggcatcgtgtaccatcttaactacatcgctatagagccggtggtgaatggtaaaattgagttcagtgaaatctccccttcacgggtagacgggaagtggggcaagttgatgtggaccggcgaaaccaacgatccaggccggtttacggctgctgccggtacccgtggcgtgctttcacatcctgatccgcagcatccggaatatactaccctcagcttatatgttttcatggaagcatttgaaaacggcgcccggccttacctccgtttgagcatcagcagcaaccggccggaagaactatgtatagaagtattccaccagccaggtggcacgcccatggagcgatgtggcatcaccgctaccatgggcaattatgcacgattgaggaaattacacctgaaggataaagtcgtgtatgcgaaaacgttatatgacgggtatgatggcaccgggttcgtggaaaaagcaccgtaccccgtacagcagctgttgcgtaataaaagcggggactacctggtaatggcgcaacccgacgaatcattaaaggagctggccgcctggccggaggatgaacaacacgccgcccgctggggctggcggtaccgccctttttatacacttacccaatactggcgcaaagaagccagtgaggccgatagttcactacaggtaagggtaaacgggcgggcgaaatattggagcggtggaagcaccgatccgaacgcatacatcaatatccccggtggtccatctttcgaaaactttgaattacgggaaaaatataatgccggtcagaaagtatattttggactgacccgtaaacccattagtgaattgctggaacagtaaccggcgccgctcgtcttaacgcataataacccaccaccgcaaaacaaatcaacggtatagtatatgccagctgcacgttgctgtaaaaactcactgcgcccaaggccagtggtatcaacgcgccacctacgatagacattaccaggaaagcagacgctgatttcgtttcgttaccaagatctttaatcgccagtgaaaaaatagtaggaaacataatagacataaagaattccaccgctagtaaaaagtaaacgcccgttctaccgccaacggctacactgtaacacaacaataatacgcacgcaatgctgtatagcagcaataatcgttgcggtgctattttccgcatgaataatgtacccgcatacctgcccgtcataaagcaaagcaataataatcccaaataggtagtcgcctctttctcctgcatatgaccactataacctgcatagcggataaagaaactggagatacaaacctgcgcacctacatatgcgaactgtgcgatcaccccccaccggaaatgaacatgcctgaatacacgcaggttaatactcaatccgccactatgctcttcatgtatttttgggaatcgtactaaccggaacagtaacgctgtaaacagcaacacgcctgcaattgccaggtagggaacctgaacggaacgtgcttcggtaagcaggtattgattcaatgcttcgggcgacatgctgctgctttgcgcagccgtgagctcctttcccgaaaggatcactttactcaggaaaaaagccgctacaaaagcgcccagaccattaaaagcctgcgcaaaattgagtcgctgcaccgctgtttcgggtgtgcccataatggtgatatatggattggcagcggtttccaggaaggtcatgccggcggctaccaggaacagggcaaagaggaataaaccaaatgaacgcagttctgcggcggggaaaaacagcacagcccccgcagcggcaatgagcaaacccgtgatgataccggttttgtaactccatttgcgcatcacccaggccgccggcaaagcaaaaaagaaatagctgatccaataggcagcgtcaataaaagccgactggaaatcattcagctggcaggctttccggagatgtggtattaatacaggaatgagattgcccgtgagcgcccataaaaagaagaggctgataataagtacagtagcaagtttcagctgacgcgaagcagtagaagccgcgggcgccttttgttggatggctgcagtggaattcataaagatgttttttaattataagcggtaagtctgtacttcgttcaccagctgtcctatatgatcgatgctgatctctacccggtcgttgtcctgtaacgtaaaactattgtccggtaccaggcaggtgccggtcatcaggaaagaaccatcagggaaagcgcagccacggtataagaaatccaccagctcctggtgactgcgtttcatctggctgatcggcacgctgtcggaatattgcacttcgttgttccggtaaatagacatgcggatgatagtgtccgggggaaccggtttatcaggcaccatcaggcaagggccaagcccggcgcatttctcgtatacttttgcctgcggcagatacaaaggattttctccttctatgctgcgcgaactcatgtcgttgccgatggtatagccttcaatagtacctttgctgctgataaataaggtcagttccggctccggtacatcccaggaagagtcttcacggatatacacggtttgcccatgaccggctacacggtgtggcgtagccttgaaaaatagttcaggacgttcggctatatatactttatcataaaaagtggcgccgcctgatatctctgattcttccatacgcgcggtgcggctccggtaataggtaacgccggcggcccatacttcctgtgaaccaataggtggctgcagcgctgttgccagtattttttcggccacggatttttcaacaggcgataatcctttcagatcttctaccacacgctggtataagccttccctgtttacgaattcattccagccggcaataacagtgtagtactgatcctggtaggcgatgagtaaagtagtagtggttttataaatacggatgctattcatttggaattatttgttggtaagaaaatgttgaacgtcttccagtgggagttgccataactgcatagccagcgcctgtaatgctttacggtcgccttcaaagtgcagggtcgtttgccggtaacggagcgattcgcctgccttcagggcccgcgcatcggaggaggactctacttcatagaaggggcccatttgtgtgccgtcggcaaggggaccatcattgtagcaattcactgcatcacctttgaatggttctttctgcaattcccattttgaatttacataacggccctgtggtactacatcataaagcaataccgtgagcgtgttgttttcaaggtcaatactgcctgcgcctcttttagccacgaggggagagaggcccagtttgccacgcgactttccgtctgcgcggaatagcagcaggctgtcttttacctgtaaattctgtggtggtatcttaccgaaataatcatccgtaatatgttgcctggcatcccgccctggtctgaaaggcgccacaatggcggtttgatcggatggtttaaacatgcccagcagccagatgctcagcaatccgttttcttcctgccagctgctgtcgcctttattggtgatggtattgtcggtttcataggctacgctgctaatacctgcaggtaatgcaaatccaatactggaaacgatgtcggcgttgttcagcaaccggatggttctgttgatctgcaattgaaaggtactgcctttataattttgaatcgttccttcctgttgataggtaatactattctccgattgcgcagttaccgtataatgtgccgtatctatcaggccgggcgtttgccagttggcaaagtcgaaaggttttcccgggggaaagaagagtgcatattgtccgccttcagggcccaaccagaagcgttcttcgccgccaaaggcattgatgtgcggcgcgtattgctgcgatgacaccaggttgtagttgatccagccaaagctctttcctttgtcgccgccggtagtgctggtcattacgcgggcctggtagtcgcctgtaaccaccagccggccgctgtcgctgccatttttcaataccacaacattcttcagatgttgttgtaaaaaggatacgtcttcaccaaaatttacgggcttcatatgattgggtgctttcgttggtccggcgccgttacagctaaaaagcgctgcagcaatacaaccggagagaaggatagatttcataacgatggcatttttagcttgataaaatatgaactatagtgatacccctcttttccagggaataaaatcatcctggccgagtacctgtgcttttgtctggtagttgccgctggcggtattgatcaccatgtccataatgcgggcggccacttcatcgatggtttcttctccgctgatgatggtgccggtatcaagatcaatgatatcatgcattttgcgggcaagtatactgttggtagataatttaacgactggtgtaacagggttgccggtaggcgtaccgaggccggtggtgaacagtacgatgttggcgcctgcgcctacttccgctgtagtggattctacatcgctaccaggagtacagagcagggcaagaccgggatgttgtacccaaccgggataatctattacatcggttacaggggaggagcctcctttcttcgccgcacctgccgacttgatggcgtctgtaatgaggccatcgcggatattaccggcagaaggattggagtcgaatccggagcctacggcttccgctctgctggcgtaatcgcgcatcagttgcacatagcgtgcagccatgtccgtagtaacgcaccgatcgctcagttcctgctccacaccgcacagttccgggaattctgaaagtattacggaaccacccagcgctaccactatatcagccactttgccaacagcggggttggcagagataccggaaaatccatcggagccgccgcattccatgccaatgcataatttgctgagtggggccggttgccgctgccagctgttggcatgcgttaacccttcaaaagtttgttgcaatgcctgtgtcatcagctctttttccgaacctacctgttgctgttcgagatggatcaccggtctatcgaagccgggcgaacgtttttcaatttcttctttgaggatactgatctgtgcattctggcatccaaggcttaacaccgtagcgccggctacattgggatgtgtgatgtaacccgccagtaatccgcagagggtacgtgcatcgtctttagtgccgccgcagcccatggtgtgcgagagtaatttaataccatctatattgggaaaggtgcgggtaggcagcgtaagtgtggccgcagcagcggagcgacctggttgtacgccctgccggaaatcctgcagcaattgttgcagcatggattcatagggagagggttcccggtagcccagctctttcaccagcatttcatgcagcagctgtacgttgcggttttcgcagaacaccagtggaataattacccagtagttaccggtgcctacacggccgtcattacggtggtagcccataaaggtgcggttttcccagggagatgtatccggcggtgtccattcggcatgccgctcaccgctcacgctgaactgaccggaagcatggcgtatgttcccggtggtgatgagttccccggcaggaagatcttcattggccagtcctaccagtacgccgtacataatgatgggcgcatctttcgggatatttcccgccgttattttatgcttggcggcaacatcacgtatagccgttacagtttgcccgccattgctcactgcggtgccggcaggaatgttttgcaaggctacccaaacattgtcaccaggatggatttgtaatatgctttgtttcattattgcttgaataaaataatttataccagtgccctgtcgaggtgtacatagccgccatccacatgaataagttgcccggtggtatggctcgattttcccgacaggaggaaggcggtcatttgtgcaatttcttctggggtggtcatgcgtttttcgaggggaatacgttccacgatgctggccagttttgcttctttgtcggggaaggtattgatccagttttcgtataaaggcgtccacgactcagctaccacgatggcgtttacacggatgctgaaaggcaacagttccacggcccattcacgggtaagcgcattgcggccaccgttggcggcagcgtaagcggaagtattaccctgaccggtttctgcggtttttgaagtgatatttacaatggcgccttttgatattttgaggtagggaagtgcatgatgcgccatcaggtaatagtgcacgaggttgcggtgcagtgattgcataaacgcttcgtagtttcctttctccagtccaacgccatcgttgatacctgcattgttcaccagcccgtcgatgcgcccgaattccgcagcaactgcggccacggctttttcgcaggcctgcggatcggtgagttccgctactgcctgtgccccctggccacctgcttcacggatacgttccagttgcaggagattatcggcttcacttctgccgataataacaggggtggcgccttcctgtgccagcactgcgctgatagcggcgccaatgcctttggcgccgccggttacgatgatgatcttatcttttaaacccaggtccatacttattatttagagggatttttttgaaatatcgccattcacctgtcgccatatattcgttggattttcatcctgaagttccggtggcagcaggtaagcggggaagtcctggtaacatacggggcggcagaagcgatagatcgctgcggtgcctacggatgtgcctgcggccggcgtagtagccggccaggggccgccatgtaccatcgcatgactaacggctacgcctgtaggaaatccattgatgatgatcctgccggctttctcccgtaagatatcgatcaaagcagcgtgttgctgcagttcttcttcggtaccgtgaacggtagcggtgagctgaccttccagcttcctggctaccgtgtatatttcttcgatgctgccggcatgaatatgcagggaagaggggccaaatacctcatgacaaagagccgggttttccaatgcctgcgctgcggtaacctgcagcaggctgggggctgcctgttgatcggcaggagtggcttcgcccagtatttgtacgccctgctcacgcagggtggcaataccgttgttatacgccgccaggatccccggtgtgagcatataaccattgggcagtgtgcttataccttgctgcagggcgctgataaaggtatcggtggacccgccggctgcggtgatgaacaaaccgggattggtacaaaactgcccggtgccaagggtaacagattgcaggaactgtgtggccagggcagcgcctttctcccggagtatccccggaagaaaaaataccgggtttacgctgcccatttccgcaaataccgggatgggtactgctcttcgtgtagccgtatcatatagtgcttttcctcctttgaaggagccggtaaaggcgatggcagataccagcggatgagcggccaggtattgccctgtttcatgggaggtgccatgcaccagcgagaatacgccatcgggcatattggtacggagtactgctttacgtatagccgtagcagttaaatgcgaagtatgcggatgtgcaggatgtgctttgaacaccacggtacagccggccgccagtgcggcggtggtatcccctccggccacggaaaatgccagcggaaaattgctggcgccaaagataccggtaacgcctatgggaatctgcatttgccgcaggtccggagcaggcgtggtgatccgcgcatttacccacgagccttccatgatggtagcggcaaacaaccgcagctgaccggtggtgcggtctctttcgccctgcagcctcggcagtggcagcccgctctctgccgacgcaacattgattaattcatctcccagggaaattatttcctccgcaatcgcctcaaggaaagcggccctttgcagcgatgttgtttttttataaacggtgaaagcctgtgcggctaagtttaaagccgaatcaatttcaccggtagtagcttccctgaattcctgcgacagccattgctgctgcgcaggcgcgaatgcccggaaggtttggtcgccttcaccggaaaagttattgcctatcatctgcaatcctgtcaacgaggttctgttcatcttcctgtatttttatgattagtttacttccaggtcgttcattgccggcagtttcggaaacggtgcgtgtggttcacgctggtaccagtacactacgctgctgatatccgattgttgcggaagataacgtccgctgctgcgccagcccagatcctggatggtgatcttcagttctttttcaaaacgtaccgggtccataatgtgccagcggtacaatccaaaccgttgctgtgatttatacaatccatcggggcgtattacctgcgataatccggaataaggtgtgcagaattcctggtagcggcctttcgtgtcgaagttgtaggagccgcagaaataatcttccgtgccggtgccgcaaatagtaggatattgtttatcgccatccataaagaattttatttctccttcgccccaccagccgttgttattaacgccccaggcgatgtaggtgcctacgtactggccttttcccttcacaccatcgatcatggtaaagctggcgtctttcacgggattattgcggcggaactgtgcatggaaatagccggcgtcttcaggcacgttagtaagcgtgtagtcgacctggtagtacaaggtcattctttctgtgttgatattttccatggtgatgcggcacttcttgcggaagggcatagcccagtagcagttgaaggcgctgcctggatttacgcatacggccagtgaattgaggggtgcatattcgccccagcccatcccaaagaaatcgcctaccggcacttctacagaaggcgtggtttcatcgtcccagtaaaaacggaggatagagtagcgccagttgccggtgggtgtcatccatatgtgctggatggcgccggggccgctaatttccgcgagggtaacggttttccccggctcaatatgaatataaggatttactttccatccctggcccagctcttttgctgcgccgcgggcattaccctggtcaagtgtggccatgccgcctttaccgggttcgcccgtaaagttttccgggctgatagaacgggttttggcatcagacaaacggtacagatttcccatgttcatctccaggccattaaagggttgctgggcgctggcggccgtccatgtgaggagcgcaataaaagaaagaagcaataactttttcatcatacgtgaatattaaaagattaggttttacgggtttctgctgaatatagctttatcgtttaagcaatcgggtaaatttttaaagatcactttcgtacgtggtcgcgtgttaccggctgccacaggattttcttaccaccagcgtagtatcaatacaaatcgcggtggtggcagtagtatggtccaggatctgttccagcagcacgcgcactgcggcctttcctatttcaaggatcggttgtctcacaaatgttacgggtgcgtaaaacaaatccagcgcttctccttcatcaaatgtaatcaccgccaggtcatcgggtatgcgtatacccagtgtattaatgtatttcaggccctctatagccaggctgttggtggcaaagaagatcgcatctgccggctgttttcctttcagcagctgatcaattgccagcctgatatcttctttcaaatgcgagtaccttgccttcttcagtaaactattacttgcttttatatcatgttgctgcaacgcatcctggtagccgcctatcctttcgctgatatggtgcagcgtggttttataagccaccatgccaatccgtttgctgcccattttaataagatgcgatactgctgttgcggcggactcacggttattaacggcaatataactggccggaatctccggaaagaaccggtcgatcagcacaaaagggatcttctgctctttcagttgcaggatctgttgctccgatccttcggtaggggtgataataaggccatctacctgccggtttacgagcacattgatcaggtcctgcgacttgtccacgttttcgtccgagctgccaaaaattacgttgtaattgtgcttttgggcctcgtcttcaatagtccgcgcaatattggcaaagaaaggattggagatgtccgccacgatcaggccaatggtaaaagaccggccgcttttaaggctgcgtgcaatatgattgggctgataattcagcttccgcgcaatttcacggatcttcttcgccatctcttccccgatccgggccttcttgtctttgttggtcagcacataagataccagcgcagtggacacacctgcttcggtagcgatatctttcagcgagactttcttcatcttttaaaaatatgcttaaacgtttaagtttgcaagcttttgggtaatttttttttgagagaagaacttttgaccaactccaggtatttgtatttttacccgcaatggtctatttttaagggcatgatacaactggaaacatttactgctgcggactttgaccgttttatatcctggatcgacaatgaagaagcattggtacagtttgcaggcccgttgtttacttacccgttaacccacgggcaactaaccgcctacctggaacaaacccaaaagaaaccttttaagatccggttactggaaaccggtgaggtgattggccattgtgaactgaattttgaaaaggaaatgccccgcttgtcccgcattctgataggcgacaagaacatgcgtaataaaggattgggaaaacaggtggtgaaagaaatggtgaacaggttattcagtactaccgaacatacagcggtggacctgaatgtgttcgactggaaccacaacgctattgcgtgttacacgcagctgggcttccggattaacccggagatggccggtaccacggaggtaggcgggaaaatatggcacacacataatatggtattacaaaaagccgactggcagatgctgtaatatttccctactttagcagttgggccggcatttgccggcagtaataaactgaagccgatcagcatggagaaaccagaccatacttcaccccctttggtgaatgaaaatcttgaaaagcttgccgccctttttccggattgtgtggtggaaggtgccaatggtaaagtggtcgattttgatttgctgaagcaggaaatcagccatgcggttgtagaaggtcccagggaaagataccgcctggactggcccgggaagcgcgctgccatcgtttccgccggtaagccggctacacaggcactgcacccggtaagaacagactccctgcactttgatgaaacggcgaatatctatatcgaaggggataatctcgaagtactgaaattgttgcagccgcactatctcgctaaagtaaaaatgatctacattgatccgccctataataccggtagaaattttgtatacagtgacaattttacacaaggcgacggaaaccatcacgcattgaacagttcaccggatgaatacccggaggcgggcagcagataccacgctaactggctttccatgatgtatccccggctgaaactggccgctgctttgttgcgcgaagacgggatcatttttatttccattgacgacagggaattgcctaatctccgcaggatctgtgatgagatttttggagagataaattttgtgagctgcctgccacgcctcacaaaaaaagccggtaaatccaccagcatgatcgccaggaataacgattatgtgttgtgctaccgcaggtcgccttacgcgcggtttaatactaccgcatttgaagcgcagggatacacccacgctgatgaatatgaaccggaaagaggcaggtataaattaaatcaaacgctggactacagctctatccagtactctgcgtcccttgattatgaaattgaaatagacgggcaggtactaagacctggaaatgtaacccgggaagaaatgctgaaaagacaacagcgtaatccccaaagcgatttttgctggagatggagcaaagggctgtatgaatttggtttaaagcatgggtttgtggtgctgaagcaatcgaggcacggctaccgcatttatacaaaaacatacgagaaggccactatttccaaagcaggcagcgggtatgcggtggaaatgaaagaaagaaccaaagcctttaccagcctcgattttattgataaccggttttcaaacgataatgccaggaaagatatgggcaaattgtttgaagggaagatatttgagtattcaaaaccggtatctctcatcagtgagctcattgcactgtcaacttccgcaggcgatattgtggtggatttcttttccgggtcagcgaccactgcgcatgccgtatattcactggcagcgcacaccgggcagcagcggaaatttatcctggtgcaggagccgcagcttacagctgaagacagcgacgcttatcatgccgggtataaaaatatttgtgaaatagggaaagagcggatacgcagagccggcaaggcaataaaagaggagaccggcgccgtgttcgacgatggctttcgcgtataccggttaggccccctctgagctataattgtattgctgcggaacaatccgctgccacttaaccaccagcggccatccctgccgtttgattttttattccattatatttgatccggtatgtccaattgctgctattccatttgttataaggtatattatcacacttaaaactttaaaaagatggaagaatttatgttgattttcagacacgaagatggcaacaaagtagcctccccggagcaaatccaggtttggatgaaacaaacgatggactggatcggcggcattgccgcacaaaacaaatttgtagaaggaaatggtttaccttttgccgacagcagggtagtgcatcataataacgtggtgactaacgggccgttcggcgaaattaaagaaaccatcggcggctacattattgtaaaagcggcatccgtagaagaagcggtggagttcgcaaaaggcagcccggtattacagggagacggtaatacggtggaagtaaggaaagtggatcgtcactaaaaggtataagcccctgtgcaacaggggctgttttaatgtatggcacaatccgaattaataccacatttgttccgtacagagttccggaaaataacggctgtgctctgtaaggtttttggcatcgaacacctgcaggcggctgaagacattgccagtgaaacgtttttgtcggcaatggaaacctggacctataaaggaattccggagaatccaacggcatggctatacctcgtggcaaaaaataaggcgaagaattattttcagcggaatcacctgtttgcggcaaaaatcgccagccagatcaagtatacttctcctggcagtgaagaacccgacatcgatctgtctgataaaaatattaccgatagccagttgcagatgatattcgctatttgtcatcccggtatttcaaaggaagcgcagatcggccttgcactccgcgtgctctgtgggtttgggattacagaaattgccaacgcctttttaaccaataaggaaattatcaataaacgtttgttccgggcgaaagaaaaactgcgcgaagagaaagtgcagatggagttcccgggggaaacggagatcaaaaaacgcctggataccgtactcaccacgctgtacctgcttttcaatgaaggctattattctgaaagccaggatgcagtattgcgggaagatttctgcctggaggccatgcggctcacttacctcctgctggaaaatgccgctaccaatacgccggaggtaaatgcattgtttgccctgatgtgttttcacgcatcgcggtttgaagcgcggaaaaatgaaaacggtgagattatcctgtaccaggaccaggacgagtcacgctggaatgaagcgctgatcgccaaaggcgcgtggttcctgcatgaagcctccggtggtaaaaagctttcccgttatcatcttgaagcgactattgcttactggaatacaaaaaagcaggatacaccggaaaaatgggagagtatcctgcaactgtataaccgcttgctgcagatctgctattcgccggtggcggcattgaacagaacatatgcattgtcgaaagccaatggaaaggaagcggccatcgcagaagctgaaaaactgcagcttacggataatcactattattttgtgctgctgggagaattgtatacggatattgataacaaccgtgccgttacccatcttcaaaaagctttatcactggctaaaacggaagccgataaacaaaccattcaaaagaagctggcccggttggcagcgatgtaagccggttcaggaaaaaagtatgactacctggtttgccagcctgaaatagaacatacaacaatcagctgctgatacgcagcgcagatgaaaatgcagtggtaatagcggcattatcccttctcaggatggtcgggttcaccatcatacgcgaagcgccataagcctgcggctgacccacaataattcctttctcttcccggagccatttggctgcttttacggtatcaacctgtttatcaaaatgcaggtcaaagatattggttcccctttccctcgccgttatttttataccgctgatgttgttcagctctttaaacagggcttgtgcttttttgatagatgcctgtaatacatcgtcgatgtcctgcaggtgatgcaaggccatggcggcatttccccagttggtgaaaatgccgccgccatgtactttcagcaggtgcggcattttgtcgatcactttcttttcaccgcacaggatagcgccgccctgtgcaccgaggtatttataaaggcagagatataccgtgtcgaagtttttcgtatagtcgattactttattcccggtaaacgcggccgatatatgcaaccgcgcgccatccaggtgtgtttttatgccctgctcccggcaataggcagtgatggcggtgatatcttccaaaggaaaaaaagtattgctgaaccttctcaccggcgtttctatggagagagcgcccaccggggcttcaaacgcttcttctgttttatgccagctgatggcctgcttcagttcctccagcgtaaaagcagcctggtcttttcccagcggaatcagccttttattaaacaccgtttgcgcggcatcggcttcatcacggtaaacgtggctgctttcctgcaccattactttgggatgatcgccggaaagcacctgtaaggccagctggttggccagtgtaccggatggcatgtatatcgccgcctctttgccggtgatttcacagcatttgtccagcaactctttcagtgtgccatctgtaccataaaaatccctggtgataggatgctgttgctggataagttgaagctgttgtatataatctgccggcctgtaaaagataccgtcgttgataaaatatatcctttcgctgtctttgtcaggatccatgttatcaaaatggggtgctgctttggataccagtggcaaagcgcccgccaatgcgctgagggaggctgctttaaggaaatgtctgcgcggaatataggtcataaacagttgtttttacaggaagacataaacctgttcatccggtaaatataacaaacgcagcacgttacttttcattgtgagtaatacttttttatatgccttcggcaggaatgtctgctgtatgcatgtccatattttcaggcagtagccaaagcatccatcctactattgccaggcagcagatccccgtgagtataccccagtcgagcgctttgctataatccggaaaatgcggactgctgttgatcacgtaataaaatacaccgcccacgatgctgatgcccagtgcagaagcagtttgctggaaagtagagaaaacgcctgccgctgcccctgcaaattttaccgggacgctttttaaaacaatgtttaacaggaaaggcaataccagaccgttgcccaggccgtataatcctatcagcagtattacattcatggtgctgacgtgtggcctgaaaagcaggagttgcagtatgaaggaaataagaatgataagtagtcctgcctgcaatacttttttcccggaccgtactatcagcttggaagcgagcacagatgagatcataaacaacaccgcatgcggaagaaagaacatgccgcagtccaacgccgtatagccgagcccgttctgtagatatacggcgctcatcagcaggaaagcggtgtgcatcataaagtgaaacagtaccgccaacaagccaatattaaactccctgatcttaaagagtgccgtatcaattaaactgcctttctgtaaaagtgtttttgtttgctggtcgcggataaaaaaggcaaatatgaaaaccgccagcagcatcaacccgattgcccacagcggccatcccatttcccttccttttgtgagtggatagatgaggcaaaccagtcctgctgtgaggatagcggcgccggagtaatcaaactgctgccccgtgtccctcggtgtttcatcgagatatttccggatagcccacagggatacgatcccaacggggaggttgatgaaaaagataagccgccagccggcgatgagaaaatgggtatctaccagataaccgcccaggatctggccaatgatagcagcaatgcttagcgtgataccataccacccaatggcctttgccctttcctgcgggtcggtaaacaacacctgtatgaacgcgatggattgcggcaccatcagggaagagctcaccccttgcagaaagcgcatgatgtttaactccagcggggtttgcgctaacccacatccgcatgaggtgagggtaaagagcagcatgcccaggaagaagatcttttttctgccaagataatcgccggccctgccaccggtaatcaggaaagaagcgctgcccagcaggtacccggctatcactagctgtacttccccatcggtggcttgtacgcctttctgaataccgggaatcgccatgttgataatgaagatatcaatgacatagagcagcggggccgttaaaataacggccagggcaatccatttggaatgcctgtgttgttttgggttcataaccttgtttgtgtgaatgtttaccggttaccctgttccaggtcgagtaaccattgtttccgccagatgccgccaccgtagccggttaaactgccgtcttctccaattacgcggtggcagggaatgaggatggagatgcggttcatgccattggcatttgcgatggcacggatggcttccggcttttgcagggcgatggcctgttgcttgtaagacctggtgctgccatacggaatggtttgaagcaggcgccacaccgattgctgaaagtctgtgcctggcataaacaaaggcaccgtgaatgtttttcttcttccggaaaaatacgcttccagctgctgttctaatacatcaaaatgtgggttggcgccctggatgatattggcgttgagtttttgtgaaagttgttttaattccgtttccagcatcttccggtcagtgaattccagtaagcaaatacctgcttccactgcgcctgcaaacatagttcccagcggcgtttccaggcgtgtgatattcattacctgcttttgtttgctattggatggcgataccccgaatactgatctgaatgaatcggcaaagccgctcagggactcgtatccggcgtcaaatgctgctgccgttacgggttcgccatgctgaatttttttgaaagcagcattaatgcggaacatgcgctggtaagcctggaaggtaatgccatgatgtttcaggaaccaccgcctgatggcgctgggtgctataccttttacagccaggtctgcgtctttgaatttccgggaggggttttcattcagctcctgcaggatcgccctgatagccggaggtgtttcatccagtttttccagcggactgcacaccttacagggccggtatccctttgtaatagcgtctttcgtggttttaaagaattctacattttcccttttgggtttcctggccgtacaggtaggacggcagaatatcccggtggttttaacccctgttatgaagctgccttcataagccacatttttatcaagtatcgcctggtacatgatttcgtccgtcagcatgtatatctttttttcaaaagtacgccagctgaacttgggtaacaaccggaaattgaacaagtattttttttagcgtacctcgtagttgtgtaactttaaatacggagataaaaaccatgctatatgcaggaagaaaaagcgagcggctgggacttcagctatttaaccaacacaggcagaatgatggaaagccctttgccctggaactattttgtaatggtgtgccgccacctgaagccgggctgtacccttctcgacctgggaaccggcggcggagagtttttaagcctgctacccggtaaagaacaacttcgtatatacgctaccgaaggatacattcccaatgtggtactcgcccaaaaacggctgcattcgtttggcggaacgcttgttcatgagtatacagatgataacctgccttttgaagataattattttgacatggtaatagaccggcatgagagttatgatctgaaagaagtatatcgtatcctgaagcccggcgggcatttcatcacccagcaggtggatgggagaagtgatctttccatcgcagaggtgctgggagtgaaacctaatgaagaatttttgcactggaacatcgattatgcgctgcagcagtttgcaccaaccgctttcagcatccttcaccagcaggatgattatggctttatgcgtttttatgatgcggaagcattgctgttttatatccgctctatgccttacttatttgaggaatacgacagctttgattttgagcggctgtcggcccggctgtcggattattttgccctgcatactttcctggatgtgcggaaagacaggttcatcattgtggcgcaaaagtaagcgcaggcaacaatatcccccggctggttgttagaagaaaagagaaacatcatatgatcatgaaaaatatcttgctttttctgttgggtttaccgctttttactttcgcccagcgggagaaattgctgtatggttacgcttatggaatgatccacgacggtaatggcggcggtggcgtgacggccaacgtggagttgctgaatcatgttattagtgtggggccgggtgtggagctcacttcttacaatgatcattccttgatcccggtatttgcagatgtgaaaatcaaacaccgcttcgggcatatagatccgtatatcaccgggcagttcggcaggaatggctataatgtaacccgtactgcggaagtgccctcaggaacagggcaggagtctgttactttcaatgaatccgggaagtatttttatggagcaggtgctggtgttgcctggcatttcaataagataggcgtgttcgcttcttatatttaccgcggctataaataccggtatcccgacagaatatcggaagaggatcacagtgttgtgttcggcgaaaaatccgtcaatgctaatgtgtttgttgtaggaattgtattttgaagcaggtgccggctgccccagttaaagatctggtcgatcagctgccgcaatgatgcaccgctttctgttagcctgtaaataactacctgcggatgtttgctgacctttacctcgcggcttatcagcccattattttccaggtccctcaaatgttcggtgagtatcttccggctgatcttcggcattttttcatgcagcaagccaaaacgattgatatcatgctctattaaatagaggatgacaggcttccacttaccgctgatcagttctattgttttactgaccgggcaaatgcctgcgtcatattcggtatgtgtaattgacatgcgtatatctttttaaaaaaaaagttgatggttaccatcctgtaactacttgcctgcgccgttttacaaatctagttttgcttgtataaaaatacgaatcatgtacaagctaccgaaaaatgagcaaacgaatgtaagtctgtatagtaacgcactcatgctcctcacttctgttcatcacgtatacggcgccatccggtaccacacgccctggcggatgcatgtgctgctgctgagtgtgcccgtactgatcattaccgttatcctggaccgggtaatcaaacaaaaaggaatgaccgttaagagtgtgtggtcctggatattctgttccatcatattccttgctgctattgtaatgattgggagctatgaagggatttataatcatctccttaaaaatatcctttactttggcggattatcagcagcacgcatgtccatgcttttcccgcccgctatgtatgaaatgccggatgatatattttttgaagtgacgggagtgctgcagggcattgtggtaattccccttggtatttatttcgtccggatgatccggcaggggatgacgaaattacaggcttaaaatatcatgaagctgttgttgtttaatcctctcaatctggcgcctgtgccggagtacatgcacaatagcgtgttcggccatttgttctatatcgtatacctgtccccagccggcttttatttttaacgcatcgtccatttgttccagttcatcatctttaaatgctgcgaatattttttctgtgaagataaatacctgggtgaggtcttccaggtaagcgtttacagtaagatgaaatgttttggcaggacgtgttagctgcgggccccgcaggttgtgaatactggtggcatagccaaagccggagctgactacatgagataaaatggtttgaaccgaccggcagttttcgtccgccgtatgcggatcggtgataacagtaagtgcgtgatcgggaatggtcctgatcacttctttcaattccgaaatggctctttcatattcatcaagcaatgcgccgatggccccctgtctgaaagtttgggtcatatgttttatgatggtcccgtcaaaagtaggacattcacctgataagaaggcgttaataatccgaccgctttttagcttcctttgttgccaggtccagcagggaatttttgatcacctttgtatatacatccctggttttgtcgctataggtaaaagactgcaggtattgttcataatcctttccttcgtaggtcattttctttgccagcaggagccatgtctcctggccggcttctttcccgaaaatatggataatggtaagggtgttgtgcgttagcaatgcatcgagataattcttatgttcctttgaggtatcttcttttgcaatgaggtctttcatcaccactgcgcccaggtcaacgctgttcgcatcatataccggctgaggcgtatcgtccgcttcccgcaggctgtccactcttttatagtaaatttcctgcgttgccttcatggtggctgctgctttctttagctttttttcgtcggccttttcatttttcagtgtgatggcagctttctttaccaatgctaagaattgcgcctgcttaacagtgtctgtttgctgtgcgaaactattcccggtaataaaaagtaacaataaagcagctgcaaaagcaaagtgtatatgcggtttcataaggtcaggatattttttaaagcagacaaatatataatatattatcaatatagtgatccggtataaaaaaataacctttcggcagattttattaataaatttacttccgcaaccaaagtagtttccaatttactaatcaaggaattcatcctgatttcattgattcattatatgaggggtttcggaattcatgaggatctgccaggagagcaggagttgctccatcgcgtagctgacggtgacggcatggcgtttgccatattgtttaaaacgcacaaggaaaatttgtataccactgttttacgggtaaccggcagtcgggagatggcggaagatgtattacaggaagtatttatcaaggtatggatgcaccgggagcgattgccgggtattattaatttcgccggatggctgtacaaagtagccgaatatgccggctttaaagtgatccgcagtaaccgccgtattgccggtgggctgcaggctttatccaatgatccgttaacgccgccggagaaagatcccgttgatatttttattgaaaaagagtacgaccagctgttggaggctgccattgcgcagttaccggaaaaacaacagctcacctaccggctcattaagcagcagggactgaaaaggaaagaggtggcagaacgattgtcggtgtcgcctgaaacagttaaatggaacctcgatcaggccaaccagtccgtccgtaagtattgcatggcgcacctgggacttaccctggctttcatgctgctgaatggtttgcaataatttttttcgtccttaccccccaattgttattcccgtggctcttatatatatgattcacaggaaaggccgtaaaaatcatactgtttatctgcctgatgaagcagggttactcgggagaattgccaacggagataccgctgcctttgccacggtatttgcgcattacaggaagcaactgtatacaaccatttatcaccttacgggaagccgggagctggcggaagatgtgttgcaggaagtttttatgaaggtgtggttgcaccgggaacggttgccggtaatcacacatttcggcggctggatttaccgggtaacggaacatgcgggttttaaagtgatccgtgagttgcgcagaaccgtcagcaacccgcagtcaccaccggaaacggataaaaaagatccgctggacctctacatcgaaaaggagctggataccttgctggacgaggctgtagcacgactgccggataaacagcaacaaacgtataagctgataaaagaggaaggcctaaaaagaaatgaagtggccgatcagctcctggtgtcaccggaaacggtgaaatggaacctggaccaggcgatgcgatcgatacggcggttttgcctggcaaagctttcccattaaaaacatacacctaagaaaatgaatgatggaactaccagataatatagctgctttatatcaccgttgtatacagggcgccgctactgcagaggaacaggctgcattcctgcagtatctgcaggaacctggtcatgaagatatcctgcgggaagtactgcgccgtggtttgcgggaacccaaaccgctgacagatcttccgccagagcgggaagaagtggtatggcagactatcatggcctccaccggggcaacaccggctgtaacgccggtataccggatggcctggttccgtatggcagctgcggcctctatagcagtattggtggccataggtggctatacttattaccgttcgcatgaaagcaggccattggccgtacaaacaccactggcgccgggtggcaataaagccatacttacgctgggcaatggtaaggtgatcacactggatagtattggaaacgggcaaattgccggtgaaaacggggtggttaaacaaagcaacggcaaactcgcttatgcagctgatcctgccggagctgttaccatgcacgtgcttaccataccgcgcggcgggcaatatcagctggagctgtctgatggtacagaggtgtggctaaacagtgcttcttatatcaggtatcccaaccgttttggtgataaagaaaggagcgtggaaatttcgggagaagcatacatcagtgtggcaaagaacgccacgaaaccttttatcgttgtttccaaagggcaacgcattgaagtattgggaacagcatttaacctgatggcctatcctgatgaagcagccataaaaactacgttgataaacggcgccatcaaagtgatccagcagggaacacaaaagatactaaaacccggtcaacaggccgccgtagcaaacaacactcccggtattaccattactacaccagacctggaagaagtgctggcctggaaggaggggaagttccggttctataatacagacatcgccaccattatgcggcaggtagccaggtggtatgatgtggaggtagtataccaggggcaattgccggaagaagaattttacggcgccattccaaaaagtgagaatgcccggcagatcctggatgtgctggaactgacacgcaaagtacattttgaaataaaagggaagcagatcattgttattcccggtccgaggtaaatttaaaccaaccagtcattgtgaatgaaaataaataaatagaaatacatcaaccaaaaagaaatccggatatgggagaacattttccggatagcagcaagaattagacgtaaaaccaacatcgcttttcagcattactttaacatccaaaccggtacaaagatatgagctcaattgtacatggcagtcccgtgcctgattgtatgccacctaaactgaccagatttataaaggtgtgtttctttgtttttacagcagcattgcttcttagcgcaaatacctacgcacaaaagattacgattacaggacggaatttatccctggagaagatcttcagggaagtagaaaaacaaacaggatattcttttctcgtcagcaaagaaacactgaagaaatccaaatctgtaaacctgaaagtaaaaaatgcctccctggaggatgtattggatcaatgtctttcagaacaacatctcacctgggaaataaaaaataaggtgattgtgattacacccgaacaacctgctgcaatggcgcaaccggtgatggtggagtcggtgccttccaacccgggcaggattttcagcggacgtgtaatagatgaacgcaaaagacctgttgtcggcgccaccatccgcgctgatgtagccgccgaccgtctgcagatgtcctttacagatgaaaaaggcgtcttcattttatctgaagtggaacttccggtggtaaaggcacagattaccagtgtaaatatagaaccctggaacggggagctgaacatagatgaacaacaacgtaccattgtcgtaaaaagtaaagtgtatcagctttccgatgtaaaggtgattgttaataccggctatcagaaactcgataaagaaagagccaccggctcttttggtaaaccggatatggagattgtcgccaaacgcaccggctccatggatatcatgcaaaagctcgacggtctggtcccgggattaaccctcgcagtgggcagcgattacgatgtggaaacgcaaaacggtaatggaaacggcgtaaaaaccaggagaagtgtgatccggggaaaaggcagcatccagctgaattcggacccgctgtacgtgatcaacggcatgatcgtaaatgatttcagtacgttgaaccccgatgatattgaaaatatcacggtattgaaagacgccgctgccgccgccatttatggggcaagagcagccaatggcgttatagtgctcaccaccaagtcaggcaaaaataatcaacggctcacggttaattacagcggctttatcaacttccagggtaagcccgattataactatatcccggtgatgaacagtcagcagttcattgccacctcaaaagaattgttcaacccggagcagtttccctggaataccctgtatgatcaaaccattccgccgcacgaccagctcctgtatgatcattaccgcgggctgatctctgacgcgcagtacaacaaaggaatggacagcctggcctccatcaacaaccggcaacagatcctggatgtgctggttcgcccggcgtttactactaatcatactgtttctgtgagcggcggaaataatgtgtattcattttatggatcattggcctatacgatgtcgcaggataatatgccgggaaataaagacaatagttacaaaataaatctcacgcagaatctgcagccaaacaggaatattaagatttctgtaaacgcttctctcattaataacgtacaaagctcaaaaaattcaatagcatctggtcctaatgtggtgccctacctgttacccaaagatgcctccgggaaaaatgtggctatgccttttttgtcgggatggtcagattccctgcggctcgattatcaggcgcgcagcaggatcaatatggattatataccactcgatgaagtggattatgcgcatagtgaaaggaatactattttcattaacctcacggctaatgcaaatatcaggatctggaaaggtttaagttttgatggtacctatggttatgtgaaatccccgggtgtcaacaattactttttggataacagggcatttatgcagcggcgggagctcctgggttttaccgtagcacccactgttaactccactcctcaatacctggtacccatcaccgggggaaccttcggtaacggccacaatgatcagcgtaactggaccgtccggaatcagctggtatatacagcagcaccacgcgaaggccgggaccacctgatggtacaggtagggcaggaagcacaggaacaattcaatttttcaactaccagtacttttttgggatatgacgaaaaactcggcacctacggcctcgtggattatgcaacactggcccagggtgtaacaggtacggtcagcggctacggctacctgcagcggccatactccattaaccaaacgctttcgcgctttacgtcaaaattcgcactggccagttataccttcaatgataaatatagtgtagacggaagctggcggcaggaccacagtaatctttttggcagcgatgtttcttcgcaaaataagccgatatggagttttggcgctaaatggcaactggcgaaagagaatttctttcagcccatcacctgggtggataatcttagcatcagaactacctatggtatcacaggtaactcgccctacgtcgggtcggcgtcaaggaatgatattctgaatgccatttcgcaggcaaatagcggcggaatagccggtgatgccttaggcatcgcatctaccgctaataccaaactggcatgggaacataccgccaccatcaatatcggcatcgactattcactgctgaaaggaaggatcagcggaggcatcgacctgtacagcaaaaccaccaccgatatgctgggcaatgtttacctgaatccgttcgccgggtataaaaccagtataggcaacctcggtaagtattccaataaaggaattgaactgaatcttacctcccggaatatccagggaaatggcttgaattggtctactacatttatattcagctataataaaaacaagctgcaggattttgaagcgttatccgcatattccaataccggtgattataaaatacaatcgttttattacatcggttaccccgccggacctgtttttgcctacacatggggaggattggataacatgggtgatccgcagataaaactgaacgataaaaccattaccaaagacccttattaccaggcgaagaatgaggatatcaaatatatgggcaccaccaatcccgttttcaacggggggctttccaacaccttccgttacaaagggatttccctttcggtgaatatgatctataacatgggtaacgtgatgcgccgcgatgtaaacaatttcagctccgaccggcccggatcttatgcgtcaggattttctttcggaaacctgtcgagttacttcctggaccgctggaaaaagcccggagacgaagccaccaccaatgtgcctgcctatgtggccaacccgaatgaagattacagccggcgcaacatgatgtattattacagggccgatatcaatgtagtgagcgcctcctatctcaagatcagggaccttacgcttaattatgaactgcccgctgcatggctgaaaccattgaaaatacagcaactgagcgtatacggacaagccaccaattttatggtatggagagccaatgatcttggtattgacccggaataccacgacatgcggcagggataccggtccatacctcctttccggcacagttacagcctgggcgtaaatcttactttataagtgaacataaatgaacagatcatgataaagaaaataatttatcctttcttatacataacgctgctcttttcctttgttgcctgcaaaaaggatttcctggaagtagtgccgctgggtaaccaggtagccactaccaccgacgattatgataagctgatgaacaatcccgttttttatatgaacgaggcttcgggagggcaggaagctgtatcaatgggagatgaaacaggtgcggaagcagctttcctgaatagaggcacggtatggatgccgcggctttttcaatgggccgacagtatctacaaacccggcgatgaaataccgtaccctttcatgttacgggagggactggaaaatatgtacctgcttaacaagatcattacagaagtaatggcatcatccggcgggtcagacacgcagaagaaacaactccttggggaggcaaaagcgacccgcgcctggctgaatttactgtttgtcaactactacgcaaaaccttacaacgcggctactgctgccacagatccgggcttccctattattgacaaagcggatattactgtgcagcggttcgatcgtggcagtgtacaaagcagttacgactttattattaaagaccttaccgacgcgctggcggatgtgccggtgcacccccgcattgttacccgcatgtcgaaacccgcagtggccgggctgttggggaaagtgtacgtgtttatgggccgttatgcggatgcgttgccattactggataatgcgtttgccgcaattgctgccaacggcgcaccggtgctgtataactataatgtggagtttgcaccgggtggcgcattcctccccatcgatccaacctttggcccgcaaggtccgggcgttaaccgcaatgatacccgggaagcaattctttctaaagtttattacaatggtcccaacagggggaatatgtttggtaccgacggactggtactgatgccggccgtcgcagccttgtatgggcctcatgatcagcgcctgctgctgtataccaatagggatctggatggtaaccttaatcccggtggcaggttgcgcaaatatggtattacctggtcgcgctacggattgcaattacctgagctgtacctgctacgggcagagtgcagggccagaacaaacgacctgggtggcgccataacagacctggaaacattgagaagaaaccggatgccggctgccgatgcgcaggttccacctgctgttgcgggcaaccaggtagcgctgataaaatatattatcgatgagcgaatccgtgaatttgcacaggaagggtaccgctggtttgatatgcgcaggttatcggtagatcccattttcagtggaaaagctatcacacgtaatttgtataacaccaacggaaccactacggtgattaccctgaggcagccggaccgcctggtgatgaaaataccgccttactttttacagaacaacccgggtatgcccgacaatccataattaaattaaaacagaccaacacgatatgaccagcattgtaaagcttgagcacctgtctcataagtatagcagctcatgggcgatccgtgatatcaatatagagatcagtaaaactggtattgtagggctgctgggatccaatggtgcgggtaaatccaccaccatgaacatcctctgcggcgccctgaaccaaacagaagggaatgtatatatcaacgggatcaatatgcgggaagatccgcaactcgccaaaagagagatcggatttttaccacagaacccgccgctgtacatggatctgacggtagatgaatacctgggttattgcgcagggctacgacagttgacaaaagacagaatgaaaccagccataaaagaagccaaggaacgttgcggcatcgaccacttcagcagccggttgatccgcaatctttccggcggctaccggcaacgtgtgggcattgcacaggccatcgttcaccgcccccgcctggtggtactggacgaacctaccaacggcctcgatcccaaccagatcacggaagtacgcgccctgatcaaagaaattgcacaggaccgggcggtcatcttttcttctcacattctttctgaaatacaagtgctctgtaaagaaatcaagatgattgaaaacggaaggattgtattctccgacagtatggacgcatttaataactatgtggaaccgcacagcgtcatcatgcacctggaaaatccaccggctgccgccgaactgctgaaaatagacggggttacaaaagcggattttcttactgaaagacaagtacgcctgtatttcaatggaagccaggacatcaccgagaagctgatcgttgccagtgtgcagaacggatggcggttgcgggagatcaatcttgataaaacagcactcgatgagatcttcaaacaattatccagtcaatcatctcaataaaaatatttaatgaagacaatattcagaattgcaaaaacagaactgcgggtactgttctattctcccattgcctggtttttactggttgccttttttattcaatgcggtatcgcctatttcctccagttacaagggtttgctggcatgcaggaaatgggcggtgagcagttaagatacatggataacctcaccatcaggatcttttccggtgacaacagcgttttcactaacgtgatgcagaagctgtatctctacgtcccattgcttaccatgggattgatcagccgggaaaccagcagcggcaccattaagctgctgtattcttccccgatcaaagtacgggatatcgtgctgggtaagtacctggcgatgctcatttacagcttactgatggtggcggccatgagcgtttttattgttgccggtatgtggcagatcaaatcaatggacagcggtatcatgttatctgctgtactggggcttttcctgttactctgcacgtatgctgctatcgggttatttatgtccagtttaactacctaccaggtggtggcggcggtatgtacttttgtgatgataggcatcctcagctacataggtaccatgtggcagggaatcgatttcgtacgggatcttacctatttcctgtctatccagggacgtacacagaagatgttgtttggtttaatcagcagtaaagacgtcgtatatttcctcgttatcatctttatgtttatcgggttcacttatttcaggctgaaatcaggcatggaatccaaaccatttatggtgaaagcaatgagatatgtggcagtagtggtaataggtctggcaataggatatgttagttcccgccctgtttttactttatatacggatactacggttcaccagcaacaaacgcttacccccaatgcccagcggattattaaagagttgggagatgaaccgctggaagtgatcacttataacaatgcattgagcaggtatgtgtggctgggcataccccaggagcgcaacaggttgttggacaactgggacctgtatacccgtttcaagccggatatcagtttccgttttgtgcagtactatgcagaaccgctggataatccgcagtttccgttttctaagatgtatcctaataaaaccgttaaagaggccgccgaacagtccatacgcgggctgggcatgaaggtatcgcaatttaaaacacccgaagagatcaaaaaaataattgacctggaaccggaattaaaccggtatgtgatgcagttaaagtacaaaggccgttctacttttctgcgggtatttgacgatcagcaggtatggccgagtgaaaccgaagtttctgccgctttcaagcgtttactgcaggctaaactccccaaaatcctgtttgtaaccggcgacctggaaagggatatttataaagtaggcgcccgggaatatatgaccatcacgaataccaaaacgttccggtattcattcattaaccagggcttcgattcagatactatttcactggcttcacgcgagatcccggaaggcatcaccgccttggtactggcagatccgaaaacaacccttagtccggcttcactggctaaactggaacagtatatcgacaaaggcggcaacctgctcattgccggcgagccaggcaaacaaacggtgctgaaccctgttttgcaaaaactgggcgtgcaaatgatggaaggcgtgatagcccagcccagcaaggatcttacaccggatattgtattgccggagttaacgccgctggcggtatcgctatccgccaatgtagccaaaacggtgaaagacagcctgaaagtggcgatgcccggtgttaccggtcttacttacagcggtagttccttcactgttgaaccattactggttaccgacgctaaaaagagctggttaagaaaaactgcactggtgctggattccgcacagattgtatatgatgcggccgccggagacgagaagaaagcattgccggtgatgatcagcatgacccgtaaagtgaatggaaaagaacaacgcatcattgtatccagcgatgccgatttcatgaataataccaacctgaacaggttcgatgtggaaaccgctaactttcctttcatcactgcattattcagctggctggattacaaagagttcccgattgatacgcaccgcccggagtcggaagataaccgggtaaaagtatcgctggatgatgtggacctgctgaagatagtatacctctgggtgatgcctggaatactgattgcctttggcgctatattgctgatcagacgtaagcggaaataaaattttatgttatttactacagataaacaaacactggaagatcttaacatctttggcaaacatggcggagattccatcttcaatatctttaaccgctgcatcaccaggggtggtgcggcggtactggatgagatgttccagtacccgctgtcagatgagaaattgattaaccgtcgcagtggtatcatccagcatttcgcggcaaaagaaaccatgttcccgtttgagaacaccctctttgatgcggcggaaccttatctcggtaatacggatgaacggaccaggctcactacggaagatcatgcggttaccaaaaaactcagcagttttattgcaccggatgccgacgctgttcagatccggaaaggagtggtcgcgcttacccggctgataaaaggactgaacgattttatttattcaccggcagtagccggaatgccttattataacacggagaaagccgctatagatgcgctgctgactgatcctgcactgaacccggtgatcctgcacgaagggaaagacaagctgcctgctgctacaatggctgcttttgacggtattttccgtttccgccaccgggacattattttgaaactgctgcggcatatctattatctcgatgtgtatatagcgatagcaaaggtggcaaaggaaaggggatttgtgttcccggcagccctgcctccaagccggttaacggtgacgctggaaggcgtatatcatccgcaggtgcccaatgccgttgccaataccatagggataacaccggaaggcaatgttattttcctgacaggcgctaacatggccggcaagtctacttttatgaaatcattgagtattgcgctgttcctggcgcatatgggtttcccggtgccggccacccggatggaattttcagtgttggatggcatctatactactataaaccttccggataatctgggaatgggcgccagtcatttctatgcggaggtattgcgtgtgaaaaagatagcgcatgaacttagtcagggtaaaaacctgctgatcgtttttgatgaaatgttccgtggcaccaacgtaaaagacgcttacgaagccactattgccattaccaaagcctttgctaccaaacgcaacagcctgttcgtgatttccactcatatcattgaggcgggagaggtattaaagcaagcctgcgacaatgttcattttatttacctgcctacacgaatggatgggaacaaacccgtgtatacgtataagctggaaaatggtattacagacgaccgccatggtatgatcatcataaataatgagggcatcctcgatatgctgcgggcaggtatctcaacatgaattaaaagacaataacatgagcttcattgctgataaacaaacattagatgacctgaacctgctgggtaaatataaatcacattccgtttacagtatttttaataaagtgcgcaccgcgggcggggaacggttactggaatccatgttccagcatccgctcaccgcgccggaagaaatcaaccgccgcagcaatacattccggtatttccaggaaaagcagctggagttcccttttcagaacggctccttccgggcagcggaaaattacctgggcatggaaaccgccggcaacagtgtgtcagcgattattattactgtgagaaagaagatctggcagtcgttgttgcgggacgaccagtttgacatcctgcacaacgggctgctcgcctgcattgccgcattaaacgcattgaaagaattgttgggccgtatgaatgataaccagcatccttttcatgaacaggtaaaaatgttgctgggtattttttccggcccccggttaaagtggcttgcagcagaaaaaggcgtaacacagctgccgctgatgaaagtggcccggtacgatttcctgctgcgtaacaccctgcgaaaggaaatggacatcatcctggaaaatatttacctgctggacgtttacatcgcggtaagccaggtggcaagggaaaagaatttctcctatgcaacggcgttgccggcagcggatcatttaatgcaggtagaagggctccggcatccggggctggaccatggcgtgcctaatcctttgtcccttcaccgccaccggaacgtgatgttcctcaccggcgctaatatggccggcaagtccacccttatgaaatcctttggtattgcggtgtacctggcgcatatgggattcccggttgccgccactgctatgaggtttgcggtaagggatggattgtatacctctatcaacgtaccggatagtttgagtttggggtacagtcatttttatgcggaggtaatgcgtgttaaaaatgtggcagcagaagtgagtcagaaaaagaacctggtagtcatcttcgacgaattgtttaaaggcaccaatgtaaaagatgcgtacgatgccaccctggcggtaacagaagccttttcgcaatacaggaattctttctttattatctccactcatattattgaggtaggggaaaccttaaaacagcgatgtgataacctgcagtttgcttacctgccaaccgtgatggaaggaactgttcccaggtatacttaccagctggaatccggcattactactgatcgtcatggtatgatgatcatagaaaatgaagggatcctggaaattattatgtcttaataaaataaatatcactcattgcgtaggcttcatcttattataaatatcgttgtaagtatcaaagttccggaatacctggctggtaggtaaatttaattgctgcgctatcgtggaaatgctatccgctcttgtcagcagcttaatggcttcctttgtctggttggtggcaatgaggcgggtaacggcctggatcagccgttcctggtaggtattccctttaacattaatgatgtaaggatgggtaataaagcttctcgtaagctcgtctaaacggttcatgaagccggtgaggttgctgtaaggtgcatctatctgtgaaaaattattccagtaaagatcatatttaacgtaatcgatcaccatatccaccagtagttcctgctcaaaattaatcccgccattattttcattaacggcaaaccgggtcatcacggcggaaagtaccggcaaaagattatttaattcaaagagttgtttgttgcccgtcagcagctcaagatcggggagtggcagaaatgcgcaatctgtaaagtccgtactttccccggtagccagtatttgcagggcgcggaccagtgataccaggaaaggatgctcccggatgagaaggtgatcgctgtcggtgagttgctggaaatttttatagtctttgaaagcatacatgattttgtccagcaccaggtattcttctgcatccctgctgaatgattgtttattggaatagaagaagaagcaattctccatatccgctttattgtgatagcggataaagaactgcgtttgataatgatcatatatgtagaatggaaagatcctgggatcttccgtaccattggctttcaggaagtacagtccattctccagttttccggaaaagatgaaccagccttcttcattattgaagcgggtgttatcggcgttgaattcaatcagtgtatcattggtgctgctgaggatggagtagctggtaagcaggttaacaggaaccagttcggggaaagtgtttttatcgtatttggcgccaaagaacaggaagctgggccggtgcggcgtatccgggttggtggattgcaggctggatgcttcgaggtttttgcataagtaatcatgcgtggctttaaaagataagatgggcgcaacggagggatagtcaaagtcgaagtgaaatgttttatcggcatctacaatgaggagatattcctggtagtagtcgatgaggttcactttcaggcggtagatgcctttgtccacaaacatatccagttcagcagtatacccggcgtaaatgatctgcagatccccgtttacgagtatgaggtgcaatccttccacaggttgattgaaagctacggtaatatggaattttacatcagaattgttcataacccacagtgttttcagaaaagttgatgatcgttttttgttcaccacttacattgtccagtaaaacataatttcctttttccagtttgtagtgccatttctcgccggtaactacatcggctgtacgcagtttgtcggcgtttttattatagagggtcacattggaattgcggttgaaggttatctcgaagttgtaggcttcttccagtttttttacttcgcagatcacgatgttatcgccgccattgtcggtggaggcgctgccgttctggattttgttatatttcagggcatacgtggggaaattgctttctatatgctgtttcaggtccagcgcggtaattttgccactgttgttgatatcggcatcgcctttcaggctttcaatgagaaaagaggtaaaggcgccccttttctggttggagtcgatagacacttcatagcttagtttcccatagatggtagaattgcaaaccagtaccctgggtacccgttcgcccactttattctgccagtcgccgataggaggcaaaccttttatcatggtgtcgttttcccggcagcagtcgaggaacaacagcacttcatcaaagattcccttgttgattagcccggtgaggtaatccaggctggagatacagtgattaatcattttgggccagaaccgcatgcacagtgcggtgttgttaaaggtattgccgatgccgtgaccagaaaaatagaaatagatgcgattggtttcgttcctgtgtgctttcgcattttctgtgatcgcttctatggcactatcaatttcatagccaatcacaatctggttgctggcatcggatttcagtagtttgatattatcggggttagaaacaagttgcatgtcggtcaggaattttgcaaatgcctctgcatcggctaccgccccggagagtgcccttttatcataatggtcaatacctattataattgcatattccatggtttatatgctttttagaatagcggttaaagtgagtgtgtcgttatcaaaatcgccgtgtttaagagagctgcatcgcaggctttcgtctgcattttcgagatcggtggagaggatcagtttattattgccgatatattgattcagttttttcagttcatcgaagtcttcataacggccggttgctttcagttgttcatgcagccccatgatttttgcatccacttcttcttcaaacaggccagacaccatgtatagcagggagtgggtgtaagcgaaaggaatgcaatgatcctttttctcgttgctttcatccatggtaaacatcttaaaatgtttaaacacgcctttttcctgcgcggggcttcctttctgcaggaagaagtctgttctgcaggcaggggccaggaagaaaacgttgttataggttacggcattgaaatgattggcagtggcttccagtaaattgcatacggcaatggcgccggcactgtggcctatgagttctatatccagcttttttccggcggcctttcttttttgcaggtgcgtatccagcaaggagaggaagtgcgtaccggcgtgcaggttgttgccggttaccccgctgttgctgttgaacatattgccggatttatctttgatttgtttccagccccatccgccgattttatcgaggtacaatttcctgaaggcttcttccatgatggtggggtagaagtcgtggtgcgtttttttgaagtagcgttttaacacggcaaaggctatctgcgctaccactttggccacaaacagcattccgcccctggccacttcatcgccttcggcctgttcatatttgagttcttctgatccttcggcactgaccagccccttggcttctgtttccagtttggcgtagtaggtgctgtagttttcgtcctcctcatctatttcaagcggggtgccgccgcgggcgtccagggatctgtcgaggtcttcaaaaggggcgatcttttgtttttctacggcaatagtttcatcgctgaggtaggtgcccccgcctttggcatcatccagaccgagtttcttggcaaccagtttggtgacgaatttcacgatttcatcgaacacgcctttcccggtaagttccttcaggtttttgaggttttgcatcactacctcagcggggccggtttcccatacaaaggccacggtgtgcctttttgcagccgcgtcggcgaagtgttctttcatgacagcagcagctttcagcccgcttttttcgctgactaatcccccgtgaaaatagatcagcagtttttcgatatctttttcttcgaggaagctaaagatctgttctacatcagccggggtagtggagaggtgacctgaatcggcaaaggtgccatcagcgcctacgtttacaaagaagattttttcaagtgcttccatgatctttttttggggttgatttgaatacacggagagccccgtctttaattgaggttattggggtattgatttggagttactcgtcttttggggcttcttttcctgatatctaatatcggtcatttttacagaaattcaaatttattgtaccgggaaatgcctgtggcggttaatagcagtccctgggtgggcggcttcaggcaccggtgcattaaggcagccgggctgccagtctttccggcatatacttcagcacctggtaaataattttccatttggcgcccggcacaatggcaaaacggttaccggcatgcacgatagtttttgcaataaaagaaggctccatcagtaaatattcgggaaggttaagtcctgctgtcattttactgcggatgtatcctgctataattacattaacaataattttcctggagaacaggtattgccgcagtcctgcaagatattgtgtgaaggcagccttggtgctgccgtatacaaagttgctcttgcgcccgcgtacgcccgaaagcgacgacagcccgataatcctttccaggtgatcgttttcgggatccgaaataatgagattaagaatagacagggcgccggcataatgcacgttgatcatccggtaactgccttcccaatccaccagtgcctgttcattggtaacctggaagcctgcggcatataccacgatgttgggtttaaccggcagactggcatagaacccggcgtgatcgttaaaagcggtggcgtcaaagtaacagatggtcagttgctcagcggctgccttcctggctttcataaacgatgcgatgtcggcggtgctgcgtgaagcggctataacatgatagcctttttccaggtataataatatcgcttctttggccacatcggaattcgcgccaagaacaaggaccgttttgatagcaggaagagtcatagatcataaaaatagtcattgtcgggagattcgttgcaggcgtttgttaaatccggttatttactgtaatcttatacggtaataaagtaacccgatgacagtacctagaattaacaggtggatctcctgcctgtgttgtttaatttttgcagcagtggccactgctcaaactcccgccaaaaataataaacttgaaaagatagacgccgcgctgacggatatcctgcaggatgcgcagggcgccggctttgccgtggctgtggtggaaaaagataaggtgatattttcaaaaggctttggttaccgggatatgacccgaaaattaccggtgacagaacatacccgttttgccatcggctcctgtaccaaagcatttaccagcactttgctgggcgatttgcggaaagagggaaaggttgattttgataaaccggctaccacttacctgcctgcactggatttttcggatagctatctcaatacccaggttactttacgtgatatgatgtgccaccgtaccggcttttcgcgctacgaccttgcatggtatctttttgaaacggattcgcgtgactcgctgctgaaacgcatccattatatgaagcccaatgcgcctttgcgcgcccgctggcagtacaacaactttatgtttatggtacagggaatggtggtagagcggttaacggggcaatcgtgggaacaaaacattgccagccgggtttttcaaccgctgggcatgagtgaatcttctatcggcactattgccctcgccgctgcagaagagcgctcacacggatatgagttcagcagggagaaaggcattaatgaaatgaagtatcacccgatagtagcaatgggccccgccggagctatcaacagcacggtaacggatatgtcgaagtggctgatcacctggatccatggcgggaagtataacgggaaggaaatcatcccggcagactatgtgaaagaagccatttcttcccagatggtcattcctggcggagaaccggataccaaaacaccgtatatccagtttgccaattacgggcttggctggatgctgctttcttatcgtggtcattaccgcgtggaacacggcgggaatatagatggattcacggcattgactaccttttacccaacagatagtattggcatcgtggtgctgagcaatcagaataattccgctatccccactaaggtgaccaatctgatcaccgaccggctgctgggcattgcagccgcgaccagtcctaaagctaaacccggcaaaagggaggaagaccccgcgcctcaccgggattctgcctccaggccgcatcctcctacacacccggcagcggcattcgcgggagtgtttaagaatgatgcttatggtaactttgatattgctgtaaagagagattccctgtttgccacattccccgatgtgacctggtacctcaaccaggaagactataatattttctctccttacgatgctgcagatacggcgattgacgtaaagtacaagtcgaacatgagagtacaattcctgatgaataacagcggggatatcgaccggctgagttttgcctatgacccgtccggcgacccggttatatttgagcgcgtactacaacaggtggtattatctgccgcctcgctggcgccatttgtgggcgcttataaaatggcctccatgccgatccagatcaaactgtcggataagcaggtacttaccatggtagtgcctgggcaaccggtgtatacgctggaagcaatcgacagcagtaccttccgtattcaggggctgaaagagtacaaggtgaagtttatcagggatgataaagacaaggtggtggcgttaacatccatccagcctaatggctccttccgggcggagaaggaataatgcgctttaaaacttatgtttgctcacggagtgtttataacacgccggattacctatatttttgataaaaaacagatcccttaccgtatgaaaagaattttcaccctgctgctgttagtggcagctatgaccacaacaacccaattaaaagcacaggacctggtaaaaggaaagcttgatttcctgaaggatgttacagaattgggcgtatccttcgactacaataaagtaaccgtaggaacagaaggaaaagaggcgaactatctcaaaagaaaaaaagcagaaaaggaagctaaagagccgggaaccggcgacaagtgggaggagagctggtttgccgacaggaaaaaacattatgaacccgagttctcagagctttttaccaaatattccgatattaaacttaccgaggattccgccagtaaatatttaatggtggtgcggacaaaatttattgaggtgggctataacgtggctgtttcttcgcagaaggccgccgtgaacctggaggttgaaatatacgaccgggccaacctgaaaaaatctatctgtaaaattatgatgaatgatatgaaaggtggaaaggggcagttcgctaccggtatgcggattggtgatgcatatgccaaagcggggaaagaactgggacggatggtgagtaaaaaagtaaaataacaattgatatctcaaaatagaaaaaaccggtgcagttctgtattactgcaccggtctggggaacattgtatttattgaatggggccgggttaccaacaatgacgttaagacacacttgttaaaaactaatattggggtgttaccgagataccatcattatacaaaccgttgccaggtctgcttttgatgggatctccggataaaaggccatcagctattcttcttgttaatccttaaaggattgtattacaggggcaaaagtatagcgcagcagccagtgaatcaactgcgaaaattcgcaggttatgctattctttattatttttacgatcaaaaagatgcatcctgataagttggggtttggaagttactcgaaaggatttataactgatgttccggctgatctgaccagcccggaagctttgcattttaaaaatacgatccgccggtttgcggatgaagccatctatatttattcgtttaaagaaaataagatgttgtatgctgacggttgggaggaattgctcggctatgcagataacgagatcagcatgctcaccattgtaaatattaccgcacccgaatatgcccctttttccaatgagctgaacgataaagccctgatgttcctgcacaataaatctattggcgacgaacaatacagctttaccatcgaattgaagaagatccacaaaaacggcacgcccatacccctcatcagtaaagtgggcgtatttaccaccgaacagggaaaggtgaccagcatcattggccactcccagaaaaatgagagcattaaattcggaaacgtgatgcgctatgcggcatacgggcctgaaaaatccgagtttgaggaagagttgaacaagcagttgttccggtattatgccatctcagaaaaagagaaagacgccctttccctggtggcggaaggttattccttcaaggaaattgccgcccggttcggggtatcgcagtcagctattgagaaaaggattttaccgatgtataaacgtttcggggtaaaaagcctgacccatctcatcagctttgcatttgcaaatcatattctgccttagccgctttatttttccgtacataccgctccaggttgagggaaagcattttttcccgttccactcctatgctgtgcagcatgttttgccaggtggcagacagcttacggtcctggtcgtcgttgcccagcacccagataacattggtatcctttaacgcggttctgttaatgtcattggtagaggagccatccacgaagctgaggaagcggtcggacgtgatcaggtcttctttcaccgggttgcccggattgatatcgtctatcaccaggatggaggctttgcgccaggtccacagcacatcggcggtggagtcatcgtcgtgttcataaaacatgcagtaaagcttcatggcggaagtatacaccgccgaatagtggcggatggatagttccgtggcgatggccacgctcaaactcgttttgccgctgttcttcggcccaaacaggaacagatgcatcccttgtgttttactatccaggaaacgcctgatcaggtcgatatcttcgggggcaatctgttcggtgctccattggctcagccggaactgaaacggatagcccggcgtttgcaggtacattttggtaagataccagtaataggtggggtagagcagcaacgccgcagttactattacgatggccctggccaccatggtatctttacataaaagggagcagaaaaacgcacccagccagaaaaacagcagatccgtgatggtatcaaaagccacattgccccaggcaggctgaaatacgtatgactttacgccgcctttcttgccaaaggttaaaggccacaggaagttgatggcctcaaataccagccaaacggcgctgatactccaggcggccgtaagtgcagcgcgcgtttcttccatacgatgcctcagcaccaggtataaaatgaatgcaggaataaaccccagtgaaaagtgaccaaactggttggccagccacgtataggtaagcgtaaccccccggtaagagtccttacctccgaggtcagccttcagctgacggaacatgttgctgtgagtaatcgttttcttcatgagcagttcgggatagcagcggttggataattgagggtaaatataataagttggcagaaataatagacccgcggcctgaaaaaagccttgttaccagggtaccatgactgcgaaaaacgaatcgttgcatgtatatttaaggttgatccgtcatttatgaagaaactatttattcttatttttttagcaggactcctgcataacgccaccgcacaggatgcggtatacctgtttgcctattttaaagacaacgggcaggatggactgcacctggcgtatagccgggatggttataagtggctggcactgcacaacgaccagtctgtgctcacgcccaccgccggagtggataagctgatgcgggacccctgcattatccgtggcgccgatggccggtttcatatggtatggaccgtgagctggaaggaaaaaagcatcggctatgcttcatcggccgacctggtgcattggtccgggcaaagggatatccccgtgatggcgcatgaaccgggcgccttaaactgctgggcgcctgaaattacttacgatgcccggcgtaaagaatatatgatctattgggccaccacgatccccggccggttcaccgccggcgattctaccggcgacgaaaaatataaccaccggctgtattatgttaccacaaaagatttccagcatttcagcccggcgaaattattatacgaccagggctttaacgtgatagatgcgagcattgtacctgaccagggccggtttattatgttcctgaaagatgaaaccaaaacaccgccacagaaaaatatccgcacagcagtcagcaacactttaacagggggctatgagaagccttctgcgcctattaccgggccttactgggcggaaggtcctacggcactgcataccgccggtaagtggatcgtgtatttcgataagtatacccagcaccgttatggcgcagtggaatctactgatctgaaaacgtggatggacgtatccgacaaattatctatgccgcaaggcatccggcatggtacggtgctgaccattaccagtaaggagtttgaattgctgaagtaagaagaaaatatcgcggtgtcggttttgttctattttccgggtaaccgccatagtagctttgagaaaaaatagatcatgaaaacagcaaatactaccaaacaaacagtactcgtattaggcggcaccggtaaaaccggcagcagggtggcagcacaactcacagaaaagggatggcccgtacgtatcggatcacgttctgccaatccggctttcgactgggaagatacatccacctgggaacctgctttacagggtattgacgccgtatatctcagctatcacccggatctggcgatacccggagcagtggatacggtacgttcatttaccggaacagcggtgaaaaacggtgttaagaaaatagtattgttgtcgggccgcggagaaaaagaagcgcaggcatgcgagcaggtcattatgaacagcgggatcagctggaccattctcagatgcgcctggtttagccagaatttcagtgaaggctatcttttagatccgctgctggccggccatgtagcgcttccggccggaaacgttgcagagccgtttgtggatgtggatgatattgcagacgtagccattgcggcgcttaccacggaaaaccataacggccagctatatgaacttaccggtccccgcctgatgacctttgaagaagcggtgagggaaatagccaaagccgccggcaggccaatccaataccaggcaatacccatggaagcatacaaagccatgctcgttgaatataacatccccgatgatttcatctggctggtcacctatttgtttgctgaagtactggatggccggaatgcccatctcactgatggagtgcaacgcgccctgggccgtgcgccgcgggacttctcagactatgcccggaaaaccgctgccgaaggcgtatggaatgcataggaagatgagcaacagcagggaaaagcacgcaatgcttttccctgcctgggttatagcgtataaacaatgagcacgcctatactgaataatacatgcgacaggccaaccgccatcacatacgacatcaccgggatggcaggcggccgcgggtggagacggataaaagtaaaccagaaccccatcgcgaaaataccgttcagtaacccaaatacgatactccaggacaaggtaggacgtcctatgccggcctgccacaggtaaaagtaaataatggcgaaaaacacacctatgaggtaatgcagtatgatgccggttaagaggtctgccggcttccgggttaaacccttatccggtgttgtatgattagtaaccatagtagcaagcactcccaccactttataatttttaccggtaatggcggtgagaagatataatgcgcccgtcattaataaagtaccaaataggcccgcagcgatcgctttcataaaaacctggtttgtatagcagccttttatcaaataataatcctattaatgcgaacacgttgcagccttctttgaaaccggttttacgatgtacggccgctacattttggggagcagtttctgcaattccgcaccgcttttctgtcccacacctgttatcggtcagggcatataatttgcggcaactgaaaggaaaagtaattagttcttcacctaaatttcattgttatggcagacgataaaaaaaacgttggcaagcaggatgatatccgggtagatagccaggacccttcagaagtggaatacctgcatcagcagtttccatctaaaacccaccaggaaattaaagacgccatcaaaaaagccgggccgatgagaagcgatgtgatcaaatacctgaatggtcattaataacccgttgcatggcggataaaatttcccataagagcttattggaacaggcgaggcaactggaggcggaagacgacctgccaggcgctattgccttgtataacgaagcgctttccaatgatccgctgaccattgctgcctataaccggttaatgatcattttccggaagcagaaagcgtataaaaaagaactggaaacaattaacaaagggatcaaatctttggaagataatgtgcatcaaaccaggactacctggatgaaagcgcaccggaaggcggcgaagctaagccaggcactggcaaaaagcctggggcaaatagatgccaaagggaaattaacaaatgaagacccggtgattactgggtggaagcgaagaaaggcaatcgttttaaaacggatgaagaccccataagtttgccgtataaaacaagcgtcttacagttatattgtaagacgctttcgtattttaaatactttttttaccgaagaatttctttttggcgctatgcaccggaactaatggcaggatggccgctgcggcttctatggagcggtcggcttcaataagactggcgccatcgcggataatcgcctggtaagcggcactgcgatcggcggaagaaggaagcttatcgtaggtgggcgccgtggatatcatacacatcacaccacgcttgtttaattgctggtaaagttccttcagagccggtttgttatccggacctacatacgccatgatatgcgaccacggaattttagcggcctcgtattcttccaacgcctgctgtgtttttacaaatgcttcgaatacaatatccttattgcggctgtggtaccagcgggcttcttccgcggtatgtaccgttaccattacgtttccttcggcatgattgtctttaatgatctttgcggtcatctcaaaaggcacatcttttttatccaggatgagcactgttttccccttgctccacacaattgcctcctgcagggtgggaatgcggaaattggtgatatttccttccacatcttttagctgcaactgtttaagttccgccagtgtataatcggaaatttttcctttgccggtggtggtgcggtccagtgttgcatcgtgcatgagcacaatggcgctgtcttttgtaagccggggatcaatttcaaaagtggcgggcgtatgccgaagggtattttcaaaggcttcgatactgttttccgggaagcctttgtttacaccgccacgatgcccgctgataaagggaatatctttcccggtatacttaaagaatgcctgcagatcctggctgttgcggatgttcagcacattcagttcaggtgattgagcctgtgtgttaagctggcaggtaagatacgcgcctgtcagcagtaaggttctggcaataacttttatcatgatcagaattttgcattgaggtgttgtaatgtaaaaggttcgtgagccgacaggttaaatactgtaacagaggcattgtcctgcaccagcatccggtaatttttcagcggcatgcccagcttatacgccaggtacaggcggtttacaccattatgcgctgctacaagaatgtttccatggtcatgttgctgtagcaggtcatggaaaaattcatccacacgggcaacgatttcgctgccggtttcgccggtgccaccggcgcggtgctgacctgggtcgtccatccagttatgccacagctgcggatcttcggcaataaattcttcctttgttttcttttcccagttaccaaaatcagcttcaataagacggttatctttaataacatccattccgccggcgatgcgcgcggtctgatatgcccgctctaacggggaagaatatacgccggcaaagttaattcctttcagttgttcccgcacggcttctgcctggccgatgccttttgccgtaagggcaatgtcggacctgccgcagtagcggttattatcggcgttccaggcggtttgtccgtgtcttaacaggtaaatattaagcatgttcataagttgaaatgtatcctttttctttcagcagttgtataaatttcaggtagctggcatcgtaggtttttacgggagatggcgaaggcagtatctcttccgctacctgggtcattgcagctgttgcctccataacggtgtggtaccatgttttggacgccgccaggatagccgcaccggcagcgccgcttacgtgtttcattttaatgatgggcaggttgagcacattgctgcggatggtgagccatgcgcggctgttgctggcgccgcctgcggtataaatcttttccaccgcttcgccgcttaactgccggatcatctggtaggcatagcgctctatataagccacaccttccatgccggcggcatagctttcaacggcagaaagtcccgcggcttcaaacccgcatgcctgcggcgccacgaacggaaacctttctccgtgttgcagcagcggccaggagaggtggccggtgggtatgatccgcaacgcctgctcattcagcaccgtaagatcaccagggaatttttgagatacccagtccgccccggtattgctggcgccccccggcatccagtatccctccgggtgccggtgacaatacaatgcaccggaaggatcatcgatataccgggtagttactcctttcaccaccagggtggtaccaatggtggtgttccagtcgccggggcaaacggcgcccgccgcaatctgcgaggcacagccatctgtcataccagctacaatggtcacgtctttcggcaggtggaggagggctgccacaccgggttgtatctttcccaacggagtacccgcaggcactacttctggcagccacgattgttgcaggggcaggtgctcccagagataggaaggccactcctgcgcctgcacatcatatcccgatttcagtgcgttggtggcgtcggttatatcaaagcggccgctgagctgcccggtgatatagtcggccgcatgaatgaacttataaagttgttgggctgcttccggatattgttgtacaaaccagcacattttcgatagtccactggaagtattaaacgacgtatagccatgcgggtgataccggagagcggtctcccggcaaagcttcccggtctccacctgcctgccgtcgctgtacatcagggcgttatgcagtggccggtgccggcggtcaacgggtacgatggtaccggacgtagaagtaacggctatggccctgataagtggccggtgcggctgcacggaggcgtcctgcaggagctgatgcaaacacgcaaggcaggcatcccaccagccggtgggcgactgctcctcccgcatcttttcatgcaacgggaaatgttcctcccggctgcccagcaggttgccggtggcatccattaataccaccctggcgccttgtgtacctacgtcgatgcctatgaaacaagctgttgccataatcgaattttaagtagttagttcatgccccggaaataatgccgggttttttcccattcagcatacaatgtgctgtaataggcagtatcaacaggatggattacttcggtagcatcctccattactgcatttacctgcagcgcctcattgcagatcaacgcgccgccaacggcagatgattgctggtattctttcctgatctgtacctttttccccgtgagattggcgatgagttgccgcagcacccggctttgcagtccgccgccacaggcccagatataatctggatcatgaccggcagtagcagccagtatccggtagtttttaacgatggagcaggcaatgtccaggatggtggcccatacaaaagagccgcgggtgagcaggtgcgataccggcgcgggaaaaataaagccaccgcgggtaagggacacttcttcatcagccagcaacgatcccagggaggccatgcaaaacgtatgggtgttttcttccagctctttttcaatcacttcataatcttcattaggataaaaaatttctttcagccgctgatagtttagcccggttacaccggcattggcttcaaatacaaagcgtcccggttctatatcacggcttgtccaggtcctttcttccgcatccagtgtatacgtgcccgttatcttcacaataggagtggtagtgcctgaaacaatcaccacgtcgtctaccgccggccgcgtgcttttgatggcaagttgcgtatcgccgccaccggctactattttcacggtggcaggcagccccagttcctgtgctactccaggaaggatatttcccagtatagtggcggagtctgcgagcggcggcagcaatgcggcatccagtgcaaaaacttcgcataactcagccgaccattgtttttgcgctacatcatacaacaatgtttccgatgcctgtgaatgctcataccgcgctacaccgctgagcataaattctatccagttgctgatgctgaggaacgtgctgcattgctgccacagttcgggcctgcgctcacggatgcccaccagtttcagggcagaaaacagggaggtaggataacgccctgtcagctggtacaccctgcttttatcggcaatggtgttttcccattcccggccacggtggtcgatattgggcaacccggtcagcgattcgccggtggcggataacagcacaataccttcgcgctgactggtagccgtaatggcttttaccaccgtgccgggaataccggagagtacctgcacggctaaacgctttacctgaagccatagctgagtaggctcaaaatacagggcatccgggtacaacggatctttgatgtaatgtatgtcttcccgggcaacgcttaatacctgtccctgcggggaagttgctgccacccttacgtttccggtgcctatgtccacaatgatgtaggtgttctgtgttgtcattggaaatgaactttaagtatgtctttgttggctaattcggctatgtgcctgttggcatgtgcataccactgcagcaaggccctgttcataatttcaacgtggtgatcttccacttcaaaggtggcgcccgcaatgtgcggggtggcaattacctgtggaaggtcaatgatcctgtaatccagttcgtccggtggttcatgatcgaaaacatctaagatagccccccggatcgattttttttccagtacttccagcaggtcttcccgttgcacgaccgaagccctggcggtattgataaatatggcctcctttttcatcattttcaggagccggccgttgatcatcccttttgtttctgcggtaaccggcaggtggatggatacgatatcgctggtagcaaataaatcttccaggcttgttttccggtaatcactgttgtattcggccacatacggatcgaagaactggatggggcagggatattcttttaccagctttgcaatcagctggccgatagcgccaaagccaaccatgccaatagttttgcctgccagctcattgcctttgaagtgcaggtaggagtcgtgcgcacctgcctgccagttgcggcctttcagccagttgatgccggggatggtattacgcaacagcatgattacattggaaataaacagttctgctacggcctgcgcattacgggcaggtgtgaagaataccggaattcccatttcagtggctttgctcactgccacgttggacggtgtgccgcggcatacgccgataaactgcagctggggattggcggctattacttttgcagtaacgtgatcgtgctctgttatcagcgcttcggcctgcgtgtctgaaagcatggccagcagctcgtcttcattgtatgcccttccatgaggcttccacgaccggtaaataatttctccgaactgccgctgcaatgtttccagcccctgctcatgataaggggcagtgattaagattttcatgtgtattataattgtatggtttccgttgtattgctgtaatgatgagatgtttttgcattgtccggcagggtgataaaccgggtgatgacggcgcttaccaggtaaagggccgccaggatccagataacgcctgcatcgcctgcgctgccgataaataatcctacaattgcagggcccacaaaaacaggtaagccggcgccgaggttcagaatagccattgccgcacctttgtcttttttcaccagggaaggtactaacgccgacaggggtacgtagcccgccaggcaggcgccccaaagtatgccggccgtcatgaccatccagaaattgccttcccatatctgtggtgcgtaataaaacagcagggtagtggctgcacatcctacgccgccgaaccacatgatagtattacgccatcccatgcgatcgcccacaaagccaaagatgaggttgaagatgatattggcggtgaagatggttccccagatctgcagccattgcgtggtttcgtagccatgtttcgccatatacatcggcaggaataccgggaaggcaaattgcgccgtggtattaatgatgcgcacaataccacccaataatactttgggttcttctttcacaatggtgagccccttgatcagttcttttacctgcgagccgccggcagtttctttcttaatacttcctttattcagtaccagtgcaaacagtgcgcccagcagcgcccagaaaactgaggtccataaagtattgaggtgcccgaagcgggtaatggcccagctggaatagtacgcgccgagtacattgagtccgccggtgaatacaaaccagaaccagcctacagcgcgacccagttgctgccgcggactgctgtaggcgatccataccaggaaggagtaggcgaacaaaggataaccaaatccacgcaatgcgtaaaagagcaacatcagcgggtagttgagccccggcatgccgtatccgacgaacccgatggtgccgagaatgtagaggatcaaacccgtgaacatggtgcgctttacgccgtagccttctgccagtacgccggaaaaccaggcggagatggcgatggtgatgccataggccgtaaacagggtggccgactgctgcaccgacatgccatgtgataccaggtatgggcttagccatccctgttcaataccatcacccatcatgaatatcatgatgccgatgtagccaaagagcagctgccggggcagtccggccttttcgaaaaatgttttgtttactgtggaattgttacctgataacatacggttgcttgtttaaggtttttcgttttatttaatttgcccactccgggtcctggattaagttgccgtttaagatgatttcgttgtatggaatgggatagaagtatttgcggtcttcgtatttgcgcacaaggttatcaaacagctgcagattgccgttggtaccgttgctgagcttgaactgtactttgtctatcaggaaataatatacgcccggtacttttgtcgccgggattttctctacaaaacaaacatccattttcccatcttcattcagatccatcagtgtgttgaggaagggtacatacatgccatcatagggcatggtgagcaggttgccgagatgccagcgcttcagatcatcgtagcggaatccttccaatgccagctcaatgcctctctcccggcgtatttccagcagtgccggatcatttataccaggaaaataatgttgctgaagatatggatctgctgtaaccggcggcgtggtaacggtgatgcccgcacgctgccgcagcggagcaatggtgaggttccagtcttccgtagtaaagttgccacgctctgcttttgcttccgcatagttcagcaatacttctgcataccggatcagtggcagggagttaaagttttctgccagaccatcggtcgctttcgcatccaccgccagtttgataggcatataacccgtataggtatacgtaaagtcgggcggcgttactacaccatcgcgggaatagttacccatgcggatgctttgtttcaggcggaggtcgcggttctttacttcctgtgcaaaagggattttattaaaatccgcttgtgcggtgaaaggcgtaccatccgtatttaaataggtgttgataaaagttttgatgaagctgtaccggccgccgtaagtggcgctggtccagtaccagttggcatcgttgaatacacggagacttttattattaacggccgccagcagtacttctgtgctgttgggtgtttcattgataaacaggttgcggtaattttgatcggtggagccggtagtcagcagtttatactggtttcctttgatcacctggttggcggcgtcaatggctttgtcgagccagtcgttcgccgtgccggcaagcttcagtttcgggtgatatttgcggatggtgccttcaaaaagacatacccttgatttaaaggcaagggctacccatcttgttacctgtgatgcgccgttatctttggtattacggatatggctacacgcatagtcgagatcggccagtacgttgtccattacaagcgtgcgcggatcgcggcctttgtaaagatccggatcgtccgcagcgaggcttttatcgtaccagggcacatcgccgaattgttttactttattgaaataaaaccaggcgcggaaaaagcgggcgagacctatgtaatgttctttggcttcgtctgtaatttttgcgttgccggcgtgttccaggaagtagttgattttgcgcagtgcgctccagctccagccagtggcttcggtggggccaaaggcgccgtagatgtagttggacagggttctgcccaccaggtaatcgctcagggcatctccccttacaatatcactgccatcgggcaaatccaggtaaaaggagttggcgtataactgcaggtccttttcggtattaaaagcattttcaggcgacagcttatcaaatggtttcaggttcagatcacggttacatgcactcatgatcatcaatccggcaaccaggaagagaatatttttcatgatcattttatttgaatgttacattgatccctatagtgtaggttttcagcataggataactcatcccgtttccggagccatcgttcagctcaggatctgagccttcaataacttccgggtccattgttttcacgtacttgtacatcgggctccaggtccacaggttctggccggttacgtaaatgcgcgcattggccataccggctttgttcaccagtgatgcggggaggttatatcccagtgtaatatttttgagacgcaggtaagctgcgttctgtaagtatttggattgtgttacctgtagttcggcgcgggagtttagcgcggtgtagccacgcatgcgcgggaagtaggcgtcgggcttttcttccgaccatacattgttcaccacatccaccggctgccagctgtaagggcggttataagcgccccagaacagggagttgtcggctcccggccagaagtctcttttaccaataccttgcaggaaaaaggagaagaagatattattccattccatgttgccggtgaagccatacatgtaacgcggggagctgttgccgataaccgttttatcgcccggatcagcgagtgagccggcgccttcattgatctttttatcgttgttaagatctttaaatttgatatcgcctggtaatattttgttggcggcggatacgcggataaagctctggtcgatgccacgggtatctatttcattttgatctttaaagtaaccgtcgtttacaaatccccagatatcgccgatctgcatgccttcatagtaggtgttgatgaggccgagtggattattgaagcgggtgatcacacttttattatcagacagtaccagtcgggcatcgtagctgaatggtttgctgccattggttttattcttccacccgatagatatttcccagccttttgtttccaggtcggcatagttgcctttgggttcggtggcgccgaatacaccggggagcggcaatccgtcggtgaacatatctttcgttttgcgggtgtaccagtcggccgtgagcgtgagccggttgttgagcaatgcgagatcagtaccaacattcagcgtggtcgccttttcccaggtaagtccgttgggaattacattgggttgctgcgtatagtcgggccggataccgttcagaatacgggccatttgcgttacgctcatggtttcgagaaacttgtaaggagcgatattgccgttgccgagggtgccatatgatgcccgcagcttcatgtcggataccactttataagggatgttccagaacttttccttggagatcctccatcctgcggaagcggatgggaagaaaccccattgctgcgtttgcgggaatttggaggtgccgtcgtaccggccgtttacttccaggaggtagcgttcatcgaagttatagttgatgcggaagaagccgccgagtgtgcgccattcgttaccgccgcctctcatggtgaagttgagtccgttggtaagggagaagtcgggcagttcattgttgatgatgccatcccgctggatgtacctgcttttcagcagggagttttcatagttatagccggccattaccttgaagtaatgtttacggtaggtatgttcataatcggcatagacgttggcggcgagatagtttgttttatcgtcgttttcgttgatcttactttcgccgcgttccagtgccacgcctggctttttgctgtagggcacgggcgtgtatatacgcgtttccacatcgttgagccgccagaaggtgagatcgccgtttacatgtactttatttttaaagaaggtagcggtaaagcgggaggtgttacggatctgcgcgcgactcagttctgactggttattaccggagataaagctgccaaagacgatggaagcgttttcggtgagtgtgccatccgggttgcggagcatggcgatggggaaggcttcatcggaaattcttctccacacgggtgtgttactgggatggtttaatatggggtagaaataatttgtttgagtgaagttgagatcattttccactttgagccacggtaacgcctgtacggagccgcgtgcccggaggttataggttttgaagttgtccgggttgtaacggaagatcccatcctgtgccatgtaccggccggagagatagtagctcacgtttttgctgctgccggaaagactgagattatgttccatggatggattgttatctgcatagagttctttcagccagtcggtgttgccgtagtaaacatattcgccggtagtgggattgatatctgttttaggcagggacggatcgtcgtttctgcgtttcagttcatcgaggtaatctaacgagaacgggaacacggagtttgctttttgcgggtgcgaggcatagtcgttccacgaggtaaatgcgtcgtcgaagtttttggcccattcgtaaccgttagttaccattttgggtttgatggttcgttcgttaatggagtagctgccggcgtagttgagggtggttttatctttcgccgggcttttggtggtgataaggataacgccgaacgatccccgtgacccgtatatagctgcagcagctgcgtctttcagcacggtgacgctttctatatcgttggggttgaggagcgaaggttctcctggtacgccatcaatgagtatgagggcgctgccgccggcgccgatggaggtggtgccgcgtacattataggtagcgctgcgggtaggcttgccatcggtcatacggatattgagattgggaattacgccctgtaaaccacgggtaacgctggtgagcggccggttttgaaatacctcgctgcctacctggtccaccgcaccggtgaggtttactttcttttgtgttccataacctactactaccaggtcctgcaattgtttggcggaggaggtgagctggaggtcgatggtgttgcggttgccaacggggagttcctgcggggtgtaacccacaaaagagaactggagaatagattcgttaccgggtacggccagctggtagcgcccttctgtgttggtggtaacgccggtagtactgcttttcactcttacattcacaccgatcagtatttctcctttgtcgttggtaacctgcccctgtactttccgggacgtttggccggataatgcacacggccatgcaagcagcaggaaacagagcatgtacattttgtacatagctgtgcagcttaagtgattcataactggattgttttgttttggttgacccttttttctataacatgaaattgtttgttgatatccgttacccgttgattcgtctgaccttttccggactgatggtggaattcatgaacgttggaacatacggttgcgcaatcgatgttacctttaaattaaacaaaatttaattaaattaaagtaaatgtaagtaaactatttaatctttttaaatattttttaagtgtagggaaacgggatggtttccaggctaacagggagttttaactataatggtggctgttgtatagaaaaggacagtagagtcttgattaataattttatatttgatgaaagaaatttaaacataaagaagaaattcaactttccatgaatattacagacagacatcagcttatcctgcagaaattgcaggaaaacgggaaagtggatatccaggaactgagtgatgccttgcaggtatcaggagtaaccatccggaaagacctcaaactactggaagagaaaaagttattataccgtaccaaaggaggcggatcaacgcagaatccttatacggtggagcggccgatcaacgagaaagagtttatcaaaacggaagagaagaaaaagatagccaaagcagcggaagcgcttatcgggatgaatgattccatcattattggctccggcaccaccgcctttgagctgacccgttacctgcatccgtcgaaacatatcacggtaattacccctgcgctgaaagtggcgctggaactatgtaaccgcccctttgtagatgtgttgcagattggcggcctcattcatcaaacctcttcttcggctgcgggttcctttgcagagcggctgctggatgatatttcctgcggggtattatttatcggggtagatgggattgatatggaatttggtctttctattacaaacctggcggaggcgagcctcaatatgaaaatgattaacctggcgcaaactgtggtcatcatggccgacagctccaaatttaaccgccgtggcataggtcgcatctgcagccttgaacaggtggattatattattaccgataacctggtatctgcagacaccgtgaaaacgctgaaggagcacggcgtgaaagtaattatagcagaataacttgttaacaccactacatatcaatccgtatggaaacaaatcacaccactactttactccggcatttcaatgaaaccattgaaatatggattacttacctcaacgactacacgttagagatgctttgccgcaaaccccgggaagacgcctggtcgctgggacaggtgtacctgcacattattgccgataccacctttttttatgagcagatgaaagctgcactggtggacaatgccaaccatgaaaaagcaatgcataaacatgccaaagccatatttgcaaagaacgacttcccggatatgttggtcgaaaacccgtccaacgacccttattcaagacaaccacaaaataaagaggagctgttgcagggcctgttgcgcgtaaaacaagccgtgaataccttatacgctgcaaatccctcaccggcaggcggaaaaaccgaacatccgggtttgcttttttttagttcattggaatggcttcagtttgcagagatgcatatgagacatcatctccggcaaaaaaagcggattgatgaacaactgttccccggataaaacaaacggggaacaaaacagctatcattcacctgaaccgggaagaagctctacttcttcagggatcacgaagaacaggacacagccggttttgctggtaacggagtgccggaagcctggcggtgtgtacaggtagtcgcctgccagcagtgttgcatgttcgagcaccgcatctccactcagcacaaagatctcttcaccagcgggatggttatgataaggataatgcgcaccgggttcaaatttgagcaggatggtttttgagcgcccggcggcttcgtcgtaccggagcgacttcacgaatattcctttgtagtgaacatttttttccacgagaggctgccattcagcctggttacttttagtgatgtagtgatggatgtctgtattcatgatcttgtttttatttggtgaagtattgatccatgctccatttgcttggaggcattgttgctaaaaggaaagcggctgcgctgaaggtgaaaacggaatagtccaggggttctttcagcccaaaggaataggtcatggtgagcgcaaacagcagggtgagtatcatggcgctgatggctgccagcgatgttttgaaccccagcaacagtaaaatacccaataatgtttccaggatggtactggctactgcgagggcagggaccagtttttgcggtgcaaatgaatttacctgtgctgtatactgcaggaattttccccacccggatgactgttgcccccataaccccagcctgcttgctaccgcggataagaagcctgttgccagtgcaaggcggagtagcagggaagcgatgtgctgataagatttcatgtaccagttgtttaattgttaacctgatacaaaggtgcggtttatagggaccccagggaatagagaatcctgcaaaaagcatgtaatatttaaagcgagaattgttctttatacagttttggggagatttctgtttgttttttgaagaagttggaaaagtagaagggatcgttgaagccgagcttataagcgacttcttttacggacaggtcgccataggtaagcagccgttttgcttcagaggtaacgaggccataaatcacgttctgggctgttttgccggcatggagttttgccagttcattgagctttgcttcggtagtgccaagcagtttggcaaattgcgcgaggggatagttatgctcaaagttatcccttactgcttccaggaatctcaggaagagggcttccggtttccagatttcatcgccacgtttcacctttgcccggttgatagataccagtatcagcgccacgcggctatgcacagaaataaggtattggtaaggctgctcctgtaattcttcccggatgagggtgagttgtgtttcgacgatctctttatccacggggattacttcattcatggcgaagtggcagaaaagcccgttgtgaaaaatcagttcaatgtccttatcatctttgcagaaaaagtccagtgtaaattccagtacaaatcctttggtattttgaagcggctgaatgcagtgtatctgtccggaggtgatagtgatcacatcgcccggattcaggtcaaatgcggtatgatctacctgtacatggagctttcctgatgtacagtataccaatacatacttcatgatgcgccttggcttgtcggggagcgggctatggtccaggtcttttatttcaatcatcctgcgtttgggtggttgtgataccgaagatagggttttaaacggtaacaggaatctgtgtatttcttttttaaaaagcttctggtggtaaatatttttatacgcatttacaatgcgtatgggaagtggatttttataaagacaatttctttattgaaaacccacaaataaattagaaatgacgtttcaaaatgtaaatgaattgaaggcaactgccggcacaacgaatggggaacttagccatctgttaggatatcttgaaccggccgatggaggagaaggggtattttattgggatagcacttcttcactagctgccaacctgggtactatatttgaggtgacgggcagtccaggcagatggatcaggaatattgatggcaatatcataaatgtcctgtggtttggcgctttaggaaatcctgctgttgattcaaccaatgcactgaaggatgccgtcaaggtagtaaatgcctactccgtcacttcgcctgatccgggtaccagctattatgggaataagcctacattgtattttcccaggggcgaccggtatacctgtagcgctaccctgaatatcggcgcaggtgtgaatgtggaaatggaggcgccggtgagttttgttgaccccactgattcactgccaggcatggtaataggaagtgacggtgcaagtaatgcatccgtcaaactcagcatccggatcgtgaaagaaaccatatcgggctggacgaatgaaagctgtatcggcgtaaagcttattaaccttttatcatcaagattaaacctggaatttgtaagttcctttaccattaacgcgcagctcatgggtagtgtgcaatgcgcctacaaccgggtggggatagggacattgaaagatggcaaaatacagctggatctccaggcgtcgggaacagacgggttttgtaatgaaaatgtttttaccggcggccggtttgccgtaaactcactaagcggcctggcgaacaaagcaagatatggtgtcaggattggcatgtcgggaacaacagcgcatattcccaacaacaatgtattttacaaacccagttttgagttgagcgcatcatacataactgatccaaccgttacggaatgccgtgccgtactaatcaaccggggaattaataaccggatatgggatgcaagaaacgagaacagtgggaagtgctccctgaagatcactggcgaggatagtgtgcagaacagtgtttatatcgggtacaccgacttatctgccaatgaggtaaacaatgccgctatccagatagaggatggaagtaaggcccgtaacaaccgggtggctaactatccgaactattataatgacgctgtcaataacagcaattgctggcaatcacttttcctgcccctgcatatcaacaggtataacgctaccagttactttttcaggggattgcactgcgccgataaagccagcagcgctgtgttaccatcaaggctcattgcaggggtaaccagcagttacgtggagatatccgggaacaccggcataggcgtttttatcaatacatcgtctgcgaaaaagtttattgtaagaaagaatgtggatacaggcttcggaggaagggtatcggtggtttgctacgacagtgcaggcaatatattgacgcctgtaatcggcgccaacctcttttcaccacatttgacaatagttaatacagggcaatttggagggtgttacctgaacaactcagatgttgaatacccaaccagctttaatgtagcggataatgtagcgtttgtaagagtaatattaacatccgggacagcgaacctgagaataagatcattttccgtggctacacttgactttaaacaggtaacagcttataccggcctggaggcagcgggcatagatcatcatttatcttatgcagcagtggtgccaacagaagtgaaacccaaaggaaccatcatttataacgactggagtataacaaccggtcatctttgctggagaaatgcagacggaggtactacctggacggagctataagcaggtagcggtatttcaacgcccgtatgcagcgggcgttgaaataccggctctattccgggcaggcgggaaaggcagttgtttgcagcgtaaaaaagtgaggcattgttttttatcacactattttagggctactaaataattattattaattttcagtataaaacattacgatgcgccatctattcaaactatgcctgttactcgccgtttatttgccagccatggctcagaaacccgccaatgaactacattttaccagcagtcagcagcagctgatcacggtgtataaaggaactatttttgtgaacggcaataaagcttttgtgcttcatgaagatattatcaactacaaaagtaaacgcaaccgcctggtggaaaacggtaaatccgtttttctcttcctggaggtaaacggcagcccgaacaagaacaggctgtatgtgtttaatatcgaccactccctggcagattccctgttgagtgcagtgagctcggatgtgaaagactgggaccgcgatggtgacctcgaattcggcggcagtgatgttacaaaggtttaccccgctgccgattcaatgtattacgttccctcgaagttctatgaaataaaacgtggtaaaattacttatgacgccgagcttacggaaaccaccgacaaaaaagtcaatggtattttcctggcctcgccttcgaccagtacggtaatacctaaaccgaagaaacggtactagccggaattagatttcggggtcgttatttttctcccgttgctcggctttccagataaggaggtcgattcccgacaacccggaagggtgggaggaagcgtcttccttatctgttttttctttctttacaaccggcgctaccggtgtcagcgttttgaaatcatttgcaaaatcagtagttgcgggccggttattttcccagaacttcgacaggaagtttaatgcttgctggggtgtatctatcttctcttcttccttcagcaattccagcagctttaaatcgaatctcaccggtaccggtttgtttttttcttttgccatagtgctaaaggtactaccttacccgcacaccaggaaaagatatccgcctggcggcagcacctaatcacttcctcaatagatcttcttgccgaaattatagatggccgcaccggacaacagtgaaatgagcactgccagtgaaagcacacctggccagatggcgccggtgccgttttcattatagcgctttaacttaaactggctccaatcaatacttttaaccggttggtcctggaaaatggccggataaaaatacaggcgtagctgttcatgataattcctgatggcctgctggaaatccaggtgctgctgaagatcggatccggcgattccattaagcgtaagctgggtttgaataccaggaagaataagcgccactgcagttgtaaaatcgttcctttgtgccagcttttgtttcatagacctggcgcccggtgcggcctggtcatcgccgttttgctgcatggcgaaataccaataccagctgaacgccagttcttccgggaacgggtattttttaaactgcggataatgccggtaaaatgaggtgagagcaacgcgcttatccatatcccatttttcgtggtatccttcccgttgcatcaccacggtttctaacgcttccggaatgggatatttccgggtaagccaaacatttaccaaagcaggtgcgagtatgttcagcactacccagcatgaaatgagcgtcaccgcattaacgctggaggactttccccgggagatgacccaaaaggagagagcaaaccagaacagcaggtacaggcttaataccacgattaccgccagcaaacggagatctgctgcaagccggaggtaaacaatcgccgcagctattaataccaacgctgtcaggtaaacggtactcatcctcaccaggaacttccgccatagtatttttagaggaacagccgattgggaacgcagcagcccccaaataccggactcctgttctcctgaaagtaaattatagctgaatgcaatgatgatgagaggaaatatgaagataaatacaaaagcaagatccatattgccgagtaacagcgtggaaggattgttaagatcggtatcatagagctgtccttccaggcccagggtggtaaccccgatgagataaggattgatgtcgcgctggccattggaaaatgccgcccagttgcgtggcatgttggccatcgaaaatttggtatgatataacattaatcccagttctttaccgaagtatttaatattcctggcggtattttctgcctgtagtttttcggctttgacaatcacttcctgctgcctgtctataaaattctttccaaaatataacccggccaacccgctgataagaaggatcagtatccctgtcaataccgttttattcctgaaaaagatcttgtattccaattgatatatatgctgattcatatttgctgttataaagttttaacccattttgctgacagcagcaggcatcccaacaaggccgccagccagcagagtaaggaaatgatggtgctgatgtgatgtgacattacctggtcaaccggtttaaacacatacttaaaatcggcctgttctgcccagtgcgcccggctgatggttaaaggtttatctttttctcccggtgtggtgttgctgattttatctttctgcaatttgttcatacgctgggcgagcccgtagcggtaaacttctgcctgatcctggaaatcagcaaacgtgttgaagtcggaggcggtcagcgccatggaaaggttctttatagccaggaacgggttcaggtagccggcagccacctggaagctgttctgctgctcaaatgttgtcgtcagcgctttctgatgatgggtataaatgccggcggaaattctttctccttcggccatcacatagccgccgtagttaaagggcaattgtttcacatcacttacgccatactgttttaaaacatctgccctgaatttcgcatagtgcggatcgtccgggttatggctgtcgccttgctggtgcaggtctgattcaacggcagccgcaaattcaattttcgatggagaggggtacactttaacgccgatcgcctgggtaatccgcggcatcacaatagtgaaaaacacccaacaggccagcagcgtagtaagcgcggccctcgatgttttgtgcaccgcggataccactacggcaatgccggtgcagatgataaagtataccgcgtaagccagtaccagtaataaaagacggatgcttgcatcggccgttacctgccagtgacttagcattgcccacaggaaaatggtgagcaaaataaccgggatgaaaagtgtaaagctgacggcaataatccctgcaatttttcccgttagcaatgccggccagctaaccccctggcaaagcagtatttttaaagtaccgttttcgcgctccgcggaaatactgttatatcccaggaaaaagatcagcaatggaacaagcagttgtaacaccatggctacactcatttccccgaaacggagcatgccattggagaagccagcttcgctgaagttgacggtattttgtttgtgcgcctccaggaaaatggatacgcccgcaaagctttcaatgccaaaatcaaagaagctcagttcatgtttatcacggaacgcgagatagccgtagtgggccatccggtgcgggtgcttatctggttttgccagccattgctggcggacgatttgtttatatttcagccgctggccattctggatgttgaagttctgccacccgatgtacatggccaggcacaatgccagtccgaggatcaatgtgaggcccagcgtggctttattccggaatgatgctttccaggtgctgcctgcaatcaaaaaaattgttctcatgcgatcagaatttataggtagcgttgaacatcaggtttctgggagagccggggaacaggcggagataattctgcgcgcctatccaataggttttgttcaggatattgcccacattcaatgccagttgtatccttgttttagccggactgtaatacaaagcggcatccagtaatgtatacgccggcagtgtgaaatcgcggatataccagggtagtttgttaccactgtattgaatgccggcgccaaagccaattccttgcagcagcgggtgatcgtccaggtcgtaccgggtccataggctgccgctgtgttttggcgtgttttgtacgcgttcgcctatgagtttggggtttaagtcttgcaggatgatggcatccacgaagctatagcctgcattaaattgccagttgggcatgatgaacccggaggcttcgagttctattccgcggctgcgttgtgcgccgcgttccaccagccggttcacatcttccggatcgttggcattcatcagcaaattcttctggttgatttcaaaaaaggaaatgttcaccatcagcagatcattcagccattcagactttgccccgatttctttaagatcgctttccagcggtttatagttgacgcctgccggcggaggtacaattaccagcgtggaggtattgccctgtggctggtaaccgcggagataagtactgtacaaattaatattcggagagatggcatagataaggcctatccttggcagcagttgctgttgggagatctttttttcaccgggaagtttatagttgctgaaatcttcataccattcctgccgcaggcccagcgtgagggtgagctgttgataattcacctggtcctggatgtatacgccgttaacgagataataggcaggcgggatctctgttttattgaaaatataatcgcccaggttccgaagtgtataaacgggactggcgaggttgaagaagtcgacattaggaaccggtgcatttacgccgttaattgttttaaagagataggcatctttctttgccggatcgtaccgtgcagcaatggttccgtctttcagccggtggccctgggcggaattttcgccgccgccacggtacttctgtgtgttaatacgatcgtatcccgtcacgatcttgtgatgtacagtgccggtgctggcgttgatactgaagtaagcgctcaggttatccgtattccatttctgttgccgttgtacagcgcgcatagcagcgagggtagggatagggagattgttttcatccacgccaaaagcgttggtggtgcggtgttcgagcaggtcttcattccaggtttgcttcatataggcaacgttgaaaaccacttttgatgtaaaggcatgggagccgctgatcatcagcatcaggtcctgtgtattgaagtaatcgttgctggcgcccatattaaaactgatgggggtgctgttgaggtttgtttgcccggcgatagccccgaatattgcctgtccgcgatccagcctggagttgctgttgttcatcaccagctccgcattcagactggtactttgattaggcacataggaaaaggatggtgaaaccaggtaggcctttttgtattgcaggtcgcggaagctcttgctgttttcgtatcctatattcaggcggtacagcaatgttttttccttattcagcgggccggtgaaatcgagggcagctcttatgctgctgaagctgccggtggagatgctgacctgcttcctgttttccgtgagtggttttttggtcaccatattgatgctgcctccggggtctacactggagaaagtagcgctggccggtcctttgatcacttcaatgcgttccaggttattggtcagcggttgattaaaaaagtactggcgtgtacgcatgccattgataatagcgccttcttcgttctggctgatgccgcgtatggcaaactggttgtagtagctgctttgggaaacgcctgttacatttttcacggcgtcggccagcgtggatgcctgccggtcggagatcagttctttagataccgaagaaatagcctgcgggatatctttgttggcagacgcgatctttgtggcagagaaggagtagtcgccataatatttttgtgcgttggtaccggtgatttccactgtttgcagttctacctttttcctggaggaatcggtgaccgcatgcagccgggtggtgtcgccggcctttgtctgggctgttgccgccgttgataaatatataaagcctgctgccaaaaacaggtttttggccattggctgagaataaagaaatttcatgaagtgtgtaactagatggtttgtaagtatagttcctgtagatcgcgggcattgatatcgccggcatttaaggtatgcaccagctgacctttgcgcatgatcccaatacgggcgcctacattaacggcgttgaatatatcatgggtggccattagcacggatttgccctgcctgccgagttccctcaccagccccgtgaattcatcggtggctttaggatccagtccgctggtgggttcatccatcaggatcacgtctgcattttttgccagcgcgatggcaatgcctaccttttgccgcatgcctttactgaatccggagagatgtttatgatgcgcttcctgttgtaagccgcaatcggagaggaaggtggtgagcctgtttttatcatacttaaaaccggccagccggctgaagtagtccaggttttcggtggctgttaagctgccgtacagcattaccacttcggggatatacgccaggtgtttgcgtgtttcggcgtcaccgggacgcacttcctgctggtggatcattaccttccctgatgtgggcgctgtaaagcccaggaacaggttgatggtagtggttttgccggcgccgttctggccaagcagacaaaaaatttcacctggcttaacttccaggttgagattgtccagcgcaacgtgcgactggtaatgttttgataaagatattgcctgaagcataaaaaagaatataagcagcgatacaccccccggatagcgggggcggagaaatcaggaaccggatgttacatccggtagcagtaaatgatttaacagaaagcgggaggtcctttatttgtacaggagagcagatagcctgaataggcctgtacgcggaaaagtgaaacggttgtttttgtaaccggggaaatgaataccaggggaggtagttgtgttggcaggaaatgatgcgactggtgttttatcagatcgcacagcttacactttacatggatagtatggaactgctgatcaccggtaggggtatgttttttcaggatcagttctgttccggccgtgcaatgatgatgatggaaagcctctatcagcggggcactcaggaatataagcaataggaatatggccccaatcctggagagtagctgaaggcggtatttttgttgcgtattcaaaatatgcaacgaagttacaattttcattaaaacggcgaaaggtttatttttttaagagcgtaacagagcgggcgtataattaagtgatggtgtatttgaagatggcctgagcaagagatagcgcatactttgcaattgcctttgacatgctttggggatacttgggagatgcctttgctatggagttgacgtggggttgatgtggaggtgacgtggacttgatcggtaaggtattgaggatcaagattttgcagagggttttgccgttgtgtttagacaaacagcaaagagaaaaatattggatgtcaatgttttatacatgtttcaaagataaacctgatcagcgaaaatatcaaaaaaaagaggttgtacttttggtacaacctcctgcaaataaaattcttttcttctcttttatcagttcttaagatcaaagctgataaaaatattactcagcgttgcgagcaacgaattagcgcttgttggcggtgtagtacctggtgtgccggtgtttcctgacgcgttaaaagagaagctattgatggtgctgagggtggccagttcgccggtagccggaaagtttgttaatgaagcggcgccttgtatcagcacatcatttacccacaggttataggtttgtgctggtaatgcataggtggaagcgccttttgtataattctctcctgcactgctgttattgcagtataattcaattttataatttcctgttttattgaataccgtattgttgatggtagtatagccgtaagtagcattgcggtaggagagggtggcaaagttgccgccgtaaaagtcgaggcggatagcagcgaaaacgccgggtgtgctaacagaagtcagctggttggtgttattaaaggtactgctgctggtggtgctgtagccaaatggaatgatcagctggccgtttgttaatgcagcattgaggttgagattaaaagtaagggcagccagcggtttcgcctcatcgatattataccaggaaagttttgccggggtattggtagaacttgcggcgacttttaaactgggaggactggcgccgggctgcaattgaaagtatcctccgcaggtggccggcagaaatacccgtccgtagccatacggtggagcggggaggaagccgggtgttccttttaccgaaacagacgctttagcggcggtagaatcagcgaaggtagcggaagcaggggcgctcagatcaaatttccaggtgatgtagggatgctcccaacctgtgctgctgtttattttgtcgtgaattgcattcagcagggagagtgatccggtggcgtcctggagcacctgccagaacatgatgccgccggcttcctgctgggcatacgccgttttattctgaatggtgggtatgccgttgtagttaactatggcgccgtctggccgccgcacggtgtctttgttttcagcaccggggtattgtgcggtgatctcgctgtacttcatggattgtaaattaccggacagggtgtatagcccgtaaaaaggcacgcccactactattttagcggccgctaatcctctttgtcctttccagtattccacgtgctgtttggcgtagctgtaaggcgaatgttcgtcgcccgctttgtcgtatgccatcacgttgataaagtcaaaggcagcgagacaggaatctgttacacggtcgcgtgtccaccaggcaacagctgcggtcagtaattttccgttgggtttgagttgagtagacaggccggtaataaatgcttcgtagttttcatcgatgttatctccttcaaggtctacatcgatgccatctacatggtattgtgatacgaggtttaccactttggtgatgaaagctgccctgttggcggaggtgagcaggttggcatactgactctgattggagccgccaccgagcgacaacaacactttaacgttattgagatgcgcttttgatacaatggtatccagcccggtgccttgtgatgcagggaagttaccatttacatccgggttaaagaaagcgatattgaggtgggtaactttggagaagtcaaaggcattgatatgatctgcgagtgtagaagtatatttaggcagataggcgactatcttaaacccggtttcttccagttgcaatgcggacatatgcgccgttttgccggcgttaagcatataccggatttttgtgcagccggaaataagcaatacaagaagggcggatacgactagtttttgtttcattttttttggtttaaatgaacggtaaataataagcggaaatatttgaatagttgttcctgtcccggtgcagcaataccgggaaagagcgatctggttgatgttttacattagcatgccatcattgttatgccactaaagaagtgatataatgatgcagcagggaagctgttttttaaaacatgcttcagtaatgatgggagatgtattttttgggcgaacggttttttacctatatttcgtgtacgtacacaaaaatagtgtttatttcttcatatccaagttttgcgataaaaaatatcaggatattgttgtggcgggcaacgcttatatatgaatagatgaaaacaggattaaattagtatttttgatgtattaccggctggtatagcaggttttgctgcaacaggcataacttcgcagctgtaagccgaataattgaatgttcaataaaccagttaatgaaagatacaaaagaagcagcattggtaggcgtgaaggaaattgccaggagggcgaatgtttccataggcacggttgacagggtattgaataaccgtaccggtgtggcggagaaaacgagggaaaaggtactggagattattaaggacctggattaccagcccaacattatggcaaggcggctggcatccaagaggcttcttcacctggcggtgctgatcccggcggcttccggtgaaacaggatactggaatgcgccgctgaatggaatcaggcaggcggctgccgcgatcagggacttcggggtaactgtggaaatatacttctttgatcagaacgataaaactacgtttactgccagggccaatgaaattttaaagaaagaataccagggcattctgctggcgcctatgtttgaagaggaatcgctgggcttcacaaaaaaatgccgggccaagaagatcccttttgtatttattaactcagatattgaaacagccggaagtcttagttacattggtccggacctttaccagagcggttacctggcggcgcatctcatcagctacctggtgagggaagggcagcaggtgctgattgtgaatatctccagggaaatggacctgcatcaccatttgttgagaaaggaagaaggtttccgtgcatactataaggcacatcctgcggatatacagatcaggaaaaccgatatccggcaaaccgattacaagtccgtgaaaagcaagttgcacaaggcgctgggcaaaacgccggtggatataatttttgttaccaattcgagggtggctaccgtaggccgttacctggaggaagccggtctggcgcacatcaaactgataggctatgatttcctcgcagaaaatatcgactatctcaaaaagtcggtgatcgatttcctgatctgccagaaaccacaggagcaggggaataagggcatcatggccttatatgatcatcttacacatgccgctgtcattgaacggcagcagtatatgcccattgatatcattaccagggaaaactatctcaattacaggaactaaccctgtttttacttctccagaaaaaaaatattttacgatagatagcattttctgaattttatttctatattcgtgtacgttaacgaaatgacggattttgtaattcctttatcgcttcgttaacgtacatggaattgtgcttttggggcgattcctcttttttacctttttttcgtgtacgttaacggtcttattttcagccatcgttttttaacagcctgtatcatttcatcgttgttgccagggagtattcagtcaaccaaaatgcgctacgctttattccggataaagtgaagccgggcgggtatttattgatcactgctgtgtacctatcgaattaggccagaaccaaaatcactaccaccatgaatgcaattgtcaagtttaaacatctgtacttatgtataacgatgttggcggcttcccggcactatgccgctgcgcaggcgcctgctgttataaaaggcatcatcaccgatgaaaagggcgctgtgattcccggcgccagtatcttcaacaaaaacagtaaggaaaccgccatctcagcgggcgatggggcctattccattaaagccgccggcggcgacagcatcatcatccagatgattggttacgagcgtgccggttttctcaccagaacacaacgcctcatgaatgtgaagctgctgtcgcgctcagaaacattgaaagatgtggtggttaccgcactcggcatccgccgggaagaacgggaactgggctacgcattttccgaagtaaagggagaggatatcaataaagcaaaagaaaccaatgtgatcaactccctggcaggaaaagtgcccggcctgatcatcaacagcaccgcgggaggtccgtccggttcgtccagggttatcatccgcggaaataccagtatcaccggcaacaaccagccactgtatgttatcgacggtatcccgatggataactccaattatggccaggtaggcgataccaagttcgcagaaggcgtggacatgggcgatgccatctccgctattaatccggatgatatcgataagatcagtgtattgaaaggcccctccgccgctgcattatacggcagcagcgctgccaacggggtgatactcatcactaccaaaagaggcgcgaagtcgaaagaactgggcgtggaactgagcagtaccgctactattgaaaaccagcttacaaaagttgatggcaaccaatacctgtacgggcaaggccgctccgggcaactgccactggatcaatcgcaggcgcaaagcactatgttcaccaactttggtccccggttggatcccagtatccattccattggattcgacggcgtaaccaggccctatgcccttgcaaaagataatttcggcagcttcttcagaaccggatcttctttgaataatacgttgtcgctcaccaatgccaccgacaggtccaatttccgcttctctgtttcagacctgcggtataaagacatcctgccgaacagtgatatccgccgtaataattttactttcagcggccggtctaaattcggaactaaactcgatgtggatgtaagagccacctatctgaatgaaagggttaacaacagggcaggactgggagatgcacccaccaacatcgggcaaaactttaacggcctggctaacaacatcgatcaatctgttttttccgatacctataaatccgcacagggcgagtacgtggaatggggtggtggcgcttaccgcctgaatccttactggatactctatgaaatgtcgaatgttacgctgaaagacaggctcaccggtgctttcaacgccacctatacggttaacaactggcttagtttcctcgcaagagcttccaccgatatcactttcctgaactaccggaaatacagtccgcgtaccacaccgctggcgctttcgggtatgatgaatgtactggaccagaagtattccactacccaggccgatttcatggctaccatcactaaaaagatcacacccgatctcaatttttctgcacgcctgggcgccagctttaaccagcgtatcaggaaaggcactaccgctacctattccaatatgacggtcacagatgtgatcagcatcaacagctaccaggataaaagcattgaagaaaataacctgcgcagggagatcagatcggcgtatggactgttcacctttggctataagaattacctgtacctcgacgctacggtgagaacagatgcttcgtcgaccctgcctgaaaataacaacgtatatacttatccctctgtatctgccagtttcatttttaccgatgcgtttaaaatgaagagcgatgtattatcgttcggtaaactcagggcctcctgggcggaagtaggaaacgacaccgacccttatatgctggatgtgtattacagtctttacccactcgcattcaatggggtgcagccggctaacctggccacgaaaatattaccaaacattaacctgaaacccaccaggacgcgctcatttgaggcgggcactaacctgaagttctttaatggccggcttaatttcgacgccacctattatacttcccattccagggaccagatcaatattgtgccggcgcctatctcttccgggttcccaaagcagatcatcaatgccggtatgatcaccaataagggaatagaattgttactgtccggcacaccggtatctaaaaagaacttctcctgggatcttacattaaattttgcccgcaatgttaataaagttgaatcgctggcagacgatgtaccgtttattgctttatcagaagcaagatggcttggcctgctggtagccgctatgcccggtcagcaatacggcgctatccttggatacgactaccagcgcgatccggacggaaacattatccttaacccatcttccctgaatcccatgcctacggccgacagaagagtattgggcaagggcgtgttcgactggaccggtggtgtgatgagcaggtttacctataaaaatttcagtcttaatgcggcattcgatatcaaatacggcgctgatattttctcgatgaccgacctgttctccgtggtaaggggcagcagcgtgaaaaccttgcccggccgcgaagaatggatcctgtccgaacaggaaaggctcgccgcgaaaaagacgccggccgaatggcaggcggcaggaaacgtaaaaggatatgtgcctgaaggtgtagtgcaaaccggcacggacgccgggggcaaaccggtgtacactaaaaacacgcgggcagtggatccttctgtttactggggcggcttttactccgatggtaatggtattgcggtaccgtttatttacaaggccacctatgtgaaggtgcgggaaatcacgttgtcttaccgcgtgccgggaaccttcaacaggaggttgggcatcaaagatgcttcggttggtttagtagcgagaaatccttttatcatctataaagatattcccaacgtagatccggattcaaattataacaacggtaacggtcaggggctggaatatggatcacttccatcaagacggggctggggaattaacctgaatgtcaagttctaatcaatcaaaacatgacagacatgcacactaaaagcaatcattcaatgagatatatactactggcgctgttgctgctgatatccgcctgcagcaagttcggtgatctgaataccgatcccaccaagtccagcaaaataaaccccgagaaccagctgatctttgcgcaattgtggttctccggagacctttccacgcaggaacgtaccaacagcattgtgctgatgccgatgatgcaacagctgggagccgcttattatgcaagggtgggaggcatgtatatcaaagacattacgcggatgtgggtaatgtgggaaaacagttatcagaatgatgtggtgaatatagtagatgccgtggaacgcaccaacggggtagcatcaaaaactaatctgaatgcgatctgccggatcatgaaagtatatactttcgccaggttaacagatctctatggagatatcccctattcccaggcaggcagcgcattttacacccaggtgaaacgcccggtgtatgatctgcagcaggacatttataataattttcttgaagaactgaaagcggcatctgcacaactggatccggctaaggacaaagtatccaatgaaattttttacaagggggatattgttgcctggaagaaatttgccaattcgctgcggatcaggctggccctgcgcctggtgaagcgtgatgccgaaaaggcaaagaaagaagtgcaggaagcctttaatgccgatggcggcgtgatgatgagcaacgctgataactgcatgacgaagcacatggatatccagaataattattcagacctgcggggtaattctgtgtcagccgccatcaatcagcagagtgccatgccgaagctggtgacgactttcctggatcagctgaaaaataccaacgacccgcgggtgaattacattccgcgttgttacaagcagaacgtgccgctgaagccctttgaaagggaagatattaccgcgcaggtaaaagccagtgtgctggggctggtgggatcgaagcccgggaaatatgtgtatgacgactgggtaggtccggttaccgtaaaactcgccaatggcgccaattataacgcagtgaacggtgatttgaaatgtgagatgaatacttgttttatgcgcaataacgctcccttcctgcatttgacctatgcagaagtggagttgttattggcagatgcgtccgtgcgcctggggctcacactgggagcggatgcggctacgcattatcagaagggggtagaggcagccatgaaacagctgagcctttaccccggcgggccggtgatccccgatgcggaaatagcggatttcttaacgaataacccgctgcagccgggcacggaattgaagcagatcaataaccagttgtggatcgctttgatgctgaacgggccagaactgtttgccaactggcgcaggaccggctatcccgaactggtagctactcccaacaatgaatccacctccctgacgataccgcggcggtttcagtatccgttatcagaaaaagagcagaacaccgtgaatgtgcaggctgccattgagcggataaacgaagatgactggctgaagagagtatggtgggacaaagaataaacatccaaacacaggaataaaaatattaactgatgaaacgatccatttatttattgctggcggtttgctgctattgtatagcaggatgtaaaaaagaagaagcggatgaacagtccgatggacggccatttacaccgcgcgtattcaatgaagcggccctgttcccggaaagccgcgatagtgtgagggtgttgatgatgggagagcaactgcccttcaccggcatgcaattttctcccggcggcaaagtggctatttcctggaaggtgaatgataaagaagtgtccactgccgatacctttgccttcaaggccaccaccggcggtgctttccgtataaagctcgatgtgtcttatgaaggcatgaccaccagccggtaccgcgacgtttttgtagtgccggacacctatcagaaaaaggcggctgccggcgttgtgctggcctacctgaatgatacggccggttataagtatatcgactggaacacgatcacgcacctggcttataaagtagccactctatcggctgcaggcgtgatggatatctcaaaaggggagccttaccggaaagccgaagagctgacaggcagggcgcatctcaacggcgtgccggtgctgctgagtgtaagcggcgcattgtcgggcgacggatggagcgtaagccagagtaataattttggcgccgtgatcaccgatgcggcaaaaagagcggcactggtgaaggccattgcaagttatattgccgcaaagaaaatggatggcgtagatattatgatgaccgacatcaacgcttcttccgctattattaatgccaacattgcggcaacgggtttgttattgaatgagctgcgggcagcactgggtgcaggcgctattatttcagtaacggtgcctaccaatcaataccacgaccgttacccggatctctccgccgccacctggctgaatgtgcatgcctttgaagatggcgtgcatgtagggccgggtaaaattccgggccagccttcaggatatgattattttgtgacgggggcgttgctgtggaaagcgaaataccctgcttcaaaactggtaatcggcataccggcgttcgggctgaggtataaccagctcgatgcaaacgggaataacctgggctggtcgtcgtacaactatattccttataaagatatcctggcagcagtgccctcagcatcagacaaggagtacgcggatatctccaaaggggtgtattttaatggcctgccattggtaacgcagaaagccacttacctgaaacagaacggcttcctgggcgcttatatctggacaggcgattatgacgtacaaggcgcgaattctttaacaggtgctgtattcaacttactgaaatgaacacacgtaaataataaaaaccagtagtatatgatggcaaagcgggtattaacagcagtgtttatattggtcatgtatctttcggtgaatggccaggcggatactttccgtgtgaaaggttttcatctcgacctgcgcatacaggtgatgaaaatgccggcgttgaaagcatttgcacggcagctgagcgggcatggcatcaacacgctggtgatggagtgggaggccacttatccttatcagcaacacgctgttatttccaaccgctacgcctatacgcgaacggagattgttgattttgtaaagtattgtaacgggttggggatagatgtgattcccctccagcaaagctttgggcatgttgaatatattctacggcactggcgctaccgggagctccgggaagaccagaaagattactcccaggtaaatcctaccaaagaagcggcgtgcaaaaccctttttagcgaattgtataaggatcttatctccacacatacctcccggtatattcatattggtggggatgaaacttacctgcttggtcactcagaagcgtcgaaacaaaaagtggcgaaagtgggcaaagggcgtttgtatggcgattacatcaaaatgctgtgcgaggtagtggtgagcctgggcaaaataccggtcgtatgggcagatattgcgttgaaatacccggatgcattacaggggttgccgaagcaaactgtttttattgactggaactatggctgggccctcaatcgttttggcgatcatgaaaagcttatgcacagcgggtttgaaatatggggttccccggctatccggagtgggccggataattatttcctgaccgactgggagaagcattttaataatatccgtgactttatcccgcaggcgcggaagttaggttaccgtggtatggtcatgacttcctggtccacctccgggttgtattccccggtgtttgaatcgggcagcgatatcacagatctctatgcgatccgccgggtgtatcccattgcggggtttgatatgctgatagccgcgtattttgaaagtttgcgtaccacccgcccgctggaagtaacgaaattcattacccggtattgcaaagatacctatggctttaatgaaacgcaggcccttgcctgctggaacgcgctgaagaaagcgccttatgaggtgtcgcagggcgcggtggtaaagccgggtgtttcgctcgccgctttgctggacagtgcgcgggaaacagccagggttttatattcccttcaaccgtctgctaataaagccagctttggtcatttcctgttaatgagtgatatcaggatctattacctgtcttgtttaatgatagaagcaaaaatgaatagtgtgaattatacccgggatcaggcggccggtttgctgcaacagctggatgcactgaagccggaggagctgaacaaacgcttttcgctgatgaatgaggaaataatgtttccggcggaaattgaaacagagaacacgttgcgtaatgaaagatggaatcagttaagaaataagctggaggccaacaaatgacacatatgaatatacagggcgtattgtacaaacggagggaagacacgatatctattgtgatcatcgggttgatgttttttatttttgggatggtcacctggatcaatgctatcctgatcccttattttaagataggctgtgagctgaataattttcaatcctacctggtagcttttgctttttatattgcctacctggtgatgtcgttgccggccggttacctgctgaagaaaaccggcttccgcaaggggatgatgattggtttctggatcatggcttccggtacactgctttttgtacccgcaggttttacgagggcttatcctgttttcctggcgggactttttacaattggtctggggctggccgttttgcaaactgccgccaacccgtacatcactatactgggcgataaagagcgcgccgcgcagcggttcagcatcatgggcatatgcaacaaagctgcggggatactggcgccgcttttatttgcggtggccatcatccggcctggtgatcaaacgcttttcaaggcgctccccgcgatgcagggaccggaaaaagaattgatactggaccagctgatccaacgggtgattgttccttatgcagtggtatctgttgttttatttttgttgggattattgataagattttctcctttaccggaaattgatactgataccgggcatggcgacacggctgctttacatgaaaaccggaaaagtgtattggaatttccgcacctggttttgggagcagtggccattttttttcatgtaggttcgcaggtgattgcggtagacagtatcattaactacgcctccggtatggggatgccattccttgaagcaaaggtatttccgtcgtatactttagcggctaccatcaccggttatatactgggtatattattgataccgcggtttctttcgcagctggtggcgttacgtatctgcactgtattgggactgttgttcagctgtatgattccttttatacagggaaacgtaacgctgctgggacaccacacggatatttctgtatggtgcattgtgctgctgggatttgccaattccatgatatgggcgggaatatggccgctggcactcgacagcctggggagttttataaaaacgggcgcctccttactggtaatggggttatgcggcaatgccattttgccgctgctgtatggatactgggccgataggtatggtttgcggttggcttacctggtgttgttgccctgctatagctacctgatcttttacgcattttatgcatttggcttgagaagctggaaccggaaaactattaataaatgataaactatctgaagatatataacggaacggtgcttacaccgcaacgcactattcccggtggttgcgtgattatcgctgatggcgttattgctgaggtaagcgatcagcagatagacgtgcccggcgccatagagatagatgcccgcgggcaatacattgcgcctggctttatagacatgcatgtgcatggcggcggcggccacgactttatggataataccatcgaagccttccatcagattgccattacgcatgcgcgctttggcaccaccgccatgatgcccactacgctgagttgcggcaagcaggatttgctggatacgctggctatttacgaacaggcggataaggggaatgataaaggcgcggccttcgttggcctgcatatcgaaggaccttatttttccatgcagcagagaggagcgcaggatccgcgctatatccgtaacccggacccggctgaatacatggaaatactttcccgttccccggccatcaaaagatggagcgccgctcctgagttgcctggagcgcccgagtttggaagatacttaaccagcaggaatatcctggcggcactggcgcataccgatgctatttatgaagaagtggtaaaaggctatgaagcgggctttacacatgccacgcatttttattcctgtatgtccggcgtgtcccggcgcaacgcataccgctatgcgggggtgatagaaagcgcttatttgattgatggcatgaccgtagagattattgccgatggcgttcatttgcccgcaccgttgctgaaactggtgtataaaattaaagggcccgaacacacggcgttgatcaccgatgccatgcgcgcagcggctatgccggaaggcccctcggtgttgggcagccttaaagatgggttgaacgtgctggtggaagatggcgtggccaagctgcccgatcgcagcgcttttgccggaagcgtggctaccgccgaccggttagtacggaacatggtggaactggccaccattcccctgcgggatgccgtaaggatgatgagtgaaacacctgcatctattctccgcatacaggaccggaaaggaaccctggaaaaagggaaggacgcggatgttgtcatcttcgacgacaagataaatattcacaccactatcgtgaacgggaaaatagtgtacacgtcgaaagaaatttctccgggtatcttatctaaataaaaaaacatgataaaggaatttaaagcgggaaaattaaccgtgaggatttatcccaaccggcaggaaatgggcagggcagctgcggagatggcggcggttaccctccggcatttattggaaaataaaaaagaagtgaatatcatttttgcggcagccccttcccagaacgagttcctggaagcgctgcagcaggagaaaagcattgaatggaaccgcgtaaatgcttttcatatggatgaatatattggcctgccggcagatgcgccacagggatttggcaacttcctgaagcaccggatctttgatgcgttgccctttcattccgttcattatatcgatggcagcggaacagcagctgcctgtgagcaatatgccggcctgctgcaaacacatgcagcagatatcgtatgcatgggcataggggagaatggccaccttgccttcaatgatccgccggtggccgattttgaagatccgctgccagtgaaaacagtagcgctggatgaagtgtgcagacagcaacaggtgaatgatggttgtttcgccacattggaagaagtacccacgcatgccgttaccttgaccattcccacgttgctggcggcgccccatatcttttgcgtggtgcccggttcccggaaagcagcggcggtatacgatactgttcaccgggacatacagcagcaatatcctgctaccatcctgcgcacccatccaggtgtggtgcttttcctggatgctgacagcggtgcgcagctaagccatcaaaaggtataaggatgcggaaactggaggtaccctttattccgttgtatggcaggccggcaccggcggaagtgagccggttgctggacaggctgcaggtgatcccgatcagctgtaacccctggccgcagtatgcgcatgcggtaaccgcagcgttttccattgcgcatagcgaagaggctattttgctcaagtattatgtaaaagagagccatttgctggcagcggcttccactaacggggatattcataaagacagctgcgtggaattttttgttgcctgcgacgatggcggcaattattataacctggagtttaactgtataggctggtgtaaagcaggatttggatccagccgtgaaaacagggctccgctgcccgttacggctacagacctgatcaccacggctacccatatcacatcggcagtggagcatgggaggagatcatttgtttgggaactgacggtgattatacctgcagtagtattcagctatcacaatatcactaccctaaccgccatgaaggtgaaaggcaatttttacaaatgcggggatgaaatgccggcgccgcattttttaacctggaatgacgtaaaagccgctatgccggatttccaccggcgggaagattttgcggatatctgttttctctgatattcattaacctataaaaagtacaaaatatgaaaagcacttttgcatggctgctggcagccatccctgtttgttttgcaaattgtacctcctccaagctggatgggccggttcaaacaaaaacaagtattcagaacagcaaagccaatacggtggccgtgaacgcgctgaaccaaaccactatccagttttcgggttatacctggatcgtaaaggaaccggctggtcagcagggaccacataataactactggagtggtgataacgtttgggtagacagcaacggacggctacacctggtgctcaaaaaacacaatgataccggccggtgggagtgtgcagaggtaagaagcacacagctgtttggatatggcacttaccaatggaagattgaaggagccgtaaatgcactggataagaatattgtattgggccttttcaactattccggcaacagccgttttgatgaaatggatatcgagttttcacgatggggatatcccaatgcgccgatattaaactataccgtttggccggctaccggcgatacgggtatcagcaatgtaacctatgcaaaggattttgtgatgagcggcacctataccacgcaccgtttccggcgggatgccacctccattcattttcagagtttgcacggctttcagaatggaaacgtgaaccagtttgaaacaaaaacgtggactgcacccacttctatcagcacgctgcaaatgccggtacacatgaacctctggctttttaaagcggtgccgccttctaatggcaaagcagtggaaatcattatacacgaattcaaatttacccctttatcttagtggcgtatgaaatctgtaccggaaagataccctgcgttggatgtgctgagaggcatgaccgttgctttcatgatagtggtgaatacacccggcagctggaatgcgatctatgcaccttttaaacactccgactggcacggatttacggttaccgacctggtgtttccgtcgttcctgtttgtggtgggaaacgctcttagcttcagtatgaggaagatgaaaagtctttctcatactgcatttatgggtaaggtattcaaacgtacagcgatcatttttgtgattgggatattactcggcgtttttccttttgtgcaggtggaagagggacattatctgtggaaggacctggctgatacccggatctggggcgttttacaacgtatcgcggtttgttactgtatcgcagcttttatgatccgttacagcagccaccgcatgcttgttgttatgagcgtgctgatattattgttgtattggtatgtgttgtattattttgggacgcaaccaggaccttacagcctcgaaggaaatgctgttggtagattggacgcgctttatttgtctccccggaacatgtaccggcattatggatttccatttgatccgctggggttattgagtacgttcccggctgttattaatgtggtggcaggttttcttacgggtagttttatccaggagaacgggaagcgcataagcggtatcgtgaagttgctgttggccgggatattgctggtggtagccggcgcgttatgggacaggtggttgccgattaacaagccgctgtggaccagctcctatgttgtgtatgccactggctttgatttgctgatcctcgccgcattgatcatcatcattgatgtatggtcgttccggaaatggacttatttctttgaagtgtttggtaaaaatcccttgttcatttacatcgttgcctgggtggtgattgtattgctgggaatgatacgcataaacgggggatccgtgagaggtattatttacaggggtgcttttaccagttggctatctgacaaaaatgcttccctgttgtttgctgttttttatatgctgctgatgtggcttgttggatatgtgatggaccggcggaagatatatgttaaggtgtaaggatggttatcttatttaagatattccttcagatacccgctgcgggttaaaaaagctttatagtctttgatgtcaagaatttccctgacagcctcttttttatcagctgccttcacaaaatattgctgtgtaatcttatagcccatccaataaccgagatcattcgggtggttgtctttcccggaaactccatatagccagtcgatatagttggtactatcgattcttgtaacaaattccctgcataacttttcctcgtttttattcccgtagtctatcgcaattttattggtggttgccccggatatcagttctcctaaaaaatcggcgctgccttcgataatactttgctgcaataaagtgggattttccatccagttcttttgctgaaaatgaatcagctcatgcgctacgataaatggaatgttgctgacatcagtttgcttttcagcgccgatgaacaaaccctgctcattgaaggttcctcctgaattatatgcaccgatcacaaaataaacaggtggatactgcgcgggaggataccagtattttaaagcgtagaacgcgctgcggcattgtttttctttctccttcatttgcaaggtggtggcccttactttttcatagtcgctgcggcgtttcctcactaccaggaataaattttcggcgcttttaatcctgcctggtgtaaacccctttacgccggcgctgccaatgtcgagataggcgctgccaaacgggttaacggtcgtgtcttttttaaagaggtcaaaagctttccagaaaacatcaatgtcttttgtgagaaaaacagcgctgtcggggttatttgaaaaagctgtttgtgaataagtaaccgtgcatgtaaatacaactattaataatgtcaggcaatatttaaacatagcaacattggttgaaaatggcttcataatgttgcaaagtaatttttttgacgcaaaattctttttttaacccgcttttcgtataattatgccatgtgccggtaacccggttaacccaaattcggaaaccatgtcaaaagaacgggcttatggaaattcatgcttttgtaccgccagcggatggtaaaaaccactttcagataggagattttaattttgagatagatgaagcacaatcgggacagggtttcgattactcaggggctttactcatcacagtggttgccaggaccggtgatgtagaaagggctgtggcggcggaattactggacgactacgagcctacgggcgaggtgaaaattacgattcccgcattgggaatctataaaagcgatgcaccggaaggcatgctgcattttacggaagacaaacacgaggcgccttatctttctattaaccgggaaaggtttcattatacgttaaaattttcaggggatgttatttttaaagatggttgggtagcgctgctggggcagttgaaaccttcgtggagtgatcaacccgtgtttgcggtgactgtttaccggaagatagataccgcacagttaaactgggaagagtactgtttcacttccgtggcagaagcagcaggcgctcccgtggaactggtgaaaaaactggtgctcaccaaccctgcattcgaccggctgccgaatgaattttatcgcctgaaagcattgcggaatgtggaaatcatggccaaatggccggtgaaaaaaatccccctggaatggctggatgataagttgcttcatctccgtgaactggagcacctggtgattgttgattcaaacctgtgccgtatccctgagtatatgaaccagcttacgaagttgaagcattgttcgtttgcaggtggaaatttatcgcgtgtacccgctcacctgatggatatgccgcggctggaatatcttaacctcaacggcaaccagctcagcgaaatagccgtattcgaattgccggagctgaaatacctgcacctggcgaagaaccaattaaaaaccctgcccgaaaatctattggcgttgccaaaaattataaagatcaacgctgccaataacccgttttcattcctgccggcagctttttcagattttgccggactggaactggatataaaaagtaagcagcagttgctggataatacttacaaagatgcagatgacaacggaccggtgaactggaacgatgaaagtttctttgcgcagtatgatgaagcattaattaaaccggtggatgagatcctgcagaaagaggggttattacaacagcgcgaagcgttacgtgcgctggtaaaaaagaccatcagttttaaatattccggcgaagaagattacgctgccattggcaaccaccggtttggcggcatgcctgatttgcccgcggatgttgattaccctgtgtactacgatgattaccgcaaggagcattataagtatgaattcatcgcccaggttaattgtgaagcgctggcgctgttgcaggaatatttaccggaaaagggaatgcttttctttttcctggaaaccatgcacaacctcggcgcccgggacgggcacctgccttgtaaggtattgtatgtggccgataattccaccctgcaatccggtaagcggttttccttcggggagcaggatttttatgaattaacagatgggcaatacgccccatataaagccgatgctacggttaaaaattcggtaccgggtttttattcctggcatgttaatcagtatcttttccggggtgtatcgaagtcgttgttgcaggatgaggcgctgctcagcaatttgtatgatatctttgaagagctggttaatcgcctgctggaaagcgatcatgaaatgaataactatggttttacgcagcatcattcccctgagttgcaggcggcgctggcctgcaaaggaaaccccgaggactggaccattctgcttaccgtaaaatcgcgcggggattttagttggggagatgccggcgacctgttttttgttatacataaaagcgacctggcgcggaaagatttccgcagggtgtatgtaactatggagagcagctaaagaaagaattggcatgtttgacattcggcatatctaacaaaagtatattgttatgaaaagaaaactggttttgttctggcagcgttacggccctcctatagaagttgcggggcttatacttttaattatcgggagtacgtatatgaaaaactccgttacctttaaaagcttcgcgatcgctttctggattgtgtgcctggtgctttatgtaataggggaaccaacgtaccggacaacccggttctggctgtttcttatacttggcttaattttggccaccagccaggtattgcagttgatcggcacatttaattaattattgggggagatttataaattatgaatgcaggaatgtttatcgccagcacatcgcttttggaggataccttttttgaaaaggccgtcctgttcattacggaatataatgagaacggggcgatgggatttgtggtgaaccaggagtatccccgtaagtttaacgagttggaggagttcaggtatagtcccccgtttccgttgtatgatggcggtccggtagaccgggagcatctttactttatacaccgttgtcctgagctgatagaagaaggtatacaggtagtggataacatctatatgggcggggattttaaggcagcggtgatgcatatgaataatggaacgatatctgagcaggacatccggatattcatcgggtattgcggctggaatgcgcaggaactcgaaggagagatagcagaaggcagttgggagatactgaaagaagggaagatgttttagtggtggacagggggatttttaaaaaagaagttattttgcacgttgattttgcaaagtaaattgataaatagtattaatatgtctacaggtgaaaatgtaaatgccagcttaggcggagatccgtatgaaaattttcgttcattgttgcagcaatcaattgtattccccagtgagtatacttttaagtttatcattaaggcggacgaggacaagatagcggagctgaagtcgatgtttgcggatgtaagtgcaaaaattacagagaccaattcttccggcgggaagtataaatcctttaccgtgcaggtgcctgttcagaatgaggaagaagtgatttcgtattataaggaggtgtcaaagattgattcggtgattatgctgtaggagctttatcatgcaaaaagttatacagggattgttataatattgacatttttcgatatgttgcatcatgattaaggccgattgcctatattcgggaacttatatataattctaatttaaatttatgaagcaaacagtacctgcctttgccctgctgcttacacttgcagcatgtggtggtgcttcgactgatcaggcgaagaccgaagaaaagaaagaagcagctgtgaccggtggcgcagcttataccattgacactgccactaccactgtacagtggcgtgctactcacaaaggtggctttgcgccccgctttggtaccatcaaagtagcggatggcagtcttaacgttgaaaacggcgctgttaccggcggtagttttgatgtaaacctgactacattggttgcagacccggcttctgttactgaaccggacaaaaaagcatccgacctggaagggcacctgaaaagccccgacttcttcgatgtggcgaagtatccttccgccaaattcgttatcacgtctgtagctcctttcgacagcaccaagcagaaaagtctgcttcctggcgctaccaatcttatcagcggtaacctgaccctgaaagacagcaccctgaacatcactttccctgcgcaaatcgttgttgctgaaagcggcgttactgctaatgcaaagttcgtgatcgacaggtcttcatggggtattaactacaaaacagaaggtagcccggaaaactggatgatcagcaaagatgttgaaattggtttcagcctgaaggcagcaaagaaataatttctttaccggctaaggtcctgataacttaatatcaaatgaagcagcctggcacatgatcgtgccaggctgttttatttcaggtagtcgctaccaaaaattcttctccgcttgacgggtggaaattatctgttctgccggtaaagtaacgtttgtcaagatcgtctaccgatattatctccaacgttttaaaaccggcttcacgtgccagcgttcgcatttcctccggtgtaaaaaaactgatgaaaggagtaccggccgcctgggcgcctttctctgctatttgttgcaggggtttatcttcttccttaagaaggtcaaatggcaggtaaaacgtcatggcaatccgggagccgggtgcaagggtggcaagctggcgcagggtagcaacgatcgcgtccctggtaagataaaggctaacaccggtgcaagccaccactgcgggttggctggtatcaaagcctgcatttatcaattgctcccaccaggaggaggtttcaaaatcaactccaacaaaatgcagccactccggcataccaaagccaagttcagttaaccgttgttgtttccaggattgggtatcaggctggtcaatttcaaatacctgtaattgggatgcaatgtccggcctgcgttgtgcaaaagtatcgagtcccgcacccagtatcacatactgctgaataccctgttcctgctgtgctatcaccaggtcttcaatgaagcgggcgcgggccaccatggatgcccggaggcgtttggtaaaatccgggctcatgtccggccgttgctgccatccattatcgggcgctattagttgaagcccggtttcatcttcaataatatgaggcatcggatcgatctgaacgtgcagggctctccataaagctgtgcgtaccgctgtattgtctggtgctgcctttcttttatcctgttccatgtgtgatggtttgggtgattaatgtgacaaaattagctgctatgccccgggtaaaattgtaaaaaaccgacaggcccttttatgattcccattcgggaaatccaggcatccgctcaatggatttgcgcaggtaaatgcccggactcacgccggcgaaaagtttgaaatcgcggataaaatgggattggtcgaagtagccaagcgaatgtgcaatgcctgtgagtgaacaaagattgcctttccgcaaaagcgctaccgaagcctggaagcggcagatacgggcataaaaaattggtgtaatgccgatgtgggtaagaaagagacgttccagcgaacgttctgataaactgaggtcatgtaatacatgcgacagccttttcccctgttgcagtgctgttacggcataatctacttttttattgctgttttcgtaaaggtgtgcctgtttttccaggaagttaaaaagacaagcagcctgttgttgtgcagaactgcaattaagcagttgttcgcttaaagctgtttttgtaaggtgactgatgcaggtattttggtcggtcagttcattagcattcaaaccaaacaccgatttaagtgctgcggggtgaaagtttataccaaccgtgcgaaaactaccaccgccatgcaattggccatatttccttgcctgcccgaaaacaaacaattgtggcagccgttcaccttcgaaaccggtaaacactgcggggttctcctggaaaataagccccggagcaccattgcacatggccgtgaaagttttttgtgatacatcgtcagtttggtgctccagggtccagaaacattgaacataatttttcagcgacggagggggagcaattacctggtaattcattttttattttctaacacgcagataccgaagataacccatttcccggtttcgggaagtcggtgggctattgttaaatttatatttaaatggctgagcatgatatatatgcaacaacagacctctgatacatatacttaaacaacatatttatctgttatggaaaataagcctaatttatatgaggttcaggtatctaaagctgtcagatgattatcagatcaagtaaaccagctctttggaaaggagctttaattccgttggcatattttatattgactttctttattgcgcaacatcatactttgttcgaggagtgggatggcgccatgcaatacctggctggtgtggacttatttgagggaaaaggatatcggggcgtgagctcacatttctggcctcctctttttacgctattaacaggcttgttcacctggatttttcaggatggttttgcggcggcgaaatttatatctgtgctttcctcgtctgtgctgctcctggttatttaccgttttgtgatgaagtttaccggcagccaggtgcctgcctttttagcgcaattacttgttgccgctaatcccacctattttctttacagtatccaggcgcaaaacgtcatgctggataccatgttttatgtaagcgctatttgcttttttttccaagcactgcagtcagcttcttataaatatctttttataacaggaattatggccggattagcggggctgacacggtataccagttacgccttgctgccctcctttataatactgctatttttctattaccggccacgggccgcctcttcaaatgtgttcaccttgttcgtggggtttgcaatagtttccctgccctggtggatcattaatacgcttaacagcggcggtccttttaatagctggcattatctgaacgttggttatggcttgtcgtaccagtcagctccggttaatccgaaatggtggtggcatgaccaggcatcctacaattctgtctggcaaattatgcggcaatcaccattagattatgggaaacattttttatataatgtaatggaggttttctccacgctcactataaaaacactgttatcgtttattgggtgtattattttattttttgtacagtttttatctacccggaaatgcaggtcctttttggcggataataaatttttcctggtgattgcaacctgcttaataatgtatacaggtttgatttcacaggcgtttatcatagaccgtttgcttttaagctggtttgccataaccggtatggctatagctgtgttgttgtatacaataggcatgtctgatccggggtggataaaattaaaaccgcttgttgccggcgcactgctcttctttttattgataaacgtaatagtgactatcaggaaaatggatatttacctggatgacaaaaacgatagcggacagctggcggatatggaaaaaataacacagcttttaaaagcgcaggatcctgatttatcccaaaaaacgatcatggccatacatccggccagcgcatattacctcggatgccggtttgtgatgataccactctattacgacagcaataatatcaatgattggatcgcatacggccatcttgctcccaaggtcattaactatgttccccgctttccgggagacctggatatcacaaaatcccctgtgaattaccttatttttaaccggcttagcagcacatatcttccccagttttcctttttgctggatgaacatacagataagattcctgctaatttcgaacgcctgttactgacaaaggacgtggcgctttacaggatcacggggatcaggtaatcatcttcaaatcaatgattcgttaagacagccaaccgccggtgaaaaataaatttgtgtagttaaataactacatgtacatttgtagtcaaatagctacataatgaatttacgacgagatgtatttcaagccatagcggacccgacgagacgggctatattgctgttggtagcttcacagggcatgacagcaggggcaatagccgctaactttgacaccgccagaccaacagtttccaaacacctgcaaatacttacggagtgcgaactactggaacagaaacaaaacggcagggaaatttattaccacatcaacgcaaaaaaaatgaaagcagtagcagactttattgaaccattccgccaaatgtgggatgacagatttaataaattagaatccatcatgaaaaagtacaaaccaaaaaaatagcagccttatggaacgaaaaacaaaaatcaatgccgaagacggcaaacaggaattagtgataacgagggaatttgatttgccggtggaattactttttacggcatacacagaacccgaaattgtggagcaatggatgggaaccaaagtgctgaaacttgaaaacaggaagcacggcggctggcagtttgaaaccagcgatgctaaaggcaacgtggtatttaaagccaatggaaccgttcatgagtttattccgaaccagaaaattacccggacttttgaaatggagaatgcaccttttgccgcccagctcgagttcctggaatttgaaccacttacagccgataccagcaaactcaatatgcatattgtatataaatcagttgaactcagggaccagatgatgcaaatgggttttgctcccggcctgaatatggcacataaccggttacaaagcatcgtaggcaaattaaaataacacatcatgtcaaagagaaataaaattatttattggattgctacgctctggcttgcattaggaatggtatcaaccggattagtacagttattcaaagaaccggatgaaacagattttacggcgcatctgggctatcccacttattttctgaccatactgggcatttggaaattgttgggagccatagcagtactgattcctaaatttcctttggtaaaggaatgggcgtatgcgggctttttctttgtcatgtcgggagccgcactttcacatatggcaactggtaccatgaacaatatttttccttcgttgttattgctggcgttgacaattacatcctggtacttcaggcctgcagacaggaaaactatttcagttaatcaataaaacaagaaaacatgaatcccaaggttgatttctattttagtaaagctgacaagtggaagaaagaaatagagaaattgagaacgattgttctcgactgtcacctgaatgaagaattgaaatgggggtgtccctgttacatgtttgaaaagagtaacatcgttttaatacatgtttttaaagagtactgtgcgcttttgttttttaaaggagccctgttaaaggaccctaaaggaatcctgatccagcaaactgaaaatgtgcaggcggcgcgccaggtccgctttaccagtctccaggaaatagtgaagctggcgcctaccctgaaagcatatatttatgaggcggttgaactggaagaagcaggtgcgaaagtggagcttaaaaagacgaaagaatacgccatccccgaagaatttcagcagcagttagataaaaagccggccttgaaaaaagctttttatgaattaacaccggggcggcaaagaggctacctgctttatttttctgctcccaaacaatctaaaacccgggaatcgagagtggagaaatatatgtcgcagattctcgacgggaagggattggatgattaagggatttcatctgatgttattgcattattctgaagaagcatgtatctttagctggtatgaaaacactatttgcatctgttatataatcccaataacatgaccagcttaaaacccttatggtcgggtgttactatctgtatgatggcgctgctgagtcaatttccggcaaatgcgcaattccgtcagttttcggtatccggtggcggtgcatttaatacgaatgatttcgactggtcgattgcaggtaatccgcagggacaatctcccaacgttttatcagaattgcactttaatggtatcacgtccctgggcttttacctggatggcgcctatcgcccgttgaaatgcctccggttcaacacatactatcaaagaaatggtgtagtcagcggcagtggtgtggataccgactataagggtgataaccgcacagatcctacctttcagcagtctttttccagcaacaggggctacctggagatattcagggcaggcgccatggctacatttctgcaacgtgccaatttcagtttgggagctggggtatcctataaaaatacccggcaaaactttgttatacttagtcctgaattaacggacctgcagagtacttatacagcaaagtggcgtggacccgagtgttctctggaaggtaattacaagatcaaccgctctttatcagtgggcgctgatatcgcttatacctggatcagttaccggggagaggcgaactggaacctgatcgatctgttcatgcatccgttaagctttgcgcaaacgtcgaagggacatggtatggactatggtttgaatatcagatatgccgttaacagctttctcgccttttcacttaacggcatgctggggaatgcgaggatttcggaaggaactgatatctcttatttgagtaacggcacgcagatttccacacagtttaatggctccgcgaataattattacggcgccaggttgggcgctatcattcagttctgatggattgcctgtttgatgaaccaggcacaaataaataaggccagttttaataaccggcatttataaatatcctgaacaatacagggaacgtcctatttttccaaccggtattttattgtaatcgctggtgacacagctgtgttgattacgactaatgaagtatccggtgaataggtaacttttcctttcagatctgttctttgccggccatctccatccaggaaatagatgctgtctgcagtcagcttgagtgcaaataccgaatctttctggatagtatatacaaaatccgctttgatatttgtccggagaccataggccgcgaaactggtgctttgcaatgtgttttcttttgccagccaggaaaatatgttgccgttcccgatctttgtccagcttccttcctgctgcgtcttgatagagtcttcccgccaatcgaatttagcgccataggtaaaaggatctatctgtaaatcaccatcgttatcatccttcccgcaggattgtaataacagcagcgctacaattgggcacaaaaaaatgaaaaaggatttcatctgtggatattttatctattttgaaaagtaaattacatttttatcttttaaaaccaggaagaagcctgtcattttttaacaggcttcttcctggtgcgcttacattaagggcaggtaaattttcctaaatcattgttcagtgtacaacaattaggagggtatggattgccgttgttcaaagccgcctgcaggtcaagtctttcactcggcgtcatgatggtgttatctgacttatacactgttggcgccaattcagcatacacatctgatcttgctatatacggaatgtagaaataatttatccaggatctgtcgctgttggaaagaaaactgccctggtaaatataactgccatctgttttagtgtacattggtaaactggtgttatgcacaatggatgtactgcttgtcagcgagctgtatcccattacagaagtgtaatcgtatgtacctgtctgatagtaattggtggaggggatattaaattgcgccagcccggaagaggtaaggttagacgtattaacggtaacaaacgaattcctgtcgaggcgcgtatgctcatgtcttaaacccagcgcatggcagatttcatggatgatcacactgttgtcccatgaatcaaaggcgaaatcagcgaggttgatgcgttgtactccgcctgttcttccgagatttgattcgctgacatcagcaccatctgtggaccagaattcgatgttggggtaagtaaatccataagtggggtcaaccagcggctcacaggtagcgttgtagaaccttacattggtattggattccatttcaagcagtgctgaacggactttctgtttctccgccagggttaaatttgacccgtatataatcctcaccatggcccataaattataggcagtagggtatatactgaatgctctggggatggtgcggccctgggcggtgttttgaaagggcacattatacaccgggtgcgcatttttttcggcgcctacatagtctggtttcttgggcagtagctggccatagagatccaggtttttgtattgttccttagtgagacggatatctccttcccaaaaataatcagctccttttttttcgaccatcgcaccggattttaaagtgatcgggccatctttctggttatctgattgattggattggttatccttgctacaggacaggaaaaacaatacggctaacaacgggaatgctttcaaatagtggttacgtttcatgggtaatgtttattggttgaaggaatactttgggttacatattatcagactatagcaaaaatgagaataggttaaacaaatgtgatacctgagggtaagcatcacgattataatactatctaaaataaagaataattttaattcgccgggaatttatttttcaaatttttaattcgtagtcctgataatgtggggggatgcccggggcatttttatatatttctgataatcagttattttttttgttataatttttcaagtgcccggtttgaataattgtaatattgacagtactaatttatcaagcgggtaaatttataccggtgcggcaaattccctgggagatgtttaccatttatctgttagcccgatctatttcttatacctgaactttttgagcagctctttttttttcgccgcgatactgttacatacagaccattttccagttctatctgcccgccttctccccggatatagcgtttgatgtactgcagattgataatatgcgagtgatgggtgcggaagaataaatctgttggcaatagttcttcaaaatctttcagggtacggctggccaccagggcagggtgattggaaaaactgatagccgtgtagttgctcttcgctttaagacatataatatcggcaatattgaaacaaagcaatccttctatcgtggggatagcgattttgccttgccgggcgccggtgtccaggttttgttgcagtacctggagcttttcttctgtcgtcactccttcgcttttgagcttgaaggggggaggcattattgatggcatcgtacagggctttaccggaaagtccgccgggatcggggggagcctcttcaccgacctgtgtaccattaaaattccggtataagcgggaatggcagaagccccgtttagcagatggaggaagtgggtgagccggcggggagttaaaggggctggactaactcctgccagatgggttcctgcctggttaaaagcgggataacaaaacaaatttgaccggtttatagaattaatttaatattagtgtatgtatcttaccagtgtgcccgatcatacggagccaggatttgatgaggcattgtatttcagcaaattccaaaagcataacattattattaatgcggagagcaatgggagtcattgtgacgatcatgccgggtgtctttctatcaaaacaatactcagtggcgaggaatggtatgggattgatcgtcacaagctggtggtaaggcccggccagttcctggttttaaacgatgatcagcgttattcgtgtcgtaccagccggggcgaaaaagtgagagggttgtcggtgttttttaaaaaggaatttgcgtcggctgtgtttagtgatatgcttaacagcgaaggagcgctgttggataattcttcttataataacagtacaatacctgaatttttccagacccttaataatatctcccctgatttacaggcgcggttatcccggcttgtaaccactattgaaagcaggggatatgatgcaactatggtagatgaatacctggtttttctgttgcggcacctgattggggtttacaaatctgacgtggttcgcggagctggtatccaggcggttaaggcaactaccaggattgaaatttacaaacggctatgcatagccagggatatcctgcattcttcttataccgaacatcttgatctgtcaaagataagtagcctggcctgcttatccatgcctcaactaatcaggcagttcaaagcggcttttcattgtacgccgtatcaatacctcatacgcatcaggctcaggcatgctgctcaattgttgcaagacacggataagcctgtgcaggaaattacctggatatgcggttttgaaaatacgagtgctttttgccgggctttcaaatctgtttatggcatccaaccggtgctcttcaggaaaaaataaaattgagcatttttgcacatcatatcttgcagcgtaggcgtaatattgagtatccatgcattttatgtttacaaaatgaagagaattatatcagtatttgcttttttgtcatttttacagttggcgcatgcgcaggaaacaatgataccgctgtataaaaaaaatattccgaattccaggagcatacccccggattatatagaagaaacggatacttcaggtttgataagaaaagtaacacaacctgccctgatacctttttttccgaagaagggaactgcaaccggcacggctatacttatttttcccggaggcggttattttgttttggcgccagccacctgttatgaaatggccagggcgctcaatgaagcaggtatcaccgcttttgtagtaaaataccgtttgccgcatgataccatcatgattgataaaacaattggtccgttacaggatgcccaggctgccattcagctggtacgcaaaagagctgcagagtggggcatcaatccccacaaagtaggcgcaatgggcctttcagcaggtggtcacctggtatcaacagcgggtacgcagttgaacagggtagtgattgaaaatagagagcagatcaatctccgggcagattttatggcgctattgtatcctgtaacgatctatgatcctgctattcccagaacccgcgaaaacctgattggtaaaaatccatctgctgcattgctggatctttatagtaccgataaacaggtcacggaaaatacgccaccgacttttttggtgcatgcggctgatgacgatgtgataccggttaaaaataccctcctgttttttaacgctttactgaaagcgaatgtaaaggcggaaatgcatatcctgcaatctggtggtcatggttttggtttaacagatcttcacagcaaggataactggtttaatttatttaaaagctggctggcagaaaatggattttagtgggtcagccgcagtatgcctactgtatcagtgctccaggaaggcatccatcgccttcgtgggtttcccgtcatctccccaggcacttaatccataatggctccagctttttgctccctgcggctcccaataaattacacctaaaccctttccatccggcacggcctttacctttttctgtacggcaaccagcatatcataggtgttctgcgctttcgtgtcttctccgcccacttctactaccatcacctcctttccgtacctggcggccatctctttcaggttattgcccaggtcatcaatagaaagggtataatcgggtttgccggtaagccagtagggatagtatgacagcccgattacatcatattttgcgccctgggtcctggcgctgtcgaaccacgtaacaaagcgtgttcggttattaccctgatccacatgaagaatcactttagacgcagggctcaccgctttaatggcatcatagcctttgttgatcaattgcgccagttgatgccagtttgaagtgcttccttcaggatagatcatacctccggctgtttcattgcccacctgcacccattcaggggtgatgccgctgttcttcaaagcagacattacatcgaaagtataatcatatacatctttcagcagctgcgggaagtcgtggccttcccaggcagccggttttttttgcttacccggatctgcccagctatcgctgtaatgaaaatctatcattacccgcatctgccatttctttgcccgtaaggccattgccaccgtttcttctttgctgcaatgaccgctggctttatcgttagatggatttacccatgttcttaacctgatcgtattgataccgtgatctttcaggatctggaaacaatcctgctccacgccattatcattataaaatttgaacccggaagtttccatctgcggtagccagctgatatcagctccttttgcaaattcgttgcgggatgggccaacggatgtttttgaggtggtacatcctgtcgatagtataaccgcgagcagtataaagaagatagtgattattgatattttcatctggctgaaatttaagtgttatttgatggtcacttttatcgttccttctttcagattttccgaagaggcagtaacaacaacttttccggtaagatctcctgctttcagcaggatagtggcaatgcctgcttccgcctttaccgggttgctgccaattaatactgcattaccagtaaccgtgaattgaatgacattttttgcatcgggcaccagtacgccattttcatccgtaatacgcgcgtaaaggaaaacgatatccgattggccggattgaagcggcttcccggtcgtatcaacattcatactgatgctgctggcttttgccggcgttctttgtgtagtgctgatcacttcttttccgttgttgtatccgatcgctgttaatgttccgggttcaaatttgtttaccgggaaggtgaacggcggatggggcaattttcccgagaaggagttctgatcgggcttttgacgcgctatcagcttcccgttcagcaaaagagccgcttcatcgcagttactgaaaaccctgactgttgttacggagggattattccaatagctggcaataaagatcatcggcttgccaaaatcgctgttcgtgttttccggtgtccggtactggctttgataaaaataataagagaatttcggtaaacggaagatatcggagatcccggacgattctatgtccggcgcgtatccgcgtttgtagtcgaacaaaagccagttagcatcgcctacggctgttccggtaagattgtcgttatgggcttcctggaaattgagcgcctgttgcagcaatgccttttcaccagcttcccgcagttgccgggaagttctttctccttctttcagatctttatattctttttgattaaaccccgcattttgtgcatagtattcccaatcgccatactcagcaatcagtattggcttccgggtgtattttttccagtagtccggcgccctggcatgttgccttgcaggaataaacacatcgtacacgtcgtccatccatccgcaggtatacacgtctgtgaaaggcagttccttatgtacaatatcgtgggactgctgcatgtactccatactcatattggtttcattcagggacgcttcccatagaatgatggaggcatggtttctgtcgcggtgaatgagatccctgatattctgatagctgttttgctgaaattcctcattaccaaaaaattgccagccgggaattgagttcatcaccagtattcctaatctgtcacaggcatctaaaaaagcgggggaaggagggtagtgggagcaacgcacaaaattaaatccggctgccctgattttataggcatcgcggaattgcgcattatccggaagtgcatagccgatataaggatactcctggtggcggttagtgccacgaaggaaaaatggctgcccgttcaaggtaaaactacctgcttcaaaccggaaggttttaacaccggtactgatttgctcttcgtccacaactttgccctgctgcaatacctgcacagtaagctggtatagcgaaggatgttctggtgaccatagcgcgggatttttgatagccacctgcccgttaaaagaaacatatcctttactgattacattttttacaccagataaaacgcgaccaacttccactcctttttcatctgttaaaattaaattcacctgtgcattttgtggccggcggtaatcgtttcgcaattctgtttttatcattaatgttgcacggctgttgctaacgttttcataatgcaacatcacgccgccgccggattccctgttcgcttccaccgcatcggcaatgtgcagtttatctttgatgatcagccaggcattgcggtaaatgccgccatagtaattaaaatcaaggtctttaattgattttcccggtggaatagcgggattgttttgattatttaatttaacgactacgatattctctccatcaaacctgacgttatcagaaatatcaatatagataggaagatatcctcctgcatggcgatatacatgcgttccattcagataaatatctgcttcgtgcatggctgcatcaaattgcaatgcgatgtgttttcccctgacggcagcagccacccggaagtttttccggtaataacaggtgccctgccattgctcctctttcttctccacaggttcaatccgtggtgtatggggcagtgaaactttctcccataaaattttatgaccagtattaccggaaagggatgcagctatttccatactatccacattcttcacaaactcccattttccgttgaaattaattttattcgcagggtgtgtgttttgtgcttgtaaactgttaataataattagtaagatgaaaagaaagatgaaccggttttgcataaatgtagtcatgggttagatggttattgcggatacccgtcgttttgtttaatgattccctttgcttcgatgatcacggcagatgggatgggaaataacacctggtatggcctggcgtttgtttttcctcttgccagggcgttggttatcagggagccgtttcgtaccaggtcctggcgtctcacgccttcgccatagagttccctgccacgttcatccagcagggcggtacgcatacctgcctgtgttaagcctgtaaaattgggaacgcctgccctggcccgcacctggtttacatattggtatgcttcgcctggtcctctttgttcattgatggcttcggctatggccagcagtacttctgcatatctgaacactaccacatcaatggcataaccaggtccgtcgccctggatgctggtgtatttcagcggaatggctcctcttaatccattacttttgttggcttccgtaccatcgcttttagtatagtggtctatgatcgttgttttcctggtgtcgttggtttcatatttattgtaaaagctccagggcatataatatcctccccagcccggggctctctggatgcttcctgcctgtttaaagtcgccgggaagtacttcctggatccagtagttaggagaggcatcattggtaggcacagcataaatgagttccttgcctgctttctttttgaatatatctgcataattatcttccagcgaataattcatggtcattatttctttggcggttgcttccgccttgttccattctttattgtgcatatataatttcagcagcagcatgcgtgcaacgcctttggaaacccttccccagttggtggcatcactgttgtatttgtcggccaggtcgggcagggcggcagtcagatccgcttcaatctgagcggaataagttgcggcgtccggcctgggtgtgatggtattatctgccagtgttgccggatcagttttggcatttacagggccgtaaaaatcatatagcacatacatcagccaggctctcagcacttttgcttctgcgatatattttcttttaatgcctgcgtcaagcgttgatttttctatattattaattacgtcggtagctttggctacgtacctgatcttgggataggtgggatcgttggcatccacccaggtggagggtccgaaggtaaagttggttaaattggcatcccaatcggtttgtaattcatctgttgtcatcaggctgcggatgaagtaagatttgatatcagcgttatacagcgcaccataccagctgccggcgccgggatcagcgttgccccagttggaggtgaagggattgtaaagcgtaatgagcgcaacattcgcatctccttctgtttgaaagaaattttccggcgccagctgggaatagatgtctgattccagcatttttttacacccggagagcggtaaaagtatgatcaggcctatcagtgccagttgatgcagcgaaagtttgcagcagtttgaaatgaatattttcatgatgtggatattaaaaggtcaggtttacgccaaaagtggcagataatgcttgcggataaggattcacttctgtaacctcgggatcatatcccttgtagttggtgagtaccgcaatattctgcatgtcgaagaacaaccgggcattccgtataaaccgggtggaccgggtaaggttatcaggcagcttgtaacctaatgtgatattccttaaccgaaggaaattcaccttctgcaggtagaaatcatttgtggtggtgggattattgccactgtagggattactggcataaccgggataaaccccgttggtattgtcggcagaccaaactcctttgataccggtaagtgtattgtgtgcgttgctgccgtttatttgtgcgggatcataaaaccccgaatagctgttgaaaagatatcctccgaagttgccgtaaacaaatacattcaggtcaaaatttttataggaaaaagtgttacccagtccgatagaaaatttcggatccctgttgccgagtttcaccacgtcattgatatccaggttaccatcgttgtttatatctgtatacctgatatttcctggccgtgcattgggcatatggacaggagcatcagcggcgcttttgataataccatccgttttccagccgtatatttcgcggatcggatctttggcgccgatgaaaggagaaagcgcaataacaggatttctttctatccagtaatttttatattgggagatattaaaagaagtattccatttaaatgcaccggtagtattacgggagttcaacgatagctcgatgccgtcgctgcgggtggagcctacatttgccgccacctggcttacggcattgttggatggcagcgggttgtaatccagcagatcctttgcttccttccggaacacgtcgagcgctcctgtaagccggtcgttgaaaaatccaaaatcaagaccgagattgattgttttgtctgtttcccaggtgagatcgggattggcaatctgtgtaatggcaatacctgtgtaataagtggagcctattaaaaatggggagcccgttccatacagtgataaggcattggtgccaaggatgctttcattaccggaggtaccatatcccgcgcgaagcttgaggttggaaataacgcccgagtttttgaggaaaggctcttcactgatgcgccatgcggctgaaagtccggggaagaaaccgaatttatgattgtcggcaaagtagctggatccgtcgttacgccctgttaaagtaagaatatacttattgtcgtaactgtaatttacccggaagaactgggaaactttgatgcggtcgggcgccctgaaagagttctggaaactcttttctttattgctggcaacgcctacattattaaaactaaaagcatctgtgaaaaaacctactgcctggagaccaaagttatctgacatacttttgtagtatccggctcctgccactaccgcgagatcgcttttcttaaatgacttgttgaaagttaaataagattctgcggtatagttaccaatattattagtggccagttgcgccattccttctggcaattgcgcgttctgagcttttcgtggcaggtaaaatttcagatcggagctttgtttatcgatacctgctactgcagtcagttttaaattatccaggatctttatttccagggttggggcagccaacagccgtttgaggctggtctggttccggataatggaaaatgcagcgggattggtaatgaggcggtcgtagcttttggtataatttcccgattcatcataaataccaatattaggcgcaaaagtgtaggcggcttgcagttggttgtatttttcggggcctcctgcattagatcctgttgctgcattgtcgctgttaacctggcttagcgttaaattcaggttgaattttacccggctgctgatttgctgttcgaggtttaccctcccggtgtaccgcttgtagcgggagttttccagcagcgctttattatcatacaggttaaaagaggcgtataccttcgttttttcggtaccgccggacacggaaatattatgttcattaatactgccctgtctcattaacaggtccagccagtctgtgcctgcgccggctttgctgatgtctgcatccgaaaacatgggattgaacgccggaacggaggaggggtctgtgttgccataaggggccaggttgttatcatataaatacttatcccgggccaaacggacctgttgttgcataaagttacccgcgtctaaaaaatcgaggtagggtttgggcgactgtatcgtgtagctgccccggtattccgttatcgcctgtccggcttttgcctttttggtggtaataagtataacgccattggcagcagcagaaccataaatggccgtagcgctggcgtctttcaatacgtctacggattcaatatctgaagggttgatgctgcttaacgggtcctggtccactccgccgtaaaaaccaagatcgccatcggcgatggaaggaacgggcgaggcgttatttaatataggcactccgtcgattacatacaacggggcgttgctacctctcggagaaatggcgccccggatgttcacagaaaggccgccgcccggctgggcgctccgcacacttaaattaaggccggctgcttgcccctgcaacaggttattaatagaagtgttggccacctgtggcaggtctttagtttttatagataccactgatcctgtaatatcctttttgctggtggttccgtaacctaccactactacttcgcctaatgccgtggcggggttttccagggcaatacgaagggtattcctgttatttaccggcacttccatagtggtataaccaatatagctgataaccagcgttccgttttccggtgcatttaaagaaaagttcccgttggcatctgttaccgccccaacgctgcttcccttcacttttactgaaacgccgggcagggcatctccgttggctttgtctgtgatctttccctttaccgggatgtcggcttttatccggtaggtgacccggatgttgttaccgctgtaagcagccatcgcaggcatagatgaaacgatggcgaaggctaagggcgccgcggtctggcaaaatagtcttacataactaaccctccacgcggaacgatgcgtttgtcgtagtttattcatatgctgggaatttataaagtgactctaagcttcaagtcgtacataattagctgggaagcaatttattgcaattcgcttccggaggcttgttcaaatcatctaacatttgtttcaatctgtcttttgttaatatcagcaggtattcaggagggggaggcagctatatttcccgattttatctaaattggttgatgattcgtttaaggattttttaaaaagcgcctggtgtctctaaaaaaatatatctcccattttttattattccacgtggctgccatgacactttcattggttccgctgttttcttttgcacaacaaccaagactctccttcaaacatattacccaggaggaaggactttcaaacagcaccattgaaacaatattccaggatagccggggatttatatggtttggtacgcgcgacggattaaaccggtacgacgggtatgaaatggtggtataccggaacgaccgtagtgatgccagcagcatcagcgacagctatatccgttatatatgtgaagacagtgaccacaaactgtgggtggctacgaataatgggttaaatctttttgatccggttaaaaataccttcaggagatttactcatcgtgcccaggaggccggcggcctcagtaacaatatggtgaactgtgtattggaacaacgcgacggcgtgatcctggtagccactaccgaagggcttaacctgtataaccgggcttcaaataccttcagtcatattttacattccggccagccgggtagcatcagcgataaccgggtcaattatctttaccgggataaaaaagataatatatggattggtactgataatgggttgaaccggttcaatccggagaacaaaacatttgaaattttctatccatccggaagcagggacggcaacgcaggcgaaaatactgtgaaggttatccaggaagatactgccggaaatctttggctgggtacacaggacaagggactttatctttttgatccctctcggaaaacctttaagggataccggcacagtgaaacaaacagcctgagtttgtcgaacgaccagataaaaataatactgagcactcccaccgggaatctatgggtaggcagcattaatgggggactggatctgttcaacccggccaatggctctttttatcattaccagaatgaacccgataatccgaacagcttgtcgcaacgaaccgtttctgcgctttttgaagacaaccagggcaatttatgggtgggtacccatcggggcggtgttaacctgtacacccccggtacggataagttcaaattataccggcaggaaaacaacgcttcttctttaagttataatgatgtaaaagcattttatgaagacaaagaaggttatatatggataggtaccgatggcggtggcttaaaccggtttaacccccggacaaatacgtttacccgttaccggtataatccgtatatgccggcaagcataggttctgatgccgtcttacatattacggaagatagcaaagggaatttatgggtgggcacctggggcggcggcttaaacctgatggaccggaaaagcggcaccttcaggaggtatgtaaatgatccggacaacaggcaatccatcagttctaactatgtgcaaaaaacatttgaggacagcaatggcaatttatgggtcgccacttattacggcggattgaatttatttgaccgggccaccgggaaattccgcaggataacaacagctcccggaggaaaaaatagcttatccggcaataatattgtatccatcgatgaagacattcaccataatatctggattggtacagacgatggcggattgaactgctatcatattaaaaaccggaaatttacctgttattttaaaagtgaggaaaaggtgcccgaccttcgggtgatattcaatgacagcaaaggacggttatggatagggcaggcggggttatatctttttgatgagaagaatgacacctttaaaatttttaccggtaaggctggtctttcgcgggagtttatcaaaggaataacggaagataataaaggtaatttctggatttccacatctaacggactgttgaagtttaacccggaaacgggtcaacataaaagatataatataggagataacctgcagggcggcgaatttgaggcgaatgcttacctgaaagccagtgacaacagaatgtatttcgggggtattaatggatttaattcattctatcctgatagtatcaaagtaaatacattcgttcccaaagtatacattaccggtttccatatatccaacagaaaggtggccgccgggcagaaaggcactccgttgctaaatgacatcaccgccacccgggagattaccctttcttataagcaggcggatttttccttcagttttgctgcgttaaattataccgccgcacagaataaccagtacgcctacaagctcgaaggactggataacgactggaacctggtaggcactgaaaggaaagcatcttataccaatttggatccgggtgagtatactttcagggtgaaagcctccaacaatgatggcaagtggaacgaagcaggtaccgcgataacgattattatcactcctccattctggaaaacatggtggtttttactcctgttgggatgcctgatgatgtacctcgtttattttgccctgaaacagcggcgaaagtttgaactcaataaattagaagagaaaaagaaggaagaaatgcaccaggtgcagctgcagcttttcaccaacatctcccatgagctgcgtacacctttatcattgatcctggggcctgtagagaaattaagacaaagccattcccatcccgaattttcccattactatcgttccatacatagaaatgcgcttcgtatgataggcctgataaatgaactgatggactttagaaaagtggaagcgggcgtgctgaaattaaaagtttctccgcataacctgagtggatttgtacaaaccgtggcagaagaatttgaagacctggcgctgcagaagcagattgaatttacttttccaactacagatacgcatttaactccctggtttgataaacaaatattggaaaagattattttaaacctgctgaacaactcctttaagtatacagaagaacgggggaagataacgatcgatatatttacctccctcagcggatttcaaccttccttcagcaatgagctgatcctcaaaaatgagttccgggcaaaagattacttctatataagggtaaaggataacggcattggtatctcaaaagaatctatcaaacatctttttgaaagatattaccgcatcacgcaatcacatctcggatcgggtgttggattggcttttgtaaaaagtttaaccactctccataaaggagatgtgtatgtatatagtgaacggaaccagggaacagaaattatcatagcgttgccatcagcagcagaaaattattccagcggggagaagacagaggggaatgtgccggaaggcgtaattgccctggaaagcgttcagcaaaaattcgaaccacagttattgctggacgaccgtcccgagcacttacctgtaccagccttgcaagacgaacatattttattggtagaagataataatgaattaaggaagttcctgaaagattcactgcacccattttataaggtatctgaagctattgacggcgcttcaggccttgagctggcaaaggagatatttccttcattgattataagtgatgtaatgatgccccgtctgaacgggattgaattttgtaaattgataaaggaagatgttgaaaccagccatattccgtttatcatgcttactgccaaagatgcgatcgaatctagaatagaaggcgttggctccggggcggatttttatttttcaaagccggttagtatcgacctgttactacttactgtccgtaatatttttgttcagaagcagaagctgaaagaacgctatatacaggattatcatatagaagcaaaagaactggtgcattctacccaggacaaggagtttatggataagctgcttggtattattgaatcccagatgatcaatcccgagtttgatgtagacgttctatgcgctgaaataggcatgagcaggacaaaactttatgagaaaataaagcacattacgagtcagaatattgtggaatttatacggactacccgcttgagaagggccgtttatattatgacacacgaggatgtaccgctctcggacgtaatgtaccgcgtgggtattcaaacgcagtcgtattttacgaaggcatttaagaaggaattcgggaaaacgcccacccagtttttgcaggagattaagaagtagtgtttgcaccagaccggtcgcatcagtggtggatccaggaaagcatctgacgtaaaattccttcctcaaaagaaatcaatacgcggtaaattctccacatctctttttcatcttccctttgccggcttcatggaaatgcaggagtatgactggtatgccgttcctttacgcagcgtaccggtataaccggcgttattgcagcggccggcgacagagattattggtacagttgctgtggatgaaaaatagcatgtgagcagtcattgttgaactttgtaaaaaataattttatgggaaaagatagaaacggaactttccatcccggcaagggaaaaccctccggcgcaaacaaagaagagggacttggagcacaggctacgcctcccgaaagaatggatgaatacgaggaaataacagataaatacactgacggcccggatgagctgtcagataatgtacatgtattacatccgaacaggaatacttcaaaagcaaatacatccaggggatatggtacccggacaagcggtaagcctgaccatgaaaaggaacaggaagataacgtacgtaaccgtttccctgcggcacaggtggaagccagtcctccggaagagctgcctggtgtattcacgaaggaagccttcaatcatctggccgctatctccggagaatattgtgtatcagtttatattcccacacatgaatatggcgctgcagtgaatgatttatcagatgcggttctttttaaaaataagttgcaggatgcacagaaaatattacaggagaaaggtctgaaacagcccgaaactgacaagctgctcggccccgggtatacactgatgtatgatgatgacttctggcgaagccaatctgccggattggccatgttcttcgcccccggtttttcagggtatgttaaaatgtctgtatcaccgccagaacaactagtggtaaatacttctttccagttatctcccctggtacaggtgatgccggcaacagaagatttttatgcactcgttatcagtaagcataccgcccggcttttcaaagcagatgcaacgggcatgaatacggtacctgtaaccgggctcccggacagcacggccaccaaccttcccgtggaaccggatactaccaatggtgataccaattatcagggtattggcggcgccagcgatacaaatatcacagcgtacctgaaagcaatagacgacattcttttcagggaagtattacatgatcagcatataccgcttttgatggcaggcgcagaggagctgattacagtataccgttctgtttcgcgatatacatatgtgtatcctgaagcgctcaccggtaatcatgaatacgatgatacccctgctttgtacaaacaggcacgcactgtattgcaaccatactttaaccaggaactgcagaaagtaaaggaccggtacgccaatcaatccgctacaggccgcacttcttctatcattgcagatatagttcctgctgcttattatgggcagatagatacactatttgtggcgaataacacgcaggcatggggagcatttgatgaaatgaaaaatgaactgcatgttgatgacagcatgactggcaacaatgaagacctgctcaatatggcggtaattaaaaccatcgccaatggcggccaggtattcctgctcgaaaaagacgagatgccggctgaaagccctgttgcagcattaatgaggtattagtaaataaaaatcttttttatggaaagcaagaacacggaaaacaaaaacacttcaaagggagttccgggaaaagataccggagataaaacctcactgggaggtaacttcaattccggtgttacatcggatgacccggagataaagaaagccatcgagaaaaaagcgacgttgctggaagaccagccgccatctgaaaaagacagcaatagcaagcaaaagaaggtttaacaaaagaggacctgccagtatgaggctaccgttcagcaggcagggcttaaatcaggtggtaaaaagcctcatagagctatggctctatgaggctttttagtaagttcgcctgcttttgcttcgcagagcaggatataataatgagtatcacccgttttatcgccatatttccccggcatgtcgactccccataagtggctacaggatggcgggctacttttgtgtaacaagcattttttatgaaagcagccacagaacgaaaaataatccgctggttacatattatactcagcattcccatcctgggatatatttatggaccggtagccgccaacccacccgccgcaaacgcggtacgatgggtgtttctgccggtagttgcattaagcggtctttggatgtggaaagggcatctgctgaaaaagaaattaaacaggcagcgaaaaccgtaagtacctggttgtaataattgattaagcaagggaaatcctatcctctttattttgttgtatttttaccgcgtaaaaacccaggcaaattgactgttaaacaaacaccccggatatgctatctttcaaaatgcagcaccaggaatttgatcctcctgaagagctgcaacacgctataaagtgcttctggtataccagggtagacttcggggaattgccatcggatttcgagatactaccggatggttacgctgaaattgtttttcatttcggaggcgactgtcacattttccaccatggaggtttgcaaccattgccatcgccatctataatggggttgcttaaccagcctgttattttaaacgcgaaaaactgcctggaagtcatcggtatcaggtgctttccctggaccgtattcgatttgctcggactgccgtccgataagaaaggcgcgaacatctttgagcatccgatcgcgcgccttcaatccacattgagtaaatgtatggagggaaagaaaatggatgaagcgttggctcatgtaaaacagtatttcctggatgcagggtcgcaggttgctgcagacagtatgctattcaaagcgggagtagctatgagagaggcaaatggtgctataccggtaagcgggatagcggcggcggctcatgctacggttcgtacattggaacgaaagttcaagcaatcttctggtcatactgtgaaagacgtgtctggtgtgatgcgcttcgagcaggtacgaaaccagttatggctttacccggataccaaccttgccggtctggctcatgaggttggctatacagatcaggctcatctaagcagggagttcaagcgctacagcggcactacgcctgcggcatttgcgcggagaacaaagaaaagaaagctggctgttgccggcgattttgtcgcgtttatacaagcctgacgagcaggcattccggaattttgtgcttcaattatgctatatgaacgctacacttgtaagccaggaacccgcacaaaatcatactatttacgatgtaatcatttccggcgcagggcctgtgggcctgttcctcgcctgtgaactggccctggccaaatgttccgtcctggtactggaaaaggcggagactccggattctttattgaagcaacttcctttcgggatacgcgggctatcggcgcctactattgaagcgctttaccgtcgtgggttactgaaagaatttgaaatacataaacggcttaaaagtcctcattcaaacgcggtacaggggccgcgccgtcaggccggacacttcgccggcattccattccacgatggtgatattgacaggtcccaatggaaatatcgcctgccaggttcaacggagaccagtttaatttctgaaatgtacgaacttgaaacagtgctgatccgccgcgcggtatccctgggggtaaccatcaggcgggggctaggcgttactggctttcatcaaaccaacgatgacgtaacggtgctggcaggtgaccggtcgtttcaatgcaaatggctggtgggctgtgatggaagccgcagtgttgtccgcaaggcgggcggttttgaattcgcaggtacggagccggaatttaccggctactctgccaaagtggatattgccgatccccagcaactcaatcctggccgtaacatgactgcaaaaggcatgtacctccaatcacagcccggctacctgatgatccaggattttgataacggggcatttcatgatgcagggaacccaattacgctggagcacattcaggaggtgttgcgccgcatctctgataccgatgttaccatcagcgcgctgcatttcgccaccacctggactgacagggcgcggcaagccactgcctaccgcaacggacgggtacttttggccggcgatgccgcgcacattcactcgccattgggaggccagggactaaatctcgggctgggagatgccatgaaccttggatggaagctcgccgctaccatccaggataaagcgccggaaggcttgctggacagctactatacggaacggcaccccattggtgcacaggtgctggactggtcacgcgcccaggtggccattatgcggccggatcctcatgcccgcgcactgtatgcaattttccgtgacctgataaatacacgcgatggcgccacctatattgcgggaagggtatggggcatttttacccgctataatctcggtgaagcgcatccgctgacaggctacagtgttcccaactttgaattcggagatggtacaggcataggggacctgatgcacgatggcgaggggatattgcttgattttgacacgaatgctacacttagagcctggacagaagcatacggcaaccggatcaggtatgttgcaggcaaagcaaaagaccagttaggcgtaaacgccatactgatacgccccgatggtattgtcgcctgggcttcggacaacgaaccggattataacgaactccaaaaggctgccgcccactggtttttgtaatgcaggaaaaaagttgacgaatgacggaaagtttgccggatatacgcttatttttaccagatcacttcctgttaaaaaaatctatatggcggatgtacacatcgtctcgtccctgagcgggggcggcatgctcaaatgggcgatccaaaagaaaatgctgaccggagaagtattcgctttcaatgacattcccggcaccggtccgctggatgatggaaaaaagcgaatggcatttctgcgcagcctgaactttaatgcagcaaactggcccgtgaatttgaggatatcgcatcccgtcctgaattgttgagggaatgcgatgaaaatggcgtgttgcagttccgggaactttccgcacatgataacctgctattgtcacattgtgataaacgctggaagcccgccgtccgggtaatagggcaaacgatggggtttagtgatccccgcaatagccttggagatgggtttgtcagctcaaggctggaacacttaattgtgagtggtcaaatcgaggcggacggaatacgcacctctatgagaacgttccgggtaaggcttgccaaaaagtgatcacaggcgctgctaacgaaaataatgcaggatgattttgctgattgtatccgcctgattaaaaaccatgagatgtccgccgcctttgatacgatagtcgggatgcacaaacctgctggcgattaccctgtcggctgtgccatgtatttgaatggttctttcaggtgtttctttattattccaataagcaatgcctctcagtgcccagcgaaaaaacaacacatttgtatcctgcaataattttgtcagttcctttttatcatttggggaccgggcgccaaaataacgataggtaagaaaattggtccgcctgattaatacacctggaataagccggtataaacccagcttcatgaaaaagaactgtattttattcaactcatcttttgtctcgacagaagagatgagtaccatttttttcactgatatttgtttggatacttccaccgctacaatgcctccaaaagaaagcccgatgatatacggattttcaaccgtgatctggctctttatcctgcctgcgtactgcgttatcgattctttgggtaacgcggggatccagttgatgtaaactttatggtatcccggaagtttcagattcatgaatatacttgaatcggcacctataccactaaaaagataaacggtcttttgttcttttttagctgtatccttcagggtttgcgcggcccccgggaagctacagaacaaccataaaataaaaagactcactttcacactttgcaccataaatttccttgcttcttgccagcgataaacgttcattgttaacgttgcagtgtgcgatattaccaaaaaaattttaaacagaggattgcactttcattacatcgtacgcatatcaatgcctatgcaacctctgccggtaatacctttgctgttactgcgaagccgtttttctcctgatttccaggtattttttgattaccggcaaagaagtaataggcaatccggatttttctcctgatatttaaatttggtttaaacccacgctggctgatgatataccggctggtaacaaatcttttttaataaaaatactattatgagaattcgtgtattgttcttcggcatttcttatttggcttttgtgtgcgcttgcaataataagggcaagcaacaggcaggcaccgctgattctatcccaaagaccgatgttattgcaacgacggagaataaatcggccaccgcacccgccacctttaacgttgatgccataccggtatcagaaaaagaattaggtgctttccccttttttactttgccggaaggtttagagaccatgaacaaacctgttgagcgtaagtttgaccgtctcttcttcgccatagacggtaaaatggtaccgctggaaggtcgcatatggaaaagtaatgttagcgaaataaaacaaggtgagtggtcccttcctttttttgaaaagagttatgatgaagccatcaaagctgccggcggcgtgaagatatttgacggatcaatttcgaaagaagaatatgaccgctacagcccgggcgcttcttacttaggggaggacggttctatcggttatacggaggaccaaatcaaaacttatatcattcgcaggaccaatggaagcaatatttatatccagctgtccggcacctccgcccagggcaagctgaatatattgcagcaggaagggtttaagcaaactatcaccatgctgaaagcggatgaaataactaaagacctgaacgaaaaagggaaagcaattctatatatcaacttcgatacagataaatccaccctgaagcccgaagggaatgatgcggtggcggaaattacaaaggcattaaaagcaacccccggtttaaaagtggccatcaatggttatacagacaacaccggtaatgatgcacataacctgcagttgtcgaaagacagggccaaggcggtgctggaggcgttaagttcatccggtattgacaagtcacgcttaagttctgaaggatttggttcagcgcagccaattgctgacaatggttcagaggagggtaaagcgaaaaacaggagagtggagcttataaagaaatagctcccgcaggtggcgttgaataaggcggcaaggctatatttgcagcccgataaataaacattaacatgaaaagattattgctttgccttgcgttcaatatgttttccctttccatgtacgcgcagcaaactggctgcaactgcgcagtgacgttggaaaaactgatgaagaaagtggaagccgaatacccgggttttggggtaaagactaaggacggatcatcctacgaagaattaaaacagcatctgaccagggaggcaaaaaatgcagatagcagcgcctgcgaaaaaatactaaaaaagtataccgatttctttaaagatccccatttatgggtaggttcaaatggttctcccttttcctccggcagcagtggttcagcagcatccctcgtgatcgacattccggatttccgggaaaaaattaagctcacgcgggatacgctggagggggtgtggtccacagaggggtataagattgggattaaaaaggggagtagaaatgaatacaccgggtttattatcgccgcagcatccacgcagtggaaagccggagatataaagttcaggttgtttccggatggttcttttgaatacctgatgcttgaccggtccaaaaaaacagggcactaccacatgcataagaaaagcatcctgtttctggatgcaataagtatggcgttggtcagagaagtaccctcaccatcggtaagtgcggcccagctggaagaaaaactgacggagctgaccggcttttatttcaaaaaattatctgcgagaacatcgattcttaaattaccaagttttgaataccggcatctccaaaaaattgaggagctgatttcgcagcaccgcatgcagatggagggcagcgaaaacctgatcatcgaccttcgcggcaatccgggaggcacaacagatgcttatcagcaacttctcccgtacatctccggaaaatcaatacggaacaccgggacagaatttctatctacccaaacttatatcgggaaccttcaaacctataaaaaaagcctggataagaatgccccgacagatcaaatagacaaacaaatagataaattaaaagaaaacctgggtaaattcgtgaactttagcggtacagataaacctgcctatatagaaaaggttgagctggcagcgaaaagcccgcggcagattgttatccttgcagataagggaacagggagttcggcagaatattttttgtttatcgcaaagcagagcaaaaaggtcaagttattgggcacgcccagttctggcgcattggattacggcaacgcatatcaggtagatttcggatgccccggttacgaggtatttattcctacttaccgggccatgcgtttgccagactatccgatagacaatatcggtatccagccggatatttatatggacagttctgtggaagactgggtggaatttgcggtgcggtatgttgaggaatgagataggtaatccaacgaaaattgtaacgatatgataaaatacgtaacctgcttcactattgcttttgtcttcctgttgttgtctctctccgtaaaagtcctggcacagcaaccaaaaatcgcaaaaggtactgtggagcggataaaagtgcacagcacattgctggaaggcaatctcagtggcgacagtgcagaccgctacgtttctgtttatttacccgccggctacaagtccggtactaaaaaacactatcctgtagtgtacttcctgcatggctacacggataatgatgcaaaattttacggcttccagaagcactggatgacactgcctcctatattagatactgcgttttcccaaaagccggatcaggaaatgatcgtggttactcctgatgcttatacccttttccagggaagtatgtattccaattcagttacaaccggaaattgggaagactttgttgcccgggaactggtgaattatatcgatagccactaccgtacccttgcacagaaggagagcaggggtttatgcggccactccatgggcggctacggagcattacggatcggggaaaagaatcctgatgtattttcaacggtatacctgctgagtccctgttgcctgaactctccggcaacggccgcggaaacgcagttcctccgggcagacagcatcaagacgattgaacaactgcaaaaagcagattttttcacgaaagcactttttgcatccgcggcggcctggtcacccaacccggcaaatcctccattctatcttgatcttccaataaaaaatggaaatatacaaccggaaatattgaataaatgggacgcgaaccgcccgttaaataatttggatcaatatatctataacatcaggaaactgaagtccattggttttgatgcaggcgataaagacagatccatcgcagaaagtatcagaacactggatgaggtactcagcaaatacaacattgcacattccttcgaaatttatgatggcgaccatatcaatcatgttgctgacaggattgaaggaaaaatgctgcaattctttgaaaaaagtttgtcgtttaaacaaaatctgaagtagggttgaggaccaattgtttaattcattaatattgcgggataatcacttatcgctcacccccgacttcatatatgcgtcaacgtatccttcaaaaattaatacctgttatcctgtgctcctgcatgagcaactatgtactggctcagaaagtggtagaacctactaatcacagtgaagagtgggccagggcgtaccagcctttccgtattgcgggtaacctttattatgtaggtacctatgatcttgccagctacctgatcactacgccttcagggcatatactggttaataccggcctggcttcttccgcggctgttattaaaaagaacatagaggcgctcggcttcaggtttagtgatatcaaaattctgctcaccaaccaggctcattttgatcacctgggcgccatggccgccgttcaggaagcgactggcgccagattcatggtagatgctgcggatgaatcggtggtgaagtccggtggcaaaacggattatgccctgggcggcgagttcagtgctttcaggccggtcaaaatctccaggctgctgcatgataaggatgtagttagtttgggagatactaaattgctggtactccaccaccccggccacacgaaaggctcctgcagctttttaatggaggtgaaagatagcagtaagacttacaaagtactgctggcaaatatgcctactattgtaacggaaaagaaattctcacaggtgactgcctacccgcagatcgccgctgactataaatataccctggataccatgcccaaaattcaatttgacatatgggtagctgcccatgccagtcagtttgatttgcatgagatacgcgaggaaaatgctctttataacccggcgctgtttgcaaagagggaggcgtacgacagggcattggaagagagtagaagggagtaccaggagaagattaagtaacaggaaagattgctattgtccggaagttctctgctcaatttcgctttgccatggatatagtccgttaaacagaccaccattgagaaatctattcagaaattccggtaaggaatcggtgagcgttaatgtattgttatctgataggtggctgatagtatatttgttttcatcctccttgtctaagtttaattcccaggtgtcacagtaaatacaatactctgccacgtgaaagccgttttgcacagaaaaatatgtgcttctttcctccccaagcgtgttatctatgatttcatctaaaggaatcattcgaaacatgtcttcgttttgttcgaatccattacaaaacaggtaaaaagtttttaagtcctgcggaagttttatacccattgtctgctcaaataagtcaatatctgctggtgaagctttatcgaaaagtgttatgccgagcattccgtggatatcctcaagttttaaaattatttctgtgatcgttggctgcatgcctgcaagatatttgaaaattccgcttgcgaagcacttatttatccaggctgctcataaatttttcaggatacctcgtaccggaaacgcttcccgcaggcatgatttcttcaatgctttgcaaatcttcagcagtaagccttaccttttcagatgcgatgttttcttccagatttttgattcgtttggtaccgggaattgtaatgatgtcttcaccttgtgcgagcacccaggcaatcgctaattgcgacggcgtacaaccttttgcatcagccagtgatttaatcttcgctaccatctccagatttttataaaagttctcaccctggaagcgaggcatatgaacacgactatcttttatatcttccggttttttatattccccggtaaggaagccacggcctaaaggtgcgtaggctaccaggccgatgccaagctcccttaacgttggcagcacttcagcttcaatatcacggctccaaagcgaatattcgatctgcaacgccgtgatgggatgaacggctgctgccttgcgtatactttttacggatgcttcagacaggccaatatacctgatcacccctttttgcaccaggtctgccattgcgccaatcgtctcctcaacaggtacggctggatctatgcgagccagtgtgtagaggtcaatgtagtcggttttaagtcgctttaagctatacatcactgcgttttggatgtattcggggcggccggttacagcacccgggcccatagcgccgttagggccgggagcaaccagttggccggtcttgacagagagaaaagctttgtcacgcttatgctgaatggcttggctgatcagcgattcgttatggccggcgaggtaataatcagcggtgtctaaaaagttgtgcccgagttccagggctctttcaatggtcgatatggattgtttgtcgtcagatggtccgtaagcgcccgacatccccatgcagcctaaaccaaccggtgataccagcggtccgttttttccaagttgtctgttcatagtcttgtgattagtttcatgaacaatattcgtggaaacagcgggaagaaggctggacaaaatccgtgaatatcaggacagatccctgaagaatgccgaaatggttttaccagtcacttttttaaataaccgggagaagtaatcagggtcgttaaaacccaatccgaaagccagctcctttacagaagcgcgctcgccatgggatatccggcgcctggcttcgagtataaggcgattagtaataaactctttaggcgaaagtccggaatgctgtttcacgatctggtataagctatctgtacttaatgccagtttgccggctatatctttaatcgtagggtgatcggtcaggttgtcctcaacaaatatttgaaaatctatccacttcgagatatgatcgttcaccggcgccttatccgtatcaaaatacgccaggttgatttcggttaacaggctattgaggtgcgccaggataagctccggatcagtatctggcgtgcttaataaaccgatgagcatttcgaagatggctttgagcctgacggcagttgctgaggtaacgcttatcttttgttggtttaaagggttaatcagaaagggatatggttttggcaaccgggaaagacaattttcatcaaagcctagtttaaaataatcgctaccatgcccagaagctggtaggcgatggatctggtgcggacgcaccatcagcaattgattgctttcaatatcgaattcttcgaggtcaacgccatgccgcgtacaaccgcttaccataaacagtataaagtaataaggtgaacgatgcgtcagctcaatctgatccgcgatctccgcggaaagatgcccgaaattcggagaaacgattctgatgggcagttgatcattttgcttatgatcgctaagcagtgacttaatagtttgcatcagcaaaaaattgttctccaaaagtactgacaatatccggatgaacgatgcttgcagggagccggcaaacaatccgaaacataaatgtcttctggaagatttccttcttcaaaactgcctggatattatcgtgtgatttttttctattaaaaagcaatctttttttgcaggtttcaaaactaatcgtaatattgcgatatgctaaagaggtaacatttatgggagctaccaaatcggatttatttactaaagaacaaaatgatatagccaatatggctaaagcgctggcacatccggcccggatagctattttgcagtatctcgttaaaaagaacgcttgcgtgtgcggcgatctcgtagacgagattggcctggcacaggcaaccacttcgcaacatctcaaggagttgaaaacagcaggtcttattcagggaactattgaaggagccagtgtttgctactgtataaatccaaaggtctggaaccaataccatagcattcttggagcattcttcaaagaggcggcggagattaaatcctgctgttaaaaaaatttgcttatatatatcgcaatattacaattatacgatgggggtttattgttaagcacctcgttgcggcacgtttcatataatcacgaagtcatacttaatactgaaaaagcatctttctatgactatccttccaatgacagcaacacatggtccacaggtattggccatttatgaagcaggtatttccaccggcaacgctacctttcaaacagcagcgccctcctgggaagaatgggaccagtcacatttaaaaaattgccgcctggtagcgacggaggacaacaggattcttggctgggcggcgttaacaccggtctccagcagatgcgtttatgcaggtgttgcagaagtaagtgtgtacgtagcgccggacgcacgaggcaaaggaatcggaaaagcattgctgcaaacattaattgagcaaagcgaagaaaataaactctggactttacaggcaggcatctttcctgaaaacaccggcagcattaaaatacatgaagcctgcggcttccgtatagtagggcggcgggaacgcatcggcaaaatgggtgatacctggcgggatacgcttttactggaacgaagaagcaaaaaagttggcgtctaataatatcctgataaaaatactatgcaaaattgtaatcctgctcaacgtaagaaactgggctttttagatcgttatctgacattgtggatcttcctggcgatggctattggaataggtatcggatatttttttccctcctcttcaggggtcatcaattccttttcctcgggaacgactaatattcccctggcaatcgggttaatattaatgatgtacccaccgctggcgaaagtaaagtatgacaagatgggcgaagtgttccgcaataccaaagtattgtccttatccttgctgcttaactggatcattggccctatcctgatgttcggcctggcagtactttttttgcatggatatcctgaatacatgaccggcttaattcttattggtcttgccaggtgcatcgcaatggtaatcgtctggaacgagctggcagacggaagccgcgagtatgctgccggactggtagcactcaacagtatcttccaggtattgctttacagcgtgtatgcttatgtatttatcacctggcttccaaccatttttggaatgaagggcattacggtggaggtttctatcagtgaaatcgcgaaaagcgtgggtatctacctgggcattccattcgcagcgggcatcatcagcagatataccctaatcgcatggaaaggggaagagtggttccaggaaaagtttgtaccatttatatctcccattacattaatagcattgctgtttaccattattgttatgttcagcctgaaaggggaactgatcgtacaaattcctatggatgtagtaagaatcgctataccactggtaatttatttcgccatcatgttcctcgttagtttcgctttaggtaaagctgcaggggcagattattccaaaaatgcttccatcgcttttaccgcagccggcaataacttcgaattagccatagcggtggcgattggtgtatttggaatcaattccggtcaggcatttgtaggcgtaatcggaccgctggtagaagtacctgcattgattgcactggtaaacgtcgccttctggcttcgtaaacgctggtacagcaaaatcgtggaagcgccggtaaccgctgttaaagcataattaaaaacgtttaaatttttaataagatgagtaattcaaaaatgaactggcagagttttaaagaccagttgcaaaaacatccggaacagatcctccaatttcaatatgctgaggacaaactggtagcaccttcttatcatatcacagaaatcaaacaggctcctataacttccgtagactgcggcggcaaagtaaacgcctggacagaaattattgtgcaattatgggaaccggttgaagtacaaacagatcgcgctatggcagtcaacaaagcattgaagatagtagacctggtggaacgcagcatcgacttaaatcccaaagccactgtgaaaattgaatttggcaatgctgaatttgatacccggcagatgtatccaaaggaattccttttggatggagataacctggtagtaaacctgcagccggatgctacccaatgtaaagcaacagatcgtggtatgacctgtggtacaccaaaaacggaaacactggcagttccggcaggattggaagctgcccaatgttgtacaccaggaggcggttgctgctgatcgttaatatttctaagaacatctaatccaatcttcaattattctatttatgaaaatagctttgttcagcgatattcatgcaaatttaccggctctggaagcattctttaaagatgttgatgaaagaaaacctgatgccatttactgcctgggcgactttgtaggatataatatctggcccaacgaggtaatcaatgaaatcagaaaacgtcgtattcctgcgattgccggcaactacgattttggaattggcagaacaagcaacgactgtggctgtgcttacaaaacagatatcgaaaaggccaacggcagtgtttcgatttcttacaccaaccagattgtaaacgaagacgaacgtacataccttcgtacactgccagcccacatcaaagtggaatttcaattaaataatgataagctgaacctgctccttgtacatggcagtccccgtaaaatcaatgaatatttatttgaagaccgggaagaaaaaagtatgctgagaattatggctgatgcagatgccgacattatgtgttttggccatacacataagccctatcacaggatcttgtcggctgaagcggaggggaatccacactacaggcacgccattaacattggatccgtagggaagcctaaagacggcgacccccgcggaggctatgtgatgctgcatatcaatgaccatagtagtattcatgataaaaacagcatccaggtggaatttattcgctttgaatatgatgtggagaaggccgctaaagcggtagaagacagccccctgcctgatgcctatgccgaaagtttgagaaccggtatttaagcttgctgtttatgcaacctacacatatttcgatctgggaagaatttagtacggaattgaaaagattcatctgccagaaggtgaatcaaggcgatcattgtaacgatattctacaggatgtttatcttaaaatatttataaatattggaaagatagaaaaggcgcagcacatccgggcatatttgtaccgggtagccaataatgccgtaacagactactatcgccgcactcgtgaaaatatagccattgatgccgcacctgtaatggcggaggatcatgaagtttttgctgaagagcatgagtatcgccttgcggattgcctccggccaatgattgaatcgttgccacaaatctaccgggaggcgcttgtatttacagaactggaaggattgacgcagcaacagtttgccgggaagatgggcatttctttatcaggagcgaagtccagagtacaaagagccagggaaaaactgaaagaagaaattatacgttgctgtgaatatgagtttgataaatatgggaatatccttgcctgttgtaagaactcacctccgggtaaaaattattgtgccagcgataccgtcatttaagtgttaagctacaggtccgtgaaggcactgtagctttttagtaattacttagtatcgtacatcccctttttcctggcccattctattttggccatttccatatctgcaacaaatgcgggggatttataccaactggtaagcaggtgccatgctaaattccgcgatgcctcattgtcgctggggtagtggattcccattagttcccttgaccaacggacttcttctgccatctttataaattgcgctcttttctccggtattatttcactgaatattaacgcctctgtaaaagaccatagggtatgtccgctgggaaaagacggggaactaatccgtgccagtgggtatagccggggctccaggtgataggggcgtgggcgtttaaaatatctttttaacctgaattcagttactctgatatcctggatacaatgtaacatcagctgggtgatggcgggaaaattctgatcattgaaccaatcaccaaccgggccggcaatataaaacagttgtttgcggttttcggcatagtcagcgtccaaagggtttattatgtttggccacgacccgatgttggctatatattctgccctgcggatttcttcccgcgttctttttgcctgcaactgtagcatataatccaattcagccctggtctgtaaggaactattggctggatatttaatataaccaggcagcttttcttcatcttctttactaagatagtaggtccgcatgagtgaattggcgagcgctcctttactatattcactccatgggaacgtaatggtatccagtctttcatttgcagggtccgcagccggactcattgccgccaacgatttgtaatgatttgatattggttctaaaggatgtacagattgcgcgtatagcggtgcattgatcattgtacttgcgactacaacaagcggcaaattcttaagacatagcatcagaccttttttcttttccattaacaggtaatttttgtgttgaagaataatatacagcagtaagacgcaggacattgaaaaaggacgcagcaacagggaaaaagggacagccattatttaccggccaatgtatattggctgtttttcggaaattttcctagattgtgcttcatttacggggtgtcagccaatcaaacatataacgaaaaagaattattgtcgagaatagcagaaggcgacgagcaggcatttgctgccatattcgaccagtattatccattgctttttacatacgtcaaccggattatccaatctacccccgaaaccgaaagcattttacaggatattttcatgaagatctggcaggggcgtgaaaccttgcagtttgtagagcgattcagcccttatctctgggtaatgagccgtcaccatgccctcaatgcgatgcgcaacctggcacgccgcagcgcattattagatgattttgccaggcaggttcctgttgtggaaacagaggaaacccgggagtggcatctttccctcatcgaccaggcgattaaacaactgccggaacactgccgtcaggtatggatcatgaaccgggtcaacaaaatgaaacaggcggaaatagccgcagcgctgggtattgcattgccaaccgtaaaaaaatatatgcagcaggctatcggcctgatcacgcaatacgtaaaagatcattcttccctgggactggccattacacttttactttctcttttttttgaaaaaaaataggattcaccgtatactttttgaaaagccaggtgtcatttataggtacgggttaatttatttcatatgaatgaacagctaaccgaattgtttaagcgttattttgaaggcacggctactgacgaggaacaccaggaattaatggagctggtgaggaagtcggacgatgtattgctggagtcagtgatgcgccggcgctttgaagcgatgcaggacactgcggtgcaggcgcccggtggtgctcatgtattagcagctattcttgaaaaaccggtacggatcaaacctgtaatgcaacattggtactgggcagctgcagctgcaatcctgctgttggtaagtgttggcggctattttcagttgacgcatcaacagcaaagtactgttgcagatgcacaaaaggtaacacatggttacgagcgcgctacgctgacccttgacaatggcgccgttgtgcagctggatagcacagggcaccgtacattgcagcagggcggcgctttggtacagcaacagggcggacagctcgtatatgcgccttcagccaacaaagatgcggtaacatataatacattgcgcaccccccgtggcggacaatttaaaataacccttccggatggaacattggtttggttaaacgcggcgagttctatccgctatcccactgttttctccgggcaggaacgccgggtggaaatgaccggggaggtttattttgaagtggcaaagaatgaagaaaagccctttaaagtaagtataaatggtaaggcagaaataaatgtactgggtactcactttaatgtaaatggttatccggatgaacgcatcataaaaacaaccctgctggagggatcggtatcaatgttgattcctgccaatcagccggtattgctcaaaccagggcagcaagccacggccagccagggagcgatcactgttgccaatgatgccaatatcgaccaggtaatggcctggaggttcgggctctttaatttcgaccgcgctaatctccagtcagtgatgaatgaactgagccgctggtacgacgtggatgtgcgttatgagggacaggttccatcgcggaccttcaggggaaaaatcaaacgtgatcttaacctggcacaggtactggaagtacttcaggatgtaaatatcaaattcagaatggaagggaaaacaatcgttgtatataattagccatcaaaaatcaaccatgtaaaaagccaaaagccggaatgcgtcaacattccggctgtaatttggcaatagtcaagtccggatagatcttgttttttaccaaaccaaccaaaattatgcaaaaaaatgtgaaaagtgtgcgggcccgcggttccgggtccctttatctctatcaaacattgccgcttaagagcattgcgttcattttaatgttttttgccacacttcatgtcagcgcaaacgtgatggcgcaggccaaagtatctatgtcagtgaaaggggaggaactctcaaaagtactggcactcacggaaaaacaaacaggctatgttttcttctttgatgaaaaattgttgtctgctgcaaagccggtgaccattacggcaaaagatttaccactagtgcaatttctcgatcagcttttccggggccaacctttaaaatacagtttgcggaacaccactattaccctttctgctaaagaacccgcgactaaccgcgctgatctgccgttgcaggagaatatgattaatagtggccagatagtaataaaaggaattattgcagatggagatggtaaatttctgccgggcgtgtcggtaaggctgaaaccctcaaagataggcaccactaccaacgacgccgggatatttatactgccggaagtaccaccgggtacttatatgctggaaatatccagcatcggctattccactaccagtagaaaactggttgtaacagataagccattagaactcgccttcacacttcagcaggaagcgatcgaacaaaaggaagtggtcatatctaccggctattccgtcaggaagcccggagagctgaccggcgcggtacagaaaatatcaggagatgaaatccggagagggatcacttcctccgatcccgcgtcattactgaaaggaagagccgcaggattgtatatttccgaacaagatgccgccgaccccaccagcagcggcggacagatatttgtgagaggccagagcagtgtggcaggtgttggcgtagaccaggtgaatgagtttgtggtgcctgcgctgaactatggcccgctcatcgtaatggatggcgtaattatgccgaatcagaacctgaaagaactcgtcaccccacaggaaatacaggacatcaccatactgaaagatgccgccgctactgcgatctatggatccagggctgctgcaggcgtcctggtagtcactaccaaaaggggaaccaacgcaaaaccccggattaatgccgaggtgaaatatggcatcaatcaacctaaccgcgggcgcatgaggtttctgaacggtcctgaactttatgacctgcaaaaacgcttctataccgaagattattcgcagaataatgccagcctttctcccatgttccctacgttggacaaatacctggagtatcgcctgcccacacaggaacaggtggataattcctacgactggagtaaatatgctttcatcaccaccaacactacggaagtaaatctctccgccagcggcggaaacgaccgcactaaatattatatgggcggctcttattataatgagcaagccactggtgttcttaatggtttaatccggaaaacattccgtctgaatctcgaaagccgtttaacagacaggctcaccgccactgttgctattaatgggattatgaatgacggtcgtcaggatcagggctacaccatcagcagccttcaaagtcttgttccctgggcaaatccttatgacgcgaacggatcggttacccaggcacttaattttaaaatgggtggaacgcagcaggtcgttgataatccgctgttcaacaggcagtataatttttcaaaacggcagtcgcaattgtttttcgggtctgttaaactggactataaaattactgattggctgagcatttccagtacgaactctggtaatcttaactacagcaaaaatacccggtataccgatgtgagaacttataacggaggcagttccttttttgccccgcagggctttttgggtactagcaccgccaatcttatgtcctatcttacctccaaccagttagcctttaataaaaaagtgaacgaacatatgttccgtgcgctggccggtatggaattcggacaaactaccgtggaagatatgctggtaaatgtaaaccatgtgcgcgccggttatccggttatttccctggccagggaaatgggcggtccggccgatttatcgctctatggcatccctactaccaaggcaggtaatattgagggtgggaaagatgttaaggccatttattcgttatttggagaggcaggatatacctataaaaaccgttacagcttaagcgcttctgtacgcagggacgcatccagtagctttggcagtgataaccgctatggcaccttctactccggcggcggcgcctgggtggccagcgatgaagcattcctgaaaaatgtaaaatggatcagttatttaaaactccgggccaactatggaaccagtggctctcaacttggcgataactttctcacaagaacgttatacgatccaaggtatacgtacagcggggccggaggcgccacgatttcggtattaggtaacccggaactcagatgggaagtaaccaaatcatggagtgcaggcattgacatggagatctttaagcgtttaacagccaccgtggacgtttacaaacgccgctctgaagacctgctacagaaggtgttattgccggctttggcaggttttccaacacaatggcagaatgcggccaccgtggaaaacaaaggggtagaactggtactgaatgctcagaatatacacaaacccaatttctcctggagcacttccttcaacatcagctttaacaggaaccagatcgttaacgtggccaatgactcgttaagacagggatattatccgcaaaacagttattatctttttaaaggagatgatattaacgcattaaaagcagtgaagtatgcgggtgtagatccacaaacaggaaagccccggtttgagaaagcgatttttgatgcgaagggcaataaagtgggcgtggaatatgtaaatacaatcgctgaagtggacgccgcttcagacagcaggcagtttcaaaccatcggttctttccagccacggttctatggcggccttaccaacaactttacctacaagcaattttcgctgagcgtattaatcacttttgcactaaagtatacgatcattgataattatgctgcttcttcacaggtgtcgcgtgttggccggctgaatcaacttgcctacaccaaaagccaggtaccctggacaacgcccgggcaaaccaatgcaaccgagccggcactttattaccaggcaaatactgactattttggatcaagcaggtatatgcgtgatgccagtaacgcctctctgcgtaacgtgcggttaaattacgatctgccacagccgctgaccaaccgcctgaagttatccaactttaccgtgtatataagtgccgacaacctgtataccctctacaataaatatatcgtaagctccggtcccgaaggcccttccgtgggcgaggcacaggactttggcaattcggccggcccgttaagcatccccaaacgatatgtatttggattacaggttacattttaattgaaagctaaaagtattaaaatgaaaaattacgctatcatatttttaatctcccttttcgccatggcctgcgataaaaggattgacgaaatcagcccgctgattaaagtggataaggacggagagctatcgtcagccgcaggaattgtggaatctaccgtaggaaactactccttgttacgcgaaaattccactccgtcttatgacgagccattgctaaacctttccgaaggccgtggcaacaacatcaccctgcggaccttcggacctgcagacaaaataagcgacggtttcttttttcaaaacagtaacagccccacactgggtttcagcagcgatttttaccgcggttcttaccagctgattgtaagcatcaataccacactggaaggaatcgataaattggaaaaaacaaacctcgcttccctccctgaggccgaccggaatagtatattgtatgcaaagggagaaaatcattttctgcgggcgcttgcttattttaacctcatcaggttatatggaaaaccatattaccagaatgcggcaggcaatacaggtgttgcattaaaaaagacaagtgatgtaaaggagatacctgcaccatctactgttaaggaagtgtatgattttatcacggaagaattgaagacagccgcacaattgatgaaaacccccgtggtaaaaacaaacagctttgccagcaaagaggctgcatgggcattgttatcaagggtgtatttgtatatggggggcagtatggccagtccggatgctacttataatcaggcggccgtaacctatgccgacagtacgttaactcaaaatggcgggaaattggcactgctgcagggaaacgattataagaacctgtttgccgatgaccaggacggatctattggccgggctaagttcgccgccaataaagagatcatctttgcatttgataacatgaccggcaatacacgcattggcatttactacaattatgatccgacttatggtatgggtgcgctttttatcccgtcttcggatcttaagcaattatttaccgcccaggatatccgcagtaattttttcaaggtcaataccggaacaggactaacagaaacaaccaaattactggtgttactttatcaattgcttacccgcgctcccaacatctttttgcgtaccggcgaattgtacctgaacagggccgaagcgtatgctaaaatgaagaattacacgatggccagggccgatctccgcaccattcacacccgcgcaggactgcccgaatcggacatcaacagcatcgccgaccaggacctgcttgctgctatcctcaaagaaagacgtatggagcttgcgtttgaaggacacgccgggtatgattatttccgcaatggcttacccatgatccggaaggccgccgataacaacgggaaagagttgatcattcagcctgacgatccaaaagtggtgctgactgtaccaaacttttaaggggactttatttacgatcatcttttgtcatagaagccttcaggcctctaaaggatactattttgcatttcaaatttcaaaaactaacaaaaaatgagttacaatctgaagatttcgaagactgtgtgtctgacgcttctttctatcctttgtttcacggttgtttcattggcacaggaaaaagctaaattatttgtgggcgacaaagcaccggagcttcgttacggaaaatggctaaaaggcacacctgttaaggagtataagaagggccatctctatctttttgagttctgggcaacctggtgtggcccctgcattgcatctatgccacatctttctgaattcgccagggatcacaaaaatgaagtgaccgtagtagcggtgaatatctgggaaaaaacaggtgacaaaccttatgaatcttccctgcccaaagtgagcaaatttgttaaaggcataggcgacaaaatggacttcaatgttatcactgacagcaaagaccagttcatgggaaatgaatggatgaaggctgccggtcaaggtggcattccctgcacatttatggtgaaagatggcattatcctgtggataggacatccgatcgaattggattctgtagtaaaggtggtaatgtctggaaattacgacgtagctgccaccaggaagaagctacaggaaagaaatgaacagtcagacgccgcagcagctccctttcagggcctgatgaaggagtatgacaaagccattaaggataaccaatacagccatgccttgcagctgctggattccggtattgccaccatgcctccctttgccggaacattcggtttctttaagttccaaaccttactggaacatgtgaatgaagattcggcaatggcttttgtaagaccatggcaggccaccaagccaggatatgtaggctctgccgctgcggtaattgcaagaaagaagggatggaagaagtcaacttatgaatatgcgttggagttgctgaatgaacagctgaaagtaccgcagatgcccgcctctatggtttatgaagagatggccggcgcttatgccaacatgggcgattacaaaaacgcggtagactaccaggaaaaagccattgcaaccgcaaggcagttcctgaaagatggtaaattcgcaggttttatcatggaagataccattaaggaatctgaaaagaaattggccggatataaaaaggagctgaagtaaaataaaccgggcatcaactacttaggtcttccactgcagacctaagtagtttttatacataacggaaaatgcctactgatcaaaatctattggcagataaataccacgataaccattttctttaagacagttaataacatcatctgcggtaaagaaaaatccttccaccctcatcatcctgtcttcatcttccaggtcaaaggttatcctcaggtatggatatatctgcaagagatcacttattatattcccggctgcaacggcggattgaacatctgttttgaaaacatttaccatcgtcataaggtgattgctgtacattactttttctttcctatcagcgaaaaagggttgaacgatacccctacattaaaatagaaacctggatcgggactggtctggaatactggcgatccgaatgaatcttcctttctgaatatcctgccggatggggttatcctcacacctgtttttgcggcaaccacaaaatactttgcgataagatgttcataggttagccctgagttgatatctaattgcctgtattcgtacttttgagaagtaccgtctatattgtacaggtaaaaggaggttctgttcatctctgctcccagcgacacacggccattggtgaatacatgctttcgcaggtaagcactttttgggagaacaacatctgcaaccagtccgttattgaatttatgctcataggagaaaattggtataaccggcgtttgtgcgctcggatcaatactgaggaggataccagctgtcatttttgtgcgttgattggctttcaggaccattgttcccgtcgctatccctctaaccctttcaaaatgcttgtcactgccatctaccaggatactggacgtatagatagttcgtttattgaacaaggtggaaaaataagtaaagttgacagatgaaaaaagataatggaaatctccctcaacagtggtaactggtcctccaacagatgttgttaaaccggcatccgtattcgtatacacatatccgatagtagcacccaggaaccatgtttttctttttataaaattgatatttgtactcacttttacctgcgaaaaactattgaccttattatcaggcaacgacttcccgtttctctccgaagaaaagttgtaaggagcggaatgggaaaactctatattaaagggacgcgtaatggtgaatttatcggcggcataagccactacccgttggcgcacatccgcgctatctttcacagcgccgggaatgctgtcaggcgtctgcgaaaagccggttaccgataaagtcagcaaaccggcgactaatgacgcggtattttttgaaatatccatcttctttattttatacttttaatgatagaccaggaaaaaaaatttatcgttgatgagacggaacaaagaaaggatttaaaccatcgcagttttcctgttttctaccaagccggttacattttatatcaaatcctttccggccggaatttggtagaagaatagcgggggtttgtataatttctggtagccgtaggatatatcgttctatatttgtgtgggatgtcagacatcctgtaatattatgaagaacgatctccgggagtcaaaggataagaagcttatacaactgatcattgacgaccggtacaggatttggcgtcatactatactattgattggattccttcctgtaattttctgcactgacgagatattggaatactccgggccctacaggtattaccggctgctatgtgtgtatggatctataatggcgatgtgttatgttaacatgaatgtgctggtgcccaggattttttttaagggacggtacgtaagatacctgatagtgctttttttgctggtatcggtgtttgtagtactgatggctaatctattgagtgcattctcctcatccgggcgactgccggcgcacctggttatgcccgacaggaaaatggggttttatgaaggaacggttatattagtccccatcatcctggtcaccaccatgataaagctcttccagcgatggatgcgggataatgaaaggatcgccgagttaaagagcatcaccctgacaatggaactgaacgaattgcggaaccagatcaatccgcatttcctctttaatatgctcaatgggatcagggcgctgctgcacagcgatccggagaaagcagacatggttatcatgaaactatccgaatttcttcgttaccagctctatgagaacaacgagacaagaacattactcaggtctgagataaattttctgtccaatttccttgacctggaaaaactcaggagagataacctaaccgttagtgtagaaagccctacagcagccacggtactcaatcatatctttctgccgcctaatcttttcactacctttgttgaaaatgcggtgaagcatagtgtgagtataagtgaggctgcgtcttacatcagggtcagcatagctgttgacgtgaataggctttatttcagttgtgttaattccacagatccgggatatataccttctgatgaaaagaacagcggattgggattagcgaatattaagaggcggcttgaacttttatatggcgctgattatggtcttgagatcacttcttccgggaatgaatataatgtaaaactaacaataccgttatgaactgtattattgtagatgatgagccattggcaagagaacaaatgcagtcaatgatcaaagaagtatcccagctggagatattggggaaattctccaatgcccccaccgcactggacttcttaaaagaaaatgaggtagatcttattttcctcgatattcaaatgccgatggtaacgggattacagtttgccgcacaattgcccaggcaaacgcttaccattttcaccacggcctatccacagtacgctttaaagagttacgagctggacgttatcgactacctgcttaaacctattgaaaaatcaaggctggcgaaagcgattcataaagcggagacataccggaagctgctttcagatgataccgagaaaagcactattgagtccaacaccgttgacttcttactgatcaaatcagagcggaaattccacaggattagttttgcggatatcaaattcattgaggggctgaaagactatgtagtcatgtatgtcggtaaccagaaactgattactgccatgaacttaaaaaccatccaccagaaactaccacaacagcttttcctgcgggttagcaaatcctacgtagtgaattcgaagtatatagattcatttgatcaccgaagtatatttctcggagatgtagagatcccaataggggaggtgtataaaagagatttcttttccgtcttttcaggcggctcgcttaacccggaagagtaaacggggttgccgtggaaacggtgaatattatacgaggttttccaggccgtaggatgccagtttatcaacgatgggcagtgcctttaagcctgtcttagttaaactgtattcaacccttggcggaatttcaggataagccgttttggacaccagtttgtttttaaccaaagcatttaattcctggatcagcattttttcgctgatgccgggaatcgttctttttagatctccatatcttattaccctgtcattgatctgatacaatattagtaaagtccatttaccacctagcagtccaagggttctccttacggggcagttttcgtcgctaggattaatttttgattttttctccattgattttcaatatttcttaccacaaagtaagtaccctaccagttggtaggtattttcctaaaggtaagcaatacatacctttacgcaatgcctgcgataaaaatgccggattttaagcatccggcaaatactcctgggatagatagaaattatacacttttaaaaccggtaagaaatgacatcaaaagaaataattgaaggctactttaaagcgcttgaaacaggagacgttcctaaagccttttcggtttttgcgccggatgccaggtggcatcaaccaggaaaccataaattttcgggtgttaaaagcggcctggaagaaataggcaatatgcttggaacaatgatggaggatgtagcaggaagtttggttgttaaaccgaatggcgcattgatggcaagcgacaatttggtagcctgcccggttcgattcactgccacgaaaggaagcaaaagcatagacatgaatggggtcgatttatttgaagttaaagaagggaaaattacgcaggtctggctattttcagacgaccagcagcaggaagatatgttctggcaggactgagtaaacagagcctattttgactggaagtccgctatggtagcggactttttgtttttctaaagcccttttaacaaattaaatgggctgatgttttggatacttgaagaaatagaagtaagttggaaatccgtttatcctggcgagtttattgcctgggcgcgcttgtatctataaataataataaaagaaagaattatggtaattgtaaacagtttcgcagaatatcaagcgtatgagggtaaagaaataggtagctctgagtggcataaaatagaccaggaacagatcaacaaatttgcggatgcaacactggatcatcaatggatccattgcaatgaggaaagagcgaaaaatgaagggccattcaaaacgactattgcccatggttatctgacgctggcgctgattccttatttatggaagcagattgcagacatccggaatgttaaaatggaaattaactacggcatagagcggtttaagtttggtcaggcggtgtttgtaaacgatgaagtacaattgaaagcgaaactcaattccatcgtcgatttaagaggagttaccaaagtagtaattggcgctacgcttagtattaaaggcaaggcgaagccggcttatacaggtgatgtggtgtttttataccatttttaatggtagtttatcaaatcaaaataatatgacgcaatgtgccagtgccggaagcggtgccaaaagataataatagcgtaatattcagccgttatatttgcatttatgcaaatggatgactggaatgatcaggacttatggcaacgtatccagcaagatgacaaggcggcgtttgaatccgtgtaccgttgtttcgttgacgtaatctttgccctggtatttaagcatatagataaccgcaatgatgcagaagatgtaacccaggacgtttttttaagcgtatgggaacaacggaaacaaattgtattgcagaaaaagatcttctcctacctgtatagtgtagcccgttataaaacattccgttacaaccgcgataagggacggacagaccagtaccagcggcaatgggaacatttcctgaacctggaccagtcgcccggcgccacccccgaagttttcgtgaaagcagaaatgctccggctggaagccaatatgagcagggaaatagagaagctgccccctcaaatgaaaaagatttaccagcttaattatgaagaaggaatggatacagcgcaaatagccacacaacttattatttcagaacatactgtaaaaaagcacctcgtaaatatcaaaaaacgcctgcatagcatggcgctccgtttgttctgatcctgccttgccgcgtgcaatattaacttaatgttaagcccgtttcaccaactacttcaatttcttcttttctacactattctttcaggaaggcacttaatgtaatgagctttttctgacacagatagtatgtatcaaaaaaccagttttaaaacgctgttagaccgttacctggaaggcagctgcacaccggaggaagaggctttgctggcccgtttctttgagcaaagcggcgagcaacagaaaccggcgcacctttccgagcaggaccaggcccgcatgtttatggccttccgggactccccacgtttcagcggacagcctgtaaaaagaagcttactggtaagcatgttccgttaccgggtatggaaggtagctgtatggcaggctgcggctgtcctgctgctattgctgggtttctggggctgggataaggtatcccgttccgggaaaatgattgcctataagcagatcagcaatcccaaaggaaccgtatccaaagtgatgttgccggatagtactgaagtgatattgaacgctaattccagcctcagttatgcggttgatttcagtgagaacagggagctgcagttaaccggtgaagccctttttaatgtaagtaaggacgagacgcatccttttattatacataccgccgggggaatacatacaaaagtactgggtacctcttttactatacgcagttatgataatttgccggaaacaaggatcacggttataagcggccgtatccaggtgcaacatgcagatacggtgctgggaatactgagtagtaatgagcgggttgtatacaaccggcagggtggcggcagtcggcatgatatagtagcagatgccaataaacaagcgggctggatccgtgggcaatgggagtacgaaaacatgtcgctgcaggagctgcaggctttgctgtttaactactacaatattcatgtaattgcgcatgggcctgcccagcagtatttgatagctaatgccaatatgaactttacgagccgccagtcagcggaagacatcattaatattttttgtaacacagctaattgccattacaagtggctgaatcatgccaccgtagaagtttattgaccatactgatctaaaatagcaaagccctgctgtaacagggcggttgctcttcaattaaaggaaataaaaaacaaatgtatgaagaagagacgtttactccaatacgtcaggctacgctatgcgcgttatttatccctatgcttatggttgctgctaatgcagttgtatccgttattttcccaatcacaggacaaacagttcagcctacgggttgagaaaggaccgctggaacaggccatcagcaaagtaagaagtgtatccggcgccagtatcgtttttcataaagaagatgtaagtggcattaatattccggcacaggatattcgccagcagccggtagaaaatattctgagaatgctgctgcgggacctgccgtttaccgtggaaaaaaaaggagctggctggtttattgaaaaagcagtaaacagtggtaaaaaagtacgtattaccggtcacgttagtgatgcacaatccgggcaggctatacctggcgccagcattgcggtgaagggtactcccggcggtacacaaacagataatgaaggcaactttgctttgtatgcagatgataacgctgtaataacagcatcttttgtggggtacgctgtgcagatgattgctttaagcggtaaaacccggctggccatccgcctgaaacaggacacaaaaacactgggagctgttaccgtggaagccaggcgcagggctggtacagaaatggccttactgacggaaagaaaaaacagcagtgtggtttctgacgccatctctgcccagcagattgaaaaaacagccagcttaactacaacacaggctttgcaacgcgttacaggggttaccattacggatgaaaaatatgtagccgtgagaggattaggtgaccgtagcgtggtggcagaactaaatggcgcccgcctctcttcctccaacccagaccgcagcgctgtgccgttagacctggtgccggccggcttgctcgaaaacctcaccatttataaaacgctcacacccgaccgtcctgccgatgcctctgccggactgatagagctgaaaacaaaagcagtaccggaaacacaggtattggaatttactgcccaggtgggattcaattccaatgtaggcatgaacggacaatacaacggtttctataataatgacctcggcttcttcggacaaaaggtaagcaagcataacctgcgcccggattttattgacctgggtaaacaatatcctggcggtttaccgcagatacagaaaatgttcattcagagccgtaacagcccggagctggctgcagaagccatgcgggtaagcaggattatgcagagctttgacccggtgcttactaccaaataccaaaaggccagtcccaaccaggtatatactgtatcctatggcaatactttcagggtatttcacgggcacgtactggggttgatagccagcgccaattactaccagcgcaccaacgatatttataatgcacaacgtaaccagtacagccttttccagggagtagtaaccggttcgcccagcatatttaacccgctttacatacctgctttcgttacacccaactatcgccggctgaataattacttaaggtataccgaaaatacgggtacgcatacactgagctatggtggactgctgggacttacctaccagttcaataaacgcaacgaaattcaggctcaatacataggcagcaggggtgcagaatccgaggccaataatcttaccggcgcctggcagaacaccggccttaactttccggtgtacaacatcatcaaccagctccgtatcacttaccgcacttttgatacttataattttcagggggagcaccaattcgtggataagccatggtcgccgcgtttaagctacaacctcagttcctccaggagtacacaaacggaccccgacttccgttccaccgacgtggcggacctgcgtactacccgtttccaggatcctaacggagtaggagtagggcaggatacctatgctttcgtgagtggcctggtgcatggagtggataacgataacagcaacattattgtggcagaccccaacggccgccagtaccgcaagctgaatgaaaccaactacaacgttaaagcagacctgagctttccttttaaaacccgcgggcttgatcagctattgaaatttggcgctaactacctcagaagacaaagggacttcaccgaaaatatattaggtatcccaggttctaccctgggaggtggcggtatacaactgttgaatgacgccaggggaaatatagatcaactggtatctcctgccaacataggcttgcagaatccctcccggtatgatggtgcaggcgagccaagagtaggtggtttcctgtaccaggtaaagaaagcaccaaataactataaaggatattatgaaacacgcgctttttatggtatgctggatgctcatgtgcagaaggacatccgcattacaggcggggtgcgttttgaatctaccgatattgaagccaatgtagatacggcggatgtatttgttccgcagaacctgaatgcacttaccggtttacccaatgcctcggtgagttacagcacccaaacgccgcatacccgttatgtgagtacctataaaccttattattccgccaacctggtatactccggtatccgggatatgaatttcaggctgggctacagcacttcgctggcaaggccggagctgcgggagcttactaacgtatacgagtttgatcctttccagtttgccgtcatcggcggtaatccggggttgaaaaaccaaaccaccaggagtgccgatttccggtgggaatggttcacggcaccaggcgaagtattatccgcatccctgttcaccaaaaccattcttaatcctttgcagcgcgtattcatttaccagtcacaaggtaaccagtctaccgctccggagtttccgctcatcatctaccagaacgatcctaataacggtaaagtatatggtttagagttagaggcgaggagagacctgggcaaattatggaggccattgaaatacctgtttatcggcactaatatattgctggatgtgagcacgattgataagaaccccgaacgcctggatgcttcgcgcatcaatgatcggcgctccccggccaccagccctgtatttgaacaggcgccctatgcggtgaatgtttacctggattatgccaatacgcagtcgggcaccaacatcaccggcagctttaatatggttggcgcaagactgatacaggtgcagctcgatggtacacccgacttgtatgacaggcccgctccggtgctcgacctggtgttcagccaacgcctgggtaaaaagtggctggccaaaggttttgccaagaacatttttgatcccgcatttaagcaggtgtatacaaacccgggtaactacgggaagtattatggcactgaatatatctatcgtcaatatcacaaaggagcagagttttcactgggccttacctataaattattctgatgtatatgaagaagaattttacgcttgtatcactgctactggttggtatgctggcaggagggtgtatgaaaataaaagaagatagtaagatacccctgctggatgttaccaacagctccgcttcgagtatccgcatgttcaactttgccagcgcagcgattgaaggaaccgaagtagccatcaataatgtgccgttaacggctttcagacaaaccggcggcagcgccggtggcggtaccacgctggggttattgctttttccctccggcatctggaccagtggcgataacggcaatcccttctcagtgcctgtcagcttgctggataaagaagggaaagcacacatcgtgttgagtagtttagccggtactcccattctggataccgttattgcaggcgatgtggtgcatccgaaggattactacctgatgagagacaacagcctgaaagtgctggaacgggataacataccgcctgcccgtgcaggatattttaaagtacggattattaacctgggcaatccggcaagcaatgtaacgggacttaatggcgcggtttctttaacctatgcggatggcactgaggtaaatcccttgttgaacaatgtagcctccggcaaaattaccgcctatgcagagctgccttatggtgcctaccagtttaaagtatttctggccaggggcgctggtatagatgtaacaaagcagctggcggaaaggccgctgcagccttattacaactcctgcaatccttcggacaatatacagcagggtattatgccgcagctgcgtacgtttaaggccggtggtgtatacagcattgttattacggagaacttctacaaaacgcttacctgcgacctgcagaacggtagtttaatcacaaacggttaccggctgataacagagctgaatccgggagtaaattatgtatatgcccgtatgcaggctgtgaatgcaatccctggtaaacaggtaacaatattggtggatggcaagccgcttggcgggcagctggactatatcgggcaaacgacccctgaaaaagcggtacagcctccgggggatatgtatgtacaaggtaatcaccaggtgcaggtaatggatgcatccggcagggaactggttaggaaaagtattaacctctaccccggagatcattacaccgtatgggcttacgagcagccaaacggtgagccggggttgctatttgaagccaatgaaatgacaggcaccgtctataccgccacttatcatcccaacggcgctggaggcggtgttattccggacgacggtaccaatggtacaccgcgcagaacacggtatccatacgcctgggagtccagattccttaacctgagccctgatctgccttatgctacgttcaccaacgattaccagctttttttacccgttgatggcgtcagcttccgggataccatgcgttatcccgctgcttatgtgaacctgccttcctgcgtgcaaccgcttcaggatgtgtcaatgatttactccctgccattcattgcgccttatcagcccgataatcccaatggcaattcagagctcggctatttcccgcggcagatccgggtttaccggtcggtagctggtccgctgccggaagtacccggcactgtgttgccggatataatgccgctggacaccaggcaggcctttattgccaatgatcacttgtataccgacccccgctttaaacaaccggaaacaggtgtatacacggtggctgtggtgggaagaacgtctaaaactgctcctgcagctgaaaaggccaggatcatcgtcattaaacataacaagtagtgtatatgaaaagatatatctccatactcttcgcgggcttatgcgcaaccgcctggccggggtgtaagaaatatgagattgaaccgcaggtaaaggatcctgcctttatacgggtattcaataatcttacaccaaccctggactttgcacatgggcagcaggtgacgccattccttacgtttttaatggatccaaaaacagatgctgccggcataccaacagatgctactgtagtaggcgatttcctcggtacccggcaattgttcagcttatcctatgccgccaatgaagctaacagctcagtgggcaacaataccactggcggaccgcttcctcatcctgacgcgcctaatcttacgccggttaagtatgagtatccgggcaatgcgcacatacttaccgccccggtaatcaatggctttgatttatcggcgtgggcacaggtgccttccggtaaacacaggatcatgtttgtgataagaccgcagaacggtattgtatttaaagatttgtctgcttccatccgcagtggtatcctgctggatacaaccatcatgctggagaaaggagaagtatatacgctggaagtgatttcccgggatctggacaatggcaaatatggcctttatatcaggaaggagcagtttattcaccaggcatttgaacccaataagctctatgtgggctttgtgaatctttccggcgaaaaaacggaagatgcacgcaatggttttatgaacgtttttccggagagggtaaaagtaacaggatcctacctgcgttataatgaccctgcgtcgcaggcttcaggcaacgtgttttacacgccggtaccggggtacgataatacctatttaaccacactcagtacccgtatggataccacaatttcctatcacccgctgcctatgttgccacaaagcgactttttttaccagggtttgctgcgtacgtacgttgacgttatgacaccagagcctgccaggcagggcactttgccttacttcagattccagtacctggatgctgatgtgccggcatatggaagcctgtttaaaacgaactgctctgcaaatcctgctgtatataataactataacgtggttactacgaacgtaaagaattatctgcctaatctaaacctggtggtaaataacaaggggacttaccatgtgtatcccacggtgaatatcatggaaattgtttacgaccgcgtgtatatgatgcagatagtgcggggatttgaacagataccttaaaatgaatgatcatgaagtacttatattttttattcttattttttttgataacggcctgtgtaaaagaaccggcggatgcgccgcaggcgactggtggcgacaggccactgctcaccattctgaagaacaactataacttcagcatgttctttagtgccctgcaacgaacggggctggacaaaacactggagggtgacgggccgtttactttgctggtaccggataacaatgcatttgcagcttccggcatcagtgccgatagtctcgctggtatagatacggcatcactggcaaaactgctgcgttatcatattatccctgcccgggttaattatacagccatacctcaggccattaacttcccatatgaaacattggcagggctgccggtatatatgggggtgcccataccaggccccaggcaatttcaaagtcttaccgccaatatcctgcacattaatggcgtagccgtcagtaaaaccgatatactggccaggaatgggcttatgcatgcgcttagccgtgttttatactacccggctgcttccgtgcaggaagtgttggataaagatccgcaatacagctatttcgtacatgccctgaaggaatttggtatgtgggaacagatgggaaaaccaggggcgcttactataatggccccggccaatgagctgtttgatcagtatggtattattgaggaagaattgaatcctgcccattataggcagacaatggtgactgcttacatagtaaaagaccatcgcttctttactactgacctgctggatgcaccgctcagtaattcacagccaggtattctcacaccggagtttcttcaggcaataaacgccggctcctttggcatctggcctcttagttacaaacggatactggacattgtaggaccgccttactggggagacccttatatctatggccctcctgcaggtttcattaacagtgatcatctcgccggcaatggagtagtgcatggcctgaatggtttgataatgatgccggacagcgcaagaattaatccttaaacaatcagaaaaaataccatgacatcttcatctatttatataaaaataaaactggtattgctggcatgctgtgttgttactgcattgaacgcctgtttaaaggcttcggatgcaccggtaacacccgccgtttccattccttttaagggaacagacctggcaggcaccctggcacaggaaaactcgcttcagctgtttaaccgggcattcaaacgcctttccctggagcaggaaataaataacggaagcggttatacgatatttgcgcctacagatgcagccatgaaagcagcgggcctggatgaaacggcgattgataaaatgaatatcgacagcctgcgcaggttggtcagctaccaggtagtctccggctcattggacgatcaatccctttcccagccggtaacagccacctatttgcttacactgagaaaaacattgatcacaaaacctggcggggcagcgacttaccagtatgcgccgctgtatgtgaaggaagatgatcagctgtactttaatggtatgccggtaaaaaaagaagggacagcgataccggctaccaacggttatatttatcccgtgaacgccctggcaactgagattacaggcagcattaccctgctggatatcattaaaaatgatccggatcttagcatgtattaccaggcgctgttattggaagacagtatactagctgtcaattacctttcgggggatatcgctttttttggagataagacgctgaccggcatgtatcccactattttggcgcctaccaacaaggcgtttgaagatgctggctttcataccacggatgacatccgcacctatgcaaacagcacttttgtggggcttgatcccaacgattttatcaccttctatttttcaccgctggattctgtccttaaaaggcatatcatttttaacggaccacttgccagcagcttctattacacccaaagtacagtaaggattttttacaacgacctgttgaatcctgtattcaataacggcaaactgaacacctacacaggcggaacaggtgaagtgctggatgctgttgtgcgatacaggctgccgcttactttttcaaatgttaatggggaagcgcatgtgaaatacagtactgatcctgctgatccttcctggcctttgccgcgcaatggagtctacacggttgccaacggttcattgtgcaagatcaataaacttttttatcccatcataaattaagcagcatatgactattacaaactgtttacgccgccaggtgttttttatcctgctgctggcactggggatcgctggctgtggtaaagaagatgcgcctgctcccggtacggagcaggatggcagcaccatcaaatatatattgaaagataacttcagcttcggggtattatacgccgccttaagcgctaccggaatgctggacaccgtggctaagcccggtccttatacggtactggcgcccgataatacggcctttagccggcagggagttaactaccctgtaaatccctatagctttcaattttttacacccggttggttacagcaggccatgcgttattccattcttccggaacctgttgccttcggcagtcttccgttgaatacagtacaggtatataaaacaaccggcggcggcaacgtatacgtgaaaacgttcgaagaagccggcgatacagtagtaaccgtaaatggtttccggttggtaagccgggataatgccgcttcaaacggttttatacaggtgctgccgcagctgttaaaccctgagctatatgctaccaccgctgctgcaatacgcagtgatactactaccgccttattcgccgctgccatgcaacgtgccggtcttacagcgctgctttcaggcagcgatgaatatacagtgctggtgccatcgaacaccgctttccagcaggctgtcatcgcaggtatgaatattaataccctggatggtatactgagcgcagacccggtaaagttgtccgcattgctgcaatatcacattatcaaaggacggtattttgaaggagacctttaccggcatgccactgttcacccggatggtatcagtacgctgaacggaggtaaagtacagattggaggtaatcccccggggttcaaagccgttaccttcctgggcgccggcaataacggccagcccgcagcaatagcaatacctccgcaatattcacccgcttcaaacaatgccaacatgccctgcggcaacggggttatccatattattaaccaggtgcttattccctaaaatttgcttattcatgaaaatgaaatacataccactgttgctgtgctgcctgtctttcctgctggcggtatcctgcaccaaagataagccggtatataccaatggcgccggcgcctccctgtttaaagcgctcctggaaaaaaaagagctcagtctctatcaggcagccctgaaacgtgcaggtatgctggatgctgcaacatttgctgatggaggaccttatacggtatttgcacccgtggattccgcctttatcaatgccgggcttacgctcgacagcattaataaatacaaccccgattcgctggccctggtgctgaaatacggtatgttgtacgggcgcattagcagcagcacattgatagggttttattcacaggatatgctgaccaggcatccttcattaaggccgaggctcaataaaaactattatggcattttcttcaatggtataccattactgccacaaggcagcagcaccctggcagatggcgttttacacgagctggcaagggtaccttttccccaatccactaacctgatggattggatacggcagcaaccggacctcactttctttgcagccgttctggaccgcactggttatgcaactcaggtggctacagccggtgatcagcggggtcgcctggtgtttgcccctgtaaatgatgcttaccggaaaataggatatgtggacctggatgccatttataacgcagacctttccctgctgcaggcgccactgcagaacatggtgcgcagcccccggttgtttaccgccgatttcataggtggatattcattctggtatgatggtttttatgtgaatgcggatggatttaccatgttcgcctccggcaacgtagcacctatacatatcatacagccggatgttatgggtaccaatggcgtattacatgtagtggaccaggttattttactcagataataattgattgcaatgaaacacaactacactataaaatattttatatgcagctgcctttgtttgctgttttgtttttacagtagccgggtggccgcgcaggaaaccagcgcaggtttacgcgggcagataaaggatgcttccgggcagccgttgcccggtgctactgtaaaagcggtgcataccgcttcaggcacaaaatatggcaccgttaccagcaccgatggccgttataacctgcccggcatgcgggtaggaggaccctatgtcattgaagtaaccttcctcggcatgaataaggaaaccagtaacattgcgcaaattgcccttggcgaaacgatgatggtaaactttgtattaacagataatgcccgcaatttatccggtgtaaccatcaaagggcaaaagacgggaccaaaggccaataactttggcgcagggcagaatatcggccgcgaccaggttcgcaatcaacccaccatttcacgcagcattacagatattacaaaggcagtaccgcaaagcacaaaggacaactcttttgccggcaccagtttccgttataacaatgtaacaattgacggtgctgttaacaatgacgctattggctttagcccttctattggcggacaaaccggttcttccggtatgcctggttcatccacccgcaccaatgctatttccctggatgctattgaagatatgcaggtatacctggcgccctatgatgtgaagattggtaacttcaccggcggcagcatcaacgccgttagccgctccggcagcaatgaagtgcatggttccgtatacgcttatggcaggaatgccacgctggtaggaccagaccataccggctctgaacttaatacaaaaatgccatcagattttcatgactaccaggcagggttcagggtaggtttccccatcattaaaaacaaactgttcttttttaccaatgaagaaattacccgccggcaagaccccatacaacaggtagccggcagcccgtctgccaacggcattctcagcatggcggatgcacaaagcattatcgactatagtgttcatcactataactttgatcccggtacggcaggtatttacaatgcatacgccaactcagagaagtactttaaccgccttgactggaacattaatgaccggaaccagctggcgatccgcaacaatactatacgctccaaagccattaatatggaacgcgaccagtttgattttcgctttggcagcattgcgtatgagcagttcaataatcagacctctacggtagcggagctgaagacacggtttaacaacaatttctccaacaatgccatcgtaggatttaccagtattcatgactatcgtacaccgctaagtgatgcttcgtttccgcaggtacagatcgtgggccgtacaccgggaaccactattttctttggcacagacagggaagcttctatattcaaccagcgccagcgcactatagagatcacagacaacctggtatggaacctgggtaaacacacccttaccatcggtacgcacaatgaattgtaccggattaattatggttttgtaaactcatggaatggcagggttacctaccaaagcatagacgactttttgaacaacaaccctgaacgcgtacaaggcagctacaactatgtaaataacagccgcgattatataatggcaaacccggtcgcagtgtttaacgttaatttctacagcgcatatatccaggatgaagtacagcttacagaccgttttactttgaccaaaggcctccgctttgacctggcaaacgtgcccactaaacaaatattaagcgataagacccgcaatgcttttacggatccttcatttggcaccacttatacttatacgccgctgaaccagataaccggtggctacctgggcaagatacagatctctcccaggattggtttccgttttgatgcttatggcgaccagtcgctggtgctgagaggcggtgtgggtatgttcacttcgcggatcccgtttgcctggttaggatatgccttttataacaatggcgacacctatggcgcctacgatcagaaaacggatggcaacccgccttatattttccagggagatcccatgcaacaccaaccaggccacggcattggtgattttgcgggtaataacgggcaggtgataacggataaaaatgccggcaaaacacaggtggatgtgatagataacagctttgttatgccaaaggtattgcgtggaagcctggcagttgattttaaggataaaaatggttttaaatatacccttgaagcgatttataccaaaacgatcaaggatgtaatgttccagcaaattaaccttacagaccgtcccacttatgccgtttttgattcggccgtgaatcatcagtatcaaccggtattccccgggcagaacaacctgaacccacagtttgccaatgcgtatgaaatgtccaatacttctaagggataccgttacagtattaccgggcaggtagcccgtgcttttcaatccggcttcggtttttcactggcttatacctatgggcaatccaaggacgtggccaatggcatccgtaactctttcgaatctaactggcaactgaaccaggcactgaatccaaatgacccgcagttggcttattccaactttgatatccgccaccggatagtgggtaatatcaactaccgcaaggcctggaataaaacatgggtaagctctttttccctgtttgtatctgcacaatcaggatcgccttttacttatggcttcgtgaactatacaccgcagaatacaccacagcaggtatcactggcctatatacccgcaaaagaggagactattaatttctttgcgcctactgaaacgcaaaccgcgggggagcaggcggctgcctttgatgcgtttattgatggcaacaaatatctgcgctcccggagaggatcattcaccgagcgaaatgcgggcagaacaccctggaatgccagtgccgactttcattttgcacaggaccttcatttgaatacatacgctaatgatccatccaaagtaaagaccatcacctttagcctggatattatgaacgttaccaacctgctgaatgcaaactggggcaaagcttatttttctcccaatacctataactctacttcaagcgtaggattattgccttatgtacctgccaaatcctcccagagttacccgatttaccagttcgtaaatcccggtaagccttattctgtggatccatttgcatcgaggtggcaaatgcaggtgggcgcgcggtattcattttgataagcgcatgtagtccgtgaagatcagcagccaaaatgatagacttgcctgacagcagcccgccggttctttactagtgggctgctgtcaggacgggcaatgatgactttgtctattccctgtatctcagttaataactgcatccatatcacttggcagtgagttgatcttcgaatatagaatctcctgccttgccggatataacggctacttttccgggaaccatattgtggcgaaataaaaggtgagatgattaatgtctgtttgttcgtatcaaatgattggtttggatatttgtgcaaatatctgggcgttaaacatgttgttaaaaagtatataaaattgacttataatcaatgtgcaaagaagtgaaatttatttttttgaaaaattccgatcatttcgccgggttaaccgtcaaaagataaattgaacaaaatgcaaaatttaaaagacaaagtcgccgctgtatttgctgcatccggtgagattgcgggagcagtagcgcgatcgttttcccaacacggcgcaaaagtgtatgtcactgcccggaacctcgatgccgtaaaaacactggcacaggaaatcaaagccaatggtggaagtgcggaagccgccaaagtggatgccttagatgaggctggaatcgataacttcttaagaaaagtcgtcgcagacaacggtaaattggatgttgtcttcaatggtatcggggcaaactacgacgagatgggaggacgtccgccgacaacagaggccacttttgcgcagtttatggctccactggagaagctttgcggttcacaattcctcacttcaaggatagcagcgaggtatatgatgcaaacccggtccgaaggaactatcttgctgcttacggctgcattgtcccggtccaagctttctaatgtggctggtattacggccgccagtgccgccattgaaggattgacacgggtgatggccgctgaatggggaggagatggtatcaaagtgatctgtatttgtcctggcgccctgctggaaaccaggcgtatctccgggtggataaatgctgctgcgcaacaatacggaatgcctgtggaacagctggtagcgcagtacaaatccctggacatattaaaaacaagtccgacgttgaagcaagtgggtgaaacggcagccttcctggcgtctgaaacaggggtagcctttaacagtcatattgtagatgtggattgcggcaagctgaacattttatagaatcctttttgtggtacattagtagttgcggcccgccgaagggccgcaactatctgttattgattaattatcttaatggaaaaagaggaacttcttttgtcggcaatagctggcgatatcaatgccttccaggcgctgtttgccggatttcaacatcaattgaaatcctacctgtatcgtttggttaccgaccgggacgatgtagatgacctgacccaggatacttttgtcagggcctttacaaaaatcggaacgtttaatcgcagatcatcgctaaaaacctgggtattcagaatagccaccaacctcgcctacgatcacttacggaaattaaaaagatggcaggcagatgcccaggacagggcggcggatctggccataagttcggaggagatccgggaggtcttttggatgacgcacgatacgtcacccgccggggcttatgaaatgaaagagcatatagactactgtttcacctgtatttcaaaaaccttacctatagaaaaacaggtggcgctgatcttaaaagacatttacgattttcaggtaaaggagatctgtctcattcttggtaaaaccgaaggtgtcatcaaacacctgttgaacgatgcgaggaatacgatgacaaatatttttgagcaccggtgtgcgttaatcaacaagaatggtatttgccaccaatgcagccatatcaacgaaatatttaaccccaaacaaaaccagcaggaagaactgatgaagctggaattggtaaaggcttcaaagaggtataaccgggagcagctttttgaactgcgcactttactggtaaaagctattgatccccttaatgcagcgggtactgattttcacgaggaaattatgaactgtctcaaaacagccattggtgaaaaaagcaatttttttgacagaaagcgggataaggcagagtaatccgttcccatgtaaaaaatgttggtaatcatctccctgtctccctgcggaattcccctggcggcataccggtagtattagaaaacaggcgtgagaaggaagccagatcttcatatcccacccggtaacaaatttcggagatactgagcttagtttctcccaatagttttttcgctatttccatacgtttttcctggatccatttgcccggactggtattcaattcttcccggaacctgcgtgataatgtccgggaagacatccccatctccttggatagaaaatcgaggcttatgacttccatgttgtcttttagcagtttgctgagttgtttttcaaagctgccaatcatctctgtaaccggaatctcataaggactttgaaattcgcgcgcaggagggagcagcattattttccttacacgtttcagctcctttgcgaaaccaaggtccgttaacaggttactgattaaatccagcccggcaaaacctccacccgaagtataaatattcccctgtttcactacaatccgggagggttcccagcgcactgcgggaaaccgctcctgtacggctcctttcaaccaccatgagatggtggcccgctttccatccagcaaaccattggccgccaggagataggaagccccgcaggtggccgcaataatggcaccatgccgttgagccgccttaataaatggtgctgccctttttgcttccactgccaataagttgtgttcgggaatagcctgtgctcccgcaccggccaacaggatcaacacgtcggcctttttagcaggttttgttgccgcattaaaagaaatagcagaacgagaaaccgcgtgtgtgtgtttagacacaaactcaaaagtaaaaatatccgagtcactcaacacatttattgcctgcaatatttctaccacactggaggcaatcgctgcataaaaaccggaaggcaaatagatgacgaaatgcatatgtctatttttgcatagtaattgtcagataagacatatcgaagataagaaacgtctggtaatattgctattcaaacaaaacaatgaaagcaataacatttaatcgcatcggcgcgccggaaaaagtgctccaattatctgaagtaccagtacctgctataaaagataacgaagtattgatcaggacaaccgcagcctctattaacccgggtgattttctatttattcagaacctgtacccggaacccaaaaagccagtattccctcagcagattgctggtaatcacggcgccggtattatagaaaaagcaggaaaagaggtagcgtttcaaccgggcgcgcacgtagcattcagctattataactcctgggcagaatatgtagcggttccggcggaatggctgattcctttacccgccggttatcctgctgaactgagcagccagtttgtaaacctggttactgcatgggacctgctgaagcagtcgggtgttcagccgggtcaatggttggtgttgactgccggcaactctgcgatatcaatattggtgactcaactggcgaaactacagggaatacatgtcatttctattgtacgtcgtataaaacaggtacatatactggagtcactgggcgccaccgtggtcatagacctttctgcggagcagggaaacagcgtacaacgcatcatggaggttaccggaaacaaaggcgtaaagggtatcattgataatgtgggtggcccggttaccggcgaattgatcaggtgcattgactttggcggtaagctaatcatcaacggcggcatgagtgctgagaaatatacactccataatttcgacattctattaagcggtctccagattcaaccgcatgtataccggtactttttcacaccaccacttcctgaagatgttaccatgctgaaggaaattgcggaaatatctgccggttttgcttcaaatgtttccggcaggcatgcactggaggattttaaaaaagccatcgaagagagtatatacttcccggaaaaaggaaagcatatttttatcatgtagttgaataacagggtagcagtgcctgtataattgttaaatttgagtgctcataacgcagttcactaagagtatctatacatggctatgaaaataaaattatgggaattgagttaccatgaagtggtacaggcgttaaagcatattgacccggtgcatgaagttgaaatcgtggaagaagtcatgatcacagaagcaaatgttcttctatgtaagtttaaggggaaaaggtttaatatctattttgacatagactatggggcagaaataaaagcagtcgacaagatagagcaggaggagctaaagatgatggaggaattaattatccgtcaattctcttagtttatatatttacagtataatagtatccctgatgttttcaccatttcagcagctggaaaaggtaaaatatacctacctgcataagcaggaactgattatttgttatgtagataatggaataactgtttacaaggaggaagcccttgtcaggctatcgtcggtttcgccatggtacgcctgtctgtttggtgactggttattatttcaaccggaaaacgaagggccggtccagtacctgcagctaggcagtctgcagccggccagtggtaccctggaaggtgattttttattatacaaggcgctgatcaacggtaatactatttatattccggccgctaataaattgctggcctttaatgagcatctgcatccagttcgtacttatatcgtgggaagagccccggtagccatttttaacgataagtatttcaggatggtaccgcatttgagcgctttttctttagcagataatgctaaaatatgggagctttctgacgatgcgttgctggaagataagaccatgcttgccgggagcttttttactttaagaaacggtgttttaattatccgctcaaagctggaatcatttaagaattatctgactggttttgacgccgataccggtgagatttgctggcagcaatacggttactttccggctacccagcatataggtgatgagatctttgtattttcttacctattcatgccggaattacagggccggctttgcattattaatagtaaatgtggggaaatacttaaagacgtcgatattaccggcgaactaaccagcaagggctttcaaccatcagatttttaccgcctggctgtccgggatcattacttatatattatggccggttatggcaaagcgttgtatgcttataacatgaaaaccgataagatcgactggctatataaatttgatattgcggcggaatggcttactgatataatatactgcaacggtaatttattcattactgatgatcagggaacgctgcatgttttcaggcaagattgaagacttgttatggttgccgggtcattgggcggcaaccaggattttactgtatggactgctggcacctacagtaataaacattgttttccaggtggtaaaaggagcactttcgctctgtttgcctggcagtacttacagctttttcaaatattttataggcggccccacccgcttgaaaccatgctcttcccgaaacctgtccagttcctcttcactcatatttttggcggccccttcactgagtttaataaagaattcttccatttttcccgcaggttgaaagaacatcaataaccgcgcttcaccttcacccatctttgaaaagctatggggcacttttctgggcccaaagacgctgtcgccgggttttgccttgtaggtaacatctccgacttttataaggaattcgcccttcaaaacataccaccattcatcctgatcgaaatggaaatggagagagggccttctttcatacgtattgattcaaacacataaatatctccgtcagtatcttttgaagaaacttttgtataaaatgtgtccccctccaagagattgatacttttattgaagcggtccgtgccagccttaactgaaaaacctttttcaattcttttctttactgattgagcaatcaggttaaatggagcataaacaaaagcccctactgctaagcatttttttaaaaattgatctctgttcatgtgctttttatttaataataacaggatttattttaggattgcaagcgttgtactgataagtataatggagcttaattgtttttgggggattatacagcaatattttacttgtgaataatattatggtagaaattacaattaatgcattcactgaaaagtgccggttagccattcgcggaaatgaatgagccggtggttgcttcccggccacgtcaataaccgtttatcacaaaccgctcagtcaatcctaccaaccgctcaacagtcctttttcatattcttttttaagcagttctttaacgtgacaaagattacaccgaacatgctttaaacctttaaacagataatcatgaaaacaaaattgctattagtggcaggcttgctgattatgtcgtgccttgcctgctcaaaaaccggtcctgaaggcccgcagggggcacagggaacacagggaacaaaaggagataaaggagataccggaagccggggcgccaccggcacggataatgtgatctattccacctggaggtcttttaccgggaaggttgcgcaatggcctataccggccataacaaagacggttcttgataatgggattatattggtatacgttgattttggctctacggtattacttgtaccttatgcctccaacgccggcgacataaagatgtatcctcagttctatgtaggcggtcttaatgttatcagcaatattgaactgaacgtttttcggttccgttatgtcatcattcctggtggtgttgcagcaaggagtgcgtcaggcgcggactacagtgattaccagaaagtttgtgcagattatcacatccaaccctgagaggtagggggcggaaactgttcagcaggaaaaggaatcccactaatttcattacatgcgtctaaaaactgattctgcaatgaaaaattgttagcttcctttttgtaacttctttctttttgatgatagaaataacggccggttactttcgccttttcatcattgcttgcagccagccaaacctgggtttcgtatccttttgccagatctccgggtgccgagctgccacccatttttgttggcacccaacccggatcaacggtattggaataaacatctttccattttcttgatacagcaagtgaaagcaataaaacataaaatttggagtcggaataagtgacatgatcaaatccgtttctggaaaaaccaatacttgcatcagcatgagtgtgcatatccgagcttaaatagattaatcgtttgggtcgttgcatcaaactggtcagaatataaggagccagggtattcactttaaatatctgctccggtgcagcgttatatactccggcattatggatgactgcatcaaactttcccagggaatttaactgttgcgccagttcctttgtttcttcgatattagaaagatcgccggtcacaatgccgtcagcacctttcagcttgccggtgatgtcaagttttctattttcatcccgcgcatgtgcaactacctgatgtcctttttctattagtgattttgctgctaataaccctagtccgtcggcagacccggtgataaatatccgtcccatatatttggtttaatacttatgtaaattaacgttcctgatcgggacgttacaaacgtttatcctttttcaaatacatgtaaggtctgttctgaatccagcacatacatgcggttgtcaaatacatgaaatacatcttcggctgcggggatcatagtacccctgcggcctgttttattggcatcgtgtatccggtaatgccataagaggtcgccggtttgtatattccattcactgatagtcgtatccaggatacctgccaggtacattttatcctctctgaatattacgttggaataaggatcgatacctgctgacttaatatgcgctgacaggtccacgccgtgaaggcgggcgccatccgcggcattgatcttccatatttccgtattcacaaagcatagtacggtctgatccgcggcctggaatctcatgccagcgcccttcaactgccagcataactggccgttaccggcatcgaggcagagtaggtagtctgtatgcccgttggtaacacctgcgtatattcgtcctccttccaactgcggacgcacgatgatctcataactacctgcaggcagtcccagttcatttatgtttacttcccacagaaggtgaccgtttgtttcgctcaaacaggagagctcctgctttttctcagtatgcgtagccaccaactgatcgccgttgccggtaaaaaggtgggtataggcgccatcagcttcccagataaggttggaatcccggaaattatatttgctcagcttccagccgtcagccgttttattgcggatgatcatattatcaccatacagcagcttgatctgcaggctgcctgtataattgaatggatattcctttttgacgttgctatctgtatcccaggcgatgatcttgtcctttgtccggatgatcacttcccggttcaccattgcggtaagcacaaaaggtgctgtatctaatgcgctttcagtaaccgaaagatggttgtctatccggataatagcattatcgctgtttttataaacaacgcctgctgctgtaatgagcggttccgttacctggtttatctggcggactaattgcatcatattattatgggactaaaattttctgctatcctttgtatttggaaatcgggtgccagggaaaccgggcccgggtccctgaaattattttttatcgggcatagtcatcaggtagctcgtcagcttttttatcaacccgttttccatttcaaaaacatcacagaatacaaggttgacaataattccatttttcgttttggcctgaacggtgccttctgcgatgactacattttcctcttctgtcatcctggatactttaataacaggcttgcctgtaaacccttcgttttcaatttccttgtcaaaagcagctttccctttatgcagataaacacccggaagcacccaggttatatcgtcagttaagcaggcaagtattttagcatggtcttgctggttgaaagcttccatgtatttggtaaccgtttctttatttttactcacgtggtttgattttgaaacataagtgaagctgctgagcagacatattataagaaacagcctggcagactttaagcagtgcatcattttgatattatttaccggttgataatagcgcattcaaacggtcaaacatgctgaaccagctttggtaggcgccggttttcctggcttctgcttctgcaacagtttggtgtagggtaagtttcgtttgcgtaccgaacgactcgaaagtcaccgtggtaatagttaccgctggccagtcttttgactttccagcttcggttgcgctgagtggggtgccttgctcattactcagctccattgtgaaaacgagtttttccggaaaagttatttcctggtatactcctgtaatccagcactctccatgcacaggatcgtgaataacagaatgaaatgtaccaccaactttaacatctatcgacttaaatactatagtgcatccatccggtgcataccagtgttgcagatgcctgggatctgtccatgcctcaaaaacaagttcacgcggcgcattaaactgatacgtaataaaaagatcttctttattagtcttcatttacctttggatttttgttgttgtaagtatttatctaatttttcaaacctcctggtccataatttcctggattgatctatccaggttactacctcatcaagttgatccagctgtacctcgcagaatctttctcttccgctttgtttgataaccagcagcccacattcttccagtattttcacgtgcagggatatggcctgcctggtcatatcaaacttttctgcgatggtgtttacgttgtacgactgtgctgcaatgaggttaatgatttccctcctggtaggatcggcgatggcctgataaacatctctcctgactttcataaatgcaagtatgtgcttgcaaatataagcgcaagtatttacttgcccaaatattttttagaatattgattttatcgtgtaaaagcaaggcgcgccttttttagtgagcgccttgttttagggtaagtttatggcatcgcctatatcgcgtattctcttatgcggtcgtgattttttcaggtcttaacaagatgttgtgctctatttctgtcatccttatgcttaaatggttaatcctggttgggcattttggtggtgtccatgaaaaatatttcccaggtgtgtccatcaaggtcctctattcgccgctgttgcataaacccgtaatccatcataggcgttggctctgttcctcctgcttttaatccatgcgccacaacttcattcattttatcaacactttcaacggataaggcaaacaggcctgcaatattgctttttgtatcagctattggctttttcgtaaatgtctggaacctttcgtgggtcataatcataacgaaaattgcatcgctccaaaccatgcattttgcctggtcgtcagaaaactgcggattgattacaaacccaatttgagtgtaaaagtccagtgatttttgaatgtcttttactgcaagattgataaatacctgtttcattttttaattttattattggttacagatgcaaagatgaaaagacaaaaatgaaaaaacctttacaaatgttgagaaagtaaaaatttatttgctatgactaaaaatcaggcttaatggagtagactaactgaccctattttcttttatccctgcaaaaataagccataaacaaaccgcagcctctccaatgaaggatgggaacagaatataagggaacaagggattagcaaagccgcgtgaaaggaacattataaagctgttaaggatataacataaccccgcaacggcatacaatatgcccaatacctttgggatatgccatgatttaaagataagccaaccgattatgatgcagtaaaatccaaaaaataccagcccgatggcatatccttgtgattgaaagtccagggccatggcagataacgctgccaattgatcaggttgaaaaatgcccgggtactctttaccgcccagaattatcaatggatataactggtataaaatattcatcgcaaatattgcatttgagatgatcacaaaaaagatcgcaaggatggtgctccctttgtagatcgggctaaataaaaggtaaaagaataatatcaccggcaacccgcaaataaagtttagcaggtcggcggaaaagcccaaacgatagaatagctcatgggattgtatgttcctggccgttgccatagcatcattgggaacagccaatgcctggcggacaaacacctgtgcgaacagcccggcggcaataactaccaaataaagaaaaccagcaattcgcgcattgctttttaaggaagggaaggagctgtcctgcattgggataaattaatatagcctgttgaatgagacataaagctattcatttacaatgattatttcaggaaaagcctcatatttacaattaacttacattccaaattatatgaaatccggtttcctattttttattataccgttatttttttcatttaaggcaattgcccaaacggtagaaccaattaagtccggtcagggagaagtggtgacgatgcattccggcatccttaaagaagatcgaaagataatgatctacacaccaaaggatgctgacaatcgggagaaaaaatatccggtagtctatatactggatgccgacaatcattttacccaaatagtagaatattctaaatacctcagccggcaggatgtgtatgttattccgccactgattattgtaggaataacaaatacagaccgtaaccgtgacctcactccatctcacagcaatattgattattatggaaaaccggataccactgctaattccccgtataagaacagcggagggaatgagcatctttttcaattcattcagaaagaacttataccttatatcgattcaaattacaaaactcaaccttaccgcatttttgcgggacactcattcggggcgctgacagccatcaattgcctccttaattatccggatatgtttgacgcatacattgccgtgagcccatccttctggtgggatcagaaatttttgctgaagctcgcggataaaaaaatgaaagcaggatcaactttatcgaaaatacttttttttagtgatggcaatgaaggttcttcacctggatcaacatttcataccgatgttttaaagtttgattccctgctcaaaaagcggaacatcaaaggattggattttgaatatatgagctatccggttgagagtcatatgaccgttactatcaaatcatattatgatggacttcggtttatctatcaccagtggccactacctccggtaagtgatgaggagatcaatcccgagatcattatgagacactataaagaattatcacaaaagtttggttatccgattttgcctgacgaagcatatgtcaatggatgggcacaatggatagtaaaaaatccggcaaccctgaataatggcattaagctactggagatgaatacaattaactatccgtcttcttcaaaagcctttgcggctttgggcgcagcatatgctttgaaaggagaaaagcagaacgctatcgcttcgtacaaaaaggccagcgaattgaatcctgcctcaaatgaaattaaatcgcgcttgttggagttgcagaaataacatagatatgccttctaccaatcaggtttttcaaatccgctaatatagacaactaagtaaccttcacatgtaagcctgttggacttacatggttcctttttgcaaactccgatggtgcaattccaaaatgtttcttaaatgcaaaagaaaagtgcgacaatgcttcaaagcctaactcaagataaatgtcggagggttttgcagcctctttttccaggagaaaacgggcttcgcccaaacgtttttgcactaaccagcgattaggcgtgtcgttaaagatcgctttgaaatcccgcttgaaggcagataagctacgcccggttaagtaggcgaaccgggcaacacttacattgaatttgtaatttcggttcataaattcttcgagatctattttcccgggaataccgtaatcaaagaatagtcccgataattctggctgcagttgcaacagtattaggagcagttcttcccgctttacatcaaaaaatgctttgtccatttctccacgactattgtagtaaggagttaaagatcgaataaacgcaggaatcagctcattgcttgccgggcgtataaagttttcagcagatcggaactttacggcatttatccggtgtttgtcctggaattgttttaagaacggttcatcgaaaacaaaaatgattttctcaatcacatactgctttttggtagcggtctgccggcccaaacggtttttacgggcaatgccatattcgcccgacttcaaggtgtaatttttatcgccgtaataaccgttcacacaccctttcacaacatagaaaaagagatgctcgccaatgaattgttctcttgctattgcaggaccaacgagagtcgttttgttgacagaagctttcatcttgatctccctaagttaatcatacttatcttaacaataataattaaacccttgacaatagggtgcgcgtctccgcaacaacgagctcctgaaattttggatcctgcaccaacatggagccgagcatgggcagtcctttttcgtcgtaataaatgcctgttttaccagactcgctggttagtaatgctgtctccaggcgtgccgcccgctttggggtgctccagtatttaatatatggagcgaccagcgggagcaaataatttcctataaaacgaaggaagccattggcgtccctgcctagtcccgtgttcggaatgaagcccggttcgatggcattgatgtgcaaccgtggcgtttcacgggatagagccagggccgcggcaaggatacattgcttggatgttgcgtatgcgtctgcccccggcattttagagccgccgggctcccattcaccgcgggcgcccgcctctacagaaataaagcggccaccgcggaagccggcggctttcgcaggtttccgcccgggatcttctactcccgaggcaacaaaagcgatatttgcgccatcaggcagatatggtataagttcctcggtcaacgcaaatggccccaggtggttcgtagcgaaggtcgtgtcccaatcctgcgcactccttgtggcacgcatttgcatgatacctgcgttgttaagtagcccggtaatcgggatatcgagcgagatgattgctgctgcagcatggcgaacactaataatatcagacagatcgcaaacgacagggaccgcatcctgccccttttctttaataagccgctgcatttgttccagctttttaaggtcccggcccactaacaccacagtaccatactttgcaagctcaagtgccgtaaggcgaccaataccggaggttggacccgtaataatgaacgccttcttattcttcaaaacagtctttgacatgattttatctttcttttaaatgatactgcaaaactcgccattaatatgcgcggcagttttcttcaaaagcccaaatttgttgtattgaaaagtccaaattggggagaccgtaatcattttggtagccggttagtttttgaaagactgtctgaatgcaaggggagaaagttgtgttttggctttaaacaacctgctaaaagattgcaaatgttcaaatcccagttcataagcgatctcgcttatggacaggtcggtggtggaaattctttctttggccctttctatcagcttttcatggatgtaatgctgtgggttttgccctgagtaaaatctattttacaccacaatgttactgagttacaccgatgttactgttatttttcagtactaagttactttagataacttagctggtctacctttgttgctcaatctttaaaaaaggaaataatgagcagattaaagaacaaagtagcagttattacaggtggtaatagcggcattggatttggcattgcccgggaatttaaaaatgaaggtgctaaaggagctattgttgggagaaataaggaaactttggatagttccgtagctcaacttggagataatttcatcgccataaatgccgatgtaaccaacatcgccgacctggaaagagtctttaaagagacatctgaaaaatttggtaaaatagacgtgattgtagccaatgcaggtggtgccgttactggggcaacatttggttctgtggcagatattggcgaaaccgactatgacaagacaatggatttaaatctgaaaagtgtttacctcactgttcataaagcactgccctatatgaatgatgggggttcgattattcttatcgcctcaaatgcggcgcatcgggcatatccgtcttttacgctttatggcgctgcgaaagccgctgtaatccattttgcaaaaggattttcaaacgaccttttagccagaaagatcagggcaaatgtaatatcaccaggtacaacagatacaccggtatttgacaggtttgttccggtagaacaacttgaagcagtgaaaaaatactgggcagatgtaatgccgataggcagaatcgggcagccatctgacattggtaaaacagcggttttcctggcttctgatgattcttcgttcatgcttggtgctgaacttcttgttgatggtggccttagctatttatctaaataattgacccgcgcgggtttgcaacccgtgtcaataaataattttcaaaatgagtaaattaaaaaaagaagtggcgagctacgcaattatcggcttcggcaatattggccaggccctggccaaggcgtttgcccgcaacggcatcgaagtatccgttgcaaccacgcgcaacccggaaagctttgcagccgccgcggcagcgatcgggccggagatccttcccacaacattggcggaagctgtgaaggcggacgtcatctttttagctgtccgttttgagtcgcacccggatgtggcgaaggcgctgcccaactggcaggggaagatcattgttgatgtgaccaatgcctatggtgtgccccctgagaaacttggagggcagccttcttccaggttcgtggcccaggcattcactggtggaaaactcgttaagggcttcaaccatttgattgctgccattcttgatcaggatcccaccgtacatggtggcaggagagttgtgttcctggcgggcgacgatgagggcgcagtagcggagattggtgcgctcgctgagaatctcggtttttcacccatcaaacttggagggctttcggaaggaggactgcttgtgcaggcgcgcggaaatagttggggtcaactgatatttaaggacctggtcaagttcgattgatcattcttgatcgcaaatttcgatacgatccttcctcatggacaaagagaatcacagtttgattgaaggaggtcgacgtcccgatctggcgtacgctcatttataggtctgcttgacgccttccagcccgggaggcgtttcgcttgaccgggatacaatagctaagcaggcggcaaatggtcttgacctgcttttttttctagaaaatcgtttgtttttataggggcttttaataaatttatttagcccaatagtacgccaaacctattttaaaaagggaaaaatagcccctgttacaaaatctcaatgcaggaatttaaacttgagtagacactgccttagagaatgtgtcaaagaatggcggcacagttccaaataaagcaacaattgaggatggtgccggaaatcagcggatagtcatttgggtcacatcacattttcttgttcacaaaaaagttgccggctcaaggttatggtttaatgaaatatgttccttcccaattgcatcagagatagaaagtggcggcattcttgttgtgtactccgtcataatttatgcttatgcaaccccgtaataaagacctgatcatcataaaaggcgcccgcgaaaacaatctccggaatattaatgtagagatacccaagaaaaagatcaccgtgctcactggtgtttccggttcaggaaagtcgtcactggtattcgataccatcgctgcggaagcacaacggcagttgaatgaaaccttcagcagctttatccggcatcgcctgccacactatggtcagccggatgccgacctgatgcagaatctaagtcctgccattattgttgaccagaaacagatcaggggaaatgcccgctctaccgttggcaccattactgatatttattcgttgctccgtttattgtattccaggataggaaaaccttttgtgggctattctaatgttttttctttcaaccatccggaaggcatgtgcccggtgtgtgatggtattggtaccacaacaaccattgacgtggaaaaattgttcgaccgcagcaaatccctgaacgaaggcgctatcctgtttccttcttttgctccgggaacagcattgtggaaacgctttgtgatgtcgggattttttgacaacgataaaaaactaaaagactattctgaagaagaatggcaattacttttataccaggaagaaattaaacccaaacacccagcgccggggtggtggccttctgcgaagtatgaaggcgtaatgccacggttcgccaaaagattcctggctaaagagccggacgacagccagaagtcgtggcagcaaccactgcggagggtggtaaccaaagggccctgccccgaatgcaagggagcgcgtctcaatgccagaatactcagttgtaagattcatggaaagaacattgcggaaaatgcggcgttgcaggtaagcgatcttataaaagaaatagcacgcatcaaagaacccatggcggctactatggtggccgccatcatcgaaagactttcacacctggatggtatcgggttaggatatctgagcctgaaccgtgaaacctccacactttccggcggcgaatcccaacgggtgaaaatggtacggcacctcggcagcagtttgtgtgatatgatgtacatctttgatgaacccagcactggtcttcatgcgcgtgatgtgcatcagctcaatttgctgatgaagggtttgcgcgataaaggaaataccgtattgatagtggaacatgatcccgatgtaatcagcatcggcgaccatatcatagatatggggccgggagcaggaaagcatggcgggcaaatagtatttgaaggcactgtaaaaggtttgctgaaatcgggtacattaacgggaacggccctgcgcaaacaaccacagcttcgggcaaaggtgagagctgctaccggcagcttgcgtgtacgcaatgccacattacacaacctgcaaaaggtaagtgtagacattcccaaaggcgtgttaacggtggttaccggcgtagccggatcgggaaaaagcagcctgatcaacggtgtgctgccccgtttgtacccagatattgtttgtattaaccagcacgcactggcaggatctgtgcgatcgaaccccgctacctacaccgggatatcggatgttatccggcagctgtttgcccgcaccaataaagtaagcgccggcctgttcacttttaacggtgagggcgcatgcccggcgtgtaaaggactcggcgtaacctcgctcgacctggccttcatggatgccgtagtaaccacctgcgaagtatgccacggcaaacgttttacagataacgtgctgggctatacgctgcgcggcaaaaatattgatgaggtattgaagctgaatgtagaagaagcgatacagttttttacagaagaagaggtcgtgcgcgtgttgcatcgtttacacgaagtagggctggattacctcaccttgggtcagccactggactccctctccggcggcgaaaggcaacggatcaagctggctgccgagcttgagaatacaggcaatatttatattttggatgaacccaccacggggcttcatttgtcggatgtggctaatttaacaggactcttgaaccggctggtcgacaacggcagtaccgtaatagctattgagcataacctggacgtgatcagccaggcggactggattgttgacatgggtcctggcgccggccgccagggcggcaaagtgatctttgaaggcacacccgctgatcttatcaaagacaagtcttcacaaacaggcatcttcctgaaaaaatatattcatccccgttagtacctgaaaaaaatactatcctgcagtgtcctgctattatgtaaattgttaattaagtttgatgtaaacatcgccattgataattttgtgaattacacggcttttattatctgataaaaatttcctttttatatggttcaatttaaacaacttttaattctttttttgctaaccggcactgcaacaattgcgcaggtaaaacctgaggaaatagccgatagtctttataaagctaaaaatttcaaagaagccggtaagtattacttaaaagcgacggagaaagtagattttaaggtcctgaaatcagataattattataacgcagcatgttgttatgccttaaacggtcaaaaagatagtgccttggttttacttacgagtgctgttaatagcggttataaaaatgccgatcaaataaaaaaagacactgatcttgaatctttgcattccttgccgggctggccggaacttatcaataacattaagacagcgaagaacagcacaacagatccgtataaggctaaactgatcaccagcgatgtaaagaacttttggaaggcatacgagctggctaaaaaagatacggctcacgcccttgatctttataagaaatactatgtggaacccgcttcaaatggacttgaggattatctgggttataaagtcaaaagcctgaataattttgtaaaatccgtaaacaccaagcctcaattttacgctgctgtacgtaaaaatactttggccgttgatcagcagaaacctcgaatgattcgaagctttgtcaagttcaaacaaatttacagcgaggctcagtttcctgatatttacttcgtgataggcgcatttaattcaggaggaaccagtactgacgcaggcttattaattggcttggatcaatccgcccggactgcagaagttcctgttaaagaactgaacttatggcagcggaataacttcgcagacctggaagctttaccacacctgattgctcatgagctcattcattttaaccagggcggacttaagggcgacaccacccttcttgccggggcactcaccgaaggcatggccgattttattggcgagttgatatcagggcacacggctaatgaacgcctgtttatttgggctaaaggcaaagaaaagcagatttgggcagatttcgagaaggaaatgtatttgaacaaggcccgcaactggatagctaattccgatcaggaaactgcagataaacctgctgacctgggctattgggtgggatatcagatctgtaaagcctactatgacaaaagcaccgataaaaataaagccgtaaacgacatacttaacataaaaaattataaggagttttatatcaaaagcggcgcaggggggatttttaggtaacctttttaataaaatttggaaaatttttcaaatcataaactggacccctttatattttaaaactggactgttagggtaaccaaactaaaaattaattttatgatgacccaaaaaggaggtgtgttatgaaagcaattatagtgacggatcaagctgcaggaaaggcaggaatgcagcttgtggagcgccctgagccgcaggtagcgataaatgatgttatagttcaggttcatgcatcggcaatgacaggggacgagctgtcgtggccctcgacctggaccgatcgagccggccgtgacaggacgccgtcgatccccggtcatgagctggccggtattgtcacgtctcttggctatggaacgacagggctatccgtaggacagcgcgtgttcggcctcacggactggtaccgcgacggtacgctggcggagtatgtagctgttgaagcgcgcaacctcgcgccactgccgttcgatgttgatttcacagttggcgcagccctcgtaatgccgggcttgaccgcatggcaggggctgtttgagcacggccgccttcgggcggggcagactgttcttgtacacggtgctgccggggtagtgggttcaatggcgacacaactcgcacgtgctgccggtgcttatgtcatcggcacagggcgcgcagaaggccgtcagagggcgctcgatttcggtgcgctggagtacctcgatcttgaaaacgaaaagctgcaagacgtcggtgaagtcgacttggttttcgatattttcgggggcgatattgccaatcagtccgcaagtttgattagatccggaggaaggctggtgaccatcgcaggtccgaccggggcccggcctgctaacggattggccattgattttgttgtcgaagcaatcccaaaccaattaaatgagatcgtccagcggctgcgcgagggacgtctgcagacgaacataggtaatacatctacgctcaacgacgccgttgccatcttcaattcgaccaatcgggtcaatggaaaaacgattatccgcgtccagccttaagtactccggccggcaaaattcgttttgagttgccttcagaacttaggcacggccccaatttgttgcagcaagctaagtaaatccggttgtccgtattcttcaataatctggttaagcgccaatcggtaaaagttcattgcctgaactttgatggattttccggttggtggaataccataaaatgttccgtcatgtgtaccccgcatggtaaaccaaatggctgctttatcctcttcagaaaccatttcttccaacgtccactgaatgtcggagaatcccgaacgcatcatgcctataatcgttaaataaccgtttggacctcttaatggctctgattgtccgggaacataaaactttgcctcgggacttataagttgctgtgccaaagtttcatcagcagtattgataaattgtacgaactgtttgaaaaaatcttcatgatatttcatggcgttattttttagcaaaattgatgcacaactgaatgctaaccaataaacaagattaagaaatagccttaatgtaggttaaggtatgaattatttcggcggcttctgtgcacggattttactaagaaattcgggagtaactcctaaataagaggctatttgaacattggataatcgcatggcaaggttcgggtattgttctaagaatacggtatagcgctgctgcgtgttggaactgaaatttagtaataagcgattctgaagttcaatcaacttttcttcaacaattaccctaaagtttctgtcaaactttggaacgtttacaaataaatataacaagtccgttttttcaatctgcagaattgttgaaggctcaagcgcttcaataaaaagtttacttggtttttcggaataaaaactgcctaagtcagcaatccaatcattttctgctgcaaagcttatattatgcgcattgcctttttcgtcagttccatacattttaaagcaacctgttaccacaaatgtataatgcttgcaaacaaagccttcttgcaaaatcatttgccttcgctttattaaacgctgtttcgttcgttcgttcaacagtttgatttcttctttgtttaaaggaagatagtttttaaaatattcaacaatgggttgtgctgtcaattctttaagtcgttttgaaagtttatgctgtttgttatagcttgccgctataccttttattagttatcgagcattgagcggttaatattttaccggcatgatcggcccttttctctgggtgtaaccattatagatttgtaatttaatataatccgatggaaattttatttccgtttggctccgtgtagtcacgaaaacgtttctttaccgttgtagtatggcgattttcatgattaacttaatgtaaacaaatcttaattacattatttcgtgtttacctttgcctcaactgtaaataaaatggagtctatttcatctgaacaacacttcagggacatctataatcaatattgggaggcgctgtataagatagccaataagaagaccaatgctcacgaagatgccttggatatagtgcaagatacctttacatacgtctgggacaatgttcacatactccggcaggttgaaaccggtaaggttagggcatacctgattacctgcctttattacagaatttttagcttttttaaggcgaaagggctcagaaacaaacacttacagttttttcaggtacaaactgaacatcattttgagcaaacggcttcatatggtactgctgaggcagacgaagagctaaccgctattaatctggcgataatgtcagagctggataaaatgccagaacggatgaaagagttatttcttcagaatcatctatatgataaatccatccatgagctggcatgtgagtaccgcatttctgataaaacagtcagcaaccaaataagtatagcaagaaaaaggctcaaaggatttgcgcgttcttatccgaccacagaacttgtcccactgattattttattcctcacaaagaattgattaatacaggtaacaatttgttaacacaacaaggccgggaagttttacaggtcggtatctaactggctgtatgaatccggaaaaatttcaaatcgacgcacttcttgccaaggttgccaacggtcaggccgatgagtcagagaaagaaatcgttcgtcgctggttatattcccttgatatgcccgataatagcgtatcaccagaggacctgtcacaggcaaagaaattaatgctcgaaggcattttaggtaagccaaccgaaggcacgcttccggggaaaagtacgtatggtaaatctcgtccggtctggagaatggcggcggtagctgcggcagtgtttacggctttactactcgggcgtgtttggctttatccctatcgggggggcataaattcatctcaggcatatgccagcaacgtactcattcaatccgacagtaccgttatttatgtccggctgcccgatagttccggtgtatgggtgaatgcccattccaggttgtcgtatgatgctgtaagttttgctgctaaggaaagaagggtaagtttgcagggtgaagcctatttcgaagtaacaaaggatccaaccaggccttttgtggttatttcaggtgctatagcgacccgggtgctaggtaccgggtttaatgtgcagacctaccaacaggacgaattgatcaagatcacgctcatccacggcagcatttcagtaaatgattcttctgccggtaaatcaaccttactccagcctcaccaacagttgcaatatcacaggaaaagcaaaacatggaatgttatggcatttaaccataatcccgcacaaaactggatgaatggaggattgtctttccgggatgcaacgctatctgaagtgctggatgatgttgcgcaccaatataatgtgactattggatatgatcaccagacagtggtcaataaaagagtaaccatagatattaaaacacataacaatatcgacactgtgctcaaaagtatcctgttcgtgcatcgtttacactatacctataaggacagccaggtgttcatctactaacaagggatgttccaaaacgatctaattatcatttctaaacataatttagtgaagccgttattttattcttccgccaggataattgccattgtattatttgtgctaacaggtttgcacaactcagctcgttcacaaaaattacctgtgcctattgttatcaaggtagaaaacgcctctgtgccggatatactggaaataattaaacggcagtccggccacgacatgtcctattccgcctccgaattgaggtctatatccgtctctcaattttctgcaagcgggagcatagctgaggtaatgactaagctaaagcaaaaaacgggtatcgagtttgaaatactgggcggtatcatctcagtcaggcccggcgcgaggaaaaaaacgagcaatagcacatcgtcttttaaattcagtggtgttgtcacagatttgaaaacagggaaacggctggacgaagtagaaatttttcttcttaacgcagtatccaggcttattgacaaaacggcaagtgataaagatggcaactttacgctaacagggcgtgattcagtcggcatgctgatttttacaaagaatggctatctcggacaaacaattactgtcatagccgagaaggtgctacaggtacgaatgaatgctaatacgaaacttatatctgaggtggtggtgtcggcaaaaagaaaacttaatacacaatcagcattactgaatgatcgtaagaatgcagcaactatttctgatgggatctcagcagaaaatatagaaaaaactggcagtattactacttcccaggcattacaaagggtggccggtgtaacagtgacggatgacaaatatgttgcagtcagggggcttggtgacagaagtgtgatcggtcagctgaatggaatcaggctttcttcgtcagatcctgataggagtgcgataccattggacctggtgcctgctaatctccttgataatatcgtagtgtttaagtcagttacacctgataaaccggctgatgcggcaggtggaatcgtggaattgaaaacgaagtcaattcccactatccaaaccctgtcaatcaccattcaacagggaagtaataccagtgttggattgggaggaaaggtaaatagctattacaatggtgatatgggattcctgggacaaaaaataaatgatcataatttaagtcaggagttcaaggcactaagtacgcaatatcctgggggactggcatctattcagcgtttgattgccggagccaacaacgatccgtccttattacaggaagtgagccgcatcaacaggattatgcaccagttagacccggtgcttaccacgaggtataaacgtgctcccctggacggtatttatagtatttcttatggtaactcttttacgattgcaggggtacaaaaaattggtgtaatattgggcgcaagttattataaccggtctgttgacattaccggtggcacacttaatcagtatagtatttatgagggtgtcattaccggaagcccctacattcaccagcccagaaatatccctgcctatatatcacctaataatccccgcttgggtaaatacctttcctacaaagaaaatacaggcacgcaaacattgaattatggttttctggccgggcttgcgtaccggattaacgcaaatcatgaattcagttttcagtatatgggcagtagaggagcagaaacacaggcttcgcatttaaacggctcttatagttatacaagcggttttagcggtcctatttatagcaccatttactcacttaagcaaacctaccgggtatttaatacctataacctgcagggagaacataagttcggaaggggtgaattagccccacgcctcagctataacctggcctcttcaaaagcctcccacaataaccctgactatcgctttactaacctggtagaatactatccccagggaggtggttactaccctgtgcccaataatggtggcggaggcgatccacaatacataggaagtccggcacattacagtctggtatccggttatgtaaccggctatggtacttatgggcttatacaggcagatccgaatggcaggcgttttaggaatatgagtgaagtgaactacaattataaagctgacgtaattattccttttaaactttttggcaatacgcaagagtttaaaacgggagccaattatttatacagggaacgtgatttttcagagtatcagatggctttgccgggggctaacgcttcagccaatgcacaatatccattgtacgcggtgaggggtaatctggatcaattggtaggctacaataatattggcgtacatccttcttcagctaatactccggaaggtgcaccgctggtgaatggttttctctacaacagccgccgctcgcccaataattatattggattttacgagaccaatgcactttatggaatgttagacctgcatcctctttctaaattgagaatggcaggcggtgttcgttttgagaagacaactattcagagtaaggtggataccgctaatgtatttgtcgatcctgctattacaaaaggcaatgtggcaccgattttcgttaacccggtttcccgttatgcagtgaagtataaaccgtattattctgtaaacctgacctacaatcttacatctcttatgaatgtgcggctggcttataataccacactggcaagaccagaaataagggaaatgaccaacatatttgatttcgacccttttcagcaggctttggtggtaggtaatccctcattaattaatcaacataccaggagttatgatttcagatgggaatggtttccacatacaagagaggtgctggctttctctctctttggtaaacaaatagataaccagcttgagaaagtttttgcgctcaatactgccggtaccagtgctgctttccctgaattcccgacaatagcctaccgcaataacccgaaccggggtaaggtatggggcattgaactggaagttgtaaaagacctgggtcgtatcacatcagtactgcagaatttttacaccggcacaaatatatcattagtacaaagcgatgtcgtaaagacagatgagcgtttggaagcagccaggatcattgaccgccaatcacccaaaaattcaccgctatttgaacaggctccatattcaatcaatgcttatatcaactatacaaatcagaagtctggcagtgacgtaagcatcaacttcaatatggtgggagagcggttaatccagattagtatggatggtactcctgatgtatacagcaacccggttgagatgctggacctcgtatggagccaaaagataacacggcgtttgttattcaagggttatgcaaagaacttattaaatgccgcctttgaagaaacctacaataatcctggtactggcagcactttttatggagataaatatatcaggagaagttataagcgtggaacagaatggatggcaggctttacttatcaattgttttaaggtaagagaatatagtattatgaaaacgaagagaatattctgtaaggcgctttgttatagcctgctgttggcaatcgtattattatcatcctgcagtaaggaaaaagaagaggctggtcgtaaagatccctatagcgaaaatatcacgccctcgcgcaccagggtggtactggcaggaggaatggatatcatggtaaatgggaaaaaattatctaattggggggctggtctaacaacagtaggtggaccggacaatcctccttatcccaccccatattttcccactacaggcaaactggggagcacttattttattcctgctgaatttatagatgccaaaggaaaagcgctggtggaattgggcggaagtggcccgggaataacaacagaaatagaagacagttatactaatccgctggattattattataacgtgcaggattatacagcaccaggtttgttgactcccataccccgaccagtagcaaaaccatcacagccgcaaaatatactcatacgggtagtgaacctggcctctgacgctgttgctggtagtggtacagatgaaacgcttagtcttggctatgcaaatggccagccggtaagtgctgccacttccggcattgctaagggacattggtctgagtacactgagataccctatggtacctacgaattcagaatgctgatagatggaacagccagacaatatccgctggcttcctccctgaacatttacggtgcagaagatttcagaatagccaatacgcttttctattatacccagcgtcgcgtattccagccggggggtgtttatactattgcagtatctctaaagatggccagggatccttttgcagtgccctacccggtaaatatgttcacagtgataacagatctcaaccctgctgtaaatctatcttacgcaaggatacaggttgcaaatgctttccccgatgaagtgctcaatgtgtttgtagatgaaaaaccgctaccgtccatcctttttgggcaggcaagtgattatgttattcttaccaccggtgtacacatgataaaatgggtgaatggaagcggcaccgtggaaaaagaacaaaaaataagtgtaaagggaggcgataatttcacggtagcattttatccggcggcagacaaacagattgccactacgatccttcaaaataacatgagcggaattattaataatgcttccaatgaagatggctccgatggtagtacagcagtatttgacccggtttcaataatggccatgaatttgcagacccgttttatgaatttttgtcctgagcttccttatgtgagcttcactgccaggaacggggcatcacttacttccggaacaacgggttatccttccgctgcagttaacctgaagtatggaacagctcctgatgccgtggcattaccttatccttatatcagcctgaataatacggtaatagaagcttatgcctcccggcccgggtttattccaggcaatcggttagaaggggtatcaccactttcaccaacaaactttattcatcttcctgctgaattttactcagatgggttgccggttggcgaagcaggtgtgtataccgtagcacttgttggtcattatgataatgtgaatcaacctaagctgattgttatcaaacacaataaatagaaagtaatgaataggattatacgtcatttatgtttggctaccggtatattattggttgccacaggttgcagaaaatcagactacaacaaggtggacaacgcttcctatctgagggtgtttaatacattgagttacgaagtagatcttaccacaaagggtaagaaagtaccttttctaactatgatcatagatccgcagatagataaagatggagtagttacaggcggagctatcattgctgattttttagatgtaagaaagccttatgcagctccagcttccaatgcggcgggtacggattacaaaaacacggagtttccgggaaaactgaaagttccggttgcacccgttattaacggatttgatttatctggctgggcacaggtacctgccggtcggcaccgttttgtattttacatcagacctattacccccgtaccctttttaacgcttcccgaaacggaaagaacggtcaatgcgcttattgctgattcaacgctagagattgcagcaggagaggtatatactatgaacctgttggagaaagatgtaagaagtccgcagctttccacgctggtttatttgcgtcacgaagtctttacaaatataccttttgccgattcgttactgtacataaacttctataatcttagtgccagaggttatgcagaggcacatcctgaaatttccaggagtattcttggcaccaatacggctaccggatgtgctattgcagacaacgtaaatctgtattactttctgtatacccctgatgtaccttatccttataccttagtgaacaatcaaaggcctgctattggacagacgtctgtaccaggttacaacaatgtgcccttgcagaacctgcagtggtcgcaggcgccaacggtggccgcttacaacgctattcctttattcgcagggaaagacacctcaaacggtatcatgtcgcgtcaatggatgcaactggcagtagcgccgtccggagtgggaggagcagggggatcgccatctccggctaacgggatgtcagtttcttttacaaatgaaagtgacgagggacgcgtccaaatatggaacaatgacctcaatcatgctgcagggtttttgctgcccagcttaatcaggcaggcggcttcaggcccttacctgcaacgttcttttgccactgtatccagtatggagtttattaataaaaagatatacctcaccagtattcagcgcgtctatgaacgaccgctgtccaggtaaaatatgaaaatgatgaaaagtaatatactatttgtaacctgcttgttcttagcgctggcaggctgtcagaaaccggatatgactgtaaaagtggcgccaggtactgctgcggtaagtactaccgccaattatttaaacaataatctcgatttttccatctttgctgcggccctggcccaaactgatctggccgattctcttaacagccagaatggactgtatactgtctttgctgtaacaaatgcaggttttaaggcaatgaatatttataccgtagcggaactggataaatggagcaccgacagtttgaggcatttcattaaaacacatttgatagcaggcaggatttcttatgaggatttccccagcgcactggatacgcgatatacgaaccggaacggggatgccttgtttatatcattgtttgaaagcgacctggcagtaaacggtgtgagagtaaaagcgaatcctacgattagtggagggagcaccggatatggtatcagcttgttaaacggtgttgtttatccggtagatgtaccgattaaggctagttcagccaatattcaggattttctgtctgcaaggccggatatgaccattttcgtggctgcgctaaaaaagtttgggttgtggaatgttatgatcaaggaggatggtctcaccgtgttagctgttccggattctgttttcttacgctatggccttacggctgcctggatcaatgccctggatacaaaccactataaaaaggtgtttatggactgctatattttaaggattagggtcttccagtcagatctttattcttttgtggatatggttaatgctccccgcattcccgttacctttcctcctgagttaatgatatcaactactgaacctgggcttgcattgtgcatgcggggttattaccacattgattatccttttgggtgttttgtttttgacctgtcaaaagaggtggcaatgcccgatggaagtggatcctcattctggttttaccagatattaggcccttatgccacaaattatccaaactacggcgatccaatgtctggctatcaggttccctatatcggagaatcaaacacgtccggcagtctgaaaggtacctatatcaactatacattgaacaacggtgtggttcatttgctgtccggattgctgttgacgccggacgatgtcaaacgctagcgaacattaaacaattactaatgagaataagaaatttagctgtattaataatcctggtatgtacctgctattcctgcagcaaagtaaaagaggtagtaccttctgcaggtgcttctctgccttatggggaaaagatcccggtgtcaaccgccaggttaattgattctattccggatttaagtattttccgggtgatataccggaattctgatgccatacactatttagacagtgcccgtacggcatcaggaaaaactgatcagcctttcaccttgtttgccccgaaagatgcagcatggcaacaggcaggttatactcttgcaagcgctgctgcgctttcaagagaacagtgtaatgcgctggtgctttacctcctggtgcctggccggttgttggcagacagcttgatgcccactgtcgggggaactatgctttacccggtaatacaagggatcaatgtgccttatgaagatgagtggggtactgtatataacgggaaatacacttatagccttgaccttgcctggcatgaaagagaggtagtgttgaacggcaatcatgcagggaccatttcctcgatgatcaacgcttctgatggcgcactatacctgctggatactgtaatccgcaaaccagagcgttcagtgtatgaagaactggtcgctgatacggcttatagcttttacctggctgcattggaaaaaagtagtgctatatacaccgaatacaaggcgggtatcagccccggcgataggaacgaagagatttttttcacaaatgctgaacctttcaataactatctgtcaacgttaaagaaattcattcctacgccagccggtaccagcaataagtttgctaatacctatattgtttttgcgcctgataacaatgcattcagaaaagcaggtttcaatgatattgatgacattgagcgatttattaataaatcctatgtaaccactgatacttacaaggatgtaagtcgcggctatccgatgtacaccaatatggattcagctttgtcttacagtttcattgtgccggcttacaccagaactgccggattcggtgtagccttcaattatgagcaaacactcaaaaatttatttagaacgttaccatatacagctaatctcgaatcgtccacggtgcaacagggagggataacaacagacactaagatagacttttatgactgggccacttttgatgaaaatacatatgagtttgcaatcaatgcaagcaacggcagcatgaagtggttatttggaaaggaaagcggcagaatctccctgcgcagaggcgatatacctaatggccgggtcgcctacatcgtaccggcgcattccaacatcaccgctttgaacggtgtgatacatcgtatcgacaaccttttattaaacccacaatgataatcccgattttaatgaaacgtatatatatcaatttactggtgatattgctgttttctgcctgttcgaaagatcccatagtgcaggaagatatctataataccagaggtatcgcagcggtagccaataacaattttaacctcaccttgtttgccatggcaatgcaatcatccggttataccgccattttgagccagcggggtcctttcacagtactggccccgtccaatgccgcattcaacctgatgaacattcgtaatgcggtcgacatcagaaatgccagcggtctcctttcagaaataatcccatatcatgtaataaaccaacagatttcatttgatacgcttgggatatcaactgttcatacatttcttatggacaacgggttgcccgtgtatataagccgccgggagaatagcagggatacagctattaccgtaaatggtgtccggcttccaggtaacgcactgccaacaccaaatgggaatatgtatttgctggatcaggtactgcttccatcaaccagtgggaatgtgcaggaggtagttggcaatgaatcgacgcttactttcttcaacgccgcagtaatgcgcagtggtctttataagatactaacctcgtctgatatctttactgtttttgcaccttcaaaccaggcgtttgttaatgttggtatcaccactacggacagtatttatcgtatggatccggcgttgctcgaacatttgctgaaagcgcatattacaaccggacggcgttttatcaatgactacatctttatggcggatgttgcgacagataactacaccgaaacgatgatagataatggtgatatacaaatgcagttgttgcccatgcccggtgctcctggccgttttcgcagcatccgtttaagcaggttaaacaacagcaccggaatgctttggagtgccagccttgtaaaagaaaatcttgcagcctccaatggggtagtccatattgtcgacaacatttttgttccataaacttaccaactcatgaattttatattcagtctttgccgggataaagtcctggtcgtattcctgtgtttaattaccatagcgttgcatacagtggcgcaacaaacagatggaagtatttccggtacggttcgcgatagcctggggagtccgctggaaggagcgtcggtcttagcatcacatacgtcttcaggtaccagttttgctgcccggactgataaaagaggagctttttatatacctaatcttcgcattggcggaccttatactgtcaccgtttcttatacaggaatgaaagcgtaccagcagaatgaaattacagtgcgattgggaacaccgcttgagttgcaggtagcattgatgccacagcatgcggttttgaaagaggttgtgatcagtacaggaaaggcaaaggttcccgcggcaaaccgacatggttccggaatgaatatatcccgtgcccagattggcaacactccaatgattagcagaagcctgcaggatgttacgcggacagtgccgcagtcttccaaagacaactcttttgcaggcaccaatttcaggtataataatattacgatagatggtgctatcaataatgacgcgataggtttcagtccttctgcaggaggaattaccggatcttccggtacacccggatccggcacccggagtaacgccatttcattagacgttatagaagacatgcaggtgtacctggcgccttttgatgtaaagattggtaatttcacaggtggcagtattaatgccgtaacacgtagtggtactaacacagtaacaggttccgtatatggctatggccgcaatgcaggtattaccggaaaagataaagctggtacactgggtagcatggataaggatttctatgactggcaaacgggttttagagttgggttcccaatagtccataacaagttgttttttttcaccagtgaagaaattacccggcggcaggatcccgctcaattgatagctggtcagcaggaagtggcgggtattcttagcagtcaggatgtagcgctgatagaggcggagacggaaaagcgttatgacagaggcttttttggaacagcaggggcatttaacaccagttccgaatctgaaaagttttttaatcgtattgactggaacatcaatgagcgtaaccagctgtccgtacgcaacaatactattcgctcccggtctttaaatcttgaccgggaccagttagattttcgttttagttcgatggcgtatcagcagaccaataaccaggtgtctacagtagctgagcttaaaacaagattgtccaacggctggtcaaacagtcttattgttggctacactacaatacatgattaccggatgcctactgctgatccttccctgccacaggtgcagatacggggtcgtacaccgggtacaaccatctatatgggaactgacagagaagcttccgtatttgatatgaaacaaaaaacatgggaaattaccaacaatcttacctggcataccggcaaacataccttcctgtttggtacccacaatgagttatatcacatcaactatgggtttgttaatgcctggaacggacgggtagactatcttagtattgaagattatcttggtaaccggccttatcgtgtaagaggaagttatagctatacaaataacacaagatcatatcttcagaataacccgggagctgttttcaacgttgacctgctgagtgcttatgtgcaggatgaaattaaagtaactgaacgatttcaaatcacacctggcataagggttgactatacattgttgccggacaaaccggatataagcgaaagggctgtggaaagtatgacagatgaatattttggcaatacttattactatacgcctctgaacaggattgacaataattatctgaacaaattacagatatcgccccgcattggcttccgttacgatatctccggcaacaggaagtggatcctgcgtggaggcgcaggatggtttaccggccggataccctttgcatggctgggttatgcctactataacacaggcatccactacggggcctacgatcagcgggcggacaaacaaccttttgtggcgggaacggaccccattaaaccttctgtaaatggtatcgctgatttcatcgcacaaaacggccatgttatcaataacgccgctgtaggcgtcactcaaattgatgttatcgacaatcagttcacgatgccgaaggtgctacgtactaacctggctctggaacatactacgaataatggctatgcacttggtgtggaagcgctgtatacaaaaacgataaaagatgttttctttcaacagatcaatgtaaaggatgctcctctttattacggctttgacaaagagcatcaaatgcctgtatatccaggttcctcagatccagggtttaccaatgtttaccagctttccaataccggtttagggcaccgtttctctttcaccggcagtatcaggaagcaatttaaacagggaggtaatttctctctggcctacacatatggtcagtctaaagatgttttcaacggtattcgtaactcaatggagagtaactggcaattaaaccaggcgctgaatcctaacaatgccgggttggcctggtccaatttcgatatcaggcataggatcgttggaaacattggctacctgaaagaatggcctaatcgctgggtcactataatgaacctgtttgtgagtgcacagtcgggaagtccttttacctacggcatcgtcaattacagtctgcagggattatcacagcaggtgagcctggcctatattcctgaatcaacggaagcggtgcggtttttccaggacgtgcaacaaggtagtacggttgtcacagcagaacaacaggcgatggccttcaacagttatatagatggaaatgcttacctgcggtccagacggggtaattttacagaacgtaatgctggtcgtacaccctggaacgttaacgcagaccttcacctggcgcaggagtttcattttggggaaagcaaacagttcgttacactttcttttgatattatgaacgtaaccaacctgatttccagcaattggggcaaagtctatttttcaccaaatacattcaattccacggcaagcgttggactgataccttcgcagtttcctgaaaaacaaaatcaaggtcaataccctgtatttactttcagagaaccgggaaaaccttattcaatagactattttggttcaagagcacaagggcaggtgggcttgagatataatttttaaatccctttttatttagtaatcatggacctagttcaccacttagttcctcaacgagttgacatgaattgatataaaatgggctaaatatttttttagtctttgcagatttaattggtctacaaagaataaaatgaaaaacacctagtacatctatgatcgcaagatgctttctggttaagcatttgcggggagttccattagtttaaactggcgataaatgaattgaacgagatgacttggagaggcactattttgacggctgctatgacttgaaatacgttgaaataattattcgtaaatcaaatcccgctgaaagtgggcgactgtagagggtttgcgccgataatggcggtcggttcaccacttagttcctgcggaaaatagccctgtttttaaacagaaaagcatgaaattcaatgctttgaacttcatgctttgactccgttggtcggggcgactggacacatttcgaactttatcatggaggatttgaccattatagggcggtttcatgcacaaaacagcacaaagtgacaaaattacatcctatataaactgatcgtcctatttttcagatcaactaatatgcttatcttatttctttagtcgaaacaaaacaaataatggatatttagaaaaacccagctgggcgagaaaggcaccatcgacaaccatagcaatcatttaaatgtttgggtaatgccaccatcaaaccgattgatatcattaacaatatagtcgtattcaaaaaattaaatattcaacaacctcatatactttaagttatgtttaaattagaggataaggtagttgcaaaagaagttagtgcaagtattctaaaattaatccttagtgctactcctggtggagcatttatcaatgaatatatagaaatacgtagtagaattaagcaggagcgatttaataattttgtttctcagctttcggaatacctgaccaataataaaattgaagcgaacgcgaatctaaaaatggaagattttggtgatctatttgaatcagttctcagacgcgttactgctaccaaatccgctgaaaagcattctcggttcagagacattcttttaaattttatggaaaatgcagaagttgaaattgatgaagcagagatatttctggatctagctaatgacttgaacgatattgctgtaataattctaaagcatcataagatattgaaaagagaatttagtgagaaaaatactaggttatataaattggaacagaatctaccagttctgaatggaaaagtcgtcagggaaatggcgttaaaggaaaaaggggttgccaacgattttgatgtggttaacctgcagcgactggatactgatttaacgataaagaagttaaaagttgaaattaaggagcttgatgcaatcaagatgccttcgttctataaccttgatgaatatacattcctatattataagcaaattctcctatcgaaaggtctattaaaagataattttgctggtaatactattggaggaagcccttttatatatatgacgatcacagaatttggcgaaaaatttattgatttcatcttgagagcctaataatttctccgaaaattatcatgtgacattataaaaatagaaaagttaagttatggagaatttaaaaagagaaattgatcaatctctgaataaaatcgacttattagatgttcaatttcaagattacgctaagcaaatgatacttccggattcaaatatgtttctccttgacatttatgcaattggaattgtaaatagagcgctatcgctaacctctggctttagtactttaattagacaacagaattttattgctgcatctcatttagtaagaccttacctagatacttatctgcaattttttgcagtatggcaagtctctgatatcaataaatttgtatcagatgtcatgaaaggggatcgtattgataagttaaaagataagaatggagttttaatgcaagacaaacacctcgtaactttagcatctattgattatgaatggatgttaaatgtgtataaagaaacttcagggtttattcattttagtaaaaagcacatattcacatcaagtaggcttaaagatccggacagcagaattattgaaggaagggttagtaagtacgataaatatgttcctgatgaatccaggctggaagctgttcaatgtatgttagcaatatctcaggctatttttaaattattggaaggctggatatggaccaagcaaaatccagaggaattagaaaagataaaggaaaaggaggcttttaaaaatcagtggagcaaaagggtaaagatcattggaaatctttataccgcattaaatgaaaagagagttagggattctctcgccttcttacacgaaaacgtactttggccgacctcagatccagagaaattccttgagggccacgccgcagttaaaagtaattggaaagagctttggaaaactacaacagaaaatatacagcctatttcattctcagtcctagaaagcaaagacattttgatcgatgcccatgtgatagttagagatttgaacatggcagtaaaagaagattataaaacacaacatttatttgaatttgataacgacctaattaaaagaattgatataattccttataaagactaatgctgcgaatcgaaagtgtcaatggagacatgggtaggtatttttgattaaatactaaaatgtaatacattgcaatattatttactataaaagcgccgtatattgtgaaatacaaacattgtgtgcaactttctataaaataaccataaacaattaatgtatatgagtaaagttggaggtcaattgatacaggttatcagagataatgaatttaagaacataacgaaggatttagtcgagagtgctatcgatacaaatttggcagaaggctttttgaaggatgtgccgtttctttcgacaattataagttcatttaatctagttactaacattaaggacagattgtttgtcaaaaaattgctaacattcttatacgagctaaaatccatttcagaggatgaaatactagatcaaattatcgagttagaagatagcaataaatacagaactaaggttggagaaaagctactttatatcatcgataagtgtgaagatcctgataaagcttcactcacaggcttactttttaaatcttaccttgaaaaaaaaatagactatgatgaatttttaactgcatcaaatacaatagaaaggacgcctttaccagacctactatattttatagacaatgatttcgatgactggggtttggatagtggcggttctgaatatgtctcctatggcttaatggagattagagtttctaaaccagaaataaaagtatcaagtgactctcgttatgattatgatgaaaaatatgcaccatctgaagaggaaatattgcaagataaaatagatattactggctttgatattaaagcttgtgttagttggaatggaagaacaattagaaagtgtttggcaaatagataggcttctctacatcgtatataaataaacctcattagtttagaagcatcaatagagaaatattctggcgagattaccccttccggcctctttaagcaaacctcttttttattttagctcaaagatcttcggtaacccaaagggaagaagcgagccggaacccgatccagcggtagcctatcttgttgcggttgcgataggctatgcggctgatagcgggttcgcggctccagttaccgctgcggataacacgatgcggtcctgttgcagggcccttcggatcatttcccggagttttaccataatagtttgcatcataccaatcgttgcaccattcccatacattgcccgacatatcatacaatcccaattcattggcctctttttgtccaacagaatgagtatttgatccgctgttgccagaagttcaggctaccgcattgatatcattactacctgcatattcaaatttcttgctctttgtaccgcctcttgcagcatactcccattctgcttctgtgggcaggcgatagtttttaccggatagggtattcagcttttttataaatgtctggagctgtattgctgcaaaaaatacttatatgcttcactatttcttccctgttgccccttgccatgcccttattctcataccggttaggtttggtgattaaaaagtagttcttgctgtcttattaattttaatactttgtatattcataaccattatgaaattcacttaactgaaagatctaataacggtatatggaaaaattttttgttgaggaaaccgatggcatccaacctgcgctggactggtttttatcattcataggaccggaagactggataaagcgaaaacaagcaattgagaaaaaaatagcttttgaatatgataatcccatgttcaaagggaaaactaaagatagcatggttccccttacggacaaagaggaccaaattggatggtatttgtatctggctgaaaagtcattgacagatccaccacaatatgaggtcatacagggggcgcgggtaatgcccatcttccaacggattggtaccgatttggaatacttaagtaaaattgaaggcctgaaaaaaaaggtcagattcctggtaaaaaagggtagagcctcggctgattcgattctctttgaaatactggtggcactattatggaccaagaatggctggaaagtatccattattcctgaaaatcctcctgcaaagacacccgatctgcttgcggagatggatggtgaaaagtggtttattgaatgcaaaaggctgaataaaacatcagattacagtgaaagagagcgtgcaaaattgctcaaaatgctatcttatataagtgccgtgttattaaaataccatgttttgctggatattacttttcactccgaactcgaacaactacctgacgacttcctggaaagggaattatcagcgaaaatccctttaatcacgaaccggatgaatgttatatccaatgatacctgggaggtaaatatcgacttcgtggattatgggaaaataaatgatcacctgaaaaattgggtagtaaaatatccatcaccacaactatattacttgatagcgggaaaaaagattgatccagcagggttttcaagtggaataaaggccagtttccaacatcacggaaaaggcacgggaaatggacagtatgtagaccaaatagcgcaagcctatggcgtaagctggaaatgtgatgcacaaaaatccattgataaaaaagcgagagacatcaaaaaccacatcattgatgcatgtaaacagcttcctgattatgaaaatgcagcaattcatgttggtcttgaaacattagacggcattgcagtagaagatcatagacacaataaaatctacaatactataaattttttcgataaaaaaaacacaggtatcaaatggatttactgccatttctttcaatcttatgctccaccggaaagcctaacatgggtctttgatgaaaccatcagttacttctcggataatccgcaccaaaagaatggccctctcgataatagatatgtaattttgccgcctggtgctaaggattcagatgacgtacactggcataagcccacaccttaaaaggtagcagtaacgttgtaaagactatgacgtcattgtggtgctaatcattcaacacattcagcactaagttgatgcaagacaaagcacgataattattcgaggcttttgcccgttggaagccctctttaaatccggggctattttgttaatctaactgacacccattctacttccatctttggggaatgcctggtcaggtaagctcaaaataaacctttactggcttgtgtttcccattccatcatcggcaggatcaccgatcatttttgaatgcttctggcaaaaccctatttatttctcgctgcttgggattgaatgattcactttatctttatatggtaacaacttttgctagaaagctacttgtttatcatagatatatattctggaggtgttactactttagtaggaattttaagcttgttgtagactaatttagccttattcgcacaacgtaaatccaaagtgacaaaatactcgcaatgtgaagcgtaaaaacaatgtaacgcatcatcaagcagattagcgaatctctcatcttgattgtaacctttcaagtcagttgttgtaaataggtgtatgaccttgtcatagaatacattagaactcggcttaaaatcaggaattgctaagtcccatacatcatcccatgttatgcttttgggtgtaccaattattttattatgcataacttgatagagattcttatatgaggggaatttttgctggcattcagtcagaaattttcgataatttttatataaggcgtagtcggtctttattttacgcgcaaagtcgtaaaggtcttcgcacagagataattgattcatttcaatctttgtctgtgggaaaatactactgaaaataggattaactgaatagattgctcggaaactattgtctacaggttgaagcctcatcatcatcttttgcattccaaagacgctttgcatcaatggatcatctaggctattaaataaactagaaaaagtggctgctgtattttcaaattcctcaactgttgattcgaggaactccaacggctgtcgataatgaattcttactttcgtttcaccccagtattgcaccatgcacaaattttttgtcatatctgttatgtgctgaaggtgagctggtgtataaatgggatttttgacatatcctctatataggtcgctaatatgagcattggaatatggagtacttattttattttcatggattatctgaagtagttttctatatattggagtgatgtcatcaggtaattcggagattttttcaaggttattaaaaacattccaatcaagataaaccatatctattttatttataactaagcggttaaaaattttctactctatatcttcgtttttatcgtgcatattttgaatctcgattattaaaggccggtaaagtgccttcaagaatatttattactgctttatttataatctcattctcaattgcaccggaaaaatatttgactaaatttttattttctttttctatctgcatttgaataatttggtctgcgtcacatacaatggccaaattgggattgtgtgttacaattataatctgtcttttttctttgacttttttaataaaatgaacaagtatatgatatacactctcattatcgagattttcttctggttgatcgataactagaggtatatcatcgttatctaatattaaatagaaaattagcagtaacgctcctcgttctcctggagaaagttcttgtaatgttttggtacctagtttgagattataaactggtaatagatagtcgaaggagaacaggtaatcgtatagtgtgctgatttcagtaccatttttcaattgactcccgatacttactggggtattagctggtgtacgcttatcatgtcttaaatggttcagaatgtcatttgtgaaattgatgaaaccgtcacttgagtcgaaattggcgtgctcaataatttcagtaatttgcttatttgcattttctattccattgaatgaacctattttcccaagattaatgtagtttaagaaagcttctggaaaagattttagttctaatgagacgtcaatttttacgttataccttatacgaagttcctcaaattcgtcaatgaatttcataaccggagagaatagctcttttctgatatctgataaagcaattttcttattaaagacttcagtcactaagctgtttctctgttggtatcttgcctcaagatcaatgagtagttgatcaactagatatttaagctgactttcatagtacgctaatgttccttcttgctgaacactgcctaaaatattctgttcttgactttcccatactctcaggtcatcaagatatttttcctgattctttgctggggcatcgagtttttcttgatggatggcgagttcttcttcaagatttgataactgagttctgagactttcagattttgaactgtctagttcagcattaattgtttcaagacgggcatcaattagacctatttcaattgccagatctaaagtgttaatattaaattggaatacgttatcagggttcaatccgtatttttttaatattaccacatattcagccgtttcagattgcagttttttcagttgactgtcaagcgttatataatgttgttgtgctctttttagctcttcttttttttgagtttcatctgtccgttccttttccttgcttgcaatttccaattctagattggcaattttctttcggagattatccagcaaagtgaatacttcatgattattattgtcactttgtccatcagataatggaggtaagggttttactgataggtgtgttgtaaactcgttcgtcttttgactgattttgctttcgagagttgtcttgaactctattgtagatttcccttcgagggagactatttgtgcatttatcttcgatatttcgccttttagatatatgatttgctcattgatgacactagatttatacgcaattaactcatccaatgattctttgtctagcctttgatcctgtggggtatgggaataaattatttgctttagttctttttcaaattcatcactatcaatatttgtacatagtcgttctaagaaattctgtggtatgtatttaactctttctacttttagtttatctggattctcatctaaccgcttcgttattgttgacccatcctcccacgtaagggtagctgagaacttttcagagagattatatggtctaacctttctgaattttgatgacgtaagaaacgaaaaattactcttgtcttgatgcgtattcccgcaaagactgataatatctgtaattgcacttttcccgcttcctttgttcccaattattgcaactaggccattattaatttgaatattaaaatttctaaaccagatatcatctaagaccgttggtgcctgtttggttacacttactgatcttataaatttagtcttgttttgcctgacccttattaataagtcgggctctgcaccaataaagaccctgtttggttcgacgagaatctgttttagaccattgaatgtcatgtctgcattaatccaacagtatttttctataggttccgatttctcattttgtagtcttccaaaaagatagtttattttgtgggcatctgacccttttatgcaaggctttggtttggagaggaatgattcatattgttcctttgtatacttaggatctacccacttgaaaaaatcgatttgtttttttgttgaggagcctaagatgtgagcatcatttattagcgacaacttaaagtaaccgtctatattagggtctatttcatcaatcccgccatattcgtcatagggaagccatattagcgaatgcttataatgcaagtcgaatttttttaggctttcaattgttttattgtaatcgaatgagacttttaaggagtcggaaacaacgcctaattgtgcaacaatacctttttcatcaaaacactccaatgaggatagccatgtgcggattttgcttattacacttgtgcagttgtcgaatataatgtggaagtttattctaatgccattggggtttttctttgtgattaagagattattcattcgcaattcaacaataggaaatattactttattaggtacaccacccaattttactacctcatcatacccatcaatactacagtagtcatttattccaattactgcagcttctgagttttcaagattagtaatgaatgttgaataatcccctccataagttttaggggaatgaacatgtaaatcccatattctccattgagaacctctattttctgccttattcattaatgtaagtctttggttatttcgaaaaacacatgatgaaatcaaattgatagataatttacccttaacagggtatttagacgttggaagaggaaatcaaaaagataaggctagaattgttttggttattttaataaaagtattgaaaattatctatcaataaatcatatgttgattatttataattttactcacatagtctttgcgaatattgggacgcacattttattgaatccagtaaaaggactgctatttcctcaaggagtatattataatttggaaaatgaggcatttcgaacagaaaagaccaatgccgcattttcgctatttgcaagcctgaacagcattacaggcggaaaaaaaaggatagggtagcagttatgctgtcctgtcgagtagggcaactagacacatttcgctccttttttgtagcagattttgaacgaattaataacttcgtaagctttaggcattatttattagtacagccaagagatgatatcagttaaaattttcgctatcagaccttattgataacaaaatcatcgctgaatttccatgacagatattgtaacttaaaacgacaaacacaataataaaatccgtacattcataatgacttatccaattggttaacaggcatttggagtaattatcaaatagaaagtatagattttttacatggcaaagacgaaatcaccaaaaatccccgctgatctgtgttataattatccgctagaatggtacactgatgcgaataatgtcccaaaccagcaatcccaaagcgaaattatccaatggttctctactggcccaggcgcacgtttattcgcccccattgaaatactcaatttgttgtataagcaagttgattttgtgtcgcagaatatttatgacggagataaagttgaaagccacttaactgatcttcccctaacagaccttcaaaagcacgtgttatttggactaatcttaaagaaatttggtggttacccgattcatttagctgaaagagagcaagagaaaactattaaaagagttgaacagctttttctctcaggtgaaaaagattcacctgaaagggagttttgcaagacggatatggatacgcgtaaagaattcatgaaacttgggttggccttcacaacatcaatacgtacaggaatagatgtaagagagatcctagcggaaatggatgagacaacagctgaaccggtgtatagaaattttgaagatctttttgatgatgctgctttaaaaggaggtgttggcccctttcatccgcagtcccgttaccttattgagagaactaggtataactttacctttaatacttggttgattgaccataaaggctggccacatggagatgaggttgcctatcgacaatttctaaatcgtctgacattcgtggaatatttaaaatatgaaaaagaccaagttgcgctgaataataagctgttagcagcagataagcaaaggtggacggtgggagatactgatgttcaggcaccagatactgaaacagaagatgataaatctgtactggtcaggaagcacttatccaaatttattgatttgttcaattctggagaagagttaaaccgagcaataacaatcattactgagtttctgaacattgcaaaagtgacaaaaaccaaacagatttttgttaagaacggctctaaaagaaagtttgcctacgctttcagccaaatatggaaggagacttcaaatgaggcgatccctcttaaatatttgaaactttgtaagaatagcttttctatttttgccaaagaggatattgatgaaaaaaactacaaaagcagtaacctatataaatacttcattactaaaacctaataccatattgcgttccccgcattactaaaatcattttttttatcacttttttcacctcgtctatttgtgtcaaataagaaattatgagaaacaatcaaacattaaaggtgagaaatctgattgaacgatcaaatccaggtttttacattttaggtgtgccgctcatttatgttggttttaaatcagctaattttgcgatttagtttatctgcattcctttatcagcaattttcattcactataattgtttcttgccccactttccatagatagaattgtgcctttttgtcaaactgtagaagtcaatacagatccgggctaaatttgtactagttggtaaaaaatagtaatttgaatagccaatttttccaattgtagtttcgttaattcgatattaaagaaaaatgaacaaaagatttaaattgcatgcgtccagccgggcagtggttgaattttgcgatcagcttatttggcggcgaattttggatagagatcttccttttaatgtcaagaatactgctgcgtcagtacaactttcgttcccggaatataggattgacaccattcagagccatctgcagcggatttttaattattatgctgatctgggatatatcggacttaggtctgctaataatgaattttatgacatcaccgacctttactatgttaaggatgcagtaattaggcccgaagaccaaataatgtttatcccaccggagcctgatatgcctgtaacacagccggattgcaaaccggtagatcctcttcgtggtttcaagcgtaaaaattggaaggcctttagggcccagcaccttagaaatctaaataagggtttagattaacttttaatttaaaagtggagctaggcatatacttggggccttgttcggcaaatttatatttgtctaatcgaaggttcattttagaaatgtaaattgaaaatagtattttattcagtccaacgatttttacggcatagaacggattccgtcaatcgctgggaacagtaaaaacagcatcctatctttacaaaactattgctgcttaatccttgacgatgcaagtgccaacaaaatgaatgtgcctgcgcctccattttgttagcacttgataaagtttggatctacaaattagtggcctggcagttggggctattgcaatgtgatttttagttctctttattcaataagtcaagattaagaagtaatctctgtatcaaaattgtcaattgtgtcacatcttctgactcccaacctcgtctatctatttctttaactacttcctgacttgtttcgagtaggctgtacccaaatttccttatatcgatgttgtctgttccattgcttcttgaattccgaaataattcaacaacagattgatctaatttttttcttattacaaaaaaaaacggaccatcaaaaaatgtgaacttagcttcattatttcccgatcctaaaatttgaatcatattttcaatccaggaattgaggacagttacaatggcgtcattccaattttgctccgggaaaaagtcattgcccacttctattgaaattattccggtaattacttttcgcttcgatatttcaagcgattttctatcaaaatttatttccatagctttaatatattggataagcagtttcgatcgtgtttgttactttgtttagccacatttcgatttctaagccatcaaatcctgttcctcttaacagtattctatctccttgggtctgtaattttgtatgtacatttctatatgcgttccttacaaccctgctaacatccttagcattcatccattcaggaaacaatgtttttaaattactaattctatttcctcctcttatatgaccagatgcaatatgatctatatcaataatgactttcttccagcttggcaatatttttttaaggtggctagcagctctgcctgttctgcctgcagcacgaattattgaacttctagtaactccactgacaactgcagcggttgcaagaccttctaaccccattgttgtaacacctgtcacaaccggttctacataatcagttacaaatataaaagatttatgcacttttcccattcctctgcgccaggcggccccagttgtactcggatcttcgtattgccgaactgcgaagccgtcttttacttcaatctgctgactttgctgtaaatctatctgagtttgaatatcatatgatctttgcaaagattgaagtttctgcagttcatacctttgacgctgttgttgccttgtcacatagtctccaatttgattgaaaccgttggtttgaaattgcattccgacttccaaaactttctgagcagtaataaatggtatcttatgcgtaacaatatttacagctccgtatccccaaccatattggccattaaatagtccccaaatcggaggatcatcgcccaaggggtcggatatggatactggattattaaaattgctattatagggactgatgccgggatacttttcagctacagggtccatctggttccatcggccaagttgtggatctagtgtgcggaagaatgcatcatattggtttaagccaatttcgtcggtttgttcaatgccgttatagttaaagttatttgttatatatggatttttcagcgccttggaactgatgccagccattgtcagaccaaagggataataatgggtttcttccaacaacggccctgcattatgattaactacaatgttgtcaaagtaaacatcctgaatgctttcgtttgttgtgtatacatacagaaagccagtttttttcattatcatcaggctcgtagccagcgtctggagctgatcaggactaccctgtacctgtctgacaccactgttttcatccaccatattcatttggtcatcaaacagcacataagccaggtaggccttaggaagagtggcaacattttgagaagggtccttatctctaatggcctggtagttggctgaagtgaaattggatgcgattggcgatccagttcctgttccattaccatgggcgccatctgatggtccagttccagtagcaaaagcctgtagtaatgcggctagcatatttgcgacagtcgtattagaggtacttgctgctgctgatttataaaaagccttactccctaattgaatggaatctccggccataactcggagtacgagggagggcccaattttctgtgagccagcagaggcatttaatttagctacataatcgtttgggttggtcgttgcatcaacaggatagccagcgggcttgttggttcggcaactattaatattggcaaataatgcattttccttagcggagaaggctgtttccattgttgctgcataggtggccttcccatattgttcagtaagcaccatccggatattaccaatgtgatcagctataaaatagtcatatacataagttggagcttgcccactggcatacaaaacacgtatacgcccctcatcgtggtcaaaagataccaggctatcattctgataaataaatccatcaacgtaatctgttgtagtgaccgaacccgttcctgataagtcggtaactttcttgcgaagcttatttccagcggcatcatatgtgtaggcaatatatcctttacccaatacagttaagctgtctggtacattcagataaagattaggtttgattgccagtaaccggttcatatctgtagttaagttcccagcagcatcatatacataatcctgggtctcattattattgatttccttaaaatctctgagtcctgattgtggatcattttgtcggtctgttacaaaatatagctggttactatttggcaggtacccatacttaagactatcaactactgcaatgctcaatcctttcattcctttttgcaacaatcctccaatattcccattggcatcgtaactcaggttccttaaactaaaatccactttgtctgaggtccataaggtactaccagcattttgttgggagaagtcagctgccaaaagtcggccggatttatcatatgagtaaccactggctctggctatgccatcccctctgcttttccactttgcacctgcaatagtaccattatactggttgacactaaagccgaagtcaaatgccagttcctcgccaaaccaatttgaggtactgttgggtgtattgacaaatgttttattgattccagtcaaatttccattgatattatagtcgtaagtcagtgtttcctttggaacactatttatgacgccgacttttttggtcctaagattgccaatttcatcatagctgtaacttccgacaattcttttggaagctggtagatcgtttagctgcgtgctgatctcaataacttgtcctccgtcatcataggaaatatttgatagaacccgtgtttcaggcgttacggtactatggggatttgtttgccggatgtaactacttaggagctttccattataatcatataaactggtaactgtctgctttccaccataaatattgtcactaattaactgaattggccttcccttatcgttgtaataaatggtctttgttaaccattgggtcgttcctaaaatcctcgtccgttggcctgttggtaaacccataacccgatgactgactcctgtaaggggggcgtcataataattggtccctttttgcggcatcccaaaatcagtggtcaatgctggctgcacaccaggaaaggaatagttatcgtcataatattgaaaagacagatctgtcaggttgcctgcaggaataaatgggaaggtaccggggagggtggcgttcactgctgtctgcagcgcatccctgtttgtggtggcggcataggcggctattctgatagatctattcagattgtcataaaaattgaccagccattgtcctttgctttttaatccagcatcacgcacaagtaccggcctgtcgcgggtatcatatactgtttcagatgaatcgacaccaggtaatttagttacaattagcctgccttttacatcataccggtaagaagtacataatcctgagagaacgtttgtaatggtccagcttggaataattttttctactgcaagcggcggaattacaaaccttaaattgtcaagttcatcatagacgaaataagtacataaccaaccaatatgggcagtaactgttccagatgtaactaatgatttttttagtatcagtttcccttccttgtcgtaaaattgctggtattgaacaccattttcatcaatggaaactgatttacctaatactcctggatcatatgtttttagagtccttggaacccctgttaccaaatcccatacccgaacagaatcagtgacagtgttcacaaaaagatactgctgattggatttttgccctccttcattcgcccaggtgttgcctgggctaaaacttttgatcagcggagaagaaggagtctcctcatatttttgctgaccgtaaaaaatactttcccctgagcctgatgggtttagtgccggatcttgtgaaaaggcttgttgactcgaaaacgggctatttttaaattttccgtcattcgtatttccggtagtctggacatatggtaggtaaattactggctgtctcccatatgcatcgaatgtctgcgggcttaccagatcctttccagacgtactacctccttttaccactgtttgaaggtttcggtttataccatccgtgtaagatgtagtttgtcttacttcccgtgttgtgcgggcagtaccggtcacattaataacatcggtcgtaggcatattaggctcccagatcctgacatagttaataaccggattctggtatgctgcggggagtggcagcggggtggctgccaggtgaaagccagaattgggtattactggtgcttgaccagaaaggtcgaaagtactattgcaaatgtatagaagagggataataaatctaattctcgggaatttcatataattggagattaactaagttaaaattactgtaccattaaattggaatgaactaattacaaggctcctcgcccgtataggtctttggaccataagtgccatcaggaaatttgtagcggtagccaactttgcacatgaagggatttcctgaaattggttcattgaaatattcaattacgcccgttatacagctgccattaatgacttttttatcaacaccactgcatgtgcattgtgttgtctgatttatatagttttgaccgttcaccctcatgtcctcctgcgccattgcatttaccattaaagagtcatcgccggtatattttccgacaggaatgttataaactcccgtaccagcgataaagccggaaccacatccttgtttagtaaacgtcttggaaagtgccgtattggaataagctttcccaccgcatgtttcaggttgcccgaaataattatagcaaatccgttttaatatatttccatcttgatcacgtacaatactcaaccttccaagataatcatactcgttaaaaacggtatttccgttaacatcagtctgagaggttaatcctatcattggatcataggtataagttgagattaccgcatctactggatatattctcacttcgtcaatggcgtctccgtcggaaaggagcattccattagtatatggcttggcattgtaattccatttgccggacaaataatatcggtaatccactctatagctccgcgaattgggcatcgtgaaagaaaccggataatcaccttctttacagcctttgcctgcgtatggcactattgtaccagtataattacctgattcaaaatcctcgtagaggaattctgatgcaagcgaaacagtgggatctgtaaaataggaataggtgaagtcgcaactacctgaataagtagattttaggccagtaagcgtgtatgtccctgcaggaagtgaagcgtagaatacactttttgggaaattgagtttaaaggtgttgaagttatctgatatccttcctgagtttaccacattacataaagttccgctataggaaatcgcaggacttccaccagaaagggtatagctaagcatcgaagaagaccctgttggggacgcatctagctgaagaaatatggttcctgcctgagccagggtgaatgtggctgttttaacgtttccgtccgtcagtactagtttcgcatttgtaacagctccttgtgttccagacctttccacatgagctgcatgagcattcgtaatttctgccgttattttctgcttaacattaccgaactcatcgccatttccccactgatagccagtctccacagttgcaggacctgacaaatgaacaatattaccggcgccgtcatagctcattatctgctggttctttatgagtgcaggggtccggtttagcacacctgaattaaaattaccagctgctgctgcagttactggaacatcagtttcaagggattgtatctgttcaactttaatatccggagcacctgtgaatttgtataccgaaaggctggaacttaacaatttctggccagtgggatttaactgccatgtttcctgtgccactggtagagaaatacagttggcatccgttaacgcttttagcaccggaaggctcgcaccattataatcttggggataataagttcttgtttgaatggtatcccccaagctattaaccacattaattttagcaggtaacaggtttgttgaattattaatatacgtcgttgaggcttgagaaaagttgccaatgctatcgtaatttttttcagcaatagaaattaaatcggtacgtccaagcaacggtttgtatatttctgaataaaatgtaatatagtatgtagaaaatgccagataaagactattgggacacatcagcatgttcctgggcttccacacaacattactatctccaacttcagttgttagcggagcgtaagcgtaaaccttttctgatagcgttttacttgctttggaaatttcctgttccttcttaatcagaccatatacccagggaaggcatctggttttgggagaatatggttggctttgggtaggtaccgctagcgggaaatcatctgggctggtaaaatcgtaaaccatttttccaatattactggttgaggttccttccagcacctcgactcgcttatagaggtgtggtagcaaattatttttagtactatgagtacttaactcttgtgtattggtgcaaggatattgtttagttgtcggtggtggggtaagaatgtcaattataatggcaactataatagtaataaacagttggttcattaccatattttgaacgcccttcatatttccgatggaattagccgcataaaggttaggtaaaataggggacatggctacgctaaaaagtaaatttcccggtctataaccagattgagatggtgggactactatcatggcatcggagacatcttgatatacaggaacttcgtatccccaaccagaagaaccaccatcagcatttacatatctatattcttttacaattttcttggtagtgtcgaccatatcatataatgtagtacgctgaactcttataccccctgataatactgccgatccattaaattgggcagtattgttctcatactcatatagaagtttaccaccagtaggcaattgaattgcttttagggcgcctattacactagaaccattcggatcaaccttcctgtattgttgaatgtagttcgtaagcattttaacgcttgctgccgcgttgtcgccattagtgtaatccaaatataaaggcaatgcattttcatatccccaatggtcaccacatttaaggtttcttccagccatagttactgttccaactttattataataggagaaactataaggtgcatctgggatgttaaactttccggttttctggacagacttcaagcaaagtctggcaaattttaaatctgatggtgtaaaagtgtagttaaatggtttggtggtatccttaaagaaatattcgtatccaaactgatggcctgaaattatctcatcatcatgctttacgataatctgttttaagggcttttcgccgggtaagtcaaccatgtcgctatcactataaattaaatttaccttagttctataatcgggaaaagtaatttcagacagccgcttcttggtaccggaaaatacattgacgatactttgtccaccctgactaccttgcccgtccgctacggtataggtgagtgcggcttcatatccaataagatattgaagatcgtagctatcatatttcagagtaattttcttgccggagattggatctttaatttcacttaggtaccatgtatttttaacagcatattcgctcacatcgtaattcggcaatgtaatctttaagcccagggatgaaacatatggtccattcttattatcaattaaattggtaagctcagattctgaaaatgtatattgtattccgctttcatcagtaataatgaaacttccgatcgttgtaattacctttgattcgccagctccgaagtattctactttttcgattttaagttttgaattatccaatggacgaatcatgccattacccgaaattataaagcttcccgatctgccaccaaattgaaactcaaaaatgtcctgttgtaaatcctttaagacatcagaatcaggttgataattgaaggtggattcaaacaatggaatatatcctgctttaagggaaattggagcaccgcggtatgaattaggggctaaatagccatctccctgccttattccgccatatgttcctccaatctgatcatcggggactccgatagtccggcgtactatcataccaccagcgaatagatcccaacctaagccaacctttgtcggaatttgattaaccttaatgccacctccgccagtataattcagggcaatgttaaagcttaggcggcctccatcgctatagttaaaaagtggaagagaatagcttgccctccctgttggcaggtctacctggccggaagcggtaattgaaattagggatattaaaataagtaggatgggataacatttgttcttcatagtatattgattttgtagataatttgataaagattgataacttattaaaaattatagccaagtcttaatttaatggggtctgtatgtggaatgtgctgactatatagaaaatcaaagaggaccatcatgttacctttcaacttgctgttgatcctgtatttcttactgattccggctaaaccactctgcgtccacttctggccagcaccgtctggtaagccggagtaattgggctgataattctgctcatagcctccatttaggaaaaaggttcccttcagtttccagtcgataaaggaacgcaggcccataccctggcctgaaaaacgaatattatcggaacttgtgcccatgcccagtttgtatgaaaggcccagtcctgcgcttccatttttatgaaacttataggctgcctggcctgcaaggtcaccggtagtaggaaaatatctattactccgttgaaactgaacattgctcccaaattccagtctttgaaagaaacgtgtagttttcatttcacttggtttaaaatccggcatttcgtcggcactatttaatgcgggaaatttattcttaaggtcgtccatctttgaccgtgcagcatccatttgttggctcaacatgcccaccgcatttggtccgcctgccgaaacacgattctgtaaaagtgtttcaacctggcttcgggtttgcaggcctgcaacagatccagcagaagtggcacttccaaaattgaataaggaggctaattgggaatttttcgccaggaaatcctggtaagcaggaattttccggatcagttcaattgcttttgcttctgccttccgtttatcctttaacgcctcggtaattcctttaacctgtttgctgtaataatatgcttgtcgtttaaggtgtttaagattgtcagcaaatgcaacattatctccaaggcggtccaacagtagttttttcctttcctgtatgtaattcttaattttctcgctgtactcaagctttccgattagttggttgatattatctgaacctgagtttatacctcctgctttattgtgcagatctcgggtgttgagacttttgtttttaagaaaggcaaatgtagtattcagcgtatcaagatagctgttatattcaatcttggaaattgaaccagatatccttccgctcattaagctagagaaatgcctcatggaatctaccgatgtggaaaacattgactttgcggcagaagagtctgatttgtacagtctattcttaatctgttgctcctggactatccatttacgcaaagccttgtcggatgtacggactaattggttttggcttctggttactttcttgttgatgtgagatatggctttacctgtaatgttcaattcagaagtatcttgagcaatgcaggtcttcgcagataatattaccagaacaaaggttaggggaactaagagtttcatgcgatttagggaattgtatgacaatggtaaattaattaaataaatgccagtttacgtatgcccgacaccgtaagaattaaagattcagtataaatactgcctacatttcacacgtatagatacgtcaaatagaatattatgttatacaacaatattaacatttgaaattgtcaatcgggctgctcgccaccccacttttcttaagggaattgcaatgctttagtttagcaaatgggaaagaaatgcgaattacgttttagtaaatcaaatgcactggaagaaatttttagctcgtgttaggagccttagaacttgtcctctatatcgcatggggttagaaatacacaattatcctataccattacttttgatactctaggattacggaatcacgagctatgacgctatgctttgattacaaatgaacttcactcaaacgcagtgtatttgcgtggcgaatttttgtaagtgaataatgggatggcaaataggttcattactaatattatttttaagtctgctaaacttgaattcactttatcattagcacttttcttttaaactgcacaaactgatagtccacagcatcatcctgagcagaagctaggaacactttttaaaaccaatgataaaagttttgtggtcttgctaataccgttttaatactatcataaaaggaggtttagttaactttcggcgcactaatcttagtgttttaaaaaaatgtaagagaccgtaagcagtgttttgatagcaccgaacggtctcttgttgctcttgtttagttgtatacgattgggtttagttatggcagatcatttttatcgacgggtctttaggctattttgatacaacatagtttattcgatacgacaacgatggtgtctcgaccgtacatgattgctccgcttcttccgtctggtagtcaactgtttcagcagacagccggttctcaggctcaatcgttttgttagaaagagacttatggcgggcaataatttcctccatgcttacttccagtagctttactgtagtcggttgctgctggtcgagtctcgcttgcaaaatcgtcatgtcctctttcacttttgctgcaacaattttggcataaacctgggtggtcgaaatttttgcgtggcccatcattttgcttacactttcgatgggtacattcttagcgagtgtaatgtaggtagcaaacatgtgacgggcatcatgaaaacggagtggtctgctatagcagcgtgcagtacttattatctttagttcagtattgagctttgaattagatatataaggaaacaacgcttcccgttcgatagacctttcatcttcccaatactttttaataatagcaagcggttgatgtaagaggggcactagaaagtaattctcggatttcaggcgctggttactgatccagcgctggccatccagacccacgaccaggtcaattggttttagcgccataaggtcaccatatgaaacacctgtatagactgcgaaaatgaaaaagtcgcgtaccatttgctgcaccgggtcattgagcttgcaagtttccaggtccagtaattcaaattcagtaatgtatttacgcacatattttttctttggcgcccggtatttctcgacacggttaacagcgagctttccactttgctgcgcccaatttaccatccgttttacgcgctcgatatgttttgccaaaccattttgacctgcagggcgatggggaatgagtgggttttcacgaatataggttttaaagccggccataaaagcgtggtccatttttgacacacgtatatcgtttgcggcgtattgatcggtgacatatgcactaatgtagcggtaggtagtgacatagtttttccagcttccccattccatgtctggtttttggtctttttcgtattcgctcattaaaattttaagggtgtaagctgcttctggttggttgatgccggtatatctgttttttactgcatcggcgttcagcacatcgccttctcgctcaatttctttataggccttcaaaactaagccggcttctgtttccagctccgtattgagctgtctcatttcatcggtgatcagtttcggtcggccttttctactgttccatagttttaaatctactgaatactttaaggatacttccctgactactttgttgacggttaacttcaaataaaggggagccaccccatctttgcctttctcggctcgggccttaaaagaaacggcgagtgtgtttggcctttccatgtcatttcattttttagtgttttaaaatcatacagcacttttctggcacacagggacacttgaaaaatgaatccactggtctaaaatggtatcatttgatatcaattggaaaacaattagttaattgatattcaaatagttaagtccattctgggaaccgaaaataaggtatcgtcagttcctgaccaagttcaccacttagttcctcaacgagttgacatgaattgatataaaatgggctaaatgttttttttagtctttgcagatttaattggtctacaaagaataaaatgaaaaacacctagtacatctatgatcgcaagatgctttctggttaaggatttgcggggaactgccttagtttaaactggcgataaatgaattgaacaacatgacttggagagatactattttgacggcttatatgacttgaaatacgttgaaataattattcgtaaatcaaatcccgctgaaagtgggcgactgtagagggtttgcgccgataatggcggtcggttcactacttagttcccgcggaaatagcccctgtttttaagcaaaaaagcatgaaattcaatgctttgaacttcatgctttgactccgttggtcgggatgactggattcgaaccagcggcctcttcgtcccgaacgaagcgcgctaccgggctgcgctacatcccgatgggaaggcctaaattaaaaatatttccctatccaacaaattttcatacaaaaattctcctgaacatcgcggcatacatatgccccgacccatacagggaaggtctttcgttcaacttcaccgcaactgtaaatcctgcccgatgaaacaatgcttttaaagtctgaaatggcacggggtagggtacccagggattggcctttgccgtttcatattccactatcaggaatacaccgtcttcctgcaggtgtgcacttattttatcgataaaggccggtttgccgggtacatagtgcagggaattggccattaagatgccgtccagccctgataggggtaaatcatctttcaaaaaatccagttgccccggttggatggtaacatggcgcggattgggctggctggacaaagacgggggtgttttatcccaggcataaatagtactgcctgtttccagcagattagccagggcataggtaaataaccctgatccgcatccaagatccgcccaaaccatttgagtcctggcagtaaccgggggatgttttatcagcgcaatagcatctcttatatccatagctcataaaggtacaaggaaggaaccaggttcgtaaatcccatactaaaccctaagttaaaacaaggataagccgtatttgataggtacggcttatctatggcttatctccaaatggaaccggccacagcctcccttaccagttaccttttttctaaactattgtcccgttcattttacccctccctttattttaatccctatttttgcggctgataatgaaaaataaaacaggcatgaaggcttatataggattatttttaataactgcactcgccgcctgcgctggcaataccggccatgaaagccagcatcagggcgactctgcaatggccgtggcccccggggaaatgcaatacgacaccgcgctggtggctaaccggagagaccccgtgtgcagaatgcccatcaaggcagggatttacgacaccgcccattaccagggtgctgttctcggattttgctcctccgcctgcaaagacagcttcctgttaaaacccgcagcttacacccttgtcatgaaataatgaagaagatactcctgatcactttactggtagccggatgtgcatcgccggcgaaaaagctgcccatactgggtgagccgggggtaacagcgcgtcaggataacgggaaaacagtatacgacaccacgtaccccgttgttccgcctttttcgtttagggaccaggacagcctcccggtaaatgaacagtcatttgaagggaagatctatgtggcggattttatctttttatcctgcccgaacatatgcccgaagatgaccgtggagatgaagaaggtgtataacacctttaaagcaaacgacggcatttttttcctgtcacacaccattgacccggaagacgattccattccccggctgaaagcatatgccgccagcctggaagtaaccagccccaaatggcggtttgttaccggtagccaggataccatttaccgcctcgctgaaaaaggatatttttctacggcgtataaagacagctctgcccccgggggctatgtgcacagcggcggactgctgctggtggataaagcccggcacatacgcggggtatataacggtactgacccacgggaaacaacccggctgataaacgatattaacatcttactaaaagaaaattgaagaaaatactatccatatggcttctgtgtatcgtgcttttacaaagcaccggtaactgctggatagtagccgcattttatcttaacaggaactatatcgcctccgaactttgtattaaccggttcgacctcatcccggtttgtaaaggcgcctgcttcctggacaggaaaataaaagaaaacgataaacccgaaaatacggtcaatacacgcctgaaagaaattatcctgttttgccagcagtatgatcctgccccggcaaaacctgtttctactgaaagccttattacctttcgtggctataagtcgccgtattccccgcaaagcctcatcaggcaggtattccggcctcccgctgctacagcgtaatttctcctgttacgttcacatcattaagctactacatgagtatgaaatccagcgaaatagctgtgttatctgctgacatgtttgacaccggtaatgattttttctggataggcagcctcggatgtatacccgataagtaccctttgctggaacagccccacaggcaaatgttctacatgctgctgtgcattgaaagcgcacagggcacggcggtaattgacggcgctgttatccggctggatcatccgaaaatcatttgtgtaaaacctggcagcatatgcagcatacatatcaaccgtgccgcccgcggtaacgttatttgctttacagaaagttttttctccctgagatataacaataatgtactgctcaacttttctttcctgaataaggaaagcattcacgaaatatgcctggaagaaaacaaaacagcagagtggaaccagatcacccggtttatgcaccaggaattttacggccggcataaaggcgccgctaatgtgctgcggtcgtatctgaatatcctgctttgtaacctcgaccgccacttcaatccccccacggggatagagcggaagcacaacaaagaagaaaaaatgcgtcagttcaagctgctgctcgaagagcatttcgtgcaacataaaacgccttctttttatgcggggcaattaaatatcacgaccaactacctgaataaactgtgcagggaatataatgggctgtccagcggagagctgatccgcaaaaggattacgctggaagcccagcgcctgctgcattacaccgggttgtcggtggccgaagtagccaaggaacttgcatttgaaagcgcttcttatttcgtgaccttctttggtaaaaatgccggcatgacgcccgaaagcttcaggaaaagtcaccggtaatttattgaagctcctcgggcagccacgaaggatagctgctgacggacttcttggctgcttccgtaacaggcacctgccacttgtcaaaaaagagggaaagatctttttgcgtggcggtgctgatacacctaaaccagtaatcccttttatctgcttctgataccgggtattgcgcggcaggtaaagcgcggtattttttgaagacgtcagcaataggctgccacccgaaatgttcaattatttcgatgtacatttttaaagcgagaaacggatcttcgcggaatttatcaaaaccgggctgccctttcatatagctctttacagcatcgataaccgcctgcctgctggctatgttttcatgattataaagccctttatgcagcacctggtcatatacatacatggtgtacaggtttaccgttacctcaccaaggccatcgaaatcaatgccccagaactggtgacgatggcccagttcatgaaaatgtccccaggagccttttgcccgcagctgcgcttcatccagcatcagggcgcaactttcatcatcgggcgccataattttatgtggcgccgtatacatataaccaaaggctacctgttgatcgatgataatcctttccgggtgaatcctgtcggccgaaatagctgccagccgggcatcggcatccatcacttcatcccagaatttcatcagcttttcagggtcgtccagtttacggatgcgatacgaaggaacagtaagcacaattttatcagtagccagttcggcccacggccccgggtagttgcggatggtatgttgccagtcggctaaactggtaacgcccaatttgaagtacggacttttaaccgccccgtttacctgtatatgaagtgttttcagtgaagtggtgtcgggcactttgatcatcaacagccctccaaacggggaaaagatggtggtcgccggttggtcgagttcaaacgtttttgtgaggtcatcagtatgacgcacataataatccatatggcttaggttgtcctcatgcacgcctatctgtgctttcagctgttgtggaatgcagtcgggggaaatggtaatcgtcaccgtatcgcccgctgccacgtataaaccggtgctgtgccaccggtaaaacacaccatcgggttccaacaacccctgggcgcctgcctttataggtatagctaccggctcattcactctcggagccgttttactcacttccccgggaaacaggctgctggcaggatggatgtaccctgtgtcggtatgcccttgctggtgttgtgtggccaggtaattttgaacattgtagatgaaccggttttttacatcagttttccagagcgggtgtgtgggagatggaatgacgggcgcctgccggtttgcaaacgttgacctgattttatttgatatagcagtggtatcgggattattaaataaatagttggctatggtgctggcgtagctgtcggcgtcagcagcggcgggtataaacagcgtatctttaaatgcggccattaacgaagaaatgtgcacatagggaggaatggagcggatcgttaatccctcttttctatcttccggttttagcgtggcggttacgtgatacatcccggctttcctgaaaagctggtttaagcccatttcaaaataactggttttttgctggcttaaaatgtcagtagcgggagaaccaaatatcaaggcgcctccttttcttacaaatgcttccaggttatttcttttaacggtatcggtaacatcctgtgtaaggataataatgccggcggcaggtgcaatgttaacggtatcagtgatggtgttgtattttttcaggaaatgtaagaacggtggaagatcgctgttaccgccccatacctgtacgctgccgcttttgttgcctgcccatgcgatagcattgcgcagcagttgctgtacgttcctgtcatctaacaggggctttttaaaatatttgtcggaccctataatcagtatcctgcctttatccagccgggaggccatgataacaggcaggtgctgctttgtatctttttcggttgcggtggcaataatggtgggtttttcatttagggggatggtgaaagtggcattatccggcgccggcggcatcgctatctgttgaacatgatccagcaggcgttgctggtcgcccgattgtgcggataacgaatgatgggagagaagaatgccgctaaaaatcaggcagatagcagtctttccggcaacagtgttgattgatgtcatgaattaacagggatgggtttaatgatacgctggtctgccaatttaataagaataaaaacagccgcagagatcttcctttgcttgataggattaaccttattccggggcaatgtgtatgattattgcagtcctgtactcaaacaaccctattatgagaagagcttacaaaaaagcagatctcccggtagcggagatccgcagattcctggaacccggtccgattgtgctggtcagttcccgctggaaaaacaacaccaacatcatgaccatggggtggcatacggtgatggagttttccccttcgctggtgggatgcatgatcacggcggagaaccacagttatgagatgatccggaaaagcggggagtgcgtgatcaatattcctacggtgaacctggtagaggagatcgttgggatcggaaatagtaccggcgcccatttggataagttccggaaattcgatctcacggaggaaacgggaaacatcgtgaaagcgccgctgataaaggaatgttatgccaactacgaatgtaaggtagccgatacccaattgctgaaaggatacaatttctttatcctggaagtggtgagcgcccgcgcggctgtttatccgaaatatccgaaaacggtgcattacaggggagggggcatctttatggtgtcaggaaaacacattaacttgagagcgaaatttaagaaccagaatctatagtatgctcactaccgttatccaacacattttactgatcttttttattttgttgctggtgatgattgcgcagaaattgaaaattgcgtacccgatcatccttgtggtgggtggactgtgcctcagcatgctgcggcttttccctaccattgaaattaacccggagctgatcctgctcattttcctgccgccactgttatatgaagcggcgtggtatacttcgtggaaggagctttggcgatggcggcgggtgatctctatttttgcttttttaatcgtgattgttacttccggtgtggtcgccgtggtatcccatgcgttgatcccgggattttcactggcactgggatttgtgctgggcggcattgtatccccgccagacgcggtatctgccactaccatcctgaaatatgtgaaggtgcccaaaaggatctctgcgatcctggaaggggaaagcctgatgaacgatgcgtcgagtttgattgtattcagctttgccaaaacggccgtgatcagcggggtgtttgtgttgcatgaagcggcagcgagctttgtggtggccattgtgatgggtattgccattggtttgctggtggcgttgatatattatgccattcaccgctggctgcctaccggtacggaaatggatgtgatcctgaccctgacggcgccctatgtaatgtacatcacagcggaatatttccacgggtcaggtgtactggcggtggtgagcgggggattgttcctctcttcccggagccagcatatactcagttaccggagccggttgcatggcgccaatgtatgggctacgattggatttatgctgaacgggctggtgtttatgctgatcgggctggaactgccggtaatcattaaggaactgggtacggtaagtctttgggatgccataaaatacggtgtaattatcaccggcgtgttggtggtaacccgcctgctttgtacgatgggcgcctccgtgttcacggtatttatcagcaggtatatcaccacggccgacagccggccgggttggaaaggtccggttattatcggctgggcgggcatgaggggagtggtatcactcgccgcggcgttgtcgatcccagtgtatatggataatggcgcgcttttccctcagcgcaacctgatcctgtttatcacttttacggtgatcctgcttacgctggtggcgcaggggctcaccctgccgctggtgatcagatgggtaaatatggaagatcccgataaacaaatccctgcagaagagcaggagcggattatccgcgaccggctactggaaggaagcatccgcttcctggatacccaatatccggaagaggtaaaggcaaatccggcgctgaagcagctgcgggaagacctggagcttcgcaaaaccgtgtccatgcacaataagattgaaggattggaccacctgttatataagaaagtttatgtgaagatgctggatcaccagcgccaggtattgcacgaactaaacaaggacccggctacagcgcacgagctgatccggaaatatcatgagctggtggatattgaagaggagatcctgagaatgaaatatgaacctgcttcctgaacctgggggcataaaataacaacagggtgcttccggtattgctccggaggcgccctctcattgccggttaacgttatattgcccggtatttacttcacatgaacgctgatcactttggccaggtcaaacatggagatctgcttcttcccgccaaataatttattcagtttatcatctgcgttgatcatgcgtttgttggcagtatcctgcagattgtgcttcttaatataatcccatactttttttacgatctccgttcttggcaatggggtggtaccaataacagcggccagttctgcagagggtgcgagtggttttttaagcccggaaccggcagatgcgcctgctgcttttttggcggcagctggtttggtggcggctggcttggctgcagcagcctttttagcaggcgcttttgctgcaggtgcttttgccgcaggtgcctttgttgctgctttctttgccggtgcttttgcagcagccgctttcttgccggtagtacttttgtttgccatttttctggttttaagatgatatgatgcagtccctggaggacatacgccccctaacatcaacacatatgccagtttgcctggaaaacgcattattcaccatatcaatttcccgccggcattggatccggagcagcgggttatgaggcaattgcaggtctttagcaatacaggcctgcttttatagcacttaattgtatctttccaccatgaaaaggagtgattacctgcggcagggaaaatctgaaaattaccaggatgccgaagagaaagggttattaaaggcgggcgaagtggccgccttgctgtcgaagaaattcaacaccaaaatatccgcaaaggaactgagcgtattttccacagaatggcaccacgccggtgttttcaagggcgcacggaatggcaggttgatcgggcgcaaagtttatttcttttcggccaccgatatcagccacatctccctggatgctatactcgccaacaggaataaggcggctgaaaaaccactgccggacaatagccccgttcagggctggtatccgcagttttttcgtatgaccgaccccgttacccgccggactttccccaagccctttatcggcatttacaaagggccggcctccaaagcgccaaagggtttcagggcattgcccgatgacgcatttgcggcagccgaaaagcagcggggaaaggaactgaagccaggagaggagccccggttttaaccgccactgcatacagattccggcttttttacttaacttaattaaagtaaataaatcatccactacatgaaaagcttgactactttgccacttatttcccggtataccgcagagcaaccccgctttaccttactggattccgttgccaacaggatttccctgatcgtgttctgcagcattttcagcttcctgttcatgtatatcttcctgccttttaatatcaatatgtggtacgaaggacaaccgctatccctgatggcattgttcctcatttttaccttatgtggagtggtagtgctgaccatcacacagtttggcctggccaggttaaaatggcggcgtaagctcaccaatgccacctacctctgctggttcctgggcgaaattgtgggcgtagccgttatggttaccatcgtggatgtaaccctcacggatacatttttccttacctgggccgaatttatcaatacccttcgttatatcgcccttattttaccgctgccttactgcatttcgctgctctggttttttaccagggagaaaatggcccaactcaaaagcctggaaaaagaacaggtggtcaaagccggtgatccctgtatcctgatccgtgacgaacatgacaaacccgtgctcaccctgcaccctggcaagttactgctcatgaaagcagaagataattatgtgcaggtattttacctctccggaaataccatcagcaaggaactcgtcagaacatccctgaaaaaactggagtcgtacctgtcgcccgataattttgtgcgtgcacatcgctcttacctggtgaatatctccaaagtggttctttttaagaaaaacacaaaaggacattacctggaactggagggtctcagtgatatcagtgtaccggtatcggctacctgtttaacggctttccaggaaagattcgcccccgtgccctgatttttacccccaatagccccggtttcgccccaaagtcaatggtaccaatgcgttccgtccgcgtattttggtaatatcgctatgccacaaggcgataaattaaacaaccaagccatctaaatcccacctgccgatgttaagatccattatcataagtatggtttgcctgtttggggcgcgccttacggttaatgcacagattgtgatttcgggcaacgttcgcaacagcgttacccaggaagtagtgcccgttgtttcagtaaccatgaaggaagcacagaacggggactataccaacgaccagggaaactttaaattctctacccggaaaaattatcctgttacccttatactgtcatcggtaggctttgaaacaaaagaaatcatcatttccggtcccggatttcagcgcattgagctgtcgcccgcatcggtactgggcaaagaagtggtggtttctgccagccggtttgtacaaaagaaaatagaatccccggttaccattgaaaggatcagcagcaaagatatcatcaactccccgcagcccagctactataacatgctgcagggcctcaaaggagtagacgttaccacctccagcctcctgttcaccaccgttaccacccgcggcttcaataccagcggcaataccaacttcacccagatagtagacggtatggataaccaggcccccggcctcaacttccccatcggcgctattattggtcttacggagctggacgtggacaacctcgaagtgctgtccggcgcctcgtctgcattgtacggctcccgcggcctcaacggcactatggtaatgaccggcaaagacccgttcaaataccaggggctcagcgcacagatcacacaaggcgtgaaccacgtgaaaaaaggaaaggccaatgatccgctggggccatcgccttactacgactggaccgtgcgctggggcaaaaaagtaaacgacaagttcgcgtttaaaataaatgtgcaatacacccaggcgaaagactggatggccaacgataccactaatgccaatggtcccggtggcccgcagcaggatcctaactataacggtgtaaatatttacgggagcaaaacatccgtagacattaaccccttcctggaaggagccctggcgcaggtgccggaactggaacctatcatttcgcccatgctggcggaaggcaggcatatggtagcccgcaccggctacccggaatacggctacctgagcagcgacgccaaaatgttcaaagccaatgtggaactgcgctataagatcaaaccgaagctggaagccattctgtcgggtaccttcggacaaggcaacgcggtatacagcaatgatacccgctacgcactcaccaacttccacctgggacaataccgcgccgaattaaaagcggagcactggtttgtgagagcctacacttcccgcgaaaattctggtcgtactattatagccatgcccacggcgcagctgatcaacgaagcctggaagcccagctacgacggtaataccggcgatggctggtacccgcaatataccagcgcattgctggaagctatgtcgcagggtaaaagttatattgatgccagcaacctggccagggcattcgccgaccagggccggcccgacgccggcagcacacagttcctgcacctgaaagacagtatctccaacattcccacctccaaaggggggaccctgtttaccgataaaagccgcctctttaatgcagaaacccagtataattttacacacctggtaaaatttgcggagctgattgccgggttaaactaccgcctgtaccggctcgactccaaaggcacgctgttcccggataacgaaggacctattgatgtagcggaatacagtgcttacgctcatcttaccaaaaaagtgatccgcgaaaaactgagcctggctgctgctttccggtatgataaaaatacgttgttcgccaaaccgcgtattaccaccagggtatctgcggtactggaagtgaacaaggaaagtttcatccgtttttcttaccagaatgcgtatagcttcccttccaatatccagtcgctccaaagcaccccgatcgattacaacagcttcgcctccggcgggtccgacaggctgctcaacggcgtataccagtttaataaatacccggcctatacgctggaaagcgtggattcattccagcgcacaaagaatcccgccgacctgaaacagtttgctttgaatgatatcaaaccgcagtccgtagatgcgttcgagttaggttactcgtccctcatcgccggcagggtgctgatagacgtgctgggttattattctacctggaaaaatttcattggctatgtaaatgtggccaatacccccggtacggcagatcccaacgccttcctggatcacagcacttatatccagtataatattgcgtataacggcgcggaaaaggtaaatacctatggctacgccgccagcgtgagcgtggacttatcacatcacttcctggcaaaggtgaatttctcgtccgatttcctgaaaaacaggaacaacagccaggtgaataattttaacacgcccaactataaattcaacatcgattttggaaataccggctttggtaagaaggaaaaattctcatttaatactaccttccgttacagaccggcctatttctaccagattggttttggcagcggtacggtacccgcctcggcagtcattgatgcacaggtgagttaccggctcctgcaggcgcattccacgattaaactgggtggggtaaatctcaccaatacctattacagaaatggcttcggcagcccggccatcggtggtatgtactacgtcaccttcgcttacaatgttttctgatttatttaaaataaatatttccaagtatgaaacgatatcctatctgtttgttattgattgccctgctggcagcctgccagggtccggaagttcaggagaagagcggttatagcacccggcttcagtttggtcccggtgaggaaacaaaaattgcggaagcctttctgtcgctgacagacagcagcagtatcaccttaaaagaagggacttataagtttgataacctcagtatcgcccaggtaaatcatatcctgatccagggcgccggtccggataaaacgatcttcgacttttcggcccaaagccagggtggggaaggcatccgggtaaccgatgtaaaaggatttaccatcgacggccttaccctgcgcgactccaaaggagacctgatcaagatcaataaaagcgagaaagtggtagtcaccaatgtgcatgcgatctggtcggtatccgattccaccagcggcgggtatgccatttacccggtgatgtgtaaaaatgtgctggtggaaaactgctatgcccagggcgcttccgatgccggcatctacgtagggcaaaccgacagcgccatcgtgcgtaaatgcaaagcctttaaaaatgtggccggctgcgaaatagaaaatacttccaatgcacaggtatatgataatgagttttggggcaatactgccggcttcctcatttttgacctgcccgacctgtcgaagcgcggtggctttgtaaaggcatacaacaactacatgcacgacaataacgaaaagaattttgccaaatccggcagcttcggttccacctggggcgtgggcaatgctgctcccggcagtggcgtggtgatcctcgccgcatctgatatagagctgtacaacaatcgcatcatcaataataactccagcgctatttcagtggtatcaggattttttattgatgaaaaagccggttcaaaaatcaacgatcactatttcccgatcccccgcaatgtgcatatacatgataacattatggaagtgggcgccgcttttccgccggcagtatacgagcatcataccgggaaaattctggtgggtatagaacagaaattaaatgcagatgatccggcgcgtaaaaatgcccgcctgcctttcattacctacgatggtattaccaccaacatcctcacaaaaggtacagcggtgaatcccgattcgctttgtatacagcaaaagggtcccaacttatttgtaaatgtggatgccatgaacatgatgtcgaaaaactggaagcccagtaccgatgttacgccttatgtatgtaaatagtgtttttattaaattttttaagggagatgaggaagtcttgtttatttgtgatgtgtttaattttatggatcgccgccacgcagagttgtcagcaacggccgtcgcctgctgcaacagccggtccgttccagtttaaacaaaaattatctgagtatggattttttaccggtgcactcaaggcattacagccgcgtaaaggcatcgtgaattatgaactggctacaccgttgttcaccgactacgccgtaaaagaccgctttattgtattgccggaaggaaaaacgatgggctacaccggtcacggttccctggattttccggattccacttttatcattaaaaactttgcatacaccaatccggcgcatgaaaagatcatgatagaaacgcgcctgctgtttaaagatccggcagaccggcaatggaaagtgatgaactacctgtggaataaggatcagcaggatgcagagaaatggatactgggaaaaaagattcccatcaccttcctggacgacaactggcgtgagcagtccaccctgtaccagatgcccaacaccaatgactgtaaacgttgccatattaataacagcgtgcttacgcctattggtcctaaagcgcgcaatcttaactttgtgcgtcatgggcaaacgcagaaccagttacagcaatgggccagcaatggcttgctgacgggaatgccttccctggaaaaagtgccacggctgcccgattggaaagacagtattcactacaccgcgaatgaacgcgcgcgtgcttatcttgatgtcaactgtgcgcactgccacaccaaaggcggcgatgcgtttaataccggcttattcctggaatacgaacaaactgccccggaccatctcggcataatgaagtcgcccgtttcggcgggtggcggcgccggcggactggattatgacgtgattcccggcgacccgctgcactccatcctggcttaccgtatgaacagtgtggaaccgggtacggctatgccggagctggcgcgcacggtggtgcatacagagggcgtggcgttgatccggcagtggattgcggcaatgaaataacgcacgcggatgttgtcttactcaggattacgctgattttactgattagtttgatttttacttttggattttataaaggatttggggagatagaagcgaacttggtctttctcgctgattacgctgattttactgattttactttttgaaaaatattggggagatataagcggaatatgtttgcttatatctccccaaaatcattataaaaatccaaaaaatccaaaaaagtaaaatcagtaaaatcagcgtaatcctgagtaagacaaaatccgcgaaggccgaaggccttctatttgcacgctccttccaccaatgggatgttgtcgaatttcagcgcttcgttctggctgttgaacacggggaggccctggtggtcgatgctgtcgggtagtgcttcgtatgcttcgtggtcggagattttgaagatcacctggcgggagctttccacgccttcgctgaagaaaacgtattttccgcggacgatgccattgctgataaggccgttgaagtcgccggtatttttatctttttcaaagtaattatataccagggtgccggtagccacgctgtcgtgcatggttaaccggagctggatggtatccctgccgaggaccttttcgaagcaatggttggatttttctttttccaccacgggtggcaatgaatctttggcagcgttggtttgctgctgctggccttgttgttggcaggatgcaaagatgcctgcaccaagcgccagtaatatgtaaggtgttttcatatattgaaagtaagaaaaatgaggcaaatgaaggaaagaggggccttttaattccacggaaaaaattgtaattatgtggcgccatagccaaatgtggcgatatatcttactaacaatgaaaaaaagagaatcctttctggccgctatgatttgtttgctggcggttgtcacttcctgtaaaagcagtgttgccctggcgggaaatcatcccgataccgctgttacggtggcgacctgtaatcaatgtatggtgatagcggagcagtcgcagcaccggattataatcgcagcaatgccttccggtgaggtgatctgggaatggaagccggaaaactccaatgtgcagccggcgcatgtaaaatggttcagcaatcccagcgacgccaaaatggtgtataacaatgaatatgtgttaatgaatgcctctggcggcggtgtggcgctgatcagggtggcggataagaaaacggttttttatgcctatgcaggcggtaatacccattcctccgagttattgcccgatggcaatattgtgagcgcttccagtaccggcaactacctgatggtgtttaaaacagataccgttcatttccccgataacgtatatacgaaaaagatacccattgatttcgggcataatgtggtgtgggatgcgggccagcaaagattgtggtcggccgccagggctcatatgcattcattcaggtataacttcaactgcaacgcgccggatttggtgcaggataccgttttttccctgccgggaacggaggcacatgatctctttccggtatatggtgaaaataatctatggctgacgaataccaccaacgtatataaatttgatgttattacacaaaagctgacgaaggccgatgtgttgcaggacaatattaaaagcgtttcttccgccgggaagggccttcccaccattgcgatccggccaaaggaatcgtggtggacggatgaggtgctcgacgccaaagggaagcggctgtttatccataaaggctggaagatctacaaagccaggtgggtagtacgcaatgcgttcagctatccggtgggcgatccgatgcatttgtgcaggtaaaacccgttaatcttcgtacttttgcggcaatgcaaaaagaaaaatactcattaggtaatattcttaccaatttaaagatcgattcactcaatgaaatgcagcaggcatcagtggacgcaaacaagcatcacaatgatgttatcctgttatcggctaccggttccggtaaaacgctggcattcctgctgcctatcctggaaaatctcgatcctgccaataaaaacacccaggccctgattgtggtgccgtcccgtgagctggccttacagatagagaaagtgttcaagctgatgggcaccggctataagatcaccgcctgctatggcggacacctgagggaaacagaagagaacaacctgatacagccaccagcagtgatagtaggtacccccggccgactgggagaccacatccgcagggaaaatatcactacggcagctattgaaacgctggtactcgacgaatttgataaaaccctggaactgggattccaggaggaagtgtctttcattattgaatcgcttcccaatatcaaaaaacggatactgacttccgctacagaatcagtggacatccctgatttcctggcgctggacaaaccggaaaagctggacttcctcccggaagaaggcacgcctgctgcccgtttaacaatcaaggaagtgctgtcgccggaaaatgacaaggtagaaacccttttccgtcttatctgctacctgggcaaccgctctaccattgtgttctgcaatcaccgcgaagcggtggagcgcaccagtaaaatgctgtctgaaaaaagtattatcaataccttctatcatggcgctatggagcagcaggaacgggatgccgccctctgcaagttccgcaatgggtctgtaaatgtgttggtaaccaccgacctggcagcccgcggtcttgatattccgaatatccgttatatcgtgcatttccatctgccacatacagaagacagctggacgcaccgcaacggccgtactgccagaatggaagccagtggtaccgccatcctcatcctgtcacccgatgaaaaacggatgccttacctcgcggatgaagtggtagaagacattgaactgcccgctacctccaccatcccggacaaaccgaaatggacgactatttttattgccgccggcaaaaaacataaagtgaataaagtggatatcgtgggattcctgtctaaacaggcgcatttgaagaaagaagatatcggtttaattgaagtgaaagacttcttctcctttgtagcagtggtgaaatcgaaagtgcagaatacgctggagatgattaaaaatgagaagatcaagaataagaaagtgaagattgatatagcgagatagggatataagtaatttaaagagaagctgtctcataaataaatgaggcagctttttcattttaggctttaaggatggttttatccacaatttgcagttgaaaaaaagggaagttgtaagtgtttacgcaccagaagttattgtgtaaa

SEQ ID NO: 7 - DNA, 472903 bp, Chitinophaga pinensis
  source 1..472903: mol_type = genomic DNA
aagcggatatccgcttatatctccccaaatctttttaaaatcaaaataaaatcccaaaagtaaaatctgcaaaatcagtaaaatcagcgtaatcctgagaaagacaaaatccgctctaaaccttgcattcgtaaacaatagagctgcaccggtccacggttttcaggcctttgcgataggagcggaagccatggaagaagccctgcaggagccggcttttgccggttttgtatttttcgctgagcaggcttacgtagaagccgtcgaataccatcgggtgttttttggccagtttgatatgatgctgtgcaagtagtttttccatggagcccggcgagaaatgatagagatgccggggcacatcgtaggcggcccagtattctctataatagtcggcgtcggaggaggtgtagttgggaacggcgatcagcagcgcgcctccgggtttcagcagggtgcggatgtgatccaggtagccgtgcaggtcgtgtacgtgttccagtacatgccacatggtaatggcatcaaattgctgcgcaggtaaagcatacagctgttcaatgggcagtgcctccactttgtaaatttctttggcgttgcggcgtgcattttcatcgggttcgaggccggtgacagtccagccgccggtttgcatataatgcaggaatgccccggtgccgctgcctatatccagcagggtgcctgtttttataccgcaggcattgcgcacccagttttgtttggagcgcagcgtaattttcctgacactgtgatataaacggttaatgagtccctgctttgtttcagagtgggaaatatattcctgcgactgatagtagcggcctatgtgggcgctatcgggcaccttttgtgtaaagcggccgccacagcctccgcaatggaagatgttgaatgtttctttcgatacggtgtaatctttggcggtaagcgcttcatgtatctgtgacgaaccacaaagcggacagttgttgtaatagattaaactcattggactattgaatacgcttatataattatttatactctccccaaacttcccgcagtacatctgcaatttctccgagggtacataagtgttccactgcggttactacaaggggcatcaggttttcatcggtgccggcagccagccggatctgtgccagcgcgttttgcacggctgcattatcgcggcgttcccgtaaggatttcaggcgttccgactgtaaggtacggatgctgtcgtcgatgcggaatacttccggtgttacctggtctgatgctgtaaatttattgacaccgatgattattttctcattattttcaatttcctgctggtacctgtatgcgctctttgctatttcatcctggatgaaaccctgttctatggcgcttacagccccacccatcgcatcaattttatgaatcagttcccaggctttggcttctacttcgttggtaagtgcttccacataaaaagaacctgccagcggatctacggtatctgccacgccgctttcgtagccaacgatctgttgggtgcggagcgcgatgcgtgccgctgcttcggtgggtaacgacaaggcctcgtcgtagccgttggtgtgcagcgactgtgtaccgcccattgtagcggccagcgtttgaatggctacacgtacaatattattctgtggctgttgtgcggtgagggtgctgccgcctgtttgcgtatggaaccgcagcatctgtgctttcggatcggtagcgcccagcgattgggtgatatgcgcccacatgcggcgtgctgcgcggaatttggctacttcttcaaagagatgattatgtgcattaaaaaagaaagacaaccgcttggcaaatacattgatatccagtcctgtgtccagtgctgctttcagataggccttcccgttagccagcgtgaaagccagttcctgcacagcgttggcgccggcttcccggatatgataaccggaaatagaaatggtattccacttgggcacttctttgctgcaataggcaaaaatatcggtaatgagccgcatggagggctttggcggataaatgaaagtgcccctggcagcgtattctttcaggatatcgttctggatggtgccggaaatctttttcaggtcggcgccctgccgcttggcgagcgcgatataaaaagccagcaggataaacccggtggcgttgatggtcatagaggtggagatctgctccagtgaaatatctttgaacagtatttccatatcttccagggaatctatggctacgcctacttttcccacttcaccttccgacatcggatgatccgaatcgtaaccaatttgtgtaggcaggtcgaaagccacgctcagtcccataacgccctgtcccagcaggtagtgataccttttattcgattcttccgccgtgctgaagcccgcgtattgccgcatggtccacagtttatcgcggtacatggtggcgtgtatgccacgggtgtaaggaaaatcgccgggctgctcgtccataggcaccggctgtgtgtataccggtgctattacaatgcctgaatcggtttgaatggttttttccatagtatctaaaactagcgttgcaatgttacataattattatggtacttcgccgctgagaaaaatattgatattttgtgtgaaagtttggcaggatactatgatcatttactgtttattaggcgcaacgatcgcgctggcgttgtatagtttatatcttgtctggaaagcaggaagccgccggctggcagccacctacagctatttgctgctggggctttcgctgggctggttcctgtatttatatggtacctgggtgtacctttctatttatgccaagtatgtttttggcggacttttattgctgaacatggccgcttatgcagtgcgtaagcacgatcatgcggctaaacctacgccgcggtggaaacaggtcagcaatggcattcttacctttatttttgtcgtaatgtctgtgctgtactttaccggtactaccggtaaaccagcgcgggtagcgctggcatttccgtttaagccgggtaaatactttgtgttgcagggcggtaaagggttacctaccaacgtgttccactttagtctgcggggggctgtttatgcgatggatatcgtgaaactgaacaactatggcgggcgcgcagggaaaatattttcccgtaagctggaagactatgtgattttcggcgacacggtatatgcgccttgcgacgggctggtgatgagggcgtacagcaataacccggataatataccacctgccatgaaccgcgggcctaaaaacaccaaccaggtattactggaaacgcccgggtattacgtgtttatggcgcacctgaaaatgggaagcgtggtggtacgggaagggcagtatgtaaagcggggcgacccgcttggctgcgtcggcaattcaggctttagctcagaacctcacctgcatatccaggtgcatgctaaaaaggccggcattccctggtaccagggaatgccgttgtatatcttatttaatggaaaaagttacctgttgaatgaggtgattaacgcgaagtgattaccgcatcaatctttttgcttccgcattaatgatctgggaagtgagttcggcaggagattcgccggcctgtaaaaatacctccaatatctgtttgttcagttccatagcgggtgcatccggaggcagttgcacggctacctggttgatcacggagatggtttgttcctttaatgttttcaccgcttcccatgtcatggccgacacatagatctgctgggtaacgttatgttcgtattctgccttgatttgctgtaccatcgcgatctgcatatccacggcggttaagcccggctgataagtgcgtcctatcaggctttgcggcgtgatgcggtctacataaagcgccattctctcgtaggcctgcagctgtaagggaagcacggcagcatttaccggctgttctttgctgtcggttgtggtatctgctgttttattcttcttaaaaagatctcttaccgttgggtatacgattgtcactgctccaactgcgagtgcgatgtataatagtgtattcaagtcaagactgcccatcatattactttatgtgcacaaatatatataaagatatttatatattgtaggataccggtttaaaataaaaaggattaccgggagatgtgtactttataacatccgccggtaatcatattcatcacaaagatgatcgttttgttaagcgagtttccccagccaggttttcattctttccactcctttctccagtttgtccatgccggtggcataagacaggcggatgcagttgggttgctggaaagcgccaccggtaacagtagacacgtgggctttatgcaggaggtacatgcaaaggtcgtctgcgtttttaatgtgcgcgtcttcaaatgatttgttgaagaatgcgcttacatccgggaacatataaaatgcgccttccgggtcatttacctttaaaccggggatggttttcagggcttcatgaatgtaggcgcggcgttttttgaattcagcaaccatttccacggcggtggtcagttcgccggtgagggctgtgatggcggcgcgctgggtgatagagcaggtggccgacgtgaactggctctggatcttatcacaggctttggcaatatccagcggtgcggcgaggtagcccaaacgccagccggtcatggcaaagcctttactcaggccgttgatgatgaccgtgcggttgatcagatctccgaactgcgcaatgctttcatgtttgccttcgtagttgatgtattcatatatttcatcggagatgatgaagatctgcgggtgtttggcgaatacggcagccagtccttccagttcttttttggaatatacggaaccggtaggattacagggagaggagaacatgaacagctttgtttttggtgtgatagctgcttcgagttgctccggtgtaattttataattgctttcgatactgcagggaacaaataccacttcaccctggcagaggctcacctgttctgaataggtaacccagtaaggggtggggatgatcacttcatcgccggggtttacaatgctgagcactgcattggccaggcattgcttggcgcctgtggatactacaatttgctccggcgtatagtcaagaccgttatctctctttaatttgtgtactactgcctgtcttacgtctgcatagccagccacgggtgtatagtgtgtaaacccttcatcaattgcttttttggcggcttcgcggatgtgtgccggggtgtcaaagtccggttctccgatgctgaggtccacaatatctatcccctgggctttcaactcgcggccgagtttagccattttaattgtttgcggctccgaaatccgtgacagcctgtctgctagttgattcatatcattacattgaattgaccggaacaaacgtacagaaaaaaaccagataatacatggaaagatcattcccggctgctgtacaaacgcagaacgggccggataaccggcccgttctgcgttttatgttactgctttttacagcaatgtaatattgttagtataaactgaacatagcgttggtaaccagtttgtcggtaccggtgctgcctttaacgcctacgatgtaaatggtatagaagttacctgcgttgaaactgccgacacgaagatcagtgctgcttgccgtggcaagtacggtaccagtgccagcttccttgatggtgatggcattgtttacactgaagctgttgaacagtttgaaagcgctggcagaagatacatcgccgttaaagtaaacgcggttgctgtcgattttttcagtaccgatgaatacatctaccgggcctgcgtttgcgctcaggttcaggaaacggataccgattttatcgcggctgtagttggattgatctgttttgataatagcagatctcatggggcttttatcccagatcaggtaagtatagtactgtgtggagtcgaaattgtaagtagtggtgaccagcaagctgtcgcctcctttcttcttcaggtcaaatttgtgcaggcctccgtaaacggcgtaccgggcgtagaaattataagtgaaatcagtttctgttactttctgatcattatcgaagaaagtacctgcgatcatactggtggaactgttcagaattgaaatctgtgcctgtggtcttggtggtgtgtaattgttatcgttcttcaggcaggaagataatccgatgattcctgtcaacagggccacaactgcccatacgcgatttttcttggttagcattttgctctcagtttttaaattgtgttattgatcggttgtttttttatcgtttggttcaaaacgggacaggtccggtaaaatgctctttttacgttggacttccgattcataaattatttctcccagtgctttgagaaaaggtttgcctgttttttcaaaagccggttgatcatctcccaatacaccagtggtatttacaaaaacactggcagacagcagaaattctgttttactggtaaaatcaacaatatatgctgtatcgctcagaaatccgtatgcccatcctggtttgttgaaaatcctgatgtgttcaggtatccggctgttccggtcacctccaaaaagcaaaaacctggtatatgcctgatagtattgttccggatcatacaccggatctgttgattcttccgggtgctgggacatacatctgtacaaaaaaaggtaatctttccctgttaaacggaaacgttgacgatttgttacagcttccggaaaaattatgctgcgcaggatattatgcaggtcggagaggggcagtttattccggtgagagaagttcatgggttggtgctcgaggtggtcgaggtgattgtaccaggcgttcccggcaaagtcttcccgcggggaaaactccaggctgctgcagcatgcgggttgctggtaaaggatcctgttcccttcgcggaagctgacggcgttggtatgccggttggcttcctcgtagaggggaagtcccacccggtggcggatctgggcctgggaatatcccatttcccataaccggcggttaaaaggttcctgccctataaactcgtaaaggcggttataggcgtcgttgtcgctgataaggaatattttttttatataatgggctacagacgggaggccggaagccgcggaatggtcgtggcgcacgccggtattcacatccgggagcggcgctgtaaaaaaaggcgtattgcgatcgaggccggggacctgcagatcgttcagcttttccagtgccagtgccactgccggcagttttaccgtggaggcgggatagaagtaggtatccggcgacacaccataataatagtctgtgaagtgaggccgctgctgcccgtcccggtctatgcgggtaaaaatcacctgtaaacggtaagtggaaggatcgctgaacacagcgcctaaccggcttttttgacttttcagcaaagcttccagaaaattatctgttgccggataatgttgggtttgcatatatttgtcgttgttatggattgtaaagcaaaggaatatatttaaaaagaccagaatccgggagctgcagatttaaaaaaagtgtgccaaccaacctgcaaaggcaagcgcatattgattttgcgtgtcttttaacaaggactttaatatatcgatttaaattctatctttgcaactcttaaaatttttttttataaacccgaaacaaacagtatgcaacttaaaggactggtaagattttttgccatcgcactgatccttatctctttgtaccaattgtccttcacgtttttggtgcggaactatgagaagaagatagagcagcaggccgagaacgatgtggccaagcaataccctacacctgaaaagaaatatccaggcagttcggaactgcagggcttctactcagataccctcaaagggtttattaaacagaggagacaagagattgtggacagtaccagcagcacaaaaattgcaggctttccatggaatgtcacctataccaaggccaaagagaaagaactgaatctcggtctggacctggtaggtggtatgaacgtagtactggaagtaagcgtggaagatgttatccgcgcattatccggtcaatccaaggatgctgcttttaacaaagcgctggaaagggcaaatgagctgaagaaaactaaccaggccgattttgttactttattcggacaagcatacgccgaggtagcaccacagggtaaactggcttctatttttgcaaatgcctaccagaaggacatcaccttcaattcctccaatcggcaggtgctggacatgatccgcaaggaatcacgtgttgccattaagaatacctatatcgtactgcaaaaacgtattgataaatttggtgtggcacaacctaatatcagcctggatgaaaataaaggactgatctccgtggaactcgccggtgttgataacgccgcccgtgtacacaaatacctgcaggcaactgccaacctggaattcagggaagtatacaagaactctccggagtttatccagaatgtattatccccggtgaacgatgctgtaagaaatgctaaggccgcagttaccgctgctcctgccgctacaccggattcagctgctgctgctaccaccgctgctgcgaaggataccggtaaagatgccagcctgacagattatctgtctaaaaaagataccagcaaaaatgccagcaaagaactgcagctgaaagaacaacaggcgcagaacccgctgttcatggtattattccctaacgtagacccacaatccggctcagtttatccgggtccgtctattggaaggattttaccaaaagataccgctactttcaaccgttacatggaactgccggctgtaaagtcgatcctgccgaaagacctggtatttgcgtttggtgctgaaaataaagaagataaacacggacctttagcggtatatgcgctgaaagtgaacccggccagccctgaaccccgtgttggtggcgcaagcatcgttgatgcccgtcaggacatggaccagaacaaccagccggaaatcagcatgaccatggataatgaaggcgcccaccagtggaaaaaactgaccggtgaactggctcctaccaatccaaaagatcccgctacctttaattatgtagcagtagtgctcgataacatcgtttactctgctccttctatacagggtgaaattgccggtggccgttcctctatcagtggtagctttaccattgaagaagcgaatgacctcgccaacatcctgaaatccggtaagatgccggctcctgcacaaattgtacaggaacagatcgtaggaccaaccctaggcgctgaatctattgccgccggtgcgaagtcctttatgatctccttcggaatcatcttcgtactcatgctggtgtactacaactcagccggctgggtagctaacattgcactggtactgaacctgctgtttacctttggtatcctggcttctatgggtgctacgttaacaatggccggtattgccggtatggtactcaccatcggtatggcggtagataccaacgtaatcatctttgaaaggatcaaggacgagctgacgcatggtaaatcttaccacgatgccgtggcggagggctacaaacgctcttatgcacctgtactcgatggtcacgttacctccttgctcaccgccttcatcctgttctacttcggtttaggtccggtactgggcttcgccaccacacagatcataggattgttcctgtccctgttctgcggtatcctggtttcccgtatggtaactgatttctggatgaagagaaaaagacattttgaatacttcacacctatttcccgtaaggtattcaaacatgccgcttttgatttcgtaggcaaacgtaaatatgcttatatcatctccgcctttgtaatggtggcaggtgtttcttccttcttccatggcttcgaccacggtatcgatttctccggcggccgcagctatactgttcgctttgagcacccgatgaaccgcgaagaagtggcagatgtgctgaagaaagaatttgactcagaagtattcgttaaaactatcggcagcaccaaccagctgagcatcactactgcttacaaaattgagcagcagagcctggcggtggataaagaagtggctgataagttatataatggcctgaagaagttctatgacgcttccgtaacgcctgacgtatttacctcccgttacattgtaggttcgcaaacagtatcgcctaccatttccgatgacctgcgtgcaggtgcggtgaaggcaacgatcctgtctattgtggtgatcttcctgtacatcctgttacgtttcagcaagtggcagtactctatcggtactatcttctctttgctgcacgacgtactggttacgctggcagtattctcctggtgcagatcctttgtaccgtttacactggaaattgaccagcattttattgctgcgatcctgacggtgattggtttctccatgaacgataccgtgattgtgtttgatcgtatccgtgagtacttcaggaccggcgctcatggccgcgacagggataccgtgatcaataaagcgatcaacgataccctgagccgtaccattatgacgtcgctgaccgtattcctgaccatcctgatcctgtttgtatttggtggtgaagttacccgtggtttcgctttcgcgatgctgattggtgtgatcaccggtacttactcttctatcttcgttgcggcaccggtactggttgacttcgacaagaagaatcagctggctaacgaaggtgagtcagtggaagtggtggccaagaaaacggctcctgctgccaaataactaagatctaactgaaataatgtttgataaataaaaacctcctggcttgccaggaggtttttttatgcagtatctttttgggagatatttatcagctggccggctgcctgaatacaaacccggcggcttcgcttccctgctggtagtctatttccatgcccatgaggtacatgccatgtgcttttttcatgatcacagggatgccggatatctcaaagaggtcgtcgtcttccatgcgggcatcgaagccgagcatataggcaacaccggaacaacctccgccttttacgcctacccgcaggtagggggcttctgtattcccctgtaacaattgtttcactacttcagcagcactggccgtaagttgaatgggagacctgttcacgttatccattatccgtatttttttcaaagttagagaaaaccaggggcggttttgcctgctggtatacccgaggtaagtggtgggtgtagttaacgcaaaaacgctttaaacacggcctaaaccgtggtcatgtacagctttgaggtggacttgaagcgcaattactttgctgtggccagttccaggaactttttatggaggtcgagtacctgcggaatcaccatatgctgctcatcgttatagatcacgtggtcgctgaggcgcattttaatggtttcgtcaatttgcttgtacatacgtgccagtacttcattgcgggttacgttgtcgcgtttcatgacgcggtgtacgcgcagtggctggggggcgaaaacggcgattacctgatcgaggtggtggaaggattctgtttcaaagaggagagcggcctctttcagtacgtagggagtgtgttgttgttgggcccagttgtcggaatcccgtatggtggccgggtgtacgagggagttgaggagagcgagtttgtctttgtcgttgaaaacgatatttccgaggagtttgcggtttaaggcgccgtgggcatcgtacatttcttcgccgaagtggtgttttacctgtgcagccagttcggggtcgcggaccataatatctttggcccggtcgtccgcgtagtatacgggaacgcccaataattcgaatattctactaacggtgcttttgccggagccaatgcctccggtgattccaatctttaacatagcccccaatttataaaaaaatacgaattacccatatgaattacggagttacgggcagatgccgtggaatagatccgcgaaaatcatctgcctgtaactccgtaaacagtaattactctgattcgtaatgcttatttagtttcagctgctttttgctgagcagtggtgtattccatgctgatagcagagcgttcgatagtgaagctggtgcctgggctaacttccatcagaacggtgttgttgtcgttcattttcttcactttaccgtggataccggcgatagtgacgattttatcaccttctttcaggttatcgataaattgtttctgcagttttgcttttttagtttgaggcctaatcatgaaaagccacataacgacaatcataccgccaaaaaacaggaaagaaacccaggagttaccaccgccttgggcaccgccctgaggcgccattaataaaatgttcaggatgttcatctctataattgatttaatagtttagtcggactatttggtaatgatattgcattggatcttaggtcctaccacataaccgtctttattgttgattttaacagaaatttctttctcggtatagcctgattttccgtggctgtcgaaaataaccttcatgtaaccggactgaccgggtttgatgggttcttttggccattccggtacggtacaaccgcagctggagatggcatcttcgatgagcagcgggctggtgcctgtattggtgaatttaaaggagtactctactttttcacctgctacaatttctccaaagttatgcaccttttcttcaaaggtgagtgcggaggattgaccagtttcgattttttgtccgttaccggctgcctcagcagcggtattattttttgcactattgttacaagccgccatcagcaggcttccacaggcgagtaaacagaacagttttttcatggcattgctattttacggtaaaaataacttttcccacttactttttcggacggtcctgtttctgtaccagctgttctttttccaggtctttcagaatgttatccaggataccgttgataaactggccgctctgaggtgtgctataggctttcgccaggtctatatattcgttgatagttactttggtaggaatggtggggaagtagagaaactcgcatacacccatttccatcagtaacatatctactgcagcgatacgttcagaatcccagttttgtaatttgggcttgatcagttcgaggcagtattcctttttgtcgattactgtgagcagaagttcctttgcataatccagtttttctttactgatcagctgcaggaaattgaagagatgcggcttattgaaataattattgatcagaatgcccatcatttcttcgtcgtcgccccagtggaggaaggtatcttccatgtgttgaaggaacggctcgcttttcgccagtatttctttatagatgaattccagtatttccttttcaccggctttagtgcggctaccttccgccgcgtaggctttgtaggtatctgtggctaccaattgattataaagctttctgagcagatcatcatctgtttgcagcttcattttccattggtccaggtttacctggaagcctttgtcgctggttatctggtaaataaactcatttcctgcaattttggtgttcacctgcaggtcctcggcagagggtaagtgtttggaagcacgggcgtgcgcatcaatttcggcgtattgtgctacctgtaccactgagttaagtaagtaggtaaagatctgacaggtttggtccagcttttcgtttaaaagtctggtggccgtgcctggcttaatactgctttgctccatcgtttccagggcataaagtgtttgcattacttttacccggatatttcttctactgatcatcttataaaaaagaactggtataagggcgcaaaagtagagaaaaatttccatattcgaagcggagtttgtcgcggagcttgccgcggaggttgtctttctcactgattcccctgattatactgattaattgtttttttgattttttttaatgatttttagaaagatgtatttatgcgccttattattcctggaaaaataccctggttggttaataataaatcaagagaatcagggcaaaagacaatcttcgcaaaaaaataatatccttttaatcagcataatcaggggaatcagtgagaaagacaaaatccgcgaaatccgcctagctgtcattttttcgggttgtttgtcatgatttgtcagtatggaagcaagtcgataccttcgtgacctgtaaatttgacccgaaaaccgccttggcacaattctcgtggacggaaggaacaatcacaaacatcttttttaaataaaaactactatggctaaacaattaagtattaaacctttagctgacagggtaatcgtgaaacctgcagcagcagaagagaagacagctggtggtatcattatccccgatactgcaaaagaaaaacctgtgagaggcaccgtggtggctgccggtcctggtaaaaaagatgaaccgatcactgtaaaggtaggtgatactgtactctatggtaaatactctggtcaggaactccctatcgaaggcgaagattacttaatcatgcgtgaatctgatatcctggcgatcgtttaagagctgtctgcgatatgaattaattcctaaaagaaaaatctcaaagtattatggcaaaacaaattttcttcaatatagacgcccgcaacaagatgaagaaaggcgttgacaccctggctgatgctgttaaagtaaccctgggccctaaaggccgtaacgtagtgatcgagaaaaaattcggcgctccgggtgtaactaaagatggtgttaccgttgcaaaagaaattgaactcgaagacgcaatcgaaaatatgggtgcgcagatggtgaaggaagtagcttccaaaactgctgacctggcaggtgatggtactactactgctaccgttctggcacaggctatcatcggcgacggtttgaaaaacgtagctgccggtgctaacccaatggatctgaaacgtggtatcgacaaagctgtgaaagcggttgttgaaaacctgaaaaaacagtccgaaaaagttggtaacgatacacagaagatcgagcaggttgcttccatctctgccaacaacgacagcgaaattggtaaactgattgcccaggcaatgcagaaagtaaccaaagacggtgttatcactgtagaagaagcaaaaggtaccgacactactgttgaagtagtagaaggtatgcagttcgaccgtggttacctgtctccttacttcattaccaacagcgaaaaaatgcaggctgaactggctaacccttatatcctgatctacgataaaaagatcagcactatgaaggatatcctgcacatcctggaaaaagttgctcagcagggcgctccgctggtaatcatttccgaagatctggaaggtgaagcactggctaccctggtggtaaacaaactgcgtggtaccctgaaagttgctgctgttaaagctcctggctttggcgacagaagaaaggatatgctgcaggatatcgctaccctcaccggtggtatcgttatcagcgaagaacaaggttacaaactggaaaatgctgacctgacttacctcggtaaagcagaatctatcactatcgataaagacaatactactgttgtaggtggtaaaggcgaaaaagaagcgatccagtcccgtatcggacagatcaaagcgcagatcgaagtaactacttctgactacgaccgcgaaaaattacaggaacgcctggctaaattaagtggtggtgtggctgtactgtacgttggtgctgctactgaagtagaaatgaaagaaaagaaagatcgcgtagacgacgcattacacgctacccgcgctgccgttgaagaaggtatcgttcctggtggtggtgttgcttacatccgcgctatcgaagccctggattcactgaaaggtgctaacaacgacgagcagaccggtattgccatcgttaaacgtgctatcgaagaaccattacgtcagatcactgccaacgcaggtatcgaaggttctatcgtagtacagaaagtgaaagaaggtaaagctgatttcggtttcaacgcccgtacagaagttttcgaaaacttactggctgccggtgttatcgatccaactaaagttacccgtattgcactggaaaacgctgcgtctatcgcttctatgttgctgactaccgaatgtgtaatcgcagacaaaccggaacctaaatctgctgctcctgctatgggcggtggtggccacggtatgggcatggactactaatatcaagaataatcataaaaactcctgcaggcaaggtcttgcaggagtttttttatgcggatcacctttccgctgtaactttatcataagatttccgtttaataacgagatagtaaacagcagcggatgaatacagttgtaaaaataatttgcgcaagcctgcttttgatactgggcgcctgttcaaagaacagcagctcggaggaactcaggatgggtggagtcacagaaaatgccatccagcagtacctgcacgagcataatgaaaccgcgatccgggacgtttcgggactttattaccgggtagacgctccgggagacagtacccatttcgtgaaagcaacctccatccccaccgttatttataccaattatttaattacgggcgaagtagtaggtacctccgtagggcccaccgatttcgatcacaggatgcttaaaaaccacattcctggctggcagataggattgcagaagatttcacagggaggaaagatcaggttgtatatcccatccgccctcgcctatggctctgtgggcgttaacggtgttatcccgcccaacgccatccttatttctgacctggaactggtaagtatccggtagatgtattatcttataccaattgtattttcaccttttaattatactaaaactgaaaccgtaactgtatgaagaaagtttttctgttgggaggattattcctgttagtgcttgccgcctgttcaaaaaaagatgatgcacctgcctataacgctattgcacaatatgatgctgactccgcaaaaattgtagcgtatatcgccgccaataatctcaccaatgtgcaacatgatccccgtggccttttttaccagattataacaaaaggaaccggcgattctgttaatgccgctgcaaatgtatgggtatcctacaaaggccagttgctggataaaacggtttttgacagcagcgacagcgccaggtttgaccttgataaagtgatcaccggatggacgatcggtattcctaaaatccggaagggtggagaaatcaacctgattattccttctatttatgcttacggcccgactgcctattctaaaatcccggcgaattcagtactggtattcaacgtgaagctgaaagattatgtgaataaataatggagaaagaaataacgtgaagcggtaccggttctgccggtaccgcttttgcatttgtattattcccccgctttccgttaattttacagataaataaaaaattagtggcacacgaatgtatttccgtatttgacatttttaagataggcgttggcccttccagttcccatactttaggcccgtggcgcgcagcattgcgtttcctggatcagttggagcaggctggcaaactggcggccgttaataaagtacaggtattattatatggctctcttgccaaaacaggtcacgggcatggcaccgacattgcggtacagctgggcctctgcggggatgatccggtaacttttgacgtgaaccagatcaatcctaaaatggatgatatccgccgcagccgccggatgaagatagcgggtaagtatgaaatagattttgatcccgttgaagatattgacttcctctttgaagaatccctgccgtttcaccccaatgcccttactttcctggttaccctgatggatggtgaacagctggcttccacctggtattccattggtggcggttttgtagtgcaggagggggatgcaggcggtggcgcccagcaggtggatctgcccttcccgatagatactgcccgccagctgctgcagtggtgcattaaaaccgggtacagcatttctgaactggtgatggaaaatgaacacgcctggcgttcggaagaacaaacccggcaagggctgttgaacatctggcgcgtgatgcaggaatgtaccttccgtggttgtcataccggtggggagttacccggcggactgaaagttggccgccgtgcggcagtactcaacaaaaaattattaaagggccgtacctatactgactatgcctcctggattgacgccatccgggcgggtggagagcatttcagctatacgctcgactgggttagctgttttgcgctggccgtaaacgaagaaaatgcatcgttcggaagagtagtaacggcgcctaccaatggcgctgcaggcgttattccggcagttttacaatatttcattgctttctgtgatggtttccaggaagaaaagatccagcagttcctgcttacggcttctgaaataggcagcatctttaaaaagcgctccaccatttcggcagccatgggcggatgccaggcagagataggtgtatcttctgccatggcggcggcagcgcttaccgagtgtatgggaggttcccagcgccaggtactgatggcggcggagatagcgatggaacatcacctgggcctcacctgcgatcctattggcggattggtacagataccttgtatagaacggaatacaatgggcgccatcaaagcaattacggcatctcaactggcgctgcaaagcaatcctgagctggcaaaggtttcccttgacgcggtagtaaaaaccatgtgggaaacagcacaggatatgaattcaaaatataaggaaacttccgacggaggactggctgtaaatattcctatcagcctgccggagtgttaaaagataccaggtaacgaattacagatttaaaagcagattacggcgaatatcggttataatataaggaaagaaccatattttcgtttatacgttatcatcatctgcttagatccgtaattcgttattttttatgcgtgttatccttgccattactcttctttccttttccctttctttatcggcgcagcaattcggaggtaatccgccttcgctgaaatggcaacagatcaacacagatacggtgcgggtgattttccctcatggtatgaccgggcagggtgagcgggtcgccaacctggttcactatcttaaccgttatacccggtcttctattggcagtcttcaaaaaaaagtaagtattgtattgcagaatcaaacgctgcaatctaacggatatgtacaactcggcccttttcgctctgaattttacctgacaccacctcctaactcgctcgacctgggctctcttaactgggtagaccagctggctgtgcacgagtaccggcacgtattgcagaacatgaacttccggcagggggtatccaaagtgttttctattcttggcgggcagctggggcaagcagcggtaaccaatatcgcagtacccaactggttctgggaaggtgatgccgtggtaatggaaactgcgttaacgccgcagggcaggggacggctcccgggtttctttgacggcttccgtggcctttcgctggcgggtaaacattacgcctatatgaaaatccgtaatggttcctatgtagattatgtaccggatcattacccgctgggatatatgatgaccagttatggccgggagcattacggacacacgttctggagagacgttaccagtgacgccgttcgtttccgcggtgtgttttacccattgtcgcacagcctgaagaagagaacaggtatgaatgtaaccggcttttataatgccgtgctgaaagaataccagccgctctggaataattatgccgcccggccggataccacgccggcgcagcctttgctgccggttgccaaaccagttaccaactataactatgtatacagtgcaggtaataatgaatgggtgatattaaagaatgcctggaataaagtgcccggtatttaccggttgaatgcttccggtgaagaacgtttgctggtgcgtcccggtattttatacgatgactttttcagttaccgcaatggccgcgtggtatgggctgctgcccgtttcgatgcgcggtggggctggaaggatttttccgtgatccgggtgtgggataacgctaccgggcatacgaaaactgtttctccgaaggggaaattcttctccccggatatcagtgaaaatggagaaaaggtaatagcagtggctaccaccactgaaatgaaatacagcctgcagttgatcaatgcgcgtacagcattggtggagaagcagttgcccaacccggaaaactggtattatacctatccgcgttttgctgccggtgaacaggctgtgatcagtgcggtaagaaataataagggagagatggcgttggttgagcagtcgctcgctacgggcgaaagcaccatgcttacgcctttcagttatactgtaatgggtataccggttgtgagcggggatacggtttatttcaccagtggcctgaaagatgtgaacaacgtatatgcgattacgttggcagatagaaaaacgtatgaagtcaccgacagggggaacagtgcgctgcatatggcagtagatccggcaggcgacagtctcgttttcagtgaattcaccgtgaaaggatacaagctgtatcacgctgcgttgaacaaagccgcctgggaacccgccgacgtaagtaaagacgggcgcagcgcctggctgcagcctcattttaaagaaggtggtaatatcctggagctggcgccgcatgattccctgccggtgaagaagtatccgcagttcacccgtccatttaacttccacagctgggtaccatcttttaatgacccggattacagtatttcactgatcggtgaaaatatattgagcactacgtctaccagtatcggctatacgtacaaccggaatgagggcagctcggatttcgcggcaggctttactttcgggggctggttcccggtattatcagtaggagccgactataccattaaccgtaatggactggatcagaaccggcagcgggtatactggaatgaggccactgcgcatgtgggcttcagtatcccgttgaacctgtcgtcgggactttacagccgcagtgtatctttcggtagtaattacaatatccgtcaccgttacctggacagcaagtacaagggaaacgatctgcagttcctgaccaacaccatcatctttaacaaccagcggatcaaggcagtacaaaacatttacacacatttcgggcagtatctcgcggtgcagtataacagttctgtgtcgggcttgtatgccgaacagctgtatgcgcggctggatcagtatttgccgggattatggcagaatcataacctggtattgcaggccgcttatcagcaacgcgataatgcgttcaattatactttcacggataatttcgtatatgcgagagggtataatacgccgtcgtatacgcatatttataagctgggagcaaactatcatctgccattggtatatcccgactggggctttgcgcagatcctgtatttcaaccgtatccgggctaatttgttttacgattacagcatggctaatttttcccgtaacaatgtggatatcaatacccgttatacttccgccggtaccgagttattctttgacacgcgcataggtaatgcactgccttttacgtttggcgtgcgtttcagtcacctgtttgaccaggaccccgtagacaatgcgcggaaccggtttgattttattataccgatccagcagttgtttaattattaagaagatggattatttaacgttgatctgaagggaaggagctttgtagaatttttcttctgcatatttgatgatgatgtcgtcgaagtacaagacatcaccggtttgcagggtttccttcaggtttttgctccacgcggcggggagggaagctgctttgaaattatctcctgtaaaatctttgtatatagcgggttgcccggtagtatcgttcagataaggctcatgtttttcaaaagtaaaagcaaatgagagcaccgggtatttgatattcttttcgtcccgcacaattaacgcggagtccagtaatttaatgacttcactttttggtagcgtgtcgctcaggtagatgccccagctgctgcggagtttcatgggtcttttgctggttacggcagtcgccggtttttttgcggattgtgcaatgaccggtgtaacagcagtggctaataagaaactaagtaacagatgtttttgcatgatagtaccgggatataaaaaaatcgcccggtatagtaacgaccgggcgatcctaaaaattataaggactttaaactttcctctatgactgcaatttttgcttcggcatctgctttcttctgacgttctgcgtctacggcttctgcttttgcgttttgtacgaagcgctcattgctgagtttcttttcaacagataccaggaatcctttcaggtattcgaggtcttttgtgagcgctgctttttgtgcggtggtatccagtgcagtttctgtaccgaggtagaatttatctttctggatcacgagggtaatgcagcctggcacgggttcctgtacatagtgaatggcttttgcgttcacctgtttggcgagcatgccttcaatttgtttgaatgcgttatcgtgtttggtttctatgtgcagtacgatcggatcttttggttttatctgatgtttgttacgtgcatcgcggatgctgctgatcacttcttttgccagcgaaccttccagcagggtagcgtgtaccggtgcctgtggggtgataaactgttttatcatcagggaatcatccgctgcacgtgccgtgagttgctggtatatttcttctgtaataaaaggcatatacgggtgcagcagttgcatcagttgttcgaagaagtaaactgttttatggtagatggaagcagggatcggttgttcgaaacccggttttgcccattcgaggtaccagctgcagaaatcgtcccataccaggctgtagatggctttgaggccttcgctgaggcggaagtccttatgcagggcggctacttccagttgtacttcattcagcctgctttcaaaccatttcacggcgaagttatctgctgcggcgttggtggcgctgtcatcttcctggcgttgttcccacattttcaccagtttaagggcattccatattttattacagaagttacggccctgttcacagctggagtcatcgtacaggagatcgttaccagcgggtgaagaaatcatgataccaaagcgaacggcatcggcgccaaaggcatggatgagttccagcagatcgggggagttgcccagttgcttactcattttacggccttgtttgtcgcgtaccattccggtgaagtatacgtcgctgaagggtttcacttctttgaactccagtccggccatgatcatacgggctacccagaagaagatgatatcctgtccggttaccaataccgaagtagggtaatagtaattgatatcctcgttatccggttgggagatgccgttgaatacttccatgggccagagccaggagctgaaccaggtatccaggcaatcctggtcctgtgtgagttcggctgctttgacggtgatactgcgggcggcaaactgctgcactgcttcagcagcggtggcggctacctcaaaggaaccgtccggcgcgtaccaggcagggatttgctgtccccaccagagttggcgggagatgcaccagtccttaacattttccatccagtatttgtaagtcgccaggaaccggtcgccgggatggatttttacatcaccgttcactaccgcgtccagggcgggtttggccatttctgccattttcacaaaccactgggtggagatgcggggttccactaccgtatcggggttacgctgactgtaaccgaggcgggtggtatattcctgctcttttacgagcaggccttcttctgcgagggcggctactacttttttacgggcaacgaagcggtcttctcctacaaaaacaacggcggcggcgctgagtgtgccatcgtcgttgagggtatcaatgatttcgaggttatgtttcaggcccaggttataatcgttgatatcgtgtgcgggcgttactttcagggcgccggtaccgaattctttatctacgtaggtatcaaatattaccggaacacgacggttgaccagtggtacggtagcaaagtgacctttcaggtgggcgtatctttcatcttccgggtttacgcagatggcggtatcgcccatgatggtttccgggcgctgtgtggcgatggtgatatattcgccggttggcgtgccggtggcgtccgtgatggcgtatttcacatgatagagcttaccctggaggtctttgtattcaacttcctcgtcgctcagtgctgttttagcttttggatcccagttgatcatgcgggcgccgcgatagatcactccttttttatagaggtcaatgaaaacggtgatcactgctttgtagtagtggtcgtccattgtaaaggttacgcgatcccagtcgcagctgcagccgagtttttttatctggtggtagatgatatctccatatttatctttccattcgaatgcatatttgagaaattcttcgcgggtgagctgggatttttcgatgcctttctcctgtttgagcatatttaccacttttgcttccgtggcgatggaggcgtggtcggagcctggaacccagcaggcgttgaagccgctcatacgagcccggcgtaccaggatatcctgtacggtttcgttgagggtatggccaagatggaggaccccagtgacgtttggaggggggatgacgacagtaaagggttggcggccatccggtttagagcggaagtagcctttatccatccattgttggtaccatttttcttcaaccgttgcaggcaggtaatttttcgaaagttccatgctattcataatataaggttgcaaaaataacggagattaaggagagatggaaatttaaagggcagtaatagttgccctttccgttatgccatctctgcgatgatttcgcaggtttgtgcaatcatttccggtgtaacatcgaggtgggtgactattcttacctgcgttggtgagatggccattacgaggataccctgttttttgaggtaatcggcgaagagctgcggagtccagtcgcctgttacttcaaagatgaggatattggtttccacggggagcatgtggccggtgaaggatttttccagcagggcctgcgccagttgtttggcgtggtggtggtcttctgccagccgggcgatattattttccatggcatagatgccggtagctgccataaatccggcttgccggaggccgccgccgagttttttgcggatacgcctggcggctttgataaatgtttcgctgccgagcagtacggagcccatggggcatcccattcctttattaagacaaacggaaatgctgtcgaatagttgaccgtatgtttttgggtcctggccggtggccacgagtgcgttgaagaggcgggcgccgtcgaggtgcagtgcgaggccatgttttttacacacgtcgcctattttcaccatctcttcccagtcgtagcagcatccgccgccgcggttggaggtgttttcgaggcaaacgaggctggtgcgggctttatgcacatcgtcggggttgatggctgcttccacctgggtagcgcggatcatgccacggtcgccgatgagggcatgtacctgggcgccggagttgaaggcgatgccgcctccttcataaatatatacgtgagcaagattactgcaaaccacttcatccccgggcaacgtatgtactttaatggcgacctggttactcatagtgccggaagggcagtacaaggctgccggtttgccaaaatattctgccatcatggcttccagtttgttgatgctgggatcttcaccgaaaacgtcatcaccggtttctgcctgcagcatagcctgtaacatgccagggccgggacgtgtaaaagtgtcgcttctaaagtcaatcattttattgaaaaatttgcaacggcttaacgaataaattagttaagatgttaatttaaatatgattctttatcaattgttaaaatttgtataaaccaacgctgtacagggactaaagcactataaaattccgttataaaactgtactttgttatatggctggcaaatataagaaggatttggtagagtggttggttagcacgatctttgcagacttattttgaaacaaaacaataaagcgcgggaaactttgtaagttaataattttaaaagtttcgaacaaaaaatttctttcgctgttatttatttataaaccaatacaatttttcatatgaggcaacttaaaattgccacccagatcaccaatcgtgattcgcaggcggtagaaaagtacctgcaggaaatctcgaagatccctttgttaacacctgaggaagagaccgttttggcgcaacgcattaaaatgggcgatcaaaaggctcttgaaagattgactacaggaaacttacgtttcgttgtttctgttgcgaagcagtatcagcaccagggccttagcctgagtgacctgattaatgaaggtaatctcggcttgatcaaggcggcacaacgtttcgatgaaacgaaaggtttcaaattcatctcttatgcagtatggtggattcgccaatccattctgcaggcgctggctgaacagggtcgtcttgttcgtcttccgcaaaacaaaattggcacctataataaagctaacaaagcttacatggcatttgagcaggaaaacgagcgtgagccttctaccgaggagctcgcagaaatcctggagatgtctgaatcagaaattaacaatatcttccaaagcaacacccgtcacatgtctctggatgcacccgtgcacgaagcagaagacgtagcaatgggcgacctgctggaaggtggagatattactgatgacgacgtgatgagagattcactccgcgaggaaatacgccgggtattaaaatccctgagcccacgcgaagctgaaattgtgaatgcttattttggtctggatggtgaaaatggcgcaacaatcgaacaaatcggtcagaaatacgatctgactaaagaaagaatcaggcagattaaagaacgtgctatcaaaaggctgcagaaagcccgctatagtggcgccctgaaatcatacctgggataaaatacctttattcattagttagttaacattaacgaaaggataaatctactaatcctctttattctataagaacaccggccttgtaaatacatggccggtgttcttatttagtgaacaccccttatttttgcactcatgcgtatgccgcttttcttactcctggttatactgatctttgccgcctgcgagaaagatatcagcgttaacctgccacaacaggaaccacaactggtggtggaaggcagatttgaaagcggctcctacccgttggtaattctcacacacagccttaactatttttcacagatagatccggcagtattaacgaatgcatttgttcataacgccactgtcaccgtttccaatggcagcaaaaccatgacactaaaggagcggacaatagataccggcaacatgaagttctttgtatacctgccggatcttacgcagcctgcaaacaacttcaccggaaatgtgccgggcacctatactttacgtattaacgctgacaataaggcatatgaatctgtgacaactataccgcagcgcggcatgaaactggactcggtctggtggacattagtgacggtggacgactccacgaaagcccgcctttgggtgaagatcacggatgctcctgcgtttgggaactatgcaaggtactttaccaggcgaaacagtgagccctatttacccggactgaattctgtgctggatgaccagctggtgaacggcacaacatttgaaattcctgtggacgccggcgttaataagaacctggatcctgatgacaggcccgatgagttctttgaaccgggggatactgttaccctgaagttttgtaatattgacaaagcaacctgggatttctggcgaacgcttgattttgcctatagcagtaatggcaatccattttcatcgcccacgaagatacttggaaatgtacccggcgcattaggctactggggcgggtatacagtaacctataaaacaattattattagcaggtaattatacatacagcaaacaaaatggaaaacaagcaacaagagcatgtacacttattgatcatcggttccggccctgccggttataccgctgcaatttatgctgcaagagccaaccttaaaccagtattataccagggcattcagcccggcggacaattaaccatcaccactgaagttgaaaactatcctggttatccggaaggtattcaaggacccgaaatgatggtggattttgaaaaacaggcagcccgcatgggtgccgacatccgttatggtttggctacttccgtggatttcagtaaacaaccttataaagtaacgatcgacgaagagaaggaaatcactgccgatgcgatcattatcgccaccggcgcctctgccaaatggctggggcttccttccgagcaacgtttgaacggcagcggcgtaagcgcctgcgctgtttgcgacggattcttcttccgtggtaaagaagtggctattgtaggcgccggtgataccgctgctgaagaagcgctttatctttctaaaatgtgcagtacagtgcatatgctggtgcgccgtcatgaaatgcgcgcttccaaagtaatgcaggaccgcgtactgaaaacttccaatatcattgtatactggaattctgaaacagacgaagtactgggagataagaaagtagaaggactgcgcatcctgaataacaaaaccggcgaaaagaaagaaataccggtaagcgcattcttcgtagctattggtcaccagccaaactccggtatcttcaaagactacctgacactggacgaccaggaatatattgttacagaaccaggcaccagccgtaccagcgtggaaggggtgtttgcctgcggtgatgtacaggataaaatttaccgccaggcggtaactgccgccggcagcggatgtatggccgccctggatgcagaaagatatttatcagcaaaagaacaccaccaataataaacaggataatgaataatggatttacagggagaacattcctgtaaatccgttatttgttgtccgtaatttccgcttatgcttaccatcgccctcgaacaggctactttctacgcttaccacggcttgtacccggaagaaaccatcatcggtaatcattttgtactggatgtggcagttcgtatacccggcaccgtgcccgtagatgatttgtctgaaacggttaactaccagggcatctatgaaatagcaaaggccgtgatggccgttccacggccattactggaagaagtggtgtatgaattaaccgatgcactcaagcagcggtatcccggtatccagcacagcaccgttaccctccgcaaaatgaatccgcccatgggcgctactgtccgcaactccctggtttccctggagaaggattactagttactattttttgggatatatatgatgtttccgtaaatttatagctataagtcaatcaacaaattcttacgctgtaaaaacctgtcctatgttgaaacggatcatggcagtttgctttttattatcagcggtactgtttgtacaggcccagagtgtcagtgaaatggtagaagaagccaggcagctggagaaacagatgaaagaaagcgaagcatttgaaaaagataaggacatcctcaaaatacaaccgtcggaactggacgcattgaaccaggccagccagttatgttcccgcattggcaaccggcagaaaagcaaagacgataagatcagttattttaatctcgctaaaagctatgccgagcaagcgcttaaggtaaatcccaatagtcccgaatccaatttatcgatggctattgcaatgggacgtatggcgctgatctccggtgcaaaagataaagtagccgcctccaaagaagtaaagaaatatgcggaactgtcggttaagtttaacccttcactggcgcagggctatcacgttttaggtaaatggaattatgaagtagccaacctgaatgcctttgaaagaggcgcagcaaaaatgctttttggcggattgccggatggctcactggccaacgccattagcaactatgaaaagtgccggcagctggaccccgcttttatcctcaactattatgaactggcccgcgcctataaagcagatgaccagcaggaaaaagccattgaagtgctgaagaaagcgctgaccctgcgcaatatcacccaggatgatgccgggatcaaagcggattgcaggaaaatgctggatgatttgcagtaagcgaaggttgtctttcccaggattaacggtgattttattgatttcgttgattgatgttgttatgatttttagattatagaagcgacttttagatttcttttcctttccatttgccactgcgcagataccagtaacttattccgaagataatgatccagtaaataaagtctgctccccaggcccagtgcagctcgctgcgcattctttcaattacaatattgcagtacaccaggtagccgataacggcgataatttccgttacgagattaattcttgtattgccggtacccaccacgccgctcattaccaccgctgctatcgccatcaggatggtgcttagcgtgataatccggatggaagggatggccatggtgatcaggtcggcgctattggtataaatgtgcagcaacgtataggggaagaggttaaccaccacgcacatggcaatagcgcatcctgcgctgagcgccacaattttccggatgatggggaaaacctgttccggccgtccctgcccaatgatgttgcttaccattgtattacaggccgccgccagcgcccaggtgaagatgccaaagaagccaaaaatactgcggagcatattggatacagcgagcgggcgttcgcccaggtgctcgatgaaaataaagaatacgaaccatccgccaatgctgaaaaggaactgcacaatcagtggtgcggatacattgaggatgttgcggacaatgctccagttgagccgcaaatagctgaacaggctgtattgcaggtgataacgcttcccgaagaggatgctgaaagcgaccccgcaaccggtaacttccgcaatcacggaggccgtggcggcgccgttgagccccatcgccgggaatcccagtttaccgaagatgagcgtataatcgaagaaaatgttcatcatttcctggaaaagcgaggtaaccgccagcaccctcgagtggccgctgccgatataaaatgcattggccatattcagcagcatgagaaaaggaaggccccatatacggatacggataaacgaaacggctgcagcgatgatatggtgatcgtgcaggcttttggaaaagaaccagggcgccgccaggagggtgagtaaaatagcgattccagagaaaaagagtccaacctgtatgccattggagaacagttgcccgatgccggaaaactgctgctggcccgctctgcgggcaatgagtacctgcatgccgttgttaaggccataggcaatcatgtacatcaccaggtagtagataccggcgatcccgttggccgccagttcaaattcgcccaggcgccctacgaaggcggtattagtgatgtgattaatctgcggaataatgagcgccaggcagatgggtcctgctattttgataatttgccgggtggtgacttccagttgcatggatctttagccgattatgggtatagcaacaaagatatggctatctgttgatcatctcccttatataaaacaacaaaacgccctcaccaattaactaaaaagagtattattgtaattcatttgaaaggttaaatatgcccgtggcttataacatccatcctgcatttacagtagacgatgaaatcctgctggaaactgatctcactgcctgtaatttactggtactggtaggaagcggaacattcagctatgtagtgtttgatccggttgcaaagaaattcctggcgttgaagtcctatcattttaccccccggaagctggccctggccgatctggagatgatagaacaggtgtttgataccgacaaactgttgtttactgcctttaaatctattttgctggcttttaataccggcggaggtgtgctggtaccgcatacgtactattcgccctcgctgaagaaggattttctgcacctgggcgcgccggagaaaatacaggaagccatcctgtcggatttgctgccggccctgccaatggtaaatgtttacagcgtggataaagacctgcttgggtttttacgcaaggagttttctacagacctggtgatacatgcccattcggccctgttgcaatcttacccgacggacctggatttccaggcaaaggacggcgtggcttttatcgaggtggatcagcaccgctttacgatgactgtttatgccggcggtaagctcctgattcaacaggaaagcgattaccaaaccgggttggatgtggtgtatagtctggtgaacgtgcttcgtcagctggagctgaatgagcagctggtgaaagtaaagctgggaggagtggtggctacggatgccggcgtataccaggagatgtataagtttataccacacctggaatggatacaacgaatcccgggtttcagttacattacaaaaatgcaggaaatcccgggctattattttcataacttatatgcgttagcgttatgcgtataatcggaggaacgagtgggggacgaaagatacaaccgcctgcaaaaatgccgcatacccggccaactacagatattgcaaaaggcggattgtttaatattatcgaaaacaacctggatattccatctttaaaaacactggatatttttggcggcaccggcagtatcagctttgagctggcttccaggggagccactgatatgactgtggtggagaaagacccggcaatggctgcttttatcagtaaaacagctttgtcgttggggattgaaaacctgaaaacggtaaaaatggacgttttcaaatacctgcagcaatgcacggagaaatttgatttcatttttgctgatccgccgtatatgatggcaacactggatcagttaccgggactgatatttgaaaaggagttactgaacccggaaggctggctggtggtggaacatacccagcataagaagttccaggattattcctggtaccgttctgaaaggaactatggcgcaacggtgttctccatttttattaaccgggaggaattaaaacgctgaccgtttatctatcaatcaatcgcacccttatgagaacttgtttattcccaggtacatttgaccctataacgctgggacatacggacgtcattaaccgtgggcttgatctgtttgaccgcctcgtgatcgggatcggggtaaacagcagtaaaacccctatgtttgcactggaagagcggatgagctggatcagggagatctataaagatgatccgcgggtggaagtggcttcgtattcgggactcaccatcgacttctgtaagcaactggacgcccgttttattttgcgcggtatccgttacgtaagtgattttgaatatgaaaaggcgatcgctgatgtaaaccgtactgtggcgccgggtattgaaacgatctttttaacgactgttccgcagtactccagtattgcatctaccctggtgagggatatttataaatacggtggagatgtgtcgccttttctgccggccgctgtgctggaaggcatcaaacgcacgaagaaataattttataaagcagataatatgaaaacgatctggcataatactaagatctcactggaccagttgaacgagatgggtggcactaccatggctacctgtttagggatggagtttacggaaataggtccggattatcttaaaatgatgatgccggtagatcacagaaccatacaaccctatgggttactgcatggcggcgcatctgcggcgctggcagaaacggtaggcagtatggcgtccggattgatcatagacccggagaagcagatctgtgtgggcatggaaatcaatgccaaccatataagaggagtgaaagaaggttatgtgcatgcctgcgcccggcccttgcatatcgggagcaccagccatgtatgggacatccgtattaccgacgatcatcacaagctggtatgcgtaagccgccttacggtggcgatactggcaaaaagatagttccgcttaaccgggatgcggaactaaacgttatcagatattcgcagccctgaatacttccctgatattttcgtaggagtatttcaggtatttttccacgttgccaggtttgatccattgcaggtcctggatgtcttcttctatttgtggtaccgttaattctgtgccggtaaacaacatccggtaccagtaggtatgttttaatacttttttatttttcatgggatagtagtgaaacgtttctgtgattttatgttccagtgaaacgttgtgcaggccggtttcttccgctacttcccgtagcgcgcaggtttcgaggtcttcccccgggtcctgtttgcctttaggcaggtcccatttgccgcggcggaacatcatgagcacttcaccgtcgggattggtgattaatcccccggcagctacgagggtagtaaaatgcagcgatactttcttgaaaagttgttttacatccggtgcaataaacactgctgcgtcttttttcccatcttccagtttctgcaatacattttccatcttttttgtatccgggttatcgtatactttggcgccgttaaagtgggccgggatggtagtggtatcggcactcagcaggagtggacgctcgttgagatagatcgtaatatttgcttgcatgccgcaaatgtaattatcaattatgaaatacaaattgagaatttaggaagatggaaacctattcccggcgctctctgcaaattcgtttattgtaattcgtaaattgaataaaatgatagtacttttggcggttgtatgaataaagtaagcgaaaaacaagttgcagaaaagttactgcaggtgcaggccgtgaagttaagccctgcacagccttttacatgggcttccggctggaaatcgccgatctattgcgataacaggaagatcttatctttcccttatgtgcgtgactatattaaatcagagttgtgcaacctggtgtttgaaaccttccctgatgcagccgtgattgcgggagtggctactgctggtattccacatggcgcgctggtagcggatcagctgaagctgccgtttatttatgtaagatccaagccgaaagagcatggtatggggaaccagattgaaggggtattgcaacccggacagccggtggtggtgattgaagacctgatttctacgggcaaaagcagcctggaagccgtgcaggccattcgtgcagctggtggggaagtgatcgggatggtatctatcttcaactatggttttgatatagcagtgaaagcttttgaagcagcgggtgtgccgttttattcattgagcaattattccgctatgattgccctggccgaggaaaaaggcattgtatctgctgacgaaatagctacgctgcaggcctggagaagtgcgccggaccagtggggtaagtagctgaaaattgtatatcacttattttgtatattcgggtattaatattacaactatgcgtatcctaaaattagtagtgttgttcctgtttgccggcgttggcgtggcaatggcacagcaaaagcagaaagctgtggaaacagcgaagatcagcacgccaaccgtgcagtgtgagtcgtgcaaaaaccgtattgagcggtatatgtcacatgaagagggcgtacaatccgtaaaagtggatttcaaaaaacatattacaacggtgaagtactataccgaccgtaccaacattgagaatatcaaaacgggtattgccaatgcggggtatgatgctgataacgtaacagcgaacccggaatcttacgccaaattgcctacctgctgcaagaagccggaagatggcggtggtatggacccgaaaaaacattaatcaacctgtttcagcctttggtgtccggcgattgccggtttactgaaggctgagttgttttttggcgtgggctttctgtcagccgtatccgcgttaccctgaaatgctccatcctttaaagcttaccgttattccgatactgtttaatccgctgaagcatcatttttctgcattccagcaaacgctttccaatctgatcctgctgaaataaatatgcgcctgctttccctgggaggttcacagcttacggctgtttccgctcagaagcactgctgaaaacgggcatattctggaaattattgccttattggaaccccgtttatagccgggttaaaagaaattcagcgcttgtttggtttcgcattttatcgggaaaggaagaaaaatacccgccttgcctactttacaatttccggtggctttgatggttacttctttattggcgaaagcgcttaatgcatttttgaatacgttggccatgttcacttccaatttcacggggaagtaaaaagtgtcccttgccggaatagaaatggtggtatcctggagggagtgacctacctgggtgtcatcaaaaaacaggtcgaagttggcatcttttagctggaggcgatagttgttcggattgtaatatgccagggtcatccgtacaatacttttggacatacctagctcatccatactgataccggctactctcacaaattgaatatccttgtttttttcgcaggagcttgctactccccagatcagaaaaacagcggctaataatcggaacactttcatcagttgaccaggtattttagtttatgtaaacctactgcaaagcttttagttatcaaaaaatcgggtgggatttgggaaacttttaacggggtaggttttaaaaacgggggaggctgcttagataattaatgcataaaacacatataaataaaaggttgttttaaagaaatatgctatcttcgtgatccttcctgagttcgctaaaattgaacaaaaaagccactaatttctttagtatttttgcgtttcggtaatcatttgctgaaagtaggttgtgctaatttatttagcatatgattaataattctatgaattgtttatcatttacttaaagttaattgttaagtatttaggtataagtgattgtcaggtgaaacgaacggaattccaacacctgcatacaaaattttgacattatgacagagaatgcaaaagagaaggtattgttaattgaatctcaatattttccgccaattgattcatataagactttaataaagcatgacatattaaagattgagaaatatgagcactatcaaaagctcagttacaggaaccgttgttatgttgccgggccaaatggccggatgattttaagtgtgccgttggcgcgggggaagaatcagcggaccgtgatgaaggacgtaaggatcagtaatgaggagaaatggcagggtttgcattggaaaacgctggtgtctgcttacaggcggtcgccctggtttgaatattacgaggcggacctgcaggttttatttgaaaagccttttcaatttttaatggattggaacctggcatgttttgaatgggtgaatagcaagctcggcattgaggtgcccattacctataccgaaagttatgaaaaggaagtgcccggtgtaacggatgcgcgcgaaagcatactgccgggcccggttacagaaagcgagcccggctatacacaggtgttccaggagcgtaccggcttcatacccggactgagtatcctggaccttcttttttgtgagggaaagcaatcattgaagattctgaaaaagggctgaatggaatagcaaataatattatttaacttgttggcttgtaattgtttgtatatttgcccgggtatttgggcttttccgaggaatacctcccgaaaaaaattaaggtggcaatcaacaaaatctttagatttgcaacctattttgctggggttcgaactgacgtaggtgtgtaaaccaggagtttcccagtgagggaaaaaaggattgttatcctgttatttttttctattactaattcctaaaattcatttgcagtactaaatgaacaacacctacacagacctggtaaaacagacctttgaatttccccaggagggctttgaagtaaaagataactacctggaatttaatggtttggatataaaggcattgatagacaaatatggaacaccctttaaactgaccttcctgcctaaaatcgggatgcagattaataaggcgaagaaaatgttccatgacgccattaagaagaacaggtacgaaggtgagtatttttactgctattgtactaaaagttcgcatttctcctttattatggaggagaccctgaagcatggggtacatattgaaacttcttttgcatatgatattgatatcgtcaataaattatatgagcgcaagaagataaataaggagacctatgtgatttgtaatggttttaagaccaaagcatataccagggccatagcgcgactgatcaacagcgggtttaaaaatgtgctgccaatcctggataataaggaagagctggaagattataagcggaatatcaggagtaaggataaggtgaaactgggattgagggtagcagcagaagaggagccaagtttcgacttttatacctcccggctgggcattcctccgcgtgatatccttgaatattatgtagataaaataaaaggtaatgagaagtttgagctgaaaatgctgcacttcttcatgaataaagggattaaagacgatatttattactggagccagtttaaccgtgtaataaatctctattgccagctgaagaagatctgccctgaactggacagtatcaatattggaggcggattcccgatcaagcactctttgggcttcgattatgattacaactatatcgtaaacgagattgtggccaacattaagagtatgtgtaaaaagaataaggtgcctgtaccgaatatttacacagagtttggttcctttaccgtaggcgaaagcggcgcggtaatctatagtgtgataggtgaaaaaatgcagaatgacagggaatcctggtacatgatcgatagttctttcattactacgttacctgatacatggggcattggagaaaagttcctgatgttacctattaataaatgggaccaggaataccaggaggtgcatctcggtggacttacctgtgacggctacgatttttatacatctgaagaacatattaacgccgtattcctgccaaagcaacaggcatccggagagccgctgtacattggatttttccataccggggcctaccaggaccagctgagcggatacggaggcatcaagcattgtcttattccttcacccaaacatgtgattgtaggatatgacaagaacgggcagttgaaagattggttatatgccaaggagcaaaccgcccagagcatgctgaagattttgggttattaaaaaaatgggttagtaatcctactgaaagccccccgattattcggggggcttatttttttcattttttttctctcagtttgataaaaaaaggctttcattttactgaaagccctatcatggcataggttagatgatattcatccggcataaggaaaataggagatgaatatttgatcttacaaagatagcgttatcggcaggtatcagtaagccctaaaagttgtaattttttctaatctgtttttaccccgaatacagtaagaatgatgaatttattatcataatgttcgaaaacgctgcaaacggtaatatttacatattagtatagcaggaataatattaatatggaagcattcttttataacacagatgtgtaggtatcatttcgcctgagaatcattgaggtagtcgacagcggagccgcaatgtttttcaatttcttcaaaacaactttccagtaactctgtttcccccttcaaaacggctgttttccctgaggccgaaaatccttttaccagtaaaaactgcttggtcaggtgttgattgatcagcgataaatgttgtttttgcttttcggcggttctcatttgttccatggaaatcaggttgcggtagtattgccccagtgccctgatgaagaacaatacatacatgcctaccgtaaacgggttagccaggtattggaaagcggatgaataaccaggtgaaacgaatatcatcacgttattgatcttgatccaggcaacggctatcaggtaggtgcaaaggatcaggctccagatgagggcggtgaacaggttaacggtaatatagcaaacgaggatactcattacccatatcagcgtgtatttggggccgaggtcctggttgttcagcagggacgaaaaaataggaaggatgagtgtggataaagaggcaaacaggccgactgttttagcgcttattccttttttcagcagtaaaaggcaaacggccagatcgagaatgatcacaggaatgatgatgatatttaccgtattctggctgagcatatttacaaagaggaagctcaggagcagcataatatagaagaaagcataatcaaagatcagtttgatcttcgcttgttcgtatgaattttctgtatgaagaagcatgctgcctatcactgctttttcagtgttcaggtaaatgctttttatgagtaaccagcctttcgggaagagctttgccatgagtgcttgcttagagaggcaaattattgcataataaacaatagcagattcaacgttcgtgtgaattatacacaaaaaagggacgcctttacaggcatcccttttaaaccctcatgttactacagcgggcctcctttttacaggaagccctgcttcccttattccactactatttctttaggggcatcctgtttgttttcctttttgcccaaggttactttcaggactccgttatcatatttcgcattaatcttacctgcatctaccagttcgctgatggtgaaggagcgtttgaaagatttgaaggtgaactcacggcgtacctgtttgtcgccttcattctttgtttctgctttcttttctgcgctgatggtaattgctttatcatctgcactgattttgaaatcttctttggagaaaccgggagctactacgtcgagcaggaaggcttccggcgtttccacgatgtttaccggaggatgcgtggtaaagtaatcgttggtcagaaaatcatcttttacatacttatttaatcctccattgagaatgtcttctactaatccaccaaatgatttgggaagcgggctgtggttaaatttaatgtgtgtcatagttcctataaatttttttagtgtgaaatcaatttttattgtttgatagctggtacagatcaaatgggataccatgccataaaaactgctattttgttagtaaaaaggttacagattatgacactatgtcattatgattgtatgttctgtgtcaaaaagtctatattgctatccatttttttactttctgggtacatataactaactttgtaaaaaatataaacagaaaaaactcttattatatgtatccagcggaactagtaatgcccatgaaggcggaattaacagataacggatttgaagaattgctgacaccagagagcgtggataatactttacagaaagaaggaactaccctggtggtaatcaattctgtatgtggttgctctgcaggtaccgcccgtccgggtgtattgctggcagtagcgcacagcgaaaagaagccagacaggctgactaccagctttgcaggttttgatggtgaagcggtaagacaaatccgttcgcacctgatgccttatcctccttcttccccggcgatagcgctgtttaaaaatggtgagttggtgcactttattgagcgccacatgatcgaaggccgttctgcgcaaatgattgctgcgaacctcgctgacgcatttgaacagtattgctaaatattcgattttttctaaattccaatttagaaattcgaaattgcatcgtactttggtggtttgattttccttttgattaaattcggctttgttcataggaagattcagatcaccaatttttttacggctatgtatcctaatttatattacgcgttcagagatctgcttggcttagagattccgtttttaaagattttccagacgtttggtttttttgtggcaatagcctttctggccggcgcctatatcttaacacgtgaactgaaacgctatgaagcactcgggttgctgaaaggtattcctgaaaaagtagtaaccgggcttccggcttcgcagggtgaattgattggaaatgccgtagtaggatttattataggatacaagatcctggggatcttttttcagtgggacaccgcttcacaggatttacagtcgtttgtattttcgggacaaggcagtctttttgccggtatcctggtagccgcagccatggcgggatataaatattacaccaaaaagaaacaggcactccctaagccaaaagaagaaacggtgctggtgatgccacaccaccgcgtaccggatattattgtaatggcggctattgccggattactcggcgctaaaatatttcacaatcttgaaaactggaacgactttgtgcaggaccccatcggggcgctgttgtctttcagcggacttaccttttacggcggcctgattgtagctgcgattgtgatcatcagttatgcccgtaaaaaacaattcaatatccgtgcgttaatcgacagcgctgcacctgcgttgatgctggcctatgctatcgggagaatgggttgtcatttttccggagatggcgactggggtatttacaacagcgcttatggagtggataccaataccggtcatgctgtaaaaatggcgcccgccacattccaggacattgttcagaaaaatgcaggtttctttcagcagcaatattcatcagtagaaaaaataccgcatgctgcttttgaaaaaccggcggcactgggctttttaccggattggttgtttgcctacggttacccgcacaacgttattaaagaaggagtacagatcgctggttgtgatggtccttattgtaaagtattacctattgccgtatatcccacaccgttatatgaaattattgtttgcctggttttgttcggcatcctctgggcgatccgcaaaagaataaagatcccgggtgtaattttcggcatctacctgatattaaatggggtggaaagattttttatagagaagatcagggtagatacgagatatgatatttttggctttcatcccacccaggcagaaatcatttccacgctcctggtaattggtggtattatactgattggcatctatcgtaaaaataatactgctgcaaataagctttcctgattatagtatatgcaacgtcactcttcattagtgcccttgtcgcacgagcacaagcgccttttatttgtatgccgctacctgaaaaaagatgccgcgccgtacgagggtttcccattggaaacacaggcaagatttgagtatatcataaaaatattccaggagctgatggtaccgcatattcaaaaggaagaatatctttttgagaaatgtgcaggccagcatgaagcgattgacaaaatgatccgggagttgcaggaagaacacctgatcatttcccgtatgtatagcactctcacagacagcaaggatatggatgccgcaatggatgtgctggcgtgcagcctggaagcgcatatccgcagggaagagcgggaattctttgagctgctgcaattggaacttccacatatcctcgataacctcaaactggaaaatccataaatgtatttaacgtgttattgccaggttttgatttaaatattaatttttcactggagttatagcaacattatgtatctgtaatattgcctcaataattatctgtatatcttatagcaatttatccttgtttgttaggctggtaaattttacccgggctattcaattagagttatgcgtgcgtttttttacagtgtagttgtgtttagttgcttaactgtcagcctcaatgtccttggcctatccagggaagacagtcttagcaggtacgacaagctggattcttctgaaatggtggctgcttccttttattataaagcaggtgaacaatcgttaggtgagggtacaatattaaatgtaccggaagggtaccgcctgctcgatggtgcgcagagccgtgtgctggtggagcatttatggggcaacccggaaaatccgaatacactgggcgtgctgttgccggcgaggatgggacctatggataaagatttccatggttttgtgatttcttttgagccttcgggttatatggaggaatcagcgatccggcagattgattacacgaaattgctgacggagatgaaagaggagttgaaaaatgataacctgctacgcagcggcaaaggggtggggcagatctccggtatggactgggcctttactccttattacaataaaaacaatcattccctgcattgggcccgcgttttacattttggtaaaaatgagccttccatgctgaattacgagttaagattattaggaagaaagggggcactctgttttacggctatcggtaaagtaacggaactggagcagattaagcagcaattagccattgtagctgctgctgcgcgttttgctccgggaaacggttacgccgattataatccgcgtacagatcagtcttcccgttgggtgcctgcctccgaatccgtagctggcagaatgctatcgattgataatcttttactcggaatcagaagtacgctttccatgttgctggtaatactttgtatggtattgtttgtttatggtatgaactattatcaccaccgccgcaagtccggttaccggaaaatcatgaaggtggatgagcgtctgaattgagaaggggaccatgccgtttttccatctccctaacatataactatttactgttaaccctggttacaaggccatggccttattccctgtttgtaaaaaacagccaccgtccttatataataccggtcatcctccattaacaccgctattttaaatagctgtaacctatctgcaactttcctttgcgccagtcgtctttttaatcgttctctgtttttttaccattcgtcactgtctatatgccgtttgtgtaatgctatgtactgtgtaatacataatacctacttttacatcgtagtagttaatctactgtagtggtttaactactgtagtatacaaaccaaggaactaaaagaaatctaaatcgtcaacgtttaaactctaaatcacctcatatgaaagcaagttttaaagctataacattaacaatgagtatgttagtgactgctttgacctcgtttgcgcagaatgcccccaaagtagccggacaagtaatccaggcaggtaaccagcctgtagcgttcgctactgtaaccttattaaaagcaaaagactcctctttggtgaaaggagccattgcagatatagatggtaaatatgaatttgagcaggtaaaacagggtaaatacctggttgccgcggtttcagttggcatgaccaaacgttacagccccgcttttgaagtagccgccagctccataaaagcgccggctgtaacactggaagccgcctccaaaaccttaaagggtgtagacgtaactgcccgccggccatttgtagagcagaaagctgataagatgatagtgaatgtggaaagcagcatcactgcatcgggtggttctgctatggaagttttggaaaaatcgcctacagtaaccgtagacaaggacggtaatatttccatgaaaggcaagagcggtgtacaaatcatgatagatggcaaaccaaccaatatgacttcccaggatgttgccgagctgctgaaaagcatgccagccaccaatgtagatcagattgagctgatcgctaatccttccgccaaatatgacgcagccggcaacgcgggaatcattaaccttaaactgaagaagaacaccagctatggtacgaatggtaatataaccgtgggtggtggctatggcttctggccccgctggaacggcgcactaaaccttaaccaccgcaacgaaaaattcaatatatatggttccggtaattacagtcaccgtgaacaacagcaggacctgggtttataccgctccctcacagaaaataaccagctgagtgtgtacgaccaggtaaacaacatgcacacaaaatccaattacaaagccggtaaaataggagcagattactttatcagtaaaggacatacaattggtgtaatggcagatttatccggcggcgaccgcaaaattcccagctatgccaccacccgtattggtaatggcagacaggtggactctatcctgaaaaccaataccaacgacgctaaaacctggacccggaatgccttcaatttaaactaccgcggcatcctggatactaccggtaaggaattgaatattgacctggattacgcaaaaaacaaagatgcgcagcatgctactatatatgcggtatcccgcgatggggctgaaaaaggtttcctgggcagcgatacttcccggaacaatcagccttccagcatcgacatcaaaactgcaaaaattgattacatacatccgctgaagaaccaggcaaaatttgaagccggcgtaaaggtgagctttgtgaaaaccgataatgatgcgcgtttcgactccctgagaatgggcaactgggtgctggatgaaaaccgttccaaccactttatctataaggaaaatgtaaacgcggcgtatatcaatttcaacaaacaatttaagaaagtgaatgtgcaggtaggattacgcggtgagcaaacgcatatcacgggtacatcagtgtcgatgaagaaccagcagcagatggaagtgaagaacgattctacttactttaacctgtttcccagcatggcattgacatataaactgaataaggataatacgctaggactgacctatagccgccgtatccagcgtccgagctatgaggatctgaatccgtttgaattttacctggacaggtatacaaaggagtctggtaatcctaacctgaagccacagtattccaacaactttgagatcacgcatacctttaaggatttcctgatcacctccgtaggatacgcgcatacaaaggacctgatgacccagatactggaatctgatgtggataaggcgaccggggatacttccattctgcggtacaaatacctgaacgtggctaaggccgacaactttaacctgaacgtaacggtaccgatgcccattaccaagtggtggatgagccttaccacggtgtcagtatcttatgcgatgtttgaaaccgtggtaaatgatcaccaggtgaaactgtcgtctgccgggttcttcggacgcacgcagcaaacattcacgctgagcaaggacttgtctgcagaagcagtgttcttttacgtatctccgcaggtgaccgaagatggcctgttcaagatgaaatctatgtgctccctggatctgggtgtttcccagaaagtactgaaaggaaaaggatctgtgaaactcaatgtaacggatgtgtttaaaactaattatttccgcggggactttgataatgcgggcagatatactgctgtttccagcaaatgggatgcgcagcagtttcgcctgaccttcaactaccgttttgggaatactaatgtaaaagcagcccgcagccgtcaaaccggactggaagcggaacaaaatcgtgtaaaacagggcggcaactaggccagcctgtttgggaagatggttttttaggtatataaggatggaaaaacgtggccctttaccgggctgcgttttccttaccaatttctccggtatacagatgtgccggtttcatcacaggaaacggcagtttggtataatttgacatagaagagagggtgtttgcaataattttgaagaaattttttaccggatatcactttcatccattctctataaataattaataattaatcagataacaaatttttgctggtaattaaacggacaaagtctcaccaaaccggaaatttccccgtcagcatcatgcaaccttttttacaattactgtctttataatgaaagcatcagccactaacttgaatcagacgccactcgcagcatatatagtagaacgctgcaaaaaaggagatgtccgtgcatttcgtgaattgtacgaagcctattcggctgcgatgtacaacatttgcctgcgtatgaccaataatgtgagtgatgcggaagacactttgcaggaggcttttatccaggtgcataaaagcattcataagctggagcgtgaggccagtatcagtgcctggatcaagcggattgtggtaaatcattgtttgaatacactgcgtaaaaagaaggtgtattttgaagacgtggatgaagtggaagtattgactgaagaggggattgatgaggcccagtttacctggaccgtagccgcagtaaagtctgccattcatagtttaccacagggttaccgtaccgtattgaatctctatctttttgaagagtattcgcaccgggaaatagcagagatgctgggtatcaccgaatccactgtgaaaacgcagtatatgcgtgcaaaggagaaagtaagacaaattgtaaaacagcaaaatgtaactcgttaatgccagacaattttgaaggttttatccgccagcaccgggacgaatttgaggaacagggcccttcaccgagggtttggagcgcactggagcaggagctgacgggcaggcgcaaaggaaaggtgatttcccttttacagaaaaactggtttaaagcagccgtgatcgcagttttgctggccaatgccggcgcgctgttttacttcaccaaaaaccgtcagccgcagcagcaggaacttgccgtgttagcgcctgacatccaggaagcgggcgtttactatacgtcgcgcataaacgaaaaactgcagttgattgatgcctatcccgattcagcgctggggctggatagcgctgcccgtaaggaactggaacttcgcaacgatacttataaagcactggagaaagaattaaaaaataatccgggcaatgaaagaatccgcgctgctatggtccgctattaccagctgaagctggatctgttggataaaattttggaagagttgcacaataaacatgtagctcccggtcaaacaaaaaaacattatgaagctgaaatttaaatgcttgttattcctgctgctgccattactggcgcaggcccacaatggagctacggcttataaaagaactattgtaaaggagtttactgtaaatgataacgccacgttgaacctttccaataagtacggcaaaatcatttttcacacatcgaacaaaaatgaaatcaaagccaccatcactgttaccggtttcggtaagaatgatgaacaggccaaagccattgcagaaatggtggaagtgaacaccaaccagagtaataacggcgtgtcgctgaacacttattacagcccgtcgaaaaacaattccggttggttttcatggggagggaaaatggattccaaagactacgtgaatattgactacgatatttatattccgcaaagcctgcagaatttactggtgaagaaccagtttggcgatgtgattgcggataaatttagttttcctgtgacgctggaaatgaactattgcacctttgatatccgcgaggcgcaggaccttctcttcaaaataaattattgtgataagggcaaggtgggcaaagcgggtaatgtaacggtgaaggggaattattctgccctccggggcgggcaactggaatcactgaatgccaattccaattacagtgagtatgtgtttagccgggtgggcaacctgaaaatttcttccaactacgatgattataaaatagatgcagtgggtacagtgtctggccggggtacttattcagatgtgcggttaaaggaactgcagcagtctattgatttgaacatgacgtatggggatgtgaagatagagaaagtgggcagtggattcaagcaggcagattttcaactcacctattcagatctggatatccgttttggagcgaggcagccattgtcgatagaagcaaacctggtaaacggggatctggataccggcgggctggagctgaagaatgtagtgtccaataaaacgaattcgaccctgcgttattctgcacatgcggggggaggaaatgattcatctccctatataaaaatacgcggtgtaaacaccgatgtaaacctgggtacatattaaacagatcagaacgccattctaaaatctttttaaaataatactacactatgaaacgaattgctgcttacttcctggttgctttgccattgttgcttactgccagtgtacttgtttccttttcgcatcagagcgatcaaagaataacgggaaacgggaatgtgaaagaagaatcccggaatgcgtctgcgtttacagatatcagcacttccggtgtgtataaggtgattatagaacagggaaatacccacagtatccgggtagaggcagaagataacctgctgccttatatccagacagatatcgccggcgacgagttaacgatccataccaagaaggggtataacattcagcctaccaaagaaatcaaagtatacatcacgctgcagaaggtagataagttgtcggccagcggcgccggtggttttacgagcaagggaaagcttaccagcgaccgcatccagctgaggttcagtggcgcggctggtgctgatctggacatccgtacccatgaactgaaggtaggtgtttccggggccagtaatattgtcctgaagggcaatacagacaaggctgattatggtatttcaggttccgctgatatttcagcgctggatctggctactgatgatgcaaagattggtatttccggtaccggtaaggcagatgtatttgtgcagaagaaactggagataggtatttccgggatgggaaaggtaaaatataaaggagaaccgaatgttacccagtctgtatccggaatgggtaagatcagcaagatataataacaagttagatttagagtatataacgagcaggtagttctctacctgctttttcttttttatatttgttgttcgaatataaaattttaagttatgccatcctttgatattgttagcaaagtagatttacagacactggataatgctattaacacggtgaagaaagagatcaccaacaggtttgatttcaagggttcacatgtggagattgagctgaataagaaagaactggtgctgaatatagaggtagaaagcgatatgaagctgggccaggtactggatgtgctggtaagcaggaccatgcgccaggggctggacgccagtatttacgacctgagcaaggagccttaccagagcgggaaggtatttaagaaagaaatacctgtacgtaatggtattaagcaggaagatgccaagaagatagtgaagatgatcaaggatgctggtttaaaggtgcaggcagccattatggatgatattatacgggtaacagggaagaagattgatgacttacaggaggttatacaaaaggcgaaggaatccaacctgggtatacctttgcagtatattaacatgaaatcctgatttttttacgaataatctttgggtgttaaagaaaattagttaactttgcaccctgtatttacaataattttgatatgaaacagggaatccatccagaaagttacagatttgtgatatttaaagatatgtcaaacggcgagagctttttaagccgctctaccgctccttccaaagaaactgcaaagtgggaagatggtaatgagtatccgttgattaagttggaaatttccaatacttctcaccctttttatactggtaagaatgtgttggtggatactgcaggacgtattgacaaattcaacaaacgctacgctaagaaagcatagtttctaagtaaaatatttttttagaagaatcccatcggcttatcgatgggattttctattttagccccctatggagcgtaactatattctttttgacacgcccgtacgtgaactgttatacccctttacgcatacaagacccattgcagcctgcagagtagggatactcactatacaggagaagtgggagcactggctgggtacgggtactagtcatttcaccgtaccgcatctgcaggacaaattctccctgttgtacaaagacaaccaaaccgttaacatcttactgagtggacatatactgccggacgccgggctggtagctgctattcttgagttacaaccggaagaggagttgtataaagacaaccagttactggctaaagtggtacaaggggatggcgcttctttgctggctccgggcgccaggaaaaattatccgggggaagtaatgggaatttataagccttgggatatctttgcgctcaacgataaagcaatcagggcagattatcagctgcttacagcaggcaggaaatctgttatcttatcacacaccaatcaacagatcaatcatacggacattttcgtggaaccaggcgcgaaggtagagtacagtatactgaacgctgctaccggcccgatttatatagggaaggatgcggaagtgatggaaggctgtatgatcagggggccctttgcaatgggagagggagctgtattgaaaatggggagtaaaatatatggcgctacaacattaggcccgtattgtacaggtgggggtgagatcaagaacagtgtgatgtttggttattccaacaaaggccatgacggttacctgggcgatgcggtgataggggaatggtgtaacctgggagccaatacttccggttccaacctgaagaataatgtgtctgaggtgaaagtatggatggagacgcagggtgaggcggtatctgcaggtataaaatgtggattgctgatgggagattacagcaggtgcggtattaataccatgctgaataccggtactgtgatcggggtgtcgtgcaacgtgtttggcgggcattttccgcccaaatttgtgggttcattcagttggggggaccagggcgcctaccgtttggcggaggctgtgaaggatgccggtaactggatggctttgaaggggaaggagcttacggaaaaggataagcaggtattggaagcattatatgcacaaataaatcagaaagaccttaaaacttaatatcacagtatgagaaagaaaattgttgcaggtaactggaaaatgaaccttacgctggcacagggtgagcagctgatcaacgatatcctgcaggcaggactgaagctgaaagagggacaggaagtaattgtggctaccccgtttccttatttgcagaaagcgaaatcgttactgaaaagctatcctggtttttatgtggcggcacagaactgttacagtgaaaaatccggtgcttataccggtgaggtatctgcggaaatgctgcaatcaataggtgttgattatgttattctgggtcactctgaaagaagggaatatttccaggaaagcaatgctatgctggctaagaagatagaccaggtgctggctaacggtttaaagcctattttctgctgtggcgaaccgctggaaataagacaggcagaaacgcagaatgcctatgtggccaagcagctggaagaaagtttgtttcatcttacagaggagcagctgaagaatgtggtgattgcttacgagcctatctgggccatcggtaccggtttaacagccagttctggacaggcgcaggacatgcatgcttttatccgttcgcagattgctaataaatttggccgtgaggcagccttgcatacttctattttatatggtggtagcgcgaagccgggaaatgcggcagaactgtttgccagcccggatgtagacggtggtttgattggcggcgcttccctggtggcagccgactttgtggcgattattgaaaagttatcttaagtaattgagaaatacgcagttataaaggctgcgtatttttttagtaaataatgctaaaaatattagtatttctgaaaaaaggttgtatattcgtattgtcattctaacagggagaattaaaatatcaggttatgaatacgaattatgaaatttcggaagaggtatttgattatttagtggtagtgaatccggatgcattggttgcgaaagatgtgacccgtatccgtcagtttgtagcaactgagttaagcgatacgatgatgtctgccgcaccggttcatgtggccttgttcaggtctgcttttcctgaacgtttccaggacgactttgtcgatatgctggaagaggtagcgcgtaaacaggctggttttgccatctatacggcaaagattgatgccctgaggcatgcggacgggcacaacagtgttttcattaatgtcgctaaccccaagccattgatcgatttgcaccgcagtattatgcaaacttttgagttgaagccacaaacattcaagccgcatattatgctggcgagaggcttgcaggatgcggaggtaaatatgattatgccattgctggcgcagcagatttttgtacgtagctttaactgtcattgttttagcctgctgaaaaggccagcgtccggtggtaagtatgagcgggtgaaagactttgtctttggagatattgagcacatggtaggttcattgtttaattatgctgctgcgtaagtagtacactataatctgatgcaggaattaccggatggtagatttgcaggattggtgaagatgttacggataaaataatttgttatcccctatatcaattttcatcaatgtttgttaccctcaagttaaccatcctttcgtactgttgctattgcagtttttcgcctgctgtcacaggttggctgtggaattgcggtagttatttgatccgtaggcacacattttcataggttgctgcgtatccataaatccggtaaatcctggttcagatagttgtttgtataaccaattcttctttttctggtatgccctgaaggtccctgcctgtaattagttttccggttgtttgtatctttgacgaatatttagtatgttttgagtgggagctgtattcatgtgatataaccccatccgaagaagaccattacagggtaaatcgttataaatttatggcaaccagaacagttgtacacaaagaaattattgtgaagggccgtgtgcagggagtaggattcagagctaatgcaaagcgtgtagccgattcaatgcatatacacgggcaagttaaaaatctgctggacggaagtgtgtggatactggcagagggaacggcggaagaaatggaagactttattgcatggtgcaggtctgggcctgctatggctgcagtgaaggaactggaaatcaccgatggtgatgtacaacatatcaaagggtttactatcctttattcataaatccctggtccggtaacagcaggtgcttcgttacctatgccaatcaatcgcagataaagctatccgtgaccggcagacaacaggcgcaaagaaattttacggggcaacgcaactgaatacaaccgtgaaaatttctttgcgcttttgtcatgcatatttagttggtactggtgtatttcttttggaaagatttatccagtgcggcttttggaacaacgatggtgatggtatttacagcgaagtaagcctcggatacatttacatagccaccaaacggactggagtttttaccccatgaattttttaccaggaagaacgttttaccctttggcgatttttcgatccccgtaatgtgcatcaggtgatcatcctgtgtaatcagctcttcatatagcttttgacgtgagtcctgtgtataagcgggttcagtcatatcaggatcgatactatcttttttcagcgtgatttccggtgaggtgagcagcgcaaagcctttgctactggcgaacccgcggttacttacatctgcatcccataacacggtgtagcctttttgaagggcagcctcggtaataccggtcagttcttttacgggcacattataataggcgccattggagaagttgtctggtacttcaatgatgaaaggtttgtaaaaaggatggtgtgtaaaggaagtcaggaaaacatagtcgtcttcattaaattttaccacttccttcgcaaagctttgcggggtatatgttttaccattatagtcaaaggtggccggcggcgctcccatatactgatcgaggataccggtgaattgtgatatccagttatccggcacaggggatactttgatgatactgtcgaggtattttttcatggctaccaccatttctgagtggttgtgaacggtggcattgccttttaacccgctgtaaacgctttccggttctatgccgtaagcggcaatggaatggattacatcgtgggccaggccgccttcatcgaaacgggcgaagccctgtcggcgcacatagtttttggctttttcgatataaatattgcgggcggtaaacatttcagagagatccagttcaggcagtcctttgcgtaaacactccgattctaccatggaagtagaggagaatgaccagcaggtgccagtcatgccctgatttttaaccggggtggctgcattgattttaccattttccagattgctgattacaacgcccttttcctgtgcacccgctgcgaaggcggtgaacagggcaagggttaaacaaaatgctttcatatacgatctcattaaattattaacctaaagataagtgaacccgtataataaaaaataccattaccgtatgaacggtaatggtacggatgcaatctgcaatagaatggcagtaaatcagttttgtatatcggaatgatatgagtttgcagaaccttttatggtaagccgttttgtttgcaggtatttctggtatttggcggccacattgtcgggttgtttaacatcattgatgaatagcccgttttcatttttttcaatcttgtagcctttttgggcatcgagcagcttgtcagcctccatttgggagatcatttctttataaaaggcggctcttttttctccttccttcgctcttttttctccttccttcgctctttctgcaccttcttttgctcttctttcaccttctctggctctttcagcgccttctttcgctctcatttccccttccagggttcttttggcattttctctgtcacgggcgatattttcccgcaccctggcagcattagcgagcgcttctgccctgtttctgcggacttcttccagagaggaggtagcattttgtgttgccaggctggctgctttaagaccagcctttgtttccttgcttatcttatcataaaattcctttgtgtttacgctggcgtatgcagcttgcagatttttgttgagtgctgcaaaatcaatgctgttcagggcttcagcggcttctttctgggccgcgctgattttgctccaatcgatatttttcagggcttttacgctttcttcctgggctttacgggcttcagcagatacttcgtcccatttgatatttttggtggcttcggctatatctgcctgtacttttttcatatccacctggttcagctgctgcatggcctgctggacgcttttttgcgcttctttaatttgctggcgcacttcgtctttgttgaactggtagtcgaatttataattgtaattaaatgcctgcgctttgttggttgttgcagtgtgtttattattcttatttacgtttacctgtgtatttacattggtggaaacgttgctctggtctgttacctggatatctgaaacatctaccgacagatcgccttttaatggcgccagtggtgctaccggtggtagtggcgccggcacaggagcagttactggttcaggggcaggagcaggtgttggtggtgggggcgccggcagaacggtgtcggtggtagcagattccagttgttcacggaatttgcgggtcgtttcatccggttcaagggcagccagttttttctgcggggtgctgtcttttacggtctttacttttgccggttgttgctggtcgttctgatcttttcctttagcagggttgagccatgcgatggatataagaccggtagcgatgatgagtacggctaaaaatttctggctataattaagatgtttagttttcatttccatgatgcgtttaatgcggtgaaacagatgttgtttactgtctgcagcagccatggtaagccggttggcggtaaggcggtattcctccaacgctaccagtgcgtgcgcatattgcagtggttgggcggtgctggctattaccaggtcatcgcagcaatgttccctttccatacggatgatttttgaaatcagccatacaaaaggattaaagaagagaattgtttcaacaattgattggaagatattcaacagataatcattgcgtttgatatgggccagttcgtgcagcagcactgcttccagctgggcttccgttaggttattcaccattgccaccggtaagaggatgaggggctttataaatcccagcatcacaggcacctgtacatgcctggagataagcagtttcaccttacggggaatctgcaatcttgcagcgagtttatccaggtgtttatcccatgcgtcgcccattggctctatgcgggttgtgcggattttacggagttgaaacagatcggacagcagtttaatgatcatgccggtcatgcccgcaatatatagtgttaccacgaaaggaaaacaaagctcaaggttgggaaacagccatatcagcgggtcctggctcggatacacggcggtaagatgaaccggctcctgtaaggtaagggtgccactgaagtgttgtactgcttctcttgcttcctgcagccgttgtacatgcatatacagcgttgcgagaaaccaggtaaaaatgcccgagagggagagcagcgacaggttgtattttatccgtgcgccggcctggggccagagttttaatactatccgtaaacatgcgtaaatgaagaacgcctgccacatggaatgaaggattgtccaacccagggcgcgtacaaagtcgcccgtaataggtaatacattcatagtactagatttacctgttttccttttgttgtttttctattgtagtaagatattgccggatcttttccagttcttctccagacgactgatggtggccgagggcctgcattaccagttgtgaagcggaaccgccaaaaacggtatctatcattttgtccagtaattgttgctgtgttttctgctgtgaaatggcggcagtgtatacatgagttttgctgctggtatcgcgctgcaacagctctttttcatgcataatctgcatcagtttgagggtagtggtgtagccggcatctttcgtttgagataagatctcatgtatctcacgaacggtgctggggcctttttcccaaagaacgcccaaaatttccaattcactttctgtaggccggatctgtttcaaagcaatgatttatggatgatgatgattgttgtacgaatatcttcgtaaacaaatgtacgatagttttcgtaattgcaaaatatcgggcggaattttttttcgcggaggttgtcgcggaggttgtctttttcgctgattacgctgattatactgattttaaggatttgatcactttttgattttaaaggatttgggaagagatcagcgaatatatccgcttttatctccctaaatcctttaaaaaatcctaaaagcaaaatcaagcaaatcagtataatcagcgtaatcagcgaaaaagacaacctccgctcaggtctccccacgtcgcagctgccgcgtggttttccggctgccatccgcgctccagccaggtgcgtcaaaaatataatgcactgcttcgcgtaaggagtgggcataccgcacatcccgccagatatccagccattcatgggtggcaatacggaagggattataggtgtgtatatttttggtgaggccatataccggtcgccgcttttccggggtgaaggtaccaaacatgcgatcccagataatgaggatgcctgcatggttccggtccaggtaatcgacgtcggagccatgatgcacgcggtgatgagagggggtattgaatatatactctataggcgccggtaatttatggatcacctctgtatgaatccagaactggtagatcaggctgatcgcctgcatactcattatcattaccggatggaacccaaggagcggcatccagagccagaaagtaaaggtgccggttaagttgccggtccatgtttggcgcacggccgtggcgaggttgtatttttcagacgaatgatggatgacatgtgaggcccagaaaaaacggatattatgactgctccgatgaaaccagtagtaactgaaatcatctgcaaaaaaacataatacccatgcccaccaggtaaagcccagggtaaacagccggaactggtaaagaaaaagatagatgccgaaaataacggctttggtgaagatcccgatgaacacattaccgaggcccatcgcaatgctgctgagcgcatctttcggttcgtacatgttctttttgtcgatcgctgtgaaaatgatttccagcagtatcagcagcacaaatccgggaatggcatatgttatcaggtcgggaggcatatgtggtaactttctgttacggaagttaacgaatttttgcggggcttcccggtaactaaagcaaaaatgcagcggagaaaaagcttccccgctgcattataatatttaaaaaacaggcactatttaaatgttctctctgcgcggcttacagcagatgtaccaaaccagcccaggatcctcgttttaccggaaggggtggtgttatgtacattgctttttacgttttccaatactttggcaaacaatccgccggaatttacctggttatttacctgggtaaggaaatcgtagctggggtgggtaagggaaagcattcttacaatggccttttcatttgcctggaaaggtttatcgtaatctgtaataccttctcttatcggtaaaatgaaagtgttgccatcggaaacgccttcatcataggaaccatcaatggagaagttatcttccaggcgcttcagtgtatcattgcggtaagagcggatccagtaatagtctgttgcaccagacaggtccctggcgtggaacttggcatagtagccttctttgccgctgatagattcttcttttgttttgaattcataagagatggaatctaccgtggtaactcttttgatactgtcgaacgcttcaaatatttcacctttcagctccacatgcagcttgtatccatggcctataatgccgatagctttggtagaggcatcgtaggtgtatttgttgtctttgaacaggaatggataagactcgccgctggtcaggtcaaacagggtgatctttgcatcgtcgatgatgggcgccgggctgttatctgtataaggtaccgacatggtgaacttaatggtttgtataccggtttcattggtaatccacgcatccagtaccggataggattttcctttcgcaatgtccaggtcgatcttgtcttcgcaggccgtaaaacccgcagcaacagcaaacaatatgaggaataatgactttttcatctgatcttgaattttggacaattagaacttgaagttatatgtgataccaggaatgatagagcctatgatagacatgcgtactgcttcccgtttggtaggatcatcgtcgttttgcttaaagtaaatggtgtaagcatttctgcgggcatatacattatacagtgagaacacccattctcctttccagcgtttcagctgtttgcctttcagtgtcatagacaaatccagtctgtgatacgctggcaggcggtagttattgcgtttctctgtactgttgtaaggaatgtcccagtcctggaattccaacctgttgtcggcgaaggtgcctggtgtgccggaggcgaacacccagttggccgacagggaagtacgtttggtgaaagtatgcgttaacaccaggtttaggttgtgggtgcggtcgtagcggttcaggaaccattcatccatactgatgccgatggttttcctttctgtgcgtgacagggtgtagcttacccaaccggtagttttgccgatatcttttttcacgtaaagttccagtccgtatgcgcgtccctgtgaaggcaacagatctgcttcgatgagcgggttcagctgcaggttagcattgtcgatataatccagctggttgtctgttgtcttataaaacacttcggcagacagttcgtaggcgtcattaggcgcattgtagaagtagcccgcagtgtactggtcagacaccattggtttaatattgttggtgctgggcgtccagatatccaggggagtaggggatgcggtattagacagttggtgcatgaactgtgtagttctgctataggccagcttcacagcgtgttggtctgtgaacgcgtaccgggcgctgatcctgggttcaaagtaatagtagcctttgatccggtcattggcgtcgaagtctttgctgctgatcaatcttttgcgtatgccaggtgttgtatctgcaaaataataagcagttcctttaccgatgaattgataggctgataagcggccaccgtactggataccaaatttctttgtgggtttaaactcgtgatccaggtatacggctgattccagtgcgtgctgatcgttgatttgtttaacgtgttgcagtgcaccttctgtgctggtacctgtgcctggtttaaaggtataatagatcccctgtaccccgaagtgcaggctgttagcggcattgatgtagtaggtaaaggaaggttttacgccgtagttaatgatgttggatgtccagtcgtaaccctgtgattcttccccgtttgctttctttgagtcgttgctgaacttcaggctataatcatacttactataataagtagtaaagttcatgaacaggcggttggtgaatacatggttccatcttacggtggcggtactgttgccccagttcatgttgatgtcttttccaaaaccaaaaacgtccctgccgaaataaccgcttacaaacagggagttatttttattgaacttgtagttggctttagcggtgagatcgtagaaattgagcttggtatctttcatatcaccttttacaaaaggtttcatcaggatatctatataagatcttctggcagccactataaaggaagatttatcctttaccagcgggccttctaccgacaaacggctgaaaatgttaccaataccgccgtttacgttgaagtcctggttgttaccgtctttcatacggatatccagtacagaagaggttctgccaccgtattcagcgggaaaaccgcctttgatcaggttgagacttttaacggcgtcggggttgaatacagagaagaagccgagcatgtgggtggagttgtatacaggtgcttcatccaggagaatgaggttttcgtcgctgttaccaccgcgtacgttaaagccggaagcgccttcacccacggtgttcacaccggggagggtttgaatggcccgcagcacatctacctcacccatgaaggtgggcatctttttcatttgctgtatatccagtttattgatgctggtattcagggtattgacggtcctttcctgtttctggccgttaacggtaactacgttcagctggctgctggtggcttccatgcttacgtcgagcgttacgttctttttcaggttaacagttgttttataggtaccgtagcccatgtaggagaactgcagttcatgttctccggccggaagcgtgagggagtaaaatccgtattggttgctcaccgtacccagactggtgccgcttttaccaatagagatgcctaccaggctttccccgttcttcttatcttttacatagccgctcacggtatatcgttgctgctgtgcggttgttgattgtcctgcgaggattaaaatgagcagagacagcaacatggttaccttagttttcataaaagtcagatgcagttttatataatgtctgttgcatttttgtagcatgcatataagacgtcgcaaaaatatgatacccctacggcgataaattatttttttaaatcataattgtgttacaacatgatttaacgaaaaaaggaaggccccggccttcctttttcaataaaatacgaagccctgtcagtccaggatggcacagttaaacccgagccgggttacaaaatctataattgtttgttctgctagtgattgagggcttacaatacgtaatactttgtcacagtcttccaggtctacgctacaggcatttacggtaaattgtgctgaaatggcgtcaataacattgtttctatcctgaacagttgtaatattggtacggaatattcccaacatagatgataattttttttgattcggaatatttttatgcaaatttgctactgttatcccatatagctgttacacgagacggattatcaattatacgaaacggatttttttatgggcgtagttattacagatgatgccaaccaggtattgctagtggaagaaattccttacgattaccataagatccgttccaggggaatgattgaagaaacccaggaactgcataaggattttggctccgcaactgtgcacgaatataatttcgagggcaccagtattgcctgttgcaaggcggaggtgtatgaaaatatccatgtttcttcagattttatggagccccgtgtcatgatgttattcatggagcagggagacattactactacccttggggggatttcggacaatttcaggttttccacacaggaacataatctcatgtttagtcccgagcaactggagactgtgggcgtaaagaagcagcgggacattctctttttgggtatgagctttacgccggcgcggttcctggagttggcggaaaacaatgggcgcgtgctggatcagctggccaataatgtggcagggaataaatccgtgacgctggccgataagtataatccccggattaccccgcgtatgcgtatggcgatggaggaagtgcggcagtgcaaattccagggaggcttgaaaaagctgttcttgcagtcgaaagccatggagctgcttgccctgcaatgtgagcagatggaagtggcgcaatcgtccggtacgcctttgcgtaataaaatcactccacaggatgtagagaagctgtattatgcgagggacctggtattgcagcatatccaggagccgttgagcctggaggagttatcgcgcaaagcagggttgaatgagtttaagttgaaatcaggctttaaagccatttttgataatacggtatttggttatttgaacgaccaccgcctggagctggccaggaagctgatattgggcggagatttgcccatggcgctcatcgcagagcaggccggatattcgtctccccagcacttcagtactgctttccgtaagaaattcggggtgagtcccgggaaagtcaggggttaaataaaaaaggacaggagcaaccaacggttgctcctgtccttttttatttaatacgccagtgtaaagcgttgtttgatatgttttggttgttccagttcatccagtaaggctactgcgtagtcggctgaagaaattttactctctcctttgtcgttgaacactacctggttggtacccaaacggaatttaccggtacgttcacctggttctatcatcatagccgggcttattacggtccagtcgaggtctgtggactgtttaatcacattgaatgcgtcgcgggtggcagtggcgccgcctttccactctgcggggaattcgggggtatccagcaattgtatgccaggggctatttccaggctgcctgcaccactaacagcgatcagtcttttgataccggattttttggtagcattaataatggcattgatagcctttatgtaagtagcggagtcgtgggcgctgtaagcgctgatcacagcttcattgccggccagcagcggagtgatttctgcttcgttggtggcgtctcctttctttacagtaagatgtgcgttggtaacggttatcttttccgggtgacgaacgatggccgttacttcatgtcctctgttcagcgcttcatttaaaatggctgatcctataaatccggatgctccgatgatggcaactttcatgatgttaatttttttgtagtgactaaataatacagcctgcccgtgctgattgttctaattgttagaaaaaatattacagtttagaggataaaaaaacagatcctctgatctgtaataaaaataattacagtacaaagatagggaagatattttaattaccaagcggattttgtctttctcaggattacgctgattatactgattcaggggatttgatcacgttggattttaaaggatttggggagatgtaagcggattttgtccttctcaggattacgctgattttactgatttaggcgatttgatcatgttggattttaaaggatttggggagatgtaagcggattttgtctttctcaggattaggctgattttactgatttctttgattttattttcagataattttataaataatttagggagatacaagcgaaaaatatccgcttacatctccccaaatcctttataaaatccaaaaagtaaaatcctttaaatcagtaaaatcagcgtaatcctgagaaagacaacctccgctatctcttttccaagaggtaggccgttgccttactgctcacctttttggccgccggctgtacggtttctgttttaacagtagggggaaccggtggctgcttggtatgaaacatttcggccagcgtgggcgcaatcaccaatgatacaatagacatcagtttgatgaggatgttcatacttgggccggaagtatctttgaacggatcacctacggtatcaccggttacggatgctttatgtggctcagactttttgtaataggtttcgccattgatttcaacgcctttctcgaaagatttttttgcattgtcccaggcgccaccggcgttgttctggaaaattcccatcagcacgccgctaactgtagcgccggcgaggaatccgcccaatacttccggaccggctataaagcctaccagtaaaggtgaaatcagagcgatcgcgccaggcagcatcatttcacggatggatgcctgcgtggaaatagccacacatttatcgtattccggtttgccggtaccttccatgatgccggggatttcgcggaactggcggcgtacttcttctaccatcgccatagctgcacgacctaccgccgcaatagccagggaggagaagatgaacgggatcatcccacccacaaacaaacctgccaatacattcgctttataaatgtcgataccctggataccggctacaccaacaaaggctgcaaacagcgccagtgcggttaaggcagcagaggcgatggcaaaacccttaccggtagcggcggtggtgttacctactgcatcgaggatatctgttttttctcttacttcttttggaagctcgctcatttcagcaataccaccggcattatcggcaatagggccgaaagcgtcgatagccagctgcatggcggtggtagccatcataccggctgcggcaatggccacaccgtataatcccgccaggtggaaggaaccggcaataccggcagccagcaccaggatgggcagggtagtggattccatgccaacagacaaaccaccgataatattggtggcggcgccggtagcagattgacggataattgattttaccggacgtttacccatcgcggtataatattctgtgatgatgctgatcagtgtacctacggccagtcctaccatgatggcgccaaatacctgtccgcgggtgaattcatgaccgcgtaaggtcatggcactttccggaaggatccagtttaccaggaagtaggaaacaatggctgttaatataatagaaccccagtttcccatgttcagcgctttttgcaccacgccggtattcaggccggagccttcgccgatgcgtacaaacagggtaccgatcatggagaaaatgatacctgcaccggctatgatcattggcagcaggataggagcgatgccgccgaatgcatcatgggaaacggtttcagaacccagtaccatggtggctaatacggtggctacataagaaccgaacaggtcggcgcccataccggctacgtcgcctacgttgtcgcctacgttatccgcaatggtggcggggttccggggatcgtcttccgggatgccggcttccactttacctaccaggtcggcgcccacatcggctgctttggtgtaaataccgccacccacacgggcaaacagggcaatactttctgcgcctaatgaaaaaccagtgagcacttcaatggttttgatcatttcagcagtattcgcttccgccccgaaatatgatttcagtataataaataaggagcccaatccgagaacagccaaaccggcaacacccattcccattaccgaaccgccggtaaaagacacctgcagcgctttagcaagactggtacgtgccgcatgcgcagtgcgcacattggctttggtggctatcttcatacctatgaaccctgcggtagcagagaacactgcgccaatcacgaaagccagcgcgatggaccagtgggagttttcatgtgtagctcccatgtatcccaatagcagggcggcaataatcacaaaataaataaggactttatactcagctttcagaaatgccatagcgccttcagcgatatgctgggctatctctttcattttgtcgtttcctgcatcctggcgtgtcacccaggagcttttaacagccgtatacaacaaagccaataatccaaaacatggaacgaggtaaactatattcatgtaagcgaaatttacaattacgtggttgacaaaaaagtttagtaattaaaaaaaataggattccaaaaaaaaatattcaaatgaatataaaacataaattattaattgtgtacccggtaaataaaattattgtacacatgggccatgggtaagtatttcaggcgaaaaaaaataaagcgctcagatgccttcccggaaggcattgcccagtgaggcgataatatcggaggcggtcatggcttcctgcgagagctgcgccgctgccagatcgccggcataaccgtgcagccacacgcccagcagcatagcggctttgggggtatagtcctgcgccagcaaaccggttaagatccccgtgagcacatccccgctgccaccggtagccataccggggttgccggtgtggttaaaatatacggcgccatcaggacaggcaatcgcggtataccgtcctttcaataaaatatacagctgcaggtccaccgctttttttgataataattccagccgcgccacatcattggcagttttgccgaataaccgctcaaattctttcggatgtggggtgagcagggatcctttgggcactttgtataacaggtaggaatatacggaaagcaggttgagggcgtcagcgtctatcaccatcgggcgttgccaggcatccatcagcgcttcgagcgatttggcggttccgggctgtttatcgatacccggaccaataccgatggctttgtaaccggcggaactgattcctttatgaaaatgggtgctgtagtgggcgtcttcatcagtgatgcacatagccgccggttcgctgatctgcatgatctgggtgccgcactggggaacatgacaggtaagcagccccactccggcgcgtaaacaggcgcgggcacttaatactgctgcgcccattttcccatagctgccggcaatgagtaatgcgtggccgtaggtgcctttatgtgcgaagggatcacgcggccggtaaatagtgcgcatcatttcgcgatcggacaggtgatatcgtgcaggcgtttgcgttatatactccgggtgcagcccgatcggcagaatatgtacatctcctgcgtagggtgcattttcgggtaacaggaaagccagtttataaaattcgaagctcagggtggtatgcgcctgtacaacgggattatgcacactgctttcgtcggccatcagcccggagggcatatctatggctataatgggatgtttgtggcgctggtcgttgataaggtgtataatacctgctacccatccgtctaccggccggctcataccggtaccaaaaatagcgtcaatgataatagcgttgggaggaagttccgggaagtcggatatatcgccgatggtataagttccggcagggtattgttgttgcaggatatgcagctgatgttcgtggtcggggcttgccttgctgctatgctgcaatatgccggtatgtacttcgtagccatgcccgagcattaaacgggcaatgaccagtccatctcccccgttatttccttttccgcaaaaaatataaacaggatgggagggagaataatgatcttccaaccaggctgcacattgtccggccgccctttccgtcaggtgtgtactgctgatgggttcatgagcgatggtgaaggcatctgcctccctgatctgtgcagcggagaagattttcatgtcggaaagttgaacattaaaattactccaaaataaggaacataaaaaaacggaccatgcttgcctcatgatccgtttgtaatgaagtggtcgccgggattaaaaagtatatcgggcagacacaccgccgatctcctcaccaagatagttggtgggtccaacaaactgtacgtaaggtttcagatcagcactgatgttcaaaggaattttcttgaaagtatattcgataccaatgatggcatccagaccgggagacacataagtacccttgcctttttccacataacggtcccagtcgtaatcgcgacggtcgtagaaacctacgtgcgcgccaccaccggcatacatgttcagttcaggcatacctatgttccagttgtattcatacaatccggtaaaagtaacatttgttttgtgtgagtgattggtggttaccagtccttcgatggcatgcggacctgtaataaagtgcttaatggtaaagcccactacccacggattgaggcggatacccagtgcagtttcgtagttggatggatcgctgctctgatagctttttttcttctgcgcgtttgcctggatcgcaattacagcaataaggctgaaaagtaacacgacttttttcatagatgtgttgtttgaatgaaacttaaaaatatacgttcagaaacgttggcttgttctctaaagtatatacacgacgaaattaattcacggttgctttgcaagaacagtgccaaccggtttgatcaggcgtagaaaaatgaatcctgcgatacctgctgcaagagaggcaacaatcactgacatgatggctataatctgcatttccctctcttgataagccagtgaagaaatgaaaatagacatggtaaaaccaataccggcaataagtccgacgccggcaagctgtaaccagcccgattttgaaggcagggaagccagtttgagttttacggcagcaaaggaaagtgtaaatatacccagtggtttccccaatatcagcccggcaatgatgccataactgatgttattatggagcgcggcgctgatatctattggtaacaggatcgcggtattggcaagcgcaaatacaggcatgataataaaattcaccgggtcatgtaaactatgcaccagtccggctatacgctcctgcggaatacaaaatgccagcaatacgcctgcaatagtggcatgcacgcctgaattgaaaaggcaataccagagcacaataccaggaatgtaataaaagatcaggcgttgtactttcaggaagttcagcaacagtggtatgagtaaaacgccgccaccgatcagtaaatattttacatcgaggtgcggagtgtagaagatggcaatggttaatatggcgcccaggtcatcgatgatggccagcgccatcaggaagatcttgagtgctaccggtacgcgtctgcccagcagggataaaatgcccagtgaaaaagcaatgtcggtggccatcggaataccccagccatgcgcataggcggtatttttattaaagaggacgaagatcagtgcgggaaacagcattccgccgatggcagccagtacgggcaaaatggatttgcgtacagaagataattctcctacggtgagttctctttttatttccatgcctaccaggaaaaagaacagcaccatcatgccgtcgtttatccataacagccaggaattgggcaggtgcaacgacccgtattgataatggtggccgcctgcgggatcaaataatgtattccagaatcctatataatcttcatgggcgccagtgttagccagtaccattgatatgatggtgcatacaatgagtacaattcctaccgcgcgactatctttcaggaaagtgtggataggggatatcagtgttttccggatgatgttaatagagttcttaatcacagcattctttttagtgaaaaatatttccgggagatgtgatattggaaatggctgcggtgaagcagccatttccaggtattgttctaacgaaaattattattgcattagctcgtacttcgttttcggctgccgtttgatatcccacttaaagttttccagcaggagctgttctttaggacgttgtgtaaacggatacacagttccttccggatctttgatcagtaccactttatctacttctcctttcttgaaaaagatattgataatggcgcactgggctttgttgacgctcatataggcgccggccttgtctttaatataattgatcgtttccgcgttcccttccacatgcatccagtcgagggtttcacccagtacataaccggtaatcacattgcctttaatctggttaaacatgcccggtccggcttcattaataataaagccgttgtttttgagcagcattttatctgctgtctggtttttggtgaacatgaggatggtatcgccgctcagctgggtggtattattagaccagagcaccggggtgccatagaagcggaagatagaatccttcgaggaatagtatacgctgtctgctacgccctggagggagtcggagaatattttcacgtgatggtaggcgaggatataacgttgctcgctggtgtctttaggtgcggtgagcgccatactgtctgcatggtgcttgatacccggcagggaatcgtgcaggaccacgtccggtatgggcgccaccttgatgtttgtcacggccgaatccagtttctgcctggttttggcgagggtactgtcggcgatgaacatcataacgtttgcggctacactatcctgttgtcgccgggcgatggaatcgccccgggtgatgggggatatggtagcggtaaatttctccggcggtcgaatattccggatgcttttcaggtttttggtgggagaatccgggatgcgtttcaggccggctacagagggaatagataagctgtcgtctggtctgatcacgcctgaaaacagggtatcagcggccatatacagggtatctttatttttttccatgatgagcagcggcttctgggtggcgaggattgttttttcgcgttggtttacgatacccctgttggccaacagcgacattttgcgggcagtatccttatataccatgttaccggtggcataggccataccggaaagtttatccatttctatgttatcggcggtgatggtgccggtactgtcttcgatggtaggccggttcccaaaattaccatagcctttttccgtgtcataataaccgctggtggcgtacatcacgcttttgtcgttattgttgatggtggtaggcgcaacgatggtggctattttggtaccggtattatacagcagttcatctgtgctgagggtgtattccggatctaccagtaatacattccgcatgaagtgcatttctttggtgtcggtgtaatagtatccttcatcgctggtgagtacgcttttaccatttacgagtttaccggttttgacataggagcctattttggcgttcatgtcatattgtagttcggggccggtgatggttactttaccgtctgtcagttttgcatcttccctgaggagagcaaggcgggtattggcatcgtagttcaggtaattaccgtagatatgaacgctgtcggcctggttaatatgtatatggccatatgcgtcgatgatattggttttattatctttcacggcactgtcgcagttaaacagggtggtaccttgtttaaagagggcgttgccgatgaagcgggtaacgctgacagaatctttgtcattcatgatcagtgagtccgcgtgaataatttcaattaccgacccggctttcggcgcttgttgggccggaaactgggcgttggccgtagctgccagcaggcagatgacggccagaaaaatccctgattttatgtatcgatgcattgattctttttattgtaccgctattgtgtcagaaggtaacggtttcgttttatcttttttgccaaacagggagaagtgtacatagcgttttggattgacgcggaggtcttccagcagcttattcaggttacccaatgagtactgaaggttgttgtacacttttttatcgttcagcagcatgcctgcagtgccatcggtggtattcagtttattgatggtctggttaaggctggtcacggtttgttgtaattgcgccagtgttttatcgatgttgccgttagccagtgcaccggtggctttctgggcattatcgaggataccggtaattttactgttattctctttcaggttaccggtaacggcggccaggttatcgaatgttttctggatgttaccgttgttgggatccagcatactgttaagggatgcggaggtatgcgtaaagttacgcatggtggtattgaggttgcggatggcgtcctggaggttaccttttgcggtggtatcgagaatggcatttaccgacatcagtacggaatcgatattagacagggtgccttccagtttttttaccagcgggttaagctgttctttcagggcgtctgtcatggagccgtctacggctgcgtagatggtatcgccgcttttcagatattcgccggcgttacccaggtcgagctgtactgttttggtacccagcagatcgctgctgatacgggccacagagttacgggggatttcaatttttttggtaatggtgatggctaccaggatacgggaggcatctttatccattacttccaggttagctacattaccgactaccaggccatttacctgtaccgcgttggctggttgtaaaccgtttacctggtggtacacggcataaatggttttattatgagaaaacaggctttttcctttcagcagattaaagcccagcacaagtaaggttatacccagcacagttaatacacctactttggtttcgttagataatttgagcatgagattcgtatacgttcacgcaaaaataatcaaaaagcatgcacggaagtggtcgtacgaaaatgttagtaataaaaaagaggaaagcggggtaataagaagggggagggaggaggcagtgtgattagcaggaagttacgaaagcatctttgaaacccagtttgcgggctttgcgcatctcgccggaggcttgttcatcggtcctgaaccggcccaggatatatttgttcagtttttttttattcatcacgatgcgttggcggttcacgtcaccgtggagcttcctgaaaatggaagctcccggtttataaaatttgtcggtgatcatgagttgtacgcagtagctgtcgccgggtacgggggcagacttattgttgctgctcctgttgctggtgtttagcgatgcggtagtgttattgcttttagccgatactttggtggtagctggctgggtgttgcggttattggtaaacctgtcgagttcctcacggtaacgcttaatggctttataaatgcaattggccagttcctgttgtccgttgttggagttgagatagtcttcttcttccgggttgctgataaagcccagttccaccagcacgcttggcatggcggtggcagacagtacccagatgcctttttcatttctttgcctggcgccgcggctgatacgtcctacccgggtaaattcatcctcgatgagggtagagaggcggaggctctggtcgaaataggcatttctcagggtgttgagcaggatgaaggtttcaggatcgtcgctcatcagctgctgggtttcttctgagttggcatcgagtacgataacggagttttgtttcagggactccattttagcgttgtttttgctggtcgcccatatatacgtttctgtgcccttggcattgctcgggtagtaagcgtatacgggttgtttaacggcaattttctttttcccttttttacggtaaacggttttatagtccaccaccttgcggatcttcccggtagaattgcagtggatggatacaaaaagttcccctttgttgtcgttggcaatctgggcttttttgcggggatcgtcgaagcggtcactttttcgtgtatacactacctttacatcgggcatgttttcttccaggatctttcccagtttcagtgccacttccagagttacctgtttctccgtggaatagctgccttttgcgccgggatcttcaccgccgtggccggcatcaataacaatagttcgtataggcttgtcctgtttatcggaaacgggatttgttttggcctgaataaatagggtacaggtgagtagtgttcccagtcctaaaatccaaaatcggttccagcgcatgattctcattttaatgggtgctgtttttcacaaaaaataaaaaaataagtttatctgttaaattaataatctgcttgttccacgcgagtttccgctacctttcgttatattaccttacaaacattacaagttaccatttgtaataaattgtataaaatcttgtaggtttgccgccataacacatgaacgctagctacaaaaataattataaaaagttttttcggcatacatacctggtttttgccggtatgttcgtcgccattccctttattatagatgcagttgcgggtgaaaggccacaagttgttacttattttaacaaaagtttggcagatactactccgctgatacggaaagataccggcaaattaccaaaaccggtacctgtttcccctgtcacagccgattccacccaattaaccaagggtgtggacaccagcggtgaaacgaccgtagataccttgttcgtaccaaagatatcaaaagacacgctggatgcgccggtaaattataaagcaaaggattcaatcatcctgatggtacccgataaacgcttctatttatatggtaccgccaacacaaagtacaaaacgattgacctttctgccgaaaaaatgaatttcgaccaggaaaccggcatcctggaggctaccaacgccaaagatacggccggtaagctgtttggcggcccggtgatgaacgacggcggacaaagctttgaatcggataccctcaaatataactttacctcccagaaagcgaagatttataatacccgctcccagtacggggaaggctacattcacagccagcaaaccaaaaaggcggcggataataccattttcggctttaaaaacgggtacactacctgtaacctggatacaccgcactttagcttccgggcccgtaaaataaaggtgatccccgataaactggtgatctccggcccggctaacctggaaatagaaggcattcccacaccgctgtatataccttttgccattttccccatcacccagggccagcgctccgggatactgccgccacagtacgtggtgaaccagcagaaagggataggcctggaaaacggcgggtactatatcggtttaggggaccatttcgacctgaccatgcgcggggacgtgtattcctatggcagctggagcctcacggccagtcctacctaccggaaacgctataagtacaacggcgggcttaacctgagctttgccaatacccgcttcggggatccggccgtgaaatcagagttcagcacctcaaaggatttcagggtcacctggaaccatagcatggacagcaaggcgcgccccggcgtgaactttggcgctgccgtgaactttggaacctcttcctataacaagtacaacgtgtatgactacaatacacgtgtaaataataatatcggatcgtctatcacgttctccaaaacctggcaggggaagccctacaacctcaccatggggttgaaccactcccagaacctgagcacccgtgatgtgtctatctccttcccggacgccactttcacggtaaatacgatctatcctttccagccaaaggaaatggtgggcacgccaaaatggtacgaaaagattggggtttcctacaatactatcctgcgcaaccaggctaacttcaaggattccctgtttggtaaacaggcgatgtttgacgccatgcaaaccggcatgcagcataatatcccgatctcgttttctatcccggtgtttaaaacctttacgttatccccagggatcaactataccgaatactggtatacgaagaaatttgcccgtaaatgggatcctaacaaatggaacccggggctggatacgcttggtgccatcgataccacctacattcccggattttacagtgcccgcgacatcagcgccagcatgtcgttgtctaccgccatatacggtatgtacacgtttaaaaaagattcaaagatcaaagccatccgccatgtgatgcgccccacgctgagtgccagttaccgccccgatctgtccagcaaatattaccatgagctgcaatacaacaaggagggcgataaacaaatggtatccgactttgacggagccatcatcggcgtgccttcccctggcgcgtttggaggcctgaacttcgggctggacaataacctggagatgaaggtgttttctaaaaaggataccacgggcaatcacgaaaagaaaataaagttgctggatggttttgggatcaacggcagctacaacctggtggccgactcctttaagttgtcgactttcagcttatacgcccgtaccaacctgttcgataaactgaacatctccgccagcggtaacatcgacccctaccaggtagatgcgcgcggccaccgccttgataaatacgtatggcagcagggaaaaatcagcctgggtcgtttaaccaacgccagcatttccatgagtacctcgttccagtcgaaagataaaaagagccaggagaaagaacagaagatcgattccatggagaatgtacagggcgctgacgccgcttttgccgcgcagcagcggcagctgcagatggtgcgtaataatcctggtgagtacgtggatttcgatattccgtggcgtgtggatctttcctatagcttatcttataccaataccgttattcccgattccgggggcgtagtgaaacgtattacccaatatgtaagttttaacggcgacttcagtctcacgccaaaatggaagattggtttgaacagtggttttgactttaccaatatgcaggtggcctatacgaatatgtatatctcgcgcgacctgcactgctggcagatgtcgatcaacctgattccgtttggtacgttccggcagtttagtattaccattaatccgaaagccggtattttgcgtgatttgcggataaaccgatcgagacagttccaggatttataacgaaagcggggattgccattggcaatccccgctttcgttatattactttgtgttgttggccaggtaataatcccacatcaggcggaatactttttctttaaaagcggggaggtcatctcttgttagtcctgtagtaggcaggggaggcaggaaatgataatcgatgcgatgcggccatgcgaagaatttctttcctaccggtaatatttttttggtgtgaaacagtaacgacggcatcaatggcacctgggtgtctatcgctaatgcaaaggcgccgtcataaaaatcctttaaaggctgatctgtgcggttgcgtgtgccttctgggtaaagcaggatgtgtatgcctaaactgagggcatgtttcatttcaacgatgctttgtttgcggcttgcttcactgctgcggtctaccaggataccacctatacggtacagcacaccaaacagcggcactttgccgagagatgcttttgcgagtgttttattgatgccgggaatttctgcagatgttaccggcacatcgatcagcgagttgtgattacatactacgacataggtttgtccgggtgcaaaatattccagtccttttttgcgtacagggcagccaatcagtggctgatacactttcatccatatcctgccaaagaacagaaatccttttgttctacgtggttccggcaggtaagaaatgatccataccgggatgaatattaccagcattgttagtgcgaacatcactaacatccatgctgcgaatattctgccgaagatatttttaaacataaggttgttttttacagtctccagtctaccggtgctattcctgcctttccgagtatttcatttgttcttgaaaaatgcctgcatccaaaaaatcctttatcagcgctgaaaggagaggggtgtgcggcctgcaatatatgatgtctggtagcgtctatcaggtattgtttatcctgtgcaaagcggccccagagcaggaataccacatcgctccgctgatcggaaattttgcggatcacggcatcagtaaaatcgccccaacctattttactatgggacgcgggttcaccggctcttacagtaagaaaggcgtttaataacagtacaccgtgttccgcccatttggtaagattgccgctggtaggtatttccagcccgagatctgttttcatttccttgtaaatattcacaagcgaaggaggaggttttacgccatccggtacggagaagctgagtccatgcgcctgtcctgcaccgtgataaggatcctgaccaagaatcactacttttactttatctatcggtgttttatcaaaggcattaaagatcaggtttccggcaggataaattactttacccaatgccttttcatgtttaagaaacatgacgatctgatcgaaataagacttatgaaattcatctttcagcgcttccttccagcttgattctatttgtacatccatagtgttcacgtcgatatttaaagaaaaataaattaaatttgatttattgggagaaatttacataaatttgcactcccaaaatgcgagttaaatatagtaatttatttcacatttcaagggaaaacaaacacataagtcttggtagctcagctggatagagcaactgccttctaagcagtaggccattggttcgaatccaatccaggacacagaaagaggaaaattgcttttgcaattttcctctttttagttttagtataattgcgtacaagcatgtttgtgccatagcgtaaacaatagtgccggtaacacgcacgaatgctgtcttccattttgcttcgtataaccgttagcgatatattacctggcggtatccttcagccagggccggcgaccagcttccagtataggcaggttggcctccgtaggcacataaatcaccgcctgcggatttttctcaatgttatcgatccacagccagtggagataggcttcattgttacgcagcgactcaccaatgatctggttggagcgggccacgccatgcgcccggatggtatctgcggctgccagcatggcggcgctttccattttggcgcgggcttcagccacggctacttctttggatgcctgtgcatgtgccagcagtgcttccccttccatgcgctgggagtatactttgtattgcggacaaccccacaatccaagtataatcaggccggcaaatactaaaagagcaaaagtagtgagtgaaataatggattttgtattcatagaggtaatgtcctgtaccgcaggacggggtttggtttggggttcaaatatagttatatattgtatatggatgggcggctttcacggtaaggcctatccggtaacgcaggattttctctttttgtatacttcttctccttcttcaccgtttattaaaattatatttgtagcgttttattttgccattatgatcgcatccatattaaccaggcttgaatcttcccggaaagagttactggatttaggtctcagaaatccattgttgaattacaagttgccagccggcaaaggtttacatattgtagaagaacaatctgctgccatttatgatatactggtgcgggaaggtaaaaccatgtcgttcctcggcaggcccgaaaaaaagcaggaagaagaagccgtgcagtataatgaaccggtatcgaaagatgcgttaaccgatacccgtttacaaaccaatgaaaaccaggtaaccctgcactcccggctgctcaatacctactatgccgcccggatgagcatggaagagcagggggtgaacattctttatatttccctggggatgttgcagtggtatgaggccgctggcagcgaagaagcgcggtttgcaccgctgatcatggtgccggtgctgctggacaggtccagcgcgcgagaacgtttccggttgaaatactcccttgaggaagtaggcgccaacatttccctgcaggcaaaaatgaaggccgactttaatatacatatccctgatttgccggatgcggaagactttgatgtaaatgcctacctggcggaagtggccgcggcagtggagcccatgcagggatggaaagtggccgccgatacagtggagctgggctttttctcctttggcaaattcctgatctataacgacctggatgcttccaaatggcagcaggaggatgatattataacgcacccggtgattcaaagtctttttggcggcggattttcagatactgctccacaactgccggatgatgtgttcatcgacaacgataccaatgcgcatgaactgttccaggtagtggatgccgacagctcccagatcatggccatgctgagcgtgcaggaaggccgtaacctggtgatacagggcccgccgggaaccggtaaatcacaaacgattaccaacatcattgcagacgctattggccgcggcaaaaaagtgttatttgtggcagagaaaatggcagcgctggaagtggtgaaacgccggttggataatatccagctgggagaagcctgcctggaattgcacagtcataaagccaataaaaaagaactgcaccaggaactgagaaaggtgctggaactggggcgcccgtctatccagaagttacaggaagaagtgttgctcctggataattacaagaaagaattgaatgattactgtcttgcagtgaatggcgctatcgaaagaagcggtttaactgcccaccaggtaataggttacctgctacggctaaacgaagaaactgcaggtatcacattaccgcatatacaattgccggatatcgcccgctgggatgctgctgcaatgaacaaggctaccgcaatggcgttgcggatacaggcctgtttgcaggaaacaggtgtgccggccaatctcgctttccgcggcagccggctcacggtattgctgccgcatgaacaaactgctcttgcccggctgttggcagatgcattggccgcccaggaagcactggtgcaaacgacttccgcgatcgcaggaaaaatgagtatcccatctcccaaagatattaacgcggtacatacgcttattgatatttgcgcgctgctggcgcgtcaaccggatctgaaggaaatagacgttgccaataaagcgtgggtattgcaaaagcaggatatcgtggaatggctgaccgcaggtgtagctgctactgccgttcagcagcagtaccaggaaatctttattcccgaggcatgggagcaaaacgtaatggagatccgggaaaacctgctggcacatggccacaaatggtacaagttcctgattggcgcgtacaaaaaaagtaaccggcaactggcggccttatgcaaacacgcgttgccggacgacaaggaagaaaaattgcagtatgtggatgcgatcatggaattccgccggcaggatacactgctgaaagaacatgctgctttagccggcaccttgttcggcagccgctggcagaaatcacataccgattggccagcgctggaagaagcaacggcctatttaacggaattgcatacacgtatttcagcgggcagctgtcctgcgcaggtagctcaatggttacacactcaccgcaacgccgccgatgcccttgcagatcagcagcagcttacgcaattgctggcagcgcagcagcaacgcaacactgcggtgctggagaagctggaaatgccgccgggacaatttcctgtgctgctggatgtacagcaatggcagttacaaacatggacagataaactacccgaaatacaccacctcattgcgtggaacaatataacggaaacggctatacaggaacagctgggatgcctgctcacaccggtgcaggaatgggaaggcggtgcaagattactgagaacagcgctggaaaaaacatggtatgaatacctggtagaaacagccgtaaaatcgcagcctgcattgcgtaaatttgagcgtgcaggtcatgaagaaatggtacagcagtttcgtaagctggacgtattgaatcttcagtataaccgcgcccgtgctgcgttacagcactgggaacaaatgcctcgcgcagatgccggcggacaggtaaacatcctccgcacggagtttaacaaaaaggcgcggcatatgcctatccggaaactgatgcaggaagcgggtttggcgatacaggctattaagccggtatttatgatgagcccattgtctatcgctaattttttaccgccggccacattggaatttgacctcgttattttcgatgaagccagccaggtgaagccggtagaagcgctgggcgctattttgcgcggtaaacaactggtggtagtaggagataataaacaattgccacctaccagcttctttgattcccttacccgggaaaccgatgatgaagaaaatgttaccgcagatatgcagagcatcctcggtttgtgcgatgcacagggtgcgccacaacgtatgttgcgctggcattacaggagccggcatgaatcgctgatcacgttgtcgaatcatgaattttatgagaataaactggtgatatttccgagtcccggtgataaagaaagaaaaggactggtatttcatcacctgaaagatacggcatacgaccgtggtaaaacccgcaccaaccctaaggaagcggaaattgtagcagatgcggtaatggaacatgcccgtaaaaatcccggaatgagtttaggggtggtagcgtttagtacctcgcagcggcaggcgatcagtgatgcgctggaattgcggcgccgtaaatcacctgagctggaatcatatttcatggcgcaccaggacgaacctttctttgtgaagaacctggaaaacgtgcagggagatgaaagggatgtaatatttatttctatcggttacggacgtacggaggaaggatatgtggccatgtcttttgggccgctgaataacgaaggcggggaaagaaggctcaatgtactgatcacgcgggcgaaaacgcgttgcgaagtatttaccaatattaccgccgatgatattgatgtgaacaggaccaagagctatggtatacaatcgctgaaaaatttcctgtatttcgcacagcatggcaagctgtacatgaccgccgaaacagggcttccggcagatagtccgtttgaagaaaatgtggcgtttaaactggaatcgctgggatatattgtacgcaagcaggtagggtcaaaaggattttatattgacctggctattgtagatgcagaaaatccgggccgttatatattggggatcgagtgcgacggtgccgcttatcattctgcccgttccgcccgtgaccgtgaccgcttgcggcagcaggtactggaagccgttggctggaagatccaccgggtgtggagcaccgattggttccgtaatccggagcgggagctgaaccgcctggtggctgctattgaaaaagcaaaagccgctgttgcgatcgacgaccaggtagccgaagatgcgaagaaagaatccccgcaagtactgacccgggaagcagtggaagcaaccgaagaagaagtgccggcatatgaaaccgcagtattaccggatgaaatccgggcgcaggaatttcatctgtctcccattggtaaactatgtaactggatagaacaggtagtaacagtggaaagcccggttcattttgatgagttagcccggcggatggtagaagcagcaggtattaccagggtgggaccccgtatccgggaaatactgcgtcatgcggtacgccattccgatgccggcaaacgcataaaaattaaaggacaattcctttggcatacttcattgcctacgcccgtggtgcgcaaccgcagccaactgccggccgccgccaggaaaatcaactacatagcagcagaagaaataggcgtagccctggaaaaagtggtgaaggatgcggtggccatacaacgcgaagatgccgtgcctttcattgccaggatgttcggctacagccgtgtaaccgaagaaatgaaagaagagatcctgaaagcgattgatctcagcattgaaaataaccaggtacaacgggaaggcgaactgctgaaggcatgataccgtacaggcgctgtactgaaaccggacaaatttaaattaataatatctgtttagcgttggtatttaggatacatccgggatggcatgtttttgcttttcaggtgtggagaagagaataatgtgagatagttatcaactttaaatttctcccgatgtttcaaaatcatctcctgatagcatggcgtaacctggtccggtttaaatattattccctgatcaatattgccgggttgtctattggcttggccgcctgctggttattgttgctgtatgtacaccgggaaaccagttatgataatttttatccgcaggcggatcgtatttaccgggctgttaatcatgctacgtggacaggcggtaatttgcacctggctactacttccgccccatttgccgcggtattgaagaaagactaccccgaaatagaacagataacaagagtagaagccgatggcggcgccgcattgaaatatggcgaaaagaaactggaagtaggggatatgttttttgtggacagcaccttttttagcgtgttcagtttcccgatagccgcaggggatgcttcttccgccctggcccaacccaattcgctggtgctgacccggagtcttgctcaaaaactcatcggcagccctgaggaggcgataggaaaaaccatcctcacggatgacagcactgcttatactgtgagcgcagtaatggaagatgtgccctccaattcccatctctctttcagcgcattgcgcgtaatgccgccggactataacgctaacggttggcagaacttcgacgtatatacttacctgttattgcagaaagatgcggatgcaaaatcgctggaaagtaagctgccggcgttttttgagcggtatttaaaaccgcgtatgggagaagtaacgtataaaatggaactgcagccggtgacagatatccacctgcattcccacctcgattatgaaatatcgccaaacggcaacatgctgtacatctatatttttctttgtattggtttgctgacgttgctgattgcctgtattaactatatgaacctggctacggcccgcgccagcgcgcgcataaaagaagtaggggtgcgtaaaagtatgggatcgggcagggaagaaattgcgcgcctgttcctgacagaatccatgttgcttactttctttgccgccctggttgctgtgggaatggtagcggtattgctgccctggtttaatgctttcaccggttcgcaggtacagttatggcagttcggactggcaaaaaccatcgttgttattataatgctggctttactcaccggtctgttggcaggtatttacccggcggtgtttatgtctggttttaaagtgatcaattcgctgaaagggaagctgggaaacagcggccacgctggtttccggaaggggcttgttaccttccagtttatcattgcgattattttaacaggaagcaccatggtggcgtatgaccagctgcagtatatgatgcataagaacctgggtttcgacaaagaccaggtgttgtcttttcatatacctgatcagcagatgcggagtaaaatggcggtgctgaaagaccagctgttgcggaatccgctggtgcagcatgtagctgcggccagtaatccgataggcaggaataatattggtggtcacggctttttctttgagcagaacggcagtatttccgaggcgtctgtagttgcgcagaattatatggtggacgcggattacctgaaaacaatgggcatcaagctgcaaagcgggcgtaatttttcagataccggtgaatcggatatgcatcattcggtgctgatcaatgaaacgcttgtgaaaatgctcaactgggatcagccactgggcaagcgggtgcagtttaagattgacgccgaagggaatcgtaccgagcgtgtagtggtgggcgtggtaaaagattttcacatctattccctgcagcataaaatagcgccgctggtgctggagatgccgccgttcccgggtgcgcaggacaacgtatacgtgaaggtgagcaggtccaatgtaccggctgcagttgcctatattgaaaaagtgtttcattcctttgatcccgggcatcagttcgattatagttttatagatcagaatttcgccaggcagtatgccggtgagcagaagcaggaaacgatatttatgttgtttgcaatgctggcattatttattgcctgcctgggactctttgggctggcggctttcacggcggtacagcgaacaaaggaaataggcgtacgcaaaacgctgggggcttccaccgcgaatattgtaaaattattatcgaaagatttcctgcaattgttacttattgccgctgcggtagcattcccggttacctggtggattatggaccggtggctgaataatttcgcttatcatgcgggcatcagcatctgggtgtttgtgattacaggcagcgcggtggtagtgattgcgttggcgacggtgagttttcatgcggtgaaagctgcgatggccaatcctgttaagagtttgcgggctgattaaaagaaggcgccgggtaagtaattgcccggcgctgcattacattaagcggttttaaaacaccgcatactgatacttccgttctgtatttcttcgtacgtgaattttatttcctcatttttatttaccagtcccagtgtatagatcattgggagatagtgatcgttggttgggatggacaattgcgcttcccggccgagcgtatgataatttaccaggtcggcgaaggcgccctgttccagtttctgtttcaccgtttcatcgaaggaaagggcccagtcgaacggtttggcattgtctgtaaacactacctgccggagattgtgcacaatgttgccgctgcccatgatgagtactcctttatcccgtagtgctttcagttctgccgccagtttgaagtggtattccggtggctggtgataatcgatgctcagctggaatacagggatatcggccataggatacatatgtttcagtaccgtccatgagccgtgatcgaggccccagtggtcatcttctataacattagtggaagtgatgagctgtttggtttcccgggccagttccggtgcgccgggtgcggggtattgtaccgcgtaaagtgcttccgggaatccgccgaaatcgtggatggtttccggttgcggggctaccagcacgtgggtgcctttggtgagccagtgggcggatattaccaggatggcgctaggtttttgaggcaagtcctttcccatgctgctgagggcgcgtgtaaagggattgtccatgataccgttcatggggtttccgtgcccgataaacataacgggcatgcggacgctgtttttaaattcgccggtaatattcctgagatcgttgagttgcatgctattcctcctgatggcagcaatgccgttgatgataaaatttatgcgaactggcgtaagaagtccgccaggcttgttttgtccagtttaagcagcagtgcgccttcaatttcctggtaaaggttgtccagatgctggttgatctgtttccctacgaggcagtcggggttgggcttatttttgctatttcccagcagggaagcctgttgtacggcgtggtatacttctgagagccggatcttatcggctggttttgccagggtggcgcctccgtttttaccttccttactttctatgagcccgtggttgcggaggttgctgatttcctttcgaaccagtaccgggttgatgttaatgctgccggcaatatagtcggacgacaacagttccccttccgcgctggccatcagcgtgagtatatgcagtgatatgggaaatcttccgttgttcattctgtaatcgactttattacagtacaaaagtacgataataggggagaatggaaaaatttatctgtgggtatagaagtaaactacgctggcaatgatgagaaccagtacgataagggcaattacgcagccattccggctgggttgcttcactgcactggctaccccacgggcgccaataagcgcctccacggcctctttagcttccagcaggccaatattggtgccggggagcttgttcatttctgtcaggtagtatttaacggcatgcaattttccggaatgcaggctcagttgtatcgctttttcctcgatggtacgtttagtaatgatgtttttccggttttccggggttgtttggtcgttcactaccttttgacagctttggcagataaacagtacgtgaaatgggtctttttccggtatggtacggataagatccgtgctcccacaccagggacatacttgtacagtgctcattaatggtggaactttttattaactgctgcataagttaataaaagttttttaggattcagcaataaatgcggtagaggggaggtcgacgatgtttgtctgttacttcaccaatacttctcagatgcctgatgcatgggtaagcattgcctaacccatgcactatgaatactgttctcatgcacttctgatgcacttccaatgcactatcaatgcactccccatgcactatctccccttagggttgctttttcaggtgtccggcaaatgcttttttgaacttctccagtttgggtttgatcacaaaagtgcaatatggctgtgatccgttctggttataatagttctggtgataatcttccgcctcataaaaggtagtaagcggcgcaatttccgttacaataggtttgtcgtacgcgccggattcctgcagtttcttcttataaaacgctgctttctctttctggtcctcgttattgtagaagatcacgctgcggtactgggtacctacgtcgttgccctgcctgttcagctgggtggggtcgtgactcagccagaaagcctgcagcagttcttcgtagctgatctttgacgtatcgtaggtaacgcggatcacttccgcatggccggtagtaccggtacatacctgctcgtaggtagggttgggtacatcaccgccggcatagccggattctactttagttacaccgtccaggtattgaaactgagcttctgtacaccagaagcagccgcctccgaaggtagcggtagccgtttttccattgttggttacttccatatctccgggcactttgtcttttttttgctgggcacaggcagaaaacgccattgcaatcaggcaaatgaatattgaatattttctcataaaaataaaaatttcaaagatgcagctttttttatatgtccggaatgtaatgctgttaagggattgcagctattcctggcatctttaaagagcctttcctttttataatttacgtaatatatgatggaggagagcgacaagttaagtaactttaacattcttttgcagtttccaggaacccaggagcgccctgaaaaccgcccaaaagcatacgtcagcagcagcaggaaccgatagtataagccggaattgccggataacgtttgatagcataatgacaacaaagatgaacaagaattaataattttcccggatcagctttctccgccaccatgttggcagcgcttttacgcgcacatgaacgtaaaccttttacgcagacacgaacaatacctgattgttggtgccttcttactttaaataaataacacttgaaatattttcctgaatctgcgttgatgcagttggaattcgacaaagtacaggcattgctgcaagagcattgcaaaacagagctcggcaaggaaatggccgcagcgctccgcctgcacacgcatatagattacgtaaaaaccgccctgcaacaggcacatgaatataaacaactcaccctgttacaggaaaattttccgaacgatttcatcctgaaccttaaaagagaactccgcctgctttctattgaaggcgctgtactaaccggggaacaggccatgctgctgcgtaaactggcagaaagcatgcatagcattgtccgtttctttgatcacgaccgccgtacccagtactccgcgttgtatgaagtgatcaaagaaacccattacgagaaaaagatcaccgctaccattgatgaagtgctggatgaactgggacaggtaagggataacgcttccccggaactggcccgcatccgtatttcgctgtaccgcaaacgtacagagctgcgccgcgtgtttgaccgtatcctgcagaagctgcaaaagctcaattacctggccgaccaggaagaggctttcctcaacggacgcagggttgtggctatttacgccgaaaataagcgcatggtaaagggtattattcatggcgaatccgatacgcggaagacttccttcctggaaccggaagaaaccattgagctgaataatgatatccagtcgctcgaaagggaagaaggacgcgaggtataccgtattctcaaagcgatgacggccgcattaagtggtttttcgtttttgctgaacggctaccacgaaatcctgggtactttcgattttatccgggcaaaagccaggctggcgctggatatggacgcaaactatcccatgctgctgccgcatgcacagcttaatcttatacaggcttatcacccgctgttgctgctttataacaggaaaaaccagaagcctaccatcccggtaagcatcaacctggataaagatgcgcatatcctggtgatcagcggacccaatgccggtggtaaaacggtgaccctgaaaaccatcgggcttattcagctgatgctgcaatcgggactgctggtgccggtacatccatcgtcccagatcgggatcttcaaacaactgatgatccatatcggggatacccagtcgctggagtttgagctgagcacgtacagttcccatctcaaaaacatgaaatatttcatggaaaacgccaacggcagaacgcttttctttatagatgaactgggaagcgggtcggatcccaacctgggcggcgcttttgcggaagtgatcatggaggaactggctaagaaacatgcgtacggtatcgttaccacgcactatctgaacctgaaagtgatggccaacaaggtaaaggggatcgttaacggggccatgggcttcgatgaacaaaccctgatgcctatgtataagctgatggtgggtaagcccggcagttcgtataccttctctattgctgaaaggatcgggttgcatccgtcgctgattgcgcgcgctaagaaactggtggatgaggggcatttccagctggataagctgctgaacaaagccgaacaggatctgcagaaagtagaaagcaaagaaaaggaactgcagaagttattgaaggaaaacgagcgcctgaagaaggaatatgaagtgctggccgacaaagagcgtaagcagcagcaatatgctttactgaagttacagaaccagatcaaggaagatgacctgcagtatctgaaggatatggagcggaagctgaagcagatcgtgatagagtggaaacgtgccgatgataaggagaaagtaatgaagcaggcagaaatcctgttgttccgccggcgtgaaaagcagcatactgaacaactcaacaaaaaagtacaggacaaatttgaggagatcaaaggccagatagaggtaggcacccaggtgaaaattgttaccaacaggcaggtgggcaaggtattggagatccgtgataaacgtgctattgtcaaaattggtaatattcctatcaatgtgaagctgagcgatcttgtgctggtgcaggaaaaacctgctgaaaaggtagaggaagggaaatgatataacggataccctgaggtggtatagagattatctataggccgtatagttggagcaagattatttaataacctatctttaccgcgtcaaaatttaaatggtggttaccgtaaaatattaaaccaatggaagtattagaacgtgttgtaacacgcaattcggatgtacaggtttataactgtgattacgcagaaggggccaactttttcatgggggagtggaatggttatgagtgcgcaggtgatctgaacattccgcatcgtcacaatggatatagtatagatatattgatcaagggccgcataacgcaggtgattgattttaaaaaatacgagatggaagcgccggcgctcatgctgatggaacctaaccaggtgcatcagcatgagatggatcctgatgcggagctcattaatctttacttcaccaacgacttcctggtgcccgaaatgcagggagtggtgagctgctggcgctgtgtattcagctccggtatggttccgctgaacgaagagcagctggaggaagtattgtcttatgcagatttgatcaggaaagagtataacagcaacaaattacgcaaggatgccatcatccgtaacctgttgaacgcttttattatagcgtgcgggcgtatttctgaaccttccggtaactggatgaatgcagagagttcgcaatataatatggcgcggcagtttaagatgctggtagatcagcattttcatgagaaagcgcaggtatcggattatgcagaaatgttgtacgtttcaccgggacatttaaatgacacggtgaaggcgttgctgggaaggaatgctaaattcatcattgacgagaaacggatcatggaggcaaaacgcctgctgtactggggtgagcactctattaagcagattgctgcgcagttgaattttgaagatgatgcctattttaaccgtttctttaagaagcattccggattcacgcctgcatcatttcaaaagagtatccgtgaaaagtacaattaaacccgtaataatttaaacgtgcgttaactttaaatatctatttttgcattgtgtttaaaataatgatgtcgcccgtgcatcattctaaattttgaaaaccgatgagaattttttagcggccgaccgcaaaccttcaattttcttttttacagtagtaacaaattgctgtgctcaaacgtataatgtgctgtaacattataggtgtctgagtgttgcggggctacctacctgtatttcacaacccgattgctgtcactgatattgattgctgcgaagcaaggctgccttttattggccttgatcgtaccggggaattttattgttagtcgtttaaaacaaagtagtatgaaaccatttaaatcaacgtttacaaatttgccggcaggcttactttatagtttttttgttctttccgtattgtctgcctgcagcacatcgcaggcaaagaatgaggctccgccaccagcatctttacctgtaattaaagcagttacattacctgctacaacctttcaggatttccctgcttcggtagaaggaacccgtgatgtggaaataagaccacaggtagatggctatctaacgaatatttcagtagatgaaggtgcttacgttagaaaaggtcaaacacttttcacgatcgacagcagaccttatgcagagcaactcaacaatgccactgcaaatttacaagctgcaaaagcggcattagagaatgcacaaatcaatgttgataaattgaaaccgctacttagtaataatgtggtatcggatgttcaattaaaatcggccgaagcaagttacaattcagcgaaagctaatgttgcccaggcacaggcccaggtagaagccgcccgtatcaatcttgggttcacaaatatcagcgcacccagcgatggttatgtaggtagtattccctttaaaacgggaagccttattagcaggggaatgacaggcgcattgactactatttctgaagtaaaggatatgcgtgtttatttttctttgagtgaaaccgatttcctcaaattcaaggaaaaatatccaggtaatagtgttgctgaaaaagtaaaaggaatgccaccggtagaattaatcctggcagatggaagtgtttatcctgaaaaaggaaaagttgaaatagtggaagggcagtttgacaaaactattggtgcaattagtttacgtgccagctttcctaatgcacaaggagtacttagaagtggtagtaccggtaaagtcagagtacctactttacatgcttctgcattggtaattcctcaggaagctacgtttgaattgcaggacaaagtgtttgtttatacagtggccgatagtaataaaatcgttacaaaaccactaaccatttctggcaaaacgtctaattattattttgttactgatggcgttaaggtgggagataagattgtattatcttctcaatctaccatgatgatgggtggtttaaaagatggtgttgttattcagccacagatggtatctatagatagcctgttgaaagcaaagccgctgctttaaaatagttaagcgtgaaagcacgccagtgttaagaacgtttacacaaaacattattcaaattgtgacgcaggcagtgttgttacacacatgcactgtttgtgttcgtgcggacataccgcaacccataattgttatttatgttaaaacgatttattgaaaggccggtgttatcaacggttatttctatcatattggttatactgggagcgttgtctttattctccctgcctacggccttattccctgagattgcgccgccatctgtacaggttatcgccaattaccctggcgccaacggggaggtgatagcccgtacagttgctacccccatagaagaatcggtaaatggtgtggagaacatgacgtacatgacctccaattccaacaacgatggtagctacaccttgacagtttattttaaacaaggaacggatcctgatattgcggcggtaaacgtacaaaaccgcgtatctaaagctaatagccagctgcctcccgaagtattacaggctgggctttctacacagaaagtgcagagcagcttcctgatgtttgtggcgatatatagcgaggatagcgttaagtataacgaactgttcttaaataactatgcaagaattaatatcatccctcagttacaacgtataccaggggtggcacaggtacagccatttggttcaaaagattattcgatgcgtgtttggttgaaacccgacaggcttgttgctaataatctttctacaacagaagtgatgaatgcgatcaaagatcagaacgtagaagctgcaccagggcgtttgggacaaagtagtaaagaatctttcgagtatattattaagtacaagggaaagttgaacaagcctgaagagtatgaaaacatggtgattaaggcaaataacgatggttctgttcttcgccttaaagatttggcccgggttgaacttggtggttatacttatactgcctcgaatttgctcgatggcaaaccggctactggttttggtattttgcaaacaccgggttccaatgccaatgaaattcttaccgaactggaacgccagattggagaatttgataaggcgttacccgatggtatgaagtttaagatcatgtacaactcgaaggagtttttggatgcatctatcgaccaggtaaaagaaacactgatcattgcattcatcctggtggccattgtggttttcattttcctgcaagatctgcgctctacattgatcccggtaattgctgttcctgtttcgattataggtaccttcttcttcttacaattatttggctttagtattaacctgcttacattgttcgcactggtactggctattggtattgtggtggatgatgcgattgtggttgtggaggccgtacactcaacgatggaacgtgagcatttaccggcaagagaggcaacagttaaaacgatgagtgagatatccggtgcgattgtttcgatcacattggtaatggcagcagtgtttgtaccagtgagctttgtgcaaggtcctgcaggcgtattctataaacaattcgcctttacactggccattgctatcgttatttctgcggtgaatgcgttaacgctaagtccggcgttgtgtgcattattcttaaagaaccagcatataggcgaaggtggagagaaaaaaggttttggtgcccgcttcttcgatgcgtttaataccgcttttaatgcaatgacggcaagatatatacggagcatcaaattcctgctgaggaacagatgggtggccattaccggattattgcttgtggtggttgctacagttttgctgattaaaacaacacctaccgggtttattccggatgaggatcaggggtttgtagttggtattacccaaacacctcccggtagttcacttagcagaacggagaatgcaacgagccagatcagtaaaattacgatgcaagatgcgggtgtgagcgatgtatgggctgcaaatgggatgaacttcgtaacaaatgcgaacgcttcccctaatgctgcgatatttgtacggttaaaagatcgtaaggagagaggtgctgtaaaagacccgactgctattgctggcggtttgttaggcaaatcaatgcaagtacatgatgccctgactttctttgttggttttccaacaatacagggttttggtaatgtgagcggggtagaaatgatgttgcaggacagaacaaacggatcgctggagaaattagcaggaacggcatggggttttattggtgcattaagtcagcggccggaagtggcaagtgcgttcactacttttaatacggggaatccacaatacaccattgatatagatgatataaaagtgaaacaattgggtgtatctgttggtgatttgttgaatacgctgcaaacgtattatggaagtagcttcgtttcagactttaaccgtttcgggaaatatagccgcgtaatggcgcaggccgatgtttcataccggatggataaaagttcgttggatgctatttatgtaaagaacaacctgggtacgatggtaccggtaagtacagtggccaaattcacacgtgtatatggcccggaaacagttacacgaaacaacctgtatagtgctgttaccattaatgctacacccaaaccaggttatagtaccggtgatgtaattaaagccattggagaagtatcgaaaaaggcattgccacaaggatatgcctatgagtttacgggtattacgagggaagagataagagccgggaaccaaactgcgttcgtgtttttattgagtgtattgttcgtattcttcctgctggctgcacagtatgaaagctatatcctgccactggcagtaatccttactgtacctacgggtatattaggtgtatatagtttcattggctttagcggcatagagggcaatatctacgtacaaataggtatgatcatgctgattggattattggcaaaaaatgcgatcctgattgtggagtttgccctacaacggcgaagggcgggctatgagcttgttgaggcggcgttggaagcagcacagcttcgtcttcgtccaatattgatgacttcctttgcctttattgttggtatgttgccattaatctttacgcaaggtgcatctgccaaaggcaatcattcgatcggttggagtactgtaggtggcatgcttaccggggtggtcctgggggtattcatcatacctgtgctgtttgtaattttccagttcctgcaagagaaaatcagccgtaagccgatagtggcagtggaagcagaacatcaggcaaagctggttcattaatagcggcagaaaaatatattatcagattcagaaaaaagacaaatgaaaacaagatatagctcattttactttttgttgttctccttagttgtagggttagcagcatgccgggtaggccgcaattacgagcggcccccggtggcgctgccgcagcagttcaataatgacactgcgccttcagacaccagcagcatagcagaaatagaatggaagaagttttttacagatgccaccttacagcagttgatcagccaggccctcaccggcaactacgatctgcagctggcagtgaaaagagtggaaacggcgcaggcttacctgaaacaggctaaagtggcctggttgccggcttttacagctaccgcatcgggcagtaccaacttcccttccaagaatagttttaatggattgaaccttgctgttaataacctcggcgaccatatcgaagattttaatatcggtgtgggcatgtcgtgggaaattgatatctggggtaagataaaacgtcagaaagaagccgcactggctacctatctgcagtcgtacgaaggcgagcacgccgtgcaaaccgggctggtggcagctattgccaacagttacttcaacctgctgatgctggacaaccagctcagtgtggcccgcagaaacctggcgctcagcgacaccatcgtaaagatgatccgcctgcagaaagccgccggtgatgtaacagagctgggtgtgcaacaggctatttcgcagcaacaaactgcggaactgctgatcccgcaactggaacaaggtattgccatccaggaaaatgcgttacgcattttaaccggtgagctaccgtcgacgattacacgtagcagcaaactgagcgacttccaggtattggactcattgccggcaggtattcctgcggccatgatcagccgccgcccggatgtacgcgccagcgaaatgggactggtagctgctaatgcacaggtaggcgtggcgcagggtagtatgtatcctacgctcactattaccggcagtggcggattaaatgccttcaaagccagcacctggtttaatcttcctgcttccctgtttggtacagtggccggaagtgtggcacagcctatcttccagcgccgccagttaaaaacacaactggaagtagctaaaattcaacgtgaacaagcggtgatccagtttaagcagtctgctcttacagcagtaggagaggttagtgatgcgttggtaaagctggacaaagtaaaggtgcagcaggaaattgctgtccgccaggtaaatactgcgcaactggcagtacaacaggctcagctgctgttccgcagcggtatggctaactacctcgaagtaattactgcccaatcacgttccctgcaggctgaactggcccaggccgatatagaccgccagcgcctcaatgcgatggtagacctgtaccgttctttgggcggcggttggaaatagccactgcaaatgacggatcaaagcgaaagaccatcagctgagtttttgaatcactatacgaaacagatcgcttaggtccgtcatttttatcataccatcccggtttacgcgttgtaaaccgggatttttatttccggaaggcttgctgctggcgggtttaaaaaataatagccgaatttttttttattttcaatttcttttatacttttgcgtccctggagagttggcagagcggtcgattgcggcagtcttgaaaactgttgactgtaacaggtcccggggttcgaatccctgactctccgcaaccacattgttaaaatggttaaagcctgtagatgcaaaatctacaggctttttgtatttagaaaaatgccggataaatgccactgatttcggttaaatgaaagcctgaaggaaaacaaaaatgttacagctactattctgcaaaccgttggtattaaagaacatgatgggatggtaattgcagttgttaacaggtaaatgaataaatagagatatccgttagttatgatgaggtacattgctatcctacttatttcttacaattctcacagcaatatatggttttcccggtaacccgattaagctgtgtcctgaaaatttcttttccaatggtgtgatggtcatattccatgtgtcaatcacttcaacattgtaggatgcgtctgtaggaagatcaataacaatgctccgcggttgtgcatcattcaaataccccaaatagtattcatgttcaatgccgacgcatgaaaatggtgcccacgtaaataaaggaacaggttttaattccccgggcgccgcttcaataatctggcggaggagcttgatccgatcggggctttttcctatcatcacaccgcctttcgaccaccataaaatatcggatgatttaccaggaagccggataggatcttcagtaacataagtttctccatgtcctacaaatcctccattggtaaaacctctccaaaacttttcagtcatggattgagcagttaaattaccccacgaccacggtatgtttccttcatatctgcattcatcaaaaataacaggctttttatatttcgccctgtactcttttgccttataagtgttttcttcctgaatgcttacatgcgtaatgtagggattggtatgatcatagaaccgaacaccattatgaatactaaggaggtggtgaaacttatctttagtagcgaattgctcaatataatagtcccagtcactcattttcttattctgcataaaatcatactcgttggccatgctccaccaaacattcttgaaagctgcgaatcgtgcaatgatgtaattgatataaaggtcgtcggtagctctgtcgagcgaactaaatccccaacggtcgtaaggatggaaaacaataaggtctgcttgaatgcctagtgaatcgagctgctttattctttcttcgatgttcctgaaaaaggcagggtttaatttgttatagttccagttttttagcggtgatccctcaaaaggataatacacaggttcattattgttccagtcatagctctttggaaaaatgcacatgcgcattttattaaaataacccttcgataatgtttggagcgttacttcggccaaactatcaccctggtgtacccagctatagcaggtggttccaaacgaataatgtggggtaccgtcggcatatgcaaaataaaaactgtcttttactgctacaggaccatgattatctttttgcgcgggagtacatacaaagcttccttttttattagtaaggtttttgacattgcttaaagttacatagttccattttccttcgtttggaggcataaacctgattttataaatgccattgccgtcgtaaaaaccaggaacagaaatagtatccttgttcttaataaatctgcctgttaggttcacatctgtaaatggatttccttcagttgacccattaagtattaattcaaagactttccatttttcagtagtatgctgcgcataaagtgagcaattgcaaataagcagcaagaaaaaaatactttgaattttcatacgtgtaattttagtatcattgaaaaaggtaccctacccggtgccagtttgataagtgccgatatttcaattaaaaatgtaaatttagcatcgacatactatcaaaactagccttatatcctaataaacatgtcaaataccgggaagttatatacatttgatgaaggacgaagcgaatttaaaccgtacggtttaacgtgcgaattatggacaccggctttgatgagaaagccggacagacacaatgaagtcgaaataaactatcttataagcgggggtataacttacctttttcagggagctaaaataactattcctgaaaaaagcctgtgtgtgttctgggggctcattccacatcaaattgttgacgctacatgttctgctccgtattatgtatgtactattccgttaacactgtttctggaatggaagctacctgccctttttattgacagcatacttaaaggggatgttattatagaagacccgggagagcattcgttgtttgatacctttctttttaaaaactggttgaaagatctttctgaaaataatgatagagaagcgactttgtatgaaatgcgtgccagattaataagacttgccaccagggtcttacctttaaaacagcatgaacgattgcaagtacaagccggtgaaattgggaaggttgaacaaatggctttatatattgcgcaaaattatatgaatccgcttaagatcgctgatatcggaagagcaattgggttacaccaggattatgcaaatgtgatattcaaaaaagcttttgatacgaccattaatgattatgtaatccaggaaaggatattgcatgcgcaacggaaattaattaccacggataaaaaaatcaccgaaatagcttttgaatgtggctttaactccataaaccgttttaacgcagcttttcggaaaatcaacaaatgtacgccgcgggaattcaaaaaaaagaataccattaacaacgcaaaccaggatggaaatgccgctgaacgcgcgtgagcaattgttaatagttcccccttcgatattacgatatcagaaaatgcttctatggtggttgaaatcatgttatcaatgtttacccgacagcatttttacaaaaaaagcttaaatgaataattttaagataaaaatcaactatctgacactaagcgcatgcctgtccataataattggacagacatgcgcgcagtcgtccgttcagccacttccatacatcctcgacatggtgcataataaccccggagaagcaccttatgtaacaaagtataatgatccggtttacatgaaatcgcaagggtttaatggaatggtaacccattggtttgttaattgcgccatcacttacgataactatgaaaagggcattatccctgaaaacagtaaagagcgcgaatggattatggcgaaagcaacggatatcgataaaaagctgatggcctgtaagaaggccggtatgcgtgtttatccatttaccgatttcattgtttttccaaagtctttatggggaaaatatggcaatgaaataacaggtaaaggcaaggtagccggtaccggaggcatggacgaacgatcgagaaagcccgatatgcaaagcaaaaggacacaggatatgcttcgtgcacaaatagccggcatatttgagcggtttgctcaactggacggtttgacgcttcgctttggcgaaacatatttgcaggacgccccctaccatatgggaggaggacccatacgtgatggtaagagcggtatagaagatcaggtgacgctgataaaccttttacgggaggagatatgtgtaaagcgaaacaagaagctgttttatcgtacctgggattttggatataatttccataacaaccccgattattatctggcggttaccaatcaaataaaaccacatccaaatttaattttcgtcattaaatatcagcaagacgattttcaccgtatgacaccatttaatcccaccctcgctatcggtaaacatgcgcaaatagtggaggcgcaatcaaggatggaagcttacggaaaaggtgcgcatccctattatacggcccaaggtgtcatagatggctggccggagacgaaatatgaaattatttttgggcgacatgaattcaacggaaaactgaacgatcctgacaacccgcggggagtaaaagatattttaagtaaaggattattaaaaggagttatgacatggtcaaatggaggcgggtgggacggaccgtatatcattaatgaattatgggcagatttgaatacatacgtcctttcgcaatacgcacagcatcccgataagtccgaagaaagaattttttatgagtttgcccgcaagcttggattaactggttatgaggccgatctgttcaggcaattaaatctattgactatagagggagtgcggaaaggacaattgaacagttataccgctaacgccgtttggtggagtcgtgatcaatatttttcagcggcagaaaacaaaaatatagttaatgaaatcattaacaaaggaaaagaaagagaagtgttggctgaaaaagcggaagcttcagccatatggaggcagatcgaagcgttatcgaaacaaattcatgtaaacaatgcagcagatcaggaatctattgaagtgtcgtgcacttatggccggataaaatatgaattgattgagcaaatgtggatattgatgattgaaaacggcatagcaaaacggaacggcagtttcaatataacggcgattaagcaggccattaaccgttacgatcttttatggtcggaatggaaggctttaaaattatccagtaaatattgtactactctttatactgatttggcttttagaaatcaacgaaacggaagcataggagagctggtcgacagtttaagaaagattttatgacgatcgttatatctatgatctagatcctttggttgctggattcctgaaacttttagaggatttgaggtatcacacataattattcgagtgtaatgggtttgtctttccttttaaaatcaaaccacattaccttatcctgcgcagctgatttcaggtataaaatattcttataaaaggcaaccccgcttccagagtatattccagcatcgaaatccttatctttctttaaacggttgtgaaccgcattaaagaaggacttaatcgtgggcattggatttttactaattaaacgcagcgcaagcaattctacatccgtatctgtttggcggccccctttgccttcaatgcaataatcaaatacgtcatctgcataaaaattcgtgtcatcattcagtgtaacttcctgagcgctgaagaaaaactgactatagtccctatccggctggtcagcaaaaacatccagtttaacatactccgcctgcaatgctgcatctcttttttccagataaagatgcacctggtatttctccatcaaatctttcacccatccacaaatacatcaaacggaacaatcacatttattaaagaagccataaattctataaaaatttatatttaaaatatcttacaccttaactaaagttaaatatttctattgttaatcatcctacggatagcagaagtaaactcaattagggattcaggctacacatttgacggtttaggctaagctatgaccgatgcctttgtcgacctttgtacaatggaaaacaaaattaaaggaaaagtagtcgctataacaggcgccagcagtggaattggtgaggctacggcaattatgctggcagcgcagggtgcaaaagtagttttaggcgcccgtcgtaaagatcgattagaagatttggttggccggatcaaagcggcaggtggcgaagcagtttatttagtgacggatatcaaaaaccacggtgatttagtgcaattggttcatttagcctgtgaaactttcgggcgtttggatgtgatagtaaataacgctggaattgcccgtttgtcgagggtcgacgctgttcaggtcagcgattgggaagagatgattgatgtcaatctcaaaggaaccctgtatggtatcgcagctgccttaccaatttttttgaaacagggttttggtcacatcatcaatatcatatcaacttccggtataaaaattgtgcccctgcagggtgtgtacgccggtaccaagaatgcagtgcgtaccatcaccgaggccatgcgccaggagtcaggcgggctataccgtgtaaccggaatctcacctggtttggttaatacagaactgatagatcatatcaaagacgaagcagccagaatagctgttaaggaaaaggcagcacaaatcgcgatcactcctgatgcaatagcagctgcggtgacctatgctattagccagccggatcatgtggaggtgggagatattgttgtccggccaagtgtacaggattaaacttaatttagcatgaatcatgaaacctgcacagcaacccattatatttaaaaccatttctgaattgatgaggggaatgggtatgcccaaacccctgcatcctttggtggctgtagtaaattacgatgctaccaggatcagccgggaaaacgcaggacgaagttttttgatcgacttttataagatctcctttaaacaaaatttcaggggtcaggttaaatacgggcagggctattatgactttgaagaagggggcctggcttttttagcgcccaatcaactggttactatgagtggtgatgaaagcagttatgagggctatacgctgtattttcatgccgatcttattcgcaattatccattaggcaaaaacatggatcgatatggtttcttcgcctacgcagtaaatgaagccttgtttctttctgaaaaagagaagaaagtaattggtaccctgtttgaaagtattgctgccgaactggataataatactgacgcttttagccaggacgtgttggtttcgcagattgaattgctgcttaattacagtaaccggttttataaccgtcagttccttacccggaaagctgtcaataatgacctgatcagtcaaatgaatagcttcctggctatccgcttcacagatcacatagatggaatacctactgttcaggaggttgcccggcatctcaatgtttcacccagatatctgacggatatgctcaaaacactaactgggcaaagcacacagcagcatattcatgaccggttaatagaaagggctaaggtaatgctaacaactacccgtatgaatattgccgaaatcgcctaccaattgggatttgaacacccacaatccttcaataaattatttaagcgaaatactgctctttcaccaaacaagttcaggcaatcttttaattagcaaaaaaatccctgcttcatccggaagcagggatttgaaagcaacttaaaaaccatacataccacccgaaacggaaatctgttctcccgtaatccaggccgcatcatctgacgcaagaaatacggcggctttcgcaatatcttcgggctggcctctgcgaccaagcggcgtattggcaataaacattgtttcatactcactgccagcagtgacgccggcactacgtgctccttctgtttccgtagcgcccggcaaaatggaattgatacggatgttttttgcacccagttctttcgacaaggaaatcgttatggcgtctaaggctgctttagttgcagagtacaacgaggcggcaggaagcggcattttgcttgcgcccgaactaatgttgataatattgccgcctttaccgctgaacagtttcaaagatgcctggatagcaagtatagcccccaaaacgttggtgttgaaatgctggtgaaagctttctgctgataccagttcaataggcgtgtatccctgaaaggccgcgttgtttaccaaaatatccaacgtgccgaaagccttttttgtttcttcaaacagcctggttacatccgcttccttcgatacatcgccctgtaccggaatggcgatgcctccattgtcagttatctccttaaccacgctatctgcgccttctttacttgtagcataattcacaactacctttgcgccttccgcctcaaaatatttggcgatagatgcgcctattccttttgatgcacctgtaaccaccgctactttgttctttaatctactcattgtttctttttttaatgcttgagcgacaaaggtaggattggtaagttattattagtaacttcgtgctgaaaagtaacagtaacataggtgtaacaaagtaacattatggggtgtaaaatagaagagtttcaacaggaacaaaagaaaagaatgaaagctgttcaggattcaatggacgtgctgaatgggaaatggaagatttctatcatctcatctatttgctgttatggcaaaaggcggttttcagatattttgaatgatgtagaaggaatttccaacaggatgttgagtaaagaattaaaggaattagaaataaaccagttggtaaagcgaaccgttttagatacacaacccataacggttcaatatgaacttacggaacacggtgatacactacaaaccatcatcagcaatctgacagattggggcattgtacaccggaagaaaattgtcgggaaataatataggcttcatgaaccgccgccgggaacgagggtaaaaaatggcgtgcgtgaaagaattaaaaaggagaacagggaaagaaggaaaaacagcagcattggtagtatgcagctgtttgagaactgatcttaaatccctgtcctttaaggcacatcattctgccaatcagagtttggccttcgcatcattcaatagtgacagcaattgaatgatatccccatccttcataaacacataggacttctcatcaaatcgctctatttttaaaaaggtggaccattgcttttttgaataaaagcagcctgcctgcaagccgcggcttttatattcaacttcagtatatacttctggtgtggtcggcattatcttgtcttttataatgtttaaagatttaattagcgcgtcaacctcatctatatcaagcagtcctatttttgtatcggatgaatatgctccggaatacgcatattcaaaacgtactgccttggtagtttctccgccaatcaggtctgtaaattgggcaacttgaatctggcagcccctcagcgatccaacgtccgtaaattgtctttgtattagagacccggatttgtttgagaaaagctctgccttgcttttttgttcttttagatctgtattgggtttcgccgtttgagaaaaagccgaatagaatggggttataattgccaaaattaagattacttttttcatagttgatggaggtttatttaaaagattttttgaacgacatcataacagttgctgctatatacttagcacgtttaagcctgaactttttctgaatcataccaatcaaccgtcttatgcagtatttcttcgaacttaaaaaggtcatcgatagttaaaatctccgtcctcgtttcttttttttgctcgtcaaaagtgccaatatattttcgcacaccgttaaaatacagtctgcatatcgtttttcgattattatcatccaacagtatggcgaaataggattgagcatcgcgatatgctatcctggccggttttatcttttgacggagcatcgtctttacaatcatgtaaccttccttttcctcttcggtggtttcaatcaccggggccttttcttctacatttgttgttgctaattctttttcagcatcagatggcgcagcctcattttcctttttcaacgcagatttaagcctttcagttatcaggtcattaatgtattgttgtattgaccttttggtaagcgtacccagttgctcaacaatttttgacgttaacatccccttatatatctgcttggcaaagagcttgatcaacccttcagaaggattttgaaattcaatatttatcagcgttttgagctcattcatatattttagctcgcttgcagtagtttgaatgctttctatgttgaaatatgacttgtgaaatttctttagttcttcaatctggttatcttttatatctgtaacattaaattcaaagaatggcttttcatccattttattctgctctgccagatctgtataaaaccggtaaattattccattggacaatagtccgaacttagcggctgtagtgtgaaagtaccggaaaagctgggagttgtgcggatccaggctttctccccaatgcttacattcgataagtatagaaggcttgccttctttcaggattgcataatcgactttttcgcctttcttgatcccgatatctgcaatgaattccggcattacttcaaatgggtcaaatacatcgtagcccagtactttaatgaaaggcataataaaagcatttttagtagcctcttctgtttgaatctggtttttaagcttttcgactttgtcgccgaagagtttaatttcatctttgaaatccatcttttttatattaatgttgttggaaatctattactgaactgctttcccgagggcatcgagccgtcgtatctgtaagttcatgtggtgcagcaccaccttttcgtaatcattggatttgtcgctcgccttactgaaaagcaccagcatctctataaacaggaaaaacaggatccacaggcaccagaaagctaatgcaacggacgatgcggataacatatgcatcatgatcgttaactcatccaggaatccggtattcgctttcatttctttttcaagtgcaggcttaatgtggagtaaatcgttttccttttgggctctttgttgccgcatggcgccaatggtggagtcaagggacggtagcaatgctattttgggatttggcaccagcgtagttccaacagtaatgtcacttatcgttttccaggtggtggtatccctgcctgaagatgtaactgttgccacgggtacccgtcttgttgctgtttgcgtagttgtggcagttgtggtggtatgtttactgatatctgcgatgtaattatctttttcctgttcttttttattaatcgtcgtatccagcgctgcaatctgctttcttaattcttcggttttcgagggtagtatactgtcaaccttgttcgaaacgtaggaaattttctctatctcaatatctttttcgaatattatctgatcgatgatcaccgcgcccagaacagacataattagcgccaggcagcatctgaaaaatcgtagtagccagctcggatggatggataagatgatttgcttttcaacctgtacaatgatgacgatggagagaagcccggccagtatgcaacccggtaaactgagtgacaggtaacggtgggcaaaagtaaaaccaatgaagaaccagagaatgcaaacgatcagcatggctgcggtgtactttttcacggatttgaatgcggcttcgctgcagttccgcaggatattataattgtatccggtgaggaagcagccgaaacggatccagagatgtttcatagcgcagggttttaaaggtttttgttcagaatcatgtgactggaaattgccgcaaggccattcctgaatccgcgggtatagctgataatgatgccatgtccgactccctcgttaagctttgcctgttcttcgatttctttgacctgcctgatgtggctttcggcaatttccttttttacggtaagctcttccaccgtatctatcattccgcttctgctcctgctggagatgtggaagtttatttgccggataaagtcgtcgtaaaacgtttttaccttccggattgatctttccaggtcattcttcaacgcgatcacattttgatccaaatgagtgatgtccggatttatcaaagcatcattgtaccctttagactcataattcttgtcgaggaaatcgtatagaagatgtagtccaccattgagcggtgtagcagctttcccgtcaggctggtctcccggtgcatccttctcaatgaaagtagtttccgggatatcgggtattgcgttttcaattgccagatggtggttgtgaccattttgacgttgccggttgaaaatattgaagaggctcatatgttttattaaatagtgattgtcggcaccttatatttattatgccctttattatgacaggattcgcaaagcgtgatgagcaagcgatcggggtactcccagggaaggcggaacttctgctcgcttgctataaactggtattgccggtgatgtacctgcaagtctttgtcgctacggcaatgcacacaacgatgcatatcgcggtgtagtatttcttttcgtcttgccttccagttggggtgaaatagaagggcgccataactgccatgcgatttaacgttcaggaggtcctgctttttaggtgttaccggaggcgacttggcaggaatatcttcctcgatatatctgcgataacattggtctcccttaaactgcaaatatttatacggcgcgtcgtttggagttgtcataatagtacaggttggagtttattgaaatataatttattgctcccacttacaaagggttctggttgtcattgctttttcaagggaaatgctgatgattcggtgcttacaattacttagcccacggcaatccgatttataatgatactttgtagcacttttgctgtcacagacatacaccgttattgggttgcagtgagtatagcttataagcagccaggtatacaggagtttcatggttcgatcggttctgaagacaaggggcacatagaactggcattattgattaagtcgtatgacaaagcctgcaacaatgaatacagccattcgactttttgtagcgttttgttgcttcgcgaaccgcctcctggcaggtttcaaatcctcccagataggtccggttatacatcatgggaaagtattcgcaggtgctgacgtgaacttcatgatcgccgttgagctgggggttgttgtttacataatagttctgtttcatagtgttgtttttaatttatgaaacaaaagtatatttcatcaacctcctttttttatgggaaaccgtaatcagttattttctttcgaaatttcttttgagatgcttatatagcacctaaatccttgcagtgggccaccagttgttcatttttggtaaagccaagtgcatctttcatctgattgagtttcttttctacgctgcttaggccggatggttttatcccgttgcgttgaaggtgcgcgggtatgtctttctgcagcattccctgcgcaagcaacgttatgatcaggatatcaaattctgaaaatgagtaggcgttctttttgtcgatcgactgcctgatatgatatggcaaataacgccggtgctgggctatttcattgatggcttctttaagcgaccggatgtcgtttcggcctttggcgacaaaaccgtctatgtcgtacttgttgtaaagttgttcaataacagccggcttgttttccaatgagaagaccaggatattcagatcgggctgtacttcccgggcagcggcaatcagctctataccaccagataatacctgcttatgatcatcctgaatgaatgataaatctgtaatcaggagatcgaaggagtttccggctttaactgcctgtgtgatcttatacaaagcatcatcgcaataataggcatgtgctatatctgtgatagccaaatcttccagtgttttctgcagagaaatattggcgctttcgatatcttcagcaataagtacctttttaatcataaggattgagctattggaatggaaatgtgaatttttaatcctttagcaggatgctcaaatgtatattgcccgtcaattcttttaatacggtttcccgtattctgcagtccgtttccatacttaacttgcggagaaataccgatgccatcatcggtatagagaatctgaagctggttgttttgacattcgaattttatcatcacggagttggcctggctatgttttttcatattgatcattaattcctggagaatatattcaacttcatgctgagcctgcgcactgatccggctccagagcataggaccgttgccgaagatcaggaccttgatttgttcagatccaaaagattccagcaggttgtcaattttaacgtgaaaagggatctttgagatagtggggttttcgtaggagatatcgcgggactgctcatacagcacctcgatcttatctattaattcctcctgatctacagacgctttatgctcaagttctgtcatgatgcggtacaagccatttgctaccacgtcatgtactttctgggaggttttaagctgatattcctgtattgcctgccgggatgcaaattcaatttgttgccggcgccggcggtaccgaaggattaaagcgattccggcgataatgaagagcaggatggttagcgccagtatgaaccgctgtactaccagctgggttttcttttgtgcattatctttttgcagctgaagattgtcggctttgttttttgcggcttcataccggattaatgcaaattggttcttcgcggcgttcttggccgtttggatactatccgtcaggtgttggtagcggataaaatatggtttcagcaggttagtggggctgagggtaataagttttgaaagtgcttcgacttcgtcgtccggactgttcatttccctggcaatttcgtaccttcttaccgcataatgaagcgccgaatcggggagggagagcgaataatagtctgatagatgcgcgtaactggcattgagtcccctgatatcgttagaatccttacggatttgtaatgcacgttgcagctcagggccggcggaatatgcagcgtttttcagccatttagttttggcatagttggaaagtacccgggcatattcttttttgttcttactctcggccagcagggatttgtataaatcgatagcctggtcatagtcgccttttttctggtaagtaagggctatgctgttaagggcaatggtcctggccttcggatgttttatatatttgagtgccttgcgatagtagtcgatagctgcgtcatagtttttaaggttaaggcagatattgcccaactcatggtaaattgagctgaggcattcctggtcttcttttttgtgttcatcaagataagtaagggatttcaacaggctttcctgtcctccgtaatggtctccctcatatgcctggatgatacccatataagtataggccattgcaatttccaaactatctgtggccccggtggcaacgagattaaaataataaaaggcagaatcgttgttgttgttattgaaaaatgattcccctttttccagcgtgggtgcagaaatcggttgcgggggttcctggttggaagtacaggctaaaaaaccgctgaggagtaggggcaggataatgtttgaggggcgcactaagaattatttctcttaaaagtatcgaatttctcaattttgaggaattattattggttggcgctaaaaaagtgaggcaagaacttcttgcctcacggagatgatacatcagggtttccttggaggaattgttccggtttcgccgccggtatcgtccaaagtggtgacctgttcgccattgttatgattgttgttattgggatggcatgggctcaggaatgccaggaagaagcctaatatgatgtgaaacattgttttagtttttaaaatgtttaagcaataggctgccggttgccgggcatccggcagcggagtttcgagtggttgaagaagcgcttcttcttttttgggaagtgtgggcgtggatcacggaagctgattgtcgcttcccaagccggtaaccggcctccgctttctttgcccgggtgtgaataggttctgtacagagtgcctcttagctaaggaggcatttacccgattgcaaaacgaagatatgtcgatctaaaaggttgatttacaaacaattccaataattccgctaattcctggtattccacttatagttccgggaatgcgggtttaattccgattattcagttctataattttatttatggcgacatcttttcctgactaccaacaactggtcatacaggcgtatgaacgaaagaagacaaacaatacgctaccacatggcttgatgcacctcacacccgcgaagctcaaagaggaatgcttgaaaagatgcacaatagatgtaaatgggcgggatgaaaaggttatcagggacttctgtggggatttgaatgtatcaagaagctgtcttgcgatcattcagcgatgcgacacggataagttccggccgttggtgaattatctgaaagggaagtctgaaaaaacagatgagaagaatatcgaactccttgcctggctgattgactttcctggcaggccctgggaattggggaaaacgtactccggtgatgatgaaaatggagctcctgtgttaaatgaggctaccccggcaacagtagatcaggaaacggcaccgggttgcccagccaccccgcccgtagctggaagggatgaatcaaccggaaatccgataattccggaaaatccggcaattccattcctgatgtatagctcaaaggaaaaggaaggcgcgggtgttaaagtcgcagaaaccagtaatcaaaaaaaattaagagggagatccacgagaacattggccgccgcggttatattatcgctggcactgggaacaggtggtatgtggtggtggaaagataatccgcggcccggcggtaactgcatgtattggcaggaagatcattacgagcctgtagcctgtaatcagaaaatagctaatgggagggtcatagcggcagatacaatgaagttgaaaaatttcaggaagataaccaggccggacaccatcacctaccaggctataggaaaggtttggtattctaaaattaacgacaagatagaatactatacagcgggaggagagcacccggtggtctttggccgtcagctgaagccaattactgtctatattatcgataagtatatccgtggaatgaatgagtgaaaggttgcccttcttcaaatcccccaaaatgcttatcttaatttctactacttagcaattaacactaaagaaccctaaagccgtgtttgatacattttttgaaaaatatccagactaccgtattatccaaaaaccgaagagcgataacgtggatgagtatattggcaagctgccggttcagctcatccaatttttgaacgcttacggatttggaacgtttatgaatggttacctgaaattggttgacccatcggagtatcaatcggtttttgatgaagcctataataataaggacaaggaaattgtttttgcggttaccggtcttggcgatttcctgacctggacgggagatgcgatacgcgcagtttacttcaaaaatggtggcgattccattatcgaaagcggggatgacatggaatggttttttaatatggatttagcggacaagggtttcttaagagataacttaaatgataccaattatctcatcgcaaaggaaaggttgggtgaaccagaatatgatgaatgctatggatttgtccccctgttaggattaggagggaaagaaaaagtggataatcttcagaaagtaaaaataaaggaacatatttccttaattgcccaaacaatgggtaagattgaatagtgaaaacagtgggtgaggcaaaattgctttttccctttccccgaatggcctaaatgccccttcttttgtcgcagatggcctttacggtgataactatagtatttatttttggactgtatctgaaaccagcataaaaaattaaatactaaaaccgatcagatgagaaagataatctacggaatcaatctgactgcagatggttgctgtgatcatacccagttaagtggcggcccggaaatccatgagtatttcacggacctcatgcgggatgctgacctgatcatctacggacgtaaaacctacgagttgatggttccttactggcctgacgtcgcaaaaaaacaatccgggacgaaatcggagatcgaatttgcgaaaacatttgacgccattgataaaattgtttgttcccggtcgttagacaaggttgaaggtaatacgagaattattcgtgagaacctcgcagaagaaatcttaaaactgaaacaggaatccggcaaaaatatttcaatcggaggtataagcctgcctggggaattaatcagacttggcctggtggatgaatattattttctcgttcatcccatcattgcgggtgagggaagaaggttgctggatggtaccggtccggctcagcgggatttaaaactggcagactcgagaacgcttccatcaggagctatagcgcttcattacgtgaaacaatgataatgcgggtattcaggtgaaagtactggtacaggtctcaaaccatttaaccaataatttaattaaaagactgacggaacgccatcggcgacaggttggttttggtcttgaacaatttactgaaggattgcaggtgttcaaaacccaactcgtaggcgatctcgctgacggagagattggtggtcgatagtttttctttagccacttctatgagcttattgtgcagatgctgctgggtattctggccggtaagggatttcagtaacccgctcaggtaacccggtgagatatttaagttttcggcaatgtaggcaacggtgggcaggcctttttgagcaagcatgccgctgttaaaataattggtgagcagatcttccagtttggtgagtatctcatggctggcgatcttgcgggttatgaactggcgctggtagaaccgctctgaataagtcagtaatagttccagctgggcaatgatcacgctttgactgaaccggtcgatattagcattgtactcctgctctatattttgcgcaatagatgcgagcatcgtttcttctttgtctgataaataaagcgcctcgtatacggagtagttgaagaattcgtattgcttgatggttttagccagcggcgtgttccataaaaaatccggatggatcaggatcatccagccctccggacggtgcatcataccaccattttcaatttccactccaaagacctggccgggtgccataaagaagagtacaccttcatcaaaatcgctggcctgctggccgtatttgaatttggcattctttacccttttcatggatattgtataaaaatcatagatcaaactgaacttgccttcggcaaggggcctggtcaggtcgtccatccgcaccaggctgatcagcgggtgcgcgggctttggcaggcccgcagcccggtgatattcggtaattgtgtgaaaatgaaaaatctgcttattcatagctttgataaagttcgttattttttatggtaagcccgggcaaactcctgagcgaaatcagcaagtttaaccttccccatttttggctggttccggtgaaagttctccagggttttaccactgtgcatagccgcctgcatttccaccagggtctccgccaacttttccggcactttagccatcttcaatccctgcagcatttgcttttccgagagcaatacccattttaaccagggcttgcctaccgcgcttccgatgatctttgccgcttcattgcaggtcatttcctcgctgcctacataacggatggttttttctttgggtaataatagcagttcctccgcaacggcatccgcaatatcttttggcgatacgaaaacgatccggtcgtctcctccataattgcccatgagcaggccggttttgccagtcagtagcgccccaaggccgtaataacgcagcgccagcattttgcccataaggcccttgcctctgatcaggtcgatggactgatagaagttggtataaaaggccgcgggccgcatgatggtaatggaggcgttaagtccgtcaaatacatgctctgcgttttcggctttcaccaggtctgctgcccaaccgctcaggagtacaacccgtttggtgccggcttctttaagtgcctgaacatagttttgcgatatccggcgcaggtaagctcccatatcaggttccgtaaaactcaggggaatcattgcataaacggcatctgccccgttgaaagtatcagtcagaaaccggacatcggagatcgagccaatagcaggggtagcgcctgttttttggatagctgcccgcttttgggcatcgctgctgacaacggttaccgcatgtccctgggcgatcaatatttctgtcagcggcaggctgatgttccctaaggaacctgtaacaataattttcatcgctggttatttggtataaatactgttctcaatatcggtaagcaagggtgcgtgcgttgggcgccattttatatgctcctgtgtccaaacgctcgatgcgggacagtcgatggcggccatctgtgagaaccagccaaaatgttcagcggctgcttccggcattaccggaactaccgggaaattcagttgtttacctatggcttccgctatcgttttaactgtaatcgcttcttcggctgaagcatgataacgggctcccggttcggcgttttccaaagccaatctgtacaaatgggcagcatccagccggtgtacggcgttccagcgattttgtccgtcgccgatataagcagatattcctttttctctggcgatattgaccagaatgggtacgaaaccatgtttatcatcgtcgccatgtaccgatggagataaacggatcactgctgtacgcacacccagcgcggctactttatctgcggcttgttcagaagccctgggccaggccgggttgaacagaggaatgatatcttcggtagccagcttgccgggactgaccagggctgtgccggaagtaacgatcaaaggacggtcagaaccggccagcacatcgccgatggtttcaatggctgttttatccacttcgcatacttccttaaaccgggtaaagtcgtggataaagccggcatggatcacgccatctgactgagcggcgccgctgcgaaggctttccaggtcttcgaggtcgccacgatgaacttctgcacctgcttcgataagcttttgagctgaagcatctgaacgggccagccctaatacctggtggccggcagctaataattcctgcacaatggcagtaccgacgaagcctgtagctcctgtaacgaatacacgcatgattgttttttcttttgttgacacaaagatgagttgctttagtgaggttgatttatccaaaactgcgtttgatttagctaaaacagggaaagaattgtgtaattaactaattttgatatccggttgtaaaatcccgggttttgtacgcacagattacaaacaaccaatttagttttagcaatgaaacataacgaggttaaaccttgcttagcattagccacctatattcattctttctgggaattgaaaggagatgacagcgaccaccaatgggaacggatatttcctgatggctgccccgggatcgttataaatttaggaggatcctgcaaaaccgacaacggcctggctactatggatcacgggaaaacatacgtggtaggagcaatgacttcctttaaagatagttttatcgacagcaacacccatctaatgggagtgtgcctgaaaccagccatgttttcgtctttttataactatgcgccacaaaatgaattgacggatcataccgttgaatttgacttagcacattcatttgatgttgataagataaataatgatccccatgtttatctcaacagatattttttggacaggaaaagaaatatcaaccagttgcttcagcctgttttaaacgatatccatatttctaaaggaatgttaagcatctctgaaatggcaaaaaataattttataactgtcaggcaattggagcggatttttaaagcccatattggattaacccccaaggagtatgtaaagatcattcgcttccagtcggctttttctatgatgagtgacaacagcccaaagaaaagcttgtcagatatagcgtttgaatgcggcttctatgaccacgcacatcttaccaatgaaataaaacaacacacgggacttacgccttcccaattttaattttgtcgcttttttccaaaagataaaccaggccaggtacttaattttgcgtaaaaggattttaaatgaaaaaagtaattttgaatttagcggtcagcttagacgggtttattgaagggccaaatggtgaaattgattggtgcattatggacgacgatatggactttggaagttttatagcaagcgtcgacaccatattttacggaagagtgagctatgatgcctgggggaatttccaacctgatgcaactaccagtcctgcagaaaaagagatgtgggagggaatacactcaaaaaataaatttgttttctcaagccagagcaggcaagatagcaaagctaccttcataggctccgacatagcaaaccgggttgctgaaatcaagcgacaagatggtaaagatatctggctatacggtggggcaagtcttattaaaacatttataaatacaggtcttattgacgtctataaagtatcagtgcacccggtagttttgggagctggcaaaccattgtttgaagatttgaaagaacgaataggtttaaggttgattgaaaccaatgttttcaagtcgggtgtagtgcaacttacctatgagccggggaaatagataccggaggatttacttgttacaaaagacagtataaattgaaacgccttcaagttatcgaaggcgttttttatcagttgtctaacccaagttgttttctcatgtcgaggttaaaatcatattgttcctcaatcgaaatggctctccgggagttttcattaatgtcttttccttcctttgtccaaagaaaaggataaaagttaaagactttatcgccgtttaactttgaaacttcgtcccgccaatttgtccacctgctgccctcataaaatttatccaagtcattgttgaaacagaagtccaggaattgggtataagtaaggtccatttgttcatactctaaattatctggcgaaaaataatagacgtttcctaagtccttgccaagccctccgccatttagaagataaaagcctccaatagcatcatcggcaattaacagaaatgatggactttcaccaaattctttaaaagatttccctttattccaatcaggaagtgtccgattaatttttgagctacctgaaccaagaatcctaatccagccatcatcaattaaaagtccgcctgtcatataaataattgcacccattggggaacgcgttgtcacctaggttttgtacaacgcatcttttgcttttgaggtgtcaaccggtaagatctcaactttgttttttgcggatttaatccactcatctacaaatatccatcccggatcagttttgttgattagttcttcaacttgtctcattttattttgggctgtcattggtaaggcatacaaggtcagcaagactattgttaaatatcgcatcataacctttgtgtagttttcgcaagctattattttttcggctatctaacaaaaaagcgcagtgactggccggataacgcagaaattattccataactcatatcgggaaaacttgcctatccgtaaaatataaaatgagctaaaaatatccgaccagatatcttttagctcattttaataattgaaccaatcaactcaaggttctgtgtgatcgtgttccaatgccttcttgaatttattatacagtgtccaatcgggattcggctggttatccatccagccataagtaaggccctcaaatcttgcgcggtagaaagtgtcattttccgggtacattcttattccgtcgtaatatcttctgaggaaatattcaaaattagcacggtcctttctgccggcaaatttttcaccttcggcgtaaccgtaattgtattcgcgctcgtactcagaaagtacaggccctgacggattagaccggggaggaggaagcgtttgggcatgaaccgataatgatcctgccagtgcaattaaaagtaccgcaactgttttagccgctgcattccattttaaacatcgttttcttttattttccataaaatagtatttaggcaatgaaattagccttccttactattaaaggatagtacaaagacgacaagtttgattccctgcataaagtcgctggtacctgataaaaaaaagctgctggcccgtatcagcagcttccgcagatccattttctatacggaggatcttatccgatttcaattgtcctgggtgctttttgctttgcttcttctttcttcggaatagtaagcaacagcagaccgttttcgtaacgggcatttattttttcttcatccactacgtccttctgaagttcgaagctgcgctgaaatgattgatagctgaactccctgcggctgtaatttttttccttggtttcttctgtatgttgtttagcagaagaaatagtgagcaggttgccatcaagtgtgatcttaaaatcttttttatccatgccgggagcggctacttctacttcaaagttatcgtccgtttcccggatatttactgcgggaacggtagtgctggtggatgaatagttattgtttccccaattaaaaagttcgcggccaaagaagtcatcgaacaaagccgggaatgcggggaactgattcccgttccttttaataagtgacatattaacctccatttttaaataagtgagcaataaataatgatctcattttaattggctggccagcctcaaaaaatttcacaatcgatatgccatggcccaaaaactgattttttttcatgaaaactgacattatttaccctcttattaagagggtaaaggttatcttgtcagcccgccctttaacttcatgaagaaggctgatatcttaaagaatcatgttaagtttgagtatggaaaatttattgaagtatatccattctctcaccaactttacaccagacaactggtgtgcgcttaccccggccttaacaacggtggtgttctccaaagatgaatacctgttacaggccggtaaagtttgtgaggccttgttttttgtgagcagcggatactgcagggccttctataacaaggatggacaggatattaataccgctttcttttttgagaatgatatcgctaccaatatcaacagcctggctaccggtgaaaagtcggctttctccatccaggcattggggccggtaacggctatccgctttgatgtaaagaagctgcgcgaggtatccctgctggaccctgctatagaagcgttgggccggaaatgccttcagcagattgcggcaaaacaggaaaagcatgccgccatgtttaaattaatgagtccgcaggaacgttacgaattcctggaggagcatgaccccggcttattgcaacgggtgtcgcttacccagctgtcttcctaccttggcgtagccagggaaacattaagccgtatccgcagcaggagataggcaccttgtttgtgacgattgtcacaggttaaaatggttggatctgtggatctttacaccattaattttaaaccatttaacaacagaaagtatgaatgcaacacaatcaacagaaaccgtacttcgcttcattaattcattgaatgaagaagattttaccacggcacgcaactgtgtgaccgatgatcttacgtttaacggtgtaatgggaacccgtaatggcgctgatgcctatttcaaggatatggaacggatgaagctgaaatataacatccggaaggtgtttgctgacgacagcgatgtgtgcctctggtacgatgtaattatggatgacaaacccatactaagctgcggctggtatcagttgcaggacaactgtatccgttcgttccaggtggtatttgacccgcggccattattggaaacggcgaaatagtttcgtcacgacagcagcccatgtttaaaaaaagccattcctttacgaatggcttttactttttcaaacattcacactagttatgggaaatatctcttttgttgattagtttacgcatattttccaggatggtatttgcttcctcgaaatgcgtatttaacttcggtaccatatccctggcataggtactgatggcggtatccttagaggctactgcattattaaagtcaaacagcgtttttttatgatcctcgatcatctgtttaatataggccctgtcaaaatcttctttcttaatatctgtcagcgtttgttctgtcgcttttgcatcgtctgtaagatctgcaggcatggtaacgcctgttttattggcaatggcctgtaattgttcattggcggcagtgtgatctttttccatcatcgcaccatactgcctcacccgttcatcccgggctttactttttgcaagttgtccaagccttatttctttaaggttagcggcagccgcagtagtgataaagttaacggtagccttttccgtttgctggtccggtttcttttgctgcccgcaggagagaagggcagccacagccaatgttagaacaggatatgttttcatcgttccagtttttgaaaggatatcaaaaaaagcgccatgcctcgaaccggggattttatcaataagatatgacacttaaacattaaacctagccttagtccgcttgcgggtataccagataccagcggcagctaatgctacagcgcctgccagcagccaccaacgggtattcccggcaggcggaatgtattccacgccgttcaccccggcaacagccgcttcatttacatacctgccggaatgcggccgggcagatgctttgaaattatctgccagcgattgcaactgtcgctgcatttcctggccggttaacggcttcccatggccggtagctaccgtttggggttgcagggccgccagttttttcacactgctctccgcagagatccagtcaggtgtgaaatatttaggaggaccggatacttttttcgattgggtgatcacgtgagacagcgactctgcctgggtggttacaaacgcatctcccgccagcagtacaccgtcgtattcgcggtaaagactgatatgtcccggtgtatgcccaggcgtatgaatatatcgccatccttccagtccgggtacggatccgtcttccggaagcatgagcaaatggccgttcagattaatcccctgtttggggaatgtccacgacagtaatgtcatcataccgccgccggcagatgggtcgggaggtgggtaggcagacctgccggtaagataaggggcttccaggtagtgcgcatacaccggcacatcccattccgacaacagcgcaggaagtgcgcctgtatgatcaaagtgaccgtgggtgagaataatagccgatggtgttgcctgcggccagaagagatgtttggccacctgcataattttatgggcggaggtctgcagtccggcatctaccagtacccaggaattattggctggctcatgaatgaggtacatattcacaaatacgtcgtgtataccccacacgccgggcgccaccgcaaaccatttcttataaagtttctcctcgattaacgtaatgttttccataccggttgttttccttccatacagcaattactgttccctccgaatgcccctgtctcccgaaaaataaaaacagttatctcaaacgggttatttattttgcggcagaagtggacaaaaaatagcgaacaatgaaaatcaacctgctcttccgccgcgggagaaaagcatacctgacaggcatcttcctgctcgcaggtagccttacctcatatgcacaaaagactaaccaggcgctcctgctggatggcaatgataacaaccccagtattggtatgggtatcatccggaagcattggaccgtggaagcctggatcaaaggaaacgataacgtctggaaggagcgcgaagctattattggcggcggtgaatacacagcctatccccacatcgacaatctccctttgatgatcaaaaacggtcatttacacagcaaaaaagcgaatataaccgcacgcgggatactggatagcaactggcatcacgtagccgccacctgcaacggcgtagaaaccaaactttacctggatggaaaagaagtgggccgcgcaaaaggcgcggtggatatcttgcccggcgccataggcaccaatgatatggactccagtacctttggcggttgtatcgatgaagtacggatatggaccaccgcactggctcccgccaccctccgccggtggatgtatcagccgttggccccttcgcaccctgactttcaggcgctgaaaggctattataccttcgatgatatgcaggacgatgtatgtcttaacctggtggggaaaggccaccaggcatatcatatgcggaatacacggaaaaagtataaaggaacatcgccgttggcggcgctggtgaaaaataacaaccctttatttgtaacaccgcatccgaagcaacaactgtttaatgcggtaactatccaaagcgaatgggatgcggatccgggcagcgctaacgacgcggtacttaaactacgtatagtggctaacggtagtaaggagccgctgaaactgactgctttgcagctggatttatcgcgcaatacccggttatccgatattacggcagtgcatgtatatgctgccggtcaaacgccgcgctccaacagcaggaaggagttgtttggaacaggtaataccccggggaaaaaaatgaaattagttttgcctccggcagatggatatgccttgcaagacggggtaaattatttcctggtaaccttcgatgtaaaaaagaacgcggtgccaggagatactttgtatgcagatgttgcttcatttgctttaaacggcaccgcctatacgccggaagcagcacccaccaacattatgaaaaccgttgtaccctcttctgcaaccaatgcaaatacggtgaagctgctgcaatggaatatctggcatggtggcgtgcacctaggaaataatggtcccggccgggtaaaggaattgctgttgcagacccatgccgatattatcagtatgcaggaagcatatggcacacaacagttcctgaatgatacgctggggtttcacctgcaaacacccgctccgggcgccaatctcgcactgttcagccgttaccctttggagcagcatgcatccggtgataattttaaatccaataccgcaacggtgctgctgccgggccgccggaaagtattggtcggcaactggtggctgaggtatgccagtaaacatgagtacaccgatttttatcccattccgggattggatactaacgactggatcagggaagacagtgaactggcggtaacagatgcccggaaaaacctggatcaggacatagacccggttgcagcggctgatacctcattgccggtgattttggcgggggattttaattcgggtagccacctcgactggaccgccagggcagcgtttttacactatggatatggtccggtattattaccggcttccaggtttatgctggaacggggttaccgcgatagttaccgggagctgcaaccagatgaagtgacacatccggcaggcacatttgcggtgatttacgggcacctgcaaacttcacggatcgactttatttattacaagggttcaggcattagtgcaatcgcttctaaaattatccggacatcaccggagatagacgacgtgtggccttccgatcatgctgcggtacttactacatttgatatacgataacaaggcgaaatcggtcactgccgcacgtttgaggagaaccgtctcagtaatgtgtaatcattttctcatagtaaccccatcctgggaaacttacatgaatgactgcgaccagtcatgttgacagaaaacaacacaggagcgaggttcgctgtatcaggctgctttacgtgtaagatggcattggtatggattcacatttgcgaatgaaatacgaaagtattgttcactcaaaaatgatgaagtatgttctatcatgtaaaagacctgcagtttaatgcccgggtatcaaaaccggatcctgcatttgctactttattactggagcagttcggcggtgcaaacggcgaattggccgctgcgctcaggtacttcggacaggcatttggcgccaggaatccatttcctgacaagtacgacctgctgatggatatagccacagaagaattcagccacctcgaaatagtgggcgccactatccagatgttattgcagggcatcaacggagatttgaaaaaagcggcagaagaatcggagatcatgcaattgctggatgggaaaaaggcgaaggaagagtttattcataaagcgattgtagcgccacaactcctggtatcttccggaggcggccctgcatataccaacagccagggcgttccatggtcggcttcctatatcaatggcgattgtaacggtgatcttacagtagatctccgctctgatatggcagcggaatcacgcgcaaaaatcacttacgaatacctgctccaatttactgacgatccatatgtaaaggaaacccttaacttcctgatgacacgtgaagtggcacatttccagatgtttgaagcagcgctggattccatacagcctaatttccctccaggcgtattgcagtcggatccgcgctacagcaacctctattttaatatgtccagcggcgcggatatccgtggaacatggaatgagggcgagtcttcccaactcggggaaacctggcagtttattcaagatcctgttagctacgtactgcaaacaaacggattactggatgtggaaccaaccggcaccagcagaaccctgcagggtgtagatgaaatagacaagagtttaagcctgcagcgaagcgaggaaataaacatggcagtaccgattggagaacagtcatggagtgaacatgccgacagcgtacaaaaaaagagcaatggaaagacaagccacactaaaaagaaataaaaaaggtaaggcgacagatgccgggtaccatcttgaagtggtttattataccgatccgctttgttgctggagttgggcgtttgaaccggtaattcaacggcttgttaatgagtatgggaaacggttgtcgatccgctattgcatgggtggcatgttatcggggtggaacaactatcacgatacgctgcatgcagttagccggcccatacaaatggggccggtgtggttgcaggcaaaacaactgaccggcgtagcgttgaacgataccatctggttcacagatccgccggcatcttcttatccggcctgcgtagcggtaaagtgtgctgccctgcaatcggagcagttagctgcgcaatatctttttaagttgcggactgcagtgatgctgaaagccaaaaatattgcgcgaaaggaagtgttgatctccacggcggaagagctggcgcaagagaaccccttgtttgatgcggggaaatttacaacgcagttaacaagccagcaagctatcgatgcgttccgggcggatatgcaggaaacaaagtataggggcatccatcgtttcccttcattattgctgcaggtaagggatacgagaaaaagtttactgctcacaggaaacaggccttttgaggctattacatcgtgtattgaccaattagttgctgagtaaaataaaatatccggattatttatccggatattttattttccattgttccagtagttcatccgccttacctggttccaggtgtttaataataaaatcaagtttttcttcccggcggtcgtcaccttcttttgattggggagatccgcagtaccacaggaaggataatcctactacctgccagataagctgaaggaattccgactgccagttttccattgtttcccgcatcatctgtacggcatattccggaacttcggcaggttgcgaatgcgccatctgctcgttcagataatctttccatccaaagtaccaatgtaatgctatggaagcaaggaatagcaaaagcgttacccagaagtaggcttttcgcttcaggtaagaggggcttttttgatttgttttcataacctgtagtgtaaacagtgaataagaattttacaggtaaatgagtaacaaaatcgagccagaccttataccagctgcatattagctttcagcgcaatttctgaggaaatagtgaaacagtttgtctgaatgatgtggttacttattaccggttgaagtgcctgttgttgctgcgttttctggtattgggggtatgattttgtaagcgtatctaaggaagaaataaaccatattactcattcttaaatcaggttattatggaaaacatactgaaccagcaacgtgatgaaggaaaggtagcaaggcgatagaaaatcaaacggccaaactgccgtccgatacttttttgcgggcatctaaaggtgcgatgggatggtcgctggcgctgcaatgcttaggcaagaaacatatcagccttttcattggtcagtgggcagcccttcctgcttttcggtgtttataataagatagttaaggtagagggtaacgattagttacatggtgaatgaagagatgaaaacagcaggtgcctttgtggcgcctgctgtttttttagatggattgctgaactggaagtaaactgctggtcattaaattgcagcgccagggttgccgcagcaggaacagcaccagcgaggcgatatcttccgggatgagcatttcttctttctgctgcatttccagtttcttttctgcgggcatatccagcaggtcggtgcccaccaacccaggttcaataagcgacaccttgatgtttgatgactgtacctcttttcgcagggcttctgaaaaggcctggataccggctttagtggcagtatacacggagctgttggccgatcttacatctgcgctgagagagccgatgaacacaatctgccccccacctttttctttcatacgcttcactgcctcatgtgagcaggccaggtaggatagcaggttggtgttgagtacatattgccaatcatcgtaggtgccttcctgtatgcccttgaatggcaccgcggcgttgttgatcaggatgtcgagacgatcaaagtgttcatctacctgtttaaatgtttcttcaattccttttttctctgcaatatccgcagtaaacccatgcacctttccttccataccagcgtttttaaatgcctgaatggtatcgttcaactccggctgatgtctgccgaaaaccatcacctttgcgccgtacgaggccagcaggagggcggtagatctgccaattccggtggtgccaccagtgatcaggattttttttcctgtgagttcttccggttcatatttaccgattgatgaaaaatttgtttgctgcataagaatactttttaaatggtttatttccaggagacagtaatctgctggtttcctttgagtttaaattcaagatgtccattgtcacacggagtgccgtttatttccgttttctcatctgttactttgatccggggtagggcagtacgtttctttatagctataatacgcatatgacagactccttttttatgtcccaatacgcggaaggtgaccgttttgccttttatggtaaagccgcttgtaggatagtcgatgaaaatgagcagcgattcgccgggaaccgtgtaatagtggcggggaatcaaagcaaaagcaagtccggaaccatatacttcctggcctacagtccccgacttgttccagccctcctgcagatcttccacgggtatccacaactgtttcgccacttccccggttttggtgtcttccgacaggcaatcttccggtaacatgggcggataataataggctgcgcgataaatatagtagcgtgtaaattcactgagcagtaacctgactgattcaggtatggggatgttttccgacatcaaaagataatccccgaaggaagaaaaacattcggtttcctcgtaaacggctgtatatggcgcttccggtagaggaaaaagcgcgaaaaaagtagggtaattttttgcataaccataattgcagtcccacagccatacatttttaaacatattagcgagacagagatagctgatattcaggaatacttcttcctttgtaagggtatataacttcaatgcggtaaaagcagagaaagccgtattgttagcctggtagaaaacctggaatccttctccctgtagcgaaagacaagctgcttttgcttcctgcagatatatttctttttgtgtaagctcccatgccagcaacatcacttttgcataaataccggctacatctttttctccgcctttgcccggtgcagtttccgcttttatcacttccaatgtttccatgttataaaacaccggccatttataattgaaatgatgggctactcttatcgcaaaatccagcgaagcgaaaagcatttccctgatactttcatgcccctgtttcatcaaccttaccaggttcattaacggatgatgaaggtaccagctatccatgaccagcggacgtttatgttcttccgatttatccagcctgtcctgtgctgcggggagccaccggaccaatgttttaagttttttatcatagaaatccggtattaccgttacaagatcccttatcatctgcatatcccgcctgctccattgctggtaatccaccaggggaagcaaaacactcagctgtaccatcagttccggaggtgttttataatcgcatacataggcgttcagaaaagcatgaccatttacctggcaccagctgccggcgctatgttccaggtcgtaccatgttttatccagtatttccggccagtggtgatattgggttgctggttttgggagatggagatatatttctgccagcaggtccataaattgctttgacatggctatttcatcagcaggcgttttgtcgtccattactacaaatgtgtcgctgatggtgtaagttttgcctgcctttaaagaatgttcatctgatacaggcagcataaagcctatatcgggccatgtgccgcccacggaattactgacggatgtttttgtttgttcacagtatttgtccagcgaggtaaggttctgaagataaagtacagatcccgaaccaggttcctttatactgaaatagatcattcctgtacgcgcgccattttgtgaaagatgtatgtcaccttccgggatacccttgtaaccacttcgtttcagtggcataatatcacgtggccagtagtgaaagatgagcggagcaattggtgtaacggttgttttacaacgaatcgccgggtgtccgttattataaaggtccagcgttaccacataggaagccgccagcgtttgcagatgaaaaacagcctggttctttttcctgacagtacgtttgatcacgatcttgtcgtgcggggcatataccgccctgaaagtaatacgggcgccttccggccactcggccagcacccataaggcatctcctgtacagtatacgtagtaatgacagtcgccggattgctggtaaaagatctcttttaattcagggttattgaatatttcattaatggccgttgcgtgaggtgaaattccttccataaatcatgtatttaagcatgctccagggttaaaatatgtacgcaccacgaggtgacgagcaagagttgtatacaggcatccaacaggtatatttttgatatcactgctttggatacatatatcacatctaccagtagtaatacaagcgctgtgcctgcgccaataatcaatgttcctatggtagcagcccctgggtgcgttaattattaaacaccgcataaaaatccgtaccagtcaggaggttagaccggaagacaacaaaaagcctgttacatagcacacgcaggcattataaacgtggatgaaaagccacggactgatatttagaagagggacagattgtacaatgttttacagggcttccatattaatggagccagtggttctgaatggcttccatcgattgacctttggtttccggcaccagtttatataccgttataaaagcgaatacacagcatagcgcaaagcaccagaatgtttgtggtgttcccacagatgccagcataacaggcgttaactgccccatgatggcgtcggcggtccacatcaccatgatgctgagtgacagcgccttcgcgcgtatgctgtcagggaatatctcggctgcaatcacaaatttcaatgggccgatggagaaggcgaagcaagccaggaaagccaatacacaaagcaagagacagatgccattaacggcgccaacgtagaaacagatgccggtcagcagcaggctcactgccgcgccggctgttccccatagatacaaggggcgcctgccaagactgtcgactttccagatcgcaataaacgtaaagagcacgtttgctgcgccaaaaaacagctggctgatgagggagctgtccagcgtaagcccggattggtgcaggatagtagggccatagtaaataatggcgttgatcccgctgaactgtgagaataatggcagcaggatggcgatcagcaaagcacggcggtagcgcggcgccagcaattgcgtataaccggcggggttagcttttgttgtagcatgcctgagcttcagccaacgcggactttccggaataaaagcgatacccagtaaaaaaagcagtgccggaaaaatgcctacaccaaacattttgcgccatacctccaggccggtgatcagcagccatccgctttgggctggtgtggcggcatatttcaggagcagcgcattgctgccataggcgctgaaaataccgatggtaacagccagctggtaataggtaaccagccggccacgcaggtggtccggggcaatttcggagagatagagcggcactacgctggaggcgatacctaccgccatgccgcctagtatgcgtgctgcaataagccaggaaaataccgggataaaagtgcagcccagcgcagtgagtacaaacagggctgctgacaggaacaacaacttttttctgccaagccggtcactgatatcaccggcaaaaatgaccccggcaatacagcctgccagcgccgacgaaacaaaccagcccagttgtgcgggcgacaaagaaaaccggtgctccacaaaaggcaggatgccggataccacggccatgtcaaaaccaaagaggaagccgcccagggaggctaccagcgtaataaaggtgagatgttgaccgcgttgctgcatgttcaggtggatgctatttgttgataaaccggatgcgatggttttaaaaaagctttgatcagtttcaccggttccccgttattgctggtaatccggcagtctatcgccgctgccggtatcacaaaagtttcagcatagtgatatatattcgtatgtccgttggaggtagtaaccgttactgcactaccttctacgagcatcatcaccaggcagttgccatcggtagttatattaacgctgttgctgaattccagccggtgcacatcgtaaaaatgtgctgcatgtgttggcaggtgcaccagccggtagtctgccctttgctctattgtcacgggggcagcaatgagctgctcttttacagccttgccctgcctgttgaaatccaggttatgaaatgcatgatctatattgatggcccttggttttccatccaggccgggccgcagccaatcgtacattttaaacgtaaaaatgtacggggtggcgctgatttccagtacaagattattggcgccggcgctatgtacagttccgttgggcaccaggaacaaggtatgtttatctgctgtatgttgctgtacaaaatccgttatttctaccggaataccaagatcccggctgttttccagtttggttctgaatattccgggatcaatcccatcctggaaacccaggtacacagtggcgccggctttgcaatccaggatgtagtaagtttcatcctgtgtaaacgtttcaccgaaatgtgtgcggatataatccatggaaggatggcattgaatggataagttgccgccgtcgaaggtatcgaggaagtcgaaccggatggggaattcatatttgaagatcggggcatgattgccgaggatagccctgtgctgcgcatacatcagccattcgaagggaatttccatcaggtagccatcgctttcaaagagcaccccgttttccggaacaatcaattcaaaagaccatgcgtaatttacttcttcggtgttgataccattgatatgtgtttttagccactgcccgccccaggcgccggcttcaaaccagggccgcaccctgaacgtggaatgaaccaactggtcaatgcccgcctgcagatcttcattaaatgcccaggcaatatgatccggccactgcgtatctgccatgatgtggatacgtggcgccagggtttgcttataatgattgagcactacccaatccacaaagtaaaaccgtttatacatttgagtactgccgccggcagtatcacagcccaggttggtaatagtgcctgcgcgcatgcggtactgcaattcatttttgggtatgtccaggtatatcagcggcgcagcagcatcggtgagcgcagcgcccacgcctgatacaatgtgaaggtcataagggccatcgaatgacaatgcccccagtttctcctcatcaaagaaatcggtgatctgtaaagaagtctttttgccccatacatcaccttcgctgccaataaagggatcgaccagctcctgaatgttatcactgttttttagcaggcaatgcgtatcatgccatttaacgtttacgcctatacgtgtaaattccgcttgcagggcagcgctgatcttatcccagaaaataccagcatagccgtctatcagcaccagcgggtgctgtaccatccatttggccagtgattcgtatcctgtctgtatcttaccattgccgagcggatgggccgggtatctgttataggtacctggtagtggggtggctgcatgttccggcagcaagggctgtgctgattctcgccagatcataatcttattttttttccacacggatcattattactcctttgccagaaatggagaaactttcccgaagtgtgtgcttgtttgtttccagtatatcgctttcagaaatatttaaagcagtggatttattctttgatgttagtgtagccgtggccgtatgaggggaggtatttaccagttgcagcaatacgccattgccgtctgccgcaggatagaggttttccacaaatacattttccccgctgatgttaaagaacaggctttccgaaggagcgccgtttgcggcggcaacaaccggtggctggtgattttccaacccgcttttgttagccgcggcagcattaaactggccatgcacccgcaggtagtaatgaaagacagtgatcccttcctggtccctccggaaattggtatgccacaggttattcatcacccaggaagaaatgaggggctgttgttccataaaggaaatccagcggggagagttgtgcagtccgccgagtagccctgcagtagggtattggcctatttcaaagagcggcgcatcgggagccgaccaggtaacgcctgtatttttcccggaaatatctacccaacgttgctgcgtataccagttcctgttagtatggggtaactgatctgcttcagcggttatatttccccaggggatgctgtaacgtacctgtgcaccggggacacggaagggaaatacaaagtgtacgctttccttgtcgccaacggcggttttatcaatcgtgttagtcagcatcacctggtcggtgcctgcggcaagttgtatttcacgggtgagggagcgcgcgcggggtgcgggtgtggtgatcagcaggctaaccaccagcgggcctttttcctttacctcgatgtttgcctgtccgctgtattgtattctttcagcagcgtcaccaggcatataggtgtattggttcaatcctgcggaatcggcaaagttgccgctatagccttttttaagcagctggatgatgttgcctgtctttgggtctacccgcacggaataaatgctgttatcgagactgtaatttgtaactgtcgcttttttaaacggcgctccggcgccgggatgaatcgtgaagcgttgtttagagaaaggaggcagcgcggttgccaggaaggcgagttcgccggtgctgagccgctgggagggcaatttcctgccgttaagatcttttacaacgtcgccggaggtgctgagggcggcgggtatgcgcaccaatgcggtgcgggaatgtcccagggtattgtaaacgtctatagcggatgtgatggtgttgctggtatatccgttgccgttagtgctgctgcgcagcagcgcttcggactggtcccgggcattcaatgcaaagccctgtttaaactgccattgggcaatggctttagggtccttcggatcggacacgctattgaaagcgccccaggtgtgttcgttgaacatgacgaggtccgtccaggtgttgcggaaggagtcggccgggtaaccggtttttcccctgatagcccagatagcgccggcctgttgcagccggtcagatgcgttccggttaatggcggtttcttttgcagcagaggcgatgccatctgtccagtattcagtgtaatcgccggtgaacacaggaattttgtctttccacccggcttcaaagtcgtggaaaaattgctttaccgaggtaataatcagtttgggagatgtataccgctcgttccatgcctttactgcgtccggcagctcagggtctataggcgcattatcgctcatggcccaggtgaggagcgtcatgttatagggaaagtggttgtgctccagctgggagagataatcaaaaagataggggttgaggaaattttcagtgggtttgccggtgtaataaggcttggggtcttctacggtaaagaagttgggtattttacttcctttcagcgtatagccgatagagtagggcgacgactgccagaagagcacctgttgtttcccggaggcatcccgccagtagaagggtttatcacgccattgccccgaactgccgatgcggtcgttggcattgggtgcgctgaggaagtacttcatgccggtgatggccgattgactgatcagtccccacgaggcgcctggaacatccccctggaacatggtgttgatggtaatgccgtaatcttttgcgagccgggcccccaaagaaaacagttgcagcaattgggcggaagaagtggcgctggtattggtgttggcgtaagtcccgtcgaggttgatccagccttttttcaccgcttcgcggaatgtttgtttcttttcatcgctggcggcggcgaggtatttatctaccacccaaagcgcttccgtgttccatttgaaccgggcttccggcggatagcctgccgtacgggcggctattttaatggcttcatcgatgttgttcatatgaatggccagcacctttgcctgtacgttggtatatcctacatctacatgcgagtggggcatgaggtatacgttccattgccgggtgggtgaaacaatgcagtgggcggtataggtttgcccggcactgagcaggcgaacaaacagctcggtgtctttgtctactgcttcgccgggcagcggcagctcatagtcaacgatgccatcggggctggcggccagcgagagactgtcttcatggccattgaagtacatatacaccattgcgggctgatagctttttcccccatgaaagcgcattcttaccatccgggcgggagtgccgtgatggttcaggtaagcgatagtgggttgcagttcaatgctggtaaaggatgctgcctgctgtgatatttcagcgccggcaggagaaagggctaaatccccgctatgtgaaccgggaaattccagacccagtgcactagcatgggcggccggaaagcagctacataacaggagttttgctactatatgcttcatatgtacaaacatacggacatatttcaatattcggaaaggatacagggttaaaaaaagggctgaccaaaagtatggtcagcccctgaaaacgtaatgttatctgctagaaacccgggttatttggcaataatttcgggtttacgtcgctttcctgtttaggaacagggaatagcagttgtttcgcggcgaacgtagcaccgaatacagttttatgtcctacaaagtcgtcccagttaccggttacatcgttgtgaactttccgggtccgtatcatatcgaaccacattttattttcgaagcacagttcaaagtaccgttgaagccatacttcgcgctcaaaagcaacttgtgacagcgcgcccagcggcgccagcttagcacgggcacggatggcgtttacataacgaagagcatctgcattaggtccgccttctgcgcggttagaggcttctgcatacatcaggtacacatctgccaggcgataaagcgtatagttaagatctgatttggccgtgcttaccaccgctaaagaatcaaaccatttgtagatataccggcctttaaaagtaatggtatcggagctgggcgatttcttcttatacttagtgtagaagaattgtctttcctgcacccttttatcacccgcagggaatgatgcaataaactgtggagtaggatatacggatccatactcatcagaatattgtgaaatacccgcgtagtttggaatggtaagcggcgtaagcggattgatgcttggtactgaagcggcatactgcacctggaaaatgaactccccaagatttttattggcggggttgatcatattcgtgtattccgggaacaggaaatagccaccgtttgcaatcaccgacttggaggcagctgccgacaatgcgtagtattgattgccaccattgatggccgcaccggcgtaagtcaggtacacatcagcgagaagtgattgaacaagccccattgatactttgcctgttttatctgaccagggcagtgtggactttgccgcggtgagcagatccggaataatgatctcatcataaatcgctttcgcttctgtacggggcaggttcaggttgagatctttgggcacttcggttactttgggaacggcgccgtataatcttaccaggtgaaaataataaagcgcacgcagcgtatgcgcttctgccagcatgttggttttatctgcatccgacacggcggcttgtggcaatttttcaatggccaggttacaggcgccaacgcccatgtataaacgttgccaccaggtatccacataaaaggaagtagcgttataactgaggttctgaaaggtggcaaacccggtttgtccgagatcactgttagccttacctgtcatgaattccatcaggttgtaagtgttacccccataagaagatgcctgtccctgtaagaaaccctgcaggtattggtacgatccgtttgccagcgcgcgtgctacttttggatcagagaggtcagcatccggcggaagaaaattcgtgggcttttgttccaggaattttttgcaggagcaactgagcaacaccagcaacgcgagtatgatatgtttagtcgttttcattttcatatttttttaatcacaaaaaaggttatcacatcaacaggtacacgatttcatcagaaatcaaggttcacacccaggttccacacgcgcgggcggggataagggaagaagtcgatgttctgtgagaagccggtgttggcgccataaccaaaattaaaggtgtctacttcagggtcataaccggtgtatttggtaatgaggaaaagattttgcacgctgccatagatgcggaacctgcggatatggcttctttgcatccaggattcagggaaggtgtaacccagagtgaagttctgtccccggatataggaaccgtcttctacccaccaggtatcaaagtgggaatcctgtgtaaatttatagctgcgcacctgggcaatatgtgtgttctgattttccggtgtccatgcattcaatacggtagccaggctgttagccagcgtctgacggtcttccacagagtgcttgaacgcagccgctgtattcacgccctgtacaaaacggatatcaaaagtaaaatcccatcctttgtatttgatggtgctgctgaaggtaccggtccatcttggataggcgcggcctataatatcatacaccgcattgccggcagaatcatattcgtattttctgtcgcccggcaagagggagtgtttggctgcttctgccgcttcatccgtaccataggtacctaaccttttcattccgtaaaaagaaccgataggctcacctacacgcaggatattagtttgtcccaggaaattgggaccagggaagatatctgcattaccatcgttgagggtgagaattctgtttttattggtagcaaaaacgaaagtagtggaccaggtaaagtttggtttctggatgtttaccgtgttcaggtttacttccagaccggtgtttcttacttcacctatatttttatacacattgggtgtgtacataccggcagaccacggaataggtgttgccaggaggaggtccgatgttttacggttatagtaatccacgttcaggttaatgcggttgtcccacatccccagttccacaccggcgtctatctggttggaacgttcccatttgagatcggagttacctatatacccgggtacaagcgttggctggttggcgccgcctattacggtttgatcaggacggtactgtggagagtactggaactgaccaatttcttggttaccggaagtaccgtagctggcgcggatcttcaggttattgatggttttactgcctttcaggaagtcttcctcagaaacacgccatgcggccgctacagaagggaagaaggcgaactggttgtctttactgaatttggaagatccgtcatacctcgcagtagcggtaaaaagatacttgtttttcaggttgtaattaacacggccatagtaggagttcattgaccagggctgtgtttctgaagtgatgttgttacgtactgatcctgccgccagtgaattccactggaagtaatcggacaggaagttttgtgtttccgccagggcattttcattactgaattgcaggaaggaaatacccactactgcatttaagctgttattatttttgaactgtttgttataagtaagatagttttctgattgccagtatttttggtaattggtagtgatcctggctataccgccctgatcctgcgacaggtgaggaagattgccggcggaatagaaattggctttgttgctgatctgatcgtaaccaaagtctgttttaaaattcaggtctttggtgatctggaactgcatgtaaaaattgccgagggtatgtacctggttattaagggtatacctgttctgcgcaatctgtacaggattcggaccaccttccagcccgggaatatcgtagtttcccgcccatttaccgtcgggatatcttaccggtacaataggtacttcttccgttaccattctcggtacgtttaaggaaccgttaccatcagacaccactctctgcgtgctggatacgagattcagactaccgccgattttcagccagtcttttacctggtcatcgaaagtggccctggcagaatatcttctgaaccatgattctatcattaaaccattctgatccaggtaaccaagggacgcgctatagagcagtttgtcattacctccctggaagttcacctggtggctggtagacacggccggtttataggtttctttttcccagttggtgttgtacagcggtttgtcgttctcgtcaaacagcagcgggaaatgctcatgatccaggatagcggtgggtgtccaggtgccgtggtccggatcgaacttggtggcattggcaaatgattcgttatatacttttacaaattgctctgaatttaaggtgggaagatgactggccagtgtacttacgtttacgtcgccctggtagcttacctgggtgggaccggccttaccacgtttggtagtgatcataattacaccgttggcgcctctcgcaccataaatagcagtggaggaagcatctttcaatacttcgatggaagcgatatcattcgggttgagcgcatttgcatcaacacccgccactccatctactacatacaaaggatccacaaaagagttgatagaaccgataccgcggatacgcaccttagctgcctggccgggggcgctgctgttgatgtttacgtccacgccggctaccttgccctgcagtgcctgtgaaatgttgggaacaggcttatccattacctgctcgcctttaagggacgccaccgcgcccgtgaggtcagatttttttaccgatccgtaaccaattaccacaaggtcgcttaaggtacttacctgtacttccaatgctacattgatggtggtttgattaccaaccctgacctccttggtgccgaatccggtgaaggagaacaccagcacggcgttttcgttgggcaccgacagggagtatacgccgtctacattggcgatggttccgctggaagtgcctttaatggccaccgtagtgtttggaatgacggtcccgtcagcggcgctggtaactttaccgcttattttgatctgggccattgcatgcatggaaaataggaggcatgcaagcacataaaatagttttgctttcataacaagtctttagtgatgaggtaatattagccggtgtttcagttgatagtagtcacaggagctgtacgtggaagtccctgtgataacaagtgagattaggttttaagattatggtaatactatgttttttaataagatccggttgacgaataaataataactgagcaggcccaattgtttattctactgctgattaattgcccacttttttaaaagtgtaatggcatctgataaaacacctgcttctccacgaaaatttcccgatccttttggcgtgccagtctgaacgtcgtaccattcaaagaagccattctgagcaatgacgcgatcggtcatgggtttaagctctgctacggcttcctgtataaatccgtttataataagcgcctggatcatgcgtccgccgaaccaggtccagtcgccggcattctgatacacataaggatgcatattcgggaactcctttgccgggtaaggaggatacaccgtgatccctatggttgcgaacttttctttggcggcggcctgagtcatttgccggttaatggccgctatttcttttggtgtatgaaatcctgccagtattgcgcaggcagtgcccccggtgtagaggatctctttttcgttgaatgagggggaaaacgggcttccgttcaaataaagatgtggtatgtatttctgtgccctgttatcccataaatgtttgcgtacatttttccggatatctgttgctattttgctccaatccttttgtgcccggtagtttgctggtttgattgccaggaaatcctgtatcgccatcacaaacatggcattatcataaatatcgaccgcccattttgttttttcattgatcgccacgccccagccggtttcgggttgcacgtcgccccagtcgatggtcgtagcgcctttaatcaatccgtatttttctgaccagcgctctttcagcagataggccatagaggcttccatccgttgcaaaatcgttttatcatttatggccaaaaaaaggaaggctttatcgccggtaacagccacatattttctaaccgcctgtatcagggaagattcctggtcggtttccacggtattcttatgagcggcccattggggagccagatcggagtaccggtactggtagcccacagttgccttttcgcgtggaataacgccgtcgggtatatttccatctgtgccttgcatacggaaaaacagcaatagcatttcttttacctgatcatgaggtaatacctgcagcgagccattaatgaaagtattgaaatccctgatccatacttcgccgtaggaagtgccggcagagaaaccggtgagtagtcttaatgcgcgggcctgtacagtatccagccggctatctgctaatacagctgccgccagggtcctggtgttatcctgggcagtcgcgtttcccgaaaggaatacaggagcagtgatgccagcaataaacggaattatagaaaagacttttttcataatgtggccccggatattatgtacaaacatataaacataatttaattattgcaagaaaagtttttaatatagctataacaggcaacttgctttataagccgttgattatctggatgctatatcatgatggacggcaggacaacaatcctccgcagggatcctgtttttttctccggaacatacatacgttcaaaataaggggggctaaaattgtttttcttgtttatttccagttgctttgcaggcatgaatttgagtatagatcataaaaatcctttaccacttcatatacaggcggaaaacctgttgaggaatatgataaaagatccacagtacgcaggtggaaagtttttacccaacgaagtccagttagcaaaacagctggctatctcccgatctactttacgtcatgctttaaacaaacttgtatacgaaggattgctgacccggaaaaaaggagtaggcaccaaagtggcggaagctgccatcagctctaaatccaagaactggctgagctttacacaggaaatgactgcgcgcggcatcatcatcaaaaattttgagctgcatgtcacctgggtattaccggatgaaaccatcgccaatttttttgagatcagtccaactaagaaagtacttaaactggaacgcctgagagggaaggcagaaggccctttcgtatatttcatttcctatttccatccacgggtagggttaaccggagaagaggatttcaaacgtcctttgtatgacatcctggagaaggattacatgacggtagctactttatccaaagaggaaatcagcgccagatcagcggacaaatttattgcggctaaactggaactggaacctggccaccccatccttgtaaggaaacggtttgtatacgaccagggcgaacgtccgattgaatataacctgggttattaccgggcagacagcttcgtgtataccgtggaaagcagaagagaatagtttaatctttcatcaaaatacaacggctcagcattaatacacaggtattaatactgagccgttctgttttacggttacgggcactgtttatagcttaggagcggctgccacgttttttgtaactaccggccatacacctggtgcagggaagcttacgcctttgttagcgcctcttacgcccgcatcctgtccgaagtaatacagcggccagcctttgtaggttaattgttttttgccagcaacggtaatgctgccaaatagtgttttatcgagagtagacggtactacgatctggtctgtttcataaataggccataccgcattgttggaaaaatcaggtttggtgaacttgttgatattaaaactgtctttaacgaaagagtaaagtgtaagacccttaccatcactgaaatacaacgttttaccggtaccctcggtgtggttttccaggtagtttttaccatcggcgcctaccagctgggcattgatcaactgtatggtatagtcaggtttggctacataccagatattgccaacgccttccccatctgttttaccgggcgcttcacgcacatttacgccacccacagcaggcgcaaagtaatacaggggccatcctttgtaagcagtttgttttttgccatcgatagtagtgatggtggtgaagtctttgatgtccagaccagtgccaagtgcagtctgggaaaggttatcgccggcataataaagaggccatactgctgcgcatccaccggcgcagttatttttgccatcaaagtcgttggagaaataataaagggaattaccgtccacatctgtcaggtgattccccaaagtggcgctggcactgagttgtaccaagggcttaggcgcaggagtgtcgggattgtcatcgtttccgccgcaggcgctgaagaaaacgataccagacaaggctatcaatgaaagcagggtgttttttacggagttcatgctgttaaaattttttttgaaatttgaaataatcaatacgctattgcgggttgttggtcagtaacaacctgtttcggtaatccgtacctatgcgtattcgataaaaacagtaaaaaggttgtctcccccgcaaaatattttcagctatttttgttgctatggtcaatgagcgtttctattcagagcaatatgaatcacaggaaaaggatacccggcttgtaatggacgtcatgtctgtgtacctgtatcccctggaaacatttaccattacagacgctgtgaaccgtgtgggagaaatgaaaggcaccagggtcagcgaaatattgaagcacctggttgcagccggactggccattaaaaatgtaacgggcaattattccctggtaccggaaatgaattttctgctgttcccggtaaatataaagcaacctgcttattcggtgctgctccaaagaacgcaacacgcagtgcatgcgttttacagcatgagcgcccggttgcaggacctgcagcaattgcttaccgcttattttacaggcgaccgctttttattatcacctcctgtaaggaaactggaaatggagctggatgagtatcaaccttatttatcctacctgctgtacttcccggcctatgcagaactgttaccttttttcagccaggaaagccttgaccggatggtatcttttgccttaaaatataacctgctgaaaatgccgccggtggaagaactggagcgttttcgccggcagtatggtgcggattttcctgagttgtcactattacaggggcatcttgatttgcctccggcagataaaacagcagatgacctttatgcacaggcggtgacattactgtacagcgggcaaccggcaaaagcactgacatcctttgaaaaaggaatcaaacgtcaacggcagtacgataaaaagaacagcctgccgctatcgccgttgtttgctttttattatgcattcacactggcggtgttgcccggtgagcaaacgaatccactgatcgctaaaattgtagcggcttatgaacgcaagctgttcccggctattaccccggccgtttgtttgctgcattttcatgcaggccggaaggagaaaggcgagcagttgttattgctgatactggaaggaggggagggcaacctgctcagctacctgtctgtattgtgtttgcagctgctgcatcccaaaagtaaattgttgcgcacttttagtaccaccgttgcaagattgctggcattaggcatggagcgtcactaccggttactgacctacgaatatttatatttatttaagggagatgattaccagggatatgaaagtatgttcatggaagccggcgccattgccgtgcacccaccggtattttcccagatggaacaaacgcccgactgggagcggctattaaatacactgctcggcgcagatacacatcttacaaaaaaagaaaaaaatgtagtgacctcccggttaatttacctgatagattttgaccggtacaaaatccagccggtgctgcaaacttcccagggcaataacacctggagcagcggccgtaacgtagcattaaagaaactgaaggaagggaaggcggaagccatgacagaacaggacttcaggataggcgccaccgtacagaaagatcattattataactacgacggggaatcttattcctttgctgaaacggtatgggaagaaattgccggccatccgttattattttctgcagatgatatcactgtttccgtggaaatagtaaaagcccaaccggagctgagcgttaacaggtcggggcaaggctatactttcagcgccaacgtggatgattatatcagtgaaacggtgtttgtaaaggaaaccaacacccgcctgaagatcatccatctcaccgcgcagcagcggcggctgctgcaaacattgcagcagatccccgtggtgccggcagccgggaaagacaagctgatccaggtgctgaagagcattggtgcgcacctgaccatccatgcggatgtgggcgatatggccgctaatatcagccggcggcctggcgacagccgcattgtaatacagctgctgcctctgggcgatggattgaaagccggtatttatgtaaaaccatttaccagtgacccgccgtattgcaagccgggcattggtgcgcataatattatcggtatcagcaacggggaacgctggcaggcgatccgggacttggcaaaagaaaagagtaatgtaactgccctgctgaacctcatccagggagcaatagaacaggacctttctgatgataccatcatttttgaagatccgctcgactgtctgcaattgctggaaattatccaccagcatcctgaactggtgagggcagagtggccggaaggggagcgttacaaagtgaagcaacaggcaggctttgcgcacctgagcatttcattgaaggaaaaggaccactggtttatgtgtaccggtgaattaaaagtggatgaaaccacggtactcgcattaaaggacctgttggatactacgcgtaccgtaaagaagcggtttattgccttacagaatggagagtacctggcactgacaagcgacctacgccgccggctaaacgaaatggccagcgtggcaaatattgaccgtaacaatgtaagcattcagccctatgccgcgccggtactggacgaattattggaacaggcgggcagcgttactactgatgcagcgtggaaagctttctcacgtaaacgtaccaacgcgatggaactggcagtaacggtgccggttacactccaaaccaccttacgcccgtaccaggaagaaggtttccgctggatgacgcacctggcggcctggggagctggcgcctgcctcgcagatgacatgggcctgggtaaaaccatccaggcgattgccttgttgctgcatcgcgccccggatggccctgcgctggttatttgcccggcttccgtggtaaataactggagcaatgaaatcagccgctttgcgccttccctgaacgtggtgttcctgcataacggtcaccgtgccagcctgataaaagccgccggcgcttttgacgtggtagtgaccacttatggtttactccaatcagaagaaacactgctggccgccgtgaaatggcctacgctggtactcgacgaggcgcatacaatcaaaaatttccagacaaaaacttccaaagcggccatgtcgctgcaggccggatttaaacttatgctaacaggaacgcctatacaaaatcacatgggcgagatctggaacttgtttaacttccttaatccaggattgctgggtacactggatcatttcaataagcaatttgttttcccgtctctaaggaacccggagagcacggtgaagcaacacctgaaaaaactgattacgccttttatattgcgacgtaccaaaacaggcgtgctggatgaattgccgcccaaaaccgagattgtaaagctggtgagcttatcacaggaggaagcgtcgttttatgaagcattgcgaagaaaagcgctggaaaatatcagggcgcaggaaggtagtatggcacagcaacacatccgggcactggcggaaatcagccggctgaggatggcggcttgtaacccgcagctggtagatgctgaagccgatatcccatcttccaaattaatggtattccgggaaatagtggaggaactggtgtccaacaaccaccgggcattggtgttcagccagtttgtaaagcatctcgacctggtaagggaagccctgcatcaactgggaattacctatctctatctcgacggaagtacgccgatatcgcaacgggataagctggtaaaagatttccaggcaggcacagggcagttattcctcatcagcctgaaagctggcggattgggacttaatttaaccgccgctgattacgtgatccatatggatccgtggtggaatccggcaattgaagaacaggcgtccgaccgggcgcaccggatcgggcaaaccaggccggtaactatttaccggctggtagcgcaacatactattgaagaaaagattattgcattgcataacagcaagcgggatctggccgatcagctgctggaaggcagtgaccaggccggtaagctcaacgcccgggaattactggacctgatcgcagaaaggtagctcagaacggcgagggactgatactggtccacccgccatcgatgataaggctttggcctgtaatatgcctcgcctgatcggaaaccaggaacagcgcagcatcggcgatatcctgcgtataagcgggtcgtcccatcggcgtgaggctggaccagatctgttcataggaaggatcgtccagcgtacgttccgtgagggtggcgccgggagcaatggtgttgaccgtaattttaaaaggagataattcaatcactaaattttttgccagcatttccagcgctgctttactcatgccgtaggcagcaagatctttatgcgcctggtggccggttacagaggaggtaaacaggatagcgccgccctgtggctgttgcttcatttgattggcggcagtttgcgccaggaaaaaagtaccgcccagattcacctgcataacgcggttaaatgcttccggtgtgtaagtgaagaagttgccaaacaaagtaataccggcgttggcaatcacaatgtccagccggccaaattgtgtcaccgccgtgttcaccatttgctgaataaaggcaatatcgcccgagtcgccgggcagggctatgcattgcccctttgccgcagtgatagcgccggcagcctgttgcgccagctgtgcatcaatatcattcagtataaccgtagcgcctttcagcgccagttgtttgcttatctcaaaaccgatgccctggccggcgccggtaacaatcgctactttcttttcaaatgtcatgagtcgttttttagtgtgagtccctggttacttcgctgccggagctgcctttcagaaagccgaggtccgcgccaagatgcgcctgctctacatgttgctggtacagttgtacatagccccgtgtggactgtggatacaccggtttccacgcggcttttctgcgcgcaatttcttcaggggaaatagctgcctccagccggcgctggtgtacatccagcgtaattacatcgccatcgcggagaatggcgagattgccgccggcagcggcttcgggcgatatgtgcagcactacggtaccgaatccggtaccgctcatccggccgtcggaaatgcgtaccatatctgtaattcctttagccagcagttttgcgggcaagccgagattacctacttcaggcatccccggatagcctttaggtcctacatttttaagcaccagcacactgttttcatccacatcaagcgcagggtcatcaatccgttttttataatcgtcgatatcctcaaataccactgccttgcctgtatgctgcatcaggtgagcacttgcggcagatggcttgatcaccgcgccctcctcgcaaatatttccttttaataccacgatgcctgataccgtattaaagggagctgctattgatgaaattacgtctttattgtagctgacagcgttagcgtaattggcgccgatcgttttgccattggccgtaatacaatcggtgtgaagatgctccagcagggcgttgatcacagctggcaatccgccggcataataaagatcttccatgaaataactgccggagggctgcagattggcaatcagcgggatattggcagaaaaggtatccatgtcctgcaggttcagttctacgcctatgcggcctgcaatggccagcaaatggatgacaaaattggtggagccgccaatggcagcgttcacccggatggcattttcaaaggcttctcttgtcaggatatccgttaagcgcctgttttcccggaccattttcacgatctcgttgccagacaattgtgccagtattttgcgggcggcatccggcgcgggaatagcggcattctgcggaagggaaagtccgagggattccaccatacaggccatggtagaggcggtgcccattacggcgcagtggccatcactgcggcacatgccggcttctgccatagcgagttcttcgttggtcatcctgccggcccttacatcttcactaaaccgccagatatcactggtgccgatactgttgccccggtgcctgccggtgagcatagcgccgcccgataccacaatggtgggaatgtttacactgcaggcgcccattaccaatgccggggtggttttatcacaaccgcatagcagcactaccccgtcgatagggttggcgcggatagattcttccacgtccatgctgaccaggttgcggtataacatagcagtaggcttgataagtgtttcgcccaatgacattaccgggaattccaacgggtaaccaccggcttccagtaccccgcgtttcacggcttctgccagttcccggaaatgggaattgcacggggtgagctccgaccaggtgttgcaaatacctattattggcttgccttccagctcatgtgaggggataccctgcttctttagccaggcacggtaaataaaaccatctttgcctccgcgggcaaaccaattagcgcttctcagtgaattttcttgcttcataacgggagtggatattttaaaagatacaataaattatggatttcaaaaatgaacagggacagattttgttatcatatggccggttatctttttattaatcttctttctctacatgataagtaggttatccatttaacagatgtttatcactcatggcaacaaaagttcaatttttattatggaattttaatttcatagcatctgtacgataacctgtataatccacaaatgaagaaactatccggattgatcctcggcatggtccttacccactgctgcctggcacaacaagccacggtgaagggtattgtatcagacacacttaatcatgtacagttatccaataccgtagtggcactgcttcaggcgaaagattctatcttatataaattcacgcggagtgatgaaaaaggacactttgaattaaagcacctgcaatccgggaagtacctcttgctgataagttatcctgcctttgcagattacgtagagcctttaacgttatcagatacttctgctgtgcaactcgataatattatgctgacgcttaaatcgcgattgctgcaggaagtcgtgatacagcaaaaagtagctgctataaagatgaaaggagataccacggaattcaatgccggcagctatgaaaccgcggcaaatgcttctgtggaagagttgttgaaaaagctaccgggtatacaggtaaacggcaaaggacagattaccgcgcagggcgaaacagtaaagaaagtgttggtagatggcgaagagttttttggagatgatcccaccctggtcaccaaaaatctgcgtgcagatatggtggataaagtacagttatacgataagaaaagtgatcaggcggcctttacgggtatcgatgatggagaaagatcaaaaacgattaacatacagctgaaggaagataagaagcggggctactttggcaaagtggccgtaggcgccggcgacaacggttttcacgatagccaggctatgttgaatgtattccgcggaaagaagaaactggctgcctttggcattgtgtccaacaccggcaaggtaggcctcgactggggcgaacgggagaagttcggctccggcagcggtgaactctcttttaacgatgatggtgatgtggaacttaatttccggggtgatgatcttgacagctgggatggccgctacggcggcgatggttatccactggtacaaaccgggggattacattattcggataagtgggaccgggaccggcagaacctgaatgccaactataaactgatgaaattgtatatcgacgggaacagtgaaagcatgtcgcagaacatcttaccagatactatttactataatcattctaaagagcatttcaataacaatattctccggaaccgtgttagtggcagctatgagcgacagctcgactccagttcatccgtcaaattacaaatagatggcggtctcgatcataaaatagccaatcggctcagcagcagcgggatggaactgaatgatataaccgtgaaccagggagagcgtaaaacctccaatgtatcggacattggcagtatgaatgcaaacttcttatggcgtaaaaaattgaagaaaaaagggcgtaccatatcactgaacctcgcggagaattattcccgcactaacggcgaaggaatgctggatgcctatacggagtactacaagcagggtaagctggattcggtgcaaaatacggatcagcttaaaaccaccaataatgaaagcattagtatcgtaagtaattttacttacacagaaccattgtctgtggcctcttcgctgctgtttaactatggcattaatatcgataataatcattccaacaggaattcctataaccaacagaccgatggtaagtatactgccctggattcgttgtacagcaatgactacgcctttaatgtgctgacacataaaggtggtatccaatacggctatacgaaaaagaagatccgcattaacataggcggcaatgtgggtcttaccagcttcagccagaaagatatgttccgcaacagtaaggtagaacgggactttgttaactggtatccgcgggcaatgttccggtatagtttttcgcagcaacggcgccttactgttgagtataatgggtataccagtcagcctggcatcgacgacctgcagcctatccgcctgaatgatgatccgctccacctgcaggttggaaaccctgcactgaagccatcttttaataataacttcagtattaattttaatgatttcaaagtaatgaccaatcgaagcatctgggcgtctttgaggtatggatccactacgaatgccatcagcgaccggaccgtgatagatacttcaggagtaagtaccagccaggctgtaaatgtaaatggaaaccggagcgcacagttcaatttatatataggctggaagatcaatccatgggacctgagagtgggaggaagggcaaatggtggcttgaacaggaatgtaaattatgtgaatggtttattgaatactacgaattcttccaatacggggctgggaatcaacctgggtaagtacaaagacaaaaagtatgaatattccctggagggagaggcgaattttaacaacagcgtatcttctgtggataaatctttacggacgcaatactggacgtataatatttcacctaacgtgagttttttcctgccgcttaaatttgtattgcatgcggatctgaactataatatccggcagaaaacagcggtgtttgctaccaacaacaatgctgctatcctgaatgcttatgtggcaaagaagtttggtaagaaagagctggtacagatcaatttgtccatgagtgatatcctgaatcagaatattggcttcaacaggtcggtgtctaccaatacgatcagtcagcggacttacagtaccattgggcgttatggcttgttgtcttttatctggaactttaacaaactgggtgcggcggctccaaaagaatagtgttatgaaaagtatcattacgagaatccgtataatcctgaccgttatattggtggtggtggctgttttcccggcacgggcgcagcacactgcttttttgcagcagggaaggatagaatttgagaagcgggtgaacctgtttgcccgcatggatgaacagagtaaggggcaggataattcatggacggatatgttgaaaaaagggatgtcgcaataccaggtcacttatttcgattattcattctcccgtcaaacgtccctgtataaaccgggaagggataatcctgataataaaaagcccatatgggaatccgcaccggccgaggtgaatgtggtatattcccggctcgatagtatgcaaagtatttcgcagaagcaggtatttgagcagatgtacctggtgaaggacacggtgcgccggatccgctggaaaatcacggatgaaacccgtaagatcgccgggtttgattgccggcgggcgaatgctattattatggactccatttacgtggtggctttttatactgatgccattgttactcctggtgggcccgagtcgtttagcggtttgcctggtatgattctcggtgtggccctgccgcacgagcatgttacctggtttgccactaaagtgttgatagatgatataaaagaagatgcgctgaagcctcctgtaaaaggaaaaccggtagacaataaaggcatcttcgaatccgtttcaaaaatactaggtaagtgggggaattatgggagtgcctatatcagggcaattatgttataattgcagaacgatccggacgtatgatgaaaagtaattctcacatatacacgcctgtacagccgtttgtaaagcagccggaggaggcggtggtataccgggagtttttgccggacctgcccttacaggaatacatttattgttactggcagcttaaaaccacccgcccgcttaccgcgccttttcattaccgggtggtggccgatggctgcatggatattttttttgagctgcatgatcccaggcagagttttgtcatgggattcagcgatgcctataccagttttccgctggaaggaagctttaattatgtgggcatccgttttttgccgggcatgtttccccggttgttccggttaaatgctgcggaaataagtaagcaggtgatctcattagaggatgtggcgccggcggttacccgttttttgcaggattgctttcatgcagaaatgagcgaacagcagttgaaatccctgctggatggttttttacgcgatcacattgcccaaaagatgtcaccggcagataaccgcctgctcgaagcggtggatctgattgtccggcattcgggtgttatcagtcttgaaaaagagctccctcccgggattagctcccgtcagttgaggcgcctgtttgaattttatattggtgacacgcctaaggtattcagtaaggtggtgcgtttccagaagatattacaatctactcattctccggaacacatccgcaggaacaaatcttacctcgatgccgggtactacgaccaggcccattttatcagggagtttaaaacgctttatggccttaccccggctaaagtgtttggtaaataagttgtccgttttttacaatttttcttctcccggctatcctagttttgctgttataaaacttagcagtatatgaaaagatggttattactgattattttctttttttctgtatctaatatttattcacaggtaaaaccaggtaaaatgaaactgaacgcaggaattattacggctaaaatagcggagagtaaaaaattttatacagagatattaggattcggggtgtcttttgaaaacgaattttacctgttgctgcatacaccggataagcaggcggagattagttttttattaccggagcatgcatcgcagcaaccattgtttaaaactgcttttaatggaaagggcgtgtatttgaccatcgaggtcgccgatgtggacaaggtatatgaggctattaaagcgaagggggtggacattaaaatagcgatccgcaatgagccgtggggcgaccggcatttcgccatacaagacccgaatggcgtgggtattgacctggtgacttattcccatccctgatgccattaacataattttaagttaatataatcttaaaagggcgctgattggtatcatacaggaaccatttttgttttacaggggttaaccaaaaaattttaaccatggcaaagcaaagcaaggacacagtaaaacaagaaatccaggtattggcaattggcaactacaaaagttatcctgatgattacgaagtagcacctgccacggtttcccagaatattcagtcattggcgaaaggttattgggacagccgggaatataaagaagtagagcgggatgagcgactgggcatcaacctggaagattatcagcattggacaaaagaagcatatgacgcctttatgaaatccaatcagcagtccatgaactagccccattcaccatttttcgatagctgcagcctgaaagtaaccgctttcaggctgctttgttattatttgatactgtttgcaaccatttctccccgactattgttttaataagacggtggattcactgccataatgtagtgggcactacacctgcttcttattttactacaccataccaagctggtgttcgttaccccctgaatacataggcttgtggctgaacctgccattaatcctaaattttcagtgcatgaaaaagcttatctgtctgttcatgatcctgggcgccggctggcaattaactgctcaaattacgccagctgcagtcgttttgccaactgaggatcttgtaacgcaaatctttggcaaaaacaaagagtcattgttgaatgactttctaagaatttcgcctttggaagaaagggcgtttcaatctgcatttcttgagtacgaaacggaaaagagtccatggttaacggagcgtattgccttgttgaagatgtacaacgaggagttttcctctattgatgaaaagaagatgaattcgcttaccaggcagtttattaacaacgatctggagttcgggcgtttgcagatgcgttatttccggaagtttaacaagctgctgggcgctaccagggcggccaagttctttcagctggacaattacctggaacaatcgacgagggcgtaccttcagaaccagttgccttttataaaagagctggaatctgataaattggcgaaaccgctgacggcgagatagatgcggattttgtcttactcaggattacgctgattatgctgattaattttttgagatttttttcaagattattatattgattaatcttgaaaaattaatcaatataatcagcgtaatcctgagtaagacaacctacgcttcttccacgaaatcctcactccgtggtatggctttgaacttctccatgagttcagggggaagtcctgtgagtttgcgtttacgggtatctatccaggcgccgtctactaatacggtggcggatttggtgccgtcgccccggaaaatttcgtgcttaatggaccagcgggagccatctgcccggcatttggtcatttcacagcttacgcgcactttgtcgttagggctgatttcccggtggtagaacagctcttcccggaaaaggatggggcccagctgttgctgtataaaatgaactgcggtaagccctacctgttcaaggagactaagcctggcctgtgcggcaaagtcggcataggccgagtggcgcaggtgcatattagcgtctatctgtgaccataatactggtccttcaaagaatatgttcatacttaaatttacggaaaagtggtgtaaaaagcccgtgtccaacaggcgggtattatacccgtgacggctatacgtaaattatcccggtagcctgatgtctgccaggggattgcttcctaacgaaatttttctaataaaaaaagtaaaacaaatttttttagaatgaattccttttatactttcgcagcctggagagttggcagagcggtcgattgcggcagtcttgaaaactgttgactgtaacaggtcccggggttcgaatccctgactctccgctgtgagggatagctgaaaagctatcccttttttcttcatcatcagcaccttcttttctccactatgagaagacatttcaagcactgcagggtgctataatcccatccaaatagtaaaaattgctgtcggacaccagtttacaagttcccgctttcatatcggtaagaaggtgaaaatgtttattcaggattttcattttttttgtcaaaagtaaataaatacttacttttaatcatgcggctaagagatcagcataaggaagctttggttaagcagaagacaatggaacttcttgtcagggagggccttgagggtttcagtgtgaataagatcgcccgggaatgccatatttccgtcaggacactttatatctattataaagacagtgatgatctcatcgttcgtattgcaaaggaagaggctaagaaaatggaggaaatgctgttggatggattcgatgcgtcctggtctattgagaaagggctggaatggatgtggaaagcgagagcagactatatgctcgataacgaaacaagcgttcgtttcctggatctactgcggcattccacctatcgcaaaataattttcgggggcactattcaaaagtttcagaaaaccatggaagcgtttcttcaaaatgccatccggaacaaagaaattgacgcgttacccctggaggtgttttggtcgcttgctttttcacccttacatagcctcattcaattacataatgaaagccagtcgaccgataaaaaatttaagctgacgaataaactgttggatcagacgttcaaaaaaatgcttaaaggacttttgcactgattttttttcaccaaatagtaagtaattacttactattaactactatttaaaatagcttttatgaacacaacaacttcttattttttggaggtccccggagccaggctacactatgaaataactggaaagggcccttggttactcttgcttcagggaggcgatggagatgcggacggcacaaaaggaatcgccggtagtctgaaagagcattttacaatcatctcttatgaccgtcgtggcctgtcacaaagcagtctgacaagcccttctgaggagcttacattacgggtacatacagatgacattcatcatttacttctccatcttaccacggaaccggtatatatttttggcaccagcatcggggcgttgcttggaatagactttctcgttcgttatccgcaacaggtacgcttactggtagcacatgaacccccgctcacgcaattcctggataaaacggcggctattaaagcggcggaacagcaggaggaaatcgaaaatgcttttcaacaggggagcattgctgaggccatgcaaaaatttgttgcgctggcgggtctcaattttaaagacaaggaacccgatgcagagttcccgatgccaacacctcaacgaactgccaatcttgctttctttcttcagaatgatgcaccttctgtccggaaataccggcttaaccccgttgaattacaacaagtggcagataagatttttttagcggccggtgctacgtccggagaaaatttagcccatcaatgtactataagtatcgctgaatttttaaagaaagaaataacaatatttccgggagggcacaatggcttcataacacatccaaaggcttttgcgatgttgctggcaacctttctcctgtccaaaccactaggtattgatacaaatgcaaatggttaaaaaacaccctcatattgtcgcaattgcacctcacctgtgtaccttgtcctcgttaactttggacaacaatcaaactaaaacaaataaaatgagaaagatcagaattttcgaacatatctcgctggatggcgtgatagaacatgatggagactacacctatggcgcctggactacaccctatcgaagccctgccggggcggcgatgctctttgaggcatacgggccgaattttgacctgatacttggccgccacacctatgatatatttagtggcttttggcctaatgccggagatttccctatggcaaatgctataaacgctgcaacgaaatacatcgccacgcacaggcccgatagcctggaatggggaccggtgcagcatttgggtgaggacattacagcggcgattcgcgatctcaagtcaacggaaggccgcgacctgatcgttgtgggaagttcgacgttaacctccttgctgctcgaccagggactggctgacgaagttgtgctcattacctacccggttttgctcggccggggtaaacgcttattggctgacagtattgacgcccgggaacttgcttttgttgactcgaaagccacacccaccggtttgcttgtcaacacttataagcacgttggatcgctgaagaaataatctttgccgggatggcacggctaattcattcatatccgtatgatggatgagtatatgaggctattaagatcgccttatctcagacttattctttgatcactgtttgccagcgcacatacgccgttcgatattgaacaataatttatacaaaaatttacaggttttgctcacaatcaatagtttataaatttggcgcacaaatagcaattgttgatcaaccagttagcaataatctaatgagatatcttatcgtcctgacattttgcactatcatatttgccggcaaggcctcaggtcaggccactgaagtttcgccggcgaatgctgccattaccaatagcatcgacagtctcgtacaaacgctgatcaccaataaacaaacagcgggctttatgctgggcatagaaaatgatcaccagcagccttttgtaaaagcatacggcattgcggatcttaccaccggaaaaccagtgaacgtggcaagtgaattccgcattgcatcgatcactaaaccgtttacggccgttgcattgatgacccttgtcgagcaaggtaaagtaggtttgtacgataagctctcaaagtatttcaaagattacccgaaaggtgatagtatcaccatttaccagctactgtcgcatacatccggtattccgaactggtgggaaggcgaaacgcccgccaatacgccaggtaactttcctatgtgtaaaaatccacacttgtacctgcaggctatgaagaaaccatttcttttcgagcctggcacaaaacattcctattccaattcaggatatgtgctacttggagaaatcattgagcaggtgagcgggcttccctatatggactatctaaaggcacatgtattaagcaaagcaggaatgcaccagaccttatgggacgagggccatgacctggacgatacctgggcaaagggttatcagaaaataaatgataccacctttaaggaaccgaccaactatacaatgccatatacggcaggctcactccgaagtactgctgctgatctgatcaaattcctggatgcgctttatagcgggaagatcatcaaaaagagcagccttcagaaaatgacaacgtatgcccttacaagtagtggcaaacctgttgatgaggccatgttctttcccaataactttgtgccgccgccaccgcctgcttacctgaaacgatatggttacggccttggatttacattgaccgagatatatggtacgcctatcgtttggcataccggcggtattgcaggttttaattcgattatgttgtatatcccgaaaagcaaaacgaaaatcatcctgttggcaaatactgaaaatggcgtaatcccaatatgggaacagttgcagcaattgatggtaaggtatcagtaaataaacgagggtatcgttttgtcgcatggagccggtctatactcatgactgtttccgcatgctttgcctgattttttccctgtgttgtcctccccaggcacttagttcgcctatcaggttttttaaagtccggctatagtcagtcgcttcataaacaatgctaaccggcgtggtggggtatacattacgtctgacaaagtcgttcaattccagatcttttagctctttagccagtatcctggaagaaatacccgtgatttcatgctgaatttcattaaagcgctttgatgattgcaccaggcaaaggatcaaagccagcttccatttcccattaataacagatagggcatcaaggacgtttttgagcgatcctgcacatgcgtcgttgtccggaaggggttcatttataatcatctccatggatacaaatgtaattacattacctaaatgtaaccgcttccctttgggtaagtagtgccatttgaccacctggtaaacataattttgcctttgataatccgaacgaaagaattgtttcaccgttaacataaaaagatgtcggtgattaatgaatttaaagttgataattattaaacaggtaaatttttatgaaacgtatccttcatttaatatcaagtctgcaagagaatggatcgcacagcattcagctgggtcgcgctatcgtcgaaaaaattcaggaaaagtatcctggcagtatacctgaagaagtaaacctggtcgatatcgaaattccacatcttacccctgctgtccttcgtacattctttattcccggagagcagctgacagaacaagaaaaagaatccgtccgtttttctgatgagatggttaaacaattattggctgcagacatcattgtgattggtgcaccgctttataacttcactattcataccgcgttaaaggcctggattgatcatataacgagggcaggaatcacttttgggtatggtgaaaatggtcctgttggaaaggttgcaggaaaaaaagtgtatgtcgcaatgtcttccggaggcatttattcagaagggcctggcaaagccaacgactttgtagctccttatctgagtgcttttcttggctttttaggcatgacagatctgacggtattccgggctgaaggattaaaagtaccgggagtgaaggagcaagccatgcagaaagcaattgacagtatagcaattgattaaaatcttcttttaataacaggtagttaatttattgtcctctggaaaaataagccgtatcacatcttccaaaacgatatttgcattttgaaaataatagcaggaaagaaattgtttgataataatggcttatttttcaggacgaaaaagaatttatgaagaagataggatttttatcgtttgggcattggtctaaccacccagcctataagacccgtacagcgagcgacacgttacttcaatctattgatttggctgttgctgcagaggaaattggtttagatggcgcctattttcgtgtgcatcattttgcagcgcagttagcctccccatttccgttgctttcggctatcggctccaaaaccagcaaaatagagattggaacgggtgtaattgatatgcggtatgaaaatccactgtatatggtggaagatgccggcgcggccgatttgatctcggaggggcgattgcaactgggtatcagccggggttcgccggaacaggtaatagatgggtggcgctattttggatatgaactggcccaaggagaaactgacgcggatatggggcgccgtaaagcgttggaattcctggataaattaaaaggtgttggatttgcgcggcctaatccgaacccgatgtttccgaatccgccgggcctgctgcgcctggagccacactcggaaggattgcgggaacgtatttggtggggagccgcttctaatgctacagccatttgggccgccgagaacggcatgtaccttcaaagttctactttgaagtacgatgaaagcggcaagcctttccacatacaacaggccgagcagatcaggctgtacaaagatgcctggaaaaaagccgggcaccagcgcgaaccgagggtttcggtgagccggtctattttcgcattggtgaacgatcaggatcgctatttctttgggcaggaaaccaaccgggtcgataaaataggaatgattgaaccagagaagcgcgccattttcggaagaagttatgcggcggagccggatcaactcataaaggagttagcggaggatgaggcaattcaggaggcagatacgattctgttgacaatacccaatacattgggagttgattacaatgtacatgtactgtcctctattttaaagcatgtggctcccggattggggtggcgttaaattttaatcgacggagaataccgggagtgtctgtcagatactcccggtatatatcacccttcggcatccagtaactcgctttgcctgtcttttacaagctgtgagtgcttcagtccccattcatccatcactactaaaacaggaagaatactttcgccgaaagccgtcaatttatattccgattttttaggataaactttttccgaacacttttcaacaacaccataaaaaagcaattcggctatttgcatttcgataacccgtagtgatgcttcccctatatacctgttgatgtcagctggccggttgatgcccttactgatcgcatctaaaatgcaacatttccatttaccaccaaacaccttacccgcaatccgtaatccgcagtccaaatcttcctctatcttttttgtatacataagtattgtgtttcgagttacaaatttacgcccttaattacttaaaaaggagatcatgtataccgaatcttttttcggttattgtttagaaaacgtttgtcggggaaatttgccatgaagataaaacgtttaaaatgaataagaataaaaatacatccacagcagacaggacttttcaactcaataaaacagattttttaccggtactgattttcgctgctatattttttatgacctggttgtttatgcatggagttaaccattttttagcattaacccccgaagcattaggaaaatattatgatttcaaatggataatcattgcgcatattaccgcaggtggaggtacattgatttttgggataatacaattttggaaaaaactcagaacattcagttggcaactgcaccgtattgtcggtttcatatacctgttggcagtattagtgagcagtacctgtgccctaatattagcatttactacaacgtacgaggtaagttgggcagttgcatttaccttacaaatttgggcaggtgtctggttatccgctaccatcatagcttattacatggcagtaaaaaaacggtttaagctacatcacgagtggatggtaagaagctatatcattaccttggggtttctgatatcaggatttgccttgaaaatccatttcatacaagagctcggaaaaacagaagacatacaaagtcccctattttggatgggctggtcggtacctttattcatttatgaaattataaaaagctgcaaaacaagccattaataatccattttttaagacccgatttttgccacttctgagcccacgaaattttctttttatctgaataatttattagtttagcgtataaagccctgataactcattgcaatgactaagtacccatcattgcaagcgccggctattccattggctgtgcgatcacagatcagcgaccctgaattgaactgaaacctcatataaccatttaaacatttccctcttatgcaacccggaaacaacgacgccctttcgacctctcttttttttgaacagctgcggcagctgacccggcatgaggttaaaagtttcgatccattatcagaagaccatgttgaggtagttttgactgaatattttaggataaacccctatcacatgcctttaagatgccggtttttgaagtggttcaaacagtatgaaaaaacgagccccagatgccacgaagatctggcatatgtcccgatttattttttcccgacgagcaggaattatgataaattatttttaaatttcgtgttaaccgtaacactgattgatatagacgatacatcccagggtgacaggactttcatgacagatttcgccatcaattgtcttgagacactaaaccctgatcccagcctgcccgtaagtgttctcgaatttataaagacgatgatccggtttctatccggggtagatgattacgtaaaggaccgttacctggagatcatggttgatttcttcaaaggatgccaggtggagcatgcgatcgaccggtggtcattaccctacgatcaatatctcgagaacagaaggaacgtgattcttttgagaatgtatacgtatgcactatggatagtggaggacaggtttgggcgtaaggaattcgatttgacattcgatatattgcgtgatattgatgaatggggcgtattaatgaatgatcacctttctgtctggaaagaaatagaagacgaagatccgggaaactggattattataagatgccggaaaaccggggaagcattcagagatgtttatgcagtgcaatttgagcagacgctggacaaaacatatgatttaatcaataagcttcatacaatcgacctggtacatcgcacggatatcgggaaaaacctgctccatttcgttgccgggatatatatttggaacaagtacagcaaacggtatcaggtcagatacagttaagcttattcaataaaagaacctaagtatgaaccacaaagaaagaatgctggccggcctgccttacaaggcatggatggacggactggcagaagagcagctggagaataaaatgaagatctatcacttcaatcaatgcccgccgcatgaaaccaaaaaaatagaacaatacatcagaagtattcttggaaaggctggtaaaaacatattggtgctggctccatttcactgcgactatggtaagcatattgaggtaggggataactttgtagccaactataactgcgtgatcctggatgtggcaaaagtgcgtattggcgataacgttatgtttggtcccaatgtttccctgttcactgcagggcatcctgtacatcccgattcaagaaactccggttatgaatatggaatcggtatcacgattggcaacaacgtgtggattggcgggcataccgtcgtgaatcccggtgttaatatcggcaacaatgcggtaataggatcgggtagtgttgttaccaaagatattcccgataacgttgttgcagtgggaaacccctgccgggtggtacgcaccattacagaagaagacaggcacttttattataaagacaggaaatttgatgtggcggattattgactgaaacctgccggccgcctggaaaaaacaggtggccggcaggaatatgatcaatagcttactttgtaatgatttctatcttccctccttgtttaaacaggtcgtgcggcacaaagtatcctttgtgctctctgccatttactttaatggcagttaagttccggcctttgcccggtttggatatagtcagcaacttgccgttgctggttctccactttacttcatcaaacagcggaacggtaacaaggtattccggatcggtagcggaaaaggtgtagagccctaatgcactgaatacataccacgacgacatttcaccggcatcatccattccacaaagcgcaagcccctcatcgccgatgccgtataaagtatttaaaatagtgtcgatgatcttttgcgatttttccggtttcccgataaaatagtatgcaaacggcgcttcatgatcgggctgattgccatggcaatactggcctatcatcgtttctacatttcttgcaatgtaactggggttccagggcacagtaaacagggaatccagtttggattcaaatcctttggcgccgccatacagggctatcaggccgggcatatcatgcggtgcaaagaaagacacctgccatgcgttggcctcgcggtacatgtattcataataagggtactgtggattgaaatttttaatccattctccattttccagtttccccctcataaagcgggtagacggatcaaacatgtttttgtagttctttgaccttgccatcagcatgttgtagttagccgtgtcgccgagttttttggcaatctgcgctactgagtagtcgtcgtaggagtattccagcgttttggatacgcctgcttttcctttcgtttctacgtgcgggttagttacatcaggatcgctgatgaatcccttttccatatattctttgatgaatggccgcgccccgccttcaacggtggcgtttttcagcagtatctggtaggcgcctttgatatcgaaatcatcgatgcctctcaggtaagcccctgcaatagaggaggagccgtgatcgccgtgaaaaaaggtaggtataaacccggttttatctcccacatctttcatagatttaataacatccagcgttacctgcggggagatcaatcccagcagcacatctttattccggtaagtatcccacaacgaaggctcggtataatagttgaaatcagctttggccacctggtgttttgcatcggtatactgcccgtttacatcgctgcgcagggcgggccacagaaaggagcggtacaggcaggagtacaacatttccttttgtttggcagtgccgccttttacctggatagacgataggagcgtttcccacttttgggtagcttctttccggatatcattataagatttgtggccgatttctttctccaggttttccctggcgttttccgtacttacaaacgatattcctattttcagttccaccggacctgtgctgccgttggctaaatgaaccatggcaaagccattgcttttgccttcttccttcttttccagttgctcaatattggtgttgaggaccgcatagaagtagatcctgccgcctgcctgctggtagccctgcaacgcggaagcccctacctgctcaatgttccagccgtttaccttattattggccctggcaaggtcaaaaaggatttgccggttcgtgttatttttatattcataccggtggtatccgcatcttagggtggaagtaagacttacgttcacatcataatcatccaggtacacctgatagaatccgggtgcagcactttcctttttatgggagaagtgagagccgaatttctcaccgggatttgaaaccggcagcacgggtatattacagaggttccagtgacctttattggtatgggtaaagccgtaaatcacggagtcttcatactcatagcccgcgccggagccatattctgtcataggacttaactgcaccattgcgttgggcaaagagctgccggggaaggtgagtccggcccatgatctccagccgtccggcaatttatagccaaggattttagggtccgtcatgggcgcagtgccgatgaaagtatttacatattttgtataggtttgactgctacctgtaaaggaagtaaaaagtattaacagtaagctgcttaaatgatagatcgtgtgttttctcattcggatgtgtttattattattgttcgccggtgtacctgatatcaaagaagctgaatgcagcattttcatccggggtgccctggaagttcagtcccggccgcgggctgcggtcccacggtgggagaaaccctatagggtatgctgttttacccggcgtaagctctttccagtttgcctgttgtttccaataaaccttacaggtaaaatcaggtagcatcgccattttcaggtataccggcttaccggtatccgtgattttttgttcgcccagcacatttctttttccatccttcactacccagaactccactttatcctggcgaacagcaatgccaacagcggcagatacatctccataaataattaatcctttgctggccttattactattcaatacggcggtactgatttcataagcggctgcataaggcctgagggtgagcgctatgccggccgtatggtggctgttgtataaccccgacacctgcaattgcgcccctgtttgccggaataccggcttcatatttctaaaatcccactgccagaaaattttccctgttggtttggcaaagttataatgaagatgaatgttctctttgcttttcggttctaccggaacgggcttcagctccggccattggtttggtttccacgacaatgctgaaattaatgcttccctgccggtaaacacattgctcgctttgttataggcatggtagatatagaagtcgttgccggcggtgtcctttacaaaggtgccatgtccggggcatttccaggcgccattgtcagacagcacaggattgttggtatcttcttcatatggtccggtgatagcggttgcgcgggctacattcaccaggtagctgcaggatacgccacaacagttacctgcggagtaaaagaggtaatagtagttacctttttttataatgctttgtccttccatgcctgaacgggcatcatctttcaacaggctgaagggattgcccgtcagcgaaagcccgtcgtcggagagtttacttccgaggatctcaatcggtctgtcatccaggccgtaggctttccaggtgatgtataattggccgttgtcgttgtacacaaatgcatcaatcgcctctttgccgtattcgatgatgataccgtgatctttgaagccatgatcggggtatgcggaggtggccacgcctatgcaggaaacgccatccgtttttcttttagccgtataataaacgtaataggtattgtggtgatagaagtattcgggcgcccagaaggacgaggaggtccaggagggagctttatcaaataagaaacctgtttgttcccattgctgcaggttatttgaccggaagatcggaaaatgcggtccccattcgctggaggtgccgatagcataaaagctgttgcccttccggataatggaaggatctgcaaagtcgcccgggatgtttgcccgcacctgctgggccattgaaggacgaacaccccccagaaggatggaaatagccagtgcaagaagtttaaatctcatctgtatgatcatttatggatagccgggtaaggtggattggaaacccggtgggaacaaaaatagaaggttatgtggatgttttttcgttaaaacatctcattccttccttgtaaagtctcattgtagggttaaaacttatcctgggtatgcctgaaaacggtcggacagttaaaaaaaacgtgtgagtatttcaaaccaggcggcagtggttaaaaagcccaccaggatgctgataccgataattaagtttatcaccctcgtgttcagcctgaactgttcggctattacgccggaggtgaccaatgtaggcatcgccgcctcaaaaatactgatccgggcgatgtcgctgcgttcattaaacaacagggctgctaccaggaccaacgcaggggccagcaaaagcttgtacaacagcaccaccgatacctgggaaatctcttttctccagccattaaattttaactggaggccgatggaaaataatgccagcggcgctacggtggccgccagtttgtcgaagaatggctccgatatagaaaggtcggttaacctgctgagtataagcgccagcacgcaaccaaggaacggaggaaaggtcaggagctttttaaggagaaagcgggcgctcacgaaagtgttattggcgccgcctttcagggcagtaataataccgaaggtagataagatcaggaacgtcatctggtcacagatgatagcgatgcttatatattgctcgccaaaataggcgataatcaacggaaagccaatgaaggaggtattactgtacccacctgccagttccagggtagcacgggtgcgttttgagtattgtttgtgacggcagtagatatgcatgaagcaccagctccccgccaccaccactacggcgcttaccaccggcaggatcatggcgggcgaccagactaccttgggcaggtatttgaaagataccgcgggtaaggcgatgtataatatccaggtgttgattcctttgtgcgcatccggatgaatgatgcgggcagccttcatgatcataccagccgtgatacagactgctatcattataaaattcatcataataccagcaaagctagtaatcagaaagaagggttaattgtactttctggtagtaccatagtacttttttgcagccggattaaacgccttttgctctgaaggcagcgggggtaacatgggtgttctttttaaaaaagcggttaaaataggaaggatctgtaaaaccaagactataactgatctctttaatagtaagcggggaagatgccagcaggattttactttccgtgagaagtctttcctgcagcaggtcgtggacggtatagcctaatttggttttcactatccggttgagattcctggattgcaggttcagcgcatctgcataaaatgaaaccggctttgcttttttaaagtgttgctcaatcagcagggtgaggttacgtatcaactgtttggagctgtttttattttttagttccagcgtatgcttttgttcgtgcagtttatttcctgccagcagcaacagggctacaaagtgaataagcatattaaagtttttcggcgactttaacagctctttttgaatcattgcggtgatatgttcataaagtaccgcggtgtcctcatccaggtccacaaagggttcgtggccgccttgctgcatcatgccgtttaattcttcctgcggatgaaaacgggtgaacagtttatagattggttcatcaaagatgagcatccagccgtcgcgctcaaaatcattcattttatgcacctgcccgggatgaaagaaaaacaccctgttggtcagcatctggtgttcctgtccgtcgatcatttgggtgccatgccctttagtgatccacatgatcatgtaatgatcgtgccggtgcgctaccgtagatagctcatgtacatattggttcatgctgatcaggtgaaccggattggtttccagcaattcctgccgcggaataaaatctttcatagtccggttcaaatttacaatatacccgcatttttatttgcggtaatgataaaagatgccggtatcgaagatggtccacctgcaggctttttgcccgcagcttttcaggccgttattggcccaggtattacaggtatagaagagatgatagctgcctttggcttcataaaaggcatcgtttctgtcgtagttggcattggtggcaatgtacaccggcatttcgccggcaggggtgcggaagctgttgctgatgtactgaaccagccgtgcatactgctctttgttcaccatgatcctgcggcagctttcatcttcgctgatgttgcggtagtaggtggcatggatcgcggcggtgctaagactaaatgctgccttaaaagcggtgctggctttgaggtcagcccaggtaggggtttccaggtaaaagcctttgtcgccccagccaaaggccagccattgtgcggtggtgtctttgccggtggtattactgaagggaatgcgggtgctccagtctatttgtccggtgcgtaccggtaataccaggtcggtgtgtactccgttggtgaggatataaatagcgatatccgcatcggacactatttccctgctggtgctcatgcgtgaaagcgtataggcggccaacaggtaaatgctgatcagcagcaccagggccaacagggaataaccggtaatttttaacatcttcttcaataatatccatttagttcagggttacaaattagcttattttattatttttgccgggaatcagttttcttaaccctggttgttgatattgctatgttcccattttggagtgactattattatctagttattattctgcagattatatgtgtggtgcacgtgctgaaatcggggagaagcagggagtggttattttttatcctgtttatcccggtgataggcgtggtggtttattttatccgcgaaatattgccggatattaccaacggcagtttcggtgagaacctgttacgtactttatggccaaacggacgtatccgggagtgggagaaaagggtacgtatatccgatacagttaccaacaaaatgcagctggcagatgcttatgcacagcaaaagcaatacgacaaagccattgcgctgacacaggagtgtgccaacacttttaccaaagatccgggtattatcctgcaactggcgcggcttcaatttctgaacgggcagtatgcagcaagtattgtgagctttgataaaatgaatacttttaaaggcgtgcggatgagcaaggcagaagatgagctgatgtatgcgcgtgcgctggagcaaaccatggaaaccgccagggcggaagaggagtaccagaaaataatccgggtgcatcattcactggaggcgatgtattattatgggttactgctaaaaaaacagggccggacaagcgaagcacgggcacaatttcaaaaaacgggacaggaaattgatctgcacccccgctatgtgaggcgaacgatccgcaaatgggtatggttatcaaaaaaagaattggctacattataaagaaaaggctccggtggataccggagcctttgtcttaacgctataaattacggcccattaggagagggcaccttaaacacaaatcagttttaaagtacatagtaagcgggtgtttcctcctgctcttccggcacgttgtcctgttcgtgcaacatttgccggagatctttttcaattttcctggcaatggtagttaccggtgtatctgtaggtttattttcaaacggatcctgcaggttgatagccattttttcgatcagcaggaacgatgacgcaatggctaccacgagtggtatttccataaagccgaggacatctattaaggcaaacggcaataacagtataaagaagatcacggtgaaatgggtgtaaagactataagtagccgggaacacggtatttttaatacgttcacatttacccattgcgtcgcagagcctggtcagcgtctggtccagggcaatttgctggtattggtttatccaaccctgttccattgcatgtttcaggtcttttgcatgtaaaagcaacaaggcagccggcacattatcatatctcatcacatagtttaattcccttcttgataataatctgtctacacctttgagcggatcagtcttacgtaacgattgtcccaaactatagcaccatgctgcctgtcgctttacaaagcgctcctggaaaagcgtgaggtcgtccgattgatacgtagtatccatcaggcttagtacctgtcttgtcagtgagcgtgaatcatttacaatcgcgccccatatggttctggcttcccaccagcggtcgtaagcctggttagagcggaatgcgagtaataatgacaacaccgttcccagcaccattggtacagctataggaataaccaggttggtgaaatcatattggtagtaaagaatattaatagccagcgaataaacggttaccagcaggatctctatccttatcttaccaaaaacataatttaaggggatattatttttcagtaacataaccttgcttttttattctgttgccagcaatagtgctgagatggtagacttgtctgccacatatttccgtttctggagttgaattttcatctttggataattgcatttgctgatcagtttctgcggatcatagcttcttttggaaggcgcattaaattcatgatcggcgggttgaatgatcaggtcgatgttttgtgccagcaggaaattgcgtaacgccgcacgggtgttgccatggaagaattcaatcttcagctggttaatggcagatgaatatttgttacggattatttcacacccatcctggaagtcggacgagatgagttccaggtgcctgctgttgcgggtgtaagtcatcaggtcaaataaagagtcgggcatttccagtgcgtgcattaatatgatgtttacctgctcgcctgggtgttgcgctacaatgttatggacataactgagtgagcggatagagaaatctgtgggtatgagtatatttttcatatctggtagcttttataacaacaaaattattgttgtgaaataagtaaccagtaagagcagcgttaaaagatagtaagaatgtggtaagaatttggtaagaaaagcagtcgctacagtgggagttcaaccctgatctcggttccgtgatttacacggctgtttacaatgatgtctcccttatgcatccggataatattcatggccaatggcaggccgataccatatcctttgaaacggccggtattagaggcgcggaagaagggagagaagatatatggcagatcctccgggggaatgccgatgccctggtctttcacgataataatatttttcttttctgtggcggcgagtgcaatggacaccggttcgttgttggaatatttcacagcattcatcacaatgttgctgagtgccagttccagcagttgttcgttgccggggatgattaatttttcttcttcttcggggaacaggctgtaatctatttccactttattaccggggtgcagtttatcgatcgtgttttttacggtgaacaacagttcatcgctgcggatctgtccccattcctgtttcttgccatcaaagccggtttgggcgaggtgcagcaggcttttggtgatgtgttccagtcgccctgcttcatgaaggatatttttcagggagtacacatatttatcctgggtacggtccttattaagcgccagttctgcctcaccgataatcgcggtgagcggggtgctcagttcatgagaagcgttgctgacaaagttattttgtgtttcaaaggcagtttccagccggtccagcatattgttaaaggtattggccagatcgttgatttcatcgccactgtcgtctacatttagccgcaggtgcaggttacgggaactgatgctttttacctgcagcatcatgtgccggatgggttttagaatatacctggagaagaaaattccggcgcctaccaggatgacgctggaggccacggcgcagatgatgaggattttgcgcagccagcccaggtattccacgctgtattgattaatagcggatacgatcacgatatacaatccctgtttgcttttatacagcaccccttcatagaagcggtcgccttctcggtaggtggctttgctttcgcggtgtacctgttcgtagaaggagttggggagggtgagttgttcatctttatgaacggtaccatcgctggctacctgcaggaaatattctttttcagcaggcagtttttcgaggtgttcttcccggatttcgttgtagatcaccgagtcggattcgtaatagggcagggtagcttttgcagtaagataggcgcgtatttccaggcgtttgtagaagtcttcgaacgagtgctggttggcaaaataatacaccagtccggtcatcacgaggatggtagaaatcgttaatccggcaaacaacagcaatatcttagtgcgtatcttcatcggccttattttctttgatcatataacccagtcccactacggtatgtatcagttctgtagggttatatttattaatttttttccggagatagttgatataaacatccaccactttggtgttcatattaaagtcgatgccccatacctgttccagtatttccagcctggacagtactttcctcggatttttcagtaaatattccagcagccggtattctgtggcggtgagctggatatttcttccgttcctgctggcggatttggtgtcggtatccagttccaggtcggccatgctgagtacagctgcggaggtaacgggaacgggtgtatctacgggcgcttttctccgcataaggctgcggatgcgggcttccagttcctgtagtttaaatggtttcaccaggtaatcgtcggcgccgctgtcgaggcccattacaatattttctgttgtccccagggcggtgagcatgagtatgggcacttccagctttgcgttgcggagggagcggcatacttctatgccgttcataccgggcagcattacatccagtataatcagccggaatgatgggttattgagcgccatttgtagtccgctggtaccatcgggggccacgcttacttcgtagcctgcttccgagaggccgcgggtaataacagatactacagcaggttcatcttctatcagtaatagtttcatgaacaacaaatataattctattcgaggtggctcacgcaattaaacagttcgcagttccagttttcatcggagaactggagccttgtgatggaagtatttttcatggcgggggtaggatgcatttgtggcaggagggcatccagcatttgccggataaagctgccatgacttaccagcagtatttttttaccggtattttccgagaggaggtcctgcataaaggaaaggcctctagttactacagactcattgctttccatgccgaggtccatcagtttccagcttggaccccaccggaggatgcgttcttcctcggtagtaccttcaatgaggccgccgccggcttcccctatacgtttatcttcaattacactatccaggttaagctcttgtgcaatgatggccgctgtttgccgggcacggagcaggtgactggaataaatgaggtcccaggtttcgccggtgagccgttgtcccagtttcagggcctgcgtgatgccttcttcatccagcgggatgtctgaatggccttgcagtttgcctgctttattccaggaagtggtaccgtgacggataatagcgatctgggtcatattgggtcttttaatcattccgggggacaaatatatataaaaggccgcggggttaatagttaaaattcccggcgcagatagaattcagcgggtttttgtatattaaaagtataatatatttgttcggagtgtcgcccaatactactttcatccctggctgtttattcctgtgatatcaacatgccctataaccggatccaattaatacagtttccttatttcttactcaaaaattaacatttatgaaacacaatgttcagatgctggctcatgccagtatgcaaaaaatgcaaaaagaatatgctgttatgatgagggagggtgtagcacctttttctttatttcaattatttaaccaggaggaattcagattggatgaattttgccagtcattcaggcctcacccttattcccgtcagcttaaacggggagcccaggaattttgtgagcggtatggtatctggctcgaaaatgcggagcattatgtcacttgcgccatatacctgttccctaccgccaatttgtaccgcatgaataatattcttaagaactgtactgtagatttttttctgaatgatacaatggggcgcgaggttttcacccacctgagtgccaatgaacaggaacacagcaatgcggtcaggcaacgtatcggaagcatggattatccttttgaaaacgcaccggaggctcatggcgtggaaatggcgaacgcagaaatgctgctggatatttaccatacttcgccggctcattggttcagggaatttaaaaaaatgtacaactatcatattgatgtaacgcacctggattgcaacacccattcccttgggcatattcctaccgtggaagaatatattgacatgagggggcatatttccgggatgcatcataccatccagctgatagagtatagcgacggacagtttcttgactggaaatggatggaagcagcaggtcttaaaactgatatgcagcgcctgcagtatgttacggctgctattggctgtttgatgaatgatcttttttcttttgagaaagaggtgatcgacaatagttcagattcgaatctgctgatgatcctggcattaaatgaccccggtcttccactggaggaaattattatcaaggctgccgccattgtacaacaactgctattggaatttggattgctggtgaacagggtgaggaacaggagttatcagcaattacctgccaactcagaaatggtagataagttggatgcacatattgcaggtttggaacgatgtgtacaagccagttgggtgtggcagatttataccaaacgttataaacggccaaattctatctggaaggaaacgcaattagtgccagctattgctgaggcagtttaaacgcattaaattattattgtaattcgccactgagtggatgcagttgctgactaagtacttttatcagaaatttataatcaattggtttttcaataaaggcactggcgccagctgccatcattagctcgcgcgactctaaaaaggcatccccggtggcgataataacaggtatatgtttcaatattggatcctttttcaggctgactaaggtatctttcccatccattatgtccatatggtaatccatgatgatgatatccggtatacgtttcctgctttcctccaatacttcagccccattggccgtcaggcaaatagagcagccggtttgggtaagaaacctggatatcagcagggcactcatttcattatcctcggcaactactacatgaatgtcactcaggtccgtcatctcttcttcatcattgttgtctggtctgatatcatcagattggcccggtaccagcggaagcactactttgaaactgtttattccggtagggctgctttctgcagtaataatgccgttcatggaattaaccttattctgtacaatataaagccccaggcccgcaccttctgtatactttcttttatcggtaataaatggatcaaatatcgttttcaatttatcatccgtgatgtggtcgcccatattaacaatatggatagaccaggtatttttgctggcagcaatgtaacagttaatggtagttcccttgttagagtatttaatggcattccctaacaaatttgttataacctgattgagtttcaaggtgtccgcaataatcacaggagatatttcaccgatactgagtttaatcttgatattcctggtttttgctattatcctgttgatgtccactaatttttcaataaatggttttatttcaaaagcttcgctgttcagtacgtctgaatttcctgattctatctgcgccatatccagcacatcatttacaatgttacgggtatggttgcttgccagtaataattgatcaaccaatggctctatccccctgagctgatcatttaattttatctcccgctttaataactgtcccacaccaaagattgcattcagcggcgttctcagctcatgtgatacctggtatacaaatatctttttaaagtgattactcctctttaactgtttattgacatcattactgtgaacataaggtttgcttaccacaatgataagtgttaaaacgcctgccatcgccgagatgcggaaaataaatgctacgtctttctgaaggtgtatcgcttctgtaaaatgataatggtaataggtttccagcagcagaagaatgcctacggccaccaccagtgatattcttctcgatgttctgtcaggaaatatcaggtatataatggagatcaggaagatgatcattgcctgcagttcaataatattactgagcaatattccaaagtagatggaggcaaaacattgtaccagaaaagtgctggcacctgccattctgtgatatcccctgtggttcagatagatcgctgaaatcgtaaggataaattctatggaagcaggtataagaatagataattctcttgtaaatactataaatatggatcctacaaccaggattaaggaggcaagcaccaggcttagtgtattaacaagtatcatcctggatattaattcatcatctgtttgcccctgtgtacctgctcttgtaattgattttactacttgttgaatccgtttaataattttaatagtcatgttaagcatcgtagggtttaagtaaagttaagctcgggatgaccctaaacaacagggcgataacagtttgtgttgcaggcaaaaaatcttttcatagaaacctaatgatcttctgagggtattatcctattgataattcttccggtgtcctctttatggggtatgaacgccggcaaccaaagttatagtatttattcctaaacttaaattcatttcatttttttcatgccatactcaaataacgatttataagtaatcagtacatttgttattatggaaatgagtatcaatcccaacgaagaaaaaccagtcaaaaaggaagacgaagtaaagccggaacccgttattcacgatggttccggaggcgcatttgaaggcacagagatggtaaccgaagagcgggaagagcaaccccgcccgaatgggccaactccttactgaataatgccgcatgccggtgcggtattaaatccttaaattaggtgtatcaaaaaagtcatgcttatgttatccttggaaaaaatcagcgaattattaggcaaagaaagcgataccctgttgcagcacgaaagcaaaactatcagtaaagacctgctgcatctgcccggaccggataccgtcaataaaatttaccagccttccagccgtaacccgcaggtattgcgcagtttgggccagttatttcagcacgggcgtcttggaggcacgggctacatgtccatactcccggtagatcagggcgtggaacacagtgccggtgcttctttcgccaaatacccggcttattttgatcctgaaaatattgtgaagctggctattgaaggcggctgtaatgccgtcgcttctacttttggcgtattgtcgtcggtatcgcgcagttatgcacaccgtattccttttattgtcaagcttaatcataacgaactgcttacttatcccaacagggcggaccaggtgatgtatggtaccgtggaagaagcctggaacctcggagcagtggccgttggagccaccatctactttggctctgagcagtccgaccggcaaattgtggaagtgtcgcgtgcctttgcaagggcgcatgaactgggcatggctactattctctggtgctacctgcggaacgatgcgtttaagaaagatgtggattaccacctctcagcggatcttaccgggcaggctaatcacctcggggtaactatccaggcggatattatcaagcagaaattaccggtcgtgaacggcggttataaggctttgaatacaggagcgtcttcctatggtaaactggatgaacgtatttatactacactcacgtctgataatcccattgacctgtgccgctaccaggtagctaattgttatatggggcgcatgggactaatcaattccggtggcgcttctgaaggagaagctgatctggcagaagcagtacgcacggcggttattaataaaagggccggcggcgtaggactgatctccgggcgcaaagcctttcagcgcccgatggtggaaggagcggcgttactgaatgcgatccaggatgtatacctgaacgaacagataacgatagcgtagcagtgggagcggaggaatgttcctctgctcacctcacctggccattgccacgtacaaaccatttttccgttaccagtttttccaatgcaaaggggccgcgtgcatgcagtttctgcgtggagatccctatttccgcacccaggccaaatacgcctccgtctgtgaaccgcgtagaggcgttcacgtatacagctgcggcgtctacctcattgaggaaacgctcgctgatggtggtatcgcctgaaatgatggcttctgagtggcgcgaagaatatttttgaatatgcgacaatgcagcgttcgtgtcgggcactactttaacggaacacttgagcgaaaggaattccctgccgaaatcttccggctgcgccgcgaagagatgcggataattgttcttttgcaggatatcgaaggctaacgggtccgcatatatgtcgactgcataatgctgcagctgcggcgccagtaatgccaggaaaccggcagctacggcttcgtccaccagcacggtgtccaatgaattgcataccgacggacgggagactttcgcattggtaacaatggcggcggcctgttgcagatcggcagttttttccacgtaggtgtgacatacaccggcgccggtttcaattaccggtaccctggagttggtgcggacaaattcgatcagttgttcggagccacgcgggatgatgatatcgatatactttacggcagtaagcatttccatcacgaagctgcggtcaacaggcagtagttgcactgcatgttcatctacctcaaactgctttaatacatcctggatcagcgccacgagaatagtgttggtataaaaggcatcggtgccgccacgcagcacgcatacgttgccagagcggatacagagggcggctacatccacggttacatttggtcttgattcatagatcacgcccactacgccgagcggcacggttttcttttgcacgagcaggccattgtcgagggttctttcgagcaccagtacattggcgggatcgggcaagccggcaatatcttccaggctggaggcgagatcgcggatgcgcgcatccgtcagcagcagccggtcctttttggggtcgtcgtccggcatgcggtcgaggtctttcttattttctgtgataatgtcttccgaccggatcaggatcacggatgccagtttgagcagcaatgcctgtttctgtgcatcagggagggtacgtatagaaacgcccgcctgctgcgctttttccagtaatggttgtatcgtttgcatgattgtttttctttataacagcacgatgtcatcggcatgggccacttctatgttttgtgctttgtgttgggtatcgagtgtgtctgaagcaattttagccctgcccacggcaatggcgatattgtcttcgttcacaatttcaatgacttccccgcattcaaacttctccagtacggcctgcacgcctacggcgaggaggctgtgacgcttttccagtgcttgttgtgcgccggcgtcaatccggatcctgccggtaaccaggctgccgctggccagccatttcttgcgggcaggcatgctgcagggctgtggcaggcacaaggtacctgttttgccggcaatagcattgagaatgccatcttctgtccggatcccaaaaataacgaccctgatgcccatccgggtggcgaggcgggcgaaagtgagcttggataccataccacctaagccgagactggatttttctttatcggccagccccagggctgccttgtcaataacatctatttgtggtactacctgcccggacctgtccaatacgccggctacagaggtgctgaacaacagcagcgatgcgccaaaacctacggctatcagcgtggccagctcgtcgttatcagaaaatttcagttccaggctgctcaccacatcgttttcattggcaatggggatgatgttgctcgcccatagttcctcataggtacgctttaactggaggaactggtccctgtcggaaaaatgctggcgttcacaaaggctctgcgctaccgcaatactataaggggcaaaataacggctgtatttattcaataataacggattccccacggctgccgcggctttgcgctcactgatggtgccgttgtaatgacgtaagaactgtttgcccgcggccacggccccggatgaaaccagtacaatatgataatctgcatgtaactctgctacctgccgcgctataccggcaattacggtttcgtcgaggtcaccattctgatgggtgatcgacgctgttccaaattttataactaatatcggtttactcaatttctgctctatttggagcctaaaataatattaaggtggcgaaattctaaatgcataatttattccggataccggaaaagccttaatttgactccttacattgatttaactcgctatatgataaagtttgtcgccatgtttataacagccactatggctgtttctgttatttatctcccagcggccaacggccagcaaacactccgtcagcaaattgccggtatcgctggaaatatctctggaaaagttggcgtatatgcggaaatcctggaaaccggggacactgtttcctttaaccgcgatcagcatttccctatgcagagtgtgtataaatttccgatcgccatggcgatgctccaccaggttgaccagcacaaattccgcttggatcagcctatacacgtaacaaaagacgacctgattgggccgagaggagtaagtccggtgcgggatcagcatccggaagggaattttgatatgccgctggcagaactgatcgattataatatccgcgccagcgacggcagcgcctgtgatgtgctgctgcgcttattgggcggcaccggcaaagcaaatgcatatgtacacaaccttggcgtaaaacagatcgcgattgccaccacggaaaaagtgcaggtgcccagtgaaatgatccagtataagaactggtccacacccatggccatgacacagttgctgaaaatattttaccgggatcctgtgttgtccgacagcagcaggaactacctgatgcacctgatggtgacctccagacccggtgctaaaagattaaaagggctgctgccggcgggcacggtggtggcgcataaaaccggtacttcgtggactacaaacgggttaacccgcgccactaatgatgcaggtattattaccctgccaaacgggcatcatctggctattacagtatttgtgtctgatgcaaaagccagcgaagaagagcgggagggcaccattgctaaaattgcaaaggcggcatacgatcattggaacaaataaaaggaaacaggcagtttcaaaaacgaaactgcctgccggaaattatttcatgtatttcttgtattcgttttcaatatccatgacatctattttgtggagttgattgccatcaaataaccacatttcccaattgtatttaacatcacttaaattgagcgtagccggatttcctttggcagaatgaaaactgattttgccgccggcaggttcaataatttttacaccttttccttccaggaaagcgcgtgcatcggtcatgtaattctggtaatcttcattgatggtataaaatgcttcttccccgttatcttttttcagatgttccagttgaatgctatctggcgtatgaagtatagcgcaggggcgtgtaatctgactgtcactttctgttacggtttgcacgggtggcgccgcatctgttgaaactttttcttccggtattttactttcctggcaggcataaaaaataaaaagcgctgcaggcaagataaagtagtttttcatggttttcatagcaatagttgtttggcatatttgttacaccttacagcagtgtaatggcataaagatagtataaaatataccccgtgcaactactgcgatatgttcatacatggataatctatcagtccttctgctccaccttgatagaaagtgcttttatcgcctggcgccagtggatgctgatgtttgaaacgttctggcagatcgggattagagataaatggccgtccgaatgcaataagatctgcttcatttcgctgcagtgctttttctgcactgtctgctgtaaaaccacctgccaggatcagccagtttttaaactgctggcgtagtaaaccgatataatttgaaggtattggtaaactaccgttggtagattgatcagagagatgaatatagcgtatatccatctggtttagtttcgggatcaggtacaaatgagtagctgtttcttcatcgtataatggtaagttattgtgtgccgcaaaaggagagaagcggatacctacccggtgtgctccggcaatatcaatggtaccttgaacgatctccagtaaaaagcgatttctgttttcaatgctgccgccatatttatccgtgcgtctgttggtatgtggatgcataaattgctcaatgagataaccatgtgcagcatgcacttctattccgtcgaagcctgcagcgatggtattttctgctgctttgaggtgcaacctgatcatttcttctaccgctgtagtgctcatggcttcaggaacgggcatgggcatggggccttgtacggtggttatactgccattggcagctattgctgatggcgccagcaaaggcccgccacccgggagattcagcggatgaccaattcttccgctatgtacaagctggaggaatatggtaccgcctttttcatgaacggcatccgttacttttttccatgcagctatttgctcgttgttgtaaatgccaggcaagcggtagtagcccaccccattggggcttatagcggtgctttctgctatgataagtcctgcgcctgcacgctgactgtaatacgtggccaccatatcatcgggtacgctgttggtagctcttcttctgctcatgggcgccatcacgattctgttatttaatgtgaatgtgtttgaggtaaccggttccagtaatttcattgctatcttttttatagcacaaaattaagtgtgcgtgtaaacatggaacaggtagaatccggggtgattattgtaattttgcaggttatgggagaaagaaatttatatacgccgtttgaattgttccaggcagatatgtcggactgggatccgcagccgaaggtgtatttcttttttgagctcattcatatccgcgaaggcagcgggtttcgtacggtgaacgacaaccggttcccttatcataaaggcagcctgtttttatttaccccgcgtgattgccgcggattcgaggaagaaacgccaacgaagtttgtatcggtccgcttttccgagatgtttgtaggcatgtctcattccgcgcctgaaaaagcacggctgggagaatggctccggcaactggagtacctgtttttttatcacaaccggcaggagcagttattgatcagccaggagaatgattgcaaaatgatcatggcgctcatctgtaatatgatggacgaatatgagaagaagccgccttattaccagcaaaacctgcagcattatgtaagtttgttgttgaacatagtagcacggaatgtggcggaagatataaatatagatggtactgacaacgctactcctttgatcagccggatgatagggtatatccggcagcatatttattaccctgatatgctgaagcaggagcacctggcgaaacaattcaatctttccccacactatatcggagagtttttccggaagcaaacgggggagagcctgcaacaattcattattcatcacaaactcaacctggtgcagctgcgggtgagctatagcgacctcaccattgcggaaatcgctgatgagctgggctttacagacgaaagccatatgagccggctctttaaaaagtattacggggttacccccgcagcctaccggaaagagcaaatccaggccaaaaatgaaggggcggaaaaaaatattcatcgaaatatttcgatatttcaaaaatagtcttacttttgtgtcatggatttagcagttatagaaaaagcagcaaatgccatcgccgacaaacatcgattatctattataatggaggttgttaagaagggaaagctggtttgtggtgatgtgtgtgggtttacgtgtttgtcgcagcctacggtgtcgcatcacgttaagatcctggttgatagtggcgtactgcattctgtgaaaaatgggagatcactggagctcacgctcaataaagagatgatgaaacagttgtctatgttctttttacaattaagttaggtacaaaacgggctgaggtgctaccgggcgggtaaccagcagctttttttatacttatatatattgatacttttaaattaatggattgatagagaaagattttctcttttttttggaaattaaacattgataaacttaaataaatcgatagaatggatcagttacgaaataaaacagctgtcatcacgggcggtaacagcggtataggatatgctacagcagcagattttttggcgaaaggagcaaaggtattaataacaggacgcaaaccggaggccgtacagcaggccgccacagcgttaggaggagagatagatagttttatcgcggaccagggcatcaccgccgattcacaaaaattagcggagtatgtgcgtgaccgttatggcaaaatagacgtcttatttgtaaatgcgggcgtagcggcgttcgagtcagttgccgatgtatcggaagcttctttcgacacgatcatgaacattaacctgaagggcgccttcttcactgtgcagcatttgctgccgctgatcaacgacggtggcaccatcattttattgtcttccgtaaatgcttactccggtatgccgggagcatccgtgtacagcgccagcaaggcaggtttaaactcattgggacgcaccttatcaagagaactggcttccaggaagatccgggtaaatattgtaaaccccggccccgtggctacgcctatctttgaaaaatcaggtattccaaaagaagcggtcaatgaagaacaaatggccaaatcattaccgataggcagaataggacaaccggaagaaattgcaaaactggtttccttcctcgcatcagacgacgcatcatttatcacaggtgcagagtacaatatcgacggaggtatcagtgttcatccattaattggttaacctcaaacaaacatcattcatgtcatctctgaaggataaaatagttgttatcacaggcggtaacagcggcataggatacgcaacagcaaaggcatttttagcaaaaggagcaaaggttttgataacaggtcgtcagcctggtgcggtacaaaaggccgtacacgcattgggccaccctgcagaaggttttaaagcagatcagtcagacatgaatgatatacggcgcctgtatgattacctgcagggccgtttcgggaaaatagattccttatttgtaaatgctggcgtggcgaaattagcaccgtttgaaacggtaacagaggcactatacgatgaattaatgaacataaacttcaaaggtgcttatttcaccatccagcaattacttcccctcatcagcgatggtggctctatcacgctgctgtcggccctgaatgcatattcaggaacacccaatgccaccgtactatctgccagtaaagcagcactgaactcattgggcagaacattatcgagggagttggcgacaaggaaaatacgggttaacacggtgaaccccggtattatcagcacgccgctattggaaaaagcaggattaccggatgaagccagaacacacctgagcagtatcacgccgctgggcagactggggcaaccggaagatattgccagcctggttactttcctggcatccgacaatgcttcgtttattacaggtgcagaatacaatgtagacggcggccttatggtgcacccgttgatcgcttaataaatgatcctggcgttgcagtgtgcagcattgtgtaaatgctgcaccggcagcaaggaccaacggatgttgtctttctgcctgattacacagattataaggattatactgatttatcttttttgatttttataatgataaaagaagattggtgtagttagtgattttaaaatcagaataaaatcaaagaaaataaatcagtataatccttataatctgtgtaatcaggcagaaagacaaaattcttgttgatttacagttaacggttgtttaggatgtttgcgaaccccattggttgcctgccggataccgcttgctatacgggtatctggcagcaactttaaaaactttaagttgtaggtttaacagcggccggaataatcttattccggtcttcgcttttttagctcatcttccggatcagtttccccagcgttttcaatccgtcatccacctgcttgctccataccggaccaaaactgatacgtaaacagttgttgtatttattctgtaaagaaaagatcctgccggggcagaagctgatcttatgtttcagcgcctgttgaaataattcaaatgtattaatggattcgtccagttctacccatagcacacagccaccctgtggccgggatatacgggtactttccgggaagtattcgctgattgcctgggaataccgtaaacactgggtgtgcagcaccttccgcaaattgcggaggtggaattcgtaccggcctatctccaggaaatgccccaccgcggcttgtggcagcgatgcgcaggcgatagagtggttctgtttcatcagcagcaccttttccttgtattttccgggcaaggtccagccaacgcggtagcctggcgccagcgatttggaaaaggaattgcacagcaatacatgaccgtatttatcaaacgttttgcaatttgcaggacgctgtttcgtaaaatacaggtcgccgtaaatatcatcttctatcaacgctatatcatacttcaccatcatgtctaccagcgccttcttatttttatccggcatacaggaaccaagggggttgttgtagttggttacaaacaggcaggctttgattttatgacgcggaatggctttgtcgagataatccagatcaatgccggaaaccgggtgggtaggtacttccagcacttttaacccaaggctttccgccagctgcatagacccataataggcagggctttcaatggcaatggtatcgccggggcgtgttacggccgacaggcacaaagtcagtgcatccatacagccactcgtagtgataatatcatcttccgtataggcgccaccccatgcaagcgacatccgggctatttgtccgcgcagcagcttattgccctgtaactcctcgtacccgatcccgttgttgggaaggttccgcagcgcatgcaccactgccttcgccattttggcggccggcatcaatcccggcggaggcgtagccaccgaaaagttcaggatgttcgggttccgcatatgactgaacacttccatcaccatatcactcacagtggcttcgctggctttttttaccggcaaacaggtacccggcatagcaggcatgcgcctcgaattaaagcggatatagtaaccggattttggcctggactcaatcagccccttcgcctccaggtgatagtacgcctggaaagccgtggttaaactgattccctgctgcttgctgagcatccgcacagacgggagtttttccccgattttcatcacatctttttctatcagctgttcgatattatcagctacctgcaggtacaggtgatcggcagtttttatcatggcaatgttgatctgatctggtcaaaagtacaaaaattaaatctgtgcggattttgtcttggctcaggcggattttgtcttggctcaggattacgctgattatactgattacctggatttttacttttggattttttgggattatttgatttaataataattaagggagatagcggcggatatattcgctgccatctcccttaatcctttataaaatccaaaagtaaaaatccaggtaatcagtataatcagcgtaatcctgagccaagacaaaatccgcggcgatcctacctccgcatcagccggcccaatgtttggatagcccactcctggtcgtcgctccaggggttggagttggtaagacggaggcagttctggtagcggtcctggcttgaaaagagggcgccgggcgtaaatgtgatcccttgctccacggcctcttcgtgtagcttccatgtgttgattttgggggaaagtaccacccataaactgatgccgccgttggggcgcgtcagttgtgtatcttccgggaaatattcctgtattgctttcgtgatctgcatggtttgcatgttcagcgattgccgcagggatttcaggtgaaggtccagtcgctgctggtccaggaatttgctcagtactaattgcggcaacatgctggtgccgccggaagcaatgaacttcagctgtgcgattttttcctggtaacggccgccaatcacccagcctatgcggaggcctgcagcaatggattttgaaaaggatgaacagtaaagcaccagcccttcttcatcataggattttacggttcttggccgctccggtgcaaaatgcagatcgccgtacacatcatcttctatcagtggcacctggtattttttcaggagtttcgccagttgttccttgctgttgtcggggatacaacagcccatggggttgttgtagttgcttacaaaaagacaggcctgtaccttcttttgtttgaaagcgtcttccagtttattgaggcttacaccggttaccgggtcggtgggtatttccaacgctttcatgcccaggctttcaatggccatcagcaacccgaagaatgtaggcgattcaatggcaatagtgtcgccggctttggctacagcgcgcaggcaaagactggcggcttccatagcgccgttggtaacaataatatcctgcggtgatacggcccggccccagttgaggcaatgcctggcaatgtgtttccggaaaggttcatgaccataaacatcaccgtacggaatgtaggaaggatccaattcccgcgctaccagctgcagcgctttctttagctttacatccggcagcagcgatacatccggcagggcgcctatcagcgaaatggttttatgcgattcactggttttccggaacatggccagcttttcattgatctccactttcagcgcagtaggtactggatctgttaccggcggcagttcaggacgcagtttttttgaatagtgtacaaagtatcctgatttttcccgggaggccacccagccctttttctccaggtggttgtatacctgcagggcagtactgatgctgatgccatgctcctggtgcagggatcttacagatgggagtttgtcgcctaccgcatatacgccttcactgatcatatgctggatcttttcagccagctgaagatatataaacccgttgttctttttcatctttccaaagttaatctgttatggtttaatatcgataattctgtatctgttttggtggtgttttttgccgttaatttgtaaccttaaactgatacgcatgactgttgttaaacaaattgcacaaacgctggtacaactctgcagggcatggcagtttccggaagcgcaggccaccctgtttcatgaaaacgcggtgaacctggagccggatggccgcaccaccaccgggttaccggctatcatggcaaaggaacaggcgttcctcgacagcatcacggaaaggcacctgctggaaatctccgatccggttgtggcagatgattatttcgccatacagttactgatggatgtaacagtcaatggcgttggccgccgcatgagaaatgaactttgtatctataaagtatgcgacggtaaaattatcagcgagcagttcttctactaaatcatcttaaaaaaatataattatggaagcgagaatggacgtgtacaaactcctgcccggcgcatttaacgccatgatgggattacagacatttgttaatgaaagcggtcttgataaaaccctcacagaactgattaaaatccgcgcctcacagatcaatggctgcgctttctgcctgaatatgcacaccagggaagcccggcagatgggagaaacggagcaacgcatttacgcgcttcccgcctgggcggaatcgccttactatacggagaaggagcgtgcagccctcgcacttaccgaagcggttacgctgataagtacttcccgtgtaccggacgaagtatacaaagctgcgcaggcggtttttacacaacaggaaattgccacgatcacgatggctattgtggccattaattcctggaaccgcattgcgatcacttccaggacattgccacaggactgattgtacccgccattaccggggcgcctccggctgaagcattagttggaggcgccttcgtgaatatatattatcttcctggcgggtaattttatattggatatgtttaataagatagcgcctgataagtggaagcattttttcgttggtatccccatgggggctgtgcttgaagtggcttcggcaatgatgttcccgggcagcccgctactggcagcccttgtggccctggcagtggtcatcgttatcagctacggctttgagttgttttcattaattaccggcaaggggcactacgacgtaatggacgcggtggccagcattattggcggtatgataggtatgttgccgggggcgctggtgtatctggcttagtcccaccaaatccgcaagaatccgtaaatcaaagatgcccgctttccgtattttcgcgacatggctttgcagaaaataatgatccccatcaatgacccggcgcatttctcctttgaagaatgcctgcgtttcctgggaagatcggataaagaatgtttgcattatatacaccagggaaaggtgcggcgtatgctgttgtcggaaggggagcctgtagtagtggaaattgcgcctggttcaaagaaagacttcctggaagccaccatactggcgcctgccggcgaagcagtggcagaagcgcccattatcaggtatatcacgcattggtggcacctggatgccaatcttcaaccgttttaccagtatacacaaacagacccgctcttaaaagggctcgcagaaaaatacaatggcctgcgcctcataggtatgcccgacctttttgaagccatcacctggccggtaataggtcagcagattaacctcgccttcgcctatacgctgcggcagcggtttatccggcagtttggctatcatgtggtagtagacaataccgatttttatttatacccgcatccaaaggtgatagctgcattaactcctgaccagcttacacccatgcagttttcgcgtagcaaagcattatacctggtggaaaccgccaggcaaatggccagcggcgcgctcagcgaggccaggctggataccatgagctatgaagccgcgcgtgaaagcctggtagcgatgaagggaatcggtaactggtcggccaactatgcgttgatgaagtaccgccgttttccgcaatctgttttattggaagatgttggattgcagaatgcaataaaaaatagattaaatttggaagctaagccttctatgccagcgttacaggagtatacaaaaccgtggaaggagcatgcagcgtatgccactttttatttgtggagatcattattaccccaatagattaatttcatggaagacggattgtatcatctacgtatagactcccccgttggaccgctgctgatcagtggtaccgtacacgttataactgctgtttcttttacagatcaacccgcggtggattttccccaggcgcccgcactactgctggattgcgcgcaacagctgtatgagtatttcgcgggcgaccgcaaagtttttgacctgcctatcgcccaggaaggaaccgcgtttcaacaaacggtgtggcaacaactaattgctattccattcggacaaaccatttcttaccagcaactcgcccgcaggatacataatcccaaaagcatccgcgcagtgggcactaccaacggtaaaaacaaactggccatcattgtgccctgtcaccgtgtaattggcagcaatggcacactcacgggttatgccggtggcctctggcgcaaacgctggctcctggagcatgagcgcactgatttatttaccggcttgttctgataaatctgatatggtcaatatttctaaaactggatctgttttcagataataatttatctcaattttgttcctgcattaccacccgaaaattctcatcaacaacgagtaatcatggaattgaaattgcaggaagaccttaaacatacagatcagttattgcagttaaccaaagatttcagcagcaggtttttatccgcaatagataaactggcagccgataaaaaggtggacatcaacagccgtgtatccgttcccggtacagggttaggtggggcggctgcgttggaagctttccggcaacaatatggcaacagcattaccgcagccgcagggccgcgctactggggctttgtaaccggcggcgttacgcctgccgcactgatgggcgattggctggccgctgcgatggatcttaattcttctgacaaaagttcagttgcctattatattgaaacggaaaccattgctttactgaaagaattattcggattgccggaagcgtttttgggatgctttgtttccggcgctaccatgtccaacttcaccggcctggctaccggccggcaatgggtgggattgcagcatggggtagacattgccgcggatggcgtagccgcgctccccggattaaaagtggtatctgccgtgccacattccagtatcggtaaagccatctccatgatgggcataggacgcaatcacctggtgcgtgttcccgcattgcctggtcgtgaaagtgcagacattgcggcgctgaaagaatatctcgaagcgcataaaggaactcctattatttacgtggccaacgcaggcaccgtgaataccgtcgattttgatgatatcgccgcactggtgcaactgaaaaaggaatatggcttctggctgcatgtggatgccgctttcggcggattcgctgcctgcagcgatcagtggaaacacctgctgaatggatgggaagaggcagacagtatcaccatcgacgcgcataaatggctgaatgtaccatatgatgccgcgatgatattttgcaggcacccgcagttgcaatcggctgtgtttcagaacgcgggcgccgcttacttaggcgatccggcaacccaatttaatttcattaatcatattcctgaaaactcgcgccgccagcgcgctttaccggcctggttttctttgatggcctacggaaaggaaggctaccgctggatcgttgaaaataatatttcactggccaaacaattgggcagcctgctggagacagacccgaattttgtgttgttgtcgccggtaaggctttgcgtggtttgcttcacgctggaagttgcgccggaagtggaagcagaagcggtacaggaattcctggatgcgctgaacgacagcggggtggtatgtatgacggccacgtcgtatgccggcaggcaggccatccgcgcggcattggtgaactggcgtaccagcggaaaagatgtattgatggcctatgacaccatgaaagtactggcggagaaaatagtgaataaatatacttatgcgtaaatcaaatacaaatgcttacatcgcgcttgccattgtaagtattttctggggaaccacttacctggcatccagcgtgggcgtaagacacatgcatggggtgatgctggcaggcataagacaggcggcagccggattcctgatcaccggattttttttactgaagggatataagttaccgggaaaaatagtgttgtcgaaattatttgtcattggtacactcatgttatgcggtggtaacggtttgcttacctgggcgctgaggtacattcccagcggactgggagcgatcattgcggctaccattcctatctggatcaccattgccagctatttcctggtacaacgtacccggcttagtttgcagttgatcattggtatgatcctcggctttggcggtgtggcgggcatcttttataattatttatcaagccttatgaacccggacttccagttcggaatcatcattggtttcatttcctgtatattctgggcattgggatctgtactcactgccaagtggtcgctgggcgtgaattacctgtatggcgcaggattccagatgtttttcagcggaatcatcatgttgctggtagcaacttttttcctgggacagcacgtggaagtagaaagttttacgactgaattgtgggaaagcctgttgtacctggtactggtaggttcggtgttttcgtattctgcttatgtgtttgcgttgaataatcttccgcctgcacaggtatctatttatgcttacatcaatcccgtggtagcggtgttgctgggatggctcatcctgcatgaaagccttacctggttaacgggtgtatgttccctgatcactattggcggcgtgtacctggtaaacagtgcggtgaataaaagtaagaaaagtcttgcagcgactgcaaaatagtaatagctataattttttaaggtagaagttaatagacagatgctcaccccggtgtttaccggacggagcatcttttcttttgttatggaaatgaattaaattgagatggatttttaaatctgttattttatggatgttattcaggcaacggagttacatacgaatgaagtggcggtattgtttgatgcctaccgcagttattatgatcaggcgcccgacttcaaaggggcacttggttttattactgaaaggattgcgcaaaaagacagtgtaatatttgtggtgatgctggatgccgaaataattggtttcacacagctgtatcccatcttcacttccctgggcatgaaaagaggctggctgctcaacgacctatacgtattggaagaacaccggggcatgggcgccggcaaagccttgctggataaagcagcggaatacggtaagtccaccaacgcggcgtggctgatgctgcaaacttacatcgccaacaccggggcgcagaaactctacgaaaaagaagggttcaggaaagacacgaactcctactactattataaagcactttaaaaaacgcggggatcgcggattttgtcttggctcaggattacgctgattatactgatttgcttgattttgtcttttttgatttttcttctgatttttttgatttttatacttaattaaggaagcaactatactagcttacattttacttctaactaatgaatatgtcaataaaaaaataaaagaaatcagaagaaaatcaaaaaaacaaaatcaagcaaatcagtataatcagcgtaatcctgagccaagacaatttccaccgccgaaggcggtcgatccccgcaccacaaagcgatggatacaaccaaaaacccctggaccattcactccagggaaatgagatatgacaataactggatcagcatttggcatcacgaggggttgaaccccgccggtggcgccggtatttatggcgtggttcattttaagaacctcgctgtaggggtggtggcgctggatgatgagatgaatatttacctcgtcggacaataccgtttcccgttaaagcggttttgctgggaaatccccgaaggaggtgctccgctgggaaaggaaacggcgctggacaccgccaaaagggaattgctggaagaaaccggcctggtggcatcccattgggaagtgattacgcgtatggcgctctccaattctgtttctgatgaagaaggggtggtgttcctggcccgggggctggagcagcgggtggctgagccggaagaaacggagcagctgatcgttaaaaaagtgccttttgaagaagcctaccagatggtaaataactttgaaatcacggattccttatcggtagcggctatacaaaaagtaaagctaatgggctatgaaggcttattaaacaaataaacccgttacctttgcagcaaatggaaaggaaatttaacgctttcaaaggtgaaagaaaagacgggcaacgtggtccgaaaaaatatgcaacgcagcggccaaagcaatctactatgattattggccgtcagccgttattggaagccctgagcacggggaagtcgattgagcgcatctttatgctgcgcaccgctaccggcgatatcatacctcaaataagggagctggcccaaaccaacaatattcccgttaattatgttccggtggagaagctcaacgggcttacccaggccaatcaccagggagtggtagccattgccggcaacgttacctacctggatctgcaggatgtgatttcgcatgttacggaaaagggagaaaccccgttgttcctgatactggatggtattacagatgtgcgcaatataggcgccattgcccgcagtgcggtgtgttgcggcgcacaggccatcattattcctgataaaggtattgctgcgctgaatgaagaagctgtgaaatcttctgccggtgcattggaaagtatcgcggtttgccgggtcaacagcctgaacaaagccattgataccctgcatctcaatggtatcaaggtgatggccagtgaaatggaaacagaaataaaattgtacgattgcgatctcagggagccggtggcagtgatcatgggttcggaagataaaggcgtgtatcctgcgctgataaaggcttccgatgtattgttccgtattccgatggctggcaacttcgaatcttttaatgtatctgtggcggccggcatcattttgtatgaagcactgaaacaaagaacggtaaatatttaagcggacccgcgggaacccgcaaagaaaatggtttactatgctaaaactagttgaatgccctcgtgatgccatgcagggctggcacagaatgatcagtacggatgaaaaagtgcagtacctgaattccctgttaaaagtaggttttgataccatcgattttggcagctttgtatctcccaaagccatcccacagatggcagacacgaaagatgtgattccccggttgcagctgtctggttccaaaagtaagctgctggccattgtggctaacctgcggggagcagaagaagcggtggtatttgatgaaatcaattacctgggctttcccttctctatatcagaaactttccagctaagaaataccaataaaaccattgcggaatccctggagcaggtacattccatgcaggagctgtgcattaaaaacaggaaagagctcgtgatctatatttctatgggctttggtaatccttatggagacccttacagcccggaaattgtattacagtgggtagaagaaatggtgaagatggaaatcggcattatatccctcgcagacacggtaggtgttgcagatcctgctactattaccggtctgttcaaacacctcataccggcctactccgacgtggaattcggcgcacattttcacgcggcgccgcacaactgggaagataaggtgctggccgcctatgagcagggttgcaaacggttcgacagctccattaaaggaatcggcggttgccctatggctaaagatgagctggtaggcaacctggcaacggagaacctcatcgctttctgtcatcagcggaaagagccgctcacactggacatgacggcattgaggggcacacagcgactggcagatgctgtttttaaagattaactgtattacatgcaatttcatttaagctttccggtagcgccattgtcttcagccattcagtacgatcatgagctattgctgatggggtcctgttttgcggaagaaataggcgaaaagctgcaggaacaccgctttaataccgtggtgaaccctcacggcattttatataatccacttagcattacaaaagccctgacttcctatctcgacgggaaagtatatactgccggagatcttttccagcacaatgatctgtggaacagctgggatcatcacagccgtttctccggccttacggcggaagccacgctggaaaacattcaccggacgcaggcggccgccacgcatgctattgacaacgccgattggctcatcattacgctggggtctgcgcatgcttatattttgaaagaaaataaccgcctggtgggtaactgtcataaggtgccggccggaaacttttacaaacgcctgctcacagtagatgaaatagtaaccgcgctggataatgtaatgcatcgcttgtttttccgcaataagaaaattaatatactcttcaccgttagcccggtgcgttacatccgtgatggggtggtggaaaataatctcagcaaagccatactactacaggcggttcatcacctggtgaacaagtttaaccggctgttttatttcccggcatatgagctggtaatagatgatttgcgcgattatcgtttttataaagaagatatggtgcatcccaatgaactggcggttaactatgtttgggagcaggtggtgaaggcgggtatcagtcctggcagccaggaattgctgcatagcattgccgaaataaaccgggcggccaatcaccggccttttaaccccgaaagcgcccagcaccgtcagttcctggcgcattatgccgcaaaggtacagcaactgatggcggctcatccgcaactgaagctggatgatctgctgcagcgttttcaatagcaaagcggagggaatgtccctccgctttaccccgtttacaacggaatgcctcttttatctttcagataaataatacctactacaaaacagatgacggcaataccgatcgggtaaatcaatcctgccaggtggttgccggtattggttaccaggatggtggaaatggtgggtaacagtccgccgaaaacaccgttaccgatatggtagggcagcgacatagaggtgtaccggatgcgcgttgggaacagttccaccaggaaagccgcaataggcgcatataccatggttacaaacagtacctggatgaatatgaggatcaccagccacatgatattcatacggcttacggtcagttcctttttgtcagctgtttccttcaggatgctgccatcggtatagctatgcacgcgggtggttttaagtaccagttccccggattcacttttggaagaattactttctatcctgaacagctctgtttgttcctgtttcagctgcacattgccgatattatccatcgctttatagatgggatagtaggcaagagcggccagcagcatgcctgtgagcatgatctttttacggccgatgcggtcggacagggagccgaagtaaataaagaacggtgtagccaggagcagtgcaatggcaatgatgatattggattgcacaaattctatgttcatggttttctggagaaaggaaagcgcatagaactgtccggtgtaccaaaccacgccctgacccattgcggcgccaaacagcgctatcatgaccagtttcaggttttccttattggcaaagctttccttgatggggttggaagaggttttcccttctttcttcatctgggcaaacaggggggattcgtgcaggcgtatccgtatgtaataggacataatgaccagcagcactgacaggaggaaaggtatccgccagccgtagttgttgaaatcatcgggtgtcatgagcatacgggtaaccaggattacgcccagcgatacaaacaggcccagtgtggcggtggtttgtatgaagctggtgtagtagccgcggcggttgtcgggcgaatgctctgccacataagtagcggcgccgccatattcaccacccagggccaggccctgcgcgaggcggagtatcagtaccagtatgggcgccagtataccaatggtatggtagctgggaatgaggccgatagcgaaggtagagccgcccatgatgagcagcgtgagcaggaacgtgtatttacgtcctaccatatcgccgagacggccaaatacaatggcaccaaagggacgcacaataaagcccaccgcgaaggtagccagcgtggcgatgtaggccagctgcggattactgggcgggaaaaacttttcagcaatgatggcggataagctgccaaagatgtaaaagtcgtaccattcaatgagcgtaccagccgacgaggccatgataacctgccagatgttttgcgaggggagcgagttcttcatacgtgttaattgtaaacgccagctttttgtactgagctttttgcggggaataagataatgaatatttacaatgagagcaaatgtccaactaaaaatctcttgtgcttaacatccgggaatgtttataaagccttatctttaataagggccaattatttacaatgaagcagggatcaaaagctcacatcacccgggttctcagtttattgttgttagcttttattacgtgtcactataccgtgaaggctcagcaaacgatcagtaacagacctaaaataggattaacgctcagcggcggcggcgcccgtggcctggcgcatattggtatcctggaggcaatagacagcgcagggctgaaggttgatattgtaacgggtaccagcatgggaagtatcgtaggatcgttgtatgcgatgggttattccgggaacaaaatagaagaggccgcccgtaagctgaactggaacagcctgttctccaatcaacccgttcttactgatatttcctatgaagaaaaacgggagtacaacaaatacatcattgaaattcctttcgaatatggtaagcctaagctggcttccggtgtaatttccggtgaagcgctgtggctggaactggcaaagctctgctggccggtgaaggacatcaagaactttgaagactttaatatcccttttaaatgtattgctactgatgtatctactggtgatattgtaacactcgacagcggggaaatagtgacctgtttgcgtgccagtatggccattccttctattttcacggctgtaaaaatcggcgaccgtaagctggtggatggaggggtagtccgtaacttccccgttatcaccgccaaggaaatgggcgcagatattgtgattggcgccaatgtaagcggtggtttgcgtagagcagaccaactggtgactccttttgatatcctttaccagctgggattttataaagatgcagacgatttcaccaaagccattaaacaatgtgatatttatgtgccgatgaacaaggagctggagaactattccgccgcgagcttcggcagcgtggactctattattgaagcaggccgcaggaaaggaagggagatgtatcctgttttcaaacacctcgcagattcactgaatgctttatatccccagcctccttttgtagccgaccggctcccgtttgccacggatatagaactgagcggcgttcaggtgaacggcctcgttcactcagatcagaaattttttttacaacggctgcatctcaagcccggtggctgttatacgcctgcacagctacgaaatgccatcctgaatgtttacggcacccgcttttataaactgattacgtataacctcgtgccggaaggatatggcaaaagccggatggatatacaggtggaggaaaatccgcttacctacgtgaaatttgcgctgaactataacacttttaccggcgccaatgctattattaatttaacccagcggaatttcattgtgcctaactcccggtcgtttgtgacagcggtgatcagtgaaaatccccggctggaggcggaatatttcaaatacctgggccgcagccggaatttcggttttgggctcagcacctattacgagaataacggtcttaccttttacgatattgattttaataagctacaaccttatcgcagcaagtatgcgaacgtgaatgtggatatgcagtataccttcaaccggaatatgtcggtgggggcaggaacacgctgggagtacattaaatacaagccgcagctgtccaattttatggaggtgcggggcagtaccaaccagctgaatacctatattaatttcggtatcaattccctcaaccagaaaatatatcctaccaggggattgttgctggacctggaagcgggacatatctataaccagcatccgggcattaaagtgagctcgcaaggggtggaacaggactatgatacgcttggtgtaagcttccacgattatcagcgcctggcgctgaacctgaaatactatatcccgctgggccgtaaatcggccatagagctggatggtaatatcgggtataatcttaattataaagaatcagtggttaatgcatttgtcgttggcggtatgaccaatatcacccggaaccaggtgcctttcgtggggatatacgagggggaggtaattacgtcaaaagtcagtgcggtgcaggtagcctggcaatacgaagtgctgcgcaatatctttgctattccaagggttggcgcagccgtatatgacggggaaatttccggtggtggaaaataccaatacctcgccggttatggcctgggcggaggctacagcagccgtttgggacccgtagaggccacggtgatgtacaatgatcagtcgggccggctgaagttttatgtgaacctcgggtttaatttttaacgcggattttgtcttggctcaggattacgctgattttattgattagctggatttttacttttggattttttttagatttttagattttcttaaaataataattaagggagataaaagcgaatatatccgctgctatctcccttaatcttttataaagtctaaaagtaaaaatccagctaatcaataaaatcagcgtaatcctgagccaagacaaaatccgcgctagtgcatccggtcgccgcggacatcgatgttttgcagtatttccgcttccattttcagccactcctgccagcggttgcgcactttttcttccgggaaatattcgttggccaggtcaataaagaggcggtagtgtcctgcttcggagatcatgaatttgcggtagaattcgcgcatatattcatcttccagcccttcgctcagcaggcggaaacgctcgcagctgcgggcttcgatcagtgcaaagatcaacagggcgtcgaggaagctgtcgtctgcatgaccacctttcacccggttatccatcagggcatttacataatcatctttccgttgccgtcctaaagagaggccgcgttttttcatttcagcaagcacctgccggaagtgtccccattcttctgtaacaataggcgccagttcctctaccatccttgttctttcagggttgcgctggatcagcgaaatagcggaagatgccgctttttgttcgcaataggcgtgatccgtaagaatgtcctgtaatgaaatggcagccagattcacccatcgtggatcggtaggcagttttagtccgagtattgatactttgctcatatgaaaatagcggttagcctgcggcttttttgcgaagataacggcaaagtttaaattgtgcatcgataaacacagatcatgagtaaagacagtacttcttttttagcgcagttgctggatgagcgcagggaacagcagtcgttccgcgaattacggctgccgggggataaagtggatttttgttccaatgattacctcggactggccaggaatgcaacagtaagggagtatatacatacgttgatggaggaaaggcacccggcgcatggcagcaccggatcaaggctgctggcgggtaattatgagtggattgtttctgtggaacgcgacctggcagattttcatggggcagcagcaggtctgatctataactcaggatatgatgccaacctgggcgtgttttcctgtctgggccgcaagggagataccatcatttacgatcagctgatacatgcgtctatccgtgatggtgtgcgtttatcggcggcgcagtcgttttcatttgtacacaacgatgttgctgacctggaaaagaaactgaaacatgccacggggaatatttttgttgcggtagagtcggtgtattccatggatggtgatctggcgccattggccgctattgcagccatttgcgggcaatataacgcacacctgatagtggatgaagcgcatgctaccggcattatcggcaacaggggagaagggctggtgcagcatctcggattaacggccgcctgctttgcgcgtattcatacttttggaaaagcagttggctgtcatggcgccgtggtgctgggttcggagatattacgcgattacctgatcaacttctcccggtcctttatctatactacatccctaccacccgctgcactggctgccatagaggcgggttatgccgcatttccgtacatgcaggcagaaagagaaaagctgtcgcagttgattgcgcaattccgcgccggtattgtcaatgcggaattgctgccgggcaccacacccatacaggcggtgctgacacgcggtaatgaacatacccgcggcattgcagagcgattacagtcggccggactggatgtgcggcccatcctgcatcctacggttcccaggggagcggagcgccttcgcattgtattgcatagttttaatacgccggaagaggtggaccatcttataaaagtattacaggcataagcggttatgaatcaaatttgatgtattttacatattacatccgatatgtaatatgagaatcatccccgcagttatcaccgcagccattaccttatcgcttacatacgctttcagtcataaactgggacagatacccccactgggaaagctgttaagtccgcaaacgggcttctggcagaatgctgaacctattggtgaatttccacgtgaacaactggtattaccgggattgtccggcaaaacggaggtttggtatgacgatcgtatggtgccgcatatttttgcggaaaatgaagaggatgcttattatgtgcagggatatgtaacagcgcgggaccgtctctggcagatggaattgcagacctacgccgctgccggccgcttatcggaaatactgggtcctaagctggtgcagtacgaccggaagcaacgccgccttgggatggtatacgctgcggaaggaacggtaaaggaaatgctggcagatccggctaccaaagtggccgtaacctcttatgctgccggtgtgaatgcttttattgccacccttacgcctgccacttacccggtagaatataaaatactggattataagcctgagagatgggatatcatcaaatcggccctgttactgaagtatatggcgcatgacctcgcgggattcgccaatgacctcgagttcaccaatgcgcgccgtttattttctttgcaggactttgacctgatgtatcctgatttccacgaagctacggaccccatcatcccgaaaggtaccgcctatccggccgccaccataaaacccgccgccccgccagacagtgtgctggccaccgcagcagcatatatgaagtttaaaacggataaaccagatccggataatggtagcaacaactgggcagtaggcggcagcaaaacccgctccggcgcgccaatcctttgcagtgacccgcatcttggcctgtcgctgccttcactctggtacgaagtacagatccatacacctggcatgaatgtgtatggcgcttcccttcccggcgcacccggagtgatcatcggtttcaacgaccacatcgcctggggcgtcaccaacggagaagaggatgtgaaagattattacagcatgcagttccgtaacggccgcagcgaatacctgtacaatggcggctatcgtaaagcagacctgcgcatagaagaaattaaggtgagaggcggcgccaccgttcgcgataccgttgcctacacggtatttggcccggttatctttgataatactttccctgataaaacagccgggcaaaccttcctggccatgcgctggaaagcgctggacccatctaatgaactggctactttcaacaagctcaataaagcccgtaattacgacgaatacctggatgcactgaacaagtatacctgtcctgcgcaaaactttgtatttgccgataaagccggcgatatcgccatctggcataatggtcagtatccactccggtggaaggatcagggcaaatggatcatgcccggcagcgacagcacctatgcctggcagggatttattcctcatgaggaattgccgcatataaaaaatccggaaagaggatttgtgagttctgccaatcaacgtccaaccgacagcacctatccatatgccctgtatggagaatatgaccttttccgtggcaagcgtatcaatgaaagattatcagccatgagcgccattaccacacaggatatgatgcagttgcaaaatgatgataagaacctgttcgccgctgcagccatgcctatgatccggaaacatatcgataccagttcacttactgcgcaacagcagccctactggcagctcttaacttcctgggattttatggccacgcccgacagcaaagcagccagcatcttcaatacgctgtgggcgcatcttgaagataccatctggcaggatgaactgcatcccaaagatactaccatcctgacctatccgcagtctatcaccacattgcaattgctgctgcgcgacaccgctttccattttatcgataacatcaatacaccacaaaaagaaacgctatcccagctgttgcaaggtgcatttgcacaaaccgtcactgaactttctgagttgaataaagcgggtaagctcgagctgggaaaggcgcgtggtacagatatcaatcacctttcccgcggcattcctgctttcagcgccttacacctgaatacaggtggtgggcagcatattgtgaatgccaccaagcaaacacatggtccttcctggcgcatggtagtgcagctatcagacaaaacagaagcatatggtatttaccccggcggacaaagcggaaatccgggtagtccgttttatgacaacagtgtaaatgactgggtatcgggcaaatattatatgctgcatattttcagcgccgaggaaaaagatgatcctgtaatccgctacaagcttgtgtttacagggaagtgataaaaataatttcaggaaaatttggctggaaataaataattcctatctttgcactccgttaaacaaaaagacggggtaaaagattccctagctcagttggtagagcaatacacttttaatgtatgggtcttgggttcgagtcccaaggggatcaccataaggagtaaaagtaagtactctaacgtaattaaaaccttgtagaagctgattctgcaaggtttttttgtttttagtggtaaagatgtgaaaagatagcgttgtggttagcaggactttattaaatagtgttaaccgtcactaatgatcaagtaatttgctcaatgcgttttctaactgtttcttatctggtaggtataattgatatttagctaataacacattgttcgttatactacttgttgcatattcaaccaggatatgatctttatatgcccctaataatattcccacaggttcgttatctccttcagatgcttcttcctttttaaaatagttgagatatagattcatctgaccaatatctgtatgatcaatttctcctctttttaaatcaattaaaacaaagcacttcaatattctgtgataaaacaatagatcaagtctgaaatgtttgccaccaatactcatgcggtattgccggccaataaacgcaaatcctttccctagttccaataagaaatgctgaaggttattaattagcttttcttccaattcgttttcaagatataggtgttgttcaggaatattcaggaactccaatacaaatggatctttcagtaaatcttctgcttgctgtacttcgtgcccttcattggccagtcttaaaattccttctttgtcggtacttaaagcaagtctatgaatagcatacttttcatttgccgttttagttctcttacgctccatttttctttttcagattgtttggcgtaaaagctaatttccagatctgaatctgatttgaggatctcaaaataatggctccatgtcatttgtgagacagtgtctcacgttttgggaaattattatataattttctcatgtatagcaggttggatctgctgaatcctttgccataggacgcggtgaggtctttggataacttgtcaaataactggcttccatattcggctttctcgttccctttttgttcatactctacaatatatcgcccgatttcccaataagtatataccaaaatggtatttatttgttgagctgcgctttcccttccggaggctaacaattgtcctattccagaaacaagctgtttatatttttgttccagtagttccatatgaaaaagttgcagagcaaatatactttaaggcatgttaatacagtgtcttaatttgatataaatgagtgctatttgttattatagtgatgtttgaaaaggatggattgaaatgatgggatttctgattcggtttgtcgtaggacaatttctttccctggttcccaataaagcttaattaaagcaatattgaaattggcaaccgcttttagttgagcttgtcgtactttgttttttatttctaatagccaatctttgtaagccttttcagtcataaatttctttgttattgccgttaaataatggccattataccgttatcattggctgataagttaaaagaacgggcatgtagaggtgaatcaatcaacagaatgaaagaggattaacgacctgataacattttggcgtatttgaatggtatttttttattggattaggaataggtgtgcttcgatgtatcagcgctgaggatttaatgacttagagacggtaatgcttgcatacagtgaaggagaaagttcgatttctgtaccataggaatcacgaaaaatgcaaaagccttcaagtcgcaagatttgaaggctttttgctttcgatatttttcctgatttttcacctatattgttagtcccttattgtcagatatatacaagttcaagtgcccatgggcctgactgttcaaaaccatccaccatcttcatgaaagagaacaattgaacggaagaacatcatagcccatgaaacagccaggagaacggtcagttatcccatcaaatcgtacaatttaataaaagggctgctccatgagctgcaagattcaagggtaccttttaaatcccgttttcaggcaggaggtaggtacaatggaaagccccggaggataggtataattcgattccacccgtttttctcactttaccggcaacatattattaatatccacggggaagctgtcgtacttattatacagtctcagatatttggcaggatcaatgggttgttcgctgagtatatccaccagccctcggaagaagccttctcttttctctgccgggttgaaaatgagtgtgagcactacctgttcatccgtatcattggcgaagccatgtggcgtgaaacgtggtacatacacaacagatccgggcaataggtgatgtgtctcttcaccagcatatacagtgagcgtacctttgcctacaataaaagtttcatccataaaacggtggtaatgcaacctggcaccgatggtatgtggtggcagtgtgatttcatatacacccaggtggctgttcgacatttcgctggttactttgaaaacaatggatgctcctcccacttccaaacgctctccttccccgggatgatgtatggtagccttgttggcgagctgatcttccagatagtctatcttcttcataaatttcatttttatgaagacaaaattccgacatgccaacctaaaaaacatttacaaatgttgatacttcaaataaaattataactcggcacgtatgcggctcagttgagtaggcgtaataccaagataggaagcgacttcatgctgtttcaggcggcgttctaacgtcgggaattgttgcaggaaggcagtataacggcttttggcagtgtcatagcgtagtgatatttcctgtggctctttttccacaacccaatgtatctccaggtaacggatatacgacgcggccatatcaggacaaagcattgtcagctttttaaattcatcgaaatcatattctaataccgtggtgttttccaacgcgcggatcgtaaactggctgggactttgggttaacatcgcactcagtgaggctgccagaaatgtttccggaaaaaaacgtttgataaccacatctccattcggcgctgtatagtactgcgagagcagtcctttcacgacataggccaccagccgtggaacctggccttccattacaaatgtttcatggcgtttgtaggtacgccttttaatgatattcgcccaagcctgttggctttcatctgacagcggatgatacatggtcacttttttccaaaagttgttcatgagtgtaaatttagaaacaaaaaattatcaagtcatagatttgaagacttttttcatccaccggccttaatattcgattatttaaaccacatttaatgctgataactcacttagaaacttcagatccggtaaaaaatagttcgatttccgtaccatagggatcacgaaagcgcgatacaattcgaaaaaaatggtatcacgcttttttcttaagagattttgtatttccatattaaaggagcgtacggataaatttaaattccggtgatactaaaacctaacttatttttactatggaaaaataatcatgatatttcaaccggattactggtaagatcaaggtgtcggtaaacaccatccaatactttggcgcctgttggcaggttagtaaaagatagccggcatggctgatcgtaattgctccactgagggttattttatagatacctccactgaaaatgcctgtaagacttgagatatttccagctacaggaaaactatatcccagggaaatagtattttggagcccattgcaaacgatcaccgatgagattacaggtcttcgctgttgacgcatatgaattagaataattacccgttatttcaatggcggtattactgccgttgccagttatataaagaccattaatttctattctttcggaagatgattggatagcaagataggattgggagtagaagaaataattgcccccttaccgcttagttgcttgtttgatggaatgactacagtattgaaggttgtaaatgttctatcttctaatattgcaatgtcagaaagtgaaagtgccgttgttagaagagacgaacagtctattgcatctttagtcccaaaccaccttacatcaataaatgtaatataaatccttttccatctggtgggagtacttccagtttttaccccaattacaacttatactttgttgtttgggcttataagatgaaggagcaacagctacctgttaaatttgttatattagttattaatgatttttgaggacgtttttatcacttcgtaacttaatttaaatacagccattttatttttcttacttattaatagcttagaatgcaacaataccttgttattattgttgtttaaggatattatagtttacattacactttttatggattccgattattcaccgattgatgctgatcattgccgggaggcattgacaggagggaataaagcaaagatatcctggccccggacctatagcataacacccatcagtattaacaggaatatagatatgaattcggtaacattgctgtgcgggcctcctcaggtggtacagcaacgttaacacctgttggcgttcgttcagcaacaggtggtgcaatgttgcaggtagttatgatactgtatctgctgcttccttcaccgttacaggccctggcaaatatacctacagcattacattgctttcatctgcactcactattcccaatggaattagttacttcataagtagtacatcagcgatcgggacggtacgtcaaggcttactgtcagtgctatgtcaatgtagcggcagcgcagccatcaggtatttcatgtcagcaccctcgtttgatgtaacagtaaatcataactaattatttcttccaggcaaggagcatattgaatcgtgtccggaaaaatacagtcagccatatttcacggcaaggcatagtaagggcggtaggtgtaatatatggcatcgccgtttatacatctttacccgctgaaggatcaatataatacttaacaatgcagcggatgtagactataaaacaggaaaaccacatggagtatatacctcttcttaagaaaaatgatgccaaagcagtagaaatagctacagctgatatggatctgttttaagtgaagaattagaggtagcgatttttacggtagctatataaatgctgaatgacatgagaagattgcccatatccattttacactgtagaaatatattgattggttttttgcttttttgtctaagccctcagataaccgctcaaacaatcaccaattatatctttaacgcctcaactggcacttttactgctttggtaacccccactgctaccacctggaccggcaacgttggtgaaggtatttccaacctgatacctataggatttgatttttggtatatgggtacccgttataccaatttatctgcaagtacaaatggctggctgacacttggctccgtggccactgctgctacacccgtcaataatttgctgtcgggaggcgctcccaggcccgtaatagcaccgttatgggatgatcttagcattggagtcacttcaaatgttacgtataaaacaaccggcacaacaggcagccgtgtattcaccctgcaatacctgaatataaaatggcccgacctggcattggcaggcgtgatatctttacaggtaaaattgtatgaaagcaccgggaagatagagtttaagtacagagaggaattagtgctggcgttattgacgtccgcatcagtaggtataacggcaatggctacaggaacagggaattttctgtccatcaatgacgccggcagcagcgccagttccgctgcggaatcaagtgtaacgggcaagcccgcatccggcacaacgtatggcttcacaccaccagtggcaatctctcccggtacgctaacattttccggcgtaacaaatagtgcaatgacgctgaattggacagatctttcttccaatgaaaatgggtttgttatttaccgttcaacggatggtgtaaactacaactttgtttcccaaacaccagctaacaccaactcttcttctcaaactggtttatctgtcaacactacttattactggaaagtatatgctgttacggaaggtgcattaagtacggccttgggtggcagtagatcaaccgtaaattatccaccgctacctaacataggcactgcggttaattttaccctttttacagtgagtggcgcaataggtaatacaggcatctccaatattacaggtaacattggtaccaatgtgggcgatatcacgggactggaaacttcctctgtgattggatccttatatattgccaatactactacggcacagggagcggtagacgtgttgtctgcctacacccaactgaatgcgattcccgtcacttccagccatgctgcggtgctgggcaatggagaaatccttacacctggggtgtataatatacctgcagcaggatctattgcaggtgtgctcacattagacgcacagggagacccaaatgcagtatttgttattaaaataggtgctgcattaaccaccggggctggcacaacggtcagcctggttaacggagcctccgcctgtaatgtattctggaaggcagaaggtgcggtcactatggcggccggcaccaccatgaggggaacgttgatcgcaaacaacggcgccgcttctatgggggccggaggtttacttgaagggcgactgttttccacattgggagcagttactttgggtccggggacggcatcgttaccggtatgtccctgtacgcctgcagcacctgctgttgtcagcccattaacttattgtcagaatagcatcgccgttcccttaacggctaccggaaccaccctgctgtgggaacggggcgctgccacggcgcctacaccagctaccactacaattggcgctaccagttacgcagtgacgcaaaccgttggcggctgtcttagtcagccagctattattacggtgaatattacggcggggccatctgcggtaatttcatatataaactctccctatcgctcggatgcaggcaccgcagcagtagcccgcacaggaacagtgggaggcacttatgcttcaacagcaggtttgtcaattaatagctcaactggtttgatagacctcgccacaagtacgctgggtacttatactgttatctacaccattgcggcagcggcaggatgtaatcaataccagactacgaccagcatcagtatcatcgctccacccagcgtcaatttaggtacagccgccaattttgcgctttttgctgttagcggaggagtgggtaatactggcatatcacaggttacaggtgatataggtactaacttgggcgctattaccggttttgaaacggctattgtggctggatctatgcatacggcaaatgcagtaacctcgcagggcgcagcagatgtgctgtcagcctataaccaattaaacgcattttttcccactgccagtcacgtggccgtacttggaaacggggaaacattatttcccggcatttataatttagccgctgcggggtcagtggctgccaccttaacactggatgcccagggaaattccaatgaactgtttatttttcaaataggaggcgcattcactaccggggcaggtactacagtaaacctggtcaatggtgcatctgcctgtaacgtatactggaaagtagaaggagccattgccatggcagcctccactactatggtgggcacgttgatcgcaaacaatggcgccgcttccatggctgccggtggcatattgaacggaagaatgttttctactttaggcgctcttacgatgggacctggtgctgtaaccattcctgtttgtgtcatggggggcacatggacgggcgccgtcagtaccgactggaataatgccggtaactggtttaataacgctgttccaacttccgctactaatgcaactatcccatccggcgctcccaggtacccgctgttaaatgcaggtaccggcgtggtaaaaaatttaaccatactaagcagcgcttccgtaaccgtgacggacgggtctctgcaaatagcaggagtaatcaataatggcggaacattggatgtatctgccggcactctaagaatgaccggtacagccgtgcagaccataccggccaatgtttttgcaggaaatcagatcaggcaccttaccatcaataacaatgcaggtgtaatactgaacggaactttacagctcagcggagtactgctggtgtcaaatggttcactgaatacaggtggaaatcttacgctgatgtcaaccgtcacacaaaccgcattgattgagggtagcggaacaggagaggtggtgggaaatgttactatgcaacgatacctggcttctggtttcggatataggtatgtcagctcgccattccaggcagccacaatcggaggtttctccaatgaagtaaacctgaatgctgctttccctaatttttaccgatatgatgagaaccaggccgcttccggatggataacggatacaacagccactcatccattggtacccatgcagggatatgccgccaatacaggcgcctcttctgctgcaatgacagccgatcttacaggagtagttaataaccataatatttcgacacccacactctataatcaccatcaggcttatacgctgggctttaacctggtaggtaatccatatccctcgcccatcgactggaatgcaactacaggatggagccgtaccaacattgataatgccgtgtattactttaatgctggtacggctgatcagtatacgggcacctatagctcttatattaatggtatttccagcgataatgtggcgggccctgtcattgctgcgatgcagggattttttattcatgtaacggatggcacttacccggtggcagcctccctcactattaataataatgcgcgtgtcaataacctggcgccggatttccaccgcgtgcctgtgttaaccgtgcctttaatccgactaacagccggatacgcggatgaaaggactgttgtagatccggtagttgtttattttgatgctgctgccccgcgattctacgacaaagaaatggatgcgctcaaactcatgaatacagatgcgctggtgccaaatctgtatatacgttcttcggctgcacccggaatctccatttatgcgtggcccggattgaaagacagtacggaggtaataccactcggacttaaaacagcacaaccgggatggatcacttttaatgcagtggatatagaacgattccctgccggcaggcatatttacctttacgacatgaaaacaggcgtacggcaggatctgcaacgccaaccacaataccggctgtacctggatgccggcgaatatgaatcaagattttttttgggattccagggaaagcctccggttgatccggtatctgccggtggtacattttatgcatacagtctgggtcggatgttatacgcagtgatcgttgaaatgtccgttgaaaaatatgaggcgaccgttacaaatttagcggggaagatagtcgtgcgcaggcagcttttcggcaacggacatcatgagctgggatcgcaattcagcaacgggatctacatcgtaaccttttacacacggcaacaaaaagtgtttacccagaaagtatttattggcaattaatgtttaggcatatgatgcaatcgaacgactgatttgtacaaattgctgcggaaaacttatgatattcttgtgaacaaaaattcttatgagtggtaacgcgctaagtttataatgccattagttctacatgtaatgtaagttcgatacttttggcaacaaaaaatatggcttataccatcgttccgaatcttgctgcttttgcactctaatttaagaggtaacagcgtaactagtctgtttttcagtctattaaagtagcgccaaccctaataaagttaagaattaaaaaagtcaacatgttatatcgttttaagtagagtaaaaagtaaatactctcacgtaattaaaaccttgaagaagcttcttctacaaggttctttgtttatagtggtaaagttgtgaaagataagtaaggatagaaaagtgagcgttacggttagcaatataaatactaaattgtgctaaccgtcacagatcccaaatgttgtgccgcgtcgcgtttgaccaatgttaagcgatgtcaggacaagtgaagttgaaacaatttttgttaaattagaacaagtgatgtctgaccagactttttaaaattgcgcctgactaacaagaaatcggtatttttgaaaacagacattattatccgttttgataaaagatgcaggtatttatacctgtttttgaggttccccgggtatcagctacattttttgtaattacattacagcatctttgtcgtgcattatcaaccaaatcctataaaacacacttaaaatgaagcaacacttctttcctattatcctggtgctgggcctctccaccgcaggatgtaaaaatcagccatccgcgggtacagctaaaccaggaaccgccacccgaaatgattgcaaccagatcacagacagtgtaggccgtgtactggtgaacctcgtaacagcccgtcagagcattcaatcatacgacagcctttgccgcatccactggaaaggcactgcacctgtagaatcctataccatccgtgcggtagacctcctggctgccatggggctgcccccggaactcgccgattcgtctatatgccggttcaaacacatccgggtatatcttgggtttcaggaaaaggtagggttcaagttgtacctcgtaccggtagataatgcctgcctgaaagggaaggaccccagcaaatggaacgccggggtggatgttatactcgacaaaggtgcaaatcccattctcgcaaatattgattcaacaggaacagctgcttacgaccagtacgtactggacctcaacgccccttgtccgaatacctgcccacagccaggaccccttaaagtataccgctgatatatgaacttttcagaaacgataatactgttatcacatgtacccgttttactcactgtagtatatgctgccgtgcactacagcaaattgccccgtgaactgaaagtgttctcctggtttatttttctgtcgggcgtgatacaattcacttccctggctttctggttcgttagcaaaaacaacatgccgctgctgcacatatacgtagcggcaggattcctttgcctggcatggttctataataccttgctcaatggattcatagatgcaagaataatatggtccatcgccatattattcttgctctttacaaccattaactccttgttcattcagcctgttcatactttcaactctatcgcattaacggtagagggcattctcattgtgatcctggcattgttcacttaccggttctttctgagtgatattgtaaaagaaacaagcggccggaatatcagtagtcttaactggatcaattcaggattgtttatctattattcttccagcatactgatattttattttggcgctgttatcactgctttcagcaggaacctgaatttgtacacctggatatttcactcattcttttccattgtcatgtacacctgtttttttatcggcctatggaaacgatcaaagacctgagttttttaaatgcattgctgccactggcggttattgtgttcatcatcggtattggggtagtgttcctgaacctgcattttcaaaagaatttgtctgtgcagaaactcaggcaggaggcattgaagagtagctaccaacaggacctgcttcgctcgaatattcatgcgcaggaagaagagcgcaaacgtattgcacaagacctgcacgatgagctaggagcggtgatgtctattatgcgcatgcatctcatggtgctcgaacagcaaagtgctgatgacacaaagcaattacaggcgcccttgcagtatgttcgtcaattgtcggagacggcgctggcaagtgtgagaagtatcagccaccgcctgatgccgccacaactggagtctttcgggttgaaggccgcactggagtcggtaacggaacagatcaaccgggccggtgaaataaagatcgaactgggttgtgaagcccccatggacgacctgccctggctggtgaacctcggcctgttccgcatcatcatggaaatgattaataatacgctcaaacacgctggtgccagatcgataagaatagatcttttccggcacggccaggaactggtttgttattatacagatgatgggagaggactgtcagatggtaatgccagcaagggcctgggtctaaagagtattgaaggccgggtgaattcgctcggtggaaaactggaaatgggcaaccaggaatcaggcggatactacgccattgtccgattaacattacctgcataatacgttaccatatgaaaaaagagatcaacataggattagtggaagaccaggtgcttttcagagaggggatgaaagcgattattaatacctggcaggatatgaaggtgatatttgaatctgctgatggttactccgtgccggataaattacgtaaggcggctgttctcccggatgtgatgttggtagatctttccctgccaccggatggcgacaaagaatacagcggtcagcacgttacccgggagctcgcggttacctatcctgaaatgaagattcttatcctgtcggtccacgatgatgagaatttcattaaccagttaattcaatgcggtgcacatggttacctggtgaaagacagtgcgccacaggaagtacaggaagccatcattgcggtgtacactaaaggatcttacatcaatgagcgcgcgttaaaggccttgcagctcagaacggtgagaactgtcaggagcaagccgcagaacctctccatcaccaaaagagaggaagagattttgcagttggtatgcagacaatataccgcagaggagattgcgcaggaactttttatcagcgtaaaaacggtgaacggccatcggaataacctgctgcagaaaacaggttcacggaatgttaccggtttggtgttgtatgccatccggaataatatcgtgtcgttgaaatagtattgttatttacgctcgtgagtcaccgcatcatcatattcaccacaatcagatcctcaactgcaaaaataacagcatatcttgtcaaaatcctgcttgttacaccattattaatttttaatctttactgattgttccggagagaataaagtaacgatgatgaataaaaagatattttttgttttgctggtaacgttatatagctgtagcctgtacgcgcagtgggattttcgaaccaactattttaagattcatattgataagcggggctttatcaccagtatgaagaatatcacattgaggccgtaccgggaattcagcccggcagataaaccatcgccgctgatgcagctgtacgatggcaagcaatattatgaaccggtaaaggcatactaccagccatcggataaattgatttcactaacttattccaatgggtcaatagcgcaggtgcgcctcacgcagcatgcgaagtacctgaaactcaccttgctatccttatcttccaaaaacaatattgaaggcattcaatggggggcatatcatacaaatatcaacaaccttttaggagagatcattggtgttgcaagagataccacggcagccgtaaactacgcgataggcatgctggcgctgaatgacaacaccctgggaggtaccatagcaactgtgggagacgccgcgccgtttcaatatatcattcatacaccggatgcaaagcgattcccattgccggataccctgcatgaaggtcaggtatttagtttgggcggaaatggcatcagcgatgtggcgttttatgcgcacaaggagccgtggtaccggattatgtatggtgatgcagcagaggtagatgaacagggacgtatttctgtttcttatcaatccagggatcgctcccgcaaacgggaaattttgttttcactgatcccgcatatggccgcaaataagcccaatcacattgaggtgcagccattagccggtgttgattatattggttcttccgtagccttatggggcagcccggatagtacggcactcctggacgtgctccagggaattgttatatcggagaaattacctcatcctgtcattaatggtaagtggataaaagacccagcctcttttgtgccggacgctcttaccgacggtggtttatacgacagcatcatatcttataccgcccgcctgggatttaaggcgattagtttatacgaccagggatttttgagaccagacaggggagctaacggatatatggatggtagcagatttgaaaggaagccgataaaaatgacggccggtaacaaatcgcacaaggaatttgcagcattggctgcccggcagggtatcctgatcggcagaacacctatcaccaattcactggcccctggcaccatggatgccagtccttttccgagcgacagcctgtgctatcagcaaaagcgtttgcttatccgcaagcttagtcctggggatacggttatccttgtaaatgatccaaaatacatggatgaaattgccagttgggagggacattgcgaagacttgaatatgataaagatcggcaaagagctgatacattacctgggtgtatcggatcagccgccataccggttgctgaacgtgaagcgtggctactggaatacagttccgttaagccatgaggaaggggatattgtttacaaactgcaggtgaccgttaattacggatatgacggggtgatcccaaacatgcaactgcaggatgagatagcaaagtattatggagaggtgtgtaagatcaatggtttggcttactatgatttcgacggacaggaattcctgttcaataacgggcatggttattactccgccaaaagattcttccgcaaaatgtttgaacatgcccgcacagttggcgtgccatatatccgttttaccggcgccacgttgtcggaaggctcctggcattaccagagcatctggaatgttggcggaggaaaaaacctgtatgatgttgataccagggagtgggggagcactaccagccagggaaaagatctgcgtgacgtaacatacgccaatttcttcccggtgggcatgggcgggaactttcctattacggccaaatcaacggtggagcagtacgagcatatacaagccatttctgtggggctgggtactacatatagtatgcggctgaaccagaaagatgtggaaagttgtccgcagaaagatgccatatttcaggtcatccggacctgggaggatgcacgcgctgccaatgcatttccccgccaggtaaagatactgctggccgatccggctaaaagctggaagctggaagttgggaacgacaaaaatacctggagattgtatgaagttaccgggggaaccaaatcacaaccaatacaattgagagccaggttataaaaaaatcaggcatccagcacaaggtgactggaaggcacacaactgcagggcaaacagttatctttgcccggttgaaccatggtaggatggatatatttaatttcgcctcgctgcaattttgtaaggcaggttccgcaatctccaaagagacaacccgaggagatatcaatatcattggcctccgcaaattccaggatagaccggtagcgctgatcccaaagtagttttttccctgatttaataaattctatcatcaattcactggattcctggttgttttgttcaggaactacggtaattgtgccaaaggactcggtatgaatatttgacgcagatacacctgccttctccagggctcccgtgatggattgcatcatagcttcggggccgcagatataatagtccatatgaatatcggacaacaatgcaaacattttctctactgtaataaatcctgtatagtcgtaatgcagcccttcaatacagccagggagtacgtggttgtaaaaggtatagatgttgaaattagcggatgtttttttcagctgagatagctcttccaaaaagctgtgctcatcttgttgattaacgccatagaaaaaataaacctctctttggggattgactttggcaatagttttcaacatgctgagcaacggcgtgatgccaatacctcccgcaatgagaacaagcgggagcatctcttctgcattaatataaaattcccccgccggccctttcgcttccaggtaatcaccttcctttacaatatcgaatatgtaggaagagcataagcccgctcttacaacaccctgatccaggatgcgttcttttttaacagagatacggtaatacccgttgttatagtggtcggaaaaactatagtaccggaaagcaggtatctcttgccccggaatatggaatttgaacattaaatgctgtcccggccggaagaccggaagatccggcgaatttaccggcttcatatacagggatacaacgtccctactttcaaacacttttttaataacttcaaattgcttgtacgatgtcatacatattgcctttaaataatcttaatctgcggcgacctcctgtctgtccgcacgtatgtcgcgataattcatatcataggcaagcactgttgaatctggctcgatgccccaatgctggcatgccttcttataaatatccggccaccagttttcatgtgctgttaaacctgcttcgagaaatttatcataagcatccattaatgctttgctccatgctttgttgccatattccattgcctcattctgtccacctaattccggaacaatccaatccctgcctattttggcatgtaacacttcatcagcccagtcataatcctggattaattcggtcaaccggttggcggtggctatcgctacatcccattcatattttttacctgttttggccggcatcaatccctgttcaataaagtacaaaatggaatgacgctccttactggtcatttttgtattcaacaggtaagaccaggtgatattaaaaggaatagttttccagtcgatatccagtgaagtaaatccgacttctcccatcatggcatgccgggcttcatcccatatctgccggatcatatctttataatagttccagggcttgtccttcgtttcatatacgatactggacatcatttcgggaacatctatttccctcattcgcttgaagtaaagcatgatcgttttgggaagcggtggaaattgcggatccagtaaaaacgactcggcgtttacccgcatattgtatacatccttaaagcgttcatccctcctgggtacaagggagatttcagcgggctgtaatgaatacatctttttgaccggcttttcaatacaagtctgggtgccgtcaagatcacctatggttgccagacagtcggttaataaattaatccattcaccgtatgcttccctggcgttttcatcgataagtgcactcaccgctttttgaccatatgcgtcaatatcttttatgtctgccagcgcctggcggcagatcctgaaagtgggatgatcaaagagccggttgttctccgcaatatgacgttccagtccgcgaaccagcgaagggatgataacaccataaattccccataccaaagcctccgtggtgggtgcatattggacttcatccaataggatatccagtgtttcgtgaggtgttgtgtccatgccatatggaggttgccgcatctcgcgtaccctgttgaaaaatggttcaacatgttctgcgaggtaatgggcatgtaatgaaaaagccattttcaattcatagataggcatagccgctatgcggctggtaaatataagactgagcctcctggccgtccaatgatagcgtttcagcctggctacactttcggtcaccgttagccctttggtaatggcatctttcatttcatgcagtcctaccagttcaggcaggcccttataaccaatataattttctgcaagcatgatgttatctggttttatggtttaattgaattgttattattctttggcgcatacctcaattgttgagcgaaaaatttaagggagttcccaatatgcgctgtccagtacggccactcatgtccacccggaaattcatcatatacatgggcaatgccggctgccttgagttgctggtgcaattgccggttatattcaatcagcgggtcaccgaggccacaatcaaaccgcatggccggcaaatggcaccggtgttgttctattgtttgaaaaacatgctcatcggccgcggataattgccggtagttcgatagttcttcttctgcaaacaatgacatctgttccagggatgtgatggaagaatggccggacataccccggaaaaggctgccatttttagcgccaatacgtaaagcaccaaaaccacccattgaaagcccggttataaataacggggatgcttcggtcacacctgcaatcttttcagacagtgcagccaccacgtcctccgcaatccatttttcaaaatcatacccgttatgcggaagataagcagatccgtcaccccaaagcccatcggagggcatggccagtatcatgggagggatttctccggaacgtatcatttccattacctggagatgcaccccggcactatgcgtccaggcccaggcgctgccataaacgccatgcagcagtattacaaccgggagtacctctgaagcgctgatacccggtggcacaaatatgcagatgtcaccacgtcccctcaaatgttgtgatttaacagtcatgaaccgcaggttggctgattcatatcgtgggtctgaaatttctatggttctgaactttgacatggtcatatctttagccgagtataataactcctttcgcattttttccctgcagcatatcctggaaagcagcttccaggttttctaaatcatatgttttcgtaatcatttcttcgagtagtaactgaccacagtcgtataagccgatgagcttagggaaatcaatttccgggcggcattttccgtaaagtggattgatgtaggttttatcccattcaaacagggtcatgtcgacggtaattgcctgctcaataccactgacctgaaccgcggtgcctccgttgcgaatcattgccaatggggcagcccctaactcagggacagcggtacattcaaatgcatagtctgccccccgtccattcgttaatgcttttacggctatggaggcccgtagcagtcctaagtcctctttactcgccgtaatcgtatgggtggcgccaaaattcacagccatgctcagtctcttttcattgatatcaatagcaataatttttgctgcaccggctattcttgccccctgaatcacactcaggccaacaccacctgttcccaataccaccactgacgtgcctggttttactttggccgcattcaccacagacccgtagccggtcataaccccacagccgataatactggccgcctggaaagacatatccctggaatagttttttacaatcgcggaagatttcaccagcgtgtattcggaaaaggtgccgaggttaaatgaccgctcaatagggactcctttccaggttgtgccggcagcatgtgcatggccgccggaatatactttgccgccggcggttacgggtgaattgttttcacagatattctgattgccctccaggcactgaaaacaatgaccgcagggagtagcccaattgagcaccacagcgtctcctgccgcaataccagtaaccgctgcaccgcatttaaccacaatgcccgctccttcgtggccaatgaccatgggcttaccccatttcagggaatcatagtctgtatgacatataccggcggcttttattctgactactacctcatcagcttccggttcatgaatttcaatttcatcaatcattaaagtgccgtccccgtttgtaagtgcagctttacatttaattgacatatttgactatttattagtttgattacaataaaagaggaggctaccccaaagccccaggaacgtgaaaagcattttaaaatggttttaacaaaaatatcctatcgtccccttgatttaagtgctgattttgatcaattattaccttattttgtcattggctacagatatttttttgtaaaccaaagcacacgaaatgaaagcacagtttgaggctattgcccagcaggaaaccacctccctgaatttccatatccaggaaaaaaaggagtttgattacccctttcattatcatcctgaatatgaattgacctatatactttccagtcgcgggatgcgatacgttggcaaccattttggctatttccgggaagatgattttgtgcttttagggcctcatctgccgcattgctggaggaattcggaagatcagcaggatatggcttctgctattgtgatacaatggaacgaagatttattgggtaatggatggctggataataaagaattcagatggattaagaaattgcaccagctggcaaataaaggcatcaggtttcacgaaaatattgcacaaggcataaaagcaagactactgaatatcgcggcgatgccgccgtttgaaaaactgatatcggtgctgcaaattctcaatgatttggcccaaacagatcaatatgaccttttatgtgaggatgggttttcctataacctgaattatacagaaaacgagcggatcaataccgtttatcagtatgtaaggttgaattatagtaagaaaattaccctgaaagctattgcagcagaggtaaatatgaccgaacaatatttttccaggttttttagtaaggtgatgaaaaaaaccttcttcgcgtttttgaatgaataccggattaatgttgcctgtaaattgcttattgaaacagatatgaatgccaaccaggtggggtatgctgcaggatatgaaagttttcctttcttttaccgtcagtttaagaagtttaaatcctgctccccacaaaaatacagggccgaatttcagaaaacacctcatccatatatcccgtaataaataattgttttatcagtgccgtttttgaatcagttcaggctggccattggaacggatttccaacttcacatctgccccgttttcacctgaatatttcccgtcgaaagtaatttcattcgcgccactggataaaaccggcagcggtttattcagatctacggtttgcagcaattgccattgccggttgtatacctgtattattttgccatcacatttcaggaattggtttctcttcaggcttaccggcaataccaatgcatcctggtgattaatgcctattgatatctgatcgaaagtcacatccggatcagactccttgctggcagcgagtgtaataataaaagacaccggttgggaagccgccgggttattaaacgtgaatgtggaaaaaaccggttctccgggttgtttcatttgttgtgtatgtttaaaataggcgttatatacaggagtcagcttatattgactgcttcctgtcatctccaggtgaaattcgtgctttaaacttcgcatctgctctttctgcgcttcgctgaaaatatgctccatacgggcttgttcccaggtgtttatcaatcccagcaactcgtctttctttccgtgtttccgcaatgtttcgaggctggtagccagtccaaatcctgcattatacccggcgccaagggccagcatccattctatatcttccggggtggtttctgggcgcagactgaaccagcccagcatggagggcatcaggttgcggcggaaaaattgctggttcttgaggcgcaattgcaactggctttctctgaagccggcgtaccagggctcaccccagttcatcctggtgtaaatatgccagaagtagtggccgggcatactggcatcattgatcacttttcctttcaattcgggtgtcaggttatcgtaccaggtttttgtaaacaactgcttcgcatactgacccatgccggaagaccagcagccttcaagtccatcgaaagatatctgcatcaggcccgtttcattaaataaccgtgcaagggttttcgccatttcttcctgcagtgcataatcggtgagaaatactttgtacggatgatccatcagtttaccaacagtatcatttgcggaatgggccgcagcattggtgccaaaggagccgcgctgacaatcaagcagtttccagggagcagaggtggataccgttccataacggataatttcattgcctataactactgactttagcgtattgttttgaaactggttgaagtaaaccgggtcactgatcccgatttcttttgcattggcatcaatagctgcactgagctgtgaataacctacttttgccaaccgcgggtcgggtaccggggttacataaggatcgttggtagtaatgaaattggataatgtatggatacctagccgcactcccttcgcttttgcggtttcaacacactgcttcatagtggtccagttctccggaaattctttcgcatgcagcttaaaatgcccccagttatcaaaaggatcgccatgatagagatagcgaaggcccgcctgtttggtaaccgctattgcttcctgcaggttatcgatgccgaaatccatgatcaggtatgattcagaagcgtgcaaagcctgtttcccccattcgccatccagcagcggatgcggtaatccttctttgagttcaatctgcgaaatagtgggtagcacatcagcattcgcaactccgaaaagcgcgatcttgctgcctgcaacaccgccatctttgaacgcaggggcgaggtaagcgctatgcccccagttttcaataacccggtccttgtcccggttgcggcaatacgcctgcaatacagctccataatcagtaggacgggcaacgtctcctctgaatgactgtttgttcatgtcatcttcctttacatccaccttgttgtggccttcaaacacgtcataggatggttcaatatcgctttcttcgttcgggtatcctccaagtgtttttacattcaacgcctggatgccgatagcaaactccttgttccgtactacgcctactacttcgcctactgtatctgcgatggtaacggggtatggtccccataatatcagctcaatattttcagaagaagttagttgtgtcagttcaaaactgatgtaacgatcgttgcgctgcacttttacttttgcttcgacacccgcctgcggataagataataacagttctgatttttttgcgttccaggcacaactccccggggcaagaatatggccttctttctttatgctcatgagcgcagtcgccttatctgcaaatatgaattccttttgcagcgcaaggctcttcatactagtcaccttcccggaattgtccagctggatactccactgcttcgttttgaaatttacctgtgcggtagccggcaaaacgactaatcctgccagaacagccaggattggaaccaggtgcttgatgagacttctctttttcatttcaatattttagatgagtgtagggagcgcgtttttcataccggccgcaaattgttcattctgcttcttgtatactaatgtatttttatcattttttgccgttttatttactggtgttggattttttaaggaagatgagatgtttgaggtatccgggatcttacggaaaaccgtaagtatcccgatttatagtctgttatattagcaagatctaaataaaacttccaaatttaaaaacgctcactatgggaaaaattgaagcgattaaaccagggccaaaacccaagaaagacaatgacgaattagataaaagaaggagagttacacctgaaaaaaagcccgactatcctcctttaaaacctcacaagcacaagcccagggattaatcacagggattataagcgtgataccattgtatcgcgcttataatttaatccaggttaccgccggaaccaattgatatctacatggccgtcagccgcaagtgttgatggattggtattgaaattaaataatgcaaaccggttggccgtccaatcgagtcccaggcccatttttaattcgcttccaataggaagaaaatccttaccattagtactgtagaaaaaagtagcaacaaagcctttttctcttgtaacggatttaaaccaaattttaggctgcttcaaattaataactgctatagtactatcattcattgccataataatttcttttctgcctgcagcttgccggacggccacataagcatagggaacctggaatatacccaaaccggcgacgtcattatctttcattccactgatatccatttctattgttccttcggaatacggaccttctacccgctgagtcaaagtgttgatggcatgaaacagggtggaggctttgcccgcttttaagcggagataccccggtcgctcagtcaatgaccatttactattatcaggattatggttccattgccattgcaatgccaatgaagtagcgtcgaattcatcagagctggcaggaacagtaatcggggaggagattcctgtaactggtttggggaatatatctacccctatccctttgttaccaaatatgggccagccatcttcccaggtaaccggttccaggtttggcacacgcccgataggaccacgatcctgcataataatagcccaccaggagccgtctttcaattgtaccataccaccctgatgtaagccattgccgggataagtatgatcatcctgcatgattactttcgcttcataagggccatatatgctgtctgagcgcaaacaaacctcccgtccccgcgtgccaccagtagaaccaagtatataatatttgttattgactttgtatagatgcgatccttcaagatatggaaaagcaggattgtcgtagatcttccgctgcggaactttcacggacttcgcgtcactatttagcgctgtaatataaagtgcctgctgtccatgcacaacatatactttgccgttatcatcaaaaaaaagccccggatcatacaggtactcattgaatattgttcttgtccacgggccgtttatatttttggcagtacagatggaaaaatgtccttccttcgtttccatcttaggtgtgcagaatcccacataaaaggtgctgtcgtgatagcggatggtagcagcccaggagccgctcagatacatatcacctcccttcatgtcatagcggggatcttcctcataccttgaaacggcatagcctcccatctcccagtttactaagtcccgggaaaccgcaatagggcaaccgggtacataatgcatactggtggaaatgaagtagaatttatcgtccacccggataatgtcagggtcgggccagtcgccccacatgagcggattagtgaaatatccattgcccagatccggtgtccagctttttgtaatttgtgaggaggcggtagtgaaataccatagcaatgtaaataatactaagatttttttcatcgatcactgtatttgtttttccggtaatgttattccccggtattgcgttcatgttcacggcgaaattatattaaaacaatcgatgttcacgtggaatttatgacagaggcagcccctgcaaaaataccattggtaatggtcaaattaagcgttgtgtaagagagcgggtaatgccgggatttcttaacaggtataagaatcagccatattgcgcgggcactttatctatgtttactcatattcatgaccctttcaattcgtggccggttatatcgttgaagcaaaatagggtatagattgaataatatattcagtactaacaaccacagcgacttgaggattccgaatttaaatgcaacgaaaatattaatccccaaaactatcatcaaaataatgatatgccctaattcagattgttttgtccggtaatgcagatgcattaaagctttggtattcttttccaccgggctggattttttgtttagtttttcccagccaatccaaaccaataatttcctgaaaacatttattccaagagactgatatattttccctccctgttcccatggcttttcggtatagtaaggggaagtaagcggggctttcaatgtttccgtaaagaaaagcacgcagcccatcaacaggaaattaagcgcccaggcaaatgcaaaaccttgcatcccaacgtaataaatgagggcataagtacaggtaatggtgagaattacaatgaaaattaaaatcaggactttccgcattgattactatcgttaagatgataagttgtttcacaacgcacgaatatacggaactctttcattttggttatggatatccttgattcggttatcattgaaagatgatgattcctgagttttgcattgtttattaatcatcaatattatggaaaatcaaatcagatcgtcagcaaacaatcaacttgtagcacttgtaacaggcgccaaccagggcgttggatttcagatcgctaaagcacttgctgccaacggctataccgtatatgttggctcacgtaatcaaagcaacggagaaaaagcggcggccgaaattggtggcaatgcgtatgctattcaacttgatgttaccctgaaggcaacaatcgatgcagcagcagaacgtattgaaaaggaacagggccgcctggacctgctggttaacaatgcgggcatatctcatgcgggaaagccgggcaggacgctggaggagataatggaagatggccgtgctaccaccgcttcactggaagaaatccgcaccgtatgggaaaccaatgtatttggcgttattgctgttagtcaggccatgctgcctttgctccggaagtcagcggccgcacgcatcgtcaatgtatccagcgtattgggctctcttacctggatcgcggatcccacttgctgggcaagggatcattttaacgttgtttacgctgcctccaaaacggctctcaatgcggttacgctggcctttgccatcgaactggaaaaggaaaacattaaagtcaatgcaacaagccccggctttacagccactgcattgaataacttccagggcacagattccgttgaagttggctcacgtgaaccgatacgcgtggcacttgacaccgatggtccaaccgccagctttaccggtccggatggcccttcgccgtggtaattgcagcacagtaaaattaattaatgaccggtggccgaaatagtcaccggttaaagttattatctttaattatgaaaaatgaacagcccaaactccctaagctggactccatagcggaacttcaccgccagctggggcttcccggtccacggcatcctatcatcagcttattggatgccacaaacggtgaaatcgatatgagccggcttccaggcggttatatctcgggtttctataagatctcctttatcaccgaactgaaaggaaagttccggtacggtcagggctattatgatttcgacgaaggtagtctcttattcactgcaccaaaccaggttgtaggtgctacaaacaattaccagggtaataaaagttattcgctgatcatccatccggatttcctgcaaggctatccattggccacgaagatcaaaaactacggctttttctcttatgctatcaacgaagcgttgcacctttctgagcaggagaagtcgactgtgcatgctatttataacattatcggggaagagctgaacagcaggatcgatgaattcagccatgaggtagttatcgcccagattgagctgctgttgagctatgctaaacgattttataatcgccagttccttacgcggaaagttgttacaaatgatttgctccagcaactggaagaactgctcaatacttattttgagcgggacaagcccgccagtgatggcatacccacagttaaatacctctctgaacaactcaactttacaccgaattatctcagcgatatgctccggtcacttaccggcctgaatgcgcaacaacatattcatcaaaaactcatcgaaaggtccaaggagctgttatctacaacaaatctcaccatcagtgaagtggcctatgagttaggctttgagcatcctcaatcattcagccggttattcaaaatgaaaacgaagctgtcgccgctggagttccggcaaacgtttaattaataagcggccgtatttcaagaaaaaacgcaaggcgcaacgtgcatttctatgcaaacacgggaaggtatccgcccggttaccggtattgtattttaatattattatcattatcttggatgaattgtttcaaaacacttttgtcaagccatgggggagcctgtagaggaagggcaaaaagccaccacgttagtacagccggaagttaccgatctggagctggtatttaaagagtgctatgcagttctcctggcgtatgcctgtaaattcgtgttgcgcgaaaccgctgaagacatcgtacaggatgtttttgtacaaatacaccggaaaagtgcctctctccaattaacctccaatatcaaaagttacctgtttcgtagtattcataacagttgcctggattatattaaacaccaggcagtgcatcagcggtatgtgaatgccgccttacccggtcttacggccgctgaactggactattttaacccggacagtccccggcaaagcctcctggagcaggacaacctggaggccagcgtgtggcgggccatacaggaattgccgcctaaatgccgggaagtggtaacgctccgttacctgcaagggcttaaaaccggcgaaatctctgctgtcatgggtatctcttcccgcacggtagaaacacaattatataaggcgattaagcaactcagaggaatcgtcaggaaagtgaactacttgttttcttttattttattgtagcctgtaatcccggtcatcccctcttttctcctttctgaaaaaaaatttaaaaaaagagtacgtagaaattatctccttgtcgtctaattaaatgacatgtcactacaccataatacaaacgaattggattatacgatcttaataaggtttattgaagggaagacaagccctgaggaaactgaggtaatagtcgcctggctgaaggcttccccgggcaaccaggcgttgtatttccaggtaaaagacatcctcgaccaggaattggcggctaaaattacggcagccgatgccgatcaaagctggcagcgggtattggcgcagttgtcggcagcagatcagccggtgacaactgtaaagaaacttagctggctgaagtatgccgcggcaatcctgctgctgatcctggctggaggcgcaggagtttacctgtttatgcataccggctcccggcccgcagccctggtaacactggtgcataaaaaagcatcggtacaaatggtgctgctgccagacagtacccggatatgggtaaagcccggcggacaggtgaagatgcgggatataaaagagggagacggacgcgaagtatggctggaaggcagcgcttattttgaagtggtgaagaaagcgcaaacaccattcagggtgcatgtgccaggcatgacagtaacggtattgggaacttctttcaccgtaaacgaagataaacaacacacggcggtagtggtaaacacagggctgatcaaagcaaccgcctttaacagggaattactgctgcatcccggggaaagagggatggtggtcgacagccagatacagatggatcatatcaacccgcagttatatgccgcctggaaagatggtgattataaatttgaaaacacaactatagatgaaataaaagaactattgtacgcgaactatggataccaggtagaaatattacaaccaaaaaaattccggggcacccggatcagcggacgtgtgctgataacagatgacataagtttatgtaaggcgctgggagctatgctggaagcagacgtgcggaaagatggccaccgggttattattcaaccaaaataagcatggtgaaagagactgtatcacctccgttatctgaacagatacgttttttataaccatattgaacaggaacaaattgaacagcaacgacgtgtagcacggtaatctcattcccattttaatgaagtagttttttaaaccaatatgtagtctttaaccaaaatttttccgttatgaaatttggatctctacggcattgcctgaagggagcgactggcctgtgccttgtactgagtgcgataacttcgtctctgcgtgcacaggatgccatggccggcatccaggaacaaacccggcaggaacgcagcagatacagcccctccgatccggccaggtcgcaaatgatattgctgaaggatgtgctggaaaaaatttatacaaaatatcagctcaggattgcactaaacgacaagtatgcaaaagatatttatctgtctgacaaagtattaaaaatggatgccgaaaaggtagtgccgtttttgcagaaaatgttgcaggggcatagtcttaagctggatgcaataggcccctcacagtatgtgattacatcggcggagaatcatgttgcggtgcgtaaaccggtggtgaagctgaaagtatccggtaccgtaaaagataaactgggcgccgcattggtaggagtaaccgtgaaaatcctcggcacaccaacggggactaccaccaatgataaaggctactatgaactggatgtggaacccaccgatgtccttgaattttcttacatcggttaccagtcgcagcaaatccccgtcaggaataaagtagatatcaacgtggaaatgctggccaaggaaggcggattgaatgaagtagtggtggtagggtttggtgcacaaaagaaaataagcctggtaggtgcgcagtctaccatcaaaccggaagaactgaagctgccggtgagaagcctgacgaatgcgttgggtggccgcctggcagggattgttgcggtgcaaaggagcggtgagccgggctatgacggctctgatatctggatacgcggtatctccacttttggttccagtccgcgcggtccgctcgtgatcgtagatggtgtgcccgatcgtagtatcaatgatcttgaccccgaagatatcgccagttttacggtgctgaaagatgcttccgctactgccgtatatggcacccgtggcgccaacggcgttatcctggtaaataccaaaaccggtaaaccgggaaaaccgcaaatcaacgtggaactcaaccaagccatcacaaaatttacacagctgcctgagtttgtggacgcccccacctttatgagattgtataacgaaggtttggagatgagaggaaggacaccgctttactcagaagagcggatacaacaacatgtttccggtgaggacccggatctctatcccaatgttgactggttcaaagtactgtttaataaatggggacaaagcagaagagcgaacctgaatgtacgcggaggatccgaatttgctacctattatatttctgccggttattattcagaagtgggtttgctgaaacgcgatcgtgtgcagtcctataattcagatataaaactggatcgatacaattttaccaccaacgtagatgccaatatcaccaaaacaaccaagcttgaattaggcgtaaacggttttatcattaacagtaactatccgggtattggtaccggcgcactttttgacctggctacacaggtgccacctcacctgataccgccgcagtattccaatggggagtggcctaaaattccgggtggcagctatcccagtccataccgtaaccttacgcaatccggttatgctacagaataccgcaacaccatccgttccaatatcaggctccggcaaaacttcgatttcattcttaaagggttatcatttaccagcatgtttgcttttgatgcttatggctggaataatcttaaccggaaaagagaagtacaaacctactatgccaccgggcgcgattcgttaggaaatcttcttacaaaaatagtagaccccgggtccaatgtactgggattcgatgtatcaagaggtggcaaccgccggttttatacggaaaccgcgttaaactacgccaacaaattcggtgaccacgatgtttccggattgctgttatataatcaatccgattatattgacgccgatgccggtacccttatttcctctattccctaccgcatcagggggctgagtggaagaggtacttatggttataagaaccgctatttcgcagaagttaatttcgggtataatggttccgagaactttacgcctaataaacggtacggtttattcccttcttatggcgtgggctgggtagtatccaatgaaagcttttttgccccggtaactaatgtgatcagctatttaaaactccgctatacctatggtttatccgggaacagtaataccggatcacggttcctgtttctcaccaggataaagagtgatggcaatcttggctatactttcggcgtacctggcaacaccaccggctatggcgggttggaagaagaccagatcggttccgaggtgagctgggaaacaggtaaacggcaaaacctgggtattgaaataaaggcgttgcatgacgacctgtcgctgattgtggaattatttaaagagcgcagaacaggcatcctgctgcggcaatatgatatcccttacgcttccggttatactaccgataatatcccttacaggaatataggtattacagagaataaaggaattgatgtaaccctcgattataataaatcgttttccggtaactattgggttggcttccggggaaatttcaacttcaatatcaataaagatgtgtatgacggtttaccaccatggcagtatccctggctgaaccgcacgggccatcctatcgaccagcgttttggttatgtagcccttggcttgttcaccgattcctctgagattacgagatctcccaaacaggccggagatgtgcgtcccggagatatcaaatacaaagacctgaatgaagacggtatcattaacagctatgaccagcaggcaataggttatggctcagtaccgcgtattgtgtatggcgttaacttcagtgtgggcgcaaaaggatttgacctcagcctgttcttccagggtgtggcaatggtagattttatgtacagcggcggtcatgccaccaatcctttttacgaaggacctacaatcggtaacctgtataccgcagtaaaagaccgctggacacccgagaaaaccgatggccggcctttctatccaagaatgtcaacccgccaggatattaccaccaattactacgaaagtacctggtggcagaaacgggcggactatatccgtttaaaaagtgcggaactgggttatacattcagcagcagtaatcttcagcgctatggattgaaaagtgtacgcacgtatgtgaacggaaccaacctgtttaccatttcgccctggaaaatatgggacccggaactgggcgatggcaggggcaccgcttatcccaacatgacttccttcaattttggtatccgcgctaacttcaaataaaacagcaccactatgacgcatcatatcttccaaaaaaatatccttttactggcgctgctgttactgtttacagccggttgtaagaaaggattcctcaatacagtaccggataatatcaccacgctgaaagatgtatttacaaacaggtcgatgacagaacaatggctggcgcgcatctacaacccgatgccggatatgtggaaccagccttacagtattccgtggacaggccagtgcgacgaagtagactatgcatgggtacaacccggtatgaactcaggcgccatcactgcggataacgccaatccatcctattggaacagttactaccagaccatccggcaggccgccatcttcctgcaaaatgcagatcagaacaaggagatcctcgcacaacccggtggtgaacagctactgaagcaatataaagcagaagcccgctttttaagagcctactactattggttgctcatgcggcaatacggaccggtagtgttaatgggagaagaacccaaagccccggaagacgatttccagataccaagaagtccgtgggatgactgcgtaaactatgtattgtcagaaatggataaagcaatgccggatgtgccggtactgcatatgaaccctgttgatcctacacagccggacgttacacaaacaggccgcatcacaaagcccattatcctggcggtgaagtcgcagatattgttatatagtgccagccccttgttcaatggtaatacggagatgggcaactttaaaaaccaggatggcgccgccttgtttaacgcctctttcgacaaagagaagtggaagaaggcagccgatgccgctaaagcagtaatagatcttaacaggtgggaattatataccgtagcagatgcagatccgttccgggcggcgttcctttcctgccggaatttattctttgatggctggcaaaaagaagcgatctggatccgtaccaactctgatcatgtggggaactgggaacggcattgttctcccaggtgcgctaacgggtccggctggaacggtattgccgtcacccaggaaatggtggacattttccgtacggctgatggcaaagctattacagataacagcagcggctatacggaaaccgggtttaccgatgccgctaccccgtattatgtaagtggtacctccaatatgtatcatggaagggaaccccggttttatgtagatgttacttttaacggatcagtgatcccggtggttccggaaaacgggcaatcaagagtggagtttttctttaccggcaattccggtaaaaacggcgcccccagggattggcccactacaggctacaccgcccgtaaaaatattcaccccaacacagatttcagaagcggccgtagtttttcccgcccggcgatgatgatccgtcttggtgaaatttacctgaactatgcagaagccttgaatgaatacgatccgggaaatcctgatatcttaaaataccttaacaagatccgtaaccggggtgggctgcctgacctggtggccggcgccagccaggcagagatgcgtaagcaaattcacctggaacgccaggtagaactgatgtttgaaggccaccgttattgggatgtacgccgctggaaagtggcgaacacgccggatcagcatcagggcgggcaattccatggtatgaacattgaaaaaggatctttcctgtctgatcccgaatttcataaaaggattgtggccttcaccagggcgcaatgggataacaaattttatttttatcccgtaccacaaagcgaaattgaccggaataaaaaactggtacagttccctggatattaatgcagctaagtgatgaacgtgttttaaaagagctggctccgtgagccagctctcttttttgctgtcatcggatgtcgcttttggctccatgattgtcgcatatcccctgcaggtgaaaaagttgggatgccgaaatttgtatcgtaaacaaaaacacacggtatgaagaagaatatgatcacccttttcctggtggctatggcagtggcggtagcaacatcctgtcagcctggcccggagaatcagcaaaaggttccggctaagccggaagacacgcttgttaacaagacggtgaagccggctgaaagcggctacgcagatgtgaacgggctgaaaatgtactacgaagtatatggtgaaggtaaacctattgtactattgcatggatcttatatgaccatacctttgaattggtcgcacatcattcccctgttggccggcaacaggaaagtgatagtggcggaaatgcagggtcatggccgcacaagggatatcccgcgcgaacttagttacgaagccatggctgacgatgtatccaggctgctccggcatctcaaaacagacagcgccgacattttgggatatagtatgggaggtggcatcgcgttccagttcgctatacgccatcctgagcaactacgcaggctcgtggtgttatcgggttcctatacccacgacggatggtggccggatgtagaagccatgtatgctaccatcgacgcaaatatgttcaaaggctcaccgatgcaaaaacaatacgacagtcttggtaacgatccggcccatttcccggaattcgtaaagaaagtcatcagtatagatctgaagccttacgactggtcgaaagaagtaaaaaacataaaggcgccgctattcatggctatcggcgatgccgacggtatacggtatgagcatgcactggcactgtttcgcgccaaaggcggcggaaaaatgggagacatacacgggctgcctcaatcccgtcttgccatcttgccgggtaccacgcacatagggatgatgcagcgcaccgattggctgatacccatgatcactgatttcctggattccgatctgaatacggctcctcctactttttagaaatacgtgactaacgtcgatatacatacgtaatcaccggtgagcaattcggttgattgtctccatccggcgacctgaagggtgaagtgcaactaaatattttatatctttaccggatatccaaacaaagcgcattttgccggtgatgttgtattgtgatattgtattgtcgtgtagtcagtgtttttattgccaagatgaaccttatcttttgtctcaacctgtttttatccaacttcatgccgaccgggcccgttgtttcaatggacaccaccgtgcattactttgtcaggcgctttactgatgaagatggcttgccgcaaaacagcgtgaaatttattgtgccggacaagaacggctttttatggctggccacagaaaacgggttaaccaggtttgatggcaattactttctcaatttcagcagcgataaccttcctggtttgaaaagcagcaggatgtccaggatctatcccaatgataccgctatagccgtagaaacagatatcggggaaatactgaccgttacagaaagtacggtaaagcatataggaaaggagctgttgggatacaggtatcagcattatgttgaaaacaaaaatgaatactatcctatcaagggattgcccgatgatcaggcagtgcgttttggaaaagagcgccctgttgtgataccacacggtacagacagttattttgcagcctatcacgatacgatctcttttatagagcaaggaagactcgggtaccggttaacgcagacccggttggaggtgtcgcgtttgtttgtttgcgatggcaggcttttataccttaacagggatgggcacataacaggatgggagaaaggacagccggtacaagtgccgcttatcggggatgtagtagctgatcctgcatttagtaaatgtaaaatggaattatactggaacctggctgcgcaccaggtttttctttataccgataaaaattgttatcaattacaggtagaaccgggagtaggcatacgtagtgcggttgtgctgcgggattttgattttcaccggaactatatttcttccatctactatgatcagcgggaaagacgggttttcctcggaagctctacaaagggcctctatgtttgtaccaggcagcaattcaatgtacataaatcggatgcttcaggggatgaagtattttatgcacaggtggcgtcccccggaaatatggtggtgacgccatcggggcttgcctttaaccagtcaggaggatacagttggctgcctttgtctttcaacagggaaagcgtgatggaaaaatatacgttggcccgtgatcagcagggaaggtattggggaagaaatgggatgacattggtgggcgtatcaccggatttcagccaggtgctgcacaaaattgaattgccctacctcatcagccaggtgttcgcggacccggaggggaatttatgggcagggggaaaatttccggggctatactatattaaaacggcagatccggccgcggcattgcagtttcttccagccaaagtaaatgaagttagctttataaaaaatggtaagccggggatattatgggtaggtacagataagggactctacagggtacatctgccatccggacgcaccgataccatcaaaggcctggaagacggacgtataagaagtgtctatattcctaaagaaggagaagtctggatctccacctataaccggggcgttttcctttacaggaatgagcgcctggtagccctgccgcaggatcgccagcggtatatggccaccacacattgtattaccgaagatgaacagggttatttctggctaactacaaacaaagggttattcaggatccggcggcaggatgcgctcgatttcgctgacggaaggcagcgcgacctttactattattatttcgggaaggaacagggttttaatacgaacgagtttaacggcggctgtgagccatgtgccttaaaatatgacgacggcgatatttctttgccctcgctggatggcctggtacagttcacgccgtcttccatcaggatggaaatgccggataaaggcatatatgtcgattgggtggaacataacctgaaaccaacaaaagcatcagaacaatttaacctgcccagtaattttcaaagcttccggctacacatcagctctccctattttggtgattccaggaacctgcagttttattattcgctggagaaagatgactggccggaagaacagatatggttgccggtgaacagcgacagaaccatcactttttcctctttgccatccggggattatcgtatccgtatccgcaaactgaaagggtttggaagagatcagtatatcgaaaaggtgctcgtcatcaacgtacagaaagctttttatgaaagattgtggttcgggctggcggtattaaccattctgatctgcctgataattttgttgtataagatacgcatcaggagtattgcccggaaaaaccggttgttggaactaaaggtaatgagccgcacccgggagttggaagaaatgatgaccatactccaggagtccgatgaacagctgcgtaaacagggttttatgcataaacgtttgcttgctgctatcacccatgatattaaaacaccgctgaagtttttgttgagggttaataaagaggaaccattatccggtgtgttgcaggagaaggaaataaaaacggttacctacgacagtctttaccgcatgcatcacctggtggataacctcatccattatatgcggatctccttcctgacgggcgcattctctgaagacactgttgacgtccaccaactggtggaagaaaagatggagattttcaatccggtatccgcctcaaaaggaatacagctcattaatcatatttcgccgggcgtaacggtggtcgtgaataaattgttgctggccgttattctacataacctgttggataatgccataaaatataccaccaggggcgttgtagagttaagtgcagaaagaggggagggtgttttaatcatacatttatccgataccggctatggtatgccggcggaagtaagggactggatcaatcacatagaaaataccggtccggttcagattgggggcagcggcataggactgatcctcgtaaaggaattgctgacggtgataaacgggaggctgtttgcctatccgggtgttaacggaggcaccagggtttccctgcaacttccgcttaatgactagttacctggtacatctgcgctttttcaatcagggcgattacatttttcacccctactttttcaaaaatacgcgttttgtaggtgctgacggtggtcagctgtaaatggagcgtttccgcaatttttatgagagggagcccttttgttagaaggttcattacttcaatttcccggggggaaagcaccgaaaaagggttagaggaatgctcctgctgccccgtaaatttacctatcagctgttccctgactgccctgctgatatacttttcaccgctaagaatcgcattgatggccaccctgaattcttcatccggggagtttttttcaatatagccatctgcgccggcctggagatagttaagggcatacagtatttcatcgtaggcagaaaaaaccagtattttaataccaggttgccggagtttcacggcgtaaatcatttgccggttgtttccgccaggcatattaatgtccaggatcaggaggtcgatattttgggcttcaataaggaatatggcttcatcaaatgttttagcctctgtaacaagcatggcgcccggtagcgagcaaataatctgtttcatgccaagtcttactatagagtgatcatctgctattagtacatttttcattgctggtttaggttagggctcataggaggtattattgtttgccggctcaaaattaacatttttttcttcgtatatatatgacagtgccgtaattttttatactatataacgttaagataactactacaacaaaagggggatgactgcactatatttgaaaatcagcctgcgtaaggacttgataagaaaagactggtaatttaaagtgtcggtatgacactaaaatgtgacggcaggggcctcatcctttccatcagaaaggattgaaagaacatgggcaaaaaccggaacaggttctacagcccggatactacaaaggattttcataggatagggaatcaataaaagatgagtgcaaagcactccaacggacagtagattgcccgggagcgccatggtacagcgttcccgggattttttttcaggtaaaagtgaagcgcgtgtagtgtaaatactacaggggtattgaactatagtgacagcagcgtatatattgtttatctacttttgctttgaagatttgttccgttgagtcatgtgaacacttctcagtttttcaggacgtactaacgatacccgtatccttttttttgtgatcttaacattacatttcctatggagagctttacccaatttccgcaacatgcggtccttacattttgtgctggcacaaatcccgttgattattaaacctgtgatgctacatgtgtctgaccagttccgcctgaaaatggctgtctgccggtcttaacaagcaaccatatctgaatacgagcatgcaaaggttccccacggaatctttcccggtctgctatgtttaacatagtggtcagggtccctcattacccaaagtttattgcattatgtccctcttcaatgttccgaatcccgattcaagatttttcagcaaaggctgtaagcgtttgttgctggctctgtttggcatgatggtgaccgttgccgcaacggccaacaccttccccgtcactaataccaatgacgcggggcctggttcgttcagacaagccatcctggatgcaaacgcagcgggcgcagggccgcacgatatcgtgttcaatgtgcacgggcagattacgctgacctcttccatgcctaccattacggcaaagaagctgaccatcgacgggcagaataagatcacgctgtattccaccggtaccaattccgtgattaatccctttgtgattaatgcggacagtgtgaccatccggaactttacgatacagaacaatggggacattaatgtggacatttttccgaacaggacgggtgttacgatcgacaatatacggtcgttcagcacggtgggtaacttcctgaatgcatttatgagggtgcagggggcgtctaccggtctgacggtgaagaatatttattccacggatgtagagcctgccggttcctcgtcactaccgccacatgttgggcgggctttttattttacaaacggcatgcagaccaacctggtgatggacaatatccaactcagcacggcagggaacgtgcgcggtggcgaaggtcttgtgttcagggatgcatcggtaaacggccttacgatcaccaatagtaatgtcagcggctttcagaatgcgattatattcgataatactgccggcgctgtggaaactgcgaataatgtgatgttcagaaatgtggccatagatagtttgtggagtggggtgtcgctgggaatttattgcgattttgttacgactaactttgaaatcaaccggaccacaatagatatgaatgtgatagggcaggatgatgatggggactatgcggttcgtttcgacaatactaccaacaacgtcacactggacaccctcaatataaatgaaaatgatatccacaatgtctggttcaatggtgctgccaccaatattacgatcaataaggcactgatggagaatcgtgtccccgggctatacgggacgaatagttttatcaggtttgaaagcacggtaaacggttttaatttaactaactccgtattgaagggagataaactcgccaatacggatgatgcagatgtcggcgttttatttgtaggagctgctacgggagtagcgatcagcaacgttacttttgatggcttccaggcggatggtataactgtaagcgcggcggccaccaatttccaggtgaccaattcaaagttcaccaataacgtggatggtattgagtttgccgcgaatgctgcaagaagtaatgtagatatcgttaactcatctttctataaccagggccgttcaggcattgtggtaaacggcgccaacgcattaacagatgtggacctggcaggtgatacggtggtaaacagcgccaaccatggtatctggttttacggcggcgcaggcgtaacggatgcacaggtaaccggttgcgtgatccatgataatggtggcgcgggtattaataatgacgcccccaataaggtaatcatctctaataactccatttataataataccggtttcggcatcgcattgcctgccggtaactgtacgtatacggctgccaccggcaaaacgccggtattggtatcctccaccgcacaggggagcgggcagtatcagctgcagctcaacatacctaatataacggccggcgcacaatacacggtagatatttatgccaatgatcccgctacgagcaaaacgagcgggcaatattatgttaccactttaacgggaatagccgcaggtacatctactcaaacaattacttacaatacaggacccggcgccaccggcctcggtttctggaccgccacgctgcgtatacccgccaacaattgcggtacatcggagtttggcaacagtatccctatgaccttccagggacccgcttgtgtaaacagcgggattcttgcatggtaccgggccgaccaggccgtgaatggtaccggctggggcgatatctccggaaatgccaatcacatgctggtaacaggtgacccggacaataccacaggcatggtgaactttaatcctgccatttattatgatggtaatgatgcgcaccgcgtacccgcttcggcaggcgtaaccggcgcatacaccatgatggggatgggcctcgtggaaggctcacaaaccggccgtgtatttaccagcaccaccggtaataaattattcggctggcacgctacaatggaaaaccggttgttcgtggaagcctggttgagtaccggtaacgcagtcaccgcaaaaggcaagctctattcctttgaaagaggggccaccggcgcctatgaatttaaaggcaacggcgccctggtgaaaaacggcactacttccgatgccagtgtatggacgctggatgtgggcggctctgcttatggggaattctcaaaagtactgattccggaagtgttcatctacaaccgtgatcttactgctgcggaagtgcagcgcatagaatcatacatggcgttgaaatacggcatcacgctcaacgcaggtgcaacagattatattaccagcgatggcacggtacaaatgtggactgctgcttccaacaccggttacggtacgcgcatcacgggcattggccgcgatgattgcagcatgctgaatcagaaacaatcgctgaaccaggatacaggtattgtaaccattgctttgggaaatgcattgaccctttccaatgctgctaataccaacactttcacacaggacaaatcattcctggtgtttggtgataacaacggcactaccaactactttactgcggtaaccagcacaaacgcaacacagcgtatgggccgcgtttggaaagtgcagaaaactgccagctggggtaatagtcagcaggtaaccctgaaactggacggcggtacagaaaataattacctcctcatcagcacagacgctgctttcggtacggttagcaaagagctgaaactgagcagcacaggaaccgtcaccctttccagcgcagacctggccaacggggctttctttacctttggtcagcagcaacggtctcccggtggagtagccactaacctgcaaacatgggtgaaagcagatgccggtgcaacggtggttgatggtaatattattaaatgggccgatcaggcggtgcagagagaatggcctttggcgcttgccaatgcacccgttagctggcagaagaataccattaactataaccccggtatcaatttcctggcgaataactatttcagcgtaccgaaattcactgaaagttatacagcaggagaaatattttctgtacaactgtctaacctgccagctacttctacagccgccaccttcccgtttgaatttggtggcgaccccaccgcggcggccggccagccaatttacgtgtataacggaagtcactatacgcactttggtactaacacccgtcccggctacgcgttaacaggcatcaatatacagaagccccatttattaaataactggagtgctcccggcagctggtcgctgaattttgatggcaaaacaataggcagcagcactaccttcccggttaacttctcaaggggaactgcgttgaatactgctatcggtgcagggcatttctccaatttcaatggccgcatttctgaagtgatcttttacaacaggcagctgagcgctaccgagcgcgcgcaggtaaacagttacctggccctgaaatatggactcactttgaaaactgctgccggcgccataaccgattaccttggcagtaatggtactacccgcatgtggaccgcctctaaaaatactggttacggcgaacgtatcaccggtatcggcagggacgataacggtactttgttgcagaagcaaagcttgtcgcagctcgacggcgccaatgtaaccatcgccgcaggcagtgatctgaccgcctctaatgccgataatgttactaatatcgccaacgatctttccttctttactttcagcgataacggtcaggcagctacgtatacccaggcggtgaacggccttggcaatattacggtgcgcatggcgcggatctataaaacagatcgcaccaactgggcgaagagtcctatcacgctgtcgctcacaggcggtaacaataacaactacctgttggtgagtaacgatgaaactttcggagcgggagataaggcatatgtgctggatgcaaatggtgaggtaaccatcgatagtgatttgttacctgacggcgcttatttcacttttgcgaatgcgcaggttgctccggcaggtatagccgccggcctggaagtatgggcaagagcagatagcggaatcgtgggtggcaataatgttacacaatggaaagaactaggcccgtccggccgtgtatggcctaaagtaaatggaaatgcggcgacatggagtcctgcatctttcaactttaatcctggcgtagggcttgccggcgctacctatttctccgtgccgcaatttgcaaatacctttactgcaggtgaaatattctcggtgcagacatctaatctcgataataatgtagccacaacacattatccttttgagtttggtggaacatatgccagcacgcaggctgtatatacatggagtaacagtaatcactatacttattttggtactgctactgcacgtaggaattttgcttaccctgcatcagtgaatgtgcgcaatgcgcatatgctgaatatatggagcgccactaatgactgggccgccggtatggacggcaaagtgctggtcacagccaatgtcaacgccgtgagttttgcttcagtgcctgtcgctgattacatcggagccggtcataattccgtttttaacgggaatattcctgaagtgatcatgtattcccgcaaactaagcgctgtagaacgccagcaggtgcaatcttatatggcactgcgctacggtcttaccttgggaatagatgcaccgatggattacctcgccagcgacggcgccactaaaatgtggcaggcttccgttggcagcggcttcactaaacatattacgggtataggtcgcgacgacaggggcatgctctatcagaaacaatctgtgagtgcagacactggtatcgttaccattgcagtcggcgccaccattgcagcttctaataaagacaatgcaacggctatcaccaacgatctttccttcttcacctttggcgataacgccgctgctaccacttacctgacaccggttaccggtatcagcggtgttaacaaccgcatggcccgcatcttcaaagcacagaaaaataactgggccgatcagaatatcactttcgaattggctggcggcaatgcacgcacctacctgctcgtgagtgctgataatacttttggcgcaggagatgctgcctatgtattaaatgccgacggcgccgttaccgttaacagcaacctgttgcctgacggtagctacttcaccttcgccaggatgatcaccgggccgaatggtgtaacagatggtattgatctctggctgcgtgcagatgacggcatgtctggtggcaacaagtggagtgactatagtaactatggcaatgatgctttgcagggtgtagtgggcagtcagcctattacagatgccaaagccctcaacttcaactacggcctcacgttcgatggtacagacgactttttggatgttactactacgcggataaatccggccacagccaccgtttttgcagttgccagcggttcggcgggagatcttttcagtagtggagcagtaggcgcaactcatggaatggaattcaggctggtggcaggaaacaagctacagtacctggagaacgccgcagcagttgtagcagtaactggtgttaacaccatccagcttaataagcctcatattttcagcgccacccagataaacaatactgcgaacggtgtacgtgtgtttgaaaactacacgctggataaccagggtaccatcaacttaacgccactcactgctaatcttatttcaataggttcccgtagcatggctgccagagccctttactggaatggcaatataggagaagtgatcacctataaccgcgtgttatcagatgtggagcgccagtcggtagaatcttacctgggtataaaatatggtattacaataggcaacggcgccactgattacctggctaccgatggttcaaaatactggaccgccgatcctgtttataaatcacgcattaccggtataggaagagatgatgccacttcactgaataccaaacagtcactcagcgtagacaccggttttgtaacgctctccctgggtaataatattgctattaccaacgaacagaatactaacaccatcaccaacgataaatctttctttgtatttggagataacggacaatctgccagctcttatggcactgttgtaaacggaacaacggctacccgccgtatggcccgcatatggaaggtggataaaaccaactggacagatcagcctatcaccctgaaagcggatgcaaacggaacgaacgtgttcctcctgatcagcactgatcctacttttgctaccatcaaccaggaactgccgctgaatgcaagtaaaaccattacgctcaactccagcctgatgaccgatggtatctactttaccttcggcgctgcggttaaatatccgggtggtgtaaacagcggtaaccttatttggctgcgcgcggatctgggcacttctgctaacgcagacagtacgcagatcagcagctggaacgactatagccctaacgggaacgacctgtcacaggcaacgcctgccaatcagccattgtatttcaacagtgctgctaacaacatgaactttaacccggtggtaaggtttaatggcgctcctcattccatgacaggtaaatcgttcctgaagactggcacctatactgctgctaacgccttttttgcagttaatcagacaactgctcttaatgccattgttttcactgagcctgccggcaccggtacgcagtttacgctgcatgccacctggggcgataatgttgtttattgggatgctccttatgttaataaccgtcttagctacaacgccggaaatgttaacaaccaagtagttctctggactgctaccgatgatatcagtcttgctaccggcaagcaggccatttataagaatggtttaaatgtggccaccggtaacaatgccagtacttttaccggtaacaacagccccttccagctgggttggaatgccgctaactcctacaatggccgtatgggcgacctgatcgtttataccaatgcgctcacaccggtagagcagcagcgcgtgaatacctacatggccatcaagtacggtatttcattgaataatggcaactccaattacctggctaccaatggcagcaccatatgggatgccactgcaaacagcgcttataaaaattatatcaccggtatcggccgcgacgatgcggaggatcttaaccagaagcaatcccggaataccgcagacggcatacaactggccatcggcttaaacagcctggctgaaacgaatacgggaaatgccaatgcatttgcggcggacaaatcctatatggtatggggtgacaacgccggcagcagcctctttaaaactccgcttacaggccaccctgtggctaactaccgcatggcgagggtatggagagtgcaggaaaccggtactgttggaagcgtacaggtggcagtgccatacgatgcgttgcccaatgccgcacaaacttatctcatcatcagtaatgatgctaccttcgacggaacggaccaatttatccctgttaccgcaactaccctcaacggcgtgaaacagtatgccgccaatgtggacctgaccaatggacagtacttcacttacggtgcatctatcaaagcgccgggtggcgtggtaggaaccagcttatggctgcgcgctgatgcaggtacttccagcactacagacaatacggctatcagcggctggacagattacgcatcagaactgaacaacgcaacacaagtaactacaccggccagtcagccgttgtatttgaacaacgcaacaagcaatgccaactttaacccggtagtgaaatttgatggtacagactatatgggtctggacatcaccaaactgccgattggcacaagcgccagaacattcttcggtactggtagcttagctaccaccgctggtggcaataaatttattctcgcatatggcgccggcgcaaccaatgtaggttccggtctggcagtcgtaggtggaaacggaacagcagattttgtaggatgggcaaacgacgtggtaagccctgcaggtaactggcaggcaggcgcatttaatgaaatggtgggtgtatgggctggtaacggcggcaacgcctccctttacagcaaaatgaaattgctgggcggaccggtagctaaggcttggaatacaggcaacgttgacgccggaataggttcctggccgtgggacaaagcccaggcatggaatggtaccgtaggagatgtgatcgtatatccggttgcgttaaccgctactgaacgtcaacgcgtatccacttacctggctatcaagtacggctatacgatagatcagactgctgctactgattacctggctaccgacggcaccactaaagtatgggatgccaccggcaacgccacctataaaaataatattaccggtatcggccgggatgatgcagaagggcttgtacagaaacaatcccggaacattaacgcaggcttccagcccatagtgggcctgggcggcattgctaccgacaatctttctaatagcaatactttcacaacagataaatcatacctggtttggggcgacgatggcgccagcacttcatttaccactgccatcaccggcaaccctgctgtgagcacccgcatggcgaggatatggaaagtgcaggaaaccggtaccgttggttcggtggcgctttcgattccgaaagatcaactgccgttaagcgccaacaggccttacctggtaataagcagtgatgctacttttgacggggcagaccagtttatacagctgtctgacgccgatctgaacggcgttccaagctattcaacctcacttgatctcaccaatggccaatacttcactttcgccagcttcgtcacttcaccaggcggcgtgccgggtgaaatgctgtgggtgaaagcagataaggatgtacaggcgaacggaagcaaccaggtggaacaatggctcaaccagagcggtcctatggtaaccgaattgcgtgctgcactgcctgcccatactgaccctattactgcatcggcagatatcgttcaagttccaaacggcatcaacttcaatccggcgatcgacttcagtggtgcagtaggtaaatcccttaaaggaaatgccggcattaactggaatacatcggccaacctgtctatcttctctgtaaataaacctgaagccgctatcacggctggcttggctggtattttctctaccaacggaagctgggttacaacaggatttacaggaaggggacttcttctgcaactcgcaggtacttatggacttgacggcgcaggatgcattgtcgcacaatccactcctgcttatgccggaccaatcatcgccaggggtgtttatgtaagcgctgccaatgcgctgaacggaactacctggctgaacggcaaacaggggatccttggcaccaactgtgcaccgggagcagatggtccgttctttgaactgggcggccgtacaggagatgacgcttcatttgacaacaggatcttcaacggtaagatccctgaagtgatcgtatataaatccgcgctcacgccaacacaggcacagcaggtagaatcctacctcggtgtcaaatacggtgttacactcgaccagtctgccgcacagaattacctggccaccgatggctccgtgatctggaacgccactgcaaacagtacttataaaaacaacatctttggtattgggcgcgacgacgcagaagcgcttgtacagaaacaatcccgcagcgtgcacaccggctctatcctcactgccggtatccgctccatcgccgctaccaatgcagacaataccaacactttcgcagcagataaaagctatctcctgctcggcagcaacagtcaggccctcacggtgagcggcaccgacctgccggtaggcagctgtatcgctgaacgcctcacccaggaatggaaaacgcagtttactaattatgatatcaacacccagccactcagcctgcagttcaatctgaacggcatcacggtggcgggtacagcagcagaggatttcaccatcatgatcgaccaggacggcgacggtaacttcgctaccggtacagtgactgaaatccctgccaccagcttcaacggcggtattgtgagcttcgaaaatgtaaacgctcttacaaatggcgtagtgttcacactcattaccagtcatcctgaacgcaccgccaacctggtgccggatgctacggtaagaacagtagcagctacctgtattgataacggtacactttatttcattgatccttccgatcctaacaaatacattgcttccattgccctgaacggcaacaccatggacgttaccaaactgtctgctgtggtggatgtgaacagggatatgaacgcagcactgggcaaaaacagcggtaccgattatggtacacagttaatgcgcagactggtacatattaattacaccggtgccaacctgacacagaacggcggtattacactccgtctcttctggaatcctgcggaaagaaccaatgcagaaaatatgctctctggtacccgcggtgtaacaggcacgcaacggtggacatggttcaaacacaccggtgattttaccgccactctcgccgacctggctcctcagggattggctaatattacagagatcaccccgtccggtacaggtcagcaggatggcgtggaatacgttgaattcagcggtattcagaacttctccacctttggcgctttaacggctgtcaaagaagtgctgaccatcaccaaaggccaggacggtacagaaggtacacaaaacggttcctttaatatcatcctgcctacatccgtaacagctacggaagatatcaccgtgaattataccgtaacaggtaccgctgttaacggcaccgactacacgtcgctgaccggcaccgttaccttccctgcgggaagtaacagcgtagccttgccggtaacagttaccgacgataacatacttgaaataacagaaggggtgaccgttacgctgaacaacgccattggtgctaccagcggcagcgcttataatatcgccagcacacaggcagcagcttctctgaacattgccgataacgacagtaatgatcctgctaaaaccgttgtaggtgtaacctgggatagtgatgcgaaagagccgtctaccaacggcgcctttaatgtgaacctgccggctggtgttaccgcatcagaagatattaccgtaaactatagcacgggtggtactgccacaccgggcgcagattatggtgtgctgagcggatcagtcatcatccctgccggccagaatggagcagcagtgccggtgatcgtaaccgacgaccagctcgtggaaaccgcagaaacagtattgttaacggtgaccggcggtacctccaccaactttacacttacgccaaatacagctgccagcaatgctaccgtgaatgtaatagacgatgagaacacaccggccaacctggtactgagtataaccaaaactgccgacgcgtcagaacctgccggtaatggcagcttcaccatcagtttgccaacaggtatcctgcctacgcaggacatcaccgtcagctataacataggtggtacagccacaggtgggtctgattataccgcgcttacaggtacggttaccatccctgccggtcagtccagtgtaaccctgcccgttagtgtaacggacgaccaggtaattgaaaacacagaaaacgtgcttgtaacgctcacgggcggtaccagcaccggctttacttataccgtaagcactaccaatggcagcgcttccgttgatatcactgataatgataacaccactgttaaccgtgtactgagcatcactaagaaaacggatgcagcagaaccggctaccaacggtgaattcaccatcagtttgccggctaatgtcaccgcatctgaagatatcaccatagcctatatacctaccggtactgccgccagtggcacagattacaccgccctgggaacaactgttctgctgcctgcaggacaaaatagtgtctccttaccgctcaccgttgctgatgaccagattattgaaaacactgaaactgttattgcaacggtgaccggcggtaccagcaccagctttacatttacagccagcagcaccagcggcagcgctacggcaaacatcacagatgatgacaataccaccgctaaccgcgttttaagtgtcagcaatgcaggtggtgatgcttccgagccagctaccaacggcgcatttaaaatcagcctgccggccaatattctttcttcagaacctattacggtaacttatacaacaagtggtacagctaccagcggtactgattatacagcgcttaccaatacggtggtaatacccgccggacagaacagcgtgacagtaccggttgttgttacaaacgatccattactggaaagcacagaaacggttatactcaccctgaccagtggagcatctaccagctttgcattcacggccagcactaccgatggtaatgctaccgtaaatattctggatgatgataacacaccgggcaaccgcatactgcgcatcactaaaaccaccgatggagcagaacctgctaccaacgcagtgttcaacatcaacctgcctgcgggcgttcttccttcagaagacattactgtaagttatagcataggaggtaccgccaccagtggtgcggactacccggcattaagcggtacagtaaccattccggcaggacagaacggtgttgcgcttccggtaaatgtgatcaacgaccaggaaattgaaagtacagaaacagtaatagcaacgctcacgggtggaacctctgccaactttacttacaccgttagcgccacaaatggtaatgcttctgcaaatattaccgatgatgataacacggctatcaaccgtgtgctgagcatcagcaatagtggtaacgcagcagaacccggtactgccggtagcttcacggtaagcctgcctgcgggaatcacttcatctcaaccaattacagtagcttattcccgggcaggaacggccgtttctgccaccgattataacgctattggtacggtaacaataccagctggccagaatagtgtagccgtaccggttacggttatcaatgataatatcattgaaccaactgaaacagtaatcatgactgtcaacagtggaacaggtggcagcttcagctttacggcatcagcaacagctaaaactgctaccgtaaatattgcggatgatgacgataccccggctaatctcgtggtaagggtacaggcagttcgtgatggagccgagggagggaacagtataagattcaatttcggcctggctccaggtgttagctgttctgaagcagtaaccataaaatatacgatagggggtaccgcaatattaggtaccgactataatgggctgtctgcgggacatttcaccggaacagctgttatttcccccggaggtggcactgccacagcgggtaccatcgtggacgatcagatcatagagggcacggaaacagtggtgcttaccatcaccagcgcctcttccgccagctttacctttacgcccgatccggttgaaggtagcgctacggcaaatatcattgataacgacgatacgccggctaaccgtgagctcagcatcaccaaaaccggcgatgcagccgaaccggcaacaaacaacactttcaaaattagtctgccaacaggcgtaacaatcgcccagcctgttaccgtgaattacacagtgagtggaaccgcaactgcaggtactgattacgctaaccttaacggtacggctaccattcctgccggtgcaaatagtgttacgctgccggtgaatgtgatcgatgacaacctcattgaaaacaacgaaaccgtagtggtaaccatcaccggtggaaccgcgggcagtcttactttcactgccagtccaacggctggtgcggaaaccatgagcattgcagataacgataacaccaccaccaaccgggtactcagtatcgtgaaactggcagacctcgaagaacctgctgttaacggcggcttcaaggttagcctgccttccactatactttcatctgaacctgtaacagttaactataccgttaccggcaccggcaccaacggtacagactatgccacattaagtggcagcgttatcctgccggcaggtcagaacagcgtggtgattcctgcaaacgtaacagacgaccagattatagaaggtacagaaacgctgattgctaccattacaaacggcgccagcaccagctttgccttcacagccagcactaccaacggcagtgcaaccgctaacatcctggacgacgataacatcgcggcaaaccaggtattgagcgtggtgaacggcggcgatgcgtcagaaccaggcaccaatggctccttcaccatcagcctgcctgctacttatacttcagcattgccaattacggtaaactatacagtagcgggtaccgccggaagcggtgtggattacaccgcgctgacaggcacggtaaccctgcctgccggacaaaacagcgtgtctgtaccggtaagtgtgatcaacgaccagctcgtggaaaacacggaaacggtaatactgaccctcaccggcggcgccagcactggctttacgtataccgttagcacaacaaacagtgatgctactgtaaatattacagatgatgaaaacgcaccggctaaccgtgtgctgagtgttaccaacaccggcaacgcgtccgaaccaggcactaatggagagttcactattagcctgcctgccggcatattgccgtcagaagacatcgacgtcacctacactattggcggtacagccacaggtggcaccgattatgccgcgcttacaggcactgctaccatcctcgctggccagaatagtgtaaccgttcccgtagttgttactaatgaccagatcatagaaggtacagaaacagtgatccttactgttagcggcggtagcagcagcggctttacatataccgccagtactaccaatggtaatgctaccgtgaacgtggcagacgatgataacaccgctgccaaccaggtgctcgctgttaccaaaacggcggatgcggcagaaccatctaccaatggcagcttcaaagtagccctgcccacaggtatcaccgcggcccgcgacatccaggtaacttataccatcggcgccggtaccgctactcctggtacagattaccaggctattaccggtaccattaccatacctgcgggtcagaatagtgtatccgttcccgtgaatgtaatagacaataccgtgattgagccggatgaaaccgtgatcctgaatatcaccggaggtaccgatacacagtttacttataccattgcaagtggcggcggcacagctactgtaacgatcaccgataacgatcatgcagccaacagcaacattgtgctgctcaccaaagtatccgacgccctggaaggcggtacgaatggtcagtacaggatttccctgccaccgggcgttaccagctctgaagatgtggtagtgacctttgctacccctatgggaggaacagccggtaatacaattgactataatttgctgggactgtccgccggtaatattgtgataccggcaggcgccaacgaagtgttcatagatgtagacgccggtaacgacggtgtcattgagggacctgaaacagtggtgctgacccttaccagcgcagcctccagcagttatccgtttacgatagaccctgcaggtaacggcgcggtagtaaatattatagatgccaatgcggccagcagcacaccggtgcaggtaattaccggcaccaatgccgcagaaccagccaccaacggtagcttcaccgtgaagctggcaggtgtggccacttctgcatggcctgttacagtaggatatacggtatcaggtacagcggtatccggtgtggactaccaggcactgggcacagttgtgatccccgccaataccaatagcgtaacggttaacctcaatgtattggacgaccagatcattgagcctgtcgaaacaatgacgttcacgctcttgtcgggtagcgctacagacggtggtggtaacgcctttatcttcccgcctgatccggccaacgatgacattactgtgaacatcgcagatgacgatgccattgctgccaaccaggtactgaaggtggtaaaaaccactgatgccgcagaaccgggtaccaatggcgcctatacggtaagcctgcctgccggttatacttccgcagccaatatcacgctgaactataacatcgccggtaccgcaacccgtaataccgactatacagttagtaccattaccctgccggcttataccaacagcatcactataccgctgagagtaatagatgacaagatcattgaaaatacagaaacagctatactgaaccttacaggtggtacagatggcaactcattcacatactctgcagatgcaaccagcaacaatgcaacggtgaatattgcagatgatgataataccaacacgaataaagtactgctggtaaccaacagcgctgatggtgcagagccggcaacagacggagaattcactatcagtctgcctgcaagctatacttcatcagaagacatcaccgtaagctataccatagccggtacggccactgcgggcagcgattatgcagccctgtccggcaccgtgcagatacctgctggtcagaacagcgtgaagatacctgtagatgtaaccgatgaccagatcatagaaggtacagaaactgtagcccttacgcttacgggtggtgtgagcaccagctttaactttacgcctgcaagcggcaacagtacagctaccgtgaacatcgctgataacgacaacaccacggctaaccaggtgatcagcattacgaaaacaacagatgctgcggaaccggctaccaatggcgcattcacgatcagcctgcctggcagtgtaacctccgcgcaaccggttactgtaaactatacgattgcaggtaccgctgtgaacggaacagattacactacactctccggctccattgtattacctgccggtcagaatagtgtgcctttaccgctgactgttaaagatgataagattatagaaggaactgaaaccgtaatagctacggttacaggtggcgcttcaccggcctttgtgttcactgccagcactaccagtggtaatgctactgcaaatatcacagacgatgatggtgtggccgccaacctggtactgagtgtagctaaaacaacagatgcggctgaaccgggtactaacggctcgttccgtatcagcctgcccgcaacttataccgcatcagcgcctgttgttgtaaattataacatcacaggtactgccactgccggtggtgactataccgccctgagtggtacagcaaccataccagccggacaaaacggtgtatccgtgcccgtgaatgtaacagacgaccaggttattgagaatacagaaacggtgatcatgacccttagcggtggtacctccggcagcttcacttatactgccagcactaccaatggtgatgctaccctgaacattgctgacgacgacaacacaccggacaacctggtgctgagcgtgatcagaacttcagatgccgcagaaccttctgcgaatggtgaattcagaattagcctgccaacaggtgttaccgttgccgaaaatgtgacagtgaactataccctcactggtacggcagcgaatggcacggattatacgaaccttggcggcacagtagtgatcccggctaaccagaacagtgtggtggtaccgctggtggtaaccgatgaccagatcattgaaagcactgaaactgcgatcatgacactgaataacggcgccagcacaaacttcaacttcacggccagcactaccagcggtaatgcttccatgaatattgacgacaacgacaatacgccgaccggtcttgtactgaacatcgttaaaaacacagacggagcagaaccatccactaatgcggcattcacaattagtctgcctgccggatataccgcttctgaggacattacggttaactataccgtagccggtactgctaccagcggcgatgactatgtgtctctcggcacttctattgtactgcctgcgggtcagaacagtatcagcctgccggtaaccgtaacagatgataagatcatagagaacacagaaacggtggtggtaacattaacaggtggtaacagcaccaacttcaacctggtggcaagtggcagcaacggcagcgctagcgcagacattacagacgacgaggccagcaccccggctaacctggtactcggtatcagcaaaactacggatgcagctgaaccggccaccaacggcgacttcagcataaacctgcctacaggtatcaccgcagcggaagacattaccgtgaattacaccgtcgcaggtacagctaccaccggcgctgattacactaccttaagcggtacagtagtgatcccggcaggtcagaatggtgtgtctttaccggtaactgtagcagacgataagatcattgagaacacagaaactgtgataacaaccctcgcaggtggggcatctgccagctttaccttcaccggtaccggtagcgctactgtgaatattgcagatgacgataacgcaccggctaacctggtactggcggttgccaaaacaggagacgcagctgaaccaggtaccagcggtaccttcagtatcagtttgccagcaggttataccgcggcggaagatatcactgttacttatacaacagcaggtaccgcaatcagcggcacagactataccgcactttctggtacagcagtgattcctgcgggacaaaacagtgtggccgtttcagtgcctgtaatagacgatcagctgattgaaaacacggaaaccgtgatcatgacgcttaccggcggtacttccaccagtttcacactcacagccagcaccaccaatggtaacgccactgtgaatattacagacaacgacaacacggcgggcaatcgcgtactgagtgtggtaaaaacaaccgacgccgcagaaccagctaccaatggcgtgtttaccatcagcctgccgctcggtgtggcagcagatgaagacattaccgtgaactataccaccagtggtactgcaaccagcgcaacagattatacagcgctgagtggctcagtaattattcctgccggtcagaatagcgtaacggtaacagtgccgataatcgacgaaaaggtgattgaaactaccgaaaccgtgatcctcacgcttacagacggtgcaagcaccagcttcgccttcactgccagcactaccagtggtaatgctaccgtgaatattgcagatgatgataatatcccggctaacctggtgatcgaagtaaccaaccctgtaaacggtgcagaaccagctaccaatggcagctttacagttggattgccaacaggatacaccgcatctgaagatatcactgtgagctacaccataggcggtaccgctacaggtggcgccgattacgctaccctgggtggaaccgtggtaatccctgccggtcagaacagcgtgccggtaacagtaaatgtaaccgacgacaagatcatagaaaatacagaaacagtaatattaacggctacgggggctacttctaccagctttactctcgtggcaagcagcaccagcggaaatgctaccgtgaatatcacagatgacgataacacgccggctaacctggtactgggcgtaagtaatgcaggcgatgcaactgaaccgtctacaaacggcagctttaagatcggcttgcctggcggagtaacctcggccgaagatattacggtgaattataccatcagcggtacagctaccagcggcaccgactacaatacccttagcggtaccgtagtaatccctgccggacaggatagtgtaagcgtaccagtgagtgtgatcaatgacctcatcattgaaaacaatgaaactgtgatcctcacgcttacaggtggtacaagcaccagcttcaccttcactgccagcactaccaatggtaatgctacggtaaatattaatgatgacgataataccgctgcaaaccgcgtgctggcggtagccagaaccgcagacggcgctgaaccaggcaccaacggtaactttaatgtaagtctgcctgccggtataacagccgcagaagacatcaccgtgaactatgccattacaggcaccgcgacgaatggtaccgattacgcaaacctcactggttcagtagtaatacctgccggtcagaatagtgtagccgtaccagtaacagtcaccgacgatcagatcattgaaggcaccgaaacggtgatcatgaccctgaccaacggagcgtctgccagctttgccttcacggccagcactaccagcggcaatgcaaccgtaaacattgcggacgacgataacactgctattaaccgcgtactggtggtaaccaacacaggtgatgctgcagaaccaggtacaaacggcagctttaatatcagtttgcctgcaggaataacttcgactgaagatattgccgttggctataccatcgcaggtagcgctactgccggttcagattatactgccatcaccggggtgatcaacatccctgccggtcagaacagtgtagccgtaccagttaccgtaacagatgaccaggtgattgagcctgttgaaaccgtgctgttgacgctcaccggcggaacatctaccaactttacattcaccgcaggcggcgccaccggcaatgctactgtgaacattgccgataatgataacacaccggctaaccggacactcaccgtggtaaaaactgctgacgcatcagaaccgtctacagccggcacattcacgatcagcctgccaaccggtattactgcatctgaaaatgtgaccgtaaattataccatcggcggtaccgctaccgcaggtacggattacagcacgctgagcacttcagtagtgatccctgccggtcagaacagcgttactgtgcaggtaccggtgatcgacgacaagctgatagaaaatacagaaaccgtgctgatgacactgaacggcggttcttctgccagctttgctttcaccggcacagccagcgccactgtgaacatactggatgacgataacaccgcggctaaccgtgtgatccaggtaactgctactaaaaatgctgcggaaccaggtacagatggcgaatttaccatcggcctgccttcaggcattacttcatcagaagccattacggtaacctatactatcaatggtaccgccaccagcggatcagattataccgccctcaccggcaccgcggtaatccctgctggtcagaataacgttaccataccggtaccggtgatcaatgacctgatcctggaaaataccgagacggtagcaatgaccatcacaggtggtgcatctaccagcttcaccttcaccggaggcggcgccgcaaccgtgaacatcatagatgatgagaacaccgcagctaaccgtacactccgcattgtgaaaacagctgatggtgcagaaccatctaccaacggcagcttcacgatcagtctcccggcgggcattattacctccgaagccattaatgtaaactataccatcggcggcaccgccaccaccggtacagattatgcggccatcacaggaaccatcatcatccctgccggtcagaatagcgtgagcgtaccggtaaccgtgatcgacgacaagctgattgagaacactgaaaccgtgatcatgacactgaacggcggcacttcttccagcttcacgttcaccggtacaggtaatgctactgtgaatattacggacgatgaaaacacagcgggtaaccgtgtgctgacagtcaccaaagtaacagatgcagctgaaccagctaccaacggcggatttaacatcagcctgcctgccggcatcgcttcatctgaagctatcaccgttaactacacgattagtggtaccgctaccagtggtgcagattataacgccatcaccggaacgatcaccatccctgccggtcagaacagcgtaaatgtaccggttactgtaatgaacgaccaggtaatagagaatacagaaacggtgatcctgacattgaacggtggtaacgctgccagctttgtattcactggtacaggtaatgctaccgtgaatattacagatgacgagaacataccggctaacctggtgctcaccgcaacaaaagcaacagacggctcagaaccagctaccaacggcggctttaacatcagcctgccagccggtatcacttcttctgaagatatcaccgttaactatacgatcagcggcacggctaccagcggtacagattataccgctatcacaggaaccatcaccatccctgcaggtcagaacagcgtgagcgtaccggtaacagtaatagatgatcagctgatagaaaatacagaaaccgtgatcatgacactgaacggcggaacatctgccagcttcaccttcaccggcaccggcaacgccaccgtgaacatcaccgacgatgaaagtgatccggccaataaagtgctgagcgtagtgaaaactaccgacgcagcagaaccgggcactaatggagcgtttaccatcagcctgccttcaggtgttgcttcttctgaagatgttactgtgaactacaccatcaccggtactgctgccagtggtacagattataccgccctcaccggcaccgtaattatcccggcaggtcagaacagcgtgagtgtaccggtaacagtactggatgatcagttgattgaaaacacggaaaccgtgatcatgacactgaacggcggaacatccaccagcttcaccttcaccggtacaggtaatgctaccgtgaatattacagatgatgaaaacatacctgcaaacctggtactgaacgttgtgaaaacaacagacgcagctgagccaggcactaacggtgcgtttgcgatcagcctgccatcaggcatcgcttcttccgaagatatcaccgtgaattatacgataagtggtacggctaccagtggggcagattataccgccatcaccggaacgatcaccatcccggccggccagaatagtgtagccgttcccgtaaccgtggcagacgaccagatcatagaagtaactgaaactgtgatcatgacgctcaatggcggaacttccaccagcttcaccttcactggtaacggtaatgctactgtaaacatcaccgacgatgaaagcagcacaccagccagcatggcgctgaccatcaccaaagatacagatggcgcagaaccagctactaatggcggctttaaggtgagcctgccagcaggtatcacttcatctgaagacatcacggtgaattataccgtaacaggtactgccaccgccggcgcagattataccgccctcaccggcaccgtgatcatcccggcaggtcagaacagtgtagccgttcccgtggttgttgcagatgaccagatcatagaagtaacagaaacagtaatagccaccctcaacggcggtacttctgctaacttcaccttcaccggaaatggtaacgctaccgtaaatatcaccgataatgaaagcagcacaccagccagcctggcgctgactgtcgctaaaggtgcagacggtgcagaacctgccactaacggccactttgttatcagtctccctgctggtattacttcatcagaagctatcacagtgaactataccatagccggtaccgctacgccgaatgcagattacaccacccttacaggtacggtagtgatccctgccggtcagaacagcgtgaatgtaccggtaaccgtatcagacgaccagatcatagaaggtacagaaacggtgatcctgacactgaacggtggcacatctgccaactttaccctcacaggtaccggtagtgctaccgtaaatattaccgatgatgaaagcaacctggtactgaacgtcaccaaaaatgcagatggcgcagaaccagctaccaacggcggcttcaccattggtttaccagccggtgttaccgcagctgtggatatcactgccacttacaccattgcaggtacggctaaaggcggcgccgactacaccaccctcaccggtacagtagtcatcccggcaggtcagaacagcgttgccataccggtaaccgtaaccgacgaccagctgattgaaggaaatgaaacagtgatcatcacagtagccggaggcaccgccaatggccttgtgttctcaccgggtaccaataacaccgttaccgtaaacatagcagatgatgataacacgggcctggacctggttgtaaatgctaccacaccaaatgcggcagaaccagctacaccaggagcgttcacgatcagcctggcaagtggcaaattacctgtggaagacattaccgttacctacacagtaactggtagtggcacagcaggcgccgactacaccgccctcaccggcaccgcagtaattcctgcaggccagagcagcgtgatagtaccggtaaatgtaacagacgacgatctgatagaaccagcagaaacagtggtgttcaccatcacaggtggtaagtcggccagcattaactacactgtaggtaccagcagtactgccactgtaaacattgcagacgacgatcacactaacctgaacctgctcgttaccgccagcaaaccggatgctactgaaccgaatgtcaacggggcgttcacgatcagcctggccagcggcaagcgcacagccgaaccgatcactatacaatacatgataggtggtaccgctacaccggatgctgactacaccgccattaccggaacaatcaccatcccggccggcgccagcagtgtaaccataccggtgagtgtactggacgacagtgaagtagaaacaccggaaacagtggtgttcatgctcaccggcggacaatcagccagctacaccttcacaaaaggtgctccgggcgacgctacggttacgatcaccgacaccgataaactggcgggcgacctggtggttaccaaagaaatcgtgacaccggcagttggtccttaccgcatgggtcagaacctgacctaccgcatcactgtaaggaatgcaggtaatatcccggtaaccgccgtgaaagcagaagaccgcttaccggtacaactggatgtgcctagtcatacttccgcagaaagaggagaggtagtagtaacgccagccactaagctgatagaatggaacatcggcgacctggcagtgggagcttccgtacaaatgacgctgacagcccgcgtaatagaaggcggacagctgatcaacgaagcaactgcttacagtacaaacatgccggacgccgacagtgccaataacgtaggggtatctgcagtaggaatagaaggttcagacttatccttcccgaatgtgatcacgccaaacggcgatggtaagaacgaaaggttcatcatcggcgggctggagaaatatccgggttcatcgctgtacatcttcaaccgctggggcggacaggtgtaccagtcgaaggattaccgtaacgactggaacggtgctaacctgaacgaaagcacctactactatatattggaagtgaagaaggagagtggaatcaaaaagtataaaggctggataacaatactgcggtaaaagacaaaaatattatctgctacaaaaaaagtaaaagatgcaaacagtactcagagcaggaataatggtgatgctgctggcgataggaatgcgtggagcagcgcaacagaacatacagttcagccaatacgtgttcaacgggttaagcgttaaccctgcctatgcaggctataaagaagacctgtatgtgaatgccgtataccgccatcaatgggccggtttccccggcgcgccccgtacgggcggcgtgtcgatagacggggtgacgccggccagtgataacaaggtggggctgggactgcagatgttgtttgataaactcggtccgcaggatgccttgtcgctttacggttcttactcctaccggattccgctggatgatgaggatacgcgccggctttgcttcgggctgggaggaggcgttacccagtactctatcgacggttcggccctgcaatacatcgataacgatgatgccgcccttccgttgggaaagaaaagtgtatgggtaccggacgcccgcttcggggtttattattacacaccgcgcttttatgcaggcgcctccatcatggacctgttttcgctctataccgatgcaacccgctacagctggaaaggaaacaactattctacgatccgcaaaacacagcacctgtatgttaccacgggtgctatgtttccgctgggcgacaacctccagctgaagccttcgatcctgatcaaggaagattttaaaggacctaccaacgtagacattaatgctttcctgctgattggtgaaaagctgtggacgggcgtctcttatcgcaccggtgtaggcgtgtggaacaaaaccaacctccagaaggacctgagtgagctggacgcagccagcgtgatggtggaattctacgctacagaaacgctgcgcatcgggtactcctacgacctcagtattaataaaatggcaggttaccagggaggatcgcatgaaatatcactaggcttcttaattccttcgaaaaatttcactgtaaagaatcccaggtatttttaaccatagtttactacccgtatgatacgtcgcactataattaccatcccgctgtttcttattgccttcaacctgtacagccaggagcagaaaagcatgtcgcaaatggctgaagcagcctatgcacggcaggagtatgcagaggcaggagcgctttataacaggattgcccgcagcaagggaagtaagatgccggtagatcagctgatgaagatggcccatagctaccaggagatcggctactttaaggaagcttcggatgtatacaaggaaatcacggagcgggccgaccggccttcgtctgcctattttgcatatggcgaagcgctccggcaactggagcaatatgatgccgcaaagcagcagtatgcgttgttcaccacctccaatgcagatagtcttaaactaaaagagattgcactgcagggttgcgacagcgccgttgtatggcttaaacaggcagcgcctatacagttaaagccggtgaaagagctgaacacacaaggctccgacctggtaaccggcgtggtacagaaaggtttactgctgatgtcaaacgggtaccgctctatggcactgaataacgggtcgcaggcaaaacctccgatcgataaacgcacggaacaaccttactataaagcatacgtttaccagcaatatgccggcggcaaccacgacatgttcctggaggaactggcgcctgcactactggccaaatacgattatcatattggcccggtgtgtttgaacaccacagaagacacgctctatgccaccatcaacatacagggcaaaggggttcccgttaccggtaaaggactggtaaatggtgttcgccagttgcagatctatcaatctgtaaaaaagaatggcaaatgggaagcaccggtactgatgcccggcatcaatgtaacgggatattcttccagtcacgcggtattaagcaccggtggcgatatattgtatttcgtgtctgaccgcccgggcggtcaaggacaaacagatatctggtacgccgaaaaacaggcagacggttcctggggcgcgccggtcaactgtggcagccagataaataccgtggcagcagaaaccttccccaccgttaacgaagacggcattctttatttctccagcaggggatatgcaggaatgggtggttatgacatttaccgcataaaaggcggcaaatccagctgggaaataccggagaacatgaaagtacctttcaactccggcgcagacgatttagggcttattttgaaacgtaacggctatgaaggttacctggcttcgaacaaaccaggcagcatgggcaaagatgatatctattatttctcagacgccgaatattttaccaggatcaaccgcagggaaaacccgccggtgataacagatcatacggcccctcctgtaactggcgaccagcctggtggaggaaagaaaggacatacgccggaagaagaagaggatagaaagaagctggaagaactgaagttcttctatgattataacagcgcatcactgctcagcgagtcccgcaggatcctggaccaggtagcggcggtgctgaaacgtcaccccgactggaagatcgtaattgcatcttttgctgataaccgtggctctgaccaatataacactgatttgtcggccttacgttgttatgcggtaatagattacctcgttaataaagggatcgattccaaacgcctctactacaccaataacggggagaacaatcctgtgaacggctgtaaggatggtgtaccatgtaaggaagaagactataagcagaacaggcgcaccgaactgcggatcaaatggtagcacttcgctgaacttataccatacaaaaaagccttcaaatcatttcggtttgaaggcttttttgtaggatattttgtcggcaggcaggtaccggggtcctttcaggtaataaagttccggatagcactacccttgcgtataaacagattttccctgatctgcagcatcttgataactattgcaggaaatccttgggcaaggtgttgtaaatatgaaaaattaatctttcatttgttgtgttatgagggaatttgtaccgtagcaagtgttatccctgatattccccgatcataacaaacgtgtcctgaacctttgtctgaagccttctgcagttttcaattcgtttttttgaagtttggaatttagattggaaaaaatatcggaatttttttaatcgtcagttaaacacttataatgattacaatatttactggtacttgattgtatggttattgtagatgtcgtttgccctatataaaaagtttagtcgtcccacaacgattaaaccatattttaccctttacccactcccgttatgatgatacggataaaatggttattgattttattatgggggctccctgcctatagccaaagggtggacactgttgctgcattcccgcagaaaacccaccatcgcatagctaaaactattgaagggcaaggggacatgtctgacaggctaaagcgccggcaactgaagctgatcgcaaaactgcagctaatggaaggcaaagccggccggcggttaaaagaagtggataccatcgcagctatgacctacctgcaacaaacaaaggacgcctatgcaaccctgctgggaaaattgaatggtacaaaagaagaagggcagagcccatatattccgcgtctggattctcttcattgcctggtaaactttttaggtgccacagcggatggaaaagatcatttaaataaagccttaaaaagtatagacgggctaaaagccgactggctaaggggagaacgtgtaaaaagtttcctggcagaaagggctgcgatgttaaatagtttacgggagaaattcccgcagctaaagggcatcaaaggcgccgcggcgaagtactcaaaggagcttttctattataagcgccgcctcgatcaatggaaagaggaactgaatacccccgcagactgggaagctacggccttgaaggcacttggcaaagttccggtattccagcaatttttacgggaaaacagtcagttgtcatccttgtttggtatgcagtccaacgggggcccgaatgtagcggcagtaactgtaaacgggatgcaaacacgcgctactgtgcaaacattattacaacagcggcttggccccgcggccggaaacctggaacagcagctggccagtcaggcagtggcgcaaggcacaggcttcacagatatccggaataaaataacctcactgaggtcagcaggaatgtccggtgatgaagcatctgcaatgcctgcctttaaaaaaaatgatcagcgtataaaaccctttctcaaaagactggaatatggatttgatctgcaaaccggcaagcgtagtgcttatcagtttccggccagcaatgacctggctgtttcactggggtaccggttgaacgaccgtctggttacaggtattggcgtggcctataaatttagtatgggcgaagcatggaacaaaataaacttcactcatgatgggatcggcttgcgcagctacctggactggaagcttgcggcgcccggcaaagggaagaccgcattgttgggtaatctctggatcagcggtggtattgaacaaaactattggtcacgttttgagaacatagcggaactgagaagtctcgcctggcaaacatcaggtttgataggagtagctaaaaagatccaataccagaagaagacggcgaaactgcagctgctgtgggattttctacagcctgccggaaatcgcgcagttgtattccggtggggatacaacttctgacaggaatcataaagatcaaaaagcaggaacacatcactgaacgctatatcgcccataccgatttgaaattaataaaagttgtattgatgaacgtattcaaaacatgcctcggccttctgaccggattattaataatgatccccacaaaagaagcgctggcacaagcacccgccccctataccgtacaggatgggaatactatttatactgtcacggcaacttctccccaaacgaatcccactattctgaatacgcttccgctgagagatgccaaagtcgcaacgcagtatatcgacggccttggccggccatttgaattggtgcagaagaaagcgtctctcatcacggaccctgccagtccgctgtcttccaccacagccgtagacttggtgaccgccagaacatatgacgtgtatggaagagaagtatattcctttttgccttttgctgccaataatacgaacggcaatacttctgtttccgatggaaacttcaaaaaaaatccatttgaacagcaggccatcttttcccaggcaatgtacccgggagaaacctatttttatggtaaaacgaattttgaagcatctcccctgagccgcactacggaggtgtatgcgccagggaataactgggttggtacagaatctgccacaaagaaaaatataaccaccaggtacctggtaaatacagtgaccgatgccgtcagatactggaccgtaacaatagcgccggtgggaggactaagcacatacgccacttcaactacatatcctccgggaaccttattcaaaacgatccggataaatgaacatggcaagcaggttattgaattcaaagacaaagaaggtaaagtagtgctgaaaaaagtgcagcttacggcatccgatgcgggaacgggaagtggtcatgccggttggctgaacacctattacatctatgatgattttaaaatgctgcgctgcgttatacaacccaagggggtagaactgatctctcccaactggttactgacggatgttaccatattggcagaacagtgcttccggtatgaatacgatgcaaagaggcgacagataataaaaaagatgcccggcgcaggcgcgcaatacctggtatatgacagtcgcgataggttggtgctccggcaggatgccatcctgggaagcgggaaatgggaatatttccagtacgacagccgcaacaggccggttgccagcggtatctggaccaccgctactacttttgcagctcacattaccgcagccgcgctcatcccgggtggaaccgctgctaattatcccgcggcaggaacctccggcctcgaagagctaagcagcaccttttacgataactacgattttctgaccgccaccgcttacgccgggcatggattgaatacaggtttctttacaggagataacagttatttttctgcagccagcaataccgcctggccctatccgcaggccgtaacttcaacaaccgccacacagggaatgattaccgggggaagggtaaaagtacttggaaccgctacctggctttatacggctacctactatgataacgatggaagaaccatacaggtgcaaagtaagaatgtgaccggcggccttgatatagcgactacccaatatacatttaacaatcagccgttgatcactgtacaacggcaggtaatcgccggcgccggtgcgcaaaccactattgtgttaactaaactcacctacgacgatctgagcagacttgtaaaagtggagaaggctatcagcaataccaccgtgaatagcggggccatgacagcctacaaaactatttcggaaatggcctacgatgcgctggggcaaataaaaagtaaaaagataggcatacagccaggtgcatccacaccactggaaacgcagcagtcaacgtataacatcagggggtggctgttgggcgtaaacagggaatttaccaacccggccacaccatcaacaccaggatcaggtaactggtttggctttgacctgggatacgataagcttacaaacgcatccgcccggaattacctgggccaacaattaaacggtaacatcagcggaaccgtctggcggtcagtaggagatggcattccccggaaatatgatttcagctacgatcccctcagccgcctgctgtcggccggctttgagcagcgaaacagcgatggcgcctggaacaacagcctggtcaattataccgttaaaatgggaagcaccggtgcagaccccgctaccgcctacgacgccaacggaaatattctccgcatgcaacaatggggactaaaattaaatgccagcagtcagctcgacgacctgtcttatacctatcttcccaatacaaaccgtatacaggcagttacagacgtatttaacgataatacaagcacgctgggtgattttaaatacaatgcggctaccaaaactaccacagactatacgtacgacggcaacggtaatcttaccatcgataaaaataaagggattaccagcgccatctcttacaatcatctcaacctcccggctgcaataccggtagcaggaaaaggaaccatcacttatacctacgacgcctccggaaataaatggaagaaaagtgtgacagaaggcagcaccattaccaatacctactatataaatggagcagtatatgagcagaaaggaacaggcccgctggtgctgcaatccatgggtcatgaagaaggccgcatccgtaatactattcccacaggtggaaccaccctggcatttgattattttctgaaagatcatctgggaaatgtgcggatggtacttacggaagaagtgaaacggattaattatccgatagcaggcatggaaaacgtaaccgacaagaataacctggcggatcccaataactatataccctattattccaacacggattataccgtaacgtcttccgtgcgtgaattgaaatcaaacacttcaaatcctcccgccaacggcactacgaatccgaataactactggaccaagctaagcagtgtggccggcgaccggaaagttggtcccggaatattactgaaagtaatggccggcgataaaattgaactccgttgtgatatgtggtggcggggatctgccaccggcgcaacgcagcaaagtccgctggcagatattttatctatcctcgcaaccaccattacaagcggaccaggagccggtaaaataactttgccacaaacaggtaccaacggcagctttttcaacccggcggtcaccggatttatgagtaacagcaacccggcgcaaaccacaaagcctaaagcatacctgaactggattttcctcaatgaacagtttgcctataccagcaccaatggcagcggtgctgaaccgctgggcgccgccgatgcctataaaacctatacaaggctcgacgcgaacggaaatgccattccggtattgcagagcggatatgtttatatttataccagcaacgaaagcaatattgccgcgttctttgataacctggcagtgaaccatatccaggggccattgatagaagaaacgcattattatccgtttgggttgacaatggcagggatatcttcagaggcacttaaaggatcagcttatccggagaacaggatgaagtacaacgggaaggagttgcagaataaagaatttacagatggttcggggctggagtggtatgactatggcgcgaggatgtatgatgcgcagatagggcggtggcatgtattggatcctgatgcagataagatggttaattattctccctataactatacgctcaataatccggtacgacttattgatcctgatggcagaagccccgaggatattgtgttttttgataaaacagggaaggagatccatagaatacaatcaaatacccagtatagaacattcgtacaaacaggagaattgacatttggtaattttgtgtcagggaagacatttacggaagcaccaatgcctaatgtaataacatcaagagaagaaagcagtacaacagctcccaaatatcaaaagtatgactatgcaatagccgccgagacattcctttttaataagaataaggaaaacgggatagttccgacatatacaaacgggactactcttggcgatccatcatctgttccggatctggatcctacactggtaaaagctatgattatgcaggaaaccgtaatgggaacctatgatggaaacaagaaggacaataatgatgcaaccacagacattatgcaatcaaatgtatactacagtgcaaaatctaatgactggagtgattccaagactcaatttggcttagaaaaagggaaaggtgtttccgatgcaacacagagtgtgaaagcaggtataggtattttatatcagaaaggcctcaaaggtgctgacggcaaaaaatggactggtggaatagattggggagaagcagtaaggcggtacaatggtggtggagtagataactacaaagaaaaagtttttaagatgaaaatggattcaaaagaacctaatccttcaaattattaaactatgagaaacagcatatgtatttatatatttttgatagtgtatttgtcgttaggatgtaataataaagtcaataacccggataaaggtgccgccgttagtatgaaaggaggtgatagtaatatgttgaacagtactgatagttttaaaatagatgctattgagtttgttaaacaggataaaattgttgacactattgatttaaagagcatgtctaaaagaataacctgttccaatgattatactgcattaaaagaggaggaaattgtagacgaattcagatttttcgaaactcagattctttgttttaattataagggagatataaggggggggcttagtgattcttcctttgtaacagcgttttataaaaaaacagtgaatgagaacgaggagtattttcaggttgagcaattacgatttttaaaaattgattctatggaagttgctggttacggagattgtataatagcatcatttgaatatttgaatccgtcttcagctaatcaggataaacctactgtaatgtttaacactgaaaggaatgaagcagttgtctggaactttagcgattggggcataagaaaaggtatgattgaactggattttaaggttagaggaggaaagcacactttatataaagttgaatatgatgataagatcaggaactttatccctacttgctataagataatagcatcaaagtaatatatcacaacaaatcctgaatatctataaaagaattttccttatgcctggctgtcataaactaatcagatcctgctatgcccttattgtatgcgggatcttctatccgcacatcgtatcctcacagaatacggcctttgatgaaatgcgaaaaattccgattacttctccggatgtcgcgtcgctgactaaggcagcagagtttcccgttacctatttcaatggcaggccggaagtatctattcccctttacaccatccgtacgggcgatctggagtttcctatcagtttgagctacaacggaggcggcatcagggtgtctgaagaggccagttgggtaggcctggggtggacgttaaatgtgggaggagttatttccaggcagataaaaggagcggatgatgatctggtgtctaacggaacgtttaagcaatattatccggacgcactgggaaatacctatcaggccggcgcccaggcgcggaattttatgttacaatttaacctgctatataaagctaacggccaggcttatacgaagccggagctttgccctttcctttgtcctggagatattgatggtgagccggatctgtatgtttacaatttcgggaaatatacaggtaaattcaccgggttttctactgctgaagtggtggatgtcagtggcaacaatgtccggtttgaaaaatcaggcggtggaattatcgccaccgatccggagggtttccggtacgaatttatggcgatagaaatgtcgatgacggcggccgggcctactaaaacggcttactatctcacaaaaatcaccagtccggctaatcgtattcttacgctgaaatataaaacgttccgcgagtacgtttatcctgcaacgggcgccggccatagcacggattataccggtatttccagtgcattcaccaacgtggactatgtaactcaaatgcccgacctcactgaagagtatatccaataccaggctgtttccatgcgggggccaatgggcatgcccaccaatgtcggcttgaacagcactttcagcacctctaccatcagaacgcttttcctggatagtatcctttttgaaaatggcgccgtgcagtttataccagacagccggaaagatttatttggcgtaaagctgaatgggatcactgtttttaataaagccggtagcgctgtgatgacagccgggtttgactatgattatttcaccgcccggcccgggaacgaatcgtatactaccgcgagcacccggccgggaataaaattgccgtatgatgagtcttaccggcggaaaagattaaagttgaaaggtgtaacggtaaagggagaagtatataaatgttattattacgaaggcgccgacggatttacattaccctacaaaagttcctttgaacaggattattggggatattataacggggcagcttcaaataccacactggtaccggattttaagcgatataatttcctggctgccattccgcaggtactaaggagctggataggcgctaaccgcgacgcaaaatttccacaggcacaggaagggatgctgaagaaaatcatgtatcctaccaaagggttggcggagtttgaatacggccttcatgaatttaacaatgcaccagcagatatcattgttaactataacaacgtgggcgcattaaataccacaacaggcgttactaccaccacggtggacatagcagcgaattgttatgtggatataaccgtgaacctgttctgtaatcagcctgcagacgcaaatccaacaggcacaggttgggactgttcctgcatattcccgccgtgtagccccgttaatatgcaaaatgcgatgtgggtaacgatagaaagagtagacccggccaccggtgcggtgagccccacggaatgggaatatgatttttccaaagatatcgtaaggaatcaaagcggcaattttgtattaaccaatcaatactttacagccggcagatataagttgacggctaactaccccgacaataaagtgggcgcgccggggcaaaaaatggcctatatctcccttaaaattccggttactacaaatgtggctccctacggaataggtggcgggctgcgtttaacttccagcagtaggtttgatccggtaagtaaaatcacatcgaagaaattgtatgcttacgaacagggcatgatgatgcattttcctacttattacagtggcctgaaaaaccaacagacggatgtattgaccggcacagacactgaagtaatagatgagtatatcacgcacacactttatgctaatccgcgccaaccgtacacgttttccgcgaacggaagtcatgttgggtatggtaaaataaaagaaaattttacaggagaagcattgggcagaacagaatatctgtacaacgtgatcccggataaatatccgcatttgtcgaaccttgatcttattcccggcactcctcctatccccagcctggaaaatgggttcctgaaaacagtgaacttctacgataatgctaacaggttagtgaaatcagtatccaacacggcagtggtaaaaaagacccaaaccttttgggctttcaaacaacgtaagcaaatgaattcacaaacggttaatacagcaaactttgacatgtacctgcacttgtctttttatcctatccagacaggcaagctgctcacagccaccagtacggaaacgatgtacgataatgtgaatacgcccggtatcaccaccagcaaaatttttgagtataacgaccgcgcttttcttcaatcggaacaactgacccgcagcgatggaacaccggttgttaaacactaccggtatcccggcgattttacggcgactaccggttggattggagagttaaagacccgcaatatgatcagtatgcccattgaagcggtgacccaggtaaatggtaaactggtggaaggaacctataaaacatttgcgctgcatgataatattgtaacccccaatgaggtatttgctgcggaaacattaaccccggcaacggtggcctttattgcgccttccggcacattgccggccgaatataaatccgccggacaactggactatgatgcaaaaggaaacctcaattattccaaatcaaataacaatatcagcataggctataaatggggctacaataagatgtacccggtagcagaatgtaaaaatgcagttccttcgcagttttattatgaagattttgaggggaacggcccgcttgtctccaataccagcacggcacacacgggaaaaggcggttacaacggatccattgcgcttgccagccagttttcagccaccacagcaggcagaacttaccgcctttcttatttcaaacagaatggaactgtctgggaacatatagatcaaccatataccgggcagtctttatcgggcgtagtggatgatatccgcatctatccgcaggacggagaaatgaccacctacacttatttgccattggtaggaatcagcagcattattacgccctccggtaatacttctttttatagctacgacgcgtataacaggttatccatgatccgcgaccaggatggttatgtgatgaaaaccttcaactacgcctattccgctactttaggtcaggataattctaccacctatcccaatgtagccattacgcaaaacttttataagcagtgtaccaccggtgagggatcgctggtgccctatactgttccggcaggaaaatatacagcaggatcccctgaagaagcaaatgccctggctcaggcggaaatcgatttgcaggggcaggcaaatgccaataccaatggaacctgcgatgttggactggccattacaagtattgtaaacgggcctggaactacgtttaccgtcaactttacctgtcctcccggtatgaacttctttatcaatctttttgctaaagatcctgttaccggaaggccatacaacgataggccattcgttgttccgctgggctctaccagctttacaggcgacatcgcaaagggtaaaacatggatattctctatcaccgcaggaggaactaattttccatccgggataagctcggcaaacgtcagctttacttttccataatcacgtaaataataaaagaggggcagccagggtatccgtggctgcccctcttttattatttacgccaatgtgtaatattttgaatactttcagcaactaatagtgcaaacgctgaaaatgaaactacaatccatcctgacaatactgctgtccttaacttttggcgccgccttttctcaagcagaaagcccgggaagcaggtatatatcggcaaagtttgaaaagtattacaacaacggtcagtttgatagcatttttgctacattttctgaacaaacaaaaaccgctttgccgttagataagacaaaagcatttctcaccaatttgaaaagcaactacgggaatatcataaagcgtacatttttggaataccagtcttcatttgccgtatacaaaacagcgtttgataaaggtgtcattcttcttaacatttcagccgacaaggatagcactatcaacgggttatatgcaaagccatatgtgccggatacattgccggtattgccgcggaatatcactgccatgcacctgccttttaaaggggaatggacggtgttctggggcggggatacaaaagaattaaactatcacgtagcggttaaattccagaagaatgcatttgatattgtaattaataaccaggagggaaagagttttaaaaccaatgggaaaacaaatgaggactactatgcatttggacaacccatcattgcgccatgtgatggagaagtagttttagcagtagatggggttaaagataatgtgccgggagagctaaatcccatgtttgtttcaggcaatactgttttgctgaaaaccaaaaacaaagagtatgttttctttgcacactttaagcagcattcaattaaggtaaaacaaggcgatgtaataaaacaagggcaattgataggactatgcggtaactccggaaattcctctgagcctcatttgcattttcaccttcagaatgtggagaacaccaaccaggcaaccggtgtaaaatgctattttgaaaagctcaacgtaaacggcgttgtaaaaacagattattcacccattaagggtgataagataagcgaaaccaggtaatctataaaagtagctcttatggattcttcattaaaaataacattgtggcatcagttcggagcatctattgacatgctcgaaaatgcgttaactttttgcccggatgaactatgggatacccctgctaagttctggtatatcgggtatcataccttgtttttcctggatttttatttgtctgatgaaacaccgatggaaaaggactttttaccaccggagccatttacgttatctgaatttggcaccgggatgccggaacgggtgtatgataaaacggagttgctgacatacctccggtttgggcgtgagaagttacggggtctgctgacaaggttaactgctgaagatattttgacgaagcggtttgttagtgagtacaaggattatagtatattggaaatactaatttacaatatgcgccatgtgcagcaccataccgcgcaactgaacctgttattgcgccaggaggtgaaagatgcaccggattgggtatccgcaacaaaagcagatttagcactttaaagcagcagcgattataaattaatatacctggcaatcaggatggtaaaatacttgtttccaggtattgccgggggtattcaaccagcataactttgcggtattaattaacccaatacacgcaaagagatgaaaaggacaacacggattttttttagtttgtgcctggtaatgatggcaggtttggcatttacaggctgcggcggtaaagacgatcctgcacccgataataaaaaagcaacctttaaatttactattaccgtagcaggcgctgatgataaggatcaggtggatgttcgcgtatccgcagggaatcatgatgccagccagtacggatcacctgtttggaaaataaatggggttacccagggaaatgaaaatgtgatgatactcgatattgataattttgtaggaggcgtaaaaacatatgtagttgaaaccgttaagccgtttaattttagcggattaagtgtaggtgtcgtgaataacgcccaggttcccggcgcggtaacgatcagttataaggccgaagtagatggcaaggtggaaacgaatgtgcaaaatgtggcgactgctgccagtcaatcttataataaagaatatacttacgtagcaaaataatttttcattgcggttaacgtcaataaatccagggaacgctttacagggcgttccttttttttgtgacaaaccggggggttacttcttggatacttctccgatacttctccgatacttaggagtcgtgtatatgttatactccccatatactccccatatagtccccctgtactccccctatagtccccatactgttccgatactgttcccatactctcaccatactctcatgatacactccccatacattccccatacactatgaccgtttccgggtcgcccgattccggcataatccggcaaaaagcggcaaaagcggcatatttgtttttttctgttcccttctgtgaatatttttgtgttgtacttcctggcgtaactgatcctttgcaatttttcgggtgtgggataacttttttatatttataacaagcaacaggttaatcaaaactaaaagaaattaaacatgaagcggcatatttttattataatttttttgatggtaagcctggtttcctgtaaatcgaagaaggcaacggaattcagagaagcaattgctcaaaaggagaggactgcattccagattttggtaggcaaaggaggccccgaggaagagaagttgatatgcctggtaaataacgatttcagtggagccctgcgtgcggtagataaacaggaacaggcatttgacagtatcatccgggagataatcgcattgccggcagaagggatcagcgaaggagctgcattaaaaacagctgccataaactattacatgtccgtaaaagatttgcaggtatttgaccgcaggataattgcaacacaacaagccatgcaccaaaccaatgcagactcgatagagaatgcgcaggacaaactattattgctgcaaaaagaaaaactgacgatgtccggggtaaggaatgaaaaaaggacagcgctccaggaagccatcgggagattcaataaagcaaacgatttataagcgcctgtaatccaggtgaaaaggccattgtacccaggtgaacagattcatgaaaacccgcgctgtgtccggaatatggccattgttaacattattttaatattactttcatttcaacataacccctccgtactatgtttgcatacatcttctaaacacagaaaaatgtgagaacgttttcggaaaagaccctaatctcgctgctcaaaaaccaaaatatccctgcatttaatgagctctattctcgttattgtaaagagctttatgatgccgcctataaaagactcctttctaaagatgatgtgcaagacattatccaggatatttttatttctatctggaacaatgcagaaaacctcgacgaaaacctgtcactccggccatatctgttcaagtcgctcaagtacaaggtgatagacgccatttataagaataaaagtaatgcacacttatccttaactgatatcggcgaaattgattttataaaggagagccatgatcccctgctcgccaaagaacttgaaacgttcttaaataatgagattgataatttgccggtgaaaatgaaacaggttttcctgctgagcaggaaacattacctccccaatgatgaaattgccaaacaactctctatatcttcccaaactgttaaaaaccagatctctatggcactcaaaagattgagggagtcgctggaaaatgctaatattctctgatccgcacattaaggaattgttatctcgcacctgccttatggtacttcaccccgtttaaagagaagtatatagcataaaggcaaacttgtggatctaaacgaaaaaaaaatcagggagctgctaggtcagtatttgaatggtacactatcgccagaggagagcgaacaggtagaggcctggtattcatcttatgatatcagccatcctgcttcaccagcattttctactgaaaaggaagaggaagaagcgcatcgggctattttaaaaggtattcatggtaaaataaaatcccagccgcaaagaacaccggtaagaaggatgggcaacatgataaaaatagcagcggcagtaggacttgttttgatttcagcaggactcactttttttcttagcaaaccaggtggtaaacaacaactggctgctgttatagattcggctgccatgaatacgattgaagtggccgaaggtaaaatgaagctggtggagctgtcggacggtactaaaatatggttgaatgcagccacgaaattcagttacccgaaacagttttcagagaaaacaagagaagttaccctgctggaaggtgaagctttctttgatgtggcgcatgaaactaaccggccgtttattgtgcacagcaagggcttgagcacacaggtgctgggcacctcttttaatattgacgcctataatttctctaaatgtgtgagaatatcagtggccaccggtaaggttggcgtgaaccgtggcaaggaagtgattggttttttaacccctaacgaagagattcaatataaactgctgttgaataaatctatcaaatccaccagcgatggaaaagcggtaagctcctggcggacaggcattattgtgcttgattatgttgactttgagagccttcaggccattctctttaataactataactacgtattgaaaacaggcaaacgggatttaaatcatcttcatttttcggcaaccatcaaaaaaacagaccgtattgaagatgtgatgaaactcctgagctccatcaataagaccaagttttctattaccgacaagacaatcgtaatgtattaataacccggtgtaatcctgtttaaacgaatgaaaataactgtagcatctttagagcgatttttacgtatttccgtattgtgtttcctttacattctcaatgccggcattctgcttggcgcagcggatgtgagggcacagaaactttccgataccaaactgacggttaattttgagcaccagaaattaacgactggcattgagaaactgaaagaattaaccggtttatattttgcatataataaagatctttttaaagaaacccgcattgccgccatgtcgttcagggatacgccgctggatgtaatattgaacaggatgctggagaaaacagatttttcttaccaggttgttaataacaatattcttatcagcttagataataataaacggaatcagcgtgcggaaccaggacgtgtatcgggcaaggtaacagatgggaaaaccggtgaagccattccgggtgtaaccatcatcgcttcaggaggctcctcatacggcagtacagatatccagggaaactatgtgctgaaactgcagcccggacaatataagctggagttcaggtacatcggttaccaggcgaaggtgatcacagaggtgatggtaaaagaaaatggaaccacttctttagatattgttttgcaacaaacctcccagcggctgaaagatgtggtaatcaccagctcgtatcgccgggaatcgcaatcagcattgtatgcccttcagaaaagaagtacggccatcaccgatgggatttctgcagagctgatacgcagaacacccgacaggaatgcaggagatgcgattaagcgggtaacaggagtaagtgtgctcgatgggaaatatgcggtggtaaggggacttgcagaccgctacaattatacgctgttaaacggagggctgcttcccagcacggagcccgacaggcgcactttcagcctggacctgattcctgcgctggctgtggaaagcattgtagtaacaaaaacagcgaccgcagatttgcccggtgaatttgccggtggcgtggtacaggtgaacacgaaagattttccggataaggattttattacactgtcgctcggaaccggcttttatgacgggcaaacagggaaagcatttttcaaggaccgcaatggcgcacgtgactggataggctttgatgatggtaaacgcgcggtccccgatgaatttaaaatgaaagccagcgagttggcccagctctatccggaagaaaggttccggatcagcaatgcgctgagcaaaggctgggagccggtaagcagcgggaaagcagagcccatacaacaggtacagattggctatggcaaaacctttaacttcaaaaatgatacgaagtttggcatcgtagcgttggcaaattaccgcaaagaccaaaccatagaccaggtggaacggtatgatcttgcacggtatagtaaatacgagggcactgccggcccgggagacacggtgaagtttatgcggtcctattttaatgaagaagcctaccggtacctggtaaatacgggagctttgttgaacatcacctaccagtttggaaagaacaagataggcattaaaagcatgtttaaccaggactttgaaacagtaaccaccatcaaaaatggcgagaaaacattaggagaaggaattggcgatattgtaaacagcagggtagtggatatgcatcctacacagaaaaccttgctgggtgcgcaactccagggtgagcaccggttagggatagaagcaccggttacatttacctggaatgtttcttataacaaaatcaggaagtatgagcccaaccaggtgcggttaggttatgtaaacctgtaccgcgcagatacggtgagatataaagaccaggattactttgtaccggaatttggttctgttgaaaattcaagtaaactgtattccgatttaaaggaggatgcttacaatatcaattttgcagtatccactccgtttaaggtggcagggcaaccgcagattatcaaagcaggcgcttttacacaattccggaagcgggaatatatcacctataatcttgggtattttgatgccgcccgcggcttaaccaccggcaatgatacacaagggttcccaagtgattctgctgtcaatttcggacagccaatcgataaaatactcagccctgaaaacttcaggcccggcggattggtagcggtaaattatgagttgcctgcaaaccaatacaccggcggggctaacctggcatctgcttttgtaaacgtggagagccagctgctcgacaatcttaaactgatctatggcgcaagggtagagttttatgccatgagcctgagcacgaacaaggagctgaaccgcaaattaccgggaagcggtggaacaggagatgaccaggcgcctatagattatatccgttataatacggatgtattgccctcggcgaccatcatttacagcccggttacttcgatgaacgtacgggcggcctattcaaaaacactgacaaggcccgagttccgggaaataagcccttataactactttgattttgtaagcgggtatatgaccatcggtaacccggagcttaacaggggaaccatacagaatctcgacttccgggtagaatggtttccttccgccgctgaaattatttcggcatctatattcaaaaagaatttgcatgatccggtggaacttaccacgcaggcaacaacatccacaacgaggtttgtacgcacgtacaggaatgtggatgaggcattggtatggggacttgaatttgagctgcgtaaaagcctctattttggaaccggtcctgaatggctccgtaacattatcatctttggtaattattcccggatacattccaaaataatgggagaaaccgcaggctccggattggaggttacacagaaattgcgggagcggccattaatggggcagtcgccttatctgctcaatgcagggttgcttgttaacgcatttaaaaatactttcagcttttcagcagcaattaatcgtaccggccggcgcattgttgttgttggaactaccgctgaagacaggtctgaaatcggggcctatcctgatatatatgaaaaccctcgtaaccagctggatatacaactttcgcaaaagcttttgaaacaacgactggaactcaggttgaacgcagccaatttgctgaacgacaggtacatacaataccaggattttgatttgaacggcaagtattcagggaacacctttgacggaacaactttttcaaggaaatcattcagtaattacacattcacaatttcttacaattttaaaaagtagcacggagaaagaaaacggttttttgatgtgtgcgcgcacaagcaggtaaagccgtaattgatttttgtactgcaaacaacggcaattgctaaacacagttgctggtgggcatgccttgtcttaacccttgtaaaggcgctgatgtccattttatgaaacccactttatcattaaaaatttcaacaaaaatgaaaacgatcagtaaactgttaactatcgcagccctgacggcatcttttgcagcgtgcaaaaaagacggaaacattgaacgtgacgtagtatccggcccagatcccaacgttgacaccattaaaggaaatgttgtaggtactgtaaatttactcgcaaccaaaacttacattttaaaaggcctggtaaccgtaaaaagcggagcgatcctgaatattccagccggaacaaccatcaaaggttatgatgtagctggagaaaaaggcgtactgttagtagccaaaggcggtaaattaaacgcaaacggtacattgaacaacccggttatttttacctctattaaagctactcctaccaacggcgattggggtggtatcattattctcggccaggcgccaaccaataaaccagcgacaactttcatcgaaggtattcctaacacatcagatgcccagtatggtggtacaacgcctgcagataacagcggtactatcacttacacacgtattgagtatgctggtggtgttttccagggtgcactcggaaataacaatgaagtaaatggtctgactttaggcggcgttggttccggtactgtgattaatcacgtacaggtaagctatagcggcgatgattcctttgagttctttggtggtacagtaaaccctacccacctgatctcttatcgtgcaattgatgatgactttgattttgatttcggctacagtggcagattacagttcctggttgctttacgcgatcctgaagttaatgaccagtctaagtctaatggtatcgaatgtgataacgacaataccggcgtagctactaacgtaccacgcacacatccgatcatttctaacttaaccgtactgggtaacaacggtgtggctgattctaaccctgatttccctgtaacttcagccactggtgttgacggatcattccaggctggtgcgcatttccgcagaaataccggcttgtctgtacgtaactccattttcctgggcttcccggctgctggtttactggttgacggaaacgttactgcagattccctgactaacggtgcgtcagaattcaggaagaacttcgttcattccaatacttcaggaaaagcctttgcagttgcttcaggaactacttcctacacagatgcaactttaaagaccttcctgacaaacgctaccaatgcaaatgttgaactggctgctgcgagcggcgctggcctggttaatccgtttaacctgagcagcgttaactccactcagttcttcctcacttccggtgctgctcctgctacaggtgctgatttcaccggtgcattctcaactggattcagttcagttacttaccgtggtgcattccctgtttcaggtggtgcaaactgggcgactgtaagatcaggttctctcggatggacaagattctaagcaattttcagaacatttaatgatggtgagattggcatatcatgccagtctcacctttgtaatataccaccgtcaaaataatataagccaaatgaacagaaactattgcctgccgatgatgctcagtgcctttctatccatttgtttgttgtcatgtaagaaggatgataataagttagaaacccaaaagccagtcgtggccctgccggaaaaaatcgacgcaaaccgcaccctgaaaagcgataccatttacacctttgcggtatccgtgaatgtaacaaacaatgccgtgctcactattgagccgggcaccgttattaaaagcaggagcgtagcagctggcgccggaagatccggttatattgctatagaaagaggttcgaaaattatggccgaaggcactgcggagaagccgatcgtatttacttccggcacaccttccgggttccagcaacacggtgattggggtggactgtatatttttggcaaagcgcctgtcagcgcttatgatgaaaataccggcggggccggtacagaaatgaccctgaccgggttaggcgcgcttttaccttccggcggcggaaatgatcccagggataattccggtgtgctcaggtatgtgcgtatcgaatttgcaggagtgggatctgccgaatcatacggactggcctgtgttggcgtagggtcaggcaccaccattgaaaatgtgcaaaccagctatacacaaacttcagggtttggcttcttcggtggaaccgtgaatgcaaagaacctggtggcatttaataaccggctggctggatttgtttattcaaatggctataccggcatgcagcagtttatagtgagctataaacatccttattttgctgcccccggaccttttatcagcacctgcgatgcattattggtactgaacgataccaaggggtacccggtagcgccggatacacgcccggtattgtcaaacgttaccgctgttggcccgtataacaatcctggttacaatagcgctttaccctggaacgccgccttaaatgtaagttatagcggggcgtttgttttgagaaattctattttgatgggaatgccaaaaggcgggattaaattcagcgacgatatcgccgcacaacggttaatagacggcacctccgaattttccaccaacctggtgcatagtaatatttccgcagatgcttttaccgtagatcccggggctgtttattcaatagatgcagccggtgttacggattacgcggtaaatcatcataacaaaatgtacgttaaaccggaagaaatcggccttaccaaccctttcaaatttgcgctgccagaactattgcccaccaccggtgcggcagctttaacgggcgccgatttcagcggggagcctttccagggattctttaaaaaggtaacttatgtaggcgctttcggaactgaaaactggatgcaaaactggacagatttttatccttttaccattaaatattaaggcaatcaacagctgtttgaacataccgggtcgtaaaatgggcttttgtttttgccttttcatgatattatggtgccatcgcagcccggcgcagcagatggtatcaatgggcgtgtttttatccaggcaaacggtgaaagacgccgggatgtctgcccttgtttaccagggaacatatcccggtatggccgccagtttttcgcataccggccgggtaacacaggaagtgggcgcccgtggggcatgggggaaattatatgccaacaaaggatctggcgccatgcgatcaaaagttttcgggttagattacaatattttatttacgctgggaaagacagacagaacccggtttgaatttggcgctgccctggataattatctccatctgagggaacagctgcattacgtaaacaatcgtgattactatgagtttatcagttccattggccccactgcccggtacagctatgtattttcatggcgtgataaacaggccggcaaaaactgggaactaagcacccgcatcttttgcccggtggctgctgcgctttccacagcgtactcggcatacgaaggacaaaccggtttgcatacgccctcattgcggaccattacccgggatattaagctgacaagctggaacaagcttaaccggttttactggaacaccggcataaaggtgaagatgtgtaaaagcaggggcctgtctttgcactatcaatgggagtactaccggattaaagaggtgagcggggtacaatcagctatgcatagtttaaccatcaactacatttttttattatgaggaatgttgtcagcatatgcatggtgatgatgctatttatcgtttcctgtgaaaaggcgattataaaagaagacaagcaaaaccctgttgctgtttttgaaagcctctggcatgcgatggataccaggtatgcactgttcagctataagaaagtggattggaaagaagcctaccggaaataccggccgatggtatctgacaaaaccagcaccggggaattgtttgatatttgcacagctatgcttgatcagctgatggatggccatgtggcccttatcaacggggagcagaagcacacttacaccggttattacaattcatatccccacaattttaatttcggcctgttaaaggaaaagtacctgccgggaattaactaccagggtacattggcgtatactttcatagaacagtttggatatctgcacattccgtcctttggggaggaattgacattagcggatatcgaccgggtgtttgagaaattggcagatgtagaagggctgatcattgatgtgagggataatgggggcggcggttctttaaaagtagacaggatcgtggagaagttgctgccggaaaagatgttgctgaagtatgatatttataagcgcggaccgggccatgatgacttccttccgccggaggccaaatacctggcgcccaggcatcctgttttggcaggcaagccattgttgatattgacaaacaggagatgtttcagttcgtgcaatgattttgtgctgtatatgtcggaattaccaaacgctgttataatcggagatcaaacaggcggtggaagcggtaccccgtttgattatgagctgcccaatggctgggtgctgaaatacgctgcttctatggctgtttctgttgaaggaacgaatatagaaggagggattgccccggatcattttgtatccaatagtttggatgatgaaagtaacgggagggatgccatttttaaatttgcattggaacacctgcaatagtttatcttaaatattagaaatgccttcttatattacaagttgaaaattattgtttatcccaaaaaagggtgtttaccggaatctatgttgatcatcttattgcgtataaccagctatggctgggcggccatagcgattgtagtattgtctgtactgttagcggttaaaatattaaaacgaaacaacccgggcggcaaacctggctgcatggggataggttatgtttcgctggtggtattttgcctgcttagtctctctgccacgcttgcgggtgtattgggcgactttgtggtgaatgcgtttaccctgccgcggtataaagcgaaggtggtcagtttttcctcttatgtatcgaaggacagtaaaaataaaaacactatcatgtatcgctccacggtagccttcacaacgaaagacggcacaccggtggaaatggaaaccgatgtatcctcctccggcaaaccggatatcggcgaggtgattaccgtgggctatgaacccggtatgtctgccgccggcgagttctccacaagtaaatacctgttaatgagtggagcggctgttatgttactggtaatgggatattttgcaataggaggtattttatatgcaatgggctggcggatggcctctttctttaattccgggatgatcctgctgctgtatttcatcatacctttggccatgctgtttatgttaggcggcatgggatacgcggtagtgcagtatttcatgggactccggcccgatatgccggtatgggcggtggtagtatgtacttttttctgcctggtgttatctgccgggatgctggggtatttccggatgcttacggacaggcgggcacgcacccgttaaatttttgtgggggctgccccgaattgcttcttgaaagcaaatgaaaaatgcgagaggtcctcgaagccaaggtccaggtaaatatcggaaggcgttttacctttttctttaataagataataggcttcctgtaatctccgctgctgcagccagcggctgggggttgaatgaaacagcttttcgaaatcgcgcttgaaagtagccaggctcctgccggtcaggtaagcaaaccggttaaggtccacgttaaaatgaaaattcttattcataaaagcttcgagatctattttccccggctcactgaaatcgaataatatatctttcatgccgggatttacttttaacaacagcagcactgcttctcttaatttcaacgtaaccagcgcggcatcatcttccccgttcagttgcatgtagggcggcagtgaattaaaatagtttttatacaaaggatggggttccagggcaatgacagcgttgcctttcacctgcttttcggctttataccccgcttccatactaaactcacgcaggaagggctgatcgaagtgaacggaaaacgatttaaactcgccgccttcgggcggtagcttgttgaacttcatcagccggttccgcctgccgagtctgacatcaccgggtttaaaaatatatgctttgttgccatcattcatgatcattgttcccgacacctggtagctgaatacatagtccggtataaactgttctccctcccgggtactggtggtgtagcaggaatacgcgataggggatggtcgtttattgagtgaaggcattattcaattgtattaatccgtttgtgtaaaattcgctgcatctgtagagacgcttaccggcagccacttttccatttcctcatttctttccgcattggcttcccttatccggtatatggcatcgcttccaagtaccaggtgtaccgggggcgcaggatgcttaaccaggttaatgattgcttctgcggctttgtcaggcgtgcctgcggggctaaagttactatttttaaacagtgttatccgggtgcccactgtcttttcatagcccgctatctcctgcgcgcagggcaaagaggccgtcatgccggtgcggaaaccgcccggttcaatacttgtcaccagtatgcccaatggtcttacctctttagccagggcttcgctgaaaccgctcaatccaaacttcgcggcctggtaaatggtgaggccggggctgcccaccctgccgcctacggagctgatttgcagtatcctgcccgaaccttgccggcgcatatatggcaacactgcacgggtgatggcgataggtgcatacaggttcgtttccagctggctgagtacctgctcatcgctgtaggcctcagcggcgcctaagatgccggcgcctgcgttattgaccagcacatctatccggccaaaatgttgaatggtattttcaatggcggcgatgatctgtgcgttgttggtaacgtccagctgcagcggatatatattgccgggatactttgttgcaagatcttttaacaggccgggacgccgggcggtggctgctaccaggtcgccacccgccagtacagctgctgtaagactccttcccaatccgcgggagctgcctgtaataaaccaaacgctggacataattttagttttatcaaaggtcggattaaccgggtaagaccggtttgctgaaacgtgcaaactgctttgttaaaaagttcagattaataaatacagacgctcctgttgatggccgggattacatccccgaaaaaaattttcctcctgcttcaccctttttcacttttctgttgcctatgatgatagtggtgatttaaatgaggcagccggccgttggttatctgcaaaaaacagcaacagcataatgcgggacaacagatgatggaaataaatccggattttattatactttgtgcggataacaatgaagttacaaagtggtttatgtaccaaccaaaatcaggtgaagtagtttctttcgaagaacagttcaaacttcactacaccttcctgtgcactgccgcgtactatgtggtggaagatgaggacgcggccagggatattgtgcaggattttttcctttattgctggagtaagcggcatgtcatccgtattacccacgattttaagagttatgccgttcgcgccatccgcaacgcttcactgaactatttaaagaaatcaggcaaaacgtcgctggaggaaatagccgtcattgaaaacatgacgcagcattttccgctggaagacaatgaagcggaagcagaccgcaatgcagcgctgtgggcggctgtagcccggctgccggagcagcgccgccggatattcctgctaagcaaccgggatggactgaaatataaggatatcgccgaaacgctcggtatctccattaatacggtgaaaacgcagataaaactggcactgcagtttttacggaaagaatgccggtggatgaatattttcatcgctttcctttttttcttaaaaaataactgacaggccttcacccttttttcataattgtttgcccttattaccgaagttatgaatgaaaaagataaagaaatagactgggataagctgctggacctgatggatgggaacagaacgggggaatccctgacggaggaagagctggcaatgctggctgcagccaaagagatgcagtcgagactgggcgcggaaaaattcccggaagaagagggatggcagagttttgtacaggccagggaccgcaggcaggcccgccgtttcacactggtgaagctggccgctgcagcaatattggtattggccataggggcagcattatggacattcctgcccaggcagcacacgccgcagctggccaacgaaatgcccgtgggcaaggtgcgcctcaagttatccaacggtcatgaaataacgcttggcggcgacacacaggtcattcaaaacaacggcatcgccgctatcaaagcaggtcagtcgtcattggtatacgatgccggcgccgatcgtgcagtagtaacggcgatggatacactggaagtgccccgcggcttacaattcaccctccggctggccgacagcaccagggtatggctcaacgccggttcccggctgatctatcctgctgcctttaacggcccgtcacgggaagtgtatgtgcagggagaagcctacttcgatgtggccgccgatatagaacgcccattcctggtacatacaggcaaaatgaccatgaaagtactgggtactgcctttaacgtaaacacctacggaccgggtatacaaaccactttaagcagcggaaagctgctggtcaccgccggccaggagcataccatactggcgcccgatgagcaggccgtttataatgataaaaatggttcgctgcaaaaaaggaccgtagaagcaagggtgttcaccgcctggatggaaggcgatctcttttttgaagatgccacgctgctggatattaccggctacctggcccggaattatgattacgtttttgtttttgaagatccaacgctcgagaaaataagttttactttagatatgcgccgcccggcggttttacaggatgtactgaaccagatcagccatagcatgggtaatttaaggttccgggtggaaggcaaaacagtgcacatcatgaaacgtcaatagttaagaatatcaaccggagtcaatcagattgccagtagccaccggttactgcttaaaccataataccaaaccagaatgagaaatttattgggcttgtccttcgcctggaaggaagcgcggcgctatgtcatgcggttaccttaccagttgttgcttttgctgcttcttaccggcaatggggcgttggcgcaggatagtatacaacaggaaatattatcgagaaagatttcttacgaggccaataaatcatctttaagcaaagtgctgaaggatctgcgtacgaagatgcatatacgctttacctataacagtgagctaatccggcgtcagccaccggttacggtgaaagtaaatgcggtttcactggaatcgttactcaaaaaactgttgcttaataccggcctgcaatttatggtggagatgggcgggatcattatctacgaacaggaggtgtctgcagaaaaggcaaccagccagtcggtgatcctcaggggaagggtaaccgacccccagggctcgcctttggcaggggtgagcattaaaggacttacctcaaaagaaatgaccgtaacacagcccgacgggatgtttatgctggttgcccgggagcaggaacaggtaagcctctccctggtaggaatgaaaacgctgctgtacaaagtgaagttttcagacgacccgttgatcccttttaaaatggataccattgcccgggaaatccaggaagttgtggtgaacgggtatcagaaaatagatccccgtttagccacgggctccgtattaaaactgaatgcagccgatatcttacagcccggtcagccatctgtagacaggatgctgcagggcaaagtgccgggactaatgataatcaacacctccggtggcgtgaatgcaaagcctactatgcgtatccgcggtacctccaccttaattggcaacgctgccccgctgtgggtgatcgacggtatgatacgccccgacccggttaatatctcctccgcactattgaataatgtactcagcggtccttcccaatccaactatgaactgatgggaaacgccatcagtggtttgaacccctatgatattgaaagcatcacatttttaagagatgccgccgctacttctatttatggtacccgcgcggctaacggcgtaatcgtggtaaccactaaaagaggaaaggcgggtcccgtggaagtaacctacaattcaaatatatctttccaggcgcgtccttcctacaaccagctgaacctcatgaattcgaaggaacgggtggctttctcaaaatcactgatagaagatggcgtggtctttaacggaagtgaaagtggtttcgaagaacgtttttcgtatgaaggattattaagacagttatatgccaggcaaattacggaagcggaattccgggcgggggtaggcactattgaaacccggaatacggattggtttaaggtgttgttcaggaaccagatgagcatgcagcatgcgctcagcatgagtggcggcgcgggtaaaaccacctattacgcttccctgagctatggcggctttaacggcgcagcgaaagaggatggcaagaaaacgtattcagcgaatgtaagtgtgcgcacgcagattggtaaacggttgaacctggacctgtcgatgcaaagcaattatataaaatccacggggtattaccagtcggtaaacccgttgacctacgcgttgcaaacaagccgtatttacagcccggacgatttttacccggtgcgcacgccgagcaacctgagggttaatgagcccgtacagttagtatggccaccgtatgtttataacatacaaaatgaaatcagtcactcggaaaacaacagcagcacacattcttccagcctgaatttatcgttggattataagatcaggaagggattgttttttcgccattcttccaacgttattgtgagtggagccgatgggttaaccgcagccgatgagcaaacatatgctattgcggttgaacgcggatggagcgcggaggtggtgcctacacaggagatgatgctgacggcgctgcccacaggaggcatggcctatatgatgaaccagaagagcatgtcgctcggaatgcggaacagtatagattacaatacaggcgtacggaaggatcgcgaccagtttaattttacgttgggtaacgaggtgagaagtgaaactgccaatggccttacatccagggaaccggggtactttccgggcaggggaaagtcattctttccgactgtaatgggcaggaaattatatagttcagaaacaatcaacgaagctatcgacaactccgtttcctattacagtacggccgcttatagcatgatgaaccgctatgtattgagcggtaccatccggacggatggctccaacaggtttggacagtattccaactccaggttcttacctaattacagtattgctgcccgctggaatgcttcttcagaaaactggtttcccgtaagctccctgatcagcgactggcaggtgagaggttcgtatggcacgcagggaaatgtggtgagcgcagtgggtcctaacctggtagccacttattcccccgttgtgggagaaacaagtcccattaccggtaaaccttacctgcacataaaaaccatgccttacccggagttgcgctgggaaaaaacccaccagtggaacctgggcacccaggtagccatgttcaatagccgcctgcgggtgaatgttgattattactcgaagaaaacaacggatgtactggacatgataaagattccttttgaatatggtatggatgtgatgtacaggaacggaagcgagttatataaccagggatgggaagcgatgatcaatgtagatgccatcagatcgcggaacacatcgctctcctttacgttgactaccagcaggaacagcaaccgggtatctgacgaaattattcccaacgactacaattccttttttaatggcagcggacatttacgcggaaaacccgtgagtggtttctactcttatatttataatggtctgaatcataacagcggtttgccgatgttcaggaatttagatctcaaggaaaagaccaataacccggatgatttcctggtgtattccggccaacttcaaccttctttcaccgggagtattcagccggtgttccggtacaaatccttttcagcggtgatgttgttttacgtgagtattggcagcagcaaacggctcaatgatcctttcccgcgtacaaatgcactgaatggggtgccggcgccatttaccaatctcagcaaagattatttgaaccgctggcgtaaaccgggtgacgaattacatacagatattcctgtagtgatggatcttttagccacccgggactggcttatagtaccatacaaagtgatcagtaacggttccgctggaaactccggacaaacatcggtggatccgttccaggcttataatatgtctgatctgaggacagtcagtaacaactatgtgcgatgcagcaatctaaatcttacctacaccattcctgctgttaagctgaggggaagcgggattaagaatttaagcgttggcgcggcagtaaataatgtttttacggttgccaataggaaactgaaagggcaggaccctgaaattgatggcatcggcaccactgcattgccgcttacccggcaatatgctttcagtctgaacgctactttttaatgtaactaatttcaataatacagcatgaagaaatcgttgcttgtaatcataggcgccttgtgtttagtgtcctgtaagaaattcctgcaggaatattctccaacagatgtaatacctaaatctacccatgatttcggggaaatattatattatgatggatatcctaccgcttccacattgctgcagccctggatggtattcctggatgacgacacccagggctatacaggaccactcatggcccactcaaatgcgccactcctgccggcgcccatctttcagtggcaaccagacatggagcccgccactgccgctaccggtaatgccatcaatttcaatacctggagtacctattacaagttgctgctgggcgtaaatgtagcgcttcagtatatggataattcaaccggcctgcaggccgacaaagaccagtttaaaggagaagcctatacattacgggcattctatcactttatgctggtgaatatttatgcaaaaccctataatgattccctcactatacccgataaaagcccgggtgtgcccatcaggaaaaccgccgacctctcggatgcttttctccgcaggaacaccgtgaaagaggtatacaaccagatcgtgagtgatctcgacagcggtatctatttgctggataaatacaaagttaaccgtgaatactaccgggtttcccatgtagctgcgcatctgctggccagcagggttttcctttatatggaagactgggacaaagcgatcagtcatgccgacgaagtgctgcgttatcacccgcagttaatggacctgaacacctggggagggatgccggatacagaaaataaaatgctgataggaccgtctaatattgaaagtatctggaactatggacagggagaggagcagttaccaaacacttattcagaggcatatgatatttcgtacgacctggtgaactgttttgaagagaatgacctgcgcaggcaaacaggattttacatcaatccggaatttatgaaagaattcctgacgcccgatttttcacagatgaagaatgtgccatccgtttcggggcattctgccgaattaaccaattcgtggagaagttccgaagcttacctgaaccgtgcagaagcctacatccagaaatacaggaaaacaggcgatggtaacgccgccgcacaggcactggtaagcctgaataccttgcgcgccaatagaattgaccgggcttctttcaccccctggatcgtaaaaccgggagatgtattgctgcaaatgtgcagaacagaacgtcgccgggaactataccgcgaagaagcacatcgctggtttgacctgagacgctacggcatgccatcgatcaaacacatctttacacccaaccaggtaacggtgcaggtgttccggttgccggcacgcgacccgcagtatataatgccgatacccaccgatgtactatcaaggaacccggcactgacacaaaatcccttattcgcaggtaagcgtttaccggaataatttctttcaactgtaaataatcatatatgagattatatttcctgatagtgctgttagtgggaatagcctgtaataaagaggcggcattaacaccggatcctgtccagcccttatatacgctcccacagggtaatcatgagtatgatgatacgatagtggcctggtataaaaaatacaacacttttgtcctgtataaatttacacagctggattatgcttataactactccgataagaaaacagatagtgcctttaatgctaatcccgcttatgtagcatccacattacagtatataagagaagaattactggacgtatacccggaggcttttttaaagaccacgctcccttacaaaattttacttgcctcctatatcggcgcagggaatacccgttcagcaaccggattttctgccaccagcagtatgctggctattggctgggccgatagtacgctgtggcaaaaaacaccggcagaacgcaagcagatgcgtggctggctgcaccgaagctatatggaacgcgttgttcggacagacggcactattgttcctgatgcattcaaagccctggcgccgccttcctacggacaggtaccgcctgccaggctcctggcagaaggcatcgtggagccatacaacaaccagctgaatgtggccactgatttcctggcatttattcaattgattaccagtcataccaaagatgaactggaagcgggcgtactgcgcagccaggtggatgaaaagggattgataagaaagaaatacgatgttgttgtcagcacatttctcaacagataccaggtagatctccaggcgatcggcaacaggccataacctgtacggagccgttaatattcttcgcattaatattttttgtatgaaaacattgaaaggagcgcaactcctgctatcaggcgtgttggccattgccggctttacggttaaagcccaaacgcccgctgctaacgctacgcagccgtcgtaccacagcgccgttatcactgctgctatcaataaggtcacgaaaaaacattaccatccaaggccaattgacgacgcctactccgcggcagtatggaaccggttcctgcacaccctggaccctaacagtaacctgttcctccaggaagatgtggctgcccttgcggtgtataaaacgcaggtcgacgatcagctgaacacaggcgctaccactttttttgatgccgcctacgcgatatatgagaaacgcgctaatgaagccagccagctttgccagcagatcctggctacccccttcgatctgaaaaagaaagaaacagtaatggccttcaggaaagatcttcccttttgcaccagtaaacaaacgcgcgaagaactgtggcgcaagctcttgaaatattacaccctgcggcattatatggagatgagcgccgccagtggcgacaccgccaaacacctcgcagctgccgacccggcactggaagccaaagcccgggaaaaagtacgcaaatggtacagcgattatttccgtcagacgaccgggcaacgcggagcggaagacaaatttgcgcagtatgtaagtgccgccatgtttgaaattgatccgcatactacctatgcggcaccacaggaccggttcatgaatgaacagctgaataaacgttacttcggactaggcatagagctgggcgtaaaagaatccgattactatatcaaaagattattgccaggtggtaccgcttaccgcagcgggcaggtaaaagagaacgacaatatcatcgccgttgccgacagcaaaggagagatgctgccggtgaacgggcttcccgccaacgaagtagccggcttgatccgcggtgaaaagggaacctccgttaccatgcgcttgcaacagccaggtgaaaaagaaagaacggtgaccgtaaaaagagatgaagtaattgacctggaaaacagggcgaaaagcgccgtgattgaaaagaatggaaaacgttttggatatatcttcctgcccctcttttacatggatccttccggtaccaaaataaacggctctgccaacgatgtagccagggaagtagaaaagctcaaggaacaggaagtagatggcattgtagtggatctgcgcggcaatggcggtggctccctcgatgaagttgtcaccatgggctattgctttgtgccctccggacctattacctggctccgcggaaaagacagtatccggatgtattcctctccggcagtggaaccattgtatgatgggccgctcaccgtattggtagatgaaggcagcgcctctgcgtctgaaatatttgccgccgctatgcaggatcgtggccgcgggcttattgtaggcacttcctcttcttttggaaaaggcactgcccaggtgaatatcaccatcggtaaaatgggtgatgctgcgaaaggcattgccgatgtaaactatggcaccatgcgggttaccacggagaagttttaccgcattaacggatcatccacacagctgcagggcgtaatccctgatgttgtactgcaggatagaatgagttcgcaatccgtaatggaaaaagatttttcgtctgccctcgtatgcgataccgtcggactgcctccttatcagcggcttacctttgggtttgattatcagaaagtagtgcagcaggcacgcttgcgggttcagcagcatccttcctttgccactatcgcagccaacacccgccagttaaaagcattgcaggagcaacccacaccgctggaactgttgtcgtttggagcagtttataagcaaacatccggatgtgagaagaatatacaacaggcgaaagaattgaaaggcagggaagtactgaccgtattgccatcgatgctgaggaacatcaatccggccatgcaaaagaatgaggccgttaatactgcttcttacaaagaatggctggagaaactggggaaagatgtttacctcgctgaaacagtatcggtgctggaagatatgctgactaacccggcctcgccgaaaaaatgataattaattaacaacaggcttcacccgttttgcggtaatgattgcctaatacttaaacgcacttaatcatgatgagaaaactgtttgcattcactttttgcatgggaagctttgctgcgtatgcgcaggaggatgtggccatcattacggccaaactggataaatccccgaatgataccttagtgaacctgtacgagccctattccggtgataccgccaccgccgtcattaagaatcaccagttcaggctaacgatgccgatagccaaaggaggaagcgtatatattatgcagataggcagtaatccggaactgggaggcgcattggtgtacctggagaaagggaaaatgaacatcaaaggaaaaggcggatattttaacgacgccactttttccggcgattcctgggtaaaggaatggcaggaagtaatggaaatgacttccccggagaaaggcgatggtaagctgtttgcggagctggagcaaaaataccataaagcgatggaaataggagatgaggatgcagcggaagcctacaataaacagggctccgaagtggagcagcggatgaaggatacactccggaagtggatattggcccatccgaattcgggcgttaccggttatattatcacggtatattttagtaagaatacgaaagaaatggaggcgctttatgatggtcttggtgaacatgcaaaagcttccaggatactgcaacgctggaaaaatccaggtaaagtagatccatctcccctctctttaaagatgaatgaagaaggagaagtacccggtaaacctggccaggtgaagatcggcgacgctgcgccggctttcagtatccctgatgtaaacggcaaagtggtgtcgctgggagattttaaaggtaagtatgtactggtggatttctgggccagctggtgtggtccctgcaaaccacagatcccttacctgaaagcggcgaatgacaaattcaaagataagaacttcgtaatggtgggcatctcactggattccaaaaaagaagcctgggtaaaagccatggaaaaacatgaactgaactggctcaatctctccagtctcaaaggttggggcgacaccgccgcagcggcttatggcgccggctacattccttccaacgtattgatcggaccagatgggaaaattattgccagggatctctatggcgaggcattggataaaaaattaatggaaacaatcaaataggttgtttgcggtaatacctcagcataacttccgccagggcaacggcacactaccgctgtgctgttgcccttttttgtttacataaaaaagatatcaactttatgcgtcctgtcattaaaataatcatcttcctgctgctgcctttatacagcctggcagaagaagggtttgtaatcaaaggaaaagtaacgggcatcatcagcggatacgtggccattcttgaacatgtggatgaagccgggaagccggcagtgctgccaccaagggttcgtatcatcaacggagagtttactttttccggtaagctggatcaccccgaattgatacagcttaaagtgagcacaaaaacagtgcagctgttcctggaaaacactacctatacagttgaatccagcctcgactcactgaccggcagttcttttaaaggcggccggatgaacgaccagttttatgcgtatcagcagcatagtaagccacaaatggaatatgtgaaagataaccccgaactggaactctcggcctggcttgccctgagaaacgcatccacagctgataaagcggagcaagggtatgcgctcctggctcccgccggcagaagcacctggcatggaaaagcattgctggcaaagattgaatcatttaaacgtaccggcgccggcgcagcattgccggaattaaaactgacggatcctgatggtcatgcgttttccatcaaagacatggcaggaaaagtagtggtactcgatttctgggcatcctggtgtgctccctgccgtgcttacattccgcagatgcgcaatcattataacaagtttaaggagaagggagtcgtatttgttgcagtgtctgttgacgacgacaaagccaaatggctgaccgctgtgaacgaaactaaaatggagtggctgcaggggcttacagaaggcggctttaaagcaggtataggtgtgcaacagaattttaatatcacctccataccacatgtggtgatagtgggaaaagacggaaagattgcccaatcactggacttttataaaaaagaccagctggaaaaagaattggataaactggtgcaataacaagaatatgatcatcaaaaaattaccactgttgctggcaattgctgccgcgatatttttctccgggtgtacagcatttaaaacacctgaaccacggcttccgaaaaaactggctgtcagggttttcaatatcacgccgcaacaggcggcattgaaaatagaagggatctactataatcctaacagtttcggattcacgtttaaaggcggcgacctggacctgatgctggatactttcctgttggggcatgtgcacatcgataccctgataaatgtgccggcaaatgcgttgttcaccatccccgtaacagtgaaaccggattttaataaactgggtcaaacgggcattaacctggaggactctgtgcatatttccttcaagggtaccatgaaaggcggtgtgggctggttctccaaaacaatcagcattgcgtatgatggccggcattacctggacctgatcatgaactgatgctatctaaggcgtttcagcttcgcagcaattactgataaaagccggcttttttttgcaacctccgtaaaacggacacgcatgttcaatgcgtagccatggaataacttcatttcatcgatttttatccattaaaatgttaattatgaagtttaattccatggttgatttgcgggcagatgtaactgcacttaatccaaatgatctgatccatctacttggctattattcacccggagatggtggtggtggcgatttttactgggatgccaccagcacagatactgataacggcggatcggttattaagagaacagccatagcggttggccggtttaaagccatcctgaatgatgttattaatgtaaagcgttttggcgcaaaaggcgttggcgggaccgacgacgatacccaggcaatagccaatgcgttggcagcatgtgttgccacgggtatacatgtattgtatttgccccagggcgagtatgcaaccacgcaggatattgcgcttacgcaggaccatcagatcattaagggagagtcgcgtgatggctctgtgattatattgaacaatggagctaaagtaacgaccaacaatacccaatacgcacagctgtttaactttacgattaaagcaccgggaggtaccggttgtgtgaacggcttgttactgaatagttcacccaatacgctggtggaagatgtttatgtaagcggatattatacagagtgtggtatccgcgttggcgaagcatgttatagcacgaggttcgtccgctgttggacgaaccaaatacaaacaggtgatggctggtggttccgcaatgaaggaaataacagcattcagctgcaaagttgttatatcctgaatacaaaagccggatgtggtatttccatctcccaggctaataacatggtgatcgacgcgccgcaattagaggcgaataaagaaggtcatatccagttctacgcggcggaaggagtgcccggtgcaataagaagcctggttataaatgatctttattcagaacagtcttgtacgcctaataaacccacctttactattaaacacgtaagtggtgtgatgaacatccgtgggttatacgtcaatggcggctatgtcaatggattcacaatgccctattttgcggactttaccggcatcattagcgggtccggaacggcaggcgtctcctgtcacaacgtgaatatccagaacataacagcagcgggatataatatagatacctccgtaaggggatatattaccggtccggctccactgaacgatctcacggaatgctgcccattggtggttacgctgccaggtaatgccgcaagtgtatctgtagtcaggaacaggagcatcggcatcgcggaacctatgcagccgttattattgggcccatacaatcctaccctggcacaagccggaggattatggtatgatgccatacaggataacctgcgttttaaagataccaaaggtgaatatattctgggagcacgtagcctgtatataccacccgttatcggcacaattcccgatctctcaaagataaaacaggactattttattccattgaacgctgtcaatgcggccattactattcctttaccggcggcttccactgttcctgcgggcctgacaatcaccatcaagaaaattgatgccagtgcgaatcctgttaccatcacctccaccagtttgatggacggcgcgggctccagaacactcaccgcgcagtatgaagcaatcacggtaatgtctgatggcagttcaatataccgggtggtttccggcgtgaatgccaatacgaatgtattcaataatacctctgtggctaaaacagccattaccaatacctttctcaatactaattacccggccgctgcatatcccgccggatctttggtaatatttaccaacctgtctgacgcggtcaccaacaccgccgaatgtagaagacttactcctactacatggtcaataaatgcaacagccggtaagctgtagcaagtctgcataaaggagaatgcctgttcaaggcagcctcctttatgcagaaccttgttcatgccgttgcccgcttatattttcgcagcagatttgcagttccagaatggaatgtatattttaacgctatgctaaaagcttcggacacaatgattgacctttcctttaatcgcagaacagccttaaaagcgctcagcttatcagccggcgctgcattgctgaaattaccggcatcagcaaaggggcctgttgaaaagccttcgcctgcttttaagtattcactgaacatgagtaccatccgggggcagaaattaggttttgttaaagaactggaaacggcgtccaaagcagggtttagctcggtggagatatggatagatacttttcaggggtatttgcagcaagggggctcggtaacggaagccagaaggatcattcatgatttaggcattgaagtggagaatgcgattggatttgccaaatggattgtggatgatgaagccacccgcaaagcggggctggaacagctgcagcgcgaaatggagcagctggcgcaaattggctgtaagcggatagcggcgccgccaatgggcgctaacggcagcaatgccccgttaattgacctgaacgtggtaacggaaagatatcttactatccttgaaatgggcaagaacaccggtgtaatgcccatccttgaaatgtggggcggatctcccaatctaaaaaaaataagccaggtgctgtatgtgatcacagaaagcggccataaagatgcccgcgtgctgatggatacctttcatattttcaaaggtggttcaaaccccgacagcatggcgtttgtaggtaaggatgccgtggatattttccatataaacgactacccggcggggatcacgccaggtaaaatttctgagccggatcgtatttacccgggagatggcattgcaccgctgaagcagatgctgcaacatattaagcaccccgggaaaccggtgattatttcactggaggtttttaacaacaattattatcagcaggatgctttactggtagcgaaaaccggcctggcgaaaatgaaagcggcgacggaggggatataaggaaatcttaactggattcccgcacaatcagttccgttttcaacaccctgataatactcttccattccgatacatcacggctgatctggtctatgagcagctgtgcggcagtgccgccaatttcctttaccggctgcgacaccgtggttaaagaaggatgaataagccccgatgcaaagtcgttactgaatcccaccaccgcaatatcttccggcacccgcaaacctcttttcttcaccacctgtataatctcaatggcagtaggatcgctgatcgcaaaaatcgcatccggcggatgaggaaggtttaaaagatgattcacataaatatgcaccttatcgaggttcaggtcatacggaattaccaggtcatcatccagctcaatattgttttttcttaaagcagccttatagccgttcagtcttttttcacttattttgagagaaggtgggccggataaatgtgcaatccttctcctgcctctttcaatcaaatgattcaccgcacggaatgcgccgtcatagtcgtcaacaattactttgggcacatccatttcatcgcatacccggttgaaaaatacgatgggaatccccttgcgctggaatatctttaaatgatcaaagttctttgtttctttagtgatcgataccaatacaccatctacctggttggccagcatcactttggtgttggctacttccgtttcataagtttcgttggattgacaaatgacggtattatagccggccttgctggccacttcctgcgcgccgatggtaatatttgggaaataagaactggtaaattccggaacgatgatcccgatagtatttgttttccgggtaaccaggctgatcgccagcatgttacgctggtagtcgagtttttccgccaggtccagcaccgcctgccttgttactgcgttcacgctggggtgccctgttaaagcccgcgatacggttgatttagaaagattaagctccttcgcaatgtcaacaatggtgatctggtgtcgcttcatcaggtttttttcttgtaaagaaacataattatatcaaaaatgggaacattcccaatttatgggaatgttcccaatggcaaaatcatcattttttttaccatcgggtaacagttagttataatctttggacacataaattctcacgatatgaaagaactgttgctctcaacctcttttgcaccaaccgtgcctgtacctgtcgccttatgccaatcatccgcattacacctgttacacgattacatggagtaacttcctgcgcccggtaattgaaccggcactcgataaaataaaaatgaattaaacagattttaatctaaaaaacacgtttgggggtatgcataaaaatggtttcttatcagcagggtatttattgcccctgctatttatcatcttccctgctacggatgtagcagcacagcagcctgccacggggtctgctgataaaatatcagttaccggaaaagtaacagaagccgcaggcaccggcctggtaggggtaacggtccgcgtgaaaaatgacaaaacctccgccatcactaatgaagacgggatctatcacatctccgccaataacgcacccggcgccacactcgtattcagctatgtaggatttctgagcagggaagtaaaactaaccagtggaagaagcgtatataacatcgtgctggaaccttccataaagggtttgaacgatgtggtagtaatcggttatggaactgtaaaaagaaaagatgtcaccggatcagtaggcgaatttaaaatagccgacctggcaaaagcaccggtaccttccttcgaagaagccctgggtggccgcgtggcaggtgtacaggtatctgccagcgatggtcagcccggatccgctttgaacatcgttatccgcggcaacaactccgtaacccaggaaaactccccattgtacgtggtagacggattcccgatggaaaatccgtccaacaacattttcaatcctgaagaaatagcctccatcgaagtactgaaggatgcctcggcaacagccatttatggcgccaggggcgccaacggcgttatccttatcaccaccaaaaaagggaaggccggcgcgccaaccgttacctatcaaacctggatgggcttacaggaaaatattaagaaacaggagatgatgagcccctacgaatttgtgaaataccaactggaacaaaattcagctttttacacgcccatctatctcggcgaagataaaacactcgacgactataagaacgtaaaaggaatcgactggcaggatcaaatcttcagaaaagcatttatgcaaaatcacagcctctccctgagaggtggtaacgataaaacaacctactccctttccggctcgctgctggaccagaacggtatcatcattaatagcggctttaaacggtaccagggaagggcagtggtggatcagcggctgaatgataaagtgaaagccggcatcaacgttaactatacagctaccaaaacatatggcgctgtagcttcgccaacacccaatggtccaacctccagcctgatgtacagcgtttggggctaccggccggtaaccggcgactccgccagcgacgcctctctcatcgatcagccctttgatccggatgtggacccgctgaatgaataccgcatgaacccgatcatttctaccaggaatgaatataacccgctgttcaataatacccttatcaccaacgcgtatgtggaataccaacctgcaaaatattttacattaagagtggccggtggtattaccaaagaagcacaacggaaagaaatattcaataattccaatacccgcctcggaaatcccaagagcagtgtactgggcatcaatggctcggtaagcaatctggaaagaaccaactggctcaatgaaaacacactcacctacgccagggtgatcaacaaagatcataacctgaatgtattgggtggtttcaccatgcagaagtcagccttttatagttatggtttctccgccagccaggtgccaaacgaatcgctgggtatgagcggcctggacgaagggactatcaataccgcgcccacggcaaaatcatctaatgcgttgatgtctttccttggccgtgttaactacggctataaatcacgctacctgcttacactgtcgttccgcgcagatggctcttccaagtttcctgttaacaaccgctgggcctatttcccttccggcgccgtggcgtggaggatcatcgaagaatctttcatgaaaaatttatctttcctgtcggatgccaaaatacgggcaggattcggtaccaccgggaataaccgggtgggcgattttgcctatctcacttccctgcagctgttcccttactctggttacagctttggtaactcgcctgcgcagggtactattcccagcaacctgggatatcctaaactgaaatgggaaaccaccgcgcaaacagatatcggggtagacctgggattcctgaaaaacaggatcacgtttaccgccgattattataagaagaatacaaaagacctgttgttaaatgcaacgttggcgccctctttgggttacctgagcggtatccggaatatcggtaaagtgtctaacgaagggttggaattttctgtgaacagtatgaatgtgcaacataaaaaattcacctggtctaccagtttcaatatttcattcaaccgcaataaagtaatacagctgaacgaaggtgaacccagttacgcttcccgcatcacctggggtaattttaacaacgcttatccgtatatcgctataccgggacatccgatcgcatcgttttatgggtttatttttgatggcgtctaccagtacagcgactttgatcaatccaacggtacctatgtgctgaaagataaagtgccgaataatgggaatccaagaagcagcatccaaccgggttacatcaagtttaaagatatcaacggcgacggacaggtagataacagcgatctcaccatcatcggtaatcctaatcctatacataccggtgggatctccaataattttacgtacaaaaacttcgacctgaacgtatttttccagtggagctatggcaacgatatcctgaatgccaaccgcatagaatttgaaaatggcgatgtcaccaggtctttcctgaatatgttcgccagttatgccgatcgctggacaccggaaaatcaaaacaacaaattgtataaagtaggcggacagggaccactggtatattcttcccgcactattgaagatggctcttatctgcgtctcaaaacggtggcactggggtataatttaccggcgccgctgctgaaacaggccaggataaaagcactgcgggtgtatgcttccgcgcaaaatcttattacctggaccaattattcaggactcgatcctgaagtttctgtaaggcaatcggctttaacaccgggcttcgactggtcggcgtatccgaaggcaagaaccatcactttcggactggatgtgaccttttaacgaaactaaaaagctgcgattatgaaatcaaacaatatcagattatctcccgttagaaaaataacaaagctcttcctgctgtgcatcctggccggcagtaccttcagcgcctgtaacaaattcctggatacaaagccggaagatttcgtaacaccggaaaattattttaacacagaggctgatctcgaaagagccctgaacggcgtatacaacaggctgatagataacttcggaaggatgtattcacgtggactgtacagcttcctggccatcagcgatgattttttctacaagaatattaccgtgaataatttaaaggtgatggattttgacgccggtcagctggatgtaggcaaactctgggaagttgcctaccagggcatcgaccgcgccaacctgttactcgaaaatgtagacaagccaaagatggatgaaaaaaagcgggcagctattaaagggcaggcgctttttctgagagcttactattattttatcctggtagataatttcggcggcgtgcccctgaaattgtcgtctacccaatcgcctgtagaagtcgcgctgccccgctcttccgtggcggatgtgtatgcggcgatcctcaatgatatgaaagcggcggagccgctggtgaacgatatcagcacctacaccaataatgaaagggtaaccaccaccaccgtgcaggccatactggcaaaggtgtacctcacaatggccggggagccgctgaaagatgtatcaaaatatgccgacgcattaacttatgtggacaaagtgatcgcctccggtaagcactccctgaatcccgattacagcgccatcttcatcaatcactccaaagatattaacgagccgaaagaatgcctttgggaaataggtatgtatggcaaccagcagggttccacccagctggcaggcggcataggtattgaaaacggcgtggaatcaccggatgataacgttggttattcaaatgggccggtacaccccagcgcgaggttgttcaacctgtatgatgccgccgataagcggagggactggagcattgcaccgtacaaatattccctcgtgaatggcgttgttaccaaagtggcttataccgctacgcagatatatgaccgcaccgccggcaaatggcgccgtgaatacgaaacgcagacacctaaaaacaggtcgtataattctaccaacttcccggtgatccgttatgcagatgtactgctgatgaaagccgaagcggagaatgcggtgaacgggccggtagcagcagcttatgaagctattaatatggtaagaagaaggggctacggcaaacctccggcaacgccggatgccaccgttgacctgccggccggtttagggaaagacgcattcctcgaagcactgcaggatgaacgggcgcgggaacttagctttgaaggggcacgcaagcacgacctgatccgctgggggttattcctgtctaaaatgcaatcgctggcggctgaagtagcagcaacagcgccctccgcatggaaatattcagggaacgcggcaaagaatacaacagccaggaacgtgctgctgcctattcctactacagaaaccaccattaatcacctggcagaacagaacaaaggttggtaacgccgcgctaaaaagtatttaatatgcgaaattcattatacctgttgatcattgttattatatttatctcctgtgcaaaggagaaagtagtcacaccgtcgctggaaataactacttcttcacttacttataaagcaggagataccgttacctttaactttaccggcaacccggataatattactttctattccggcgaacccggccacaactatgcgttcagagaccgtaccaccgcagaaaatgatctgcagataaatttcaagacatgggtacaatttgggatgatctataaaaatctgcagttgttggtgtctaacaactattccggtgtagccgataccaccaatgtaagggccgctacctggacagatatttctgaccgagccgttttttccaccgggcaggacaatacaccgtcagggactatcagcctgaaagattttgcagacccgaaaaatacggctgcccgcatttacgttgcttttaaatacacggactataaaaaaacacagggacaaaaccgctgggtagtccggacctttgaagccaacaacatttcagcagatggtgtagtatcgccggtggcggtactatccagcggaggatggaaagcattcgattttaaaaacccggcatccgtgtggacggttactaccgcgcagctgttgatgtttggcggtgataagaatgcggatgataatgaagactgggtaattaccaaagggctggatcctttttatattaagccggatgcgggtgttgcactgaaaaatatcagtaccgtactgccttcgtataaatatgtttacactaaaccgggtacttacaaagtagtatttgatgcgtccgcggtacgttataatggagaaaaaagaataacaaaagaacttactttaactatcaccccatagctgaaaagcgggggttaaacggaaacatttgatgaacactgtaatcgatacgtcagtcattattgtattttccttatttattatgctggtgggtttttccttttccaggacaggaagaaacctcaagtcgttttttgccgcaggcgaatcagtgccctggttcattggggggctctcacttttcatgagcttcttttctgcaggcacgttcgtggcatggggatctatcgcctataaatacggatgggtagccattaccatacaatggaccatgtgtatcggcggactcgtaacaggattatatctggcgccccggtggaaggctaccggcaaccttaccgcggcggagtttatccgcgaacgcctgggggtagatgtgcagaagatctatatctacatctttatggtggtatcgttactgatcaaaggttctgtgctgtattctgtggccaggctggtaagcgcttcactgggactgccactgatgccgtctaccgtggtgctgggcctgttcatgattgcttataccgccgttggcggactgtgggcagtaatggtaacagatatattgcagttcgtaatcctcacggcggctatattgattattatccccctggcctttgatgccgccggcggtgtgcagcacttcctgcacttttcacccgaaggttttttcagcgtagtgaacggggaatatacctggggctttatcctggcctttgcattgtaccacgttttttatatcggcggcaactggacgtttgtgcaacgctataccagcgtggatgttcccaggtctgcatccaaggtggcgtatcttttcgcaggactgtatatcatcagccccgtgctatggatgctgccgcccatgttatataaaagtatcaaccccggtttgcagggactggaaacagaaaatgcctacctgatgatgtgccagcatgtattgccggccggccttatgggactcattcttacgggcatgtacttctctacgtccgcatctgccaataccgcgctgaacgtggtgtcggccgtttttacgaatgacatctacaaaggttccatcaacccaaaagcatctgataaaaaactgatgagtgttgcacgcatatcctcctggttcttcggacttggtatgatatgcatcgccttaattgtgccttatatcggcggcatcgttgaatttacactgagcataggcgctgtaaccggtggcccgttgctggcgccacctatatgggcgctgttttcaaaacggctaacaggaaaggctacactatatatcacgggtatcagcctggctaccaatcttgtatttaagattatccttccactggcgtatggcaccggtttaagccgcgccaacgaaatgctgctgggtgtaggattgccctttgtaatgctggcgctgtacgaagcatacgcttattatagaggactcaccagcaatgaatatatacagctcaaagcactgagaacacaacgcagggaaaccgttcgcgaaatagatgagaaagaagaactggagataagaaagcaaaacaaattcggcctgaaagtaatcgctttttcgctttcatttattgcattgctgttattcggactgtgtttcttttccgggaaaagcgctacgctggtagctggtattgccacggtgatcctgttaacagcagccattccgctacgggcatcccgcaaggtgaaagtagacccggtaatctcaccgtcagcacatttggtaaattaaaaagcagatcctttgagagaaatattatcagccggtatcttatactatgcagtgtgcgtttgctgtatacctgcaccggcacagcaacaaaccgcattggccaacaacgcgctgcggctttcctggaccagcaaaaacggggaatggcatattaaagaggtggccgttcacgggcaatccctgccgcataccagtggcgaatacaccctgctgtatacgaaagagaagcccggaaatacacccatcacattatacgataagtcgggtaagaagagcagtttcctggagccgcaatacaaatacattgttcctttatgggaagcagccctgaaacccgttcccatgaatactgccggcgaggccatctatttctatccttcttccgttaaaaaaaataacggggagctggtcttcacgggggaaaataataaggctacggttacttcctcctggcgactggatgaagtctttaaaacagatatcctggtggaaatatcattgcaggcaaaggaagacggctactattccctggcaacacccacgctggctactgttccggaaaatgaactggcctggggaggcataccgggatactttcaaagtaatgcggtggagaaagatattataaaagcatacgcctatatgcagggcatccccgataaaccggtgattgtccgcgagagaacggcggccaccttgtcgcctttcatccaaaccaaaaacaacctcacgctggcggtaatacccacccccggtaccggaagggatccctgggaagatgacacgaatacgcagagtgactggctccttggtctttcccttatgaacaggaaggcatcgcttacgcctacactctatcacccggtgctgggagaaaaaggctccctcctgaaaagaggagagaaggtgactttttctttcaggtactcgctgcagaaggccggctggtatacggtgttcaagcacgccgtgaacgatatttaccatttcaacgatttcctggcgctgaaaaagacgcgacaatcactcaccagccgcatcttatccatgcataaatatgtagtgaataataagacatcattatggaacatcgaaaattataaagggatcgatatcggcgcacaatcttacctggggggtgtgtatggatcggaaaaagatgccatgaagaattccgattatggcgctatgtggatgctggccggcatcaccggcgacagcgtactgcagcaaacgcgcctgccttatgcccgcaactttaaattacagcaacaggataatacgcccggctttttccacggcgccgcagcaggacaatattatctcacaaaaagtaaaagatttacagaagaatggggaccgtatgtagaacccattggtctcacctattacatgatgatggacatgggtaatgtcctgctgtttaatccacgcgatacggtattaaagcaagaactgcaatctgcagccgataggttgctcgcctggatggcgcccgaagggaaatgggcggtggcttacgaccatgcttcgcaaaaggaaatgtttacggaagtggaggacctgcgtcctactttttacgggctgatagtagcctggaaaatattgaaagataaaaaataccttgatgcggctaaacgtggcgccgactggttcatccggaatgccaccgcgaaaggacatttcctcggcgtttgcggcgatgcccgttttgcgccggattttgcaaccgggcaaagcgcccaggcactgctggatctttacgatatcacaaaagatcgcaagtatttgcaggccgccgtgcgcaccgcgcaattgtacacgacttctatttatactcaccctgttccttccgccaaaagtaaaaaggtgaacggtgtattacggcaggactgggagataagccaggcagggctcagcttcgagcatggtggtatccttggttctgccaatcatcgtggacctattttgctggctagtcatgccggtatgtttgtgcgcatgttcaccctcaccggcgattccctgttcctgaacatggcccgcgccgccgtgctcggaagagatgcgtttgtagatagcgctaccagcgtagcctcctactattgggatgtgatgaataaaggcgccggtccttatccgcaccacgcctggtggcaggtgggatggatcaccgattacctgctggctgaaatggagatgcgttcatccgggaaagttcaattcccgagaggatttattacaccgaaagtagggccgcatcaaacctatggttttgccgcagggaaagtgtatggtaccagtgcggatttgttgttgaaagatggattgctgaaaacaaataacccttacctcgattactattgcgctattaatcttaaagagcataagctgttcctgctgttgctgaacagcgacgacgatccgctgaagtgttcgatagacattgattacaccaaagtactgcccggtaaaaccataaagccggttgcctgctaccggatcagtaaaaacggcagtaaaaagaccactgaaataacgccatcattccaggaagacatcccgccttacggactgaatgtaatagaaataaattatgagctgttggctaagtagatatttattcctggctgccataggatgcctgtgcagcgtatcatcagtacaagcgcaaaccggctacttgttggaagcagaagatttccagttcaaaggcggttggcaggtggaaaaggtgccgggcgaacaagtgtccggtaatactatcctccgcgttttttccggtaaagtaaaagccgcggatgcgcttaccgtgatcaacagcaaagctgccggcacatttactatttgggtacgtaccccggattatcccgccaataaacccggcacgcgtttgttccaggtagccatcaacgagcaaccgctggaaaaagaaccagggcagcatggcaaggaaggctactactgggaaaaggctggtactgctacgcttgatgccggcgaaaatgtagttgcgctgcaggatacaaagggtaattttggaagatgtgatgccatcttcctggccactgccggctttgatccaaatacagaaccgctggcatcactccagcgttttaaaataaggccactaacggtgaagtatataccacctgctccggttacaccggcagccggtgtgaaaaatatttccgggcaaggcactgttatcgctggtattagcaacggtaaactccgcctgcaattcctgcaaacaactgaccggcagatagtagccagtaacagtatccggaaaggcgatcagtggatcgatatgcaaacgcatggcgaaggaagcaaaatattcctgcttaccgccaaagatccgcagatcagctttggcagtttcttcccttcctggaacggaccggcagcttccggtagtttccaaagccgcggcaaaacgttcacggtactggctgctgaaagtcttaccaatccctttcttgcgggcacactacaggaatgcctgccggttgccgtgaagcagttatcggataaaaaactggatgtcacctatcagactgccgcaggagataccctgaaaggtacctggcaactggcgcctggcaataatcatttactgctaacgttaacgtatataccaaaacaggcgggatattacagcctggcagttaccggttttgaaggagtaaaaaaagaagaggtaaccgccatacagctgcctcccatgtttcaataccagcgcatcccggatcacccggtgatgctgccttctgccatgatgccgcagccattggccatcatggaaacgaaggagaggatcgctgtttttgtttccggaacaccggccgatttcccattggattggggagaagcaggtacttcgccgatgggatttaccattaagaataaagagaataacgtacagccggtagcgttatcgccggtgctgggactggatgattccaggcgtgccgccggtgaggctgtcacccgtgaatttgcactgggtgcattgccctctggctggaacgatgcactggcgtatatatcagacagtatctataaagtaaaggactatcgcatacagggacccgtttctctcacagaaactgttttcaatattacagacctgatccggaacgacaccgcagcgggctgggcgccggaactgaaaggcttttacgatatcgaagcagatccgaaagtgacgcccaccgttgtgcaggctgcgccactggcagtggtttcagcggcagtgctggaaaaggacgaagcgttttacatcagcagggcattgcccactatcgagtatacgctgtcccgcagcgggttccgctggtcgaggggcattgccggcacaccgtttaacaaagataaacagtcgctggtgctgagcccctaccactcgcagtttaccacggcatactacgagggcttgcatcaattgcttggtgaagccaatccctggctaaaagaaatagcgcttcccggaaataatatcaggtcagcgaaaggctattcagtgaacattcccgcctggacacaggaactggcagcttaccgtttcaccaaagataaaagctggctggaggccgcaaagaaacatgcgaaggagtatattgcaacggaagtatatggcactaaaaccgcaccattaggcaagcagcctttttataatgcatctttctacgcctattggtgggatctcacagacctttatgacatcacaaaagatacgttcttcctgcgcgctgcggaaactactgcttttcagacgctggcgggagtaagggtgtatccggaagtaaaggaacagctgcaaacgattcatccgggcagtacctacgatggcaacactacgttgtggtggaaaggcggagagaaataccgcctcgggtttccaagaaagaaaggcgatgcaccggagaaacaggtgccgcaaagcctcgtatctcccgttggactcggatttgagcaaccctttacattctttgatccgggcaagctggtgcgaccggtattcatgagcagctgggcgcctcacctgttacgtttatttgctgaagataaccggacgatttttgaaatctatgcacgcaatgccgtgataggacgcttttcaaactaccccggctactatgccaccgggtttactgatattacgatgcagccggatttcccttataaaggtccggatgtgagctctgtttattatcatcatattccgccgcatctggcgtttacactggatttcctcatcaccgaagcaatacagcgttcccacgggaaagtgagtttcccctatggcaagcaggacggctttgtatggtttaataaccgggtatttggaggaggcagcggcaaagtattcgatgatgaaggcgtgcgcctctggatgaaaagaggactggtgcaaataaacaacccggccgtaaattatgtcaccgctatttctcacaaccgcttctggttgtttttactcaatgaatcgcaggaaaaagtaaccgctgatattcttcttggaaaggaagtcgcggtgcaggataacgtagttgctgcctgttatgccactgccgctgctccgccggccactgttcccgtgaacaaccgcaaactgcgtgtgcccgttaccggtaagggattttctgccatctctttcccgctgaagataaagagagaagtgaaaagtataccgccggtaaagaatggtatgcaggtgctggatctgggtacagggattggcaaatgttatgcattcaggatacgttcgccctttggatgggatgccatatacacctacctggaatcgccgcctgaagcggggttgcagaccagcttccaactgaatggagaaagccgtgttattactgcctatccttatgaaagctcgttttatcccgtgaaaatatcagcagaagcggtgctgaaagtaaaggtcaccaccggaaacggacaagtgaaagaagggattgtcacatttgataacaactgatcgcaatatgaagcattattttatcctggtactatgtatgggaatgtcgttggaaatagctgcacagcataaagaagaagcggaaagagctaagctcattgccctttcacaggcaggcgcctcgcctttatatttttacccggctgatactgtgccattaatagcccccggcaacttcaacaacccggcggaatccaccgtgcgcaacggagcgcctcatttctttcaaaaagttgcgtcaggaaaaccggtgacgatcgggtttataggaggaagcattacgcagggtaatcaatgctaccggccacaggccacccgttatatccagtcgatgtatccatcggtaaccatgaaaggcatcaatgccggggtatccggcacaggcactgatcttggcgcctgccgcctccgggatcagctgctgcaatatcaccccgacctggtatttgtggaatttgcggtgaacggcgcctatacagatggaatggaaggtattgtgagacagatacgaaagtatgatcccactatcgacatctgctttatttatacgatccataacgaacatacgaaaatctacctggaaggcagcatccctgaaaacatccagggccttgagaaaatagcggatcattaccagctgccatccatacatcttggtatggaaatatccgtgctggtaaaagaagggaaggtggagtggaagagtgacagcacagctataccgggcaaaattattttttcccgcgatggtatacacccgataacagccggtggcaacctgtatgcagcggctattgcaagaggcatgaataagttgaagcaacacaccgctatttcttccaccacattacctgcaccactgatagcaaataactgggaagacgcgggcatgtatgccccgcaggatattgctgcattcagtgctgactggagccgcgttaataccgccaattccccgcaaaaacagtttacaggatggttcccctatattatgaaagcaacgcagccaggcgcttcctttacctttaaattcaacggcagcatgtttggcatttttgatatcggtggtcccgaaatggggcagctggaagtaatagtggatggtaagccggccaggctcgccgccgccggtgtaaaaggcgcccgccagctgaagatagtgaacgcaacagatcccaatggcagtaacgtaattaaccggttcaataacttttgcaataataggtaccgcggtcaatacgagttcatctccctggcgcccggtattcataccgtcaccatccggctatcttccgaaaaagcagataaagtaaaaatcctgggagataaacaactggaagatattaccaggaaccccgctaagtacgataaaaccacggtgtatatcgggaagatccttttaaggggaaagcccctgtaacaacagcaactttttatgggaacattcccgtgaaatgggaatgttcccaacttttttagcggccctatattttgaagttacgatgcgcaggctgttaatttgaaggattaaaaactgatacggtattaattatttcacgttcatatgcggtgcttgttaatcatacttctattattgcctgttcagattgcacaggcaactgataccctgttgctgcaaagtccgcataaaacactgtgcacaaaactttttacagcacacggcgccctcctgtaccagctgcaggctggcaagcagtgggtgatcatgccatcgcgcatgggcatcagggtaaacaacaaaaccaccggcgtccatgtgcaacaaatgaccatctccaaaagggagataatccgggaaacacatcccacgcggctgaatgcagctgtagctaaacaggagtgcattgcctatacgatcgccataaaagagcctggtaccacctataccatagaatgcaggatgtttgataacggctgcgccttccgttatataatagatggaacagcagataaacacgtgcaggaagaattaactgcttttactgtgccggcttcatacggtgtatggtattttgaacggaacaacagctggaaactccagtcgtatgcagggttatggcaacgctctaccatcagtcagttatccaccgtgtcagcacaaggccccattcagggaaagccgctagtgattgaactgccacaaaaaaaatatgcagtgattactgaagctgcgttgtatagctatagtggcatgcggctcaaagcctccgccaatggcagcttgcaggtgaacttcacagaaggcgataccggttttgtagtgaaaggtacattagttaccccgtggagaacgatcctgtatgcagataacctcaacgcaatggtgaataaccaggtgattgaaaatctgaatccgcagcccgacagccgtttatttaccgatatcacctacataaagcccggtaaaagcgtatggagctggattacgagagatgaacactatatggagcctgcagaagagatgcggtttatagacgccgctgctgccctgggctttgaatattcgttgctggatgaaggctgggaaaccaaatggccccataaatgggaacagctgaaaatgctgtgcagtgatgcagcaaagaaaggggtacgtatatgggtatggaaaaactctaaagagataagagacaccgcgcagcgggatgttttcctcgacagcgtagtgatggcgggtgcggcaggcattaaaaccgacttcatgaacagcgaagcccaaacactgatcgcgtttgaagagggcctgctaaaagcaacggccgccaggaaactgatggttaacttccacggctgccaggcgcctaccggagaaagcaaaacttaccccaatgaaatgacccgcgaaggtatccgcggcatggaactgaatattatgaaagaaccgatcccggcatggcataatgcggcgttgcctttcacccggttcctctgcgggcacggcgattatacccccggcttttttagcaaccgcggacatacaaccaatacgcatcagctggcactgctatacctgtttaattcgccgtttcaatgcatcgcggaaaacccggccactttgctggataatgatatttataaacccattctcccactgctgaaaacattgccggtaacctgggatgaaaccattgtgctgcctggcagcgatataggcaggatggccgctttcgcccggaggaaggggcgcgattggtacatagccgtgattaacggaactgacagtgccagcacatttaccctgcagccatcttttctcagtaaaaaaataaaatatacagcaacactgatcacagacacgcctgatggcaacgcttttgcatccacatctccggagatcaatgcaaaatattacaggaaaataatgatacccgcaacaggcggtttggttttacggttagcagcacataataatgaaaacgactagaaaactatatggtcatatcggattgttgtgcatcgccgctaacatggtgaatgcacaaagccgggtgtctgtaaaccagcagaatattgttatcaccactgccggccggtcgtacgcattcgctccgtcatttgtggtattatataacgccacggatcccggtatggcgctaaagcccgccggtattaaaaaagttgaatacaatgtgcttacctggaaagtagccgatagcgcgaaggccgacttcaaacaaaagaaaataagtgcttcggttgccggcgacggcttcgacgacaggatactgcgcagcaaaaaagaatacagaaccgcgaatatatttaacgccggggaaaggatggaggtcgttgcagatagcattgaacaaaagaatgacacggttttcttccgtttcccctcttcccaaaaattccggttaacggcttatgttatcacctccgccaaaccttaccccgtattgcagtacagcttccagcctttgcaggatggctattacagcattggttataccggcgcgccggcatctgtaaaggagaaggccactgccatatggcagccactgatctggcaggaaaagcggatcccggatgccgcctatcttacgccggcatttatggctacactgcccactaccatggtatacgacggcgctgctaccattggtgtgctggccgcaccggagtaccttccttttcagccgttgcccgtactggctaacagccagtttggtattgcactgctcaacccgcagcaacaattgcagccacaggtatatgcacctataccgggaggttacggttcccgcatgaatgccgggcaaacattccgtttcggacttcagctggtagcggaaccacttgccatcaacaatacttatgaacggattgcggaaaaagtatttggcttccgcgattaccggcacaatgatatctcttcgcttaatagtacgctggataatatggtggactatgccatgtccggctacgcctggttcatcgacagcctcaaaggctgcgcttactccacagatgtaccgggcgctgtgaaaaatgtttccagtcttaacccgctggaactggcgctgataagagatgatacagcgatgtttgaaaagagggcgtatccgttaatggagtttatgttgtcgagggagaagtttcttttcagccttgacagcacccagaagatccagagtccttcccgcaggttaaaaggtccggtagcgccattgtcggagttagcggcgctctatgagctttcaggaggcactaatgatttttacctgcaaatgatgcagcgggaatataacaacgaccgcatacgcaatctggatgtaaaagaaaaaggtaacaactggattaacgcgatgcagctgtaccgcgccaccggcaataaaacctacctggatgccgcagtaacaaaggcaaagcaatacctggaacaacgggtgtaccagccacaaactgcttttgatgatacgttctccggcagcttctttttctggcccacttataccaacaggtggatagagcttttacagctgtatgaactcaccggcaataaaatattcctcgatgcagcagtgcagggagcccggaattataccatgttcacctggatgtgcccagtagtgcccgacagcctgatcaccgtgaataaaggcgggaaggcgcccatgtattggtacctgcaatccaaaggacatcagcccatgtattaccccgaggaaaatgcgccggcctggcggctttcggaaacaggactgacgccggaatcatccggtaccgccacagggcatcgcgctattttcatggccaactatgccccgtggatgttacgcctcgggtattatgcgaaagacagctttctcctcaatgtcgccaaagcggccgtgataggccgctacaggaacttccccgggtatcatatcaacactgcgcgaactacagcttatgaaaaagcagatttcccgctgcatgaacataaagaacagagcgtaaattcttttcattataatcatatcctgcctatggcttccatgctgctcgactacctggtaacggagacctatatacgtagcaaagggagtattcattttcccgcagcgtatattgaaggatacgcctatctgcaaagtaatatgtatggtatgcagaaaggatctttttaccaggataagaacgtgcagctatggatgcctgcaagattactgcgcatcagcaatacagagctgaattacatcgctgcaaggaaggatcataaactattgctggcttttaccaatcagtcagcgcagcccgttaccgccacagtaacagtaaaccccgcattggtaaaaccggccgccggaagtaaagtgatttcatacaccggcgcggcgccgcaacaaaccaaggacagcacctttgttgttaccgtacccgccaacggcatagccgccgtagtgcttccggatgtaacctatgcaggtgccgggtttcagcaacaaatattatcagggaccaataaccgcagccgggattataccaggctcagcaccggcaacgcacacgcgatgctgtttaagttcggcagttacggcaggcgcctgtatatctacctggaagacgatgataccaagctgaaaaatgtctccctgtattataccagtaataccaagaaagaagcaaaaatcacggataccacctacccgtttgagtttacggtaccattaccggaacaacaaccggtgaaattccgtttagccgtaaccggtatagatggaaaatcagcagaaagtaaaacagttgtactgggagaaaaagaataattatgtacaatacaccggcacagaaaattttcaggaccacagcagccatcttactggctgcgagcatccacgtgtccgctcaatccgtacacgtaaaagattttcatgccatccccaacgatggcctggatgatgccaaaggcatacaggacgcactgaattatgcaaaagcaaatagcattcctaccatattatttgacagcggccggtacgatctgctacaggtaagcgccactgcattgaacgcttacactggtctgaaggaatatgcagggctgcatttacagggagctgcagcagcggatcatacgccggctacgtggctggtgaagaagaatccgcagcagaataacacgatactgccgccgcatatgcgtttcgaccagtgcaataacctggtgatggagaacctggtattcgataacgatccgcagtatgctaccgcgggaacagtggtggagaaagatacttcgcatgtagtggtgcaggtgtttgacggattgccggctgtaaacggaatgggttgctatactgctaacatatgggacagtgcgacacgtatgttgaaacaggtgcccagtcttactttcgttgatgagatagccacgcagcaactttactggcagctggaaacaagggagcaaaagaattatatgcggatgaacaacgctgcctttgcatcacggcttgccgtgggagatatagtgtcgtggcactttggcgggcaaaccatgttccagctggcaataaacaactgcgatgatcttgttctcagaaatatctcgatggttaacatcgcaggatttggtatccatacttacgcctgcaaaaacattaccgggcaacaggtggtattcaaagccaccggccgacaactggcagtaggtccgcgcgatgcctggaaaataaacagctgcgatggcctggtagcaatagatagtatgtatgtggaaggtgttcgttgggacggacagaatgtacacagcgccttcttccaggtgaaggaacggctcgcatataataaaataagggtgtggaaaagatataccggcgtagcgcctttcttaaacgacagcatcgggttttggaatggaaataacgctgtcagtaaaatgccggtgagctggcagctggaaccagcgggagacggcggtatttatggtatcatcaccttgcaggattcactgcctgattttgtacaggcgggaacgcttatcacggtgtacgagtgggacattgatgactaccggttgtcgcacagcaccttcaggaacatcgccgggtgcgcgggtgttatcaaatgcaccaaagctacgctgcagcaggtttcctacgatcatattatgtaccctgcgttggtgctgggtacggaaattaccacgcataatgaagccacttttccgcaggatgtgatgatccgggaatgcaactttaacgccagcggctgggtgtcgcgcatcggtaaaacaggattggtggggattggcaacagcggcacggaagcaatggcaataggaaccatacagtttgatcactgttctttttccaatgcacctatcggcattaatgccagtggtattaaggtgttgaaaattaccaataatcatttcatctcggtgaatcaatcttataaagtaaacaatagtaacaccggccaggtgatctttgaaaataatactgaacaatgaagatgaagaatatactattcgtgttattgctgagccctttcctggtgatggcgcagggtacttcaaaggcgccgctcagtggcgtatggacgtttgcgttagaccccatgagcaggggcatacaggataaatggtacgctgcggattttgcttcagcaggctttgataaagtacaggtgccacatagcttttcagtggataagcgctattttttttataccggaacggcctggtattttaagaagttcaatgcgcctgttgtgcagaaaaacgaacgcaccttcctgcagtttgatgccgtgttttataaagcaaagatctggctgaacgggcaggtggccggcgggcacgagggcggctatacgccttttgaaatagaggtaaccggcttactaaaagataaaaatacactcgccgtatcggtgaataatgcgtgggatactaccactattcccggggctaaggccagcgacgccaaagaagcgccaaatgccacccagctatatgcctggatgaattatggcggcatcaccaggccggtgcatcttattacacggcccgcagcctttatacaaaatataaaggtagtggccgaaccggatctgaaaaaagggaatgcccgtatacaggtaatcgcttcgctgaaagattacctgtcgcccgatgtaaaggtgaacatctatcaatcaggtaataaaaataacatccgctttaaacaaatatctgccaatgcttcgcaagtaacactggaaggcatactgtcatctgcgaagttatggaaccaggatgcgccgaatctctacgaagctgaagtgattgcaggggcagacaccatgcggaaaacattcggtatccggcggctggaaattaaaggcacgcaactgctgctgaatggtgagcctgtccgcatgggcggttgcaaccggccgctggattaccccggatacggttcccttgatccggatacggtgctggagaaggacctgcagctgatcaaaagcggtagcatggaactgtcgcggatcagtcattacccggtatctgaaagtatgctcgactgggccgataagcatggtctccttatcatcagcgaagctggtaactggcaaatgacgccacgccagatggccgatccgctgatgcgggcaaagtatcagtcgcagttgaaggaaatggtggagcgcgactggaatcatcccagcgtaatcgcctacagcctgggaaatgagtttcaatcgcaaacaccggaaggtatttcctgggtgaaagatatgggcgttttcgtaaaatcactggatgccagtcggctggtcacctttgccagctttaatgtatggcgcgaatttgtaaaacgtccggaagatgaagcgtccctgtatgtggactttatcagtaccaatatttatggcaacgatcagctgccacatctccagcatattcatgaaatatatcccaacaagccggtttatatcagtgaatttggtatgcggctgccgcaaagtggaaaagaagaagaccgtattacttatttcagaagggccatgcagatcttccgccaatgcgattatctcataggagcttctgtatggacgtttaatgattacctgagccggtatcccggaacagatgcaaacggttaccgtgcatggggattggtggcgcccgacaggacactgcgtgcggtgtatcctgtatggcaggaagaattttctcctgctgttattgaactggtaaagatgaatgaagataaagccattgttaagatcactgcccgtgttgattttccttcttatgtactatgcaattaccagctcaggtatggtaataattcactggagctgcggacgctgaaaccgggtgaaagccaggaggtgaccatacctgttaccggtaaggcactcacagtagccttggtgaaacccggcgggtttgtagtagtcacaaaaagtataaaggaataatacacgatcaataaaattataaccgtacaatcatgatacaatctggagaaacaaacagtcgctcttttcccggcatagcgcttaacgcggacctggttatcaccggtggcggcctttcaggcgtgtgctgtgccattacagcggccaggcagggattaaaagtagtactggtgcaggataggccggtacttggaggaaattcaagcagcgaaatccgtttatggatactgggcgccacctcacatatgggcaacaacaaccgctgggcgagagaaggtggcttggtagatgagatcctggtagaaaacacgtaccggaacccggagggtaatcccgttatatttgatatggtgctgctggataaagtgaagaaagaacctaatatcaccctgttgttaaataccgccgtatatgcagtggaaaaaaaggatgccactaccattcgttcggtgaaagctttttgcagccagaaccaaaaggaatatttattaagcgctcctttattttgcgatgcctccggcgatggggtagtgggcttcctttcaggcgccgcttttcgcatgggcgctgaaagcagtgaagaattcggtgaaaaatttgctccttccgccacgtatggagaactactcggacataccctgtatttctacagtaaagataccggcaagcctgtaacattcatccctcctgaatttgccctgaaagacattacaaagatcccgcgttttaaaacattcaatgcaaaggatttcggctgccgcctctggtgggtggagtatggcggccggcttgataccgttcacgacacagaagacatcaaatgggagctgtggaaggtgatatacggcgtatgggattatatcaagaactccggcaatttcccggaagcagccacacttaccctggaatgggtgggcgctattcccggtaaaagggaaagccgccgcttcgaaggtgactacatgatgaaacagcaggatgtgattgagcaacgtacccatgaagatgcagtagctttcggcggctggtcggtggacctgcaccccgccgacggcgtttttagtgagaagcctggctgcaatcagtggcatagcaaaggcatctaccagattccataccggagcctgtatagcaaaaatatcacgaaccttttcctggcggggcgcatcatcagcgcatcgcatgtggcctttgcctctacccgtgtaatggctaccgcagcatatgtatcgcaggctgttggagtggctgcggcggtttgtaaagagcaacatattttaccggcagacatttttaataaagggcacatcaccactttacagcaacgcttacttaaaacgggacaatatattcccgggttaacgctaaaggatcatgaggacctggtacaatcggccctgatcaccgcatccagcgagctggtgtttaaagagtttcccggcaagccgctcctgaaacctttaaccctctccgttgcacaaatgctgcctttgcaaaaaggagaagtggcgccctttatttttcatgcagatgccaccagcaacactgaaatagaagtggaactacgcgtgagtagtaagcgcggcaactatacgccggatattaccctggcaaaacaaaccattccgttacatcctggcagaaactgtgtggaccttcgctttaatacatctttagaaaatacggcctacgcatttgttactttcatgaaaaacccgttggtgcaattgcattttacagagaagagagtgacggggatactgtcggtgttcaacagcgtaaacaaagccgtctccaattacggcaaacaaacaccgcccgaagatattggcatggaagcatttgagttctggtgtccgcaacgccggccggaagggcataatatcgatttaaaatatcaccagggcataaacttattcaaagcagaaaatatccgcaacggaaccgaccggcctgcatccacgcccaatgcctgggtagccgactggaacgatccgcaaccccggctgacgctgaaatggaatgcgccgcaacagatcagtaccatcgatctgttcctcgatacagattatgatcatccgatggaatcagtattgatgtcgcatcctgaaacggtcatgcctttttgtgtaaggcagtacaggattaaagatgcagctggaaatatagtagcagagaaaacaggtaattaccagacgcacaaccgtattcaattccagcaacctgttacaacggatacgctggtcattgaactggaacatccgtctgccaatgtgccggcggcattgtttgcggtgcgttgctattaacggagtgttcctttttattcctataacataagtatggagagccttcagatcgcaggatttgaaggcttttttatgatgggaatggagatgaatcattaacgtttgagcagggaccttaatatattcacgctaaccgtcaggccgcatctttccagtgtagccagtacctgctctgctgattgcggaggactcattaacctgtttacctgtgcgtggaatgctttcagcaccctggtttcatccaggctgatcaggcttttgataaatttgtcaggtgtttgcgcttccagctgataaggttgtaaccgttttgaaggaaagtctttcaggttattagttataatcaacttcgcatcgcctttaatagctgctgccagtacatgccggtcatccggatcgggcagttctatgctgtttataagctgctgataggctgatatacgggcatccggaaatgcactatccatggcagcctgtagactttttaaacgctttaatggtatttcaggtttatttattaacaggttcctcatccattcttcctgtatctgattcgtccatttgggcctgtatagtttaatatctgcgaggcttaataaaatatctcgcaaaggagcagggtataacacatttgcgtctaacacagctaccaatccggtcgaattgatcatcagtatcccatattaagtttctgtgattgcttagctaaaaagttgagtttattggtccggttcttttgtagctgtttatcataagcaataatatcgtttaacaggattctccggtgtgtacctaccttagtaaatggaatttctcccttattcaaaaggctcaccacatgaggtcttgatacgtttaatatgtcggccgcctgttgagtactgatttccgcgtcgctgggaagtaaggtaattgattttccatctgccatattgtcgagtatcgtgtatagtaacctaaatgcctttgccggaatcgccctcgttttcttggtattgtctattgtaatagcaatacttttactcttggtttgtaatattttcctggaaatctcatacatctcattaataaaatacctggctatttcctgatccgatttcgtagttttttgtgtaatggcttccataatgcaattattgttgatacgtatacaaagatacgtaaacgaaataaacgaaacaaaactttgtctgaaaatcctccaccatcccctcattccggctttctttttgtgtcatcccccctggtacaaaacatcttctatgacacaaccattccaggtcgccatcagacaaccggtactcgatgatctgaaagcccgcattctcgccaccaggtggccggacgcaataaatccagccggctgggaatacggaatgagcctttcctacatgaaagagctggctacgtattgggcccatgattttgactggagaaaaactgaagacgccatcaatgcctggcccaattttatcatagaaattgatggctataaaattcattacctccacgtaaaaagtaaatacccggatgccattcctatcatcatttcccacggctggccaggttctttcctggaaatgctgaaaaccatttcttatctcacggataatgaaacactgccattcgatgtagtggtgccgtcactcctggggtttggattttcagataagccggcaaaagaaggcataaacgcctcattgatggcccacctctgggtgaagctgatggaagggctgggctatgacaaatttatagcacagggaggcgatttcggcgccattatcgctacgcatatcgccatgcggcacccggacaagctgaccgggctgcacatgaactatattccgttcaactataagccgtttataccgcctggtgaaaaactgacagcagaagaaacggctgcacagcaaaaaaacgctcagttcttccaggcggaaggcgcttatgcccaggtacaaacaacaaaaccgctcacgctttcatatggcctacaggattctccggtaggactgtgtgcatggatactccagatcttccgcagcttttcggatcccggcgcagtgctggagcagttattttcaagagatgaactgttgtcgaatgttaccctgttctggatcacacaaacgatccattcttctatgcgtttataccatgagatccggaaagaaccgctggcgttcggagaaagtgatttcataaaagtacctgttggcattgcacgctatccttatcccgttagttttcctgcgcggaaatatgttgaaagaggatatcatgtttgctattggagagagatgccaacagggggacattttgccgccatggaacagcccgaactttttgcacaggatgtaagcgcatttgcgaatactattttatcaaagcagcagtagatactttaggcactcatttttctcctggcatttaaatatttccgcacgggaatatcgtacaataccatcaccaggtaggagaagcccaccaaaaggagggtgccggcggtgatgataaatgccagctgcatggttccgggtttatacgccgcatagtaattggcaaagatccatatccctgcataatgtgtcatataaagcggataagatatcttcccggaaaaaacacacaagttttttaatccggaagtaagcctcgcgccagttccgagtgcaatgagtaaagggaaataaaacaataccaccagcacttccaccagccagttccattgaaaatgaggcatcaggaacggcaacatcagtaagaccgacagcccgatgaagcccagccggttctttatcatccagttgaaacggaacaccagcagtccggccagaaaggaataggaaatacgcacagcgccatcccagaagttatcttttccccagccacccatcaggttccctgcgtgataaccgactacgacaatacccgcggcagccagcaaggctaatacgaccaggtagcgccggcttagtttaacgagaataagcgcatacaatatattggccacgtattcccagaacagcgaccacgcaggcgcattaaaactgaacaggttaaaaccccggtccatcataagtggaaagggaatcaggaggatactggtaagaaagaacaacgctattttgccaaatccatataattccgggtgaccgccgaacggatcaaaaagaaagcccaacagccccaatacagacccgaaaataaccaggggatgtaacctgatgatcctcgatttaaagaactccctgacccccattttgccaatgcggttatcataggcatatccaatcacaaacccggataagcagaaaaagaagtcgaccgccaggaaaccatgtcccacaaagttcttactgtaatcagtataaactacttccataaaatgaaaaacaactaccgttaaagcggctattcctcttaatccatccaatatttcaaaatgctgtttggttcttagcaggtccgggttcaatttgttcacgttcattaaatactgttatatataatatagatgattggctgctttacagccgctaaagggcggtaaataaatgacattatttctaaatttcctaacaatcaaagctggtgtgccttttgtgaacggggttactataaaatatatatagtatggaaacaacagatatcaccgtttatatcgacaataagccttaccgttttcacatcgacgtggattacgagaatgacaaaaccacctaccgggtatccaccgatgaggagcacagcgaaaagctcgattttatgccgccacacctgcagtttaacgaagacggggaagtgaccctgaaagagcggctgcatacggtagagcaggagcagattgcgcggcttatctggcaggaaatcattgacaagatgaaaccatgaaacggtatgtggcacgtttgccacagccttgtctccggtctcagccatagaaatgatcagatgccaatatagtatcaaaatttgctaatcactttgaattttttagcaaatgatattataatttgatctcactgtattcccgttcccacagggtggttttaaagtgaggtcatttaatgaaaacaactgaaatcatcagcgaagaatgttatgccatccgcctgcagcagggcgacgaggtggctttccgttatattatggaccggtattttgcggtcattactaattttgcgaagaggattgtcgtgaatcatgctatcgcggaagatgtagcagaagaaacatttataaaattatggaacgatcatgcaaaggtcggttcctttcaatctataaaggcgtttctgtacatcgccgccaggaatgcctgttttaatgaattgagaaaagagaaaaacctgcaataccgccatcatgcctatgccgccagcatgacgggcgaagccgatttcgtagccaacgaaattatccgcgcagaagtaaaagcagagatattaagagcagtgaacagtttacccgtaaaaatgaaaagagtattccagctcggcttcctcgagggcttgcccaaccgcaaaattgcggaagaattgcagatctccgttaataccgttaaggcgcagaaattccgcgcactggaactggtaaagggaaaactccagggaaaagatattcttccctttgcattaataatactggcggcatttcacaaagattaatccccgtcttcaaaaaaaataaaaaaaaactttctcctccactaacccgaaatgatccgggcagtgtatccactatataacggcattaattttttctcagcaaagatgtgcagcccgtggccctgtaatgtgtggtcgcagtggtcatggctgcatactattattttctatggaagaaaaagacgtacaacagctattatatatcgccggacttatttaccggcagcgatcgggggaactggatgaagccgagcaggaaacggtggacaactggctggcagccagtgagcaaaacaggcagctgttccgggaactttccagtcaggatctggaagccatcacgcgcaacgaagccgatccggctaacctgcaggcatctgttgaaagagtatacctggccaccggcattaaacccggaccagcacgtatatatataagtaagtggagaacctggagatgggccgctgccgtacttgttcttactgttgccggcgccgccggcctgcagctggcaaaagagaaaagtaaaccaatagcggccatccataccaccgatgtggcgcctggtagccgcaaagccacgctgaaactgggcaacggcgctaccattatcctcgacgacgcgcagaacggcgtaatcgccaaccagggcaaaaccgtgatcaaaaaatcgggtaatggccagctggtatacgatgcatccgcatccgttaccacagaaataacttacaacaccattaccacaccaaatggtggcgaatacgaagtaatactgcctgatggctcgcacgtttggctgaatgcggcttcggtgatccgtttcccggcagcattcaccggcaatacccgtaaggtggaaattaacggggaagcgtatcttgaaatagtaaaaaatgaaaaagcgcctttcatcgttgtttccggcaaacactcggtggaagtactcggaacaaaattcaatatccattcctatccgaaagaagaagatatcaccactacattaatccagggaagtatccgcatcgccgccggtaaatataccaaagtgctgcagcccggccagcaatcgctcgtgaacaccagcagcaatagcaatatccggctggccaccggcgtaaacatggatgaagtactcgcctggcggaatggcaaattcatttttgacgacgcctcacttaaaacagtagtgagccagctggaacgctggtacgatgtaaatattgactatgccggtatggaagactaccgcttcaacggcgaaatatcaaggaatgtaagtctttcgaaagtattaaagatgatggaactcaccagtaatatccactataaaataaacgacaggaatatctacatgacaaaataagcaaagcaaaagacaaaaaaaccggaagcgcgggaacgctgccggttatcgtcaggctaatggggacttcgtatcaataaaatccttcaaccttaacatcgcaaatgtatgaattttatcattcatcgcaaggaccatctgcgcctatccaaaccggtgccagggaattgctttatcaaccattccaaagtactcctggttatgaaactaactgctttactcttaacaggtatctgcctgcaggtcagtgcaacggcctggtcacaggaggtcaccttatcagagagaaacgcgccgctaaaaaaggtattgcagcagatcagcaaacaaagcggttacacctttttttacgatgcccgttatctcaacgaagccaaacgtatcaaccttgacatcaccaacacgccggtagataaagccctggacgcctgtttcgcaggccagccctttacctacgaaatgctggaccgcaccattattgtaagaagaaaaaagacagaggaaaaaacggtcgcaccaacggcagttatcagctgggtactgtcggggaaggtgatcaacgaaaaagaagaagccctgcccggcgctaccatcaaggtgttgggcacacccaaaggcgtggtaacagacgtgtttggaaaattcctggtagaaatcggcagcgaaaacgattccctgtcggttaccttcatcggttataaaacacagatcatacaccccggcaatcagaaaacgatcgtcgtaaaattattgcctgacctcgaaaaccaaaaactcaatgacgttgtgatcgtaggttttggtacgcagaaaaaaatctctgttacaggcgccgtatccactgtgaaggtgagcgaactgcagcagtcttccaccgcctccctgtcaaataccatcggtggccggcttcccggtatcattacccgccagaactccgcggaaccgggttttgacgccgccagcgtatttatccgcggcctcggcacgttcaccggtaacaagtcgcctctcatcctggtagatggtatcgaacgcgatatgaacaacctgaacgtacaggaaatagaaaccttctcagtgttgaaagatgcgtcagctaccgctgtttatgggatccgcggcgccaacggcgtaatcctcatcaatacaaagcgcggcgctgaaggccggcccatcgtttctttccgtacagaaaccgcccgtctcaccggtatgcgctttcccagttatatcaacagctacgaatacgcaatcctggcgaatgaagccatgaaaaatatcggcaagcctcctttctatacggatgaacaggtacagaaatacaaagatcattcagatccttacctgtacccggatgtagactggatagatgtagtactgaagaaacataccatacaaaccatcaataacctcagcgtaagaggcggtaaccaaacattccgctactacaccaatgtaggttatacgtttgttgatggtctttataaagaagacaaatccgttccttataaaacaaataccagcttaaaacgctacaatttcagatccaatgtagatgccaatctctccaagaatcttacgatggacctcagtcttggcggcatcattgaaaacggcaacgctcccggcctgcaaggcggcgccccggaattattcgatgcactgagatggacgcccaacaacgcttaccccataaaaaatccaaacggatccatccccggattaggcacttttctgaatgaaaacccctttacgaaaagtacgcaaacgggctaccagaaaaggttccggaacacgattcaaagctcgctcggcgctacctgggatttgtcgtcgctggttacaaaaggacttaaactgagaggactctttgcatacgattactacggcgccatgaccaccgtgcgcgtgaaaagcccggcgtcttaccagtacctcggcccggatgccaacggcgtagaccagtatcagctcatcaaaacagagcaggcactcggctactataccaactccggcgccaaccgcgccgcctacctggaagtatctgccaactacgaccgcagctttggcgatcaccggataggagggcttatattaggtaaccggcgtgaatatgtagacctgctcgcaggaagttctatcgggaatatccctttcaggcgacaaggactcgccggccgcataacctacgattataactccaaatatttgctggagtttaacgtgggctacaatggctcggagaatttccccaaaggaaaacgatacggcttctttccctccgcagctgccggttggctcgtgtccaacgaaaacttctggaataaaaatatcatcagcttcctgaaaataagaggctcctacggacaggtaggcaacgaccagataggcggcgccaggttcctgttccagacaaccatcgataaagcccccggccatacctggtttgatccgtactatatgttcggcgccaatcaaacctaccagacaggcgctttcatggaaagccgcatcggtaatcagaacgtgacctgggaagtagctaccaaaggaaatatcggggtagatatggaactgctcaacggaaaaattaccctcaccgtagatgcgttcaaggaacggagaaatggtatcctcatcgcacggcaacaaatacccatatcagcaggttacccgtcagggatcataccttatgccaacctcggaatagtgaacaataaaggcgtagatggaaacatcgaaataaaaaacaaaacaaaatcaggcttctactattccatccagggtaacttcacctacgcccacaatgaaatagtagaagatgattcacctctgagaccactggcctaccagaacagccgcgggcaaagcatcgaccgccccttcggctatgaagccctcggcctgttcaaagaccaggcagatatcgacaaaagcccttcgcaatcgacgctgcaatcggtaatacgcccaggtgatatcaaataccgcgacctcaacggagatggtaaaataacacccgacgacagaacctatttcggttacgcacgcaacccggaaatcatgtatggcttcggtggcacggtggcgtggaaaggagtggacatgagcatatttttcaccggcgcagccaaaacaagctacctgctcagcggccgcagttcgtatgcgttttcaggcggagtagggaattacaacgtgatgcgcgaagtatacgacaaccgttggataccgggtgcagataacaccaacgccaaatatcctacggtgattgatatcaacaataccaacaactatgtaaccagcacgctctacatgaaaaacggcaactacctgcgcctgaaatctgcagagatagggtatacattcaccaaaaccctcaccaaaagggtcggtatcagcagcgttcgcgcatttatcaacggcaccaacctcgccgtatgggatcatatcaaaatagcgaatcctgaaattgataacggggaaagtctctacccgctgcaaagcagcatcaatgcaggtgtacaggtaaatttttaaagcattaaaatcattaggatgaaaacgatcacaacatattgtacgttcctgttccttctcctggcagccgtgtcctgtaagaaagacttcctggataaagcgccggatgatgatctcactattgccgacgtattctctaaccgcgattacgccaacaactatctcaccaacgtatactcacacctgccggatgaaatggtatgggcagataataaagataatccctttcatggcgccgcggatgaactgaaacagttctacccgccgtcgttttgcaacagcatgacttccggcgcatgggaccctaattccaccgtgattaatccctgggccaggaattatgcgggcctgcgcaaagcaaatatctttattgaaaatatcgacaaagtaccgttggatcaattctatacaaaggaagcgcgtgatcgccagaaaggagaagctattttcctgcgcgcattctaccatttcctgctggtaagattatacggcccggtacccatcgccgacagcagcatttcactggataccgatttcaagagcatccggcggcaacccctggaaaagtgcgtggcatacatcgtatcacaatgcgatcaggcagctgcactgctgccgacccgtattacctccgaaacagaatacggacggcccgccaaatctgctgcactggcgctgaaagcaagaatgctgctgtacatggccagcccgttgtttaatggtaaccccgactatgtgaatgtaaaagaccatgaaggcgtgtcgctgttcccggcttacgacgccagccgctggcaggcagctgcagatgccgcaaaagcctgtatcgatcagacacaggccgccgggtatgcgctctatacttctcccggtaataacccggtgaaaaactaccaggaaatattttacatgaacaacaaccaggaagtattctttgcctataatgatggtacctacgatggcctggatgtttataacgaaccgcttagtctcgccggatttactttgcatgcgcctacccaggatatcgtggaccagtatgaaatggcaaacggacaacgccctatcaccggctacaccggcgatcattcgcccatcatcaacccgctgtctggttatacggaaaccggctttaccgatactcccggaccggataacctgtatgtagccggtaccagcaatatgtatgtaggccgcgaaccacggttttatgccagtattaacttctcggggtcggtgtggaaaacgcgtaccggcggactggaattctggttcaagggggccgacggaaagcaacgtgcaggcggaggcaattacagcgtaacaggttacctgctgaagaaattatctgacccgaattttgtttttaaaccacaggagaaaagaacgctgcgcacctggatcttcttcaggctgggagaacaatacctcaactacgccgaagcgttgaatgaagcacagggccccgtggccgatgtatataaatatgtaaacctgatcaggaaccgctccgggctgcccgccctgccaggcggattaggcaaggacgaaatgcgggaacgtattcatcatgaaagacaaatagagatggcgtttgaatcgcaccggtatttcgattgccaccgctggaagatttctgaaacaacagataacgccaacatgtatggattaaatatctatgcaggagaatcaaaaacagatcctgctttctttaaaagaaccgtttttgaacgccgggtttttgaaaagaaacattacctgtggccaatgctgaaatctgaaactgataaaaatcctaatctacttcaaaacccaggatggtaataaaataaaccggatgaaaataatactgatgatgttaatcctcctgccactgagcgtggcggcgcaggaactgtataagttccccgcggatgcagatacccgttggatcagcttcgagaaccgctccggcgccaaagggagggcaggaatagaaaacaaaggcgccaaaggacatgcatgcgatacactgaaagcaggtgggagtgtaaccttactggattacgccggcgccggaatcattaacaggatatggctcaccacttcccataaaccggaagcgctgcggtccattcatatcgatatgtattgggaaggtgcgtccaaacccgcggtatccgtgcctttgggcgatttcttcggcatcgggctggcacgtagaacgccgttccagtgcgccctgttttccgatcccgaaggacggtcatttaacagctatatccctatgccttttaataaacatgcaaggatagtgctggtgaatgaatcaaaggaaacgcacctgttgttttatgatgtgaatatcaccgcgctgaaaaagccgcaaaaagacctgctgtattttcatgcttactggagcagtaatcaacaaaccaaactgggagaggattttgaaatactgcctgccatcaaagggaagggccgttacctgggcagcaatatgagcgtaatagcggatactgtgtatggcaacacctggtttggtgaaggcgaggtgaaaatgtacctggatgatgatacgcagtaccctacactggcgggcaccggcacagaggattacataggcaccggctggggacagggtgtgtttgcgcacctgtaccagggctgtcctattgcagatgcggcaaaaaaacaattcgctttttaccgttatcatattccggatccggtttatttccatagtggttgccgcgtggtgatacaacaaatgggtggtggcgggagagaccagctgcgggaaattgtaaaagccggtgcgcgtttaaaagtggtaaccgttactacaccggccaccctggttaaaatcctggaagaacctggctacccggatctcttcgatgaaaaattccccaacggctgggttaatttttaccggttggataattattccgccactgcttatttctatctcgataaaccggaaaataacctgccggcgctggcgccgttgaaggaacgtttggcgggtatactgtcaccaacaggtaaatgaatgttatgaactggaaccaactggatctgtggatagtcatcagttatttattgctcatgctgggaatgtctttgtggcaccggcgtttctcgggctccaacctggaaaactttttccttggcggccggaaaatacccggctggttgaatggaatttcctacacggctgccctggtaagcccggatgctgctacaggttatggcggcctcgccgtggtaacgggcgcttttatttcctggtggtacctgagcaggtttggactcgccttgttttttggcggcgtattgtttgctgttttctggcgacggctaaacctcttcaccacgctggagttttatgatcttcgttttcccccgcgtgcggcagcagccatgcgcttatggatagccatccggacttctatgatagccatgccggcctggacaggcatcactttactggcggcgtataaaattatgggtcctgcattcgggcttacaaaggcagaaacactttacctggtagtgcccatctctttcctgtttgttttcttttcaggatacaagggagtagtgatttccaacctgatccagatggtgatattttttgcaggcacgcttacactggccgcgctcacattggcgcatttcggcggcgctgccgctatgacggccgcgctgggtcatgctttcaatggcacacatccggaagtattacaactcatgccaccaggtgaacatcccgtattcccactggccgccgcaatggcctggatggtggggcaaagcattggttacggcggcgatgcggcgccaatgggcggcgcaatggaaggacaacggatcctgtctacccgcacaccggctgaagcgctcaccatgtacgtggtaactgccatcagcatgttcctgctgctgctgctggttacgcttcccagtatatccgctgccgttatatggcccgaactgcgcgtggaaggcgccgaccgggaactggtatatggaaaactcatgaaaacaatgctccctgccggcgctatgggattgctggtagctgcgatgatggccgccaccatgtctaccgttggcgataatctcaactttgggagccaggtgctggtaagtgatatttaccgccgctggtttgtaaaaaaggccagcgaaaaacattacatgctcatcggaaaaattggaatggcgttgatcctgtcgttggcagtggcagtagtattcaacgtgagcattatcactgatgtggccatttttatgttgcaactcagtgcggcggaactgccggctaactgggcacaatggtggtggtggcgtttcaacggggcagcgcgtatcgctgcatccttcggtggcgctgctattttttgcatagtggtattggggcctaaactattaatgtacctgcacgttccctgggcgccgcaactggtgctgccgtggtggtggcaaacattggtagtgatggcgcttaccaccgcgctgtgggttacagttgcgttgatgacaccacctgatccggccgaactgctgcattcattttatgaacgcgcacgtccactgggttggtggaagcaacacagcggcaatatgatacaacctattgtgcgcggaatgggtattgccgtaattggttttggggctacagccatgctgatcacagggttaacacaggcatggtttgcacgttactggccatgtgcctggctgttgtctggttcgctggtgttattttttgtttttagaaagatggccaacaggtacctgtcgtggctggccgccagggcaacggtgagcagggctgtactggagcagcaatccttcgaatctttatctcaaaaagtataaaaaaataattatgtctgtaagaaaagaagtcaggacaaaagaagaacacgtactatacctgggcgattgggtatttcacctggggcccacgtttatagaaacgccgtttggcacagaaacaaaagatgcagatctgcatttctatggcgagcgcttaacagcagcactggaacatgtggcggatgttaccacgcttgccaactgggagctgtaccgccttgcgccgggtaagctggaagcgttcctggaggaatctgtaagtcttattatcagcgatgtggaggcaaaatgtttccatctttaccccagctttttcgaccgctcccggcgggaaaataaagtggttacattccccgacaggcttagccttattaaagaatggatcaatgatggcggcggactgatgatgctcggcggatggttgtcgttcagcggtgtgcagggcaaatcagggtggggcaggtgtacactaacggatgcgttgcccgtgaaatgcctcgttactgaagacctggtagagtcctccgctggatttactgcagaagtattggcgcctgatcatcccgcggtgaaaggcttgccatggcatgcgttcccgcccatatttggttacaatgaagtaagtgctgttggcaccggggaagtgctggtgcgtgtaaaagaaaccggtcacccgctggtggtagccggcagctatggaaaaggcagggtgttgacctacatgtctgatcccgctccgcactggggaatcaactttgaattatgggaaggatatgatgccttctggcagcaatcattgcaatgggtaaagaaacaaaacaggtaattgatgaaccgttccattttacgcgcaggaacagccgtagctgatatcaccccgccgctggaagccggattgcttacctcttcagtagaagggcgttacgatccgtttacggcggtgcggttgccgctgaaagccagggtgctggcgcttaccaccacaaccactaccgtcgcactggtatcgcttgacctgttagggttaagcgataccgctaccggcgggtggaaagtattcaagcaggggttgtcggatgaaatattgccggagcacattattataacgtgcacgcatacacacaatgcaccggaatcggtagccttatcgcaattgtatttaacaccggtatatcgtacatggttacacgaagtacagcagcaaatacgtagtgctattcatacagcgctgaaagaggcgcgcgcaggtaccatcagcatcagcagcggtgtgctggaaggatactcgctgcaacgccgcatacccacgccgcagggcatcgtgatgtccgattccatgcagcccgttacaccagaactgatgcgccgcgaaccggctgaccgccgcgtgcatacgctccggtttaccggggcgaacgggatcatcgcaacagtggtgcatgcggtttgtcacccggtgcatgaaatgtgcctgccgcatgtatcgcccgatttcccgggggagctctgcaacgcgctggaagccaccggcaataacggcatggtgatgtttatcaatggcgccgccggtgatatcaatccgcctacggtatccggagggcccgccactgcaaggcaacatggcgccgcactggccgcagtggcgcaacaggatacctacagcgaatcgctgcaaggcaataggctgctgttcgcacatgatgaaatcacttttggaatacgtgccgctgccgtcatcaacaaagaagatgcgcacgccagggtaaatgtgatcgcaatcggggagctggccatcgtctttctcccgggtgaaccatttaccactaccgcattggaaatagaaagcgcgtctccatttacgcatacactcgtcgcggcatatgccgaaaataccatcggctatattccggatataaaaggattcgccgaaggaggatatgaagccgggcccggtaagtggtcattcctggaaaccggggccgctgctatgttacaggctaccgccctccgcctgctgaaccagttaaaaaacaacacatgaaaaagaaaatactgctgagtgccctggtatgcctgttgtacagctgcatacaggtatatgcgaaagataaaacgctgttgttctgcggcagcaataaaaacggtctctatttccttttaacacaggaaggatataaactgaaacagttcagcactcccgctgctgccattactgctgccaccgatggcgcggcggtattcatcgtatcagacacttaccccgcaattgatccggaaaagcgtattacggaagcgttgctggcggccgccaaacaaaaacacctgcagctatatgttgaatatcccgctgcattcccgggtctcgatattcctgcaaaaccgctggaaacgaggctggaacgcggcgtggtaactaccggcgatttcggtgcgccgttacagcccatgagcatactgggtatccataactgttatatcctgccggtgagtgccaatgatccgttgattgtactggctaaagtagtggggttcgataaagcagaatatggcctggacagcaccaaatcatatccgctgctgtttaaacaggacggcgcttttattgccaccactgcattgagtaactttgagcgcggacgatacggtcccgcggcttccataaaacaggtgtggacgtatatccttgcccgtatgaccggcaacccgcacctcgttataaagcactggcccatggatgtaaaacccatgtatggccgcaacgcgacactgcccggcaacgcaaggctcaacgccatccggaagggaaccgcctggttctttcatggccgcttctttgtgcatccggcctggcaaaaagaatgggaagaatacaactcccgcgaaatgccaacaggcccgccaataagtgccgataagcccgatggcgacggctcgctcggcatcatggagggacatacctccaccatcaattacgacggtacccagcaataccgctactggatgcgcgcagatgtacagggagaagtaagcatggccctttctgccgcaggcaggttgctgaatattaaaagctatcagcagaacgccgtaaatcttattaactatacgttgaaaacctccaatatgagggccggcccaaaacgggatcccaacagtcccgcctacggccttataggctgggcaacgcctaaccccacaactttttacggagatgataattcaagggccatcctcggtattattggcgcttccgcttacatgaataccaaccagtgggaccaggagatggctgccgccatactggctaatttcagaaccacgggcaaagatggcttccgcggcgaacggctggaagaaaaagatatcattaaaaacggctggcagttttacagcaaccgttccttcgtacatccgtccccgcattttgaatcgtggatgtgggcactgtacctgtggctttataacaaaacgaagtacgaaccgctgctgaccaaaacaaaaaatgcgatccgggtaaccatggaaagttatcccggcaactggcgctggggcagcagcatgcaaacacaacgcgcacgcatgatccttcctttagcctggctggtaagagtggaggacacgccggaacaccggcagtggctcgacaaaatggtgaccgaaattatgaagtaccaggatgaaagcggtgctatcagggaagaactgggcgtaaaagggaaaggaatgttcaacccgctgaacaccaattctgcctatggttccgacgaaggctccctcatttttaaaaacggggaaaaagtgtcgtgtcagttatacacctgcaattttgcactgtttagtttgaatgaagccgcgcgcgcaacaggcaataaaaagtaccaggaagccgccggtaaattgtcggcctatcttacccgcatacaggtacaaagcaataaacataaagatctcgacggcgcctggttccgtgcattcgactacgggcggtgggactactgggcctccaattcagatgcaggctggggcgcctggtgcacgctgagcggctggatacaaagctggatcatcacctcacaaatcctgatagaacaacagcagagctactgggaagtaacacaaaagtcagcgatcagcgaacccgcaaaatcattgatcaataccatgcttaaatagttgtatgaagatgaaaatatctttgctgttgtggtgcctcaccggttgtgcattatcctgccgggcaaacatccgtttgccgaaggtgctcagcagcaacatggtgctgcagcagcaaagccaggtaaagttatggggatgggccgatccgggggaacacatctccattaccacctcatgggatcagcagatatacaacgtcaccacagccggcgatgccagctgggcagctactattaccacgccggcagcaggcggcccttttaccattacgctgaaaggaaataataccatcacgctgcaaaatatcctgttgggtgaagtatgggtatgttccgggcaaagtaatatggaaatgtgcggaaactggggactgaaagacatcaaagccattcagccggctgctgataacaacaacatccggttctttaaaattgccaaagcaaccgccgcacatccacaggatcacctgaccgcccaatgggttgcgtgcgacagcgccgcactgaatactttcagcgctgtcggctatttctttgggaggaaattaaatgaacagctaaaggtgcccatcgggcttatagatgccagctggggcggtaccgctgcagaagtatggacaccagacagcattgtaagcaacaacccggtgttaaaagaggcagctacgcatatattgcccaacggcatgtgtccgcatttgccgggtgtggcctggaacgccatgctggcgccggttacacgctatgccattgccggcgttatctggtaccagggagaaaataataccggcaccgccgccacttaccaccttttatttacggctatgatagatgcatggaggcaggcatggcgtcagttgctgcctttttattttgtgcagatagccccgtttaattaccgcgaaaaaaataccggcgcactgctcagggaagcgcaacaacaaagcatgcaacatcctaataccggcatggtcgtcaccaccgatattaccggcaacgtatacgatgtacatccggctaataagcatgatgtaggctaccggctggccgactgggcgctgggggaaacttatcaccgccagggatttagctacaaaaatccgttgtttaaagagatgatgataaggaaagataaagtgatcatctcctttgaaaatgcgcaacagggactatcagtaagaggcgatagcctgacggagttatttattgcaggaaacgaccggcagttttaccccgcccgggctactgtgaaagaaaacacactgatggtatggaacaataaagtgaaacaacccgtggccgtgcgctacgctttcagtaacaccgctatcggtaacctgttcagtaaaaacggtctgcccgtagcgcctttccgcaccgatcactgggaggtgccaacaaaataaatttatccgcatgaaacattttgtctttttattactcatgatatcattcactggtttacaggcgcaggacctcgccggtctcacactcatcaaagagcatgtaaccacaaaacggatcagcagttacgacaaggccggtggtccgaacgacaacctgcaacacattgaaaacggcggtaaaaggacccttgtggatatcaaaggcgccggcattattaatcatatctggatcacgatgtggcccgccccggataaactgagccgcaacgatgtgatcatccgcatgtattgggacgggaaaccatatccttccgtgatatcgcccatcggtccctttttcggacaaggctggaacgaatcttacccttttacatcattgccactggccgctgcaccaatggatggtaccagcctggtgagctattttgcaatgcctttttccaacggggcaagaatagaaatagagaaccagtcgggcacggaaatacaacctttttatttttgcgtggactatgtggaaatgcccaaactgcccgccaataccggccgctttcatgcctggtacaataaacagctcatgggatcgcaggatagcatagaaaacgagcattggatctttggccccgaagggcaaaataccgatggccgcaataattatgtaatagcagatatcaaaggcgaagggcatttcgtcggcgtaaattactatgtgcaatcgcccacacctttatggtatggagaaggggatgatatgatttttatagatggagaaacaataccgtccctcaatggtaccggtacggaagattattttaataccgcctggggccccaaagtattatatatgcacccgtatttcgggtatgcaagggtgaacaacgatatcggtacacttggccgcacgcatctttatcgctttcacatcaccgatcctatctattttaataagtcgctgaagtttaccatcgaacatggtcataataacgagatgacactcgatcttgccagtgtagcctattggtacacaaaggaagcgttgccggtaccggacatcccggatgccaaagcccgaaagcccatgcccgcgatcaactcatacgatatccaccgctggcgcaatgagtggcggaaaaacaggggcaaggatccgaagttatggaactaactatttcatcatcatacatctcactaaatgaaaaatatatcctggttattactgctgctttttagtatgtcttgtacgggcaaagcaaaagactccaccgtggcgccgccaccggcgcccgcggataccaccttctccaatccgctgctggatggcggcgcggatccctgggtgtataaaaacggcaatgcttattacttcctttgtaccaatggcggaaatattaccatccgtaaaaccgccgccatgtcggaattgagaaatgccattcccaaagtggtatggacgcctcctgccaccggcgctaattcaaaaaatatctgggcgccggaactgcatcgcctgcaaggcaaatggtacctgtattatacagccggcgctacatccgacctggctacgcagcgtttgtttgtactggaaaatgaggccgcggaaccattggagggtgtttggaaagacaagggaaaaataggcgatccgcaggccgattttttttctatcgatggtacggtgctgacttacaacaacaaaaattattttatctggagcggccagatctccgggaaagatatcacccaacgcatttacatcgccgaaatggaaaatccctggaccctcaaaacaggcagggtacagatttccatgccggattatgactgggaaaaacacggttcaccggtaaatgaaggcccggaaatactgaaaggccctgatggacagatcatactgatctactctgccagcagttgcggcacagatgactatgcactcggtatgctgcgcctgaagaaagacggtgatccgctcaatcctgcacactggaccaaagccggccagccggtgttcacgaagagcgttatcaacaccgtatttggtcccggtcacaatggcttcttcaaatcgaaagacggaaaagaagactggatcatttatcatgcaaatcctcatgccggccagggctgcggcggcgcacggagtccgcgtatccagccgtttacctggcgcgccgatggcactcccgattttggggaagcccttaatccttattataaactcaaaaagccctcaggggaataatactatggctgtttttttaaaagaagggaagagcgaagcggcattaaaagctaccgatgcccgggtaaaggaaacggtagagaaaatgatcagtgagatagaacagcacggcgacgctgccgtggtgaagtattccgcttccctggatcgctggtcgccacctgctttcctgttatcggcagaagctatccgggagattatagcacgcacaccggaccaggtgatccgcgatatccagtttgcgcaacagcagatccgtttttttgcggagcagcaacgcgcttccatccttgatatcgaaatagaaacactgccgggcatcttcctggggcataaaaatatcccggtcaacagcgtagggtgttatattcccggtgggagatacccgatggtggcctcttcgcacatgagtatcctcaccgcaaaagtagccggcgtaaaacgggtcatcgcctgcacaccaccgatcaacggccaggtgccggaagccactgtttgtgccatgcaccttgcaggagccgatgaaatctacattttaggcggcgtgcctgcactgtgcgccatggcaataggcaccgggtccatcaccccggtggacatgattgtagggccgggaaatgcctatgtagcagaagccaaacggcaactctatggtagggtaggcatcgacctgtttgccggtcctacggaagtactggtgattgcagatgaaaccgccgatgcggaaatggtggcctgcgacttattagggcaggcagaacatggccccacctctccgggtgtgctcatcaccacttctgaacagctggcccgtgaaaccctggtggagatagaaagacagctcacctttctttccactgcagacatcgccagggtggcctgggaaaataatggtgccgtgatattggtaaaagacgaagcagaagccatcgccgtagcagacgaactggccagtgaacatgtggaagtgctcacccgcaaccccggtgtattccttgaaaaaatgaccaactacggcgccttgttccttggtcctgaaaccaatgtagcttacggcgacaaagtgattggtaccaatcatacactgcctacccgtaaagcggcaaagtataccggcggactatgggtaggtaagttcctgaagaattgtacctatcagcgttgcacgccggaagccagcgctatgattggtgaatatgccatgcggctgtgtgaactggaaggatttgcaggacataaagcacaggctgccctgcgcgtaaagcgttatggaaaaaactagcccgttttggcctgcacgtataccttctggtattgcagcggcgttttgtgtgtgagcagtttgaactgccggttgaaattggagaggttgttgaatccacaggtatagcctacctgcgacataggcaggttgttttctatcaacagtttacaggcatagccaatgcgtacttccattaaaaactgccagtacgttttcagtgtcctggatttgaaataccggcaaaaggaattagggcttacgttggccgccgcagccacttctttgagggtgattttgttacggaagttattgaaggtataatgatagatcttgttgatgttatcggtgttgatgatgttgtaggaactggcaaaaccaatgctcgacagcagggtacagtcttttgaaccggcgatggtgtccagtatgttgagcagggaggtgatcctttgtacctgcccggctttgaggatgttctccatttcccggctgatcagttcacgggtaacgccatgaatccggatgccgtgcctggcttttgcaagcagttcttttattgctgtcagttccggcaggtcaaggaaaccggcgccccagaagtggtccccgaaatgtatggcaatggcttctatctgcaacccgggttgatcctggaagtaaatggcatcgctccgccacatgtgcggaagttcactgcccagcagcaccaggtcgccatcttcaaatctttccatactgtcgcccaccagccgcataccgctgcccttgcggatcagcgtaagttcaatttccgggtggtaatgccagtgattataaaggtaagggtagatgtcttcccggatgctgaacgaatagttatggccggtgtcaaccttacgcagaatcggtttcatacaacggaattatataatgaagctaatacaatttatgatagttgcaaaacacatacacccgctgaaatcatgcgtgacaacgtatttacggtatacctgcctgctggtgcttgtcctctgtaaatccgtgctgccgcttcaggcccagcgcctccccgtgatacctgccggcgccgatgcataccggatgtgggacaaatggccttcccaacggttcggaatgcgaacttatatgagaagcacctacgaccgctccggcagtaatgaagcggccgacgccagccactatcttttcatgaacggcgaaacggataacgttacattggatgtaacgggaacgggtatactttatttttttcgtaccaaccactggcacggaagtccctggcatttcactacggacggacagaaacataccataaaagaaacggctaccgaagatcctgtaaatgccctccggaacattaaagcaagcgccttcatcccggctgcgccgtttccccgcccgctggcctggacctggggcgacaccaaaggagcagacctcatctggacccctattccattccgggaatccctgcgcatcgcgtattcccgcacacactacggcacaggatactacatttaccagttgtttgccaacccccgcaatctttcacaacgcatcaacagctgggatatagaaaaagcacccgacaaagacgtagtagcgctgctcagtaaagcagggcaggatattgcaccggtacatataccaaccagccagggaacggtagcgctcaaccaggaaaaggtaacgttgacggatatacgtggtatggcggtagtaagggcccttaaattcattattccgcttgcagacgcggaaaaactggaaagactccgcctgttggttacctgggacgatgcctccctgccttctatagatgcgccgctcagcctgttctttggcgcaggtaccctgcacaacgcgggcgcccgggaataccttgtaaaaggctttcctatcaatatccgctatgatagtatccggcaaaatgtagtgctggcctgctactatccgatgccattcttcaaggcagcaaagtttgaactggctggtatcacacccggggagactttcattaactatgagattcgctaccagcaacagcaattgcggcccgcattcagcagctatttccatgctacctaccgcaattttccatcaccggaattgggagaagatctaacgttgctggatacacgtggaatggaaggcaaatccgaatggtcaggcaattttgttggcacctcttttatttttacacatagcggcgatcttggcacgctggagggagacccgcgttttttcttcgacgacagccaaacgccgcaggctcagggcaccggtacggaagagtggggtggtggcggcgattactggggcgggaggaatatgtcgcttccacttgccgggcatccctgcggcgtagcccggaaggagcaggcaaaagataaaaaagacctcatccactcggcataccgtttcctcctcgctgatctcatgccctttggacgcaatgcccgcatccagctggaacatggtgtggacaatcgctctaccgaacactatgaatctgttacctactggtatggactgcccgccccctctttgataaaaacagatgaactggatatcggtgatccgggcagtgaacaacaacatggctattattccctgcaggcatctccggtagaatccattgtttcccgttacgaactgggtgttgattcgcttatcattaaaggacagggcagaaaggaaatctaccccgtacacacagaagatggccgttataccaccggggtgtcggaattcaccatccgcctcgatcccaccaacgttggtgtgctgctgcggcgtacactggattacagtcaccctaatcaaaaggcggcaatatatatcgcagacgacaacggagacaccacccatcttaaatggaagcccgccggcacctggtacctggccggcgccaatacctgcatgcatagcaatccgccaaaagaactggataaaagggtgtacgaagtgcaaaccagtaaccgccgcttccgcgatgatgaatggctggttccggccgcccttacaaaaggacgcagccgcatcagggtaaggatcgtatttgtaccggtagaacaggaactatacccgggatttaaattcccggggaaaaacgcatggagtgaactgcgttataccgcctatagctatgtggtgcctgattttaaagattaaacatcttccagcaggattttcaccatgttcttgtaattattgataaactggtgagagatcttataattttctgtggcggtataactggttttttggatcccgttttctgtcagctggtaaataagggcatcggggtaagccattacaataggggaatgcgtggcaatgataaactgcgactgctgcccgatcagctggtgcattcttgtgagcatggccatttgccgcgtaggggaaagcgcggcttccggttcatccagtatatacaggccattaccggaaaagcgatgcaccagcaaagaccagaacgcctccccatgtgattgctcgtgcagggacacgccgccgtaactgtcaatcacccgccggcccatgccttcccggtccagttcttcaatgttggtacccacgttgaaaaaactctcccctcgcaggaaaaagccatcctttgcgcgcactgccgccctggctacccggatgtactgatgtaacacggaatgggaagcacgcgtggaaaatgtgaagttcaatgatccgccttcggggttaaaaccacaggccaccgcaatggcctctatcagggtggattttcccatgccgttttcaccggaaaggtaggtaaccttcggatgcagctgcagggttgaaaagttttttaacgcgggtatgttgaaaggatattcccccggtgtggtgatcttgtccctgttgagtgtaatggccgttaatcccctttgtgtaagcatagccttgcctgttagtgtagttgttaaaagaaagtaacctttccgctgttcatatcgtaaacgccgcctgtaatgatcagttgcttctttttttccatttctgcaataatagggctatttttacgtatattctctaccgttagccttacattttgctcgcaaacggcatgtacatacgactcatttttgctgttcatatctcctttaaattctttgatgctggtaactgccggccgtatttttgacagcagcgcggttatattgcccagttttacattatcgatggccgacttaatcgcgccgcaatgctcgtggcccaataccaggattacctttgcaccggatactttgcaaccgtattcaatactgcccagcatatcttcattcacaatattccccgccacacgcgccacaaacacatcgccgatccccctgtgaaaaacatcttccacgggtacccttgaatccaggcacgacagaatcaccgccttaggaaactggctcaatgccgctgcccttaccctggaagaagtattcctgaccgttaagcggtcatttacaaagtcctcatttccctcttttaaaatatcaagcactctttccggcgtcaatgactgctgttcgttggacgacagtactttattttccaacacatcggtgctgtctatagcaacctccttttttgtactgctggtatcgctgccttgttgtaaccctttttcgttgcccgggttgccacaggcgtataccaacaagaggagcatgataacagataattttgcaggtatcttcataatttttttttagatgattaacggaatgcttggcatgtataagctaacaatccggcaaataacattgttttattttccggaaagataagcgaataatgatcacagccttgtataaaagtacaacgcccgcgcttggcgcaggcgttgcaggttatggtaatgtatcgtttaaaacaatggtgtaaccagtttaataaaataaacagtattaaaatctgttttgccggtaagcggcagtattttctggatataggtattgtctaccggatcggggggaacgatgccaaagtcatcgtcgttgctcactgccagggtagtgctgttcaccagtacaataccttccggtttatcatgcgggtaaccggcgatatctttcaacaggtcaaccaccagcgatttggaaacggttttgatgcctgcagcctgcagttcttcatcggtcagcacttctactgttttgccattcaccagcttgccgcccgcgccgtcgccggcatcagaaatatcagtagctgccgaaaggtcgattttatagattcttttgatcagcgatggtttaaccggatcgccggggaattcaccgtcgcgctccagcaccaggaaggtactattgctgatcacggtgatttcgctgttagcggtatttttgttttccagtttatagaggtattgcttagtttgaccggaggcgatatcataggtgaggatgcgggtaaacagggagtttttcaccgcatctttggtaggattgtataagggcgactgcataatgcctaccagtgttttgccgtcaggggtaatggtaagcccttccatgccacgattggcgcggcgcatcgcaaatactttagggatcttcctgccgccggtgcctgtaccaaaaggattgatcctttccagtgttttgccgcttctgtcgagatgcaccaggtgcggaccgtattcgtcactcaaccagaaagtaccgtcagctgctaccgtaagcccttcacagtctatgccttctgcatctacaggaagtgttttgccatccttatccaacgccgtttccccggtaccgcctgatcctgcaggattgggaagccccgttacgggtacgtttgcagcagatttgatatgaatggtttctaccagtacgagcgagtcgccattcagcttgaattttccgatctgtggattaaaccccggtacggcaaatactttggagtccttgatgataccgtccgcattcggaccgcggtcggtcatcaggtaaaaataaccaggctgcccgggcacgtttgcaatagaagatccataaccgccattgtaaactttcacaccggccatgttggtggtcattactacagcaccagccagggtggctttggcaggataagacgtattgttgttatcaggaggggtgtcgtttttctgacaggcaaaaaggaacacaaatcctaatggagcaaagtagcgtactacagtcatagtggttgatacgtttaaggcgcaaatgtgccctttccgtatgaagactatgttaccgcaatattatcaaatcgtgaaattgctattcctttttgggttctctttctacggtaatgctgcactcgccgatcagtgccgccagtgcgccaactgctgcaaaaacgggcgccagtaatgcacccactacgccaatggttagcgggaaagtcatcagctcctttccttctttatctgtaatggtaatcttccgtacattcccttcagcaatcagctctttgatcttttttaagaggttttcgccgtggagggtgaaagtttcttttgtggtcatagtctacaggtatttgtcttttaaggtactaatatttggtgggataacggtgatgttcatacatctgtcagctctatccacaccggcgcatgatcactgctcttttcccaaccgcgcacatggcggtccacgccaccggcaacgagacggctatccagttgcgggctcagtaaaaagtgatcgatacgcaggcctgcatcgcggccatatgcattacggaaataatcccagaaggtatagatcttttcatcagggtatagtttccggatggcatcagtccagccctgatccctcaggttcctgaatgcttcgcgcgtttcggggcggaagagggcatcatccacccaacgttccggtttgtatacatcctgttccgtgggcattacgttatagtcgcctgtcagtaccaccggtgttttggccgccagcagctctttggcatgcgccgtgaggcgtttgaaccagctcagcttataatcgaacttaggaccgggagcggggttgccgtttggtaaataaagacaaccaatggtaacgttattaatttcggcttctatataacggctgtggatatcctcgggatctccggggagcgctcttcttatttctttgggttcacctatccgggaaaggatggctacgccgttccagcttttttgtccgtgccagatgggggagtaacccgcatcgcggatagcctgctccggaaatttttcaggaggtgcttttaattcctgtaaacaggccacatcaggcgccgtttcctttaaccagcgaagtaataccgggagacgtccgttgacgccgttaacattataagtggctattttcatggatgctgtttattcatttgggttcgtaattagcaacacaatcacgctgccatgtgctttgtgaatataggcaattatctgtttccgtttgccccggcaaagggaaaaaacttacttttgtaacctgttatcaacaggggtagcaggttttataaataacggaacatcatggcaaagaagcatacatcacaaccacacatacaccagtcgggctttcattttttaagtaaattaaaagagaataacaacagggactggtttaatgcccacaaaacaacttatcagcaagagctgggcctggtagaagaatttgcagaagcactgctggccaaactttcggtgcatgacctgatagaaacgccctccgggaaaaagagcctgttccgcatttacagggacacccgtttttccaacgataaaaccccttataaaacacattggagcgggagcttccggcgcgccaccaaattccgcaggggcggatattattttcatatagaagaaggcaacagcttcgttgcaggcggattctggggtcccgttccggaagacctgaagcggatccgggaagaaatcgcgtttgatccggcaccgctgagaaagatcctcaacagtaaatctttcaaaacctattttaaaacactggagggagaacagttgaaaactgcgccgaaaggttttgccccggatcatgaagcgatcgacctgttgcgtcataagcagtttgtactggtaaggaagttcactgataaagaggtgttgagtgcagattttctgaaagaagtaaacctgacctttaaagccatgcgcccgtttttagattacatgagcgaagcgcttacaatggatcccaatggtcttacggagtaattgccctcgttgaggcagttgcctgttattttcatacattcaggtatggacaagctacagcaggccatcaacgtttttgataaacgtgcggtccaataccaggataaatttatggacgtagcattataccacgattcatttgatcttttctgcaacagtattcccaaacaagaggcggctgttttagagatcgcctgtggtcccggcaatatcaccaaatacctgctgcagcagcggccaaacattcacgtgctgggaatagacctggcgcccaatatgctggaactggcccgcagcaataatccgtccgcggagtttatgctgatggatgccagggacatcctccggctgaacaaattgttcgaggggattatgtgtgggttttgcctgccatatcttagccgggaagaggccgtgaaaatgatcggggatgccgtccgcttactggcgccgggtggcgtgttttatatcagcacgatggaagatgattatgccagatccggcattcagcgctccagtgcgggcgatgagctgtatatgtactatcatcaggctgattacctggtgaatgctttgaaagaaaacgggtttaagataatggatcttcaacggaagcaataccccgccgctgatggaagcactacaacagacctgatcatcatgggaggactataacctgttgagaagaaatttaatatcttacagcttaaatcatctctgtgaccaacgatatttcctccatttttgacaaagatttttcaggcgaatcagccgttcgccgccgcgatataatgccgcttgcgctgagaatatatgcctgggtttttatggtttcttccatttattcgctgttaggcaactgtttccggtatatccggtatcctgatgtatttaagttgaatgaattcagtcttaccgtaatattttctattgccactgccgtgttgcttccgctgataaggttcctgcctaatcttttaattttgctggagaagaagtacgctatactgttatccctggtagcggtggcgatttccatactggtggggtgctacagctcttacattagtatggctcacgggatgatgggctacgtggtagtggccacgaatattttctggttgttagtagatatcccttatctcatgatcctgctaaggatcaggaaggactgggaaaagggcatgggtcggcctcagggaatataaggtccgcccggttctccccatccccacttcggcatcggttcatccggcttcaggggcacttccgtttccctggagttgattacggctatacgtgttccccattcgatatacgccacaaaagcagacctgaattcgggatcatccgggaggttcagcgtgtcggccgtttctatcagcagttgcacccatcttttccggtgttgctcagtgaggtgtttcccgaggtgtttttggatcatcttaaaatgagagccatcttcttcactgtacatttttggtccgccgaaaacttccgcaataaaatgcgctacatgcaattgatgtgaaggcgacatatgccggaatacgggcgctaataattcatcctgcaataccttttcataaaaggcattcatcagcttttcaaatacgggcataccgccggcccattcgtatagtgtgggaatttttttctctgaagtcattaccgggtgcttgattatgctaaagataataattaagcagccaagttagcaggagtaacaatgcaaaacaagcgcctaccaaaaagtaggtggggttattcacccggcgccgggatgaagcagcaccgggtgaaattattttagttcatcagcttctcaatagaattgtatagcattgttttattaaaaggcttctccaggaacagatctgcaccgttagccagcgccacatcctttgcagccgcatccatccctgatatcatgataatcctggtggccggatatttttccttgatataactgataaagtccagtccgtacccatccggcagccggttatccagcaatacaatggctggtggctgctgttgaaaatattccacagcatcggaaattgtttgtacatgctctatctccatctctttcccgtcgagcaataaattgatgagcaaacacatttccccttcatcttccactatcaggagcttctgtttgggcgtggtattcgtaagattatgttccataaaattaatttaaatgtaattattgacgcgggataaaagtttaaaaaccgtaccaaagcaaccggggatgaattatctttacaaatacctttatcaacggttaatatatttcaatggaaataaaagatttatcaccaaaacacttatggcagcattttgctgaactgaacgccgttccccgcgcttccaaaaaggaagaaagagtgatcgcttttatgatggatttcggaaaacgtcttggcctggaaaccacaaaagacgccatcggtaacgtagtcatcaaaaagcctgcaacccccggcatggaaaaccggcaaacggttatcctccagtcgcacctcgatatggtgcatcagaaaaacagcgataccgtatttgactttgatacccagggcatcgatatgtacgtggacaacgactgggtgaaagcccgtggtaccacactgggtgcagataatggcatcggtgtagcggctatcatgtcggtactggcggcaaaggatgtcccgcaccccgctattgaggccatgtttaccatcgatgaggaaacgggcatgaccggcgcgaagcaactggaccccgttaacttttccgggaagatcctcctgaacctcgatacagaggaggaagatgagctgaccatcggttgtgccggcggcatcgacaccaatacaaaaggcgtttataaggaagtgcccgcaggtaaaaacgccatcgcatttcaaatcagcattaaaggattactgggcggccactccggtatggaaattcataagggcagggccaacgccaataaggtgatgaaccggttactgtataaagcagcagggcaggtaaacattcagctggccagtttagatggcggaagcctccggaacgctatcccccgcgaatcacaggccattgtggctattcaggctgcggataaggataagttcatgaacgttatcagtgaatttgaagccactataaaagaagagtataaaaccatagagccctccttcgtactggaatgtaaggaaacggcgatgcctgcgctggtaatggaccctgcctatctcccgcagctgttgcgtgccatctacgcagtgcccaacggtgtgttccgcatgagtcctgatatcgccggactggtggaagcatcctccaacctcgccagggtacaggcaaaagaaggtgtttttatcacacagtcgctgcaacgcagcagcgtggaaagtaccaaaagcgatgtagccactgccgtaagcgccgcattcgaaatcatcggctgcgaaataaaccagggcggcgactaccccggatggaaacccaatgccgattctgcaatactccggttattactggccttgtataaagatcatttcagccacacgcctaacgtaggggcctgtcatgccggcctcgaatgcggtatcctgggcgcacacctgggcaacccggatatgatttctttcgggcctaccatccgcggcgcacattccccggatgaaaaggtgcagatctcgtccgttggaaaattctacgattacctgctgcatattctccgggaaataccggttaaataaatgtagagaataaatgttgtggttgtccgcttccgggcaatcactttcccttcggcatataacggaaacggatcatcgcattttctgtttctgaagaagtaacttttagttcatagcgcttgtcgctggttaaaataaccattttagaggtgttgggcggaatatcgccgaggttattggcatgtaataccagctcctggtattcctgtgtgctatctgctgtaagatgaatgcgcaacgggctgccggtaagctcctgccggtcagccacttttaccccattgaaaaatacggttacggtatcgtgatcaacggtgccgtaatcatacaggctgatatctatacccggactgctgatatcatagcttccctgtacccggtttttccgttccggcgctggtttcgctgcaagtggtactgtatctggtttgggtggaggagtagcctccgatggaggaaatgttttcccgctgccgggaatttccagggcagcaattttcgctccgctgagcttcgataaccgcagcaccctcttcgtatgcactttcccggtgtactttgaatagctgatcatgcttccctgcaacactgtttctccatcaatatcaaacaatttcaggctcatgactgccagccgggcgctatgatttttggggatggtgagctggttgaattttatctcttcaaaacgccagttatcggcactgtcgtttcgttggccggtcaccgttagttcgccgtacaattgcggtgtttcgtaaaaccaggcagtgccggtgtatttcccggcggcggtttgttttatatccataatgtaactgccggtgccataaaaccatccctgtgattcggcggcagcgtagcctttccatacgccttcgagattttgcgcacggagtgcggcaaacaggaggagtccgcagcaggtcaacaatattgttttcatccggttggttaacatatggccttaaagataaggtttctacgcatgcgccggcaatgcggttactggttgtaaccgttgttgccggaaaaggagcccgccaataacgatggttaccaggccttgtagcaaaacggtgtttggggtacctatccattgggaaatagcgcctaccagcagtccgccgagtggctgcatgccgaaaaatgccatcgcataaaagctgatcacccggccccgcatcgcagggtctacggttgtctgtatcagggtattgctgatcgtgatttgcgacatcatgccaaaaccagctacggtggcaaatatcagtgcaacaggataaatggtggagtgggaaaacaacacaagtcctgcgccgaataccagtgtgttaaacgccaggatcttccgcaggtttttccctggtttcagggaagcgaggaaaagagctccgcaaaatgcgcccatcccgatggcgctgtctatcactccaaaggtggaagcattgcccttgaaaatatctttggcatacaccggcatcagcgtgctgtaaggcaataccagcaggctcacggaagccagtgtgactaatatcagtgaaatagccggagtggcccggatataggcaaacccttctttcagctctcccagcatattggtagtacgcactttgggcgtataagcgggcagcttcatacacagcaacgatcctattacggcaataaagctgatggcgtttataccaaaacaaatgtcttctccgaatttttcaagcgccagcccggcgatgccggggccaatgagcctcgacaaatttaccatcgaggaattcagcgccagcgcattgggaaggtccgctttgttctccaccatttcatataccagcgattgccgcgcaggtacatcaaatgcgttgatgagccccaggaaagcgcttagtccaatgatctgccacacctcgtagtgcttaaagtaaatcagcaccgttaacaaaacagcctggaacatagatgcaaactgggttatcagcaacagcttgtaccggttataccggtccgaagccacaccgcccaggaaggaaaaaacaaaggaaggaaacatgctcgcaaaaagggtgagccccagcatgaacttggaatgtgtttgcgaatagatcacccagctgaccgcagttttctgcatccaggtgcctatcagcgatatggactgaccactgaaatataaccggtaattacgactcttgaaagcattaaaagtgctgatgttcatgttagttccccgcttttattcgtactccaccaatttggataaaggcccgatggctgccagcaggatcgcctgctcttctttagtgcaaacctcgctgatcgccttgcctaaccattcgtcccgctctttccgtacccgctcgatccgcgctttgcccgctgccgacaaggaaatatgaatcttccgcttgtcgtggggagaggccgtcctgttgattaaattcagctggaaaagatgctggagtaattgtcccatcgattgcggcgtcattttctccattaccgccagttctgccgacagcaggtaatcgtgctggtccagtaataccagcacagaacgctcactctgcgatagctcctcatttgccggcgatagctttcgcagctttctcaccagcctggcaagaagtggacggagttgtgcggcaagttggtgcggatttccggaagccatatagtaaggtaaagttataagtttaccttacaaatatagtaaattatttccggagaaaataaaaggaatagttacttccctgagaaacggcttagcgtttcacgcgatacgccaagataggcggcaatcaatgttttgggaacccgttgaaaaagcgccgggtattgtgccagcaactgttcgtagcgcgactgcgcatcattgttgagcagcgacaggatccgctgctgtgacgccacatagccggaagtggcttttacccggaaaaaatgctccattttatgggaagcttcacagagcttttttttattttcgaaagataaacacagcagggtagatgcttcaatacaatcaatgttcagctttgcagttgtttggtttacgtacgcatggtaatcggtgatccaccagttttccatcgcgaactggataatatgctccttaccggcttcattaaaatatgccgcttttaacaagccgcttaccacaaaatattcatgtcccaccaggttgccctcctgcaccaggaactggtgcttacgtaatttcttttcggtgaagtacgactgtatatgatcgaattccgtatcggtgagtggggagattacttcaatatgttgccttagcgcattactcataagatacaaattaacataaaagctgtgacctgtatcacaattaaatggtgatctgtttccttttgcaacatatttataaataccaactttgtgcaaaaatcaggtaaatgaaaactaaaaaaacgggcttattgctgttactgttgccctttctggcttttcaggcatatagccagcatacaaaaacaaataatcatcagtctatgaaaaaaatacttattgtggtgacttccttcagcgaagtaaaaagcaccgggcataaaaccggtacctggatagaagaatttgccacaccctactacctgtttaccgataaggggttccaggtaaccattgcgtcacccgcaggtggaaaggcgcccattgatccaaaaagcaccgcacccgattatagcacggcatcagtaaaaagatttttcaatgatccggcagcccaggaaagattgaatcatactgttttgttgaaagacgtgcaggcagcggattatgatgctgtgttttatcccggcggacatggccccatgtgggacctgtcagataatgccacctccacgcagctgatagaaacattttatgccgccggaaaacccgtggcactggtatgccatgcacctgctgcactgaaaaatgtaaaggataagaatggcgcgcctttggtaaaagggaaaaaagtatcggcattcaccaacagtgaagaagtagccggacaaaccaccgctgaagtacctttttctttggaagatatgttgaaggagcgtggagcaaactatgtgaaaggggccgattggcagccctttgcagtagccgatggtaaccttatcaccgggcagaaccctgcttccgcacagttaacaggcgaaaaagtaatcgcagccctgggcgtgaaataatataacaatagtaatagaaagccttcagacatatacggtccgaaggctttctgttatcaggcaaccaccacgggtggatgcagtttgtgatagtaaacataggaaaccaccaggcttacaaaaaaagaagtatgacctatttccagcaatacactgtcgccgcttgataaatgcgccaccgccgcggaaatcagggttatgccaaacccgaagtaggcgaactcccggagcttcggcggcgtaaagggcaacaacagcgccagtgagcccagcaccttggcaatggtaagttctatccggaaccagttgggcagccccaggtgagcaaaggcgcctttcatttcaggattgaaagcaaaattaaaggcgctccataacattacgccggtaaggataagtgtggctgtccagtaaatgattttatcttttttcatgatgttcagtttgatcagttgaatttgtaaacactcaacaggatgatgatgaaaacgaaaagtaattgtatcgtgtggaacaaacggatgttgcccctgatcttttgaacagtgccggcagatgtttcaaaggatttctttaactgctttttctgccgctgtccgaaaaggaaggtgttgaggataataacgatcaccaggccaaacttcacccggaaccacaactgctcgccaaaaacaccatgcgtcatgtacataatgcctatgccggaaagaatgatcagccctattcccactctcattaataccgggaaaacagagatggcctgcattaccgtggcggctttgcttttatccacgtcgtactgcttccagaactgccggaagcctacaaaatccgctaccgaagtaccggcgaagagaagaaatcctatgaggtggagcacaacgaagccctggaaaataatctgtgttgacatctgactatgatttttatatgacagaatcgaaataatataagtaaatgtataacggaaatatagtaaaaacaaaaaatccggagtattttttatattattgcttcggaaataaaatatctggtatgaataaagccgtagaactgatgactgaatggggagcgtttgatgatcagcatccggaaagcagcattgaagaattttgcaggcattacctggcacgcaaacaaacacggaaagcggttccgccggaagggaagtttctgccggtacaaagcgaaggcgttttgatgcgggtaataggaagaatctttaaactacacactatttacacggtggcggcgctggacggcaccggtatcaacacaatcgatgaatattcattgctcaatacggttgcccagttaaaagaaccccggaaaacagaagctatctacgcggcgttgcaggagctgtctaccggcacggataagttaaaccggctgaaaaaactcggctacctcaccgaatatgacgataaagaagacaagcgctccaaacggttaaaagtaacgcccaaaggagagaaagtactgatccaatgcaggcggcggatcagccagctcgcggaagtaatgttccacgacatgaccgatgatgaccgtaagttatgcgtgcagctcctgaaaggcgtggaaacaaaattcgccggtatctggcaatcgcacaaaggaaaagattttgaagaaatctatgcggagatcataacggataaaggttagtacttcatatcaaaccgcccgtcggtcatacgaacggtatcacaacctgctgttatcagcgtacaggtaaaggtgccggcaatgactttttgctcggtgtccagcttcgtgataaccagctgtccttcctgctgcacctttgccgcatccatgccaatatactcacaaccggtattggtgcgcattagcagccgggtatatacaaaggctacatccgtcgcaggcgtggtaacaggataagttcccgttttatttaagttggtggcgataatctggaaactccgctgcacagagtcgccgaagtcgaaccgggtcatggatacattaaaacttccgttcctggtactagggtcataatatgcggagggattgggcaggcctacacttccgcgtggaatgaacaccttcccgtttaccaggctgccaatagtatttttaccttcctgtgtgatggagggcagcgtatccggaagggaggaaggagggatcacggttccccggccgcagtgaatactaaacagggaaaaggaaagaagcgctatacagaacagttgtttcatgggtcttattaagaggatatgaaattaggatattctctaaataaaacgggaagggccggcaaaaattgccagcccttctgagtcattttacgtttacttatctacatccatgcagtaagtaacgcagtgccatactttattaaaatccttgccttcatgttgtccgctggcttcttcggtaaaagtaccttccagcaggtagcggcctgcccatgcgggtgaaaaagtaacatcaccagcctgaccggctttgaatttcttagtccatccctccggcgactgtacgattacttcaccggcagcaggaacagccttcttatagcttaactgcacggtggccggctgatgcagcttgtttgcttttttgagattcgtcagcatggagaaatccgtatgttcttttgcgttgtctgcgccggttaaagtattgttgactttcaccagccccatcgcataataatggatcttactgccgctgtatacttcctgcacggtatgatcaatagctaacaggtgtgtgccggcaacagcaggcgtaaaggtggcggtgaagtaattgccgttggcggtacaggtcagtttctctttttgtccgtcgggttttaccaggtacagtgtaaaatctttcatattactgaaccagtgctgaatagaatcgcgctcgttatcggcatattctcccaggaaaactttcacttcctgtgcctgcccgatcttcccggtagtaacggtttcgatccagatagcatgggcaaaaagtgattgaaggctacagcataaaataacagaaaacaggaatttcttcattatatcttaatttataaatggcgcatcatctgcaatgcggcaaagctatgccggcagagggccggccggtaagcgaaaagggaatattatttacgcaatcgggaaaaattaggcgctaatttattgaaagagcgcttcattattccgatggcagtatccactgtaatccttttataaaggtaggcagctgcgtatccatatgtcccaggttggaataaacatctccccggtaagtaacctttggggagatagaagtcgttagttgcaccatcagtatctgcagggataacgccccggaatccccggcctccggttcctcctgccctccgaatgtaaagtaagccctgacattcgtccgcatgctgtcctttccccgcgctgttttcagttgctccggcaaatagtagtggttataatgtaatgccgggctcgccgcaatatacccgctgaaaccggtggaagcgcccgccagatcacggtaaagcgcatacgccgtaaaataaccgcccagcgaatgtcccatcagtacgcgcttcgtggtatcggtgcgatattgccggtctatcaccggtatcagctccctgtgtacaaacgacaggaatttatcggcgccgccactggtgctcatttcatattccgggatggcaacaggataggtgtcatcccggttccttaaggaatccatctccggaaaatctttataaccaatacccactaaaatcacattcggcgccaatcctactccggcatatttattcagggtaactgccatcacatcaaaatacaggttggcatccaggaggtataccaccgggtatttttgagattgctccggatggtaatcatccggaaggtttacgaagatagaaaaggaatcagccaccgcttttgaatacaggcgcatcacggcagttttgccttgctcgtctgccacaggcgcacatccggccattagcagcaatacaataacgggagtaacataacgggtcatggctgtgaatttagatacattctaaagtatcacttatttctgtttacaaaatgttatatttaaactcatcttttcctgaacaaacaacaaatcctccatgagtaataccgcgaatgaaagagccgccatgccaaaagatagcagcgttttagacagcaggagtttgcagaacagctacgccacgctgataccactgctcagggaaggtatgcgggtgctggatgttggctgtggtacaggcgccatatctgccggtatcgccggcgcagtgggtaaaacaggaagcgttgtgggcatcgacagcagcgcgcacctgattgctaaaggaaacacggatcacgcggatctttccaacttaacactgctggaggcagacctgttcgcctacaatccggcagaaaaatttgacgtcatcgtttctgcccgtgtgctgcaatggttaagtaatccacgcgaagcactgctgaaatttaaatccctgctaaacccgggcggctatatttctattttagactacaaccatcaccagctggaatggacgcctgcgcctccggaaagcatgcagcgcttttataaagcattcctttcctggcgtgcagatgcaggcatggataatgaaattgcggatcacctctcggggctttttgaagaattgggctttcatcacatcaccgtgttgaacgccgatgaaatatacacccgcggcgaaaataacttcgcagaaaaggcaggcatctggtccaaagtagcggaactaagaggcccgcagatggtggaaagtggttttatcacagaagaggagcgcatccgtgtcgtcacggattaccaggtatggatcgcggagtcagcgcaaaagatggtgatgaaattgaaagatgtgcaggcacggattactcccctacatacgcactaaacttcagtacccggtccttttcaatggtaaatgcctgtccgcagtcggcgctgtaagcggaaacaccaccgcgggcttcgtccttgtaggtaataccatagcaaccactggccgtggacgatcggatcaccatcacataactgcgtttggccgctaccgttatatgcggtttgatagtaaccggctccggcgaccagctcaggctgtcgcggggaatggccgcctcatacagcgcttttcctgttgccggtaatcccttatcatctgccgggtaaatgctgatatgcaggtcgtcgtccggatagccgcttttaaaagcagtgatgcttacagccgtaagcacgcctgagcgggtaggagtaaagctttgcgaacgctgcatacatccgttaatgtcgcactggaaccggaagccttcctgcccgctgctgttgtcgggcttcactttcataacaggagtcgaagcagcgcgcaagggcagctgtatgctgtctttacaaacaataggttcaatagcgccgtctgctgcaaaggaaagcggcgcccagtaataattagccagcgcttcattttttgccgcattgttccacagatcactgccatacaggaaaacgctgtcgccgttgagcttaataagagatacaaaagacggttgtccaccgcaggatcgatcgctgatctttattccatcggaccatgggcccagcggcgattccgcacggcgataagaagtaccagtacctgcacaatagccgcaattaggatcggagtacaacaggtagtaactgccgaagcgccggaagagcgccggcgcttcggtattgcctttcgtcactgcttttacatgctctccgctgccagtcagataatcggcactgagcttttcaattacaatggtgccttttgtttgccagtcggtatacgcaatataagcggtgccatcttcatctacaaaggtatcatgatcaccgttgttcaacccggcgatagcgccgttgctgttcactgccatccggggctccgccacttctgtaaacggaccggtgggttgctggctggtaaatacgcggaagccggtacggttatcatatacattgatccacagtacatactgttttgtttttttattatagatcacatgcggcctgaaacagccataggtactgccattacagcgggtttgccataccggtgtgcgggcgttaaataaaaagcctttgtcggtccactgctgaagatctgtagaagtatatactttaaatccgcaaaagggagcctcttttctgccccattcaaatccacagccatagctggtaccatagaggtaataggtaccgttgaaataagcgatttcaccgtcgtgcgcatcaatggctgcgccggcagtactgaagcggatagtttgttgttgctgcgggttgaagttaacaagcgacgaattcgtttgcgcatgcacgttatacatcaataacaacaggcagcaaaccatgttaaatatcgccttgcgctcttttccggtattccgtgggcgtaaatccggtcttctctttaaagatcctggagaagtaaaacgaagaatcaaacctgagatcatacgcaatttcttttacagatacagcgggatcattcaatagctccctcgctttctctattttaagttggatataatattgaaacggagatagccccgtgtattgcttaaacgcttttctgaaccaggagtaacccacctgcaactcttctgcggcctgctccggggaataatgccgggaaatgttggcgcggaataacagccgtgctttgttcatcagttcttctctctctttattcccgcttgcctgttgcttcacgaggtagtggatgtttcccatcaggtgaagcgctgcgccggcaatgagcggctggtagccagggcgctcctgttttgttttttctataataagatgaaacaactgcagggtaccttcctggtaaccgatatataaacagggcttttccctggtgaaaaagttttccttcaggaggttgtcgagcacagggcctttcatgcctacccagtattcatcccagccggtttcggcgagtggccggtagcggtgcctttctcccgggaacagcaggataatggtaccgccttttatttcctgctgccggcagctgtcggactcaaaaatgcctttgccgccggtgatataaataacctggtattcattcaatacccttcctttcttccaattaaaatgatgatgcgccggatgatctttccccgggtaaatgcccgctgctgccacctgcgtacaaccggtattcagtacccaaatgccccagcgctcatcttccctgctcacgggcagatacttgtaatagttcatcataacgctttcttctttatataaaaatataaaaagccggaaaggtttcggaaagtaataagaatttccgccacccgccgggattgtatcataaagtacaaccgaaatatcaaataattcatcgcaccgcgactagctttatcacaggatccggttaccattcaaaaaattgcgttatgaatacattaaaagtgggcctgtttgggataggcctcgctgcctattgggaacagttcgaaggactgcagcagcggttgtcggggtatattgatattgtgcatcagcagttgcagcactacggcgccgatatcgttcacctcggcctgatagacacgccggagaaagcttttgaagcgggcagccgtttccggaaagaagacgttgatctgatctttttatatgtaaccacctacgcgttatcttccacggttttaccggtggtgaaacgcgcaaaggtaccggtgatcgtattaaatctctctccggccgcggccatcgactatgccgcatttaatcagctgccggaccgcaccaccatgaccggcgaatggctcgccttctgcgccgcctgcccggtgccggaaatagccagtgtattcaaacgtgcacacattcctttttaccaggtaactggtatgctgcaggatgatcctgtggtgtggaaagaagtggaagaatggatcgccgccgcaaaagtagcccacaccctgtatcacaacaggctgggcctgatgggtaactactacggcggcatgctggatatttactccaatcttaccctgcacgcagccgtgttaggcggacatatggaaattattgaggtagatgaattatcaggactccggaatacggtcagcgaagcggaaattgccgcgaagctccgggaagcgcaacagttgtttgacatacaacccgattgctcaccggaagaattgcaccgcgctgccaaaacagcggtggctttggataaactggtggcaaagcaccaactgggttccctggcgtattaccataaaggaagtggcaacgctatcaataaagataccatgagctccgtgatcatgggtacctctctcttaacggcacaaggcatcccggtagcgggggagtacgaagtgaaaaatgcgcaggccatgaaaatcatggacagctttggtgcaggtggttccttcacagagtactatgccatggactataaagatgatattgtgctcatgggacacgatgggccctgccatcctgtaatcgccgccggtaaaataaaactgaaaccattacaggtatatcatggaaaagtaggaaaaggattgtccgtggaaatgtcggtggcacacggcccggtaacattactgtctgtagtggaaacagccgatggaaaattgcagttcctcctggcggaagggatgtcggaagccggccctatccttgaaatcggcaacaccaacagccgttaccggtttcccacaggcgccaggaatttcgtggaagcatggaatgcgcacggaccggcgcatcattgcgcagtaggcaaagggcatatagcgtcaaaaataaaaaagctggcggagttgttgggagtggaggcggtgcaggtctgttaacaccgcaataatcgctgtatatttattcaagttttacaagcggtcacctgctgtatcaaaagcggacatattatttaaaaaataactttttaaactattggaacgtatgtaacttttggtatggcatgttttttcaacaggtgctgtaactgatactgactatcatgataagcaactacttcaggattgcatggcgcaaccttgtccgcaataaagcattttcttttatcaatatcctgggactggcgctcggactggcctgcagcctcctcatgatcctgtgggtacaggatgaaaaaagcatggatggatttcatgccaacagcgataaactataccaggtatatgtgcgccagtcgtccggtggcaaagtgaacgccggctatctcacacaggggccgctggcggcagaactgaaaaaggaagtgcccgaagtagaatactccagcggcttcgaggtttttctgccagtaacattacgcgtagatgataaagtaatgaagatcaccggcgcctatgcaggcgctgattttttgcagatgttcagctacccggtattacagggcacaaaagcatctgccatcgataaaccaggcaccatcgctatctccaaacacctcgcggaattattttttggcagcccggaacaggcgctggggaaaacactgcgttatgaagacacggtaagtctttctgttactgcagtgtacgaggtgccggccaattcatcacaacaatttgagtacctccgcaactgggaagattttaccagggacaatgcctgggcaagaaattggggcagctttaacccgctgacgtatatccgtctccgtgacaatgccgatgcaggtaaagtagccgccaaaataaaagacttcgtttataattatcagcaacgcaacaacgattcctatactgaactgggtttacagccttacagcgaaaaatacctgcacggtgtattcagcaacggcatacctgatggcgggcgtattgaatacgtgcgcctctttaccctgctggccatattcattatgctcattgcctgcatcaattttatgaacctcgcgacggcgcggtcggtaaaaagagcaaaggaagtaggcgtgagaaaagtagtaggcgccctgcgctcttcccttatcatccagtttatcggagaagccatgctgctggcatttttttcactggttattgccctgttggtagtgatattactgctgcccgcgtttaaccagctcagtggaaaacaattggcattacccgtttcacaaccagtattctggggtactttactgggcctcacggtactcaccggcttcgtggccggtagctacccggccttgttcctgtcgtccctgaacccggtacgggtgcttaaaggcagccttaaatttggctccggcgctaccaatttccggaagggcctggtggtgtttcaattcaccctgtccatcctgttaatgataggcatgtttgtgatttaccgccaaatggattacgtgcaaacaaagaacctgggctacaaccggcagaaccttatctatattcctatcgaaggcgaattgatttccaaatacgatgtattcagggaagcggcaaccaacctgcccggcgtgctggctatttctaaaatgaaagagtcgccaacggtgatagaacatcataaaggaggtatcagctggtcagggaaagaccccaatgatgacgcctcttttgcggatgcggcagtgggatacgactttataaaaaccatgggtctcaccttactggagggccgcgacttttcccgtgcattcgggaatgactcagggagttatatcctgaatgaaagcgccgtgaaaaggattggttaccagcatccggtaggacagccattcacactcggaaatgttcccggtaccatcgtgggcgtgctcaaggatttccacttcaactccatgcacgacgccatagagccgctggtaatccgcctggatgaaaaacctaagtggggcaatatcctggtaagggtcgccgggggtaaaacaacaccggtgctggccggactggcagggatctgcaaaaacttaaatcctaacttcccctttacttaccagttctccgatgaagaatataccaagctttataaaagtgaacagatggtaagtcagctgtgcaactactttgcctgtctcgctgtattcatttcctgtctcggcttattcggactggccatgttcaccgccgcgcaacgtactaaagaaataggcgtgagaaaagtgctcggcgcttccgaatccagtattttcctgttgctgtcgaccggtttcctgaagccggtatttataggaatgctcattgccttcccgcttgcctggtataccatgaaccaatggctgaatcacttcgcgtataaagtaaacctcgattggtggatctttggcggggctgggctcatcaccatcatagtggctttagtcacggtcagcttccaaagcatccgggcggcggccatgaatcccgtgaaaagcctgaaaatggaataatcctacttattggggtgctatttccccattataccgctaaaaatgctgccacagcaatggcatgtggattgccggtatattcataaacgcaacattatgaaagtacttggcatcatcctcattattgctggtattgcaatgatcgttatcaggggcttctctgttcaaacagaaaagaaagtggtagacattggtcctgttgaaattaataagaaagaaaacagatggataggctggcccacttatgccggcggtatcgtagccattgtaggtgtggtactggtggtatcgggtaaacggagagactgatcaataacaataacgactatatgcagaaatgagcgcctcccccgggcgctcatttctgcatttggggtacgcctgccaaaaaagtgtggtaattcatcgtaatcagataaaaaagtatgcttttatgctaactccctgcaataattttatactatcgccggcgaaatatcgaaaccctttttattcaacatttacagcaacacaataactccctgtatgcgctgcatcaacaggtaaaggaacctttatgtctgcatagcatttcccgtcttttcaaccataaaaattccactaatgaacaaacaaacaatcacccggaactacatgattacaggaacattaatgctgctgctattggcagcctgctcccgcaaagaagcggcagtaacaccggaaacgactccgcgcccggtaaccaccgaactaactaacggtattgggaatggcgtaaacctgcagccttcctactacaacggcggcaatgtaaacttcgcatgggcgctgatgaaacagcaaacaaagatcaaaaccgtgcgcattgaaattgaaccaaccgtaagtattacgttggcgaaatcctggattcagcaggcaaagaacaacggctttgcggtgatcgccacttatcacaaagcgagtgtattgggaagcgacaatgccagcgaacttactgcggccgccaactggtggaagaataactacgctgcattgagccaggcgggatcatttactgtaaacctgatgaatgaatggggcagtcataacatcagttccaatgcctacgctgctgcgtataattccgctattgcgctggtacggcaggtatacagcggagctattattattgatattcccggctggggacaggaaacccgtaccgccgccgaagccgttaagggaacgaatggtaccaaaataaatgatgtgaacattatcctgtctacacacatttatcccggcgcctggaaccagggcagaaaccgtaccctcatcaatgctgatctcgatgaaatggctacttccggacgcccttgtatggtaggggagttcggcaccggctccggcagcgccaactggtccggcttaacgaattatgccaaatccaaaggatggactgtattgggatgggcatggaatggcgatggtggcagtctgaatatggttacaccctcctgggccactaatcccaccgctacttctttcagtaccaatagttacttcactactatttacagcctgctgtaaataacaacaggttttcaatatctacagccggccccgtggccggcttatttgttatattgcaggataaaacctggaagatgtcgacatccctgttggatcaaagcaaggatccgctgctcaaaactttcattgccggtagatcagatcccgcattgatgctgttgcagcactttgtctcacaatatgaaaaactgggaaagatatacctgtatcccaccaaatctatgatgggtatcggttttggcgataggcgggtagcatggatcacacagttgggaaagaattttgtgcacatcgtattcccttttgaaaaggcgtatcccgacaatttatgcttccagaaaattgcgcaggtaccgggcgataaccggcagtttaatcatcatttccgtatgtatctcccggaagatattaatgaagaaatacaacagtttatgcgcctgtcgctgttataaccggttttaagtatatttaggaagaaacctgtataaaatactgtcatatgaatcaccaccgccctgcctctaaaaatatgattgaatccatcctggtgctgttgctgttgctggctttgctgctggcactgtatgatgtgttgcggctgttttttggtattctcacatttgcactgatcttttccgtttctttccatcacctgtttgagcgcatggttgtttggttcaaaggccgccgtaaactggccgccaccatatatgcggtggcgttagttgccatcattgccctgccggttacttatttcattgccgcgctgagttcacatatccgggaagcattgcactggattggtaacgtgaaggaaaacggattgccggcgctgcccgaatgggtggttaccatgccatatgttggcagcgatatcgtggacttctgggagcatttgcaggaaagtccccgcgaaactttgtccaccagcgtacatgaacaacaggtaagagtggtgctgcatcatattatcaccagcggcgcaggtattctcggtgcagccggccaactcatactcggcatcattatatctgcatttttcctggtaagcggtgaaaaagcagtacggcctatcagggctactgcacagcacctgctgggacgtaaagatggcgccgatctgttgaacgctaccacgatggccatcaagggcgtgtctatcggtgtaatgggtacggctttcatcacagcggtggtggcgtttatcgggcttaaaattgcaggcatcccctttgcgcttggcttgtccgcgtttatctttttcctggtagtgatccagataggcccgctcgtggtttggatcccattaaccatctggatggctacacaaggtcatcccggtatgacgctcttcctggctatttacggtaccggcatcctgataggggaagccatcctgaaacccctgctcatcgctaaaagcggcaaactgcctttcctggtattattcctcggtgtaattggcggtatggctgcatggggattcaccggcatgttcaagggcgctatcattgtagccgtattctataccgtatttaattcctggctgttgcgtaaagacgccgcccacgcttcacatgctgcggaataggtagtatcttcgcccacaagcaccagatgaattatgaaagcggcaagtatcagcgatataaaaaaagaattaactaccctgcctccggcagagctgtcggccctgtgtttgcggctggccaaattcaagaacgataacaaggaactgcttacctacctgctgtttgaagcccacaacgaagaagggtacatcgccgccgtgaaagaagaaatcgacaaagggtttattgaaatggccggtgataaattataccacgccaaaaaaaggctgaggaaaatcctgcggataacgaacaagcatatacgatatactggttccaaaaccgccgaagtagaactactgatctatttctgtacaaaaatgaaactgtccggtttattatcttcctatagtgttcagttaaataacctctacgaacaacaggtgaaaaagatcaccaaaatagtgtctgcactgcatgaagacctgcagtatgattatctccggcagctgaaacggcttacaggcgaggactaaaatgcttcagcaaaattaatataaaagccctgccagttgcccggcccgaaacccatatcaaaccgcaggttggtattgttcttcgagtccacccttatccgcaaccccaggccatagctgagatggaatccttccagcgacagatcactatagctatctgctacccggccggtgcccacccatgcagccgcgccaaaaatattccatataggcgcacggtactccacctgtgcatctaccagcacgttatcccggtaagcgcccatatagtagccccgcattttactatcgccacccatctgggccaactcataaaatggtacatccccgttggtaaatgtagtagtagcctgtaaggccaccacatgtttcagccagggattgaagtacttgcggaggtcaatatccacccgggtaaactggtatacacttcccaggaaatcggggtgccagatcacagtgccaatggcataagcgcctttatagggattatagcggttatcacggctgtcgtacgcggtgctcagcccaatacctgtgctgaagccaccttccaggccaggatagttttcctttaccaggaaactgttactgtcgggcttcacactaaaataatccgatacggtaacggctacaccgccatagaaatttttaaaccactgccgcaaagcggtagcggaaaactggaaccggctgtattctacttcctgtatgctgtctttcgaaatatcatttccgatcccgtaaatatattccggttgttttttataattaacatagctcatgatcacatacctgttttcttttaagatcatttcggtagatacagacgcgttaatcctgccgttgctggaaatagtgaacacttccgataatttggagggttttgaaacggtatctttcctggagaaatgtaacaggttatatttggccagcccgaaaatatgcccggcctctgtagtgtaggagtagagcggcaccgggatgatcttgaacagtgcttcggcctttttattaaattgatcgaacttcgatattttcttttgcgtggtatccgccgggatgtgtgaagtatctgcttgcgccaggcccaacgaataactgcataacaacagcatcgttatgagtatggggcgatatggcgcagtaagcatgcagtatacgtttacaggatgatacagcaagaccaccgctataagccggtggtcttgttgtatttattaaacgcaccattcgtggcttttgttcaataaaccggttaaatcaggtttgttgccttcacaggaaaattttattttggagggtgttgatgaattaaagaggctttaaaatgaaggcatgaaaattctatttgaaacgccgcggctgcaggtccgcacttttgccgctacagatgacgcattcgtcctggaattgctgaacacgccctcctggctgcaatacatcggcgaccggcagatccggacccttgcagatgcacaacgctatatcatgaataacctgttgaagctatacgtcgaacaaggctatggcgcatgggtagtagtgctgaaagaaacagggaatcctattggtatctgcgggttatttaagagaaagtaccttgatcagcccgacctgggatttgcttttttaccggcctttgaaggcctggggtatgcttacgaagcggctaccggtaccattacctattcccggcagcaattgccgtttccaaggctgtttgccattacccaaccggataatcaccggtcggttcgtttattggagcggtctggatttacccggcagggcaccatccttccacccggagaagcggaagaactgatgttatttgatcttgaattaggaagctgactgccgccgtttccggtaggccatcatcctgcttcccgccaggtaaagcaacgaccccacacacaataccaccagtcctgatctgagccatgtagcagcggttacagacaacccgattcctgtacccagggctacataggcagcgaaacaaatggggcactttggcagcagtacgagagtgatgcccggtatcagccatcgtacgccttttacaaagcgttgcctcaaagtaagcggaccggtggtttgcgcggcggttgttttgcgggcgccgctgcccgtagcggcgccgcaggaacaatgtgttttcataatacttagtcttctgaacaacaggaacccggcgttttctctttgtgatacctgccggtattatctacatgtcctttctcttcgtatttgtcgtggtgccgtacccacgatgttaaatcgccacgttcgttgatttcattacgtcccagcggcgctatatccaggtagttgtaagtagcgagctgtaattcgccaccacggccatacgtggaataggtgtgataaatatcgcctgcttcatctttataaaaaacgctgatgccctggaggtcttccaaatgatgcggcaatccttccacgatatcgtagttgtaatacaccttaccgctttccaggtcctctttacggaaagacacgtgatagtcgtagttgaaatcactgctttcagaagatacccatttgaagtgccagtccatacgcttacggaaagcctccagcgcaggcaacggtgcgcgtgatatcactacaacggacacatcatgatgctccaggtgaggcaatacgccgttaatggaatctgctgcaaatgagcaacccacacaaccttctttttcatggggaccaaacataaaatgctggatgatcagctggctgcggccttcaaaaaggtcagaaagggtgaccttaccctccggaccatcaaatacatagttcttctctaccttttcccatggtaatgccatgcgctcacggctaagctcatcccgcaaacgggtatattccttttctttttgcaaaaacttcttcctggcttccagccactcttcggaggatacaactttgtgcgggggaccgggtttaacagcactatctttaaaaccagtcgttacaggagtactcatgattttgtgattttaatgtcttacaaatctccggagttaatatgtaaatgtagatgggtgaatgcgacttatttagggggtgattgtgccaccggaaagtagtaaattcgtgttgtaacagacacaaactgccatgaagactgtttctttgcttatttatgaagatgccattttatcttccgtatccagcgtgatagatatcctgctgggcgctaaccgctttctggttggagccggaaaggaacctgcctttaaactggagctggtcagcgaaaagatgaagaatatccaattgcacagccctgcgcagtttatctgctataaaaccatcgatgaagtacaacatacggaccttatcctggcgccggcctttgaaggcccgccggatacggtgctggagaagaataaggcgttggtgaactggatccgtaacatgcatgccagtggcacagaggtagccagcctgtgctttggaagctatttcctggccgaagcaggactgctcaccggcaaatcctgtacttcccactgggcggcactcgacgatatgcgcaggcgctacccggatatccatatcctgccggataaggtaatgaccgacgacgatggcgtttataccagcggcggcgcctttatttcattgaacctggtattgtacctgatagaaaaattcagtggccgcgacacaagtatttgggtgagtaaaatgttttcgatagatatggaccgctttaaccaggcccatttcgccgtgttccagggacaacgccgtcatgaagatgaagacatcctcaaagcgcaggcctacatcgaacaaaactacgatcagcagatctctgtggaacagatcgccagccaggctaatatgagtaaacgtaattttgttcgacgctttaaactcgccacacacaatacgcccatggaatacctgcaacgcgtaaaaatagaatccgccaaaaaagaactggagaaaaatgccatcaatatcagcacactgatgtacaatgccgggtacaacgaccagaaagcattccggcagatatttaaacggtacaccggtttaaccccgcaggaataccgtagaaagtactcccgcggcggcgtggagatgaattaagcattattccgtccgcaaactttttacaggattcatcagcgctgctttggccgactggtaactgaccgttagcagtgtaatgacgattgtaccggcgccaatggctataaaaagccagatcgatacgggtgtatgatatgcatagtgattcagccacatctgcataaaataccaggtaaggggagtagccaccagtaaagcaatgatcaccggcttcacaaaatctttcgacagcagcaacaaaataccagacaccgtagcgcccatcactttgcgtatcccgatttctttggtgcgttgttctgccatgaaagcagccagtccaagtatacccaggcaggaaataaaaatcgcaagcacggcaaatacagtggtcagccgcgcaatgcgctcttcatcggaaaacttcttcgcataaacctcatctgtaaaagtaaaatcaaagggtccctcggggttaaactttttaaatacgccggcaatcccggttaatgccgtccgcataggcattgcagggttcacgcgaacagttaacgcattatatacgccgtattccaggcaaaaaaccaccggctgcaccggtgcatatggcgattccattaccatgtctttcaccacgccaatgatcatgtgcggctcaccacccgcctgtataatttgcccgataggatgtttaaatcccgttagcttcaccgccgcttcatttaagatcagtgcgcccgtatccgtagggaagctcctggaaaaatcgcggccctcttttatttgccagccaatagtatggccgtaatcatgcgataccgttacaaagcccaaaggcgctgcaataccgggtactttaccttcccaactcaggtcgtcactattgccgggattctccgtggtaggatgcgacgccttcgccatatccgccaccgcaccgctttccagtaaagcagccctcaattcattgtaaggcgcaccaaacatttcaggggtgttcatcgtgaggttaatcaatccctcccggctgtagcccaccggacggcttttggcatattgaatttgctggtacacaattacagtacctatgatcagggcaatggatacgctgaactgtactaccatcagggcgttgcgggggagcaatgaaaaacggcccgtagtaaaacctccttttaatatttttaccggctgaaaagaggataaataaaaagcaggataactgccggccagcaggccggtaaacacggcaaaccctgttcctgccaaccatagcaccggcgcgtcaaatgggatcgtgatctgtttttcagtgatccggttaaacagcggcaataaaagccacaccatgcccaccgccactataaaggataaaaaggagagcagcagcgattcggcgaggaactgccggacaagacgtccccgcgaagcgccgatggctttgcggatacctgtttctttggcacgtttggcactcctggcggtagacaggttcatgaaattgatacaggccagcagcaacaccaatgcacctataacaccaaacaaccacaccaggcggatacgcccgccgcttacctgcccgttcttaaactcgttatataaatgccatttgttcatcggatgcagcaacagcgtttccttgcccgcctttacatgctgttgcacaacgccgcggatctttgcactggccttatccatgtcaatgccctcattcagctccacgtataatttccagtaatgggtatcccatttggatacttcctctttcagccacggaatggtagtcacggcccggtcccacggaaggaacagctgtgtgccataaaaagccgtgctttgcgggagatcttcatacacacccgccacctgcagatcagtgcggttatccatgcggatcgccttccccataggatcggaactgccaaacagggaagtggccagcgactggttaatcaacactgcggcgggcgttttcaacgcatcccttttgccctgaatcattttgagcgtgagcatctcaggcaaatccgggcctgcccacactcccgattgcgataactttttatcacccacggcaatcgtatgggtgaagttgggataaacaatagccacccgcttgaaatcgcctgcataattattccggagttcatctgcgagtggaatggcaatagcttcaccggtagtggtttcaccgttgatggtttgtacatccattacctgtgccagccggttatgatgatcatgccagtgattaaatgacacttcatcccatatccataaccctatcagcagcgtaactgccataccggtagccaaaccaataatattgatggcagtgtaacttttattttttataagatgacggaaggtaaatttaaacaattgcatgcagccgctatttttaatgggtgccggaaaaataatgccggaaccggattcttttataaataacaaatttatacttttgcagatattctaatgtgtccgttttcaatacaggcggcggccggttttgaaaacaacctttctccttatctttccctaattttagcgttttcaaattggcagatgcgtatgaacagaattatctatagcctgctgttgctgatgggagtaaacaccatcgcatcagcacaggaattgtatatgccccgcaatattaaacaggcatatgtgaacggaacccgggacaaaagcggcgcacccggcaagtattactggcagaacaaaggcgtgtacgatatccggctggcagtaaacccgcccgaccgtaaagtaaccggcagcgaaaccatcagctatgtgaacaacagccccaatgcattaaaaaacatagtactccgcctcatcgttaacctgcataaataccaggccccccgctccgggtatgtgagcaaaaactttttaacggatggcatcaccatcgatacattgctggtgaatggcgtgaagctaaaagttaataatgatgtaggcacgctctcgtatgtagtattgccaacgccattgcagccgaaagacagcctacagctgcaaatcgcctggcactacgacctctccgtgcaaagcggccgggaaggcatgttggatagtacctcggttttcatggcctacgcatatccccgcgtatgtgtatacgacgattacaacggctgggacggactggatcataccgaccgggtagagttttacagcgacttcaacgactacaacgtatcggtaactgtaccaaagaacttcgtggtgtggggtaccggcgacctgcaaaatgcttcagaagtgctgcagcccgggtttgcaaagcgccttcagcaatcttataccgctgataacgtaatgcacattgctaccctcgatgaaatgcagcggaaagtggttacccgccagcacaacacgaacacctggaagtttaaagccaaccacatcgcagacgttacctttgcggcaagcaaccattatgtatgggacgctgccagcgtaatcgtggacagcagcaccatgcgccgcgccagcgtacaggcagcctataacgatactgccacagacttccatcactcggtagcgttttcgcaaaatgcactgggctggttctcgcaccaatggccgggcgtaccgtatccgttttcggtaatgacagccgtacaaggctttgcagatatggaataccccatgatggtaaatgatggttcggccgggcacgacctcagctttgcgcaattagtgcaggaccatgaaatagcgcatacctattttcctttttatatcggcatcaacgaaagccgctacgcctttatggatgaaggctgggccaccacttttgaataccttattggcattgcggaaaaagggaaggaggtagccgataacttctacaaaaaattcagggtcaccaagtatatctttgacccgtccacggaagaagaccagccgattatttccatgtccaaccaggtaagcggaatgggctacagcaacaactcctatggcaaagcatccttgtcctacctcgcggtaaaagacctgctgggcgatgagcggtttaaaaaatgcctgcatgcttatatggacaactggcatggcaaacatcccatcccctgggattacttttattccttcaatacggcggccggtgaaaacctcgactggttctggaataactggttcttcagttataactacatcgatcttactctatcagatgtaaaacaagagaagaaaagtataaaagtgaagatagataatacgggtggtttcgctatcccgtttgacgtgatagctacttttgccgacggcagtacggctacctggcatcaaacacccgctgtgtggaaagccaataccaaagctactgtgctggatctggcggtgaagaaagaagtaactgctgtgcggctggaaggcaacctgttcatggatgccaatgcaaaagataatagctggaaaaaataataacaggaggggatcgcatcccgcgattcccttattcctctttcagtaagccgtttattttacagtactccacggcttcttcaatactgtttacctggaacttgcgcaggatgttcatccggtgcgcttcaatggtgcggatgctgatgttcagcgattcagcaatgtctttattattgagtccctggctgatcatccgcatgatctgttcctcgcggcgggaaagggagatctcctgcgtgccgctgttgccgggcgtttgcctggcatcaagatatttttttacgagaacatcactgacttccccgataaaataatatttcccccggtggatggtgcggatcgcgctgaggaatatcttattactcgtatctttcaaaatatagccgctggcgcccatttcaagggctgctgctacgtagtcgggttcatcaaaaaggctaaagaaaaggatcctgccacggggatttttttccagcaggcgggtactggtttccagtccgttcatacccggcatgcggatatccatgataataacatccggttggataacggctaaccgttgcagtgcatcttcgccgctgctggcttctcccgtcacttccatgtcggcttcactgttgatgagctgtttaagaccgttccggaatatttcatgatcatctactaaaaaaacgcctatttttttcattgctaaaaagttattgccaactgtacaattgttccggtgttgggtgttgaattgatttgaagcgttccgcccagcaattccgcccgctctttcatattacggatgccattcacctttttggcctgttcggaagagtaaagctgctggctgtcgaaatgaaaaccgttgccgttatccctcaccgtcagctgcaggaaattggccgtaccgtcaatatctatttcaatggtatctgcatcagcatgtttgatggcattgttcaatgcctcctgcaagatacggtaaacgcctgtctttacttcctttggcagcggcgccgccgctaaggtgtcttccagctggaagtctataccaggggctgtttgccggcaaagtttaatcagttcatcaatggcggcccgcaagccgaaatcttccagcacactgggtaacaggtcggcgcaaatccgtttggtttcattgataatgctgtacatcatggtattcaccatggcaatttcaggatcgtgctgcatactccggtcttctatctgttccagcttcatacgcaggctggtgagcatttgcccgatgccatcatgtatttcagcggccacccgcttacgctctttttcctgcccgttgataatggaatacgaccgtatgcgctgctccgtttcctgtcgcagcaatttctcctggttggccagttgcacctgctctgttaacttgcgtgcgcgctcttcggcatctaccagcccgcggataattttccggatgcgggtagataacgggtagaagatcacccctgcttccagcatcagcgtaaacagcaccagtcccagcacgatgtattcaatttccttcaggttgcggatgcgttctttagaaaatcggtcgtagtcgaatacaatcagctccatacccagcaggtacgacttttcataggccagtatcgtttgcacatacggccggatgcgctccggtttaaaggcactgtcgctgtacagtaccgtaatcattttactggcggcatcccatatttcctggtggggattgcggataatctcgaacatctgcttcagctcatcctggtcgtttgccggtaagttgagaaagttactgccggcctgtaagccttcgtgcgatttctgccactgcttcagcgtattgataaattctttccggttatcatctatatccctgccggattccagtagcagcgccagtttactcagcgtttgactgtacgttcgcagctttcctgcaaagttgattacatgcgaatcattcatctggtggttcagcgcctgctggatctttatctggctgaatacagataacaacgcaatagtagtgagcgccaccgcgtagaggatggtgaagatcttaaaaatacttctgtcttcggatacaggatgcataatgttaaagataaataaaacccgcgcccggtggcatcacaccgcaatatgtttttccagttccgagtgcttcagctcttccgcggtgccatccagcaccatccggccacggtccatgaaatagtaatgatccgttacctggttggcgaaatctattttctgctccaccagtaataccgacagtcccttttgctgtaccagctgttgcaggatactgccaatttcctgcgcaatggaaggctgtatcccttctgtaggctcatcgagcaacaggagggaggggttgcttaccagtgccctggcaatagacagctgttgctgctgcccgccgctcaggttaccacccgcgcgtttacggaaatctttcaggatgggaaacaggctatagatctcttcttccgggatctttgctttccggttgggatgcgcttccagtcccagcagcaggttttcgtataccgatagtttcgggataatttccctgccctgtggtacgtaagcgatgccggcctttgcttttttatgcggcggcaatgctgtaatgttttcattgttgaaaacgatactgccttcctgcgcgggcagcagtcccataatcgttttgagcagcgtggttttccctacgccattgcggcccatcacggtggtaacggcgcctttttttacggcaagggtagtgccgcgcaaaatgatgctctgtccgtaagcggcagagatattgttgatggtcaataccggtgtgctgatcataatgtttcaagttgagcgttagtacggcctaaatagcaatcaattacccgctggtcattcttaacttccgcaaaagtgccttccattaatcgtttgccacgaaccagtaccgtcaccagttcgttggctatctgttctacaaatttcatatcatgttcaatcacaatgatgctgtgcgctttggacaactccagtaacaacgcaccggttttctccgtttcttcatcactcatgccggcagcaggttcgtctatcagcatcagtgtagggtcctgcaataccacgatggcaatttccagccattgcttttgcccgtgcgaaagatcgccggccagtttatacattacgttggtgagcgacagcttcacggctacgctgtgtatcctctctgccagcgccggtgtggatttgaagaagagggaagaaaagatgtccttcttcattttggccgccagcaacaggttgtcgtgcaccgttaatcccgggaaaacggagggcttctggaatttccggcctatgccggattccgcgatctttacttcggttttccccaggatggatttgccattgaaaaatacttcgcctttgtcggcttttgtttttccgcagatgatatcgaggaaggtggacttgcccgctccattcggaccaatgatcacacgtagttctttatcgcgcaaactgaaatgatccaggttcagtgcatgtacaccgccaaatgataccgccaggttgtttacgttgagtagcatatcagtgtgtagtttgaggcgttttaaaccgggcagcggagatcttttgtttgatagtctccagcaggcccataaatcctttatcaaaatataataccgtgatcacaaacaggaagcccagtataaacagccatgaatccgggaataaactggtgcagatgctatacaggaagttcaccagcaaggcccccagcactgcgcctttcaggttgccccggccaccgagcgctacccacatcaccatttccaccgatgcttttacatccatacggccgggtgtgatgatgcctgtttgcggcaggtataacataccgcctaccgcggctaacagtgccgccactacgaaaaccgccagcttgtaatccaccactttgtaggcggcgtagctgatacgcgattcactgtcgcggatcgcctgcaatactttcccgaacttggagttggtgatccggtagcagaaaaaataagcggcacacaatactgcaaaggagatcatgtacagcgcaagttttacggaagatgaagagaggttataacccagaagggtgttgaaatcggtaagaccgttggtaccaccaagattggtttcattccgtaaaaagatgagccacatcgccagcgtaagcgcctgcgtgatgatagccatgtacacgcctttgatccggctccggaacaacacaaagcccactacaaaagcaaagagggcagggattagcaggcatagcgccagcgaccagccaaacgaatgaaatggttgccagaataacggtaacgtatctattttattccacgccataaaatcgggcaatacagcgcccgccgccactgttttcttcagcagcaggtgcatggcaatgccatagctgcccaaacaaaagaagaaagcctggcacatggaaaggatgccggtatacccccagatgagatcaatacccagtgccgctatggcaaagcagaaataccgcccccatacagaaatggtattcacggagaggagccccgacaggtaacccgccggcaacaggatcgcaaaaattgcgatgaacaatatataatacagtggattgtttttcgttttcatatgcccggtttttaatcttccgcaacgcggcctttgtcaggaaataagcctttgggtttatactgcatgaacagcataataaacaccaggataaacactttgccgtataccgcctggaaaaaggattctgatattttggtgaagaagccaatgcccagcccggagaagatagtgccggcgagtttgcccacaccgcctgttactactaccaggaaagaatctacaatataagtttgtcccatgtcgggcaccacgttgccaatcagcgtaatggcgcaaccagcgaggccggccagccccgagccaataaagaaagtaatggatgccacacgcctggtttctatgcccaggcaggcgctcatctgccggttttgtgtaacggccctgatctgtaatcctagcctgctgcggtacagcatcaggtaagtgaacaccaccatcaacagggtgagtacaatgataaaaatgcggttatagggtaaggtaagatgtggcgatacctgccatccaccggataacagttgcggcgttttcaccgctgtaagatcgccgaataacaaacgggcggtttgtatcagtattaagctcacgccccaggtagccagcaggctttccaacggcttggcgtacaggtggcgtatgaccagccgttcgagtatccaccccattgcgcctgctaccatgaaagaaaggggcagggcggcgaggaagaaaagatctgtttgcggaatgcccagtgtgtgggtgaaaaatacctgcgtgcaataagtagtataggcgcctatcatcataaactcgccatgcgccatgttgatgatacctgccagtccgtatacgatagaaagtcccagggcaatcagtataaggatgctgccaagactcagcccgctaaagaagttctgtatcctttgcaggctgtcgtagcgtttctccaggctgatggcctgtgctgcggcatagtgggctgtttcctggtttaagaacccggcttttgcatagtttctcagcagcacgggtgcattgtcgctccagttgtcgccgatactgtcaatatacgctttggcggcagcggtgctggcggcgctgtataagcgggcggcgtacaacacatctttaccggtgcgccgcgcatccgcattggtttcttttgccagtgcggcctgcaggatagggagtgtggcgctgtcgcccgcgtttttcagctgagtataagcgaggatacgtttttgcgcatcgttgctgaacaggttcagcagcggggctatccctgccagttgcagccggtcggcgcggggaatgtctaccgtttggagggctgacaatggtaacaacagcggttgcccgctgctgttggtaaggagtctgttatcgggataaagggagtaaagccggtaggttccttctccggtcggtttgctgtccaccgttaccgccttatgatccagcaggtacagctttttatcattgatcgccatcagcaaaggaaaggtggccggtatccggagggcggccagtctgccaatagcctgcgttcgcacggagtcgttagttggttgcagcagctgtgcggtgtagatggaggcgctgtcctgtgccgctactttcaggggtagcagcagtaagcagcacatcagcatccgtagggagattttcatcgcatcgtatttgataatttggaaatagcctgtctttttaaaaagtacccgcttattttttagcgtaagtaccgttgtggttcacccagtcgcagtctttatcaggagacgttaacggcgaccatggctgcggatccacgagtccttcggatttccagatgatatcaaattgtccgtcgggttttatttcgccgatcacaacgggctttgccaggtgatgatttctcgggtccattttaaccagtccgtcgggagaagggtaatccagtccgtacagtgcgttgcgcacttttgatacatcgaaggagcctgctttttcagcggcttttgcccagagataaacaccggtgtaagcccagcagataggatcatctgttactcttttatcgccgccgggtaatccttttttggcgcagaaggctttgaagtcggctacaaactttttgttttcgggcaggtcgttcgactggaagtagttccatgccgcgaggtgtcctaccaggaattctgtgtccatagagcggagttcatcttctgccacagaaaatgccatgatggggcaggtagcggcagaaaggccctggttggcaaattctttatagaaaggcacattggaatcgccgttgatagtagaaaggatacaggctttaccatctgctgcaaagcgttttactttagagatgatggtttggtaatcctggtgatggaacggcgtatattcttcaatgatattttctttcgggatgcctttggagagcaggtatgctttcaggattttgttggcagtgcggggaaatacgtagtctgttccgagcaggtagaactttttatagccgccgcctttttcactcataaggtattccgcggctgggatcagctgttgattgggggtggcgccggtgtagatcacgctgttggagcattcttctccttcgtattgcaccgggtaaaagagcaggccgttgttctgttcaaaaaccggcagtacggatttgcgggatacggaagtccagcagccaaatacggcagatacttttttatcgatcagcagttctttggctttttctgcaaacaggtcccagtcggatgccgggtctacgatcaccggttctatttgtttgccgagtacgccgcctttggcgttgatttcatctactgccatttgcacggcatctcttaaagatacttcagagatggccatggtgccgctgagtgagtggagcacgcctattttaaccgtttctttggaagtggcagagtcgctgctgccggcttttccggcgctgttgttacaggatgaaaagagtgcggtggcgccgaggagcaggatgggtagttgtttcaggaaagcgtttctcatgtgttgtattattttataaagaagatgaatgaatgcgtatgtcctttagaaaatgaagaattgagcctgcagccagagttgtccgaatgtttttttcgtgtagtcgtcggcggtagcagtggccacgttgtaggtacgggtagtataggagaggcgcaggttagtcccggtgccattgaagaagtagtttagtcctccccccattacagtgctggagttcatcttatcaaagttggtgggttttacggtgccggcttgtgcggcttcggcgcttacatcctggttttcgtaccggatccagggttgcagttttgtttttttgaagtagtagccgagttccaggaactgaacggtttgtttaggaatgagggtagcaaaggagtatttggaatccagtttggtgccgccggtcatgtactggaaggctgcatttactgtaatggagcctgcatttcccagcgggtggtcaaagaatacatccgtgctgaggttgtagtaggtggcctgtgcatcgaatcctgcggcccatgcgagtgttttaccattgcccagtttggtgccggcatagtaatagtccttttccgcatcgaggaagttgtaggcaacacggcctacggtacggagtggtgcgccgccatctacattgcggccggtgaaaactcccagccggtattccagtttatcgttggcaaggaatccgcgggcgttgatcccgagatcgcggccaaagtttccctgcagcgggctgttggcaaacaggttataagggtactggaagtaggtgaagtcgttggccattaagccggcggcgccctgtaagccgttacggttgttggacaccagctgcatccctgccaccagctggaaggcattggtgaaagtatattccagttgtgcatccagtatgatgggcgacacctttacattcttctcgccattggattgtatgccgatgggagaagggatttccgtttccataaagaagctggcctttttcgtaagctggccgcccacgagtaccctggcgcggtaaatggaaaagcccttgttccagtccttcgccgttttatcgttactgggggtgccaaagcctgtttgctcgccggaggcgaacatatgaacaatggcgcctacctggatagaaggtttaaaggggaggtctgaagcctggaaaagggtgatagcttttgcgctgtcgttgctggtatttaaagaagcgggcagttcaattaagtaaccgcctctctttttctttttagggggatcgttgttttcggctttcgcaataaatggagcagtggcaagtatgaagataaatgtggctgacaatttcataaaataagtaattaaaaattagataatgtacttaagtacttttttggttgatcgatcagtatacttaagtataaaagtagaagattaatttacttaattcatataatttttagaaaaagtattaaaaatcgtgtgatgtgctgataataaacgtacatataatttattataatataactgttgaggctgttttttacttgattaagtaagttgatttatagtatgttgtaagataatataggaggaccaggaaaaattttgcttcccagttatactcttatatttaataatattatatatattaactatgtaacgatagaatggaggagcaacctatctccggataaggtccgaggcagtgttgctgccaccccgattttgagataagccatagataagccgtatttaagccttagataactcgtatctattagatacggcttagctatggcttatgcgtaagtaaactatgggtatacttgaataaacatgattggataccagcatgagctttacacgcagtaccgggaggacatggccatgcaggagaaaatgaatggttttggagaaagtggcctcagcgtttcagccagccggtgatactcatcctgggtttatgggtgagctgcacttcatgttccagttcactgcttttaaagaaaacggttttgccgctgctgggatctacctgctgcgcatcgccattggcatggtaaatagatagctgccccccatcggcgggcaaccagccggtattgaggtaaatgatcatggaatattgacggctgtcgttattgcggaactgatccaggtgtttcttataaaagctacctgtttcatacaaggtgtaatgaaactcatacccggtaatgccggtgtagcacgactggttcaggtaagctacgaaggcatccatcacatcaaaaaaggcattttcatgcgcgttgttgtgttgcctgtcgagccagtaaataacatccccgcgaacggatttgtcctggttcaccagtgactgattaccggtacctgcggccagcatatttttttcggagtgaagatgaaacaggttttcttttaagtcgttggaaagctgactgcttaaaaaattttctgagatacctactttgctttcaatgaagctgttaattaatgtgtcaaaggcctgttgcaaaaaggggcgtgcttataggaacagaattattcccattccggtgaaggtagcgggaataaacagatttagcatcattagtagttaatattctcgtaaaacaggttaatatctgcgtgtattttattttgcaatctggtaacttcacggcgaaagtacctgccacatgaccgaaaacaacagcgccgcaccaacgcaacaggaaaaagagaagcgctttgcggcgctgtttgaactgtttaatgcgcgcctggtactctttgcaaaatccatgctcccggcaggagaagaagccgcagatcttgtccaggaggcatttgtagcgttgtggcaacggttggaaagtttcagcgacacatcggctatcaaagtattcctctatctcaccgttaaaaataaatgcctgaacatttacaaacatgaaaaagtaatacgcaggtaccagcaccgtcaactccccgaacaggaagaaaaacacatgatgctccggctgatagaagcagaagtggcaggcgaagtacaacaggcattacagcaactgcccgccggctgcaggaaggttatttatctcagctactttgaagggctgcgtaatcatgaaatagcagcacggctacaggtatccgttaataccgtgaaaacgcagaaaacacgcgccttgcagctaatgcgcggactattgaaaaaacagccgttacacctgctcgtctttttaggcaaagtattttagaaaaaaaatctttaaaaaaatccacttcttctttcacccactttttaaaactggttgtttatgtactaccagttatggaaaataccagcaaacacctagtcatcgcgcagctgatagccaggcagctggcgggaaacattacgcccgcggaacagcagcagctgcaggcatggaaaaaagaagatccggctcatgagcaattatggcagcaactcacccatcccggttacctggatgaacgggtgacggcgcttggtgaaacggaaaataaaaccgcatttgataaactaatgatgcaggtacgccacctggatgccgcaccaggtataccagtgcttacccggaatagccggcgaagatggctgcaatacgctgccattgccatgcctttattggcggccatttccatgggatggtacctgcgtgggaaacaggcttctccgccagcggtgtacccggtgaacggcaccggcagggaaggtgcgccggcagcatggcaacagcttgttacgccaaaaggaatggaggataaagttgtgcttcccgatggcagccacgtatgggtaggcgccgctacctcgctgcggttccccgccacctttagcggaaaggaacgccgcgtggaactggacggagaagcctattttgaaatagctgctgatccgcaacacccttttgtggtgcataccagcaaaacaactgtgcaggtgctcggcactgcctttaatataaaagcgtataagggtgaacgttatgaacgcaccacgctggtatccggcgccgtaaaagtatccgcggcaaacagtaccaacagccggttattggccccgggccaacaggcggtggtcaatggcgctatcgctgtggaatccaccgacgtggacgctgccctcgcctggaaaaggggagtgttcattttccgcagcgaaaagttatcggacatcctggaagaattatcccgctggtacaacgtagtgattgttaccgaatcatccgtagatggtaacgcgcatttcaccggccgcattatcagaagtgaacaattagatgatatactgcaattcctcgaagcaaccgggaaggtacatttctcccgggaaggccagctgttaagggtaagcgctggccgcagaaaaacagattaatacaaccaaatcagttattccatgtaagcaggatcaaaaagaaaaccgggaatgcgcgaacactcccggcttataatgccaaacaacctgtatgtactgtgaaaagggaacagacaggtattgtctaactattatgctaaacaaagttatgaaaaaaattggatgctccgggtacctcccggacgacaaactattgctggtattcatctcccgtacaatgcgtattaccttactccttacactgatgtgcatcttacaactgcgcgcagccagctactcccaggaaattaagttatccgtttccctgaaagaagcaaaaatttcaagcctgtttaatttccttcagcaaaagagcgactaccagttcctctacaatgatgaagacctgcagaagatgccggtcatcactatttcccttcatgatgccaccattccgcaaatcctggatgccggcttcaacgggttaccactgggctaccgcatcactaacaaaatggtagtagtatttgaagcgcctgaaaaaatgccgcttcagcaggaacacaccattagcggcatcgtgaaagatacagaaggaaagccgctggctggtgttagcgtagggctgcaacattccgccaatggcacacaaaccgatcagaacggacactacaccatccgggtaaaagaaaacaccggcacactcgtattttcctttatcggctaccagagaagagaagaagccatccgcacaagaagcgaaattaacgttgagctggaagccagtatttccgcgttgaacaatgtagtagtgattgggtatggtactaaaaaacaggtaaatgtcaccggcgctgtatccagcgtaaaaggaacagaactgaaacaaagtccttcccccaatttatcgaatgcactggcaggccgcattaccggtgtaattgccaacaaccgcagcggtgagccgggaaacgatttttcgtcgatccttatccgtggcaaaggcaccctcaacgataacagcccgctgatagtgatcgacggtgtagccaacaggggctccttcgaacgccttaactccgatgatgtggaaagcattaccgtgctcaaagatgcttccgccgctatttacggcgcacaagccgccaatggggttatcctcgttaccacaaaaagaggcaaacctggcaagcccgttatctcctacaatggcagctatggcgttgcacagcccacctatattaccaaattactcaatgcagggcagtacgccacctacatgaatgaaaaatatacccggtccaataaaccccttttgttcacggacgaggatatacgaaaatataccgacggcagcgatccgctgggtcatcctaataccgactggtaccactcggttctcaaaaaatattccccgcaaaaccgtcatgccctgtcggtaaacggcggcagcgaccgcgtggattattttatctccggtgaatacctttaccaggacgggatctatcgcaaatcagctaccaactatcaccagtataacctgcgctccaatgtaggcgccagcatctccaaaaacctgaaggtagcggtggatgtttccggcaggatggaagaccggaaatattccaactacagcagcggcactatcttcggcgaaacattatccgcttatcccacgttacctgattattatcccaacgggttgccaggccccgggctggctggcgggcgcaaccctgtgctgatggcttccggcgctaccggctataacaaggtgaaggatttcttcgtacaatctaatttatcgtttgatctgaaattgcccgccctcacacccggcctgtcgctgagcggactggcagcctacgatttccagttccataacgataaaacattcctcaataactgggatgcataccggtacgatcctgccacccagaaatataacaacgtacgcgatgcagaaagccccatgcggttggatgaaggattccgtcattacaataataaaacctataacctccggctggcctatgaaagaaaattccatcagcatgaggtaagcggttttgtggcgtatgaacaaagtgaaggatataacgaaggcatcaccgctatgcgcaaaaattttctcagcgaccaggtagaccagatttcattaggtgcggataaagacaaagacaacagcggttcagcagcgcaggtggcgaggcgaaatgtttttggaagggtgagctatggttatgcggataaatatctggcagaaattatcatcagacatgacgggtcttttaattttcctaaaaacaaacgttggggtaccttccccggtgtttcagtagggtggcgtatttcagaggaacccttctttcagcaatcggtgaattttatggatcagctcaaaataaaggcatcctgggcgcaaatggggaacgataaaattaatccttaccagtatattttacagtataataaagataacggggtgtatttcggaaatgatccgcaaagagtacccgggctttctgccggcatttctcccaaccccaatatcacctgggaagtggctgaaacaaagaatgtgggcatagaagcatctttcctgaaagggatgtttaccctgaatggcaactactttacttcccgccgctccaatatcctggtagcgcggaatgcctcagtgccggcatctaccgggttaacgggcagtttgcctccggagaatattggtattgtaaataaccacggatttgaagtggaggcagcacaccaataccgcgtgagtaaagatctgagctatagtctaggatttaactatacctacgcgcaaaacgaagtggtgtttaatgatgaagcggccaacatcccatcctggcagcggatccagggccacccgatgaattcctggctgatctataaaactacgggcatctaccataaccaatctgaaatagatggttccgtacacccggcaggaacccagcctggtgatatccgctatatagatgtaaacgatgataagaaaattacttccgacgaccaggtgcgggtttttgaaagcactacgcccaccagtatttatggcattaccatgggcgtgaactataaaggaattggtctgaacgtgctgtggcagggacaggcaggcgcaaagatgctgattcttccgtcgcagaacggcggcgccttaacaccacccttatggatgtacgaagaccgctggacggccactaacgtgaatggcagtatgcccgcatcattcgatcgtgataatgacattaccaaccgccagtcggatttctggttgcggaacgcttcctttctccggcttaaaacagtagaactttcgtatactttcccggctgccagtctttcccgtttcaagctgcagcagctgcgggtatacgccaatggctttaacctgctggtgttcagccaggtgaaaaagtatgatccggagttgaacaacgtaaccggcaactactatccgcaaacgaggatctttaatatgggcgtgaatctttctttctaaattatcataattaataatcatgaacaaaacgatatataaactttttgcagcgggcataggtgcatgggtaagtttatctgcctgcaataaagatatcctcgacaagcaacctccgatgagctactctgatgaagtgatgtggtctgatctgcggctggtggaagcttatgtgaattcgaggtactggatattgccccactttatcgacgcttccacgaaagccagtactaccggtctttccggcgcttccgacgaaggttatgaccactggaactacgaaggcgaattccgctttaacctcgggcaaattacgccggattacaccggcctggataactggaccgatgactatgcatatatccgcagctgtaatattttttttgaaagaatagcaggggtgaagggagatgaagacctgcgtaaccggctgaccggtgaaatgaagttcatccgtgcctggtgttactttgatttgctatgccgctatggcggtgtgccgctgattacaaaatcgtatactattgccgatagcagtttcctggtaaaacgtgatacttatgaagcaggtataaattttattataaaggagctggatgaggcgttgccactggtgccctacgtttataacagcagcaataccggtcgcattacgaaaggcgccatactggctttcaaatccagggctttgttgtatgctgccagtgcgctgaataatgctgccggtgacaaagccaggtggcagctggcggcagatgcggccaaagccgtgacagacctggccgcgcagggatattaccagctggatcaacggacagattataaacagctctttcttgataaaaaaacaccggaagcaattctctccttcggcatgaatgccacttatggcgataactatattgatgtttatatttatcctaacggttcacatggatattccgcgtatgtgccttcgcagaatatagttgacgagtttgaaatgaagaacgggaaacctgtcacagatccggcttccgggtacgatgccacacatccctatgacaaccgcgacccacgcttttatgcagatatcctgtttaacggcgccccgttcaaaggcagaacggtagaatatttcacagggggcatggacagcccgcaaagcaacgtggataactggaatgcgagcctcaccggttataactggcgcaaatatgcggatgaaaccaatacgaatatcgatggcggcagcgcgcagaactggattattttccggctgggggaaatttaccttaactatgcggaggcagcctgggagcttggcgatgaagtgaacgcgcgtaaataccttaacctggtacgttcccgcgccagtgtgaatatgccggacgttaccgctacaggtaccgcgctgcgcgaccggatctatcatgaaagaatgattgagctttgctttgaagggcaccggttttttgatgtcaggcgctggaagattgctgctatcaccgataataagccattgaaacgggtaagcattgacaaaaaggccgatggtacttttacgtatacctacccgacgctgcaaaaccgcaagtttaatttaaataattacctgtttcccatacctaaagaggagatgaataagaataatttactggtgcagaatccaggctattgataaatatttcgtccattgtttccccttttttttaatttgatgatacatgaatcgtattcgcacgttattactcagctgcctgttaacgggcatttcctgttacgcaaccgcgcaggaggcccgctgggaactggccgcagatggcggtatccgctggacggtaaaagattcccggccgcataccgatcacattgaaatgagcggcaagcaactgtcggccatcatcacctatggcacaaacgaacagcgggaactgctgttaaaaaaacagttggtgttcccgatgctgcgcaccattcccaataatacccatgccagcctgaaagttgattttactggtagtgagctgccgccggtgacggtagatggtgtgctgctccggtctatacctgttggtttttatcttaaaggaatgctccgcattcattcccgcagtaatacagcgatgggggtaacagatctgctttccccttctgtagataaggctggttttatacaattgcgtgagctggtgaataatggcagccgtgtttgccatgtgcaggtggacagccttgtgaaagaacagcatactgcggctgataaaggcgtgtacggggaatatgccatccgttcggaagtaaccgggtatggcagctttgatttgcagcccggagagaagcattccgtagcgataatttattccgcccgtaaaatgagtatgcctgcttaccatttttcgccgggttatgagttgggaagacgggaagcttttgtgcaggagctgatgcggaaccttgtgctggaaacacctgatgatactattaaccgcggcttcgattttgcgaagttgcgggcaacggaaagtatttatgacaccaaggccggactgatgcacggtccgggtggaggggcctattatgccgctatctgggccaatgatcaggcagaatatgccaacccgttttttcctttcctgggaaatctcaacggcaatgaatcggccgccaacagtttccgtttatttgccacttatatgaaccccgcttttaagcccattccaagttccattattgcggaaggggatgggtactggaacggggctggcgaccggggtgatcaggccatgattgcttacggagccgccaggtttgcactggcttccggcgatactgctatggcgcggcagttgtacccattgattaattggtgtttgcaatacctggagctgcacaaaagggcagatgggatcattacttccgatgccgatgagctggagggacgtttccctgcgggcaaggctaatctttccaccaatgccctggcttacggggcataccagggtgcggcttacctggctaaagcactgggctatcgcgatacggccgcattgtataacaaacgggctacgcagcttggccgcgacatggaattgttttttggtcgccgtgtacagggatttgatacctaccgttattacgaagagaacactgtgctgcgctcctggatctgtttgccgctggtgatggggcttaatcaacgccgggatgcgaccatgaaagcgctgttatcgccttatttgtggacgcggaacggtatcctcactgcggccggtgatcatactttctgggaccgctccacactgtatgctttccgtgggttattttttgcgggggctactgataccaccctgaaatacctggcgtattatacccgtcagcgtttattgggtgagcatgtgccatacccggtggaggcctggccggagggggatcagcgtcacttgtcgggcgagagcgcgttgtattgccgcgtgattactgaagggctttttggtattgttcccacggggctgcggagttttgacatgtgtccgcggttgcctgccgcctggaaccagatggctttgcgccatatcagggctttcggcgcggatatggatattaccgtgaaacgtttgggcgggcaatggaaggtgaccgtaacaagtaaagggaaaacggtattggcgaaaaactgggacggtatttctctgatcccggtattattgccgggttaaaaaggaggagggtatttttttgagagaaattgttccgcgtcctccaaatgtgccttaacctatttacatttgaaagatgaacttaattggtaacatcatctggctcatcttcgggggcttttttgcatttatacagtatatggtcagcggttttctcctttgcctgacgattatcggtattccgtttggattgcagtgttttaagattggtttctttactttgtttccatttggccggcaggtgagagacgtgccggggcaaacgggttgcctggccacgatcttcaacattatctggatccttatcggcggtgtatggatagcgctcacgcacctggttttcggtctgctgcttactatcaccattatcggcattccctggggccggcagcattttaagctgatgagcctgagctttacgccttttgggaaagaaatcttctaacggttgtgtgtgccgctattggcatgactattggatttctgttttcggactaaaaactgaaatatgaaaaagatattgtttgcagcagcagctgtaggtactgcagcctccctggttatcttatatctcagaaaacgtcaacagggacaggatttgctggaagacgccaaagattccgtaaagaaatctgccggtacgatgcgtgattacgtgcgtaaagcaaaggcagaggccaatggaatttatagtaacgcaatggggtaatccagataactttttgaaagcgcgtcctgtcacgggacgcgcttttttttatccagtcgaaattaaatgcagctgatttgccgggaaaatagtaggtttacggcatcagtattttcaccacatatctcctcccggttaccaaaaaccggttttccccggaaagggacagggtttcctttctttaatatttccacactattttaatgcaaacaggtgcttatgtgcacatttaaccaggtaattacatgtcatcaatatccaataaggccattgtactggccgcattcaaacacctcaccggggagcgcaacaccggtgtaatagatacttatcttcatggttcctacatccagcacagtcctatggtaaaagacggcaaggccggtttgctggaggcgctggcgtacctgaagcagcaacccgctcctgcagaggcaaaatcgcccgtagtgcgtgccatcgaagatggcgattacgtaatgctgcatatggatgtggcttttatgggtaaaaacgtggcggttgtggatctttatcgcctcgaagaggggaagttggcagagcattgggatgccacgcaggaacagccgcaaaatgcgtctataacggagggcgccactgccatcactgacctgcatctcactgccggtaacaagatcattgtagaacaatacctccgggagcctgatgccgcgctgctgtcgcccggttatcgttcacatgatatgggttattcagtactggaaaaccccagggttcaccgcatcataggagaggggaactttgtaatggcgcaatgttccactgcagatgtagtttgttacgatatataccggctacatgaaggattgctggccgagcactggcgggtggcacaggctattcccgcaaagctgccgcatagtaatggaatgatatagtttttttacagctggaatggccggtcagtgaaacttttcgtgccgttccagctttgcgatgaaatcgacgatacgcttcgcccttgtttctgcctttttcgcgttttgtaaccggaagtaaatagcgaatttattttgcttgttcagcgtttcaaagaaagccgccgcctttttgttcttttttaatgccgccataaaatcgtccggcaccgttgcctcactctgcgtagcgtaggccttttcccagcggccatcggcctttgccagctccacctggtggatacctgcaggcttcatcttcccttccgccgtaaggcgctctatatgttttgtattcctttccgaccagatgctcttagcccgtcgcggcgtaaatttttgtataaaggatttttcatcaacggacttcgactggccgtcgatccacccgtagcacaacgcttcttccagtgcctgggcataattaatagaagggattttggtatcttttttatacatgcgcagccatacgccatcttcctgggcatgattctttgcgagccatttctcccactgctgctgggtttcgaagaaaagttcgggtagttctttaggagttgccataggtataaagatagggatttgatgtacgtgtatgcatgggggttagcattttttttaagaattatttggaagttttaaattaattcctacttttgcactcccattaaatgaaacgattccctagctcagttggtagagcaatacacttttaatgtatgggtcttgggttcgagtcccaaggggatcaccataaagaatacaaacagtatcaaagccgcataaatcgcacgatttacgcggcttttctgttttccggctacaaaggtttatcattcaaaacgaaggtgaatggtaacataaaaggttacacctgcaatacttaattttagtgtaacctttctctctgtaatgcttcactgatcagggttttaggacttcaaaccaaaacaattaacaccaaacaacaccaaaggcgttaacctaaacccacaaagaacatgaaagtcagtcaagaattatcaatttcattctggttaaggaaggacaacaacaaccccgacagcaaggcaactattatgctgcggatcaccatcgacggacagcgcgacggtttctcgctggggtaccaggtggaaccggcacggttcaataataaagcggccgaagttgccggcaaatcgatggaggccattgagattaacaagcatattctccatgtgaggggagagctgatccggcattataatcttctgaaggcacaagggcctaccattactcccaccatgttaaagaacgcctatctgggtgttcacatcgagaaaaagaccctgatacaggtgatcgactaccacaacgcaaaattcaaagagaaagtagaaaaggaaaaacgctcagacggtacgctgaagaaatggtacaccacgaaggaaaagcaggttgctttcctgaaggcggtattcaaaatgcccgatattccgctggaacgaattgagtatgcgtttgcggaggactttttcgatcacatgacccttacagaaggtatccaggataataccgccatgaaatacctgaaaaatactaaacaggtcttaaaactggcggtccaaagaaaatggcttagtgtgaatcctctggaggattacgtgtgtacctatgtaaacccagaacgagatattctgagcatggaggagctaagcactttatattataaagatttcaagattcctcgcctgcaggaaaccaaagacgcctatctttttatggcacttacaggctatgcatacaaggatgcactgatgctgagccctgataatatcgccaaattctttgacggagaagactggatcattaaaaatagagaaaagacctggtgccgtgaaaatgttcccttgttacctatcgcaaaggaaattcttgccaaatataaaaatcatccctactgtatagccaacaatgtgcttttaccaatcaatagcaatcagcgtttcaatggttacctcaaagaggtagcagacatttgcggtatcaacaaaaatcttactactcataccgcccggcatacttttgcaacaaccgtcacgctggccaacggtgtgccgctggaaacagtaagcgcgatgctggggcataaatcaatacgtaccacacagatctacgctaagattgtcgccggtaaagtgagtagtgacatgaaaaccctgaaaaatatctttaaccttgcactgccggactccctcatgtgcgcagctgtggcttagttgagttgtcagggcagaaatgttgtttagtttctgctctgactttcttgatatttatcaagaattagtattgacatatatcaagaatcaaaattgataaatgtcacaaaatggtttgcataacaaatgcataacaacaacaatgcacccaaaagtatttcttgcaggcaccgtttgaatcccggaatattaacccaagtcatgtgaaaggttacggccaatcatttggacaatcctgacgcgtgcttactcaaaatcatccattgatatgcaataccagcattaccaattatcctattttgaaaaattaattcgtgttgaccttaaaaatgcatccgccacgcaaaaagaacctgacagtaagttctttgctttcaccaccaccgacgtcattaatcaaaaggaaagcatgctgcaaagctttggccgatacctttatgatcttggcaaaaagaaacagatcgagtggtatatcagcatgcatcaacagcagctggtgctacttttagaccaaatggcaatctacttaccggaagccgatgttatagatagtgaggtatcattaacagacattacctggttaaatctttacaaggtaatttatttaagcctcagcgaacttctatcattcctggagtgtcagtttgttcgctacctggacattgactgtaaggttccatcatcatatcttctgagagcaaagaataagttcttcaatgatgttgagaggctaaaggacgatttcgaagaaacggccacggaaaagcgcttgatatcaatagtattccagccttttacggacttggtaaaggctgaccggactgggcttttgataagttaccagcagctgtattttctaaaggaaatgggggataagctgtcagaattactggaggacgtggacgatgaagttgatctgacagagaaagtgaaagatttattgctgtatcttaacttcaatagtatagaatatttccactactggacggagactataaacgcagaaattgacaatctgcctaccatccgggaaaagcttgatcggcttattttccttcagaaaaaagccagccaggcaatagctaaacccggtttcatttttaaaagactgtacgctccacttcaaagtcagttattgtcctggttggccgatgaaattacttatcagaaggagaaatccgctttagctcatagtagtcataccccggatgaattaggccgctggaaagattttaaagtacttaccggtttttctgttccacaacttggtaatataatcaggctattggtggataacggtttatatctcaataagaacaaaacagaagtgctggacttcttttctcatttctttactactgttaaacaggataccatttccgcaggaagcctgcgttcaaacttttataaagatgatgcagctgtatccaaagcagtccggaatattctaaccgatcttattaagtcttctcataaatgaataagccttgatattttctttgcattggagtatctcctatggcgatactaaatttgcagaaagcgctatcgccatataattctataaaattcttcttattaataatcaaatagttacagggggtactgttacccccgtgactgttcttgcgtagggaataacttttcttttgctgccataccaaacaaaccccaaacgtatggcactagaaattttaacccgtgaagattttgcaatcttcaaagccgaattattccaggaattaggtaaattattcaacaccccagccgttaaatcccgtaaatggctcaaatctcacgaagtccgtgaactccttagcatttctcccggtaccctccaaaacatgcgtattaacggcacacttgcctacaccaaaattggcggcttgatcttctatgatcaggacgaaatattaaagctgctggatggcaaaaagaaacctgtaaaacattcctgatgaagacatcagctcataccaactatatcaggcatatgaatgccttcttcgcacaggtgcggaaagatgatcggttacatgccaatcatgtcagcctgtacatggctttattccagatatggaaccagcatcactttaaaaaatcctttcccatcctgcgcgaagaagtcattgcattgtgctgtatcggctctatgaacacgtatacccgctgcataaaagaactccacatctacgggtatattatatatcaacagggcaggcttacactccctggaattgttaccatccgttcattccctggctcttgcgatgacgatactacccagcttcaattatttgatgaattaaaaggaggtgaatcaggcatgagcagtagccgttccggtcgcaaaagtgataccgatacttgtatcataaatgcgattacgccgtgtcgcaaaattgcgactggatcgtatcgcagaaatgcgactatgccgtgtcgcaaaagtgatactataccagtcgcaattttgcgacgcttttataataaacaaataaacaattataaacgagagagagaaaagaggctctcgctctcaaaaaaaaattataaaaatgaaattaaaaatccccaactcgatcagtatacaccccgcgcggaaaatgcagatgctgccgggcgtgttctccccaccttgtcccaggtgcaggaattttttaataccaacgtctacccggcgatggaagcaggcaagtttttccaccactaccaggccaatggctggcaacaaggcggtgggacgctgattatcgactggcagtctgccgcccacaaatggatactgaatattccttctcttaaaaccgtaacccatgaccgaaacaccaaacaaccaaccgggccaggaaggctccatgtcaatgaaaacaaaagctactcagaccccttatgactactacctgttaatgcagcagctggaagaacacggaaagaatatctatggaatccacttccgaattgaagatatggatcggccggtagtagtgaaattacttgcttatttcctccatgacgccgctgttgccaccgtcgaaggcgtagatttgcataaaggcatactgcttaccggtcccattggatgtggcaagacctccctcatgaatctgacgagaaatttagcggcagatttgtacaggccgcagatgatttcctgtagagatatcagttttgaatttgggaagatagggtatgatgtcattgcccgatatagcaggaacgcttttttcccttactcgagtattccaagggtacattgttttgacgatttgggactggaacagcagattaacttttgggggaataattgcaatgtaatgggggaaatattgctttcacggtatgatctgctgatttcaaataaaatgttgacacatgtaaccacaaacctgaataaccaggaacttgaagatgtctacggcaacaggctaaggagtagaatgcgggcaatgttcaatctcgtcgcttttgattcctcaacaaaagataaaaggcgttagacttgactaatcaatttttttggttttgttctcattaagcagggaaatgctttttttaggcaaaagttcgatataagctaaaacaatttgaaaagaatagctgttaacagtcattatattaaaatattgttttgtggtcattcctggaaaccctttcaaattgtaagtaattatccccttttaatggtatcataagggccttttaaatcatgtaatacccgcattcctaagcagcaacatctcgcaatcgccctcagtcaccctcaaaatcaaaatcacagatgaggcgaatatttactatcctgattgtgttattttttgtttgtttacaattgattgcggtgcagggagtcgcgcagcttgttgttacggcaactgccacggatgctacctgctccggtaatggcagcatagccacgcataccgtaaaagctgttgctcccattgcatttgaactgcgcaatggcactacaggcgctgtgatcagactgtcgcagtcggatagtgtatttaataatctccaggcgggtacttatcaagtggcggtgtatgatgcaaataatggtaccgtaccaatattgagtaataaagtagtattgaaaagtacgtatgtaccaatggcgatcacaagcgccagcaaccgcactcctttgccttatttgtgtacggccagtaatagcgcgggtattttagatatttatttcaattatggagtggcgccatatactataacggttatttcggggcctacaattcctgcacccatcatcaccaataataaatcaactcctattaccggactttcttcgggaagttacgttgtgcaggtggcagatgcctgtggaaatacagctgttacaaatagcgtgacggtaaatggtaatgcgagtgcatatcctgcaaatctgatagcagtcctgggaagcaatcctgttaattttactttgaatcagagcacaaactgtggtactacagcaagtcttgctgtagtaaacagtgttgggcaattgcggtggtatatggagtatccggcaggttccggtaattttacagataccattaccggctctggtacacaggtgccgctgccttatgtagcccctgatcaattacagggaaagcagtataaattatggatacagcatccgtgtacaggtttgtggcaaacgactacggtgaatattcctgtttccggactcagtgcgaaaatatccactaattatgttgcggttaataactgtgattccgtatatccggtgatacaattgaattttccgacattgagcccgggtagttcctctccgttttattgttatccggtacatattacggtggctaataaggccactccaggtagctatatttttgatactaccctgactaacagggggcttgcttatcagtcggcctatcccgctgcttcgggaacttatgttgttacgctcactgacggaaaaaataatgtcatctcacaggaggtgactgttattgccggtaaccctaacgacctttctttcagcaacagttatgtaggttgcgattcaattacaggttcaatccagttttacaatatcaaagcccaggggccctttcccgtaaagctacacctggtgtcttaccccggggtaacagatttatcgaaattcccggacctgacctataatagccaggtgtcatcttatgtcaccgcgtggacagggcttccggtgaatggaggtacggccgttgtacaaactatttttccctgcagaacagttaccactaacatacctatcaaaacgcagatccccgtaaattcgccgaaaattgattctgcctggataaccattccggttacaggttgtagctccggactagttaatcttaatttcagaattcaggtaaaagatacacttggtaagacctattctacaccatcttctacgcttccgatggattattatgcgttgaagataatgggtgctagttcaccggtgtataatactacagtcctgaataatatcacttccggcagaacttataccgtcgggttagtgccgaggtatggagatggtaatgcctgtacacctgttagccagtatactgtagaggtgccaaattatggtgcgccggtatttgatatgaataaaacttatggccttgtatgtcctggttcagctacaggtagaatggttatagtggttaatggtttcggtcccttccagtaccgcattaccaactatggtactggtgcatggcaatcttccaatgtgtttaacaatctgccggcaggcaattatacggtgcaggtaatagatggctgtagtgccacttcctctcaacaggtaaaagtagtggatggcgcgggggcctctctgattaagccttttggcatccgccaaacaaccggggatacttcctatgtatgtgtgggcgacagcgttagtcttactgcggctccagtgggaccgcttgattccctgagatggaatatcccacgggattccacaatacgcgactcgctggtgatccggataccacattttaatacttcaaacaacggtaattatatccttcgtgcttattcttccgctggttgcgtgttgcaggatactctgccgatagtggcagtaccggctccggacttaaatatcacagaccctgaaccgctatgcacaccggaaactgccgacctcaccgcaccggccgtagttgccggtagcagtggattcagctcattggaatacttcatggatgcagcaggcgccaacccggttcctgatccatcgaaagtgggtgtgcctggtatatattatatcgtagctactaacgcaaacggctgtacggtaactgccccggtgactgtaaaaatatatcagtcagccactttgatgggtgaccttagcggtaacgtggtttgtagtggaacgcccttcagctttaacccggaaacagatataccggtgactgcaattacctggacccgcgccgcggtcgcaggtatcagtaaccccaccgccaatggcagcggtccggtaaatgaaacgctgatcaatacaaccagtaacccggttagcgtaacatatgtctaccatctggaaacagctgacggatgtggcagtgatttcattgtcaacctggttgtgtcacctttacctgtactgacttcgtctctcaccccgcaagctatttgcaaccggcagaaattcagttatagccctgtaagcaatgcaaccggcgccacgtttagctggacaagggaagccgtagccggtatcagcaatccagctgccagtggaacaggcaacccgaatgaacagttgatcaataccacccgtgcgatacaaacggtgcggtatatatttacaatagcagctaacggctgtaccaattcacaggcggttacagtaaacgtgaatccagatgtcaatgtactggggctttctttcccggaattgtgtaatggtgaaacggcacccattacacacctcacaacagatgcagatgcaaatgcgggaacagtggatatccgttggtacagtggcgcttctaatggagttcctgccaatggctatggtgatattccttcttttaccggtactaatactactgataatatctggaatgtaagcgttacttcctgggcagtggtaaacggatgtaatagctctcttaccgttaccaagccagtggtgatttacccggtaccgaaggttacggttcctgcaaatgcagagatctgttccggtgaaccgtatcaggcgcccgcatttcagaagaataatgtggcggtaactgtcaggtggactaatgatcatcctgaagtaggtctccctgcgaatggctttaataacctgcccgccttcaatgccatgaataatacgcgggatgccgtaacagctacaattaccgcattgcctgctatggatacaggacgttgcataggggatgctaaaacttttaatattaaagtacaacccttcccggatgtaataccgcccaatgatatcattacctgcgcagggggcaatgtatctgtgtcacccttacagcttacagctaatggcgcttatgttaagtggcataatgatcatccggaaattggcctgccggcagatggggtgggtgacatcccaccatttgctgcggtaaataacacgggtgcacctataaaggcaactatcgatgtatcatctggtcttgccggcgtatccggctgtgtgggtccggtacatcagtttacgatcactattaatcccgctgcgcagctcaatgatttgcaatcactcgaggcatgtgtgggcagcctggtaacgccggagccgtttagttcctcaaatgtaacctggacgaacaacgaccccagaactggattacctgcatcaggcactggcaatcttccttcattcaccgcaactaaccttaccagtagaccgatggtgtccactatcaacgtgtatgccaatgatgcctgtggtaattcagttatgaaaacaatgaccatcaccgtgaatcctgtaccggaaacggtgaatattaatttgccgccgggagcatgtggtggtcaattgataaatgtgagtccaatggaatcagacgttcagggcagcaccttcgcctggaaaacagatcacgctttttctactttacctccggatggtacaggcgatattccgccttttaccgtctataaccagccagtatcggatataggccgtattatgatcacaccttcctttaggggatgtaccggcccgactaccacctttgaactgccaattggcgcccggccggatgtgattatgccttataatcaaatggtgtgtaatggtagcatgatagaccccattgagttccatagtaccacaccggaagatgtaatgtatgagtgggtcaatagtaacccgggcatcggcttaccggcaagcggtataggatcgattcctccttttacggctatcaataccggcacagagtcagtattcgccattataacagtgaccgccagtatcggctactgtagaggtagtactgccgatatggtgttggttgttgaccctacgccggtggtacaggtaaatacgccaacacagaatacttgtgctggtaaatccactacgggaatagattttagcatcaatttagcaaatgcctctttatcctggaccaacgatcatcctgaaataggtctgccggccagcggcaggggtgatatcagcgcctttacccccgtgaacaacaccaatgcgcctattacagcggttataacggcaagggctgaactaaatggttgcgtcagtgcaccggttaccgcatctattacggtgaatccgaaagtgcaggtaagcccacagccggaacagacggtgatcagtgaaagcatgatgctgcccattaactttaccggcgctcctgcaaatgccacctacacctggacaaataaccgtcctgatatcgggctaccaccttccggtaccggcaacattccggcaatgccattatttaatcacacaggatcacctgtcaaagccgttatcaccgttactccgcatgccaatggttgtgatggggacccggtagaaatgattgtgaccgtattgccattgccaatggtatatgtacccggaaaccaggaattatgtgcgcaggaaataacgcaggaagtgatttttgatggtacttatggcgtaaatggagaatatacatggaccaatgatcatcctgaaataggtctcgctgccaatggcacaggaaatatcgctgcattcacggcggtcaataccacaaatacgcccattgtagccagcattacggtaacaccggttttccagggtgtagcaggggcgccggtgatttttaccattactgtaaatccaatacctgtagtttcgggagatggttctaaggatgtgtgtgccggtgattgggtcgataacccgcttacttcgaatgtgcctggagcagtgatcaggtggacgaatgatcatcctgaaatcggactgccggcagcaggagagggctttatccgcttcaatgcccaaaacaataccaacgctgccatcgtagcaaatatcaccttcagggcagattataaaggatgcgttgggcaggcacaaacgattcagtatactatacatccgttaccggttataacggtaccagctaacacggcttactgtaacggcaatacggtaccagcaggaatacccggcagcactgttaccggtacagtttacagctggacaaacaatcatcctgaaattgggctggctgcaggaggaacaggcgatattccttcctttgttgcggtaaacaatacggctacacctatcacggctaccattacggtagtgccggatgccggtggttgtccgggcgctgccaaatcctatacgattgtggtggaaccgtcaccaaccgtagccaggcctgcgagtcaaaccgtgtgtaatggtgctgctacaacaccggtggcctttgctgctggcgtcagcagctctctgccgcacgctgcaaataattacagctggacgaataatacacctgctattggtctcgctgccagcggtaccggtagtataccatcgttcactgctgttaacaccggcacaacaccagtggtagctaccatcacagtaacgccgcaaaacggtagctgcagcggtactccgcaaacattcactattacggtagatccaacaccggatgtaacagtaccggctaatcagtcgttctgtaacggagacaccagtacgacattgaatttcaccagcctggtaagcggcacactgttcaactggatcaacgaccacccggaaattggccttgccgccagcggtaccggtaatataccggcatttataccggtaaacaataccaatggagtaattacggcaacgataactgtaacgcctgtgagaaacggctgcacaggtacaccgaaaatatttacgatccttgtttctccggatgcgtctcttattattcctccgtcacaggaattatgcagcggcgcatccactacggccattgcctttggaagcggtacttccggcgccgtttacagctggaccaacgatcatcctgaaataggtttggccgccagcggtaccggtaatattcctgccttcaccgcttccaatagtggcagcagcccgattatagccacgcttcacattacagcaggtatgaatggttgtgcaggcgcagcgggtgaaatgaccatcaccgtgaacccaacgcctgttgccggtattacgggaactccacaggcagtttgtgcaggcgctccaacaggtaacattactttcaccggcaatgccggcacattgtttaactggacaaacagtaacacttccattgggctggctgccggcggtaccggaaatatcgacgggttccctgcggtaaatacgggtacaacaccagccgtagcagtaataacggtaacgcctgtattaaatggatgcgccggcgcgccggttacaggtaatattacggtgaatcctgctgttagcatgactacaccggccagtcaaaatatagtaaacggaactgctaccaccggcgttaccttcagtggtacagcagcaggcatgactttcgactggacgaatgaccgtccggatatcggtttggctgccagtggcagtggcaatattgcagcctttacaggtatcaataataccggccaggctatagtggctacggttactgttacgccccatgcgaatggttgtgaaggggaaccggtaacctttaccatcacagtagaacctacaccaggcgtggtggccccggataaccaggaggtatgtaacggtgcgcaaacccaggcggttatctttacggggttcccgccggctacaactttctcctggacaaatactaatccggctattggcctagccgcgagtggcaatggcgatattgccgctttcacggctgtaaataatggtaaaacaacggcagtagccagtattacagtggtacctgttaccctcggcgttccgggtgtacctgaaacatttaccatcagcgtatatccttcaccggtggtaacggtacccgcaaatattactgtatgtaacggtaacagtgtaagtgccgactttgacacagatgtgcctggaacggtatttaactggacgaacgatcatcccgaaataggcctggctgccagcggtaatggagatattgccgcttttgttccggtgaatactactaatacacctgttattgccagtattgttgtcaccccggtgttacacggttgtccgggtacatcgaaaacattgaccattactgtcaaccctgaaccggtagtgacacaaccggccaatatacctgtttgcgataacagcacggtgagtgcagtaacctttaacggcggtgtaaccggtactactttcagctggaccaacgaccatgccagtatcggattagctgccagcggtaccggtgacattccggcttttactgcgcagaataacacgacttcaacagtaacggcacagatcaccgtaacgccatctgcgaatggttgcacaggggcgccggttacttttacgattgccgtagatccgttaccgatagtagcagatcctgccgacagaaaagtatgcagtggcgcaacagtaccggctattgctttcagcagcgccgtgagcagttcgctccctgcaggtgtaccggtgtacaactggaccaacgacaaccccggcataggactggcggcttcaggtaccggtagtataccatcgttcactgcggtgaacaatggtaatactacactggtggctaatatcacggtgacgccaagtgcaaacggatgtaatggtatctcccaaacctttactattacagtagatccgatagcagaggtaacagtgcctgccaaccaacaattctgcaatggggctagtgcaaatgtccctgctttcagcagtaacgtggctggtgccacgtttacctggacgaacagtaatccggctattggcctcgctgccagcggtgtgggggatatacccggatttaccgctgttaatggcggtgccgcgtcaattgtagccaccattacagtaaccccggttaataacggttgtagtggtagtccggaaacatttacgattaccgtagcgccaaccgccggtatcaccataccggataatatagtggcatgtaataacagcactgtgaatgctgtcacctttggcagtgatgttccaggcgctaccttcagctggaccaatgacaacactgctattggtttggcggccagcggtacaggcaatatcccggccttcacagctgtgaacaccggcgcctccactacacaggcaaacatacgggtaaccaccaatgtggacggttgtccgggagtcaccggtagcttcctgataacggtacatccaacgccggatgtagcggctaatactgcgcaaaccctttgtgcgggcgcgggtacagatcctgttgtttttaccggcaccgaacctggcaccgtatttaattggaccaacaataatcctgctatcggcctcgctgccagcggtaccggaaatataccgccattccaggccaccaataatacttcagcgcctattactggcattataacggtaacgcctgtaggtaatggttgtgccggtacacctgccacgataccggtcactgtgaatccggcggtgacaatgaatcagcctgccagtcaaacggtagatagtggtgccgtcaccgcagctgttaacttctccggttcgccggcaggcgttactttcagctggactaacgaccatccggaaataggattgcctgctaccggcaacggtaatattgcatcctttaccgcccgcaatactactgcgcaaccaatcgtcgccaatatccgtgtaagggccacggcgaataattgttcggatacgatattaacatttgcgattaccgtgcggccagtacccagtgtagtggtgccgggtaatcaagagctgtgtaccggatccactactgcgccggcagtcttcagcggtgctgcgagcggtaccacttataactggagtaatgaccatccggaaataggactggccgccacaggaagcggtaacatcagtgcatttaccgcagtaaatacaaccaatgcaccgatagtggctaccatcagcgtaacaccagtgtcggacggcgttagcggtacagtgggaacatttacgattaccgtgtacccggtaccggtagtaaccgttcccggcaacgataccgtttgcaataacagcagcgtaacagccgctttcggcagtaacgtaccaggtacccgttttgaatggaccaatgatcatcctgaaataggaataccagctgcagataccggcgatatcaatggtatagtagtgacgaatactacaaccaccgcgattacggccaccattacggtaacaccggtgttgggtgattgtcgtggtgcagcggcaacctttactatcagtgtacaaccaataccgcaggtaacagcgccggcatcgcaggaagtatgcaacggcgctgccattgaaaaaatcacctttacaggtgctacaccggcatctgcctttgcctggagtcatggtcatcctgagataggcgtggcagctagtggcactggcaatattccggcctttacggcagtgaataatacgacggttccagtggtggatactttcacggtagtgccatttataggtggttgtgaaggggctgccatacggtttgtcatcaccgtaaatccaacaccggaagtcaatcagccggtggatcaacaggcatgtaatggcgatacattacctgctgtattactttcgttggtgcgtaccagtaacgcacatacggctactgaaacattcacctggactaacagtaatcctgctataggattacccgctgcaggtataggaaatattccgcggtttaaagcagttaacaatggcagtacaaccgatagtgctgtgattacgattacacctcatcaggcaggttgcgatggcatctctaaaaaatataccatcaaagtactgccaacaccggatgtaagcaagccggctaaccaggtagtttgtcacaacaaaaacacggctgcaattactttcacgggtagtgtaagcggtaccgtattccgctggagcaatgaccatccggaaataggtttggctggtagtggtaccggcgatattgctgcctttactgcgcaaaacaatactgatacagcgattgtagctaacattacggtaataccggatggaggcgcttgtaacggtagcgttcaagtgtttactattaccgtgtatccgcaaccgcagatgcagttacctttcagtcaggtggtttgcaacggcagtacgacgcaggcggtaaccttcagcggcagtctcaatggcacggtctacaactggacaaacaatcatcctgaaatagggctgccggcaagtggttcaggtaatattactgcctttgccgctaacaatattaccggtcagccggtagtagctaccattatagtaacaccggtgatgagcggttgtgacggtccggcaatgacctttaccattaccgtgaatcctacagctgtggtaacagtaccagtaaataaagtggtttgtgcaggaggtcagatctcaggtctgaatttcagcagtaatgcagacagtaccatttttacctggacgaatgaccatccggaaatcggattaggcggcagcggggtaggtaatattccggattttactgcggtggatactttagatgtgccggtaacggcaacagttactgtaacgccggtcagcaatggttgtccgggtacttccggcactttcaccattaccgtgaatcctgtaccacgggtaattgtgccggaaaatcaggggctctgtaataatgtgatgactatacccatgcatttcgaaggtaatgtaacaggcgctacgtatagctggacgaatgaccatccggaaataggtttggcggccagcggtagcggcgacattcctgcattcctggcaaagaatactaccgactctgtgctggaggccattattacggttacaccggtagccaatggttgtccgggtacaccacaacgtttaaccctgacggttagtcctactccgggagtagtggtgcctggcaatgcagtggtctgcaatggagataccgttacccggaaagactttgcagcaagggagcaggacgcgatcttcttcagctggacgaacgatcatccggaaattggtctcgctgccagcggtataggttatatttcaccgtttgccgcagttaacactaccaatgcgccaatagtcgctactatcctggtacggctcaattataacggctgtgaaggccctgccagcaggttcactattactgtcaatcctacggcgatgattacggtacctgccagcatatctgcttgtagcaatgaaaaattgacacccgcagcattcggcagtaatgtaaacaacactacgttcaggtggacaaataccgcctccattggtttacctgcgagcggcacgggcaacctgcctgcatttacagcaataaataatacggattcaattatcagggataccattactgtagtggctactacaccggatcagtgtacgtcacaggaacaaatgttcatcatcacagtaagtccggtacccgatgtaaccataccggcaccagcagtacaaaccgtgtgcaatggcgacagcctgccgcctgtattgttcaccagcacggtaacacaaacggaatacagctggacgaatgatcatccggaaataggattgcccgcaaccggcaaaggcaatatagcagccttcagagcggtgaatactactaacggggcgatcacggctaccattaccgtaacgccggcagccaatggctgtagcggagccggtaaggtattcaggattaccgtgaatcctacaccgttggtggctaaggtagcatcgcaggcggtgtgcagcggtggcactgtaaacagtatccattttagcggaccagtgaatggtactgtgtaccagtggaattcagccacaccaacaaatggtattattactgccggtaccggggatatccctgccttccaggcgtttaataacagcgataccacactcgttgaaagggttatagtaacacctgtattgaatggctgtagtggtttgccgcaggaatttacaatttctgtctatccacaggtatatgtacagcggccacaggatctggaattatgtgccggaaataaagctgctgctattacttttaaaagcaacgtagccggcgccttgttcagttgggttaatgacaatccggccatcggcctggcgtccagtggtagtggagatattgctgcctttactgccagcaacaatactacgggaccagtaacagcaaatatcagggttactccatctgctaatggctgcaatggcgaatcacaaatattcacaattgtagtgaatcctgtatcaacgatggctacacctggaaatcaaagtgtatgtagcaatacacttacacagcctgttgttttcagcatgggagccgacagcagcaactactcctggaccaacgacaatccattcatagggctggcgcctgcaggagtaggaaatatcccggcctttgtagccaccaataacaataacgcaatcacgcaggctatgattacggtagtaccagccggcaacggttgtgcaggtaagtcagtcaattttgatattattgtatctccaccggctaccatggacaaaccggcagataccgcaatatgtaaccggactttggtaaccctgcctgctttcagcagccaggtatccggtgtggcctatcgctggaccaacagcaatccggctattggtctgccggcatcaggaaatggtaatattgctacgtttaccgctattaacaatagcaatgcccctataacgggtgtaataacggtgacgcctgtactaaatgggtgcgatggcacaatacagacatttaccatcactgtaaacccaggggcaggcctgacggatattattaccaatgatgttactgtcacttataataccgctgccgtgcttaccgcctccagcaattccgttagcaacccggtattccgctggtatagtgacgcaacgctcacacacctcgtatttacaggcccccggttcactaccccgccattaactgccgacaccactttctatgtaaccgtagcaggctcgggtgtgtgcgagagcagtcctgctgatgcacgttctgtacacataacagtaagtgcaccggctgaaaataaagtggatgtggcagtgaagaaagtgtctgaatcaagacaggtagccgggggagaaacttttgattatactatcactattatgaaccatgggccggatatcgctcataatgtaatactcactgacacactgcctgagcaactggagtatgtaagcaccagcggcgccggtgccagctataatagtgctacacgtgtgttcacctggagtttacctcaaatggaggcaggggcgcagcaggatattcgcattacagtgaaggcgcttagttcaggtgaagtacgcaatacggcaaaggtgagcacaaccgatgaggatacagatctatctaataatacctctactgatatcaaagaattacttggactccggatacccaatattattacgcctaatggagatggtgcaaatgataaatggaggatcatcggattagaatcgtatccgcaaaatgaagtcagcatctttaaccgctggggtaatatggtttatgaaaaacagaactatggtaatgactgggatgcgcacgggcttaatgaaggcacttacttctatgtactgaaagtaacagacagcaatggtaaagtgcaatcgcttaaaggatatattactgtcttgcgttaaatcaaatgactatgaaaaagatgattatttttatcgttctgctattgtacacgaaagcgcttcgggcgcagcaggacgtactttttagtcaatatatgtttaatggcatttacattaacccggcatatgcaggctatagggaacagttaaacgtgcatgccttttaccgggatcagtggcggaatttcccgggtgctccccgcacgatgtcggcggccattgatgccagtgccaacaatgcaagggttggactggctttccaggtaatgagtgatcagctaggtgctgaaagcaacacttctgcctatggcagttattcatatcgtattccggtgggcgaccttgaaaaagacaaccggctggctattggtatcggtctgggttttattcagtacagattggatgggtctaaatttgatccggaaacggttatagatccatcactgatgtatcgcaaaaagacggtactggcgcctgatgtaaaggctggtattttttatagttctgatcgcttctatgcaggggtttctgtagataacctggtagtacaatatgtaaaaaataaacaggatcctgaacactatcttcctgataagaaaatgcattggtatgctaccgctggcatgttgttaccggtatcggaagtaatacagcttaaaccttcttttttattgagagatgatctggccggccctaccagtcttgatcttaacctctttgcgctttttgttgagaagctctggctgggggcttcttaccgcacagcagtacgtttgtacgataagtcgtacctggacaggtcacttacgaaaccggcggcatttgtggctatggcagaattttttatcgcagataaaatcaggctgggatatgcatatgatcttccattaaacaggataggagacttcaattattctacccatgaaatatcagtgggctacttctttggtagccggaaagggaagatgttaacaccccggtatttctaaatagtttaaggtgatgataatgatgagaaatatattttgtacttgcctgataatgggcagcctgtcgttacaggcgcagtatgttctaaaggaagcagagaaagcggcagctgtttatcgtttcaatgaggcaatacccttgtatgagaaggcttacaggaataagccttcctcgcgtgctgcacgtggtttggcaacggtatatgcatcgatgcgtaatcatgagcaggctgcccgatggtatgaccaaacactgaatttgccaggttatatcgcagatgacatccgtcagtttattaatgagcagatgtataatgggaaatacgacagcgtacggcaggcgcttcacaagtatgctgattcactgcctgcaccattgttgtcgcgttggtatgcctcctgtgattccgccgcctggtggatggctcacccggtggatgccaggctgcaaccactcagcgcgtttaatacagcggccgcagaatggggcgctttcccttataaaaataatcatgtcatgttctcatccgacagggcgcatcccagtaatggctatacaacccttatccgctggtataaccataacgatataagtttgcatacttcagggtggactggcaggccgtatcttcagttatttaccggaaatccggctgatagcaatagcgtaaatatcttaccagataaaaatatcaacagtggttatcactccggtggattatatttatctctcaatggagatgttttattttttaccagtacaagagacataaaagggaaaaacagttttttaaagaaggatcagccctatacggtgaatatggaaatattcagtagtatttaccgtgtagctgacagcagttggacgttccctgccaattttaaatacaataatccgctgaaatattcggtaggagacccctttcttactgaggacggtcgccgattatattttgtttctgatatgcctggcggtttgggaggaacagatatctattatgcagataaacaggcggacaatacatggggaaatgccgtgaatatgggggacagcatcaacagcacaggtgatgaaagatttccttttatcagcacacgtggccatctttattttagcagcaacggacgggtcggcatgggaggactggacatttataaggtagcggatttcggtaatgcggtatctatgcctgtaaatatgggatatcctgtaaacagtccacaggatgattttgcggctgtatttacagatagtatcggttatctttcgtcagataggacagggggtaaaggcagtgacgatttatattctctgacattggaaaactaccggccaccgttatcgcagaaagagactttacctgataagccagtagtcatcgttcaaaaggtagtcgttcctttgccggaaaaatggatattggaagacatttactttgattttgataaatggaatatccgtccggatgccactattggtttaagcaggcttgcgactattatgaagcagcaacctgctatccgtgtccaactgggcgcatacaccgactgccgtggcagtaatatctataatcaggtactttctgagaagcgtgccggagcggcagcctcctggctggagagtaaaggaatatccccgacgagaattaaggcagtgggatatggggaaagtaatccggtaaaccgctgtgtgaatggggtaatatgtacagaggcagaacatcagcagaacagaagggttgaggttagaatagatgaggagtaacccctgtataagcggtgccggttattcggaagaagaacatccgctaatcaacagacagtaatcatagttgtaaagggactttcagaccttatcagcacatcgatccaaaaataaagcggcctataaaggccgctcatactaagcatagtcatcgaaacattcaactttatagcatttaatgatattttttaccggtttggagatgaaacaccccaatgctgaaaaagttcatttctttaactgtaacacccaatttaattctcatttgtgaaaaagagcgtaaggtgaaagggtgaattcgacagtagtaagagggaattgtaaaaattatatattgtttgcactagcgctttaggcaaacgaatcttcttcaaggagcacgattaataaacatttaatcctggtttttgttgttaatgatattacttccttttccttgcataaacaaactaagttgaatgatttgataattcataactaattaggtttatgcgatttattttctctctcagatcggcttatatttttctgttgttgattctatcaatcctccgaagcgtagcgcaaatcagtgcaacgcatattaattccatttctactccacccaaagtgaaaacctccgtaggagacctggtatttaaggatggtatcccggacgcctcatctgcacagcggatttatgaggaatcagattatttacatggagtagatgcctttgtaaacggctatgctgttgtatctcaatgggcaatcaggcaagggtttcatgattttggagtgaaggataatgatgtgttggtcttttccaaattaatggatgcgagttcactatttcttacagccaatgcagatacgtattacttctggacctatgtggatttatccaaaggtcctatggtggttgaaacgccaccgaacacacttggggtaatagatgatatgtggtggcgctgggttattgattttggtctgccagggccagacaggggccagggagggaagttcctgattattcctccggattataaaggacagttacccgaaggcggctatttcgtatgtcatagcagaactaaccaggtaggagtattgggcagggcttttcttgaaaatgatgatccggaacctgcggataaaaatgtaaaagagcatttaaagatatatccctatgttcccggcggattgggaaccagtattggtgcttttctgaatggtaccgccaaattgggcgccaatgcaactcctcctgcattacggtttgtagaaggtagcgggaaaagtataaatacaattcctcctgccgatttttcctttttcaccatgttgaacgacgccgtacagaaccaaccagttgctgcactggaaccggaaattgctggtcactttgctgctattggcattgtcaaaggaaaaacatttcaaccagatgctaatacccgcaaagtattggagcgttccgtaactatggggaatgcgatcagccggacgatctccttcaggcccagaacatcagaaggtttcaattattatggcgacaatagtcattgggtgaatcccctgtttattggcggttatgagtttcttaggccaccacctgaagtaacaaaacagggcatagagcagtaccctgatgatggagcaagaaaactcaatgcaagaattgccatgttttatgctgccaccggtataactcccgccatgtgtatgcgcctgacgaacattggctcacaatatctgggtgcttttttcgatgcagccgggcaagcctttgatggtgctgatacctataaattagtactacctgctaatatacccgcagcaaaattctggtcattgacactttatgataatcaaactaggtccatgttacaaaccgaacagcatttcccgcgtgctggtagtcagaactaccccacaccagctgcgcaaaaacaagcagatggaacttacacaatttacttttcaccgcgcaaacctgcaaacgtgtcagatggcaattggattcaaacagttcctggaaaaggctggtttgtgctgttgcgtctctatagtccgctggaaccattctttaacaaaaattgggtggtgccggacattgaaccggtaaaataaaaactgtgtttcatttcaccttgtaatacataactatagcgacatgaagagaataagtttatacctagtattattatttatgatagcagcttgccaacagcaactataataacacatgataccggtaaccatgaacagcaggaattgaattcctcctttaaggtagagatgacaggagagttgccaagtgctgcatccactggtttattatttgatgaaatggattaccaataataagcattggccggattgaaggtgggactacgttttagtaatgaccgattcgtcccaacgggcagcagactatgatgaattctatcagcgggcgtcctacttctttgaagctgttacctattcaaaggctgtgataacaaaatgccaaatataggccaggcatacgtaggcgcctatcaggatcaaaacagacaatggctggatgaaggtctcactgcggcctcagtcggcaaaaaggtcgccaggcttccgcttgccccttccgctgcgcttcagggtctgcgctccaccctgtcacccttttcgcactccctcagcctccgttcgggtagctcccagtctggctaagggttgcttctaacattggtggcttttatgcccgccatcccttcgctaccc

SEQ ID NO: 8 - DNA, 415863 bp, Chitinophaga pinensis
  source 1..415863: mol_type = genomic DNA
taacggattgataatcattctcaactgccatcacaatggctaatttttgctcaaaactgtattttctgcgtttatccataaaaatgccccctaaaagtgtctaacttttagggggcagtacatatattcgcttttatctcccttaatcctttaaaaatccaaaagtaaaaatccagctaatcagtaaaatcagcgtaatcctgagccaagacaaaatccgctctacgccatgcggtcaactactttctttagcgtgagtccctgcactatgatggagaatagtaccacaaagtagctggcagagaggataatttccttatagggagattccggcaacgacagcgccagtgcaacggagatgcccccacgcagtccggcccaaaccaatatggtaatgcttttataatttgttttcagggagcgctttaatacaatggcggggatggtaatactcagcgcccgcgcaatcagtacaaatacggtggccattaaaccggtgaaccaatagttttgcaggaagggcatgatcacaatctgcaacccgatcatcacaaagaggatggtgttcagcagttcatcgatgagactccagatgttgtgaaaatagtgttgtatttcttctgcattttttgttcccagggaagtattacccaatatcaatccggcggaaacggccgccagtggaatagatacgtgcagtatagcgcctaccacagaaattaccattaccatggataaggataccattacaatgatattgaagtcgtctacacgcttcatggtcctgtaagccacaatagcggaaacaacacccagcaggatcccgccgaatacttcctgcgaaaacagggcggcagcatgtgatagagaaacatgactatctgtttgcccggctacttctttcaggatcacaaataacaggatgccagtaccatcattcagtaaagactcgcccccaataatggtttcaagggcgggcgggacttttgatttttttaagatcgataataccgctaccggatcggtaggtgaaatgagtgcgccaaacaacaggcaatataccagcgggatgtcgatgtgcagcagttcagtggcccagtacaacaggaatccgaatataaaagtagagccgataacccctacggtactcaataccagcacgggataccgctgtgcttttagtttattgaaatcgaaatgcaatgcgctggcgaaaagcaggaagcctaacattacgtccagcagcgtaccggtgaaatcaataccgttggtgacatctttaataaaagtgaatgcgccggggaaaattttacccgtcagggaaatcagtaaagataataacagcgaaaccacgatcacacctatggttccgggaagtttaatgaatcggttgttgatgtaggaaattaatgcactaatggtaactaaagccgttatcagcgtaaatgtgttcataagtaatcgaataatgccggttaaaaaatcaggttcctattgttgctacagtagttttaaaggtagaaaaaaatgtagcaaatcaaagtcccaccggcattataggattattttttcctggaagacttagcatttacgttaaattctaatgccattttaatccagtattgtaattgtttttttgtgtgcagctcaccttcatctacaaaaataaatcctttcatttctttgcccccatgaatcattacttcggcgccggaagaggattcgactacctcgtctgatttagcaggatcaattcttaccatcattttatcgggccgtacgcccacgcacattttatcgtttaccatgaaacacaggccaccaaacattttcttttccgtgatgttatcggtggaagcataaaggatttcgcgtacgcgatcagcgagtttttcattgaatgccattgagctattttttgggagatatgaaggtacgacttcctttaattaccataatattgtaatgaaatttataactatggcaggattggatactttttaccgcttcctgaagcagctgcatccggtgtctgatgacgactggcagctgttatccgaagggttatttgtgcaacaggtgaaggaaggagcggtgttattgccggagggcaaagtgccgcgggagctgttcttcatttgtgaaggtatattgcgcctggtaaagtatacggatgacggagaggatattaccatattttttctgaaagaaaataagtgtgccaccatactgggcagttacctcgaagaaacgccctcgccttacgtactggaggcggtatgtgatgcggctgtaattgtattgcataaggaatacctcatgaggctatacgaaaagatcccttacctcagatccctgatagatcagattacccggcaaggcttgctggaaaaggtgctggcccggaacgaatacctgggactggatgcctcggagcgttaccggtatttcctgcaaaaggaaccggatattgtttcccgtgtaccattgagtactattgcgtctttcctgggtattacgcagcagtcgctcagccggatcaggaaaaatggccgcctttaatgctttttaccatttgttaaatgacgcctgctgccggctgccgaattttgtgttcataaaaaattataattatgaatacggatctgacaggaaaaaaagtattggtattgggcggttcggccggcattggtttggcaacggcacaggcggcagcggtggcgggtgcaacggtgatcattgtttccagtaatcttgaaagagtaaataaagcattggcgacgttacccggaaccgcgcagggctttgcgctggatctggggagtgaagcagcggtgcgtgacttctttcacacatcaggcgcctttgatcatctggtgtttacagcaggtggcgccttcccgttcgggcaggtggaaagccttacagccgcggaattgcaggaagcatttcaattacgttttttcggtgcattcaatgccgtaaagtatggcagtaaaaatatattgccggggggatcagtggtattgactaccggcatcgccaacttaaggccacagcagggatgggccgccggcgcctgcatttgtggcgctatggagggcttcacccgcatgctggccatcgaactggcgcctatacgtgtaaacgcggtgtcgcctggtattgtgaaaacagcactctgggcaggaatgccggaggccgatcgcgaagccatgtataaacaggctgccggcatgcttccggcaggccgcgtgggccagccggaagatattgcgcaaacttatttatacctgatgcagaatggattcagcacggggcagatagtagtggcagatggcggcgccgtactggtttaatgcgcaatggtagcggcgccaggcgccgctgccacagccgttttgatattccggcggcataccagtaatataaacagtgccagcagggaagtgccgcacatggtgatcgccatcggcgtagccgtgtgcgtgttatacaggcttaccaccgtggaggcaagcgcacctattcccatttgtgtggcgcccatcagggaagatgcgctgcccgcatttttactgaacggggcgagcgataatgctgtcgtgttgggattgataaagcccaggcagcaaaggtagatgaacaacaatacgatgataccgggtaatgataaaaagttattccaggcgcagacaatgaaaacaagcccggtgatggtttgacaaagcagcgccaccggtactatctgctgactgctgaaccgtttcaacaacaggctgttcacctggctggaaccgatcagtcctaccgaaaggcccgcaaagatccaaccatacgctttgtcactgagcttataaatatccataaacacctggggggaagctgatacataagcgaacagtcctgagaaagaaactgcgcctgcaaaagtgtaggtataaaactgaggttcactcaccaccgacaggaagttgctgataatgggaccaggcttcagtgacatcgacgtgtccggcttataactttccggcagccagaggatggtggctatcaggatcagtgcgcccataacgcccagtaccaggaatactgcgtgccagctaaaggcgctggttacataactgcccacggtaggggcaatcatgggggacgttcccactacgagcatcagcagtgcaaatactttggcattgtctttcacggggaagaggtcacgcaccatcgcaacagaagctactgccgcggcgcagctgcctatggcctggataaagcggaggataatgagcccgttcagggaagacacatacatacagccgatagaagaaatcacatacagcacgagtcctatgaatagcggcttcttcctgccaaaccggtcgagcaacggaccatatagtaattgtcctgctgaaatcccaataaaaaagctcgaaagcgataaggccaccctggtaggatctactcccagatcctttcctatagccggaaagccgggaagatacatgtcgatcgagaaagggcctagtgctgtgagcgtaccgagaatcaggataagaaagaaatatttcgattttgaaagttcgttggtcaaaataatatggctttaaaaaatttccctgcaaaagtaagaagaaatacgccccttcggatgatgtgactgttatcttcttttgattttaccgtggggagacaagcattcgcgtatttattcctgtgtaatattgatcaggaaatcatacagtcctgtttcgccggggatgttcagtttcttgcgaagccggtaccggctggtttccacgccgcgtacggaaatacccatcgactgggctatttctttggtggtaagattaatgcgcaggtaggcacaaagtttaagatcagtggtggtcaaatccgggtattgttttttaagggtgcgcaggaagttgttatgcacttcatcaaagtgttgggagaactgcgcccagtcttcttcgttattctctgcttcttcaaataaccgcatcacttttttgaaagaaggaagcgcttccgggtcattggttttctttacgctttgtatcagctcttcacggatattggatatcagtttgcctttttgtaccaggtgcatcgtggcggtggccagctctttatttttatgttgtacgtctgattccagtttttcattgcgcagccggatcagctgtttctcgtttctttccagctccagctggtgttgaaaaatgagatgttgttgttcctgcagatgtttgtctttctgtgcagcaaattttttcttctgacgccggtacaggtaccaggtcagccccgcgagcaacagtatatacaccgtcttcgctatataggtttgataccaggcgggtaaaatggtaaaagaataactggcgggagcggagatattgccgaggttatcttttgcctttacccaaaaagtatatttcccgtaagggagattggtatattctttttctgttttggcggtccattcgccgggttgtttatcgaagccggccagctgatagctgtaagtgatatgattgccttgttccgccgggggagccgtatattcaaaatgaaaactgttgaacgcattggggagtaccactggcggctgcgcaccggccgtttggtagccgccatacagcagggtgtctttccggctggtggcttttatttgtccgagtaatactgacaggccggcatcatgacgggaatattttttatagttgagatgataaatgcctttgtcgccgccaaaaaagatattctcctcattaaaaggataaatgaactcaaagccgccaacgattttcccggtgagttcggggaaccaggtaattgtttgctgccggggtttcaatactcccggctttttatctgccaccagccagatgttgccgctgctgtcttccgaaagatattgcaccgctgcatttttcagcggggcaaacaatccctgcgacggaacaaattgctgccgggcttcatcaaattcatagatgcctttcatggtggcggctaccatccgttgttgaatacggaaaacgtaattattgtaggtggacggcagcccgtctttttgcgtgaacaagcggtagctcagggcggtgtcattttttagggtgagcaggtatacacctcggtaggggtgggaggaccagatacgttgctgtgggtccatcgccaggaagcggagggattcgtataaaccggagacgtgccggttgacacgcacctgtgggccgttatagcggataatagccaggccattataacagccggtaagtatgttgttggaaagcggcaggtaagcccagcagcccaggtctttcagcactgcagcagccttgttgccggtgatttcaaacgttccttcctggtgggccatcagcaggtgggagccgatagcagaaaggttccatacctggccacgggtgttggccaccggctgaaagttgcctttggaatagctgaggtctgcaacggtgtccagtggtgtgctgtatagtccatcagaagtgccgatgtaaaggcgctgattaaacacctttgccgcataagtggtaagcgaattatgtttggcgggtagtatctgtttaatggcggtattgtaacgcagctgatctataccgttgtccagcgccagccagatattatggcggggatcagcaaacaggcggagcacattattattctgaagaccctcgtccatgctgaattgctggatcacgctgccactattggcattgatgataaagcatcctttggagaaggtgcccaccgccagctggccgtcacccagcgggatggcgcaataaatacggctgctccggaaaacactatctgctgctgtttgcagcgggagtaactgttgcccggtgatacggaaaagcccatccttgagggtggcaaccagcagggtatcatttttttcttccaggaaagcggtgaccaggagagatttgccctggaagccggtgcaaacaggttgccatttaccgtttaataatttcagcagtccctgtttcaggtcctgcgcgtaaaggccgtgggccgtgctgcccattattttccattctacgggagcattgtacacgtctatctgccggttacgccagccgaatattttattgttgcttttgaagtaaacgccattgttgaataatgcaatattccagatgtctgcaaattctgtttgcccggcggggatatactttttgagagaagtatattccaggataccatttttattgggcagataatacccgaagtcgtcctgtgcgccaacataaatcttcccgtccggcgccacctttaccgcgcgcaggcgggtgttgttgggtacggggtacagcttccagtaattgccgttgaaggtaagaagcccttcattattggcgaaatacaggataccgttatggtcaatatcaatgtcccaggtttgcccatttccctggtattgggctttactgaaattcaccacagcgggtagtccgattgtattctgggctaataatatttttccgtggaataaaagggccagcaacaacaaatgcttcatctaaaaagcgttttactaaatgtaaaatttttttgctgatgtaggtaagatgtaatgaagatagattagctatcaatgttttaatgtcctttgaagtagaaatgacgtagtgccggaaatgattttatgcttttaaatagggatcttggatattcttatttttctttttaaagagacactgtacatgctgaaattccacgttatagcactcaccttattgctggcttctgtgctgcctggtaacgggcagggatatctgaaaacccgcggccacattattgttaatgaaaaaaacgagcaggtgatcctccggggaatgggcctcggaggctggatgttgcaggagggctatatgttccgcctgggtaatatcggccagcaatacaggatccgcgaaaagatccgggaactgatagggcctgaaaaaacacaggcattttatgatgcgtggcttaccaatcataccaccaggagggatattgactcgatggcggcatgggggttcaattccgttcgcctgcccatgcacttcaacctgtacacgctgccggcagatgaggagccggttgccgggcaaaatacctggctggaaaaagggtttgcattgaccgactccctactgaactggtgtaaggccaatcatatgtacctgatccttgatctgcatgctgcacctggtgggcaggggaacgatctgcctatttccgacaggcaccccgaaaagccatctctctgggaaagccaggctaaccgggataaaaccattgccttatggcgcaagctggcagcgcgttacgccaacgaaccctggataggcggttatgatattatcaatgaacctaactggggatttgaagacgccggggataaaaggggcaccaaagaaacaaagaacattcccctgaaacagctgatgacagccatcaccaaagccatccgggaagtagatcaacagcatatcatcattatagaaggaaatggtttcgggaataattacaagggcatactgcctgcgtgggataataacatggtgatcagctttcacaaatacggcaacttcaccaataccgcttctatccagaatttcctggatttacgggcgcaatataacctcccgttgtggctgggggaatcgggggaaaactccaataactggttcacccatactatcagtatggcagaaagcaatgatatcggctgggcatggtggcagctgaaaaagatggggggcaacaatcccctggaaataaagctcacgcccggttaccaggcgctcctggattactggaacggcaaagggcccgcacctgcggaggatgaagcctatcgcgcgctcatggaatttgcaggcaataccgggatcgaaaataatatttaccataaagatgtgacagatgccatgttccgccaggtggcttccggtaaggccattcctttccgggaacatatcatcaaagacaaggctgtgatccgcgcggtagactatgatctgggacgaaacctttcagcgtataacgacctggataccgcgagctaccattatacgccgggtgttaatacacaggggaaccgcggacacgcttaccgcaacgatggcgtggatataaaaaaggaggatgatgagtttgtggtatttcatattgaaagcggcgaatggctgcagtacactacccgggttgccgctgccgggaactacacccttaccgtaaaaataaaagcagataccggtagtgttgcccccaggtttaagatcagcagcgatgacaacgtgctggcggctgatattgccgtgccatctgcggggcagcaggtggtagtgaaaaatatccgcctcacaaaaggggaacaccggatccggatagcctttgtgcagggtggcggtgtgtttaccgggatgacctttgaaagaaagtaagaacgcataaaattaactccacgtttgatccattagccttatttgttcaccttttctttaattgtaaattccatgaaagaaaaactgatctccattagcgtaggttccgtcctgttagtggtaatgatgagcgcctgcaaaaaagaggcgaaaacaaccaataatctgcaacctttggatgcccggcctgctgcagtagcagtgcaggcggcagcagcagcgtacacgctgatctggtctgacgaatttgacggcaccagtgtcaacacttccaaatggtcttttgaaaccggtccgggtgttaataatgaaaagcagtattaccagtcgtccaatgccagtgtgagcaacggcaacctggtaatcaccgcgaagaagcagtccgtgaacggctggccctatacctctgcgcgaatgaacaccgccgggcattttaccacgcagtacggccgtattgaagcgcggattaaactggcctccgggcagggactatggcctgccttctggatgctgggcaataacattggctccgtgggttggccgaaatgcggtgaaatagatatcatggagcaggtaaataccagcaacactgtttatggcactattcactgggatgccaacggtcatgtttcctatggcggcacttccagtaccactattactgattaccacgtatatgcggtggagtgggatgccaatgcaatccgctggtacctggatggtaaccagtttgcaacagccaatatccagaacaatatcaacagcacagaagaattccacaaccagttttttatcatcctgaacatggctgtgggaggcgatttccccggacaaacgattgatgaaagtaaactgcctgccaatatgtacgtggattacgtgcgggtatactccatttccaacagcggtggcaatgcgcctattggcagcaccattacgctcaaaggatttaataatgcttttgtgagcagtgaaaacggcacacaggccatgacctgcaaccgcactactgcacagggatgggaacagtttaccgtggaagatgccggcggtggtaaggtggcattgaaaagccagggtaagtatgtttcttcagaaaacggcgttaatcccattacgtgtaaccgtaccagtgtgggcgactgggaaaaatttgactggatagtaaatacagacggcagcatcgccctccgcggaaataatgggcgatatgtgtcgtgcgaaaacggcacgcaggctatgacctgcaaccgtaccactatttccggctgggagtcgttccggtattaaatgatataggttgatggatcgggccggccgtgttaacggccggctttcctatgctgtagatcaactgttccatgatacttcctttacgccggtatctgcctgtatatctgcgatcagcttgcctacaatggttttatccatgcttctgaaacgtaccgtgataaagaagaaactgtctgtttgctcgatgttgcaggaagtaatattgagcgcggtgttttgaaataatttatctgctacctcaatggatttgctccgttcaaaagtgatgatgcggatagttttttgttcaaagcggctgaggaatcttttttctaccggctgcagcagccacaggatgatgatggcaatagcggtggcaataaatgcggcgaaatacatgccgccgccggtggcgagcccgatagctgctaccgtccataatcccgcggcggtagtgagcccgcgaaccacgccttctttcagaaaaagaatggtgccggcgccgataaatcctataccgctgatcacctgtgcggccaccctggaggggtccagtacaatgttaggctgccccaggatatcggaaaatccgtaagcggaaaccatcatggttaacgccgcacctacagacaccatcatgtgggttctaagaccggcagcccagtccttccgttctctttccaaacctattataccgccaaaaaccgctgccagcgataatcttatcaatatttccatccagggtatcatactactaatttacgcaataaattttctttcatcctgtggaggttgtctttctgcctgattacggtgattattccgattatagccgggcttttaaagaagctcaaaatttgtatcttgacatcaattcatttatatttttcgcatgcttccaatcaaactacgtttactcattgccgcagcgcttcttttttccgttacaacccgggcgcaggtaaagttccggacaatagcacccaacgtcacccagccgggattaaagacagtgcattcgccgcatcttgccgcagaacccgctgtgggaaacaaccgccatcagctgatagtgatgattcccggtaccggcggcacggccactgatttccgtacattcgacagttcttttgctgccatgggctattatgtgatcaccccggattatatgaacacggtgatcaccacagcgtgttccaaaagtgaagacagtacctgttttgatcatttccgccaggaaattatgtttggtacgccggtgagtgataaggtagatgtagattctgccaacagcctggtgaaccgttttacaaaactggtggtgtacctggctgcgcaggatcgtggctggagtgagtttgtacgtaatggacaagtgcgctgggataaagttattgctgcaggtcattcgcagggagcggggcatgcagcatattttgggaagcagttccgtttgcgtggagtgctgatgttttcgggcccgcaggattacctgcaatattttaatgcgccggcgcattggcagcaggagcgtggtcgcacgccggtgaacaggtattatgcgtttctgcatgttgcagacccgtttaattaccagtaccaggtgcaggatgtaagtgcggtgaaccaccaggcggtaaccgataccacgatggtgcagccgggaatgcccgttcactccaggaatagtatccttgttacggatgtggatcgtaaagataaacacggatctacgctgggaacagacttcatagccgtgtggaaatatatgatcagcggggctaccaggaattaataaggaactggctaacggtctcgtgtaaacgatgaactttgtcctcctgttttttattctttatcttcgcgggcgttcgttaccattctatgtcaaagaagaagagaagaaaaaagaagaagcaccagggaagcagcagtttagccgttatcgttatattgatcatcgctgcatttgcggtgactacctgttcccggaaaattaccggagacaatgaaaaatctcctccaaagaaatcatctcacaaaaaaaatactacttccggcaccagtgcatttttactggcagaagattttgaaccgggatccaaaacaaattataacagcggggacgtggcattatccagtggtacctggaagtttaaggatgccgtcaccggcaacctggaggaagatcataaaacaggtacacaggcattgcgtatccgggacaatggtatggccgggatgaaattcgatatccttgtaaaaggaacggtaacggttacactaaaatttgccgggtacggggacgacaaaatgggcacatgggagttgtgggcatcagtgaaccgcgggcaaagctattttcgtgtgggggatcccgttagtgttacgtccggtgtgctgaaaacagccacttttaccgcgaaaagtacgggcactatccgttttgatatccggaaaacagatcccggcagcagcaggattaattttgatcggttccgggtcactgccggcggaaaggacacatcggttaagccggtggagaaaccggcagggagcgacgacgacaacctgttactgggcaatcccagcgatgccagtggatcgttggtgatggcgaataattacctgatggataaggaatattacaagctgtcgtataaccgtgacaggggaacgcccaattgggtggcctggcatgtatcgcggaaggacctgggcaaaatgtcgagggccaatgatttcaggccggacgccgatattcctgggaactggtaccaggtatcccaaactagttatatgggcagcggattcgacagggggcataattgtccgtcgggcgaccggacggccacccgtgccgccaatgaatccactttcctgatgaccaatatgatcccgcaggcgcctaaccacaaccagcatttatggaagaacctggaagaatatacccgggagctggtgatgaaagggaacgaagtatatgtgatcatgggcagctatggcagcgggggagccggcagcaagggactggccaaaacaatagacgggcgtaaggttaccgtgccggaccatatctggaaggtcctcgtaattttaccggaaggaaacaatgatttgcagcgaattaataagaacacccgtattattgcagtgaacacaccaaataaaaacgatgtaaatgcgaggtggagcgcttacctgacatctattgaagagatagaaaaggctaccaggtataagttgcttgacaaggtaccgctggtgataagacaggaattagtaaagaaaatagatgcaggacaggagagaatgtatcgttaaaaaaaatattatgttgttctgataattaaattataaattgcataaaattattatgtttttgtagtttgtaaactaatatccaaaaaataaatcatgataagttcctataaaaaccagattggcataattttattgaaagtactgtagctacatgtaacttattgaagccttagatcgttattataattagaagctaacttaaagtataactggccgattattaatggaaataaacctacacttttcttgattatatgtacatataacaagacaaatactgtgtacacaacgaaagaaatggcgtaaaataattaggggtaaaatggcgttatactagagaagcttaacaatatgagctttttaaacattaattttatatctaactaatatgggtgaaagagtgtcggtggccttacttgttactacatacaactggccggaagcattaaagcttgtgctggatagtgtactggtgcaaaccgttctccccgacgaagtcattatagctgatgatggctccggagaggctaccagggatgttgtagaggcattcagacgaaaaaccaatattccggtgaagcatttctggcatccggacgaaggtttccgtaaaactatcatcattaaccaggcaattaccggtacttcttccgactatattatccagattgatggcgatattgtgatgcatgagcttttcatcagggaccatatcagtgaagcggaaaaaggatattttatccgtggcagcagggtgttgttacaggaagagattaccaggaaatacctgaacaatggtcaatttgagcgggtatcttctttcagcagagacgtgagaaaccggattaattcacttcgcattcctttcctggctccattgctgattaaaaagagtcagcgttcccgtaactggatcggttgtaactgtgctttctggagagaagattttctgaaagtgaatggttataataacgaattgaaagggtgggggcacgaggatattgaactggcagcacgttttatcaattccggtttataccagaaaaaggtaaaattaaaagcggtatgttatcacctgcatcatccttttaattcccgtgtacacgaaaacatcaactacagggtttacctggataccttaaaccacgggattgcctattgttccaacggctacaggcaccatttaacgacggagtaaataatcaaaaaagatatttcataaaaaaggccaccaatcggtggcctttttttatttagttactaaacgtttgcatttcaatgagccgtttataaataccgttgttgctgagtagttcctggtgggtgccttgctcggccacctggccgttatccagtacaatgatcaggtccgcgttctgaatagtgctcaggcggtgggcaatcaccagggatgtgcggttcttcatcaggttattcagcgcatcctgcaccattttctcggattcggtatccagggcggaagtggcctcgtccagcagcatcagcggcggattggagagcacggcgcgtgcaatgcagatacgctgccgttgtccgccggagagcttggaccctttatccccgatattggtgttgtagccgtcttcggttttgctgataaaatcgtgtgcgttggcaatcctggctgcggcctctacctcttccatggtggcgtcaggtttggcaaaagcaatattgttaaagatggtgtcattaaagaggatggactcctggtttacaacgcccatgagtgcccgtaaagattccattgtaacagacttcaggtttttgccatctatcaggacgctgcctgactgcgggtccatgaaacgggggatcaggtccatcaaggtggattttccgccgccggaagggcccaccagcgccaccgtggagcctttgggtatgctgaggtgaatgttattcagtactttcttctcgccgtaggcgaaagaaacgccatcaaaacgaatctcattggtaaagccgtttaaggtagcagcatcgggtgcgttggtgatagccgattgctgatcgatcagctccagcaccctgtcgcccgccgcaacgcctgaatggatattgctgaacgcagtggaaatagcttttgccgggcgcataatctgggagaagagggcaatatatacaacaaaggtagatccgtccatatccccctggttattgataataagcgaaccgccataaaacacgataccggccaccattaagacccctaaagtttcagaaacgggcgacgccagttgctgtcttttagccattgagcgggatatcttggaatacttgcggttttgttcatcaaagcggttggtaataaatccaacggcattaaatgcctttacgatcctgatgccgttcagcgcctcatcgaggtagctgatcatcatgccgtaagtttgatgggaagcggtagcctgttctttcagtcgttttacaatccgcgatataatgaggccggctaccggaatcaccagcatcgataccagcgttaatttataggagataaggaacaggatgacgaggaaagagatcaattgggccggttctttaaataacacctgcagggtaccggttactgtatactgtactacctggacatctgatgcaatcttagaaatgatatctccctttctttcattgctaaaataaccgaggtgaaggttcattacattgttgaatactgatttacgcaggttcagcaaggtttgtatgcgcaggctttccatggtacgatctgcgaaatagcggaacaggttgcctattaatactgaggcggcaatacaggcgcaaacaaattccaggcttttgattttaccatattcactggcaatagtggtggtgtaatgtttaaatactttgaaaatatcaaaataattgtccggcatgggaacaattttctgattgaggtccttgttgaacaacgtttccagcaaaggcgccagcaatgcaaggttcagcgtgctgaatattacagacaacagtacacagatgatataggggatcgcaaatttattaataggtttagcaaatgataataatcggaagtatgtcttcatattttaataataatcgtataatgattaagacggtgcataaaaaaaaccgcatcgttgctgatgcggttccttaagttttaatttcctttttatcaataacttaaagaatatttttcggtcgcacattcaagccagcagatcaccagtaaaaactgcaatcagggctcaaaaatagcccttttggcttaattgtcaaaagatttgatcgccatcggctggcggcgttatagctgcgtgaggatttttagcgccccggtgtctttatattgaaccatcagttgtttcaggtgctcttttaaggtagcggtgagtttctctgtgcctttccggccataaagattgtttacctcgtgcgggtcctgcttcagatcatacagttcccagctgttggactccccgtagaagcgtaccagcgtgtattgttctgtacggataccgaagtgcgggtatacatggtggggctccggaaattcgtaatagtggtaataggcttcttttctccagggaacatttccggcatttgctttcagcagcggtaaaaaggaggtgccttgtatatcagcgggtacttttacgccggcgatgttcaggaaagtgggggcccagtcgatgttcagcatcagctgattgatggaggtaccaggctttattacgccggggtatctgatcacaaaaggtgtacgtaatgattcttcataaataaagcgtttatcaaaccagccatgttctcccatatagaagccctgatcagaggcatatacgacgactgtattttttgaaaggcctgatttatcgagatagtccagcagctggccgatgttcctgtcgagcgattttgccgtggccaggtaatctttcaggtagcgctggtatttccattctacgagggcatcacctgttagtttttgttcatcaaattctttgctgatcttattttcatagtaatcaataaatgcctttttttgttccggcgtaaagcggccgtagatccctttttcgtaattggcatgcactttcaggtcttctttcaggcgcatggttttatcgatggtcatgtcctggttttgtgctgccaggcggtttttgtaatcatctttgaaagtggccgggaggggaaatgttttatcgtcgtatgcaccgaggtcctggacatccggcagccattcgcggtgtgttgctttttcgcctactaccaggaagaagggtttggaagtatcgcgtttgttgagccagttaacagaaaggttggtaataatattggttacatagccttctatgcgggtggtgtcgtttggaccgatgatatcagggttgtagtattggccctggctgttgaggatacgccagtagtcgaacccctttggcaaactgcctaaatgccatttacctatccaggcagtctggtagccgttttcctgcagcagggcagggaatagttgctgttctacattaaaccttttctcattgagcgtgtagccgttgatgtgactatacttaccggtaagcagggtagccctgctggggccgcaaatggaattggtgaccagggcatttttgaaaatggccccctggctggcaatccggtcgatgttaggtgtttgtaccagtttgctgccataggcgctgatagcctggtaggcatggtcatcggagaaaatgaaaataatattagggcgttgttgctgcgcatagctgctggcagtgaagaggagtaataatccccaggtttttttaagatagtttgcggagaagaatttcatgttcaaagttttatcttttgacgggttatgttccgtggttttatcaaagatattttagcggccaccctccggcgaccgcatctcaaaaaaatcacttttccgccaccaccttaaactcctcaaacaccacctcaaacggcaacttccccggtgcagcggccacagggcctatctgcactttaccaccgggaggaaaataggccagtcgcagcatatcaaatttcttattatcaaaggaatattcaatctgtacatagtcgcctttacgcagtaacttcagccacatgcttttggggctatcgtggcgcggaactaccgaccagtcggatacttcacgggttaccacggcgcttacgttctgtacgccgtctacatattcgataccggttttaatccagtttttggcgtccttgcggatcatcaggccggcctggtggaacaactctttataatgtccggtaatttttaccgtggcggtaaaatcgccttcctgttcctggaaataaaaagggccgttatcgcggatgaagccgtagtgggttacctgccagtagtcggtaccggggtcaacggtcacgtttatcttgttgtggtctgctgaccatttctgaggagtgttataccattgcattgtttgtgcttttagtcccatactcatcgctatgaaagcggataatgctaccagttttttcatcatgtttccgtaaaaattttctgtaagatgataaatattctccggaatgggtaatttttagtgatgggtagctgctccggatttgttaactttaagaaccctctttaacccgcctgttaaatgttatgaatatgcgcgaagaaaaccctcaagtaacaaaaagaaagtctgttgccattattgtagcccatcccgatgatgaaacgctgtgggccggaggtaccatcctgtttcatccgcagtggaactggaccatcatcagcctgtgccgcgccagtgatacagacagagcccctaaattttttaaggcattacaattgtacggagcacaaggagttatgggagatatggacgatggtcccgaacaaacgccattgccggaagaggtggtggaaaaccaggtgctggcgttattgccggtgcagcattacgacctggtcatcacccatcatccgcgcggggaatatacgcggcacctccgccacgaagaagtaagcagcgccgtgatccggctgtggcaacaaggcaggatcacagcagatgagctctgggcgtttgcttatgaagacggattaaagtcctatttcccggaagctattcctgaagcaactatttatcatgtgctggataaagatctctggcaacgaaaatacgaggtgatcactcaaacgtacggatttaaggtcgatagctgggaagcagccaccacgccgctggcggaatcattctggtgttttaataacagcatggaagcccatcagtggctcaacagtttaccgtttgaattatgaaagtacttttgttatttgattatccgccggctcccggtggactggcaacacaaggaaatttattgtaccatggcctgctggaaataggtgtaactgcgctggcggtgcactacgactcaccactggaaaaggaatggtactacaactcgtttaagccggatgtggtggtgggcgtaggttactggggatattgcccgcagttgatcctgcatccgcagcaatttggtgtgcagccggttccgtggctggtggccgatggatatatcgccaactaccaggaggtgctgaataaactgccgctgatcctcgttacctcgcagtgggtaaaggaaatgtatatacgcgacggcatcaacggcgataaaatcgccgtactgccggttggttgcaataccaacaggttcgcgccgctgcctaaagatcatccgcgggtgaaagccgtgcgggaatcaatgggcgtggcgccggatgagctgatgctgctcaccgtaggcggcgacgcctgttcaaaaggagccagggaagtcatgcaggcgctgtcgcaactcagcagtgaagtgcccggcaactggaagtatatctgtaaagtatggccgcagccgcgcaccagcatacaaaataaagccgacctggcactggcggaagaactggggctgggtggcaaggtgcaatatattaccagcattgtttcaagggaggagatgccttatctcatcaacgcctgcgatatttatgtggccccatcgcggctggaaggcttcgggatgccacaggtagaagctggcgcctgcgaaaagccggtgatcggcatccgcgcaatgggcatgctggatacgctggtagatggcgaaaccgcactgctggccggtgtggcagaagaaattgtgctgaatgaagtgatggttggtaaagagtcgggtttcgagacggaaaagaaggtcgtattttctacgccccgtacagtggactaccgggcagatatcaacgatatcaggcagcatttgcaacggttaatgacagatgccgcctacagggaacagttaggaaaagctgcaaggaaaagagtaatagcaaattttgattaccggttgatagcaaggcagtttgtgcagctgatgcatgaaaaacttaatatccgctgaacatggaagcttcttcctggttaaccatcaacgcagccagggatgccgccctgaaggtattgctgcataatgtaaacggaccgtttcacggcctcccccgcactgcgggatgtggatatcctgagccatatacaagggatctgctgctgtcctttttaggcgtaggcgttaccggcaaccccgtgctgatcaacagcatccggaaggtgcttgaaacactggcgaaaaatcaaacgccacacggacatatcccttctctcgtacacgacaaacaggacctgggcgcgagcgacaccacgccgctcttcctgctggcagcaggcatgtatcgcaagctgtcgggtaatgagcagttcctcgaagaagcggtgaacagatcattgcagtggatggaataccaaagtccttcagatcgttacctggtggcccaacagcctaccagcgactggcgcgatgaacaatgggtgcttggttacggcctctttgtaaacacgctcgtgtatagttatctccgcatcctcgggcatcatgaacgcgcagagaaagtacggcaggcaatgggcagatttaccatcaccggtggggtgcagcaccggcatgtacacgaaggactggtcgtaaaacacaaaccctattacgccatgtggtcttataaggtattgagcagcgaacggttcgacctgctgggcaacagcctggccatcctctccggcattgcagcccccaccagggcagcggaaatggtatcctggatcgaagacgagtgcgcggaactgataaagaataaccaattggctgtaaaactgccgcctaacttcttcccctatacgaaaccgggcgacaacgactggcacgaacggtatgcttcttttaatcttccaggggaatatcataacggcggcatctggccttttatctgtggcttttatgtagctgcactggtagcggcaaaaaaataccggctggcagaagaaaaactgctggagctcacccggattataactatctccaacagcggcacggtggattatggtttcaacgaatggctgaaagcccaggatggtaccgcaaaagggcaggagtggcaaacctggagcgcagcactgtacctgtatgccgcgaaatgtgtggaagaaagacgtaccccgttttttgaagaaatgagaatgcggtaacctgtttcatgataacttgatgaaagattagtgaaactcgttcgtcaattgatggtaactttacgcgcattatcccttgtttaaacttatgaagatgaatacttacagatccctgctgctggtggcagttctgagcactacactcgctgcctgcggaagccttgaaatggccggaccggataacgttaccccggtaataccaccgcctaccacaccacctgtaacaggcaataataaaattgaaggtacctggaactttgcaggcgtccgtgtaaacagcatcgccaccatatcggaatccggcgccaaagccacgctctacaacgactacaccaccttcaataataaaggggtaatggtgattgatggaagtactttcaaaattacaggcctgagctattccattgatgcggtgatccggaatgtcctttacatggatggcgtactggtaagcgatatgcaaatgccttttcagatggatatggatccatataatgcatccaacccttataaactggtgggagcagattccatttatttcagcgcaggtgtaatggaaaccccttcctatggaggcggcactacagaagtacaggcggcaggcggaaaaatttcctggagcggagatacgctgttgctgacaatcaatcttaaccaggtacaatctgccgctgttatgtcaggttttgaagtgatgaagctggtaaaacaaaaataaaacagtcaccggttattttccggaagaaagataaccggtgatgatccttattttttgcgggcatcagctgcctgccagatggatttgatcgttgcttcatcattcatcccgtccgggcactgcgcggagcgtgtattggcgcggtatttcaatcttggcatcctgcgtcccaacgtaactacacgggtaaccggcatctgcaaatggccattggcgtcatgcgctgctacccattgatgtgcatattgcaaccagttgtgccggtattgttccggttgctgataaaaccagctgatttcatcaaagccccacgggtaaatggtagtggtatccggcacaccggggtgatcgctgataccaaaattatccaactccaccaggtaaggcattgacgcggctttccagccactgggtgtaataccgcctttgcttctcccgaaaagggcatctgtaaaacccatttccaggataccttcctgtggatgcgcagggaccgatttaatacgcaacggaaacgagttaaaatccagtaagcttttgccatttaccaccataccgcccgatggcgtgtgtgcatcgagtaacacccagtgatggcgggtgtgatcttttgcataggcccgtaatttttccaggaaggccgcccattccgtcagctgcggatcttccatgcctatcagggcaatttgcccgaggtgcagcgcttcgcagcctacttccatataggtgccggccaggaacataaaccagagctgcgtttccacccgcgtaatatcgggtacgctgttgcctttactccagtgattgaccagtttcccttttgtattcagcatgctgtcgtaacggaaacgccggtcttccgacggtaatcccagtgctttgaatgcccatgccggaacaggaatggtgtttacctgttcactgatttgctcaaacagggcggcctggaaaattacttccgggtcatttttctgtacttcctgcaccagccgtttggcctggtgaagaaaatctttgttgttgagcaccgattccccgccccagcggtaaatggccctgcctatgaactttgcgccaatgttcctgatcaggcggatatcatcttccttgttgggatagggcgcatcggaggcgtaaggatctactgaaagaaattcagtcatggtaaccgcatgatccaggtaatattccagagcggggcgggtaatgccttttccgttgaaggagggtggttgtgagcgggcggtcatggcccacaaactaatgcctgcagccagcaatgctgctgccggacgctgagtgaatgctaacatgtcgtggaataaattttgaaaacaagatactttttttcgttttccgggaataacatttttggttgtgtggtacaattgtttttatattggggtcattaaaacgagccagccagcatatgagtttactgccggatactttccccgtcctgtctacgccccgccttcacctgattgaaattgaacattcgcatcagccggatctgttttacctgctcacggataaacgggtgacccggtattatcatgtaatcccgttgagtgaggtggccagtgttcgcccggttattgatctttttaaaaagcgcttttccgataagcagggcatccgctggggtattgcccttgaagaaaaaacatcgttgatcggtttcatcggtttcaataattatgaaacagaagatacggttccgctggtgtttgcgctggtacaggaatactggggcaaaggctacatggccgaagccattgaggccgtggtgcagtattgcttctccaaactgggtctgaaaaaaatcgttgcagatgtattacccggcaacgaagcctcggaaagggtgctgactaaagcaggattccatcatgaggccctggtggtgaaggggatgatctgggacgacaaaggatatgatgttaaccgctatgtaagggattacaaagcgcccgacctgtaagcatctttattgtccgcggttcaggacgcagcaatacgggttcctgtaaacaggaacaataaagacactcacaggaattacagatgtaggattaagcttttttagcggcagttttcttgggagcagctttcttaggcgtcacctttttatcggcggctttgggagtgttggcttgagctttgggtgcagcagctttttcggcagcagctttcttcttcggcttggcaggtccttttggcttatctgtcagtcctgctaacatcgctttagtggccttttttacgttccggagaaactttttctctcccagcttctcttttagttcgcttaatgcggttaatacttcggctacttttacaccagcttcttttttaagatgcttgccggtcggtttactcgaatcagtcatggagcattatttatttacaaaaacaattatattcgaaattaacaattaaataatattggcaatgttaagttttataatgccgtgatttataaagaatattctgatcttagcgaaacggaaatcagctataaattcattatattggggtaggctaccttccttgtgtcggagcttgttattgttttaaccataggggtatgggttcaagagatgttattattataggtgggggcttatcgggtctcaccagtgctattcatttatcgaaagcaggattacaggtaaccgtaatcgaaaaaagtaaatatccttcgcacaaagtatgcggggaatatgtttccaatgaagtattaccatatctgcagtcactcggggcagatccttcggtattacatccttcccggatcaaccggttaatcatttcagatcattatggtaaaacgctggaaacgacgcttccattgggaggtttcggggtaagccggtatgcgttcgaccagttcctgatgcagaagatgaccgaaaacggggtggagttaattgaagataccgtcaccaacgtggtatttgaaaacgaccgcttcttcattgataccaacagctatggcgttttttccgcgccggtggtgttgggcgcttatggcaaaagagccgcactcgatggtaagcttgcccgtccgttctttaatgagaaatcgccctggctggccgtgaaatcccactaccgtggcagctttccggccgatactgtaggactccataatttcgacggcggctattgcggcgtatcaaaagtggaggatgatatcctgaatatctgttacctggtgagttacgagagttttaagaatttcaagcagatagaatcacaccgggagcaggtgctataccgtaatcagcacctgaaggatatttttgaaaacagcaccgcgttgttcgacaaacctttaaccatcagccaggtgtctttcacagataaagaaaaggtactgaatcatatattgatgatcggcgataccgctggtcttattcacccgctttgcggcaacggcatggctatggccatacaaagcgcacagatagcatccgataaggtgctggaatatttttcagctcccacccggaaccgtttattgatggaacagaactatacgaaagcctggaacaaaatgttcagcggccgtatgcgcaccggtcgtgtactatcccggttgttccgcaatgaaaagctttctgctaccatgatgaaaggactgatcctcttccccggcctgctgccgggaatcatccgtcgcactcatgggaaaccgttaaatgccgtaccggaatgcgtgtaaacacccggcaccggagccaggctaccgaaatcatggacgatttcagtatggaaggcgatctgctgaaggctacgttggataaaatcgcacaaatcaacgctttactgggcggcaaccgcgtcacccttgaaggcgttgcggccctcctgaaagatattcctgccaatcagaaagttaccatcgtggatatcggctgtggtaatggtgacatgctgcggcaactgtcggacaccttttgttcccatagaaaaataaaactaaccggcatcgatgccaaccaggccacggtaacgcatgcacggaatttatcaaaagattatccgcacattgagtattattgtcaggatattacacagttatccttccgggagcaacactatgatattgttttatgtacgcttacactgcatcactttaaagaggcagaaatcagggagctgatgaaaatcttttaccggcaggcccggaaaggagtagtgatcaatgatctgcacaggagcgcattggcataccgcctgtttcaactggtatgctttgtgttcaatttaaacaggatggtcagggaagatggactggtatccattctccggggatttaaaaaaagagaattacaacatttatcggcagaacttaatattgatcagtattcccttaaatggaaatgggcgttccggtatcaatggataatcaataaattatgagcgttaaaattcagactgtcacaaaagcactaccgccttactcaagaaccaccgccgaaattattcccttcctatcattatggctccagggccaggaagaaagatttatccgcaaggtgatcaagatctttgagagcgccggcgtggataaacgctattctattatgggacctgaagaagtatttaccaatacttcttttgaagataaaaataatatctaccagcgggagatgattaccctgggccggacctgcctgcaaagcgcgctggataaagccggtttgaatggaactgacctcgactatatcatcaccgtgagctgcaccggcatcatgatcccttctttagatgcatacctgatcaacgaactgcagctgcgtcaggatattatacgcctgcctgttactgaaatgggctgcgcagccggtgtgtcggggatcatctacgcaaagaaaatgctggaagcaaaccccggtaaaagagccgcagtaatagcagtggaatcgcctaccgccacgttccagctggacgattattcgatggccaatatcgttagtgcagccatcttcggcgatggcgccgcctgtgcgatcctctcttcccatgaacaggataccggtccggaaattatcgcagaagaaatgtatcacttctatgacgcggaatacctgatgggattccatctctccaacaccggtttaaaaatggtgctggatatagaagtacccgaaaaaatagaagcacactttggagatatcgtacaccctttcctggcaaaaaataatcttacgatcgaagatatcgaccacctcatttttcatcccggcgggaagaagatcattaccctcgtggaagaattgttccgcagtatgggaaagaaactggacgataccaaggaaattctgcggttgtatggcaacatgtccagcgctacggtgttatatgtattggaaagatttatggagcagtcgttgcctgcgggcgataaaggactgatgctgagttttggaccgggcttttcggcacaaagaatattattacaatggtaacagagtttgcatcttactgggcgttaatactgggaggcagcagcgggcttggactggcatccgcgcgtaagctggcggcacatggcatgaacatttgcattgtacaccgtaacacccgcgtggaattaacggatatccagcagcagtttgaggagatcaggtcattaggcgtgcagctgctgacgtttaatacagatgtgctcaacattgaaaaacgtgcagaaattttgcagcagttgcaggaagctatgggtacggggcgtatccgttgcctgttgcacagcatcgcacggggcaacctcaaagcgttgccggacctgcaggcggatgatttcaataccaccatcgggcacatggcggtgagcttgtatgaatggtcggcagatatattgaacaggcaactgtttgctgcagatgcacgtatcctctcttttacaagcgatggtagttacaaagcaatggcgcactatgcggcggtatctgcggcgaaggcggcactggaatccattacccgcagcatagcgctggaatttgcgccgcacggggttagggccaactgcatccgtgcgggggtgactgacaccgcatcattgcggaaaattccgggcagtgaggcattgctggattacagcaggaagagaaaccctttcgggcagctcaccacaccggaggatgtagcgaatgtagtatacctgatgtgccgggacgaagccgcctggatcaatggcgccattataccggtcgacggaggaacacatattcattagcgtatgacaaaagaagagatcctgcagcacttaccatatgcaccgcctttcctgtttgtggatgaactggcatacatcgatgaagaaaaggtaacgggtatatatacttttcacgcagatatgccttgctataaaggccactttaaagggttgcctgttacgccgggtgtattgctaacggaagtaatggcacaaacggggctggcttgtttaggtatttatcttttgagagaagagatccataagcaattgcccacggtagctatgacctccactcacatcgacttttatttgcctgtgccacccggtgaaacggtgagggcggaggcaacgaaaatatacttcaggtttaacaaattgaaatgccgcgtagcgttgtataatgctgccggcgcattagtctgcgacggaacgatggcaggcatgatcatcaataacaaaaatgaataacagggttgtcataacaggcttaggagtggtagcgccaaacggcaccggcatcgccgctttccgcgaagcgatcaaaaaaggtatatccggtatccgttatgatgaacaactggctgccctgaaattttcctgccagattgcaggtaagccggaggtttccgaaagcttgcggcaacaatattttgaagagctggaattaaggcagctgggcagttccggtattatttacggcgtaatagccggtatgcaggcctgggcagatgcgggtttgccaatagcacaggaaacgcccgactgggacagcggtactatttttggcgccggtagttccggtgtggagaaattccgcgaagccgtttataaggtagatgatttacaggttcgccgtttaggcagcactgcggttacgcaagccatggccagtggcatcagcgctttcctcggtggcaaactgggacttggcaaccaggtaaccaccaactcttctgcctgtaccaccggtgcagaaagtgtgttgctcgcctgcgaacggattaagtacggtcatgccaaacgtgtgctggccggcagtaccagcgacagcggtccctatatctggggtggctttgatgccatgaaagtaagcacctttaaatataacgaacgcccggaagccggttccaggcccatgagcgccaccgcgagcggtattgttcccggtagtggggcaggagcgctggtactggagtcgctggacagcgcgctggaacgcggcgctactatttatgcggaagtactgggcggtcatattaactccggcggtcaacggaacggcggcagtatgacggcccccaatcccgctgcggtgcagcgttgcattaccgcggcgcttcaacaggccggtgtgcagggcgctgatattgacctgataaacggtcaccttaccgccaccggaaaagacgcggaagaaatagccaactggtgtagtgctcttcagcgcagcgggaaaaactttccttacatcaatgcactgaaatcgatggtagggcattgcctgagcgcttccgggagcattgaactggtagcggcggcactgcagctcaaggaaggttttatatctcccaatatcaactgcgaagacctgcaccccgatattcaggcactggtagaccgggaaagaattccggaacagctattgtataaagacataaatttagtggcgaaagcgagttttggttttggagatgtaaacgcttgtattattctgcaaaaatacccgcaaccttaaacgaaataacatggacaaagaaacattcattgagcagttaagagaaatagtaaggccctatgctaaaaatcaggaagcactggccaccatcagtacttccaccgattttatcaacgatctcaaaattaattctgccaacctggtagatgtggtactggatgtagaagagaaatacgatatcgtgatccagaacgaagaaatggaacgcatgctgaacgtgcaggcggccctcgatatcgtggaagccaagctcaaagaaaaatgatcggcaacgacattatagatctccgggcagccgccatggaaagccgtattcaccggaaaggtttcctggaaaaattgttcctgcccgaggaaatcaggatgatccgtaatgctgccgcaccggcagtgctcacctggttgttgtggagttgcaaggaagccgcgtataaaatagtgaaccgtaatacctgcgaaagacgatacgctccacagcgatttatgtgccaggtggaacaggatgttacatccgatatgattgccggcaactataccggcacggtggtatatgaacagcatacctattattaccagagttttatcacagatcattacatccatacctgtgcggccacaaatccccggccggtgcaggatgcagctgtgtttataaagcaggttgccggcgaagactatctgaattttatgcaggaagtactttccccgcaggagtttttttataaagacgatcatggaataccgtatatccttcaccgtgaaaatggcaggcgctctcctgtttctgtaagtcatcacgggcaatattgcggaatcctaaaggtggattttagcctaccggtaaccaggtgacgcccggcctcctccctaacaaacaatacccggaaccagtcattaaattaggtctccacccctcatcatgatcaatttgtaggtatgtatatacataatgctaagaaagcaccattatggagcaaaatagcatcaaaatggcatgttattatagccgatatttaccattattaaacaaccagacagctatagtaaaaattcacgggcctccccgttgtataagtacagtgtacaattaattgcagaaaattatgttccaacgttgtgtcagactcaccatctgctctcttgcatttttatacgcgtgtaataatggcgatacacccggtaaacagcaggaaaaattgcctgaaattgtagattacaattttgatatacggcctatcttatcggataagtgctatgcctgtcatggtccggatgccaataaacgggaagccggtctgcgcctggatattgccgacagcgcctataaagcgctccgtgaaacaccgggcgcacatgcgctcgtacccggtaatcctatggcttctgtattgtaccagcgcatcagcaccacggatacttctatgcgcatgcctccgccatcctccaatatgtcgcttagcaactatgaagtaaagctgattgaaaaatggatcaaacaaggcgcaaagtataaaccacactgggcctttgtggcgccggtaacaccgccgctgcccaaagtaaacaaagagaaatgggcacgtaatgaaatagaccattttgtattggcccgcatggaagagaaagggttggaacccaatcccgctgcggatcatgagagattgctcaaacgcctttgcctcgatcttaccggcctgccgccatcacccgaaagaatggagcgctttgccaaagataccagcgacgccggatacgaacgtatggtagatgaactgctgcaggacagcgcctatggcgaaaagatggcagtgcactggatggatgtggcccgttatgctgattcgcacggctaccaggacgataactaccgcagcatgtggccgtggcgggattgggtgatccacgcatttaatgaaaacctgtcttacaaagattttattacctggcagatcgcaggagacatgatccccggcgctacccgggaacaactgctggcctccggctttaaccgcaatcacaaaattacggaagaaggaggtgtaatagacgaagaataccgcatagaatatgtttctgaccgcaccaatacatttggtaaaagcatgctcggcatcaccatcgaatgcgctcactgccacgatcacaaatatgatccgttctcacaaaaagaatattatgaactctttgccttctttaataacgtaaaggaagtaggactggaatcggcggtgggcggcccggaaacctacgccaaaacgccctatatggagatcacgaaagacgatctcaaaggagtgctgaaatttattaataaacaggacagcaacaggctgatcgtatctgtaatgggagagaaagacactacccggaaaacgtatatccttggccgtggtaactatgacaaccctacgctggaagtgcaacctgaaacgccacatgcggtgctgccgtttgatgtgaaacaatatccggccaatcgcctcggactggccaactggctgttcgataagcgaaatccactcaccgcaagagtgttcgtgaaccagcaatggcaggaaatattcggcaggggcatcgttaaaagtaccggcgatttcggtatgcagggcgatctgcctaccaacccgcaactgctcgattggctcgcggtggactttatgcagcacggctggaatattaaacgtctcatgaaacaaatggtcatgaccaccacctaccggcaatcgaccgccatttccaaagacaaactaaaagcagatcccgaaaatatttacctctcccgcggaccgcggttccgtttacccgcagaaggagtgcgcgacctggtgctgaaaagcagcgggctgctggtaccggtgatcggtggccccagcgtaaaaccttatcagcctaaaggcttatgggaaatggctacatctggcaggggaatcctggccagctacaaacaggaccatggtgaaagcctgtaccgcagagggttgtatacctttatcaaacgtacagtgccaccgccctccatgatgatctttgacgccagcaaccgcgaccagtgcgaagtgaaacgagcaaacaccaacacgcccttgcaggcgcttatcatgctcaatgatcctaccgtgctggaagcttccagggtactggcatccaggctgctgcaaaaagataataacagctccaggaatatccggcaggccttccgtttaattgtttgccgtacaccgcaaccacaggaactaaccttgctggagaagtattatgaccagcaacagcagctgtataaacaacagccggccagcgcagtaaagttgctgcaacatggagaatacccgatggcgcaacacctcgacaatgcctcatgggctgccatgatgcaggtgatcaccaccatctataacctggaggaaacactttcaaaaacataacgatcgtatagtcacgcataataaaggacgatgaaaaacgaattcatagaacaccacctgaatatgaaccgccgcaagttcttgtcgcgcctgagccttggcgtaggcagccttgccctgggttcattactggtacctgacctctttggtaaaaacagcggggaagaagcgcctttcattcccggcatgccgcactttgcacccaaagccaaaagggtaatttacctgtttcagaatggcgcgccctcacaactggagagcttcgattacaaaccgaagctgcgggaaatgatgggacaggaactgccggcttccatccgtatggggcagcgcttaacaggcatgacatcgggacagtcgtcttttccgctggtaggttcgcactacgattttcaccagtatggcgaagcgcgcgcctgggtcagtgatctgtttccgcataccgccaaaatagtggacgatatctgtattgtccgttccatgtttacggaagcgatcaaccacgatccggcccttacctttttccagaccggggcacaacaaggtaaccgcgccagctttggctcctggatgagctacggcctcggcagcgaaaataaaaacctccccgcattttgcgtgctgctgtcgagaggtaaaggaaacgggcaaggcgtatattccaagttatggtccaatggatttttagacagcatccaccagggcgttcagttcagcagtggtgaaagtcctgtgctgtacctgaataatcctgaaggcattgacatggctaatcgccgccagatgctggaccagctcgccgcattgaatgaccagtcgtataaagaatttggcgacccggaaatcaatacgaagatccagcagtacgaaatggcttaccgcatgcaaacggcggtaccggagctgacggacctctccaaagaatcggacgatatcattaaactatatggaccggattgcctggtgcccggcactttcgctgccaactgcctgttgtccaggaagctctctgaaagcggcgtgcggttcatccagctgtaccaccagggctgggatcagcatggcaacctgcccaatgaaatggccggacaggcaaaagatgtagaccgtgcttccgcggcattgatcactgatctgaaacaacgtggcctgctcgatgaaacgctggtaatatggggcggtgaatttggcagaaccaactactgtcagggtaaaatgactgccgataattatggccgcgatcaccatccccgttgcttctccatctggatggccggcggtggcgtaaaacccggcatcgtatacggtgaaaccgatgaattcggatataatattataaaggatccggtacacgtgcacgacttccatgccaccatcctacacctgatgggactggatcacgaaaaattaacttttaaacaccagggacgccgttaccgcctcacagatgtggccggcaaagtaatccccggattgatggcctgataaatactgttataatggaaagaagaaaattcatacagacgtcggcgttagtaaccgcctccttttatatttcccgcgatctttttgccaaaccaaaaggaccggtatacggccacaataatatgcggtatgcgctggacaccaaatggggaacgctcgacagcagccggtacccggtgaaagattgccatgaaatggtgcaggacaaaaaaggccgcatcatcctgctgaccaacgaaacaaaaaataatattcttatctataataaatccggcaaactgctggaaaactggggccatgaattccccggcgcacacggacttacactcagcaatgaaaatggtaccgaatacctgttcattacggataccgagaaacaccaggtatacaaaacaacgatggaaggtaaaattctgctgactatcgactatcccgctgaaacaggcgtgtataagaagaaagaggaatttgtacctacagaaacaaccgtggcagacaacggcgacttttatattgccgacggctatggtgcgcaatatgtaatgcgctatgaccgcaatggtaaactgctgggttattttggcggaaggggtcagggagatgaacacctggacaatgcccacggtatcgtggtagatcaccgcaaaggcacgcctacgctcattgttaccgacagaacacggaattgctttaaacgcttcagcctcgacggacagctacaggaagtaattgcgctgcccggcgcctgcgtatgccgcgcggttataaaaggcgatcacctgtatgcagccgtattacgctcgcctaatatggataaggaaggcagtggttttgtaacgatattggataaagacaacaaggtagtttccaatatcggtggcaccgcaccggtatataccgatggaaaactgcagcccatgcagcaggcagagaaaatatttgtacatccgcatgacgtatgtgtggataacgacgggaacctctatgtggcacaatgggcctcggggaaggtgtatccttataaactcaggagggtataatgaccgcgaaacagacatccagatggcaaagcgcaggcagcagcctgttatttgccggaaatatttttatccttttcctcgtgatctttggcaacagggtggtgttacctccctggttgcaggtgctggggcgcatgcatcctttgctgctgcattttccaattgtactgattcttgtagcatgcattttaacgtttatccgtttgcgtgagcctgctgctgaagcgtggaaacaacagctggcatctgtgttactgcttaccggcgcactcagtgcagtcgttaccgttatcatgggcctgtttttatcaggtgaagaaggatacaacggcagtggcactttacagtggcacaaatggagcggcgtgacaatgtgctggctggcctctttcttatactggtttggacaatcggagaaaagccggccgctgttacagaagggcggtgtgctcatcaccgcggcattgctggtgatcaccggtcacctgggagctgatatcacgcacggcgaaaactttgtgctggcgccggtaaacccggcgggtaaaagaccacaggtgcccttcgaccaggcgctggtatatgaacacctggtgaaaccggtgttgcaggagaaatgtatgaactgccacaatgcgggcaaggcaaaaggggagctggcaatggagctgccgcaacaactgctgaaaggtggaaagagtggtaaactgtttgttgccggtaaaccggacatgagcctgctgatggaaagactacacctgccactggatgccaaaaaacatatgccgccggcaggaaagccgcagcttacaccagaagaagcggacctgttgtattactggatcaaaggcggcgctgattttaaaacaaaagtagccgcattacctgcaaaggatagcctgcggttgctggccgcagccatgttagagccagccgcatcgacagctcctgtatacaactttgccgcagcagatgaaaagctggtacaaaagctgaataacaattaccgtgttatttacccggtagcgttaaatgcagccccacttgtagttaactgctataataaagatcagtttaacagcaagtccattgaagaactgctcccgctgaaaaagcagatcatagaaatgcacctgcagaagatgccggtacaggatgccgatctgaatatcattgcacagtttccggagctgcgcgtgctgaacctgagctttactaacgtaaagggacaaacgctgtcggccctggcaaagctgccgcacctggaaagcctttcgctgtccggcacccccgttaccttacagcagctacaggtactgaaaacagcacctgcgttgaaggagttatacctctggaacacgggactcactgctgctgaactggacaagctccctgctgcatttaaacaggtagccatcatcaaaggatttacagacgatggtaaacaactattaaaactgaatcagcctttattactgaataccgcttctgttttccacagtacggcacaactgctgctgaagcatcccataaaaggggtggagatccgctacactactgatggatcagtaccagacagcatcaactcgccgctgtttaaagacagcctgttgctgcaaaacaataccaccatccgtgccattgcctgcaaaaaaggctggtacgccagcgacccggtgcagttcagtttttataaatctacgtatatccctgacagtgtggtattgctcacgcagccggacggaacttatgccggtagtggcgccaaaaccttatgcgatgggcagaaaggcggtatggatcagggcaacggaaaatggctgggctatgtaaaagaacctatgtctgccatgctgcttttcaagcaggccatacccttgcagtcagtatcggtaggcatcttacgaaatattaacgggtatatttttccacccgccaaaatagaaatatggggtggggcagatgcacaacacctgaagctattgaaacggattattccggcagcaggaaaaaaagacgaccccgccgccgctatggaaatagcggcagctttccccgttaccaacgtttcctgtgtaaaagtagtgatggaacccctgctgaaaataccgggctggcatcctggtaaaggaaaccgcggatgggcatttgcagacgagctgttgttgaattagctgttgaaattcgcctacctttaccgggtcatcgtagccggtaaagaaatgaaacaatataaatacgaagaaatagcagcgaacattgaaagtaagatcaccggtggccagtatttacctggtcaccggttaccttcagtaagaacattgaaggcacactacagcaccagtttgagtaccatccagagcgcctatgacgatctcctgttaaggggcctggtggaaagcgttccccgttccggctactatgtaagcgcccggccggctgctaccggtaaagtaactgaaaccatgatagtaagggatcctgttttcaggaataacctggcggcgatttcttctgaaaaccggcaacgcagcgcactatctgaattcaacgtggcggctcccggcgatttgttgctgccgcagcagttgttgctgaaaaccatgcagcaggtgatccgcgaaaaaggagcggcgctcttaaaatattatcctgccaatggtttggccacattgcgtgaaagcattaccaaacgcgcagcacatcacaatacccgtttacaatctgatgaattgcttatcacagacggcgctttacaggcagtatatattgcgctggcagcggtgtgtgagccaggagatgtaattgctattgaaagtccctgtatcttttctgtattagaagtgatccgtgtactgcggctgaaagtggtggaaattcctgtgcgcccgcaaacaggatttgatctggatgtgctgaaggaagcctgtgccatacatgcttttaaagccattgtcgttacaccgaattttcataatcctaccggcacactgctaacggatgatcaaaagcagcaactgctgaaagtcgcgcaagcccacaacattgcgctgatagaaaacgatatttacggtgagctgccgttcaacggccagcgtccttccaccatccgctccttcgatagtagtggattggtaatgacctgttcctcttttgcaaaatcgctggcgccgggtatccggttgggatggctgtcggccggccgctttttccggcaggcagaacagatccggtttgccgtgggcagcagcgtatcgcctgtgtaccaggaaacgatgaataaaatactggaaggcagtgcttatgaaaaacacctgcgcgttttccggaagcagctggccgcacagtgtgagcagagtttgaaactgatcagggaatgtttccccgcggggaccaaagtaagtcgtccgggcggcggttatcacctgtgggtgcagctaccggaaacgctggatatgaccgccttttaccgcttttgtgaagataccggggtgagatttacaccgggatcggccttctcttttacaggcgcttatgaccattatttccggctggtatttgccgataaatatacaccggcaaaggtggcggctatacgaaaagcgggaagctacgcggtagcccacagctgagcattcctgtaccggttatatttcggctccctgtatttcgctgcgcagcggcggactgctactttcgtggctcattctttcaaacaaccggacatgagtactatcattacaaagtttgcagtggcatcagacaagatgattgatgagctgttataccttacccgcacctggctggcagagcatcccgaaataaagatggaagggcaatacacccaaaaaatcctggtgaacagtatgaatagtttttcaagtcagtggttcatcgtatatgcgggggaggaaccggcgggcttcgcctttcttaccgatggcggcgtgcggccttcattcctggaagggaagcggatcgtacacctgtcggctttcgcgatattgcaggcgcatgccggcggaacagcagcagcctcattgctggaaaaatgcctggcggtatataagggccgggatgccatgtgggcagagctttccgtagcgccgggctacctggaagcaaatggctttgtgaaaacagcaggctatcttgtaaaagagatgcagtaagggatacgtggaatgataaaagtaaatattatcttaacaacccattattccacgtataatttttacccatgaggtccaggtgttttattttattattgatcctgctgtatcaggtcccattatttgcacagcgggtaaagattgcctgtttgggcgcaagcatctgtgccggcgcccggctgcagcatcctgaaaccgaatcctatcccgcgcagctgggaaagctcctggggccggactttgaggtgaccaactacggcgtaagcagtaccactttactgaaaaagggcgatcatccctattggaatacttccgggtataaagctgcattggcaagtgaaccaaatattgtgctgatcgacctcggcggcaacgacagcaagctgattaaccgcgtatatctggatgaatacgagcgggattatcacgacatgatccgtgcattccgggcattgccttcacacccgcgtatcctgttgcttcagcccattgtttcttttgtgaaagacactacccagatctgggacccggtgattacaaagcagattttaccaaaggtaagacaggtggcttatgaggaaaacctggagttggtaaacctgaacgcactgctgatgggtaaacctggactcatgccggatggaattcatcctgaactggagggcactactttgatagctaaaacactttttgaggtactgcacccggtacgggatacagcttttaacgctattggcccgttacccggcgataaaaagatctcctcattttatggctactgctgcgcggattttaatttcaggggacgcgcctgtaaagtggtggcgcctaagtttgcggctgccggtcatccgtggatctggcgcgcccgtttctgggggcatgaaccgcaaacggatatcgccctgctggaacggggttatcatgtggtatactgtgatgtggctgaattgtttggcaataaggaggctatacaattatggaacgggtattattcgttgttgcgcaaagccggactggcacataaagcagtgatggaaggcatgagcaggggagcggtatacgtgtacaactgggcggctgaaaatccggataaagtagcggctgtatatgtagataatcccgtgatagacctgtgcagctggccgggaagccagtttaaaaaacaggtcgcgcaacgtaacgagtgggaagctttcaaaaaggattacggttttacttccgatagcgctgctatgctgtttaagggaagcccgctctataaaataagggaaatagtaaaaggaaagtacccaatgctgcatgtgctggcagatgcggatacggatgtaccgccagaagaaaatacgctgccgtttgaagagaaaataaaagcgctcggaggagatataatagtgatgcataaaccgggattcgcccatcatcctcacagcttcccggaccctacacctattgtagattttattttaaaagcggcaaagtagttaaacagttagctttccgctttacgcagaaagctaactgtcatgcgtttattttaccagccattccagcttatacatcccgcggaacctgtcgtaagtcagcagttctgcatcccgtttaaacagggcatccatctgatcggccagtgtttcatgcgcagggaaggcctgttttacattccaggcggtcagcgtttgtattttaccgttaggagcggagaagtacattttgtactgatcttccggaccggctttgggagaagtgggtatttttctcttatacagcaataattgcgggtttttattcaggatctggtaactgtggttgccctctacccggtaaacatcaccgttggtgagctgataagcaaatatttcatttttgttgatatgaatatttttgccattatgctccagggtgacataacttttaggcgcaagtgtatgcagatgaatcctgggtgttttgttgctgttatccttggtataactcaacccgccggacaggtaatcatccatgctgcgataaatgccggtaatcttcttttgcgcgtctgctgctacattgatacacatcaacaagcagatcaggtaaaaaattctgctacagtattgcatatgtctatcggtttgttttggtgctactattaatttagcaaaattagccgataatttattaccaggacatgataaaaatcattaaaaatttcctaaaaattgatttggtaagatggttattttatttcatccggcacttacaaaaccggcaggtatacataaaacgtacaaccttcattcaactgtgattcagggtaaatatatcctccgtgatttaataccactttccggcaaatggttaacccaatacctgaaccgggatagtcggaaaccctcaccaaacgtttgaaaatagtgaatacctgatccgcgtatttttgctcaaagccaataccgttgtcgcggaataccagttcatagtaacgtttgtcagtttccagctttggaacggtagcctgtttttccggtgatagtatgctcacacttacccggatcaccggttcctggtcattaaatttcagggaattatcaagcaggttatgaaagagctgattcatctgtaacggaacagcttttattcgtggaagcggtgatatttcaatatgggcttttcttttcttcagatcgggttcaagatcacgcaatacgtttttcataacaacgttcagatctgtttcaataaacagatcttcatttttattcagtttggagtaagtcagcaggtctttgatcagcccggacatacgcgaagccgaagcaatcattttttccaggtattctcttaccggttgccgtgccgcttctgcgctcatagcaaggttaccaaaggtttgaattttgcgtagcggttcctgcaggtcatggcttgacataaatacaaaatcttccagttccctgtttgtccgtttcaattcttcattggctactttcaatgctgtggtgcggtcttccacatgttgttccagcttatccgaatagttcctggcagcttcacgcgctgccacaaaaaaggtaatgtcattggtaacgcacataataccggaaacatgaccattttcttcatacagcggttcaaatgtaattctgacaataatatcttctggtttgccaaagcggatgatctttaatggcagttcaccggtaatatatcttttaccgctggtgtatgccttctctatcatgccttccattccctgtgatttcagctctggtaaggcttccagtagtggtttctgcattacttcttccgccgctctgccccagtattgcaattgtatttcattggctacctcgatattcattaacagtcctttcaataagcagatggctaccggcgcctgttcaaataaatttttcagttgttgttctgcatggttgcgcaactttaaaattctaatatgcgattttactttcgtaagcagttctacggctgaaaagggtttcaccaggtaatcgtctgcaccggcttccaatccatcgatacgtgcttcgccaccggtgcgtgcagaaaggaagataacaggtatctgcgctgtagccaggttaccacgtaaacgttccagcagatcttttccattcatgaccggcatcatgatatcgctgagaatgagatccggctttttgcgctccacttgctccagtgcttccagtccgtttttggcagtcgtgatataataatatttttcgagtagccttgccaggtggttacgcatatctgcgttattgtctacgatgagcacgtgtgcccgttcagggctgttggcggctgtttgggctttatcaatagccgctaatgcgtcgttgcgttgttgtgcctgttcatatgcatgtacattcgaaaaagcgatgctgaaagcgttacccagtaattcgtaaaaattcaaataagtttcgtccagcgttcgtctggcactcacgccggcaacaacaaatccccatggccgctgctcgccggcgatatttaccggcagcacaacagcgctgtgtggcgcttccgggtagggaccaaagggaatatggccaaagtggctgcccaggtcagttatcactcccggttgcagggattgtaacgcttcgtcgaaagaccagttaactcctgcagtatccgcatcaatccccgcggcggctatcacacaatggttatttactttgctatccagctggtataacagcaggaaagggatatcgcagctgaagtcaatcgtctttcccaatattgcttcgcatatcttttcagtagtttctgctttgcctatcagggtcgacaaatcacgcaacacctgcgtccggcgcgcagccagcactttatctgttgtttcggtaaccgtgtgaaaaatgcctcccacttcgccggcttcattccgtatgggcgcaaacgagaaagtcatgaacgcttcttcgaggtagccgttacggtccaggaacatccgctggtctttgatataggttccttctcctgactgtccgcgggtgaaagcatcgcctaccacgggcagtgctgtttcccagcatacccggaagctctgacccatagacatgggatgtttatcaccacagacaagccggtagctatcattgtagatctgtatagtatcggggccccaggcgattaaaacgggaaatgtggaagcaagacacagactgaccgttgttatcaaactttggggccagcattcaataggtcctaaggatgttgccgaccagtccatgcttttaatcagcctgcccatttctccaccacgagctaaaaattgatcccgatgtttcataggcgtttggtaatagggcacatatagttttgtttgaatgagtcaaaagcggagattatctttatcctttccatactcaatttaaacaaactaccttgaatagcaagattctgcctctgatcgctgcaataatagtactcacgcagcacccgttgaaagcccaaaccaaccgtttacccgattgggcaatgggcggctttgtaaggcccgccggcgtaaatcccgtgatccgcacagattccacagcgcatttttatgattcgctcctgcaaagggaggtcgactgggagtcgaacgacacctttaaccctgctgctgtggtgaaggccgggaaaatagtagtgctctaccgcgcagaagataaatccggtatcaagataggtacgcgtacatccaggatcggctatgcagaaagtaaaaacggggcttctttcaaaagaaaaaaaataccggtattatatccgcgtaacgatgttcagcaaacctatgaatggccgggtggctgtgaagacccccgtgtagctgttaccgttgatggcacctatgtgattttctatacacagtggaaccggcaggtaccccgcctgggagtggctaccagtaaagacctggtcaactggaccaagcacgggcccattttccggaaagccggcagccgtttcgtggatcagccgcataaatcggcgtccatcgttaccatgctgaaaggaaagaagcaggtgattgcaaaagtaaatggaaagtactggatgtattggggcgaagccggcgtatttgccgctacctctgataacctggtggactggcaacccgttaccgatagcagcggtgcattaaaggcgcttataaggcccaggaagggctatttcgacagcgggctgacggagtgtggtccgccggctattatgacggataaaggcatcctgttgctgtataacgggaagaatcagccgggtgaaagaggcgaccggcgctttaccgcaaacagctacagcgccgggcaggtactttttgataaacaggaccctgaaaaagctattgcccgcctggatgtgccgttcctgcgtcccatggaagcatttgagaaaagcgggcagtatgccgcaggtaccgtgtttatagaagggctggtatattttaagaagaaatggtttttatactacggctgcgccgacagccgggtagggatggctgtatttgatccaaagcacccggcgcccggagatcccctgccataaccgttcaccattaaatttccgctatcatgcgtaaccgttttttttcgttgcttgtaatggttgctttttttacagcatcatccgcaaacgcgcagtatatcgaaaaagtagtttttgatacaaaagatagtaccggcaatttttatcttgccgtaccgccgctgtcccatcagataaaaggcgtggtggtggtgttgtctaatttctaccaattggataacctggtaccggaaacaaagctgcacaacgtggcctgtgccaacgacctgcttactgtttttgtttccatgcaggaacaactgtttgccgataccgccgtggtaaaccgcatcagcaccgtgatacagcatgtagccaataaatacaaagccgatacgtcgaaatttgtattggccggatacgagtatgccagcaatatcgcgctgcgctatacggaattaacccggcagttccccgccgcctatgccatacatcccaaagccgtttttaccgtcagcggcccggtagatctgaatggattgtggcagtggtgccaacaggtgatccggaaaaaaacaaacgacggacaaatgggcgacgcaggttatattcttgataaaatgacccgcgaaatcggtacaccagcggcacgcccggaacgctaccgcgccctttcaccgttcaaccgggaagatacggccgcaggcaatgagcaatacctgcaacgtatgcccgtgcgcgtgtattatgatacggacatcgcgtggctgttgaaggaacgccgcaacagtttgtatgatacctatattcccgatgccactgaactgataagcaggctgctgctggccggcaacggagacgcggagttcatcgcttcaccgcaacccggcaaacgcatcaacggcgcccgctacgcagaggcattttctattgtagatgaaacggaatgtatccaatggatcaaacgtacactggatatttttgacccggtaaactggaaaccaccttataagctgaacaagccgaagggctggggaacagaacatttccaggtgccggtggactttgccccggagatccgctataaaggtgtggaagatatccgctttgcaccaggatggggcgacagcaccagcgcggaacactggtcgtatgctttcctctggtggctgaaagataagcccgtggtaaacgcggctacgctgaatacctatctcaccgcttattacaatggcctggtaaaacgtaacgttatcggccgcaggatacccgcggaaaaacaggttcctacggtcgtcgatatcaaaaaagtaaaaacattggaaggagatgtggaaacctacggtggcactatccggatgttaaactatatggtacagcgccccattgtgctgcactgtaccatacatgtaagcaattgcgaatcgcaacagcgtaccgccctcttctttgaaatttccccgcagcaggcgtcccatgctatctggaagcagatggacgggctatggagtagtttccgctgggagtaaggattattgcccgccggggattgagtaaatatcaaatacgccgcccttcatcaggtcggtgtgcaacaggcgcgtggtactgtatggctttccatccttttttatggcgccaatagatacaggcgtgcttttagcctccacacggatggtggtagtggtatgcgcaccggtatgaatgacaatacgctcaaaagtgggaatggtgatggcatattccggcgccacggggttcaccgggtaaaatcccatcgcagcaaatacataccaggcactgatctggccggcatcgtcattgccgcataaccctcccggacctacgccgtattccatggccctgatttcacgggtatgcgcaatggttttcgtttgcgcgtttacgtagttatacaggaaagggatctggtgaccgggttcattgccatgccagtattgatggtttaaaaaaagactatccagcgcctgttcaaattttttatttccaccggttattttaataagaccgggaatatcatgcggtacataaaacccatactgccgtggcgttccctcggtaataaaaaacattttcttgtcccggtcgggatgctcataccatttgccggaggcgtaccggccgtttacatctcccagctgcggatcaaatacattggcataattgccggccctttttgttaaggctgcataatctttttgcttatgcagtgccttcgcaatggtagatagcgcgtagtcatcaaacgcatattcaagtgtgcgcgatacctgctcacggctatgaaaggcatacggcacgttatcttccaaaggtacatatccgtatttcaggtaagaagataaagccctgcggcccttgccttctttataatcagctatagcagcggtgtcaaacgcattttgccgcatgaggcgatacgcttcttccacatcataattccggatgcctttgttataggcagatgcaataaacggaatggcatgatcaccaaccatggctgcagtgtaattattccagcaggggaagatcggcagccagccaccctgttgccctttcaggatcagcgaacgtaccaggtcgttgatcaacgtggtgtccagaatttcatacagcgggagttgcgcgcggtaaatatcccacatggaaaagtcgtcgtagtaattgccggaagccagttgtttcacctggtaggattgcgcaaaagcagggtaggtgccttttacatcattgaagaggcgcgggtgctgcatggtatgatacaatgccgtataaaagattgttttatctttttcggaagaaccggttacttcaattttccccagcgctttattccatatatcgctggctgtttttgtttgtgcggtaaaatcccagtgattgatttctgctgcaagattttccctggccgcatcaatactggtgaaagaagtgcctacacgtatccttattacactgcccttatgcaccttgaattttacagcagcgccgatacctgcatagtctttgatgctgtcttccgccagaacggtgttgtcgcggaagacttttgcatcactaaacacttcttcaaactgcaccacgaagtatccgctaaaacctgctggctgtccctgaccctggtaaatgcggaacgcggggttatagccggagatctcctgccgccggcgatcgatatacacagcgcctttgccccggtcgctgttaggcctgatcactatatagcagtcatcctctttggtgaagctgaactgcatcatgctgcaacgcgcggtggcagtgatggctgcgtgtatcttgtctttgcccagtaatgtgctgtagcaggcgggcgaggctgtttcaccggtgtttgaaaacgttgaggcgtaaccgtcaggtgtggttttgagttcgccgcaaacgggcataacggtcatactgccatagtcctgtgtgcaggagccgctgagccagtgtgtgccccggaagccggtgaaaagtgagtccgtgtaataatacggcgccacacatttctgttcggtgagcctggtttgcggggtccactgcgtcatgccaaaaggtgtgcccaccgcgggaatggtattagccagctgctcggtgccggcgccatgtgccagggcggtgagagtagtacttttggaagtgccggtgaacgggtctacataagccaacagctggctggtttgtgccaaagcacttgccataccagctgttaaccataaaaaagtacaaacggttttacgtaccatcaatatcctttattttgtttgatcttatccttgttaatatctatctggctttgtggtactggtattacgaggttgtcgctggtaaggtccgctactaacctgatctgtgcttttttgctgttgagtaccggaatcgccctgccggtgcggacgaggtcgtaccagcggtgaccttcaaacgcgaattccacccgtctttcattttctattgccagccggaacgatgcctggtcgggcacgttggcggccgttttttctgcgagtcctgctcttttgcggatcatgttcaggtaagtgaatgcttcaccgccgccctggtagcctatttcattaagggcttccgcatacatcaataatacatctgcataacggattaccgggaagttattaccattatcgttcttggtggcaggtacatcaaagtacttctttacaaaataataatttacggtagccccgctggcatttacataagaagtagccatggaaaagctcttcctggtgtcgccggtttcataggcgctttccatatcaggggtcacctggttattgccatcgccgccaaacttcactacggcgtcgccggagttttcgggcgcgaacgagttaggcagcggattgccttcttttacgccacctgatttatattgtacatcaaaaacagattccttattatttttcttgcttacatcaaaaacgtcggcatatttatccaatatggcgtaagtgccggagctgatcacttctttcagctttgcagcagcatcggggtatttatgttgcgtgagcaatacctttcccagcaaggctttggcggcgccacgggtagccctgcctatatcggcgccggtataactcaccggcaatgcggcttcagcagctttcaggtcggcttcaatttgtgcgtatatgctggctgcaggatcacgggtatattcatatgcctggtcggcattggtgatttctgtcaccaccaaaggcacatcaccaaaggaacgcaccaggttgaagtataccagcgcacggagaaactgcgcttctgcggagaagcgcttcttcagtgaatcactcatagctatcggcgtaatcctcgacaggatggtgttgctgcgggaaatggctttgtagctgtcgttccagcgggcggccacaaaaggattggtagttttgatatagaagcggtcaaattcatcctggtctgtcacggagccggaaggcaccgggaagttgttatcggatggaatatcaccataaatataagcgttgccaaatacgccgcccgactgcagggagccatagttggcattgagtgcatttttaaaatcgtctgctgttttgtagaagttttccgtagtggccgtggaaggcgggacctgctccaggaagctctttttgcaggccgtaaatgaaacagctgctgcgaggaatatgtatatataatttgtgcgcatgttcgttaattttttagcaagatcagaatccaatatttaccccaactacaaatgttctggccagcggataccggccatagtctacgccgctggttaaagcgccttcgtaattacttacttccgggttatagttcaggtagtcggtaaacgtgtagaggttttgagccgagagatagatcctggcctgttgcaggcggatgtgctgtaatattttttccggcagttggtaaccgatacttacgttttggatacgcaggtaggtagcatcttccacccagcggctggagatggcgttgttgttgccggtggtgcgctggttggcgcggggaatgatgccgttgcctggtttgtcggccgactgccagcggttcaacaccgtggtgagctggttggcgctgccttctacgttttcaaagaagcggcggctgaggttcagtatctctccgccttgctggccttgtatggccaccatcaggtcgaagtttttataccggaaagtgttggtgaggccgtaaataaaatcaggctgactgttaccgatgatggtgcggtcgtcagctgtgatctttccatctttatttacatcttcatacttcacatcaccgggtctggaagtgatgtcgtgtggaaatttatcgaggtcggcctggttctggaagatgcctatctgtttgtatccataaatgttaccgatcggttttccgattatcgtgatgttggtttcgtttacgccggaattgctgcggatgggatctcctgtaggacccagtgccaccacggtattgcggttaaaggaaagcgtggcgttggtgttccaggtaaaggcgccggttaggttacgggtggcaagtgaaaattcccatcctttattttcaatagcgccaatatttttaacagcggtgctgaaacccgtgatagtaggcacatttactgccagcagcagatcgttggtatttcttttatagtagtcgatgccaatgccaattctttcgtggaagaagccgatgtcgatgccggcgtcgaactgtttgcttttttcccagcccagttcatcgttgccaagcgaaactgcacccaaaccatttacgagcgagttgttgaaactgtagttatctgcttccagtttagcgaggtaaggataatcttcagcgtattggttattacctgccagtccgtagctcacacgcagtttggcgttagagatgacaggaatgtttttcataaatggttcttctgtcaacacccatcctacagaacccgcggggaatacgccccacctgttttggctgccgaagatggaagatccatctgcacgcagcgatacattggcgatgtacttttctttgtagttataggtagcgcggccaaagtaggaggtggaagtattggcagttctgaaagaagtgacggtactcggtaacccggcagcattcagtgtaggcactacgtcgttggcgtaagaggtaccaatcgcctggcttctctggtactggtatttataggcctccatacccagcaacacatcgatgttatgcgggccggtggctttggtatagtttacggtttggttaaacagccagctggtggtttgatcagaagacgcttcacccacggcctgtgtaggcggcaagatctggttcagcggcatgcgggatgttttataggcatttctcctggtggagcctacattgaaattaccggtagcgcggtaactgaaatctttcaggaactggtacgatgcatacacattggtaagcaaattggtggtgatcagctcattcggattttccgtgatattggctacggcgttggtgatgccaggccagccataaggcactgccagcgcggtttgcgaggtgtaagcgctatggtcggcgttccagacaggtgtcattggtactgcagataaagccgcgttgataataccgttgttagcccagtgaccatcactgtttacatcgttctggattttatataccgggttgatattggcgcccagcttgaaacggtcggtcacgttgatgtctacattcgcacggatggagtaccggtcgagtgtggatttttcaatgatgccatcttgtttcaggtaggcaccggttaccaggtattgcgcgttatcattgccgccgctggcggttacctggtagttgttgatcattcccttgcgaaaaatcatatcctggtaatcatacgtaggcatggcggctaccttctgcggatcgtcgaagttgaaccactcaaacagatcgccgcgtggataacggtaacgcaaatacgaagacgggcgcgcactgttggggtctgatatattggcgccgggtacgttatcgaggtaagcattattggaggcttctttggagaactctgcaaactgctgcgagttgagcacatctatctttttagagagctcctggaatcccgtatatacgtcggcgttaaaccttgttttgccggatttaccgcgtttggtggttacgataagcacaccgttggagcctttggagccatagatcgcagtggaggaagcatctttcagcacatcaatgctttgcacatcgttgctgttgaaattgctgaacacactggcgtccacaatattgccatccactacaatcagcgggttggtacctgcgctgatagagccgaagccacgtacttttatggcgggggtagcacccggggcgccgcctgtttgctgcacgatcacgccgggaatttttccctgcataccggtggccacattggaaataggcatgtcacgcatttcggccataggcacggaggcgatggcagcggtaacattccgtttcttttgggtgccgtatcccactaccaccacattattgagcgagcgggtttcttccttcaggatgatgttcagcggggtagcgctgccggcggcaatttccacggaagtatacccgatcatactaaaaacaagaacggttttttcatccggtacccggacggtaaaatgcccgttaacatcggtaatagccccgccaccaccgtttttgatggtgatggtgacattgggaagcccgctgcctttttcatcggtcacttttccactaacggtgatcacgcgcgcagaggatagcgtaggatctgccacccgcttctcggtgatcacaatggtattggcattcagcgaccaggtaagggcggtgttttccagcagcaggttgagtgtttgcagcacggatcttcgttccgcgggcaaagtaatatcatcatagggagagagctgtgcggcaacataagcaaacttaaaggcgctttgctgctggatttgcttaataccttccttcagggattgccgtttcaggtttacggtgacgtctacttcttccaatcgctgcgctttgccgggagcagcaatcagcatattgatgccgaaaagaaaagcagaggcgagtaagcaacttagtttcatataatacgcaaacgttcgctttgggaaaaggcgtagccttcccctgataagaaatttcatacctttgggtagtttttaaatgtttaccgaaatgtttaagacaaccggctatactaactagtccttagtatagcctttttttaaaatcgtttatccagccagattatactgtcctgtcctttttcccattgagcgtgcgttagctcacagatcacatccagcgcctgtttcatgggatcgttgataaaattaccggtgaattttttaacgcgcagggattcatccctgaaccggatatcaataccataatatttgttgataagtggaatcgctgcttcaaaggaaatatcttcaaataccggctcgtcttttttccagaccagcacttctttcatattggctttggtcaccaaaggggcaatggcggccttgtccagtattaactgatcaccgggcagcagttctgctaccacggcgttattagctttttgcacctgtactttgccggtagtaacggtaacggctattggcgaggcatcccccgcagccctgatattaaaggaggttcccagcacccgcgtcactatggcgccggtatgcaccaggaacggtttgtttttatcgtgcgctacttcaaaaaaagcttctcctctcaggtatacttccctgctacctccatcaaaggcggcaggataatccagctggctgttttcattgagcgtcaccacgctgccatcagggagggtaattattttattggacgactgctgcgttttgggaagtgccgcggtaagggtaggagcgggctttgtaaccggcagcagccaccaggcgctgagcaccgccagtagtacagcggcggcaacggccatccttttgtagaagggattgcgctttaccgtcattaccttgagcatatcaacctccccctcccggatctttccctgcagctttgtatacaattgttcccacgcaggctcctgcgccggccggggcgtacgctcccagagcgctgccagctcctgcgaaacaaggtcgttttccgacagctccgccatcaatgcccagaactcttccagctcctgcggactacagtcgccggacaggtatttttgcagtaatagttttaatcttaacggattagacgacatatgccagttatataactgcaatgacgacaaaaaggagggggtagtactaatcagtcagaaaataaatctgacagcagcaggaggtacacaaaaggggtaatatggttattcagcaggtattgcttaatgatcttcaggctgtcggtgatggtatttttaacggtgttacgggataaattcagttctgtggctatttcttcatgcgtcatgcccttttcccggctcagggtgatcataaggcggcgctggggcgacaattgtttataggcgttgttcaatatctcccggcattcgttgttcagcaggctgtagtcggcgctttgttcctggtgggcctccatttgttcgctcaccagtttctgcaacctggcgtttttagcggccagcttgaagaagtccatcgctttattgtaagccaccttgaacaggaacgcgtccatattttggatatgggtgatcagctccctgcccgtccacaacttcaggaatacgtcaatcacaatttcctccgctacctcccttgatttggtaacagccagcacatagtgatagagcttctttctatggtgttcgaaaagttgtttgaaggcagcttcatctcctgccgcgatgttggtcagtaattcagtttcattatacatggaattcttctcttagttgatatccggaacgtggttcgacaaatatattttttttccggagaataatttttaaaatctcggggagatggccgcgtcgccttcggcgactttaaaattgtcttggagcaggattacactgattatgctgatttttcggatttgatcatttggattttataaatgattttgggagatatcagcgaaaatatccgcttatacctcccaaaatcatttataaaatccaaaaagtaaaatcaacgtaatcagtaaaatcagtgtaatcctgctccgagacaatttagaatcgccgaaggcgatatcaggagaatccgcttaatttgcaagccaatgaacaatacttatatgacacaaccgataaaactactggctatctgtggaagcacccggcaatcttcttccaatcaccatcttataaaagcgatcacggaactgggcaagggcacctttacggtacaactggtggaaagtctcaccaccatcccgcattttaatcccgaccaggacatggacgccaacagcgcaccggaggaagtgcaacatttccgggcacaactggccgccgccgatgccgtgctgatatgcaccccggaatatgcaattggtgtgccgggaacacttaaaaatgccatcgactggaccgtctcctccatgcacttctccaaaaagcccgtcgccctgatcaccgcaggtacttccggccataaagcgcaccagtcgctgctcggcaccttactgatcatcgagtcaaagatcgctgaggcagcgcaactcgttatctcctcagtaagaacaaaaatcaacgaccagggcgtgatcaccgacccacccacggaaatgcaggtacgaaaactgatccagaccctggccgatgtggcaaccggcaaagcaacagacctgttgccggcgccgtcgctgctctgaatcacgttcggcgcgtaggttgtcttactcaggattaaacttatttcactgattaccctgatttgatcacttttggattttaaaagattcggggagatagaagcggaaacgcggattttgtctttctcactgattacgctgattttactgattatatcttttaaaagattttgggagatataagcgaaaatatccgcttatatctcccaaaatccattaaaatcaaaaagtgatcaaatcagggtaatcagtgaaataagtttaatcctgagtaagacaaccttcgcgtttccgcttctatctccccgaatcctttaaaatcaaaaagtgatcaaatcagggtaatcagtgaaataagtttaatcctgagtaagacaaccttcgctgcattatttcacgctgtacttcacttcttcggtcacgcctttccaggtgtcggtgcggaaaggtgctgccgggaagccttctttgttaaagaggttgtcttccaggttatcatctgcccagccgtagcgtactgctaccggtgtgcttacttcgtctgcatacactactactttatcgccgtcaacgaatgctttggcgtagtggaattgcttgtcggcgccggctacttcaaatccgcggatatagccatatttatctttcaccataaggccgctgccggtgctggtaaagctgagggttgccttgttgccgtttacctgtatggattggtatatggggccgctgaaaacgttgttttgtccgtaggtgtcatgtaatgctacggctgccagccttttgcctacatcctgtttgttttttggatggatatctttggattcgccgatgtcggtagtaacggccatgccggtattaggtacctgcagggtgagggtttgggcttctctcagctccgcccacttgctgcctttctggctggtgccgttgctggagttgaagctggccagctgtacaaagtaaaagggaaagtcgccctggtgccacagccggcgccagtcgctgatcatcagcgggaacgctttgcggtactggtaggcgcggtcggcattgctttcgccctggtaccagatggcgcctttaatggcaaaaggcagtaccgggttaatcatggcgttaaacagcaacgatgggtagctgttggggccaacggcggtgccggggttcagcgccttttggatgcggaaggaccagtcgcccgtaagggattgcttctggctgcctgtttgcagaaaaatattctctgcatctccataaaaaccaccgccgccggtattatcttctatgcttactgcaattacattagtaccggcttttaaaacaccggccgggatgtgataggtacgggcggcatcatagcctttggtactgcctacctgtgtaccgttgatgtacgtaatatcgttgtcgtcgatggtgcccaggctgagttctgctggtttgccggcatctgctgcagatacctggaagcttttacggaaccatacgataccgtcgaagtcggggagcagctgctcttcccagaggccggggactttcatttttttccaggactggtcatccgtattggcggcagaccaggtggccacggtggcggcattgggcaggccgccctgtaaattctggataagctgttgctgcctgtttttggcggcgatggcagaggagtccatgttcagcgtgggaatacgttgcatcatgtcgccgaactcgtcgctgctggtcagcccctctttgctgatccaggtttccacgatggtgccgccccaggaagtatgtattaacccgataggtacgtgtgtttgttcattcaatgctttggcaaagaagtagcctactgccgtgaaatcggccgtgttttccggtgaggccggtaaccaggcgcttttattcacatcatccagcggcgtcaccgacatcgctttgggcaggtaaaaatgccggatggcagggttggcggattgggcaatttccttgttggcgttggttacgccgtttacatggaattccatgttcgattgcccgctgcagatccatacgtcgcccatcaggatgtcgtgaaaactgatatcatttttgccttttacggacagggtataggggccgcctgctttttccggctgcaggaataccttccatttaccgttcttatcggcctttaccgttttttcctgttgattgaaccggatagtgaccttttcattcttatcagcccaaccccataccgggatcggcttgtcgcgctgcagcaccatgttgtcgccgaaaacgttgggtaaacgaacgtcggcaaaactgaaggaacttatcatggttgccgccagcaataaaactgtttttttcataattgtggtattgtctgtattgtggggtacgcccctgttgaatcatgtgcgtataaatgtaaggaagacaggcattattttataatttttcaggagaagccggtaaaaatgacgcatgtacccctgaaagaggcccagccacggccataagaattatgtaaaagatagcatgaattgtataacagtcccgcctcccgggcatcgtaattttacatcatcaaattaattattcatcaccagataaaagaatcaacatgaacgcaacacaattcaaaaccaacatcaaatgctccggatgtattgcaacggtaacgcctgtattaaataaactggtgggcgcagataactgggaagtagacctggccagccccgacaaaatactcaccgttacaaaagaaaacctggataaaagcgaaatcagggtggcgatagaaaaagccggttacaaggcagacgccttatcgtaataacaggcagcatggagtatattatcaacaagtaaaaactaacagacatgaaaaaaatattaatggcaggcatcgtattggtagctgcatttatgcaacagggtatggcacaggataaaactgtttccacacagttatctcccttactttctttatactacaatattaaagatgcactcgtgagcagcaatgcggaagtagcagccgccaaagcagatgagtttgtaaaagccgccgcccaggttgatatgtcatccatgccgcctgctgttcacaatgcctacatgccgctggcagcaaagctcacggcggatgcaaaagcaatagctgaagcaaaaggtatcagtaaacaacgcgaacatttcaaaacattctctgataatttctatcagctcgcaaaagctacaccgctttccgcacagccggtataccaggaatactgccctatgaaaaaggcttactggttaagcagcagcaatgctgttaaaaatccttactacggcaaccagatgcttacctgtggtaaagtaagcgataccattaaatagtctttaatcattcgtatgaaagcagtattcctgtatataacattgatgagcctgtgtagtatggttgctgcacaggcttctttaaacactgcgccaaaggtagtccgctacgatttatacgtaggcgacagcatggtatactactccggtaaaatgagccatgcacttactatcaacggcaccatccccggacccgtcctgcactttacagaaggagacactgcagagatttatgtacacaacacattgaaagaagaaacgtctatacactggcatgggctcatcttacccaatcagtacgacggcgtttcctatctgaccacgcggcctgttaaagccggtgaaacacacctctaccgctttcccgtggtacaacacggcacctattggtaccatagccatacgatgttccaggaacaaagcggtatgtatggcgcaattgttttccatgaacggaaagaaactaccgctaaagaatatacgttattgctgagcgactggaccgatatgcatccgcataccgtaaaccggtacctgcacaacgccaacgactggttcgccatcaaaaaaggatcggtgcagagctacgccgaagccatacagcataagcatttcaaaacaaaagtgaccaatgaatggaaacgcatgaatgcaatggatgtgagcgatgtatattacgaacgcttcctgtcgaacggtaaagaaacagatgaacagccgcaatttaaagccggtgataaagtaaggttacgcatcataaacggcagctcctccacttatttctggctgaactatgccggcgggaaactcaccgtagtggccaatgacggcgccgatgtggaacccgtggaagtagacaggctcctcgtgggcgtatctgaaacctacgacgtaatagtgaccatcccggataatatgcagtatcagttccttgctactgcggaagaccgtacccgctccacttcgctgtggctgggacagggcatgaagatgcccgctaagccattaccccgcctgaaatatttcgaaggcatgaagatgatgaatgatatgatgaaaatggatggcaacctcgataccagcactggtatgcaaatgagtaaccaggtaatggatatgaacacggtcatgtatcctgaaatcaccggtgatgataagcgggtgaaacacgcaggtcatgatatgcaaaacatgcaaatggatagcactgccggagatatcgtaaccctgaactacggtatgctgcgggcgccggaaaaaacaacgctgccgcccggtcccgttaaactcctgcattttgaactaacggggaacatgaaccgttatgtatggagtatcaataacaaagtagtatctgaaacagacaagatcttaataaagaaaggcgaaattgtacggatcgtgttgtacaacaacaccatgatgcggcatcccatgcacctgcacgggcatttcttccgggtgctgaacggacagggcgaatactcgccgctgaaaaccgtactggacattatgccgatggaagtggatacgattgagtttgccgctaccgaaagcggcgactggttcttccactgtcacattttatatcacatgatgagtggcatgggacgggtgtttagttacgaaaattcaccgtcgaatccggaagtgccggaccctgttaaagcctaccgcatgttgaagaaagacgaccgtatgttgtacccgatggcgcgcgtagggctggaaagcaccggtagtgatggtgaaatcgtagtagcgaatagccgttaccgtttgtctaccgaatggcgtgtaggattaaacgaccgggatggttatgaaagtgaaagccatttcgggagatatctcggtaagaaccagtggctgttcccttacatcggttgggacgtgcgttaccgcaaaatggatgaaccggagaaaaatctcttcagccagaaaaatacaaaggatttcaggcaggtatttcatgtgggcgtggaatacactttacccatgctgatcgtggcagatgcttctgtagacacagatggtaaaataagggtgcagttaacaagagaggatgtgccacttacaagaaggttacgttttggttttatggtgaacaccgataaagaatacatggcggggttccggtacattgttacaaagaactttgcattttctacacactatgacagtgacatgggacttggagcaggtattacattaagctattaaaatatacagcaatggaacatcagcatcagcacaacaccatgaaaatggagcatgcgcatgcatccatgaatcacggtgcacatcacgatcatcatgccatgatgatcgccgatttcaggaaacgtttttatgtagtgctggtgctgacggtaccggtgatgttactatcagaaatgattcagcactggctgggcatttcttttacatttctgggagatggatatgttttgctggtattatcttctgttgtgtttctttatggcggatggcctttcctgaaggggtggtgggaagaaatgaaaagccgggagccgggcatgatgacgctcatcggctttgctattacagtagcctatgtgtacagcgtggctaccgtattcggtttgcccggcatggattttttctgggagcttaccaccctgattctcatcatgctgctgggacactggattgaaatgaaatcggtgatgggcgcctcgcgggagctggagctgctggtgcagctgatgccggatgaagcgcacctggtacatggcgatcatgtgatggatgtaaaaaccgcggaactgaaagcgggagatgttatcctggtaaagcccggggagaaagtggcggcagatggtaccatcctggaaggcaacacgtcgttgaatgaaagtatgcttaccggcgaatccaaaccggtggaaaagcaggcgaacgataaagtaattgccggttctatcaacggcaatggcgctatcagggtcactgttacgcatggtgtggccgactcctatctttcgcaggtagtgaagctggtgcaggatgcgcagcaatcccgttcgaaaacccagctgctggccgacaaagccgcgcgctggcttacagtaattgccattttatccggtattgccactttcttatactggtggttgagcggccgggagttgtcgtttgccatagagcgcatggtaacggtgatcgtgatctgttgcccgcatgcgctgggcctggcggtgccgctggtaattgcgaaatccaccgctttatccgcacggcatgggttgctcataaaaaaccgcaccgactttgagaattcgaggaagattaccactattgtttttgataagacaggtaccctcaccgtaggccgttttgaagtggtgaggtttgattcattgcagcagggtatttccaaagaagagatcctggaaatggcggctgcgctggaaggcagttccgaacatcccattgctgcggggattacaggtaaagcaaaagaaatgcagcttaccccgccggcggcggaaaatgtaacggccatcaccgggaaaggtatcaccggcaatattgccgggaaagaagtgcaggtggtgagtcctggttatgtggccgaacagttcagggatgccgctaccgcctccattgagccgggagaaaccctggtatatgtgataaaggacaacaaggtagcgggctttattgcgctggcggaccagatccggccggaatcggcaggcgccattgccacgctgaaggaaaaccggatcaaaacggtgctgctcaccggcgataacaaagtggtagcagaaagcgtaagtaagacgcttggtatggacagctatattgctgaagtgctgccgcaccagaaactggataagattaaagcattgcagcaacagggcgaatttgtagccatgaccggcgacggtatcaacgacgcccccgcgctggcgcaggccaacgtgggtattgccatcggcagcggcagcgatgtggcggcagaaacggccggcatcgtactggtgaacagcaacccgcaagacgtagtaaacctgattttatttggtaaggccactttccggaaaatgatccagaacctcgcctgggcaacgggttataatattgtggcgctgccattggccgccggcgtgctttataaagagggaattatgctgagccccgctgcaggagcggtgttgatgacagtaagcaccgtggtggtagccattaatgccagcctgttgaaagtgaaaggttccgggaaataaataatcactaaattgcaataggattatgaatgtgatataactgattttacaactgtattgctttgtcagctatcccgcgaatgcctctcaaaatatagccatatgaacatcggtcaactttttcaccgtgttgtaaataccggaaccttccgccaggaggaatcgctggcaaaggtgaccaggatggttaatactttttctgttgttaccaccacgctttgccttttattcggcatccttgcttacatgggtaccgggaaatttgacctgctgatccctgcttatatagaagccggacttttcctcggcgtatttttccttaacgctgtaaataaacccgttttagccagcatcgccttcattgccattaacaatatcgccatcgtttatttcagcgccgtaatgggcatgttaacggaagtacacctgttattcctgttcctgctcggggcgtcgctcatgattttcagaacacgcgcgctggtggtggccagtattgtggtggcggtggtgtcggtaacggcctgcgaaatcaattattactatacactgatcactcccatggaaatggggcatagccagcaatttatgatccgctggataacgctaccggcgatcctcctgctggatgtagctactatcttcctgtatgtaagaaaactaaaaacgctcaatataaaactggcaaaagcaacggatgagaaaacgatctttgtcagggaaaccagccatgaaatccggaacccgctgaatgccatttatggtatcagccaggacctgatgatgaaagcgcagaaagaggaacgttatagtgatatccgcccggaaatagagcacctgtattccgctacgcataatgttttacagatcatcaataatgtgctggccatttctaaaatagaagacggcgcagcccatgctattcaccccgaatcatttaatatccgcgaactgatttccgacaagatcatcgtataccaatacattgctgatctgcggggaataaagatcagggcagatattgcagaagatatgccctgctatatactggcagataaaaacaagctcgcacaggtgctgaataacctgctgtttaacgccatcaaatttacccgcaccaacagcctgatttcagttggcgttttgtgcgaagaagcacagtggcagttcatggtaaaggaccagggccagggtattccagcagcggacctggtgaccctgttcacaccgtttaaatcaggtaaaagcgattttgaaggaacgggtcttggattaccgatcacaaaaaaatatgtggaaatgatgagtggaaagattactgttaccagtataccggaagaaggagccacctttattgtgcggttaccattaacggtgagttcggcgccgtcgcctgcccagggaggctggatggagttaacgctccataaagggctgaaaagcctggtaattgatgataatgagatgagccagctggtattgtccagctttctgcgcaggctcggcttcactaccatagtggccggcagcggggcagaaggtattaacaaagcaatggatgaaaaaccggatcttattttcatagatagttatatgccgggacttagcgggaaagatacccttcaactgctcggtgatatacctgctttaaaaaatattccggtgatcgccgtatcgggcgatgcattccaggagtcgatcgatgatatgcttggcgcgggcgccagggaatatatctctaaacctattgatcttaaactgttgaacagcaccgtaaataaagtgttgttccaatagttacgcatatacgtactgatagcgggtagtatctttaccactccagtcgatgttgcctttcatcatttgtcccaacgttaaaatatacttttccagtaccggccgtacgccagctgcgcatacagcggtgagcacatcggcggtgttgttgaacaatgcaacttcggagttgtggatcttcacggcctgttctaccgcctggtccagcgtaagctgctggtgatgtttcagcagcataaccaggttcagttcatcgccgagttctgattctttcgagaaggagtagagatcgttggcccagcaaatggtacggctgcaatataatcccatgttttttacctgcgggttggcgcgcagatcggcgggcagatggatggcgcccatcagggtagccagttccaggaaaaagttggcgccgccgatctgggggcggaagcgcatataatctttcagggaaatattgcgggcatgatctacgtgttgcatacgccacaaattggccgtaaaggcatctttcaggctgcgggcgaaacgcgtctgccaggcccggttgctgatccggcacatccgctgccagatatcgctcatggcagccagcaggggaccgccgctttccagcgtaaacgtccggccggtttgcagtatctgcatcatgtgatgcgccatacgctcaaagccggtgttgaattcattaggcgccagcgcatcgagatgatcatcccacaaaaaaagaagcgtgttaaaatcgctcgcaatacataaagaaaagaaaggtgcatccgggaacatcctggctaccatccaggtgaacttctgatcatgataagcattccaggagctttcgtctgtagcaagatgaaaagtatgcacccaaccagtggtatgcgcatccgcttcatgtacctgcgggtgcaggcgctgaggatagggacaataaaggtccggacgggaaatagttgtaaacatgacacattgtatttaaaagtgaatagataaaagttgacgttgatagctggctttcgattacttttacaaaaatctcaatgtacctggcgacgtgtgaaaaaatagcaggaacgcttctgcaacaatgaacaattgaccaattcagccgttatagttataagcaaattatcaaccgttactgtaatcaaccatcataagcaagtgaacaaatcgcgcaattcaaatcagtcaatagcataagtattatcaaccttaaaactcacatgtatgtggacttgtttacgttcctgcaaacgcggaacattttctttatacctcatgctctgctgtactgctgcagcctttgcccaaaacattaaagtcaccggaacaattacttccaccaaaaaggaagtgatacctggcgtttctgtattactgaaaggtactaaaacaggcagcgtttccgatgcagccggtaactattccatcaacgcaccggccaacggcgtactggtctttaatgccatcggctacctgcgccaggaaattcccattaacaaccaaaccactatcaacgtcaccgtagtggaagacaacaaacagctgggagaagtagtagtcaccgctttgggtatcaccaaagctaaaaagagcctgggcttttcggccactgaaattaaaggcggcgacctggccatgaccaatgaagtaaacccggtgaatgccctgcagggaaaagtagccggcgtgcagatcgaccagggcgcaggcggactttttggaagcaccaagatagtgatccgcggtaactccaccctccgtagtaacaaccagcccatttttgtgatcgatggcgtaatcgtggataatggcacgttcagcggtacgggccgcgactttggtaatgacctgaagaacctgaacatggaagactttgagtcggttaccgtgctgaaaggatcatccgctgccgcattatacggttcccgcgctatcaacggggtcatcctcatcactaccaaaaaagggcatgaaagaaaaggtttaggcattaacgttagtcagacgtttaatgtattcaaaccttactccggccccgacttccagaatgaattcggcggtggcaccgtaggcaatttttttactgataaccgcgatcccaattacaaaccgaacgaacaatggagaacaaaagtgttccccacagacccggccaccggtaagccgtatatcgaccggcagataggacgggaactggagaactggggaccccgctttgccggccaggacgttatcaactacgacggcacccccacaaaatatgtagcgcaacccaataatttcctcgacgcatttcaaaccggtcatggttccgctaccaacgtgtcgctagatggcggtaacgaccgctccaccttccgcgtgtcttacacccgcgaccagagcgaaggtattgtagctaaaaacagcctgctcaaaaacagcgtggaagcacgcgttacccatgtgatcaataaattcctgagcgctgatgtaagcaccaactacacctacttcaccggaaggaacccgccacggctgggtggcctggatgcctttgcttcctataacttcggtaaactgtttacctggatcctgccacgtaactatgataccaggtactggatgcaaaaacaacattacaccagcgcactcggcggcgctcccaacccggcagatcctaatgaaacgaacaagtcgccggaatcccgcttctggtttaatttatatgaaaacgattatttccagaatgagcaaaccatccgcgggcgtgtagccattaccgctaagctcaccccctgggctaacctggtactggaaggcaacgtaaataacctgtacaccaaaaatgaaaacaaggaactgggacagggacagaatttcaccggtggcttatacggtctcggacatacgagcaaagaaagttatttctttaaatggatgggaaccattaataaaaccctcaccaaagatcttgacctcagcggttacataggcggtgaaacccaacgtttccaaactacctacaattacagcgaaacagtaggcggactcagttaccccggcaattacttcctggcaaactctgtagagaagccaagagcagaaggcgggctgaaaagtaagaaagcctttaactctatttatgcaagcgtggacctggcctggaaaaaccagctgtttgtacagggtaccttccgcggcgactggtcatccgcacttacctataccgatggcagcggtaatttcttttaccagtacccggctgtcagcgtttcctggctgttctccgaaacctttaaactgcctgcatggatttcctatggtaagttaagaggtaatatcgccggactgggtaatgacaccgatccttttaatatcaaccccggatttgcgtttaacggttacacttcttccggcggcctggatctgcccatctctacttacagccggtaccccgatccgcttaccggtaaatttattgcactggtacccgatctgaaacccgaaagaaaagtagcaaaggaactgggtgcggaaatgcgttttctcaaaaacagggtaggctttgatgtatctgtttaccaggataataccaaaaaccagatcctcgatattggcactccgccggaatccggactggaaggcattatcatcaacgccggaaatatccagaacaggggactggaagtgatgatcgatggaacaccggtgaaaataaacagctttgaatggaacaccagcgtgaactactcccttaacaggaacctcattaaatcgctgtaccccggcagaacagagtacgacctgaaagccaatgtaggagaaatcagtacctgggctattgtaggtaaatcctacggtaccctccgtactaccatccattcaaaagcataccaggccaccgacgccaatggcaacccggtagccgatcccaataacggcaaacctgaactggcctggcgctccgatgcacgcgccggatttcctgcccgcagcaataccctgcaggatgtaggtgatatcaatgcaaagttccgtgcaggatggagcaatactttccggtttaaaaatctttcgctgaatgtattactggatggcaaatttggcggcgactttgtactgcttacctaccgttatggcacacataccggtgtattgcccaacacgctccagggaagggatgcagaacatggcggcatcacctggacgagcaagtatgatcagcaaacctacgacgacggacttattccagacggcgtatttgccaaaggccagatggtgaccatgcccgatggctctcaggtaaatgtaggcggcatgacctatcagcaggcttatgaaaaaggttttgtagaacctacgcacgccccgcagttttattatcgctatggttcttcttccaccggtgtttccgattactggatcaaaaagaattcctggatttcattaagacaggtgtctttagcataccagttttcaccggcactgtgcaagaagctgatgctgaataatctcagcgtggcgattattggccgcgacttactatacctgtacaattcattgccttttaattacaatcctgcttccaacaactccaataacacggccttctccggtgaagaaggatttctgccgatggtacgctccattgcaggcactatcagggttgggttctaaggggaattaaattgtacaaacaaaaaatcaagatcatgaaaaatacatttcaatatataagaaccggtttgttgctggcactgctgggcgttagttcgtgctctaaaaatttcggggatatcaataccaaccccagtctcgtttccaagccggatgtgaagttccttttaagttattcgcaggataagatcattacctaccagggtacagaatgggtgtgggaaagcatggaacagctgatgcgttttacgcagcatgttacttccagtccgtacgaaatcaccaacaatgtaaatacccgctataataactactacctgcaaatcttacctaatctttttgagataagaaagcaggtagaggcgatgccgaataaagatgcgtaccagaaggttgctatggccacctacgtattacaggtgctccacgggattaaagtaacggatatgaacggctccattccttattcacaagccattgaaggccgttaccaggcgcaatacggaccggtatacgatgagcagcccgccctgttcaataactggctttcacaactcgatgcggccattgcggtgctgtccaataattcactgcctgcgcaggtaggctacggtcaatcggacattttttaccagagcgactggactaaatgggtgaagctggccaacacgcttaaacttcgtatagccgccaggttagagaacgctgataaagcaaaatgccaggccatttttcagcaggtattaaaagacgctaccgggcctattgatggtgacgattcacaggtgaagtatctcaacagcacctatacgccctttggcaacgggggagacatagattaccgcagccgccgctatgccaccacttccatcatggcgttcctgaaaaagagccaggacccgcgtttaccggtatattttgaaaagaacgacctggtaggcggttataaagattcgctgacaaaatacaatgttacattgcctgctttcattaatcccaacgatccgctgatcatgtaccagggcggtccggccgactggaccaccaatcccgctgtggcagcgtatatcgggaatggatttattgtgagtcagtataccaaatacaacctgatatcgcccatcaaccgcaggttcttttctcccaaactgaactcggctacgggcaatttcctcgatgtaccggttacctacgccgaaacctgtttttatatagcagagtttatacagaaaggatatgccggtggagcggataccaaaggaacggcggaagactggtataagaaaggtattacatcttccattcaaactatgaatgcgattgcggtggcagccggttctactaccgcctacacgggcaccggtttaactgaaatcaatgcctatctgaataatgcgcaggtgaaattcaatggcgttaataacctcgaacggatctacatacaggcttacctgagtatgtaccggcaggctaatgaagcgtatgtattttgcaggcgcaccgggtatcctaaaacgggctctgcttactatggcagggaaacttttaatgagctgataccgcgccggttctggttaacagatccaggcgaagtaaacagggccaactggaatacggcgatgcagcagcagggctttacgcccaatgcgcaggatttgcctacactgagttcgcaaaggatctggtatgataaacaggcgccggattttggaaagggattgtagagaagtggtgttacccaaaggagctgcctcatttataaatgaggcagtttttttattttgcggttgaaagagaattaatatggtaaatttgaatttcagtggccgattaataagtctctttattacttctccaatacttctcggatacatctccaatacttctcagatacttaggactcgtctatgtgtcgtattccccatacagtccccatacagtcccgatacagttcccatactctcacaatactctcatgatacactccccatacactccccatacactgggactatttctgaccgcaacagattccggcataatccggcaaaaagcggcaaaaccggcaggtttatttttatgcatttatgcagaagagtaacttcgaatctcaaactttcggcagggtactataacgtggcggctatcctgttaacggtttctttcagcgctgttaaagaagaggtactcgtcaccttattgactttcatccggataattttatccttctttcttaccatgatcagctggaagttatcgctgtcggtttgaaagaagccttcatcgccggtgttatcgagtagctggatgttgccattgcggcggttgtcgtccaatataccggtgtaggttttttgtgcagcagctactgaacggtacttttcatagttgtagtacacattaccggttttcccggaaacggggtccgattccacggctgtaaaagcgcagcggtacttcagtgcatcgcgttcctgtttttctgatttcagggtgagtaatgcaggctggcccagtattttggcggcgtctgcgggagtgaggtagaagtagggaacagtatctgtggcaaagcctgatgaaatcaggggaagcagcaggaatagaaagagcagtgttttcataacagtatcagttaagaggaattttacacggttgctacttttcttgtatcacaatgtcttattgctaaagcgtcttgttgtattgttaatgaagttacaacttcctgtttgataagactaataagtttcccggtaagtcagaagccggatacatcaatccggcacggcgtgaaaattcttaatgctttctttttttgctggacgcttcggtgttgattttttctttctgccccaccagatgagaaaacctgtaacaggtaaagaagcggcaatcagggcggcgaagaacatcaggagccggcccgggagtccggcgatgctgcccacatggatgtcgtaattcatgcgtaccgctttctctgccacggtggcgtctttatacttaccgagataggaaggcgtaatttcccggccggtatgctgatcgaaatagaggtagtcggcatcataaaactggtggcgaccagggtaggccctggcaatgatggctgcggaatcgttggcgggcagggaaatgctgtagcctgcggcctgcggataatggtccataaaggatccaaatacctggttaatgagggtgctgtctttcaccggcgcatgattaccggatttcaccggcacggcacccggccttttctggccgccgctgaatacccagaattcagcctgcgccatccaggtgaagctccataccaggccggttaaggcggcgaaaataacgatccagctggcataaaatcccagcacattatggagatcatagttcagtctttttggtgaagcatccagcttaacgcggaagctgactttccggcgggccttgttgcgcggccaccacagcacgatgccggttaccagcatcaggaagaacaccaatgtactgcatccgactataacgccgccggtttcctgcgggagccacaggtgcatatggccttgcaggataaaatgaaagaactcatcgtcgcggttaagcaccttctgcactttggccgtatagggatttacgtatacgttgtagtagtgatagggtttcttttggaagaactgaaccacggccgctttgtctttcccctggtacaggatgcggaatgccttttcgccacccatgctggcttctcccgctgtacggatggcggttacaggctgaaagggctggtcctgcggagttacgtgctgataggaagccgtgtattcagacaattccggttcccaggcgtaaatggcgccggtgatggaaatgatgaatacaatgatcccggaaacgagtcccagccagagatgcagccaaccgaatatttttttgatgcgcatgtgttaaaatgtaaaatgaaagcacagcgaaccgtgctttcatggatgtatgaatggcgaaaaccctatagtttgatcacgaggttcaccgcatagttacgtggcggctgcggctcgccccatggaccccaatacatcgtatttgaaacattatccagttttataccgatgcggtaaccaggccggtcgtagaacacggtgctgtttacgagtgcataggcagggaagaacaaggtattggcatcgtcaaaaggcgtttcgctgttgtaaaacaatccgccgccaatgccgaggccctgtagtttccctttcaccagccggtagctgatccaggtgttggccatatgcttaccgccggagcgcgcaggtcgtttccctacgttagcattggctttggtgatctcgctttcattgaacccgtaaccggctgtaatgttaagtccagggaaaggattggcgatcacttcggcttcaaagcctttgcttttctgcgatccatcctgtattgaaaaggccgggtcttcgggatttgagcgcagcttgtcggtcacgttaatgtcgtatgcgctgagggtaacgtttaatttgcgctcaaacagttctgctttcacgccgccttcccattggttggcctgttccggcttgaagaggttaccctgtttatctgtttgggcgctgtaagtaaagccgttctggtagttggcgaaaacagacagctggtctttgatcagctggtatactacgccgaattttggagagaaagatgatttgctgtagctgccggttacattgccgttcagcaggttggtggtgccctggttatctactttatcccaacggagacttaacatcaacagcaggcgatccgtaaaattgatcacatctgaagcatagatgccgtagcggtcaagatggcttttatagaagttattcgcctgtgcagtaggagtagggaacataggataaattttttccatcatcaggaacctggtaggtgctgaagcgctcaccgtatcgaggatgaagcgggaagtataagttggctgcgtgatatcagccaggtaatccagacccaccagtatacggtgtttgatggaaccggtatggaaagtaccattcaggttctgctggagctgaatagtattgtagttgtgactatacttctgaagctgacgggtgatgctatcttttcccggcagccagttgccggagaactggtactgttcgcgggcgttcacaccgccggtggagaatacggtggtggtgttccagttactgttgatcttataattcatttgtgcgaatacgttatatccggggaaagtagatataagatcattggtataaaaggtccgcttatagtatttacccattgcctctttgtaatcagtaacaccggctgccgggttcagataggcgatggacggtgttccgcggttacggaacgtttcgaggtctacgaggaagctcagtcgctcattagcctggtaagagaaggcggcagacaggaaatagtttcttttgaagcctgcttcctggaagctttcctgggcatgcctgccgaagtttacgcgcagcagtgctgttttttccttattcagtggtgcattcagatcgatggtaatgcgattcaggttgtaacttcctgcggtcaggctaacatctgttttgaaggtatcgaaaggttttttggtcacacggtttaccagcccgccataagatacggcgccggtgccaaataatgtgccggaaggacctttgatcacttcaatcctttccaggttggatacgtctaccgttaccagctggttggccatcataccatttcgtatatagttctgcgtgcggaagccacggataatagtagaggtacggccattgctcaccgtttcagtggaattcacgccggctacattcttgatcgcatctttataatccacgataacctgctcctgcatcaactcggatcctacaatgctgtatacctggggattttccaggttcttcaacggcatgcgggctacgtaatctgtttctttttttgcaaatttattacgaccgcttgctacaatcacttcctgcaaagtttgtttggaagcactgagttggaaatcggcttccgcagtttctcctgctgttacggtcactgaacggctgatcacatcacggccggttataaaaacctccacggtatatgtgccgggagtaatattgcggagtgtatacgttccattttcgttggaggtagtttgtttgcgggaatctttcaaacggagtcccacaccaggaaccggtgtgccgtcttccactgtaacgcggcctttgatggcgccgtgtgccggatgctgcgctttaacagccgtgcttaacaaggccagtaacgcgcatgccattgccaatgcaataactctcatgatcagtttttaagatttagggaatagtgggaatgctacaacagacgaacatagtatttatgttcgcaaaggtaggaggcaggaggggcacaaaggaatcggatcgggaatttggtttactcaatcgggaaaaaaaagatagcaggaatcaggtccatataaaaagagggtttacttctttataaggacctttagtttagcggtataaaggatgctgtactaccgttgcgactgggttcttcccacaacaatttacaaagtttacattttaagttacaatcaggatccttgaagttaaaaggattaaagtaggttcgctgtatcaagctttaataggatatgaaaaataaaggaacctttttgaatagcctgctcactatgcccgctgaactaattcactcttctgtacaggctcaacagaaacatggcgctaaggatgtcgttaactggctacatgtctatgaaagcaatgcagcgatgtttctgttcccgataattaaatagaaaaaattatgaaatatgcacacgtatatgtcctcttccggatgcttgtttttcatacttcctgcggacaaaaccaaacaaacgtaccacaggataatttcagtaaagaacataatggctactccgagtctcaacttaaagagttggctacctccaaggtacctatgagtcaggttcggcatgtaaagcaggccagaacattttacaaccagggaggggcttgccaataacatggttatgtctatttatgaagataaaggaggtaatatctggttcggcggaaatgggctaagccgttacgacgggaaatcctttcaaaattttacaacgaaagacggacttcccaataatggtattaaggctatcatggaagacaaaacagggaaattatggattgccacatgggacgggccttgtttttatgatggaaaaacatttaccgttttaaaagacaaagatggcaaagtgtttaaaaacgtttggtcaataatcgaagatgaaaaaggaaacatctggactacaggtagcataaatcctcctggtgggtcagtctgggcgctttcacgttatgatgcaaagtccttgtacaacaaaaaacctgctgtaaccgaaatcttgtcaagaccaccagcttttttgggacttttagaagctaacgatggaagtatttggtttggatccggaggcggggtgcatcgttatgatggaaagacctttacagactttaaaaagtaaagaaagtcagaaataaagtaatagccagccattttaagatggaattgtgcttcaggcggcacatttttcagcatcggcaagtggctgactagtatttatctctgacttagaatacctttattgctactccagtccttcaaatatttttcctgcggccacactcaacgcatcttgtgcagtgcggtcggcttcattcgttaatatcacaataccggtattccgttcagggtaaacgacgcagtaactggaaaatccaaacgtgccgccgctttgccagatccttcttataccgttgctggttttattcatctgccagcttaaccccatcgcatagctattgatatcgccccaggcaggttggtgtgttaattttactaccgggttgttttcatcggtttgcaggcggacatattgcagcatatcggccacggaagaatagatgccgccggcagccagcaacagcgggggattgtatggcatgatccgtccctgttgattatagcctttcgccgcattatcaggaagtgccgcagtggtgtatttcatctgctgcggacgggtaatatattttcttaccagttgggcgtacggcatgccgtatatgcgttccagtatgaacccaagtagttgtgcccctgcattggaatatttgaaatgataaccgggaatggtatccagttgtacctggtgaagatcattgaggaaagcagccatggaatagtcgtgctgcaaactatcgatcacgcctgggatggaatcatcagggcgctggaaaagatcgcgacggtcgggcagcatgaagggtaagccggaaacgtgtgcaatcaggtgtttcagctggatagcatgtgctttgtattgcaggttgggatagtcgccgttcaggtaaaagcggatgtcatcatccagtttcacttttttatctgttactgctttggccagtaaatagccggtaaatgttttggaaacggaacctatttcgtagggtgtgttgggagcggggaggtttgttttactgtaacggtagatataggtctgtccgccggtatatacccctacttctgcactaacgcgggcgttgtcctgcataaaaatggtgagcgcagattgaacaagactgtccacttttgttttatgaagattatctgttgttacctgcgcctgcgaaagaagcgttgataagcataaaagaaatgcggggataaaatgtttcatgttggttttttgaaaacacttatcctaagagaatgccatttggcacagccttcactgttatcttcttatatattttaaaataaaaatacctgtatcgaaaatgaacaccgggtgtacgcaggcgcactacactacgggtgcagtggccctttacttacttcttcgcctgctttgtataccgctgctattttccgggtattcttaatatcctgtgcagggttggcgtccaggatgatcaggtcggccgttttacctttttctatagtgccatagtgctgatctattttcagcgcagccgctgcatttttagtggcaatggtaatggcctgtaagggagtcaggccggcctgtacgagcagttccatttccaggtgttcggagaatccctgtgtgcgcaccggttgcgcgccggagtcggtacccagtgctacgatgatgccggcatccgctattctctttacatttttcatcgctgtttcaaatgcatggacattccgttggtaggagggggagttctttaacttatcctgataggcaggcgaagtaatcatttcatatacgcctggttctaacgacgctttgaagaaaggatcattgatccactccggcttacgggcatagatatacgcatattcatccagtgaaagggtggggatgtaaatgactcccttggctttcatctgttgtagtaatgctgcgtcaatttcctggtcacggatgctgtgggcaatgatgtccagcccgctggcaacaagacctttcgcatcttccagatagtaaagatgtgaggccacagggatatgatgtgcatgggcacgggtgatgagcgccttgtaaatagcagggtccattttaggagcagaaccgccaaaatcatctacccacatttttattaccgttggctttaccagcgccacgctatccagttgtgtagtagcctgtgccaccgtagcggggtgatatacatacttcatcggcggacccccctgtgtaccggcaaatccataaccggctgaaaacaggcgggcgcctggcagcaagccgtttacagaggagtcgcgtaacccggatgcaaacagcatcggctgatcagatcccatcacgaggatgttggtgatgccatagtccgcgtactttttcagttgtgataatatgttttcgcgggtatacggatcggtgctgttatcgttgcctttcatcatgccaatatgcacatggccgctggtgatagcgggcataacggttttgccggtgccatcaattattgtggcaccaccggctggtaaatcctttccggttgcagcaatttttccatctttgatgaatatatctgtatgttccgttggtacgccaccgttaccatcgatcaatgtcacgttcttcaacaggatggctttaacaggtggtgttggctgaaaggcagccagcggtaacaaagcgaggaggagtaacagataatttttcatatcgttgggctttatggagaaataaagataggaaaatctcgctaccccactatccccattataaaaccaatcgcctcttccgaatgcaatgccgccgtcgactccatcgtcatcctcgccgtttcacccgctctggcgcgcatttgtttttcatacgcggcgatggcagcatgcacatccgggaagttttccccggtaagcaattgtcctaattcaagggcatccagcatcgccatgtttacgccttcgccggcatagggaggcatcaggtgtgcagcatcgccaagcatagtaaggtttggtaatgcttcccaggtttgatcaaacggcatgcagtattgcgggcgtactataaaattagcattggcattttcaaacagttccagccagacgggatcccagccggtaaaggtggctttaaaccaggccagtacctgtgttttatctgaaaaattgaggccactggttttataccagttttcggcggtgtttatcccggtataaaatacaaggctgccgtcgcctttggaacttacgattaaagattgcgcgtcacccagtgcaaatacttttcctccttttaccagtgcatggatgttagggcaggtggttgctgcatcatatacggcgccttccacgatggtaacgcctgcataaaaaggctgaatgggcgtgatatacggacggatctttgagttggcgccgtctgctgcaatcacgatgtcggccgtggcagtgctgccgtttttaaataccagctgccagccgtggaggtgtggcgacatagacacaaactggctgtcccatacaacggtgtcgggttccagcgaatccagcagtatttctttgagcggaccacggtcaatttcgggacgcgacctgtcctctccgccattttcatggtcatccaggataatggcggcgtgtttgtccacaatgcgtagccggtcggcgccggggcggtagttggccctgaatgcttccgtcagccccgcttcttccagtgcctttaatcctgattcctcgtggagatccagtgtagcgccctgtacccgtgcttccctgttaatatcccgctcgtatacttttacgtctgcatggttcatctgcagtatcctggccagtgttaatccacccggacctccgcctacaatggctatttttttgtgttgaatgatgctcatgttgttgtttaatttatttcagcattcctttgatcactgcgttgcagcattccagtatcactttttctgtgatgagttgtttgggtctttgggtataatcaaaatattcatttaccaggtccagcagcggggcaaataatagggcacggagaatatcgggatgaaaattcgggatcacgccttgttttacctgttgcttaaaaaactggtggatgggtttaaaatactgtccctgttgtatgttagcctgctggtatgctttattcagcaggggggaggttttcccgttttgaagcaatgcaaaatgcgtcctgttaagggtcaggtaccggaagctgttttgccagagcttttttacgccggtcgcaaagtccatacccgcgtgaaagttttccagcacggctttttcatacgtctccagtacttcttctatataaagttttaccaggagatcttctttatccctatactttatataaatcgttctgggcgatatgttggccgcttttgccagcttctgcatggtgaggttttccagtccctcttcagcaatgatctgcaatgcaatggtgcggatggcttcctccttctccaggtttttaggtctcatgcaataaatgttactgcaaagtaagtaaatgtttgtttacttacgaaatctttcttcctggagataataaaaaaagctgccccggaacatgcttgttccggaacagccttgtctttcaggtgccactattaattttttatttcgccgggaattacttccactacctgcttcctgccaccccgcagtatgtctaccgggatcttcctgccgatctgtttgtcggataatagaagatgcaggtcatcaactgaagtaaccggtttattgtcgaatgcaataatgatatcgccgatatgcagttcgctgttgtagaaattaccatcgggaacggtttcaaacacgtatacacccgtgtgaatattgagtttgttggcggcaatcatcctgctgctcaggtttaccggctgtgcggcaatacccagctgcgccctgcggatcttcccgtgcaggatcagctgaccggcaatctgcgctgccaggttggaagaaatggcaaagcaaagtccctgtgcggaagcgataactgctgtattcacgccaattacctgccccagggagttgaccagcggtccgccgctgttgcccggattaagggcggcatcggtctggatcacattgtcgatcagccggccattgctggcccgcagcgtacgccccaatgcgctcaccacaccagcggtaacggtatattgcaatcccatcgggttaccaatggcaatcgcaatctgccctacctgcagcgtggaggagtctgccagcggcatcgctttcaaccccgtttcgtcgatcttcaatacggcaatatccgtggaagggtcggcccccttaatttctgcgtttacgcgcctgccgtcaacaaacgacaccttaatactgtcggcgttttctacgacgtggttattggtaataataaaaccatcggaagaaataatgaagccggaaccagtgcctccctgcgttcgcctttcccgcgttcgctggtcgcttacttttttctgtacttctatatgtaccaccgattcggctacagtacccactacgccggtaacggtttgagaataggcatccaataaactcttatcgtccgacacctgttgtgtgagaaatgaaattgagttatccataatgtacaggtggctcaaatatatctccagtttattccggatgccgttttgacatttgatgaaccggctttatgccatctttactttttctgcacttgaaaattataattatttggctattttgacggggaatgtttttcgtctaataaggaactatgccacaggcacaaccggatgccaatcccaacccggggcagaacccgggttacaaattataaatcataccgcggagggaaagcgatttccctccgctactcaaaccataatgtaatacagttgccgatagcatcaatcagcttcttgtcttttacaagatccattttccacccgcttttcgcgcaacgtataatgccaatggcttcatcattgagcatcacttctgcttcatagcacacccctttggcacaggtttccgatataggcaccgcttctcctttatagcttttaccattcaattcaaattcaatcgggatcaccgtgctctccagctgtgccacaaattttttcaggaaggcaatcaggtgctttcgttgtgtaggtcccgaagtgctccatttgcctttatccgcacgcttgtgcgcaatcttgaatttgaggcccgtcatggtagtggcatagtcgttggcatcaagcttcaccgcactttgatgggcaaggatataccagtgatacgccgtacccaccggcacaccggatccttccggcgcctttcctgttctgcgcttggtaacagcataagatatttcccagagatcgggtgtgatcttcgtttctttccagtcgccctggtcatagtgccagtgatgtccccggcctatctgaacgcctgtatattgtttatcgccaaaggttttgaatttatcgaaagaagtgaccttactctttttagcgatgctgcctgtttttttggctgccgcttttttgggcgctgctttctttgtggcagcagtacgtgtactttttcgtgtatttgttttcgtggtttgcatagtagccattgtactgaatttataagtaacaaaagttgagtatacataagagggcgtccaaaaaacaaaccatgttgtgcgcatggcatagcgtttggtttttacttcatctaccaaataccagcagctatggcaaatcttaacggacacatggtttttgaggccgcggtgcacagcagtgaagcacacgccttttataaagaggccttgctgcacttagaggagagtggggcagaatttatgctgggtggcgcttttgccatgtttcattataccggcatttaccgcgataccaaagatcttgatatcttttgtaagtggacagaataccccaaaatattgaaatacttcggcaaactggaaggatatacagtagaattaaccgatgtgcgttggctggctaaagtattcaagggagaatattttatagatatcatttttgatacagtcaataacatttgccgggtagatgatacctggtatgaacacgctgtgccggccatttttgaaggggtgccggtaaaactgatatctcctgaagaactgatctggtgcaagatatacgtacagaacagggagcggtacgacggcgcggatgttaaccacgtgatcctgcggcataatccactcaactggaagcggatcttattccggctggatcaacactggcatttgttactgcagcagctgatcaattttcagtttgtatacccggcagattttcaccgcatcattccccgctggcttttcgccgagttaatgcaacgggcgctggaacagtatgagctgccaccgccaacagaaagggtttgccggggacctgtgattgatcagacacagtatgccactgatataaaagaatggaattataaatcatctaccataaaaacggtttgattatggcagcagctacacaaccaacgaggatagcagcggtaggcgatctgcatataggcgccaacgacaaagggaagtggacggattatttcaaagccatctccgctaaggcagatgtattgctcattgcgggcgatctgaccgataccggtgatgaatcagaagcacaggtattggccggagaactggctgcctgcaccatccccgttgtagccgtattaggcaatcatgattacgagaaagggcggcacaaactgatccggcaaatcatccaggaaacccacgatgtacatatcctggatggcgaatgcacgatcatcaacgggataggatttgccggcgtaaagggtttcggcggtggattcgatggtcatatgctctctatgttcggagaagatgaaatgaaagctttcgtgcaaacgggggtggatgaggctttgcggctcgacagggcgctggcgcggctggaccaggaacatcccgatatccggaaaattgcactgatgcattattctcctgtattggaaacggtagtgggagaatcacaggagatctacccattcctgggctgctcccgcctggcagaacccttaacaagacgtaaggtagtggcggccttccatgggcatgcccatgtggggaagctcgaaggccagatcaacggcctgaaagtgtttaatgtagcgaaacccattctgtctgaggccggttattcacccgccttttttttatatgaagcataggtttgtagagatatttacaggtattgtgcattttattctatagtgtatgaacgaacaatttaccagctacagtcagctgatctttgataaactgcataactggtttattaccgcggttaaaatgacgcccaattttatactggcggtgatcatctttacgctgtttttattgctggcgcgttttacccgtaaaatcacctaccggttttcgcaacggttgtctgaaacacccgccatctccaacctggtatccagcttattctatatcctgtttttattgctgggcttatttatttcgctgaatgtattgcggttggataaagccgttacctcattgctggcaggcgctggtattatcggactggcacttggctttgctttccaggacctgaccgccaattttatttccggtatttttatcactttcaaaaagccgtttgaggtaggtcatattattgaaaccaacggttttaccggcagggtagatgccatccagctaagatccactaccatgatcaccgcagatggcctgcatgtcattattccgaataaggaaattttccagaaacctattatcaatcattcactcacaccactgcggcgcattgcactcaccttctctattccattgtcggataaactgaaggaggcggaaaggatcatgacagatattgtagtgcagatgaaagaggtagtgccggataaacccaaaacagtttggtacagcggtattgatggaggcgcggtgaaagtgatcctgagttgctgggtgagcaacgaatcggatgatgcgtatgaacgcactacccacgaattgatcacaaaagtaaccacgtcgttaaaagcggcaggtttgatgtaaaaagcaggaccggcaatagagccggtcctgctggtttttacggacgtacaatggttgttttttcctcatgcccgcggtggcacccgggatcattattccaatgacgtatagccatccgggtgagcagcacattggccgcaataaataatacaatcaccagtatggaagctactttagtgatagtgcgaagggccggtttttttgaaaatccgccaaaaacataaccgataataaataccatgctggccgcaaacagcacacgcagcacgataacaattccaagtcccataatcattctttttaaaggttatttaattttacccagcaattgctgatcatctgtccggccccagtgcgggtacacatctgtgccggggttgcccagcttttgcaggctttctgtagccagtttttttgcctgttccttatcgccgccccacattttcggggtgtagtattttacccacgccgccacatacaatgcgcgtggattaccagggtccaatgccagcgctttctgaagcatctgtccggacagtacgccgtatttacggccgtaggtcatcggattgatgaacaccctggtacggtataccatacttagtacggtgtatacttccgccagttcttttttctgcttagtgctgtccagcaaggagagcgctttttgcgccattgcttccccgcggtcggcgaagggttctatcttttcgccgtcgtcctgcaggaggaacccggtctttgcattacacagcgccgcatagtagggcggcagccaggccggttgttcgctgataccggaaaatgttttctccagcgccgcataatccttcaccgtttgggcctggtccagttggttaacggcttgctgtaatgcattggattgcgccatgctgctgtagcctgatactaacataagggcgcagataaataactttttcatgttgatgtgtttagtgttttataaattattattaagaaagtcgtcggtacggtctataccgaaactcataaatacgccgatgaaataaccacgtgtagccggcagcgttaccggctccctgaattgcccgtttgcgctgtattgataaccgaacacctgtttggttccaaagaggttgttaacacccatcgcaaagccggagaagtctttccacttccggtttttaaagaaggagcagaggtaagccacgtgcaggttggcgatgttatatgccttagtggtgccctggtccgtaataccgtgggtactgatattatagtagggccgtcctgctgccagcgcccaggaaacattcacgttggtgctgatctcccggaaaaactttttaacagccaccgtggtggtatgcggcgccgtgaaggaaggccggagggcataaggataatcaagatagttacgtttggtatccaggtaggtatacgttatccaatagtccaggtctttgatactttttttatcccgccagaaaagttcaactccctgcgcatagccgttcccgttattgctcaatgcgggtattattttaaccaggttgcggtattttttataatacaactctgcccggaagaaacggttgttggcttttttggtgtagttcagcacatagtgggtagcgctggaaaaattgagatcacggaactggtaaagaaattcgttggccggctcctggtaaaagatgccataggccaggttaaactggctggcatcagggaggcggtaagcaaggcttatcctgggcgctgccaccagcttgcggagcacggtagcatattccatgcgtacaccggctttggcggcgaggttgggggcgaggtaaatatcgccttcggcaaaagcggccgacaggtgatccgttaaggcaatagcgctgtcgttggagaagcctttatcgcgggtataaaaatgttcagcgccaaagcgcagtgcttgtcctttggaaaagaagcgggtgaatacaaccctggcctgcgcaaaatcagtgcggatggtgtggctgcctgttttataagggagagatgaaacagcggtattaccttttgcatccgtgaggctgttggccgtagcttcgcggttatagctgtacacggcgccgaggtccatcttccagttgttgtccaggtagctgcggaagctgagattattgtagctgttccagccgcgcacctggtaccctgcattgagcacggcactgtcgatgtctggtttgcgcatacccacattactgtagctccagttgctgtacagtttgagcatacctgttttgccggtacgtatcctgaagttgaagttgccatctgcatatgccggtcctgcgaaataatcaggtacctgcggcactacgctgttgtacagcgattgattgctgtaattaaggttcacgccataactgcttttattatcctgggcgaggtgctggaaacccgcgcccaggttggcggggaacacgctgaagctggcggacgttttttccggcaggtcggtgctttccatgatgagcgcgctgctcatggcggagccgtataaagcagagtatcctcctgagctgaacaggatgcctttgaacaggaaggggttgatgcgggcatactgcggcacgccgggaacagcggggtagttgggtgttttgagcagggtaccgtcgatgaactgccgcgtttcatcaccggtgccaccgcgtacaaaaagccctgattgttcaccgatctgctgggcgccgggcagggagcgcagcgcctgtgcaatatcagcattactgccggctaccgttacggcgtcgataggagtgagcgaggcgcctttggcgcggtcgctggcttcaaagctgccggcgcttactacaacttcctgcaagggacgtttactttttatagtggtatcctgtttgctctgcgcgtaggcggcaaagggaaggagtgcgatgaaaaataaccctgttttcatgacggttagtattataaccgcaaagctaccgggaggagtgactgttattttggagagtagacgggaagggaaagtgtagcgacaaaacaggaacggttcaggattgcagcatccgggtgacgttctctttatagaattcactcaccggtatttcaatattgccgatgcatacaaggtcgcgtttcactgtagtgattttcttcacggccacaaggtaggatttatgcgtgcggataaaagcgccggcaggaagtttttcctccatcgctttcatggtcatgcgggtgagcacgggtttggccgtaccggacaggtggatcttgatataatcttttaatccttctatataggtaatgtcggcggtgaggatctttacctgggtatattccacgtttacaaaaaaggaatggtcttctgcaatcgccggccttttcaggcggaacaactcactggcacggttacacgctttcagaaaacgttcaaaggagaatggtttaagcaggtagtctactacctggaggttaaatccttgcagtgcgtattcttcataggcggtaacaagaatcaccatgggaggttgctgcagcgattgcaatagctgcaggccattcagccggggcatctgtatgtccaggaaaataaggtcaatgggttcctgctgtaatacctccagtgcttccatggcattgcgacaggtttttaccagttgcaggaagggcacctgccggatattatcttccagcaattcccttaccagttgttcatcatctacggctatacaacgtatcatgtgagcttcagtgttagggtaatatgaaacagcggtggttcgtccctgatctgcagctgatgccgtccggggtacagcagttgcagtcttgtttttacatttgccaaaccaataccagagttttcgtctttgctggcattgggatcgttatcgtattcattcagtacttcaaagataagcacatcctctttcatggccagttgtatatcaatagcaggatgcggcgtatagccggtaccgtgtttgaaagcattttccacaaatggaatcagcagcataggttctatgttgttgttgccggcagcctgactggcggccattttcacgttaatggccacttcgttgccgaagcgcagcttttgcagggcaatgtaactgttgaggtacaggatctcctgggaaagcagcacctttttccccgtatcgtacagcatataacgcatcaggtcggatagcatgagaagcgccggttccagctggtcggattttttcctggcgagcgataccaggttggttaacacattaaacaggaaatgcggactcacctgcgaacgcaggaatttcagttccgaactgagttgctccgcctgttgttccttctgccgtctttcagcgcgcagcatatctgttacccggcagtataccaggctgataaaatataccgccaccgacgggccgaacacaaatttatacgctgccaggtcccgcgcaacatccgggaaccaatgtgccatgatcgtatattttaacgggaacgacagtcctatcagcagtataaccgcagggaaataaagccaccaataccgcctgttccacaacctgggatacagcaccagggcatggatatagaagatagccatatggataacaccggaaagggtaaagaacaagccaggcaggctgcctatccggtagccactggctgcactggaaacgatatagggcagcaacagtattacgctccatatcactatatgcagcgcgatcgtaatttttttcagggagatattttttttcatctgctgtccggataaagctactgatttttataaagctagccgcattaacggcgttcattaaggaagaatagacgtccggggtaaatgtgcagacaacaccggcaggcagcgcgacagggaagtatttatcatattcagagaaaataccattattatagctgaatgcattgattaattttgatggccattaagatctaaatttcctgttatgataaaacgcagtatcgggatgctcattttattgatgagcgcttccctggtttttgcccagcaatatgaagccaactggaattccctcaacaagcggggcattcctgcctggttcagcaatgccaagttcggcatctttattcactggggtgtgtatgcagtgccgtcttatgccgtggtaggccccggtggttattccgaatggtactggtacaacctgagaggcactaaagaaggttcccatcagcaggtacaggcttttcatgataagaattacggaaaggatacgccgtatgaaaattttgaaagccagttcaccgcttcgttgtataacccccagcagtgggcatcaatattccgccgctccggcgctaaatacgtagtacttacttccaaacaccatgaaggctattgcctgtgggacaataaacaggcaaacgaatcctggggtcattcctggaacgctgttacgggaacgcctaaacgcgatttgctgggtgatctcacagacgctgtgcgcaaggaagggctgaagatgggctactattattccctgtacgaatggtttaacccgctctggttaaaagataaacaacggtatgtaaaggaagtaatgacgccgcagtttaaagacctggtaacccgttacaaaccttccgttatattttcggatggagaatgggaactgaccgatacggcctggcaaagcccgtcgctgctggcctggctgtttaatgagtcgccggtaaaaaatgaagtagtggtagatgaccgctggggcagtaatacccgtggtaaaaacaacggcgctacctatcttacttctgagtatggcagcggcatgcagcccggcgtcatctgggaagagagccagggcatcgggcaatcgtacggctataaccgtatggaaacggcggacgactacaagaaaagcgcggacctggtactgatgctggtagatattgtatcccggggcggtaacctcctcctggacataggacccaccgcagatggccgtattccggtgatcatgcagcaaaagctgctggacatcggcaaatggctggaagtaaacggggaagccatctacgactccaaaccctggaaggtaagccagcagtggagcaccggtaaacgccccgaaacgaaggaagccagctatatgtctggttacaacatttcgcagctggtgaaaaaatcagatcagcatgccaacgtggaattgtttttcacccggaagccgggcgctttgtattgctttgttccggcttaccgtcagcaggtggtgatccgcgattatacgccggcaaaaggcgctgtggccactgtgctgggcagcactaaagctgtcaggtggcagcagaaaggaaaggactgcctggtagacctctcgggcctccgccctggggatgtgccggatgggctgctggtggtgaaaatgaaaggataatattaatggcatacggaataacagagagaaggcgccatgccttctctttgttatttttaccattgccgtagttttattaaaaaataattttaaaaagtatatttttaaaggaacagaaaatcactttcgttcccatgctcctgaaattcagttacgggttgatagtttccacgttattactatcctgcacctcaaaaaacactgcgcaccgcacctggcaggtatacggcggcagtaaggaaaacattcactacagcgccttaacggaactggataccagtaatgtatcacaattaaagatcgcctgggcataccgtaccggcgacaccgcagaacgcacacagatccaggtgaaccccatcgtggtaggagaatggctgtacggcgtttccccacagctgaaactatttgccgtgcaggcggctacgggaaagccgtactggacatttgaccctgtaaaaaccggcgaaaagaatgctttccagtttaatccctgcaggggcattacctattatgaaaacggcggcaaagaacaacgcattttttatacggccggcagccggctgtattgtatagatgcccagagcggggtgcctgttaaagcctttggcgacagcgggtatgtggatcttcaccgcgatatgggccgtaacatggatcaactcgatattacctccactacaccaggcatcatctataaaaacctgctgatcgtaggcacccgcgtaggagaagccgccggcgcagctccgggctacatccgcgcttacgatgtgcacaacggccggttgaaatggatttttcataccatcccgcaaccgggagaagaaggctatgattcgtggaacgacaaagacgcatggcaacataccggcggggccaactcctgggcaggattcagcctggatgaagagaaaggtatcgtgtatgccccggtgggatcggctacagatgacttctacggcggcaaaagacccggcaacaacctcttcgccaattgcgtgctggcgctggatgcggccaccggcaaaaggatctggcatttccaaacagtgcaccacgacctgtgggaccgggaccttcctaccgcgcccatgctaataaccgtgaagaaagacggccggcaagtagaagcagccgtgcaggtgacgaaaacgggattcattttcctgctggaccgccgcaccggccagccgctataccccgtaacggaaacgcctataccggcagataccaccttacccggggaatgggcatcgcccacgcagcccatgcctaccttttttaaaccatttgtgcggcaatcgctgtcggagaaggacctgaacaccctggtgccggattcgtcccatgccgatatcaaagcgcggctggcatcgtataaaaccggccacattttcctgtcgccctccaggcaaggcaccgtgatctttccgggctttgatggcggcgccgagtggggcggacccgcagcagatcctgaaaccggcatcctgtacgtaaacgccagtgaaatgccctgggtgctcaccatggtggaggcaaaggatcagcacccttccgctacggaaacacaactccaggcagggaaacggttgtataccgccaattgtatgtcgtgccacggaccggagcgcaaaggcggcggtaattttccatctctcttaaatatccaggcaaagtatacggaaacagcattggaacaactggtgaataccggccgcagaatgatgccggctttcaaacagctggacagcagcgagaaaaaagcattagccgtttttttactggatgtaaagtcgaaacaacaacaaccttttactgcaccgcggaaaaacgtagatgcatatacgaatttaccttaccgcaccaccggctataataaatttttaacgaaagaaggatacccggccgtaatgccgccctggggcacactgagcgccattgaccttaacacgggaaaagtgctgtggaaagacaccctgggcgattaccccgaactgaaagcaaaaggcattcacagtggcacggaaaattacggaggaccagtggtaaccgccggcggcctgctgttcattgccgctacggccgacagcaagttcagggcttttaataaaagaacaggtcagctgctgtgggaaaccgacctgcccgcctgcggctttgccacacctgcggtgtacgaagtggaaggaaaacaatttgtggtgatcgcctgcggtggcggtaagctgggaaagaaatcaggagatacttacctggcatttgcactttaacagtcatcattcaacattcaaaatatcttttactatgagtatttcaagaagaaatttcctgttgaaagggagcctggcgatcgccggtaccgcgctgctgtcaaacgatctgctggcagccacagtacgtaagcccgtgctgggtatacaactatattctatccgcgatgatatgaagaaagacccgttgggtacgctcaaacaactggccgccatgggatacaaaaatgtggaacatgcagggtacagccagcggaaattttatggctattccgccaaagagtttaaaaaactcctggatgatctcggcctgctgatgccaagcggacatacagtaatgggcaaacagcattgggatgcagcaaaaaatgatttcaccgacgaatggaaatataccgtggaagatgccgccatcgtaggacagcactatgtgatcagcccttggctggatgaaagtctccgtaaaaattacgacgactttaaagcctatatggacgtattcaataaaagcggcgctttgtgtaaaaaatcaggtatgaagttcggctaccataaccatgattttgaattcagccagcagctgaacgggcaaaagatcttcgacctcatcctgcaaaacacagatccttccctggtggcgcaacagctggatattggcaatatgtaccatgccggcggtatcgcattggatattattaagcaataccctggccgctttgagctgatgcacgtaaaggatgaaattaaaacagacaagggagaaatgggcggtaaatacgaaagcaccgtattaggcaaaggcatcataccggtgaaggaagtgattgatctcggtaaaaaatccggtggcaccaaacactttattattgagcaggagtcctaccagggacaggcgccgctggatgctgtgcgcgacgacctggccgtaatgaaaaagtggggctactagctgcttcccgtctccactaaaatataatcactataatcagcgtaatcagtgagaaagacaaaattcgcgtatgttatgaagatgaaaatgatgcccgtcaccgccgcactgttactgttcgccggtatgtgctttggacaaacaccccgtgtttttaaaacatggacaccggccactaccgacagcgtttatgcgctggaaggacagggatggaaaacaggattgaaaagctattacgaccgcctgcccgcgaaatcagaaaaagaagtgcggccaccggtctggaacttgtcgaacaacagcgcagggcttagtctccgcttcagaacagacgccgacgaaatagtcatcaagtacaccgtttccggaccggtagccatgccgcacatgcctgctaccggcgtaagcggggtagacctctacgccaaaagcatagacggacaatggatgtggtgcgccgggaaatacgacttccgggataccatcgtataccggttcacccggctgaagaaatacgatcaccatgtaaagaatatcgattatacactttatctcccgttgtataattccgtaaaatggttatctgtagatgttccggaagaaagcgtgttcaagcccctgccggtccggaaagctgcgcctatcgtggtatatggcacctccattgcacagggcgcctgcgcatcgcggccgggtatggcctggacaaacatcctttcccggcagctggaaacgccggtaatcaatctcgccttctccggcaacggtcgcctcgagaaggaagtgctcgaccgggtagccgaactggatgcccgtctctttgtgctggattgcctgcctaatctcaccggcgcacaatatgccggcgcggaactcaaaaaacgtataaccgccgccgtaacattcctgcaacagcagcggcccggtacccccatcctgctaacggaacacgacggctacaccgatggtgaaatggattccacccgcaaagctgcctatacgcaggtgaacatcaccctacgggaagtaagggactccctgctgaaagccggcgtgaaaaacatcagcctgctcacaaaagaagaaataggccaggacattgaaagcatggtagatggcacccatcccaacgatattggtatgatgcactacgccaatgcctatgcgaaaaagatccgggaaatctttcatgaggaaggcggcaacacagctaccaccacaccgatcacccaacgccgcgatgcggctaactacgactgggaaaccaggcatgaggaagtaatggcctggaataaagcacaccagccgaaagtagtgttcatgggtaattccatcacgcatttctggggcggcaaccccgtcgccacagtacgccggggaaccagctcatgggataaatactttgagcctaaacaggccgtgaatatgggcttcggctgggaccgggtagaaaatgtattatggcgcgtacaacacggcgaactggatggtattactccccgctatattgtactgatgattggcaccaacaacctgcaggtaaacactgatgaagaaattgttggcggcattaagttcctgctgcaacaaatacaggccaaacaaggcagcactaaaatcatactgatgggcattctgcctcgtcgcaatatggaaagcagggtagtgcgcattaaccagctgatcgcaaaacacactgccggtaaaaacatacaatacgtagatgccggaaaactcttccttcaaccatccaggaaaattgacgagcaactatttaccgatggcctgcatcccaacgaaacaggctacgaaaaattaggcgccctgattaacagatatttaaaggtgggggacaattaacatttaacggcaagtaataaaaattggcagccggttattatttcctacattagatgaaatataaccggcatttaacagtggtctcatcagaataggaagagaagtcgacttaaatattttgcatgagtactcattataaccaggagccacattttattattgccataggcgcttccgcaggtggtttggaagagctacagtctttttttgaccatactccactggcacaagcttcttatgtgattatacagcacctttctgctgattataaaagccggatggcggaaatattgtcccggcacagtcagctgaaggtcacggaagcagccaataatatgctggtagaacctaaccaggtgtacctgatccccagccagcaatgcatgaccatacaggatggccgcttgttgctgaaagacaagaacagcagtccggctccccacaaaactatcaatacctttttcaactcactcgcattagacagcgaatatcagatcatagccgtcatactttccggctccggtgatgatggcagtgaaggaattgtgaatatcagcagggcgggaggattgattatagtgcaggatccggatactgcccagtatagcagtatgcctctggaggcaattgccaccggtgcggcagatcatatactggcccccgcagatatgccaatggtgatcacccaatatgtaaacaaggcgaagagaagtattttgccccctgttacgcaggtaatggaagataaaagtgtgatcgctattattgacctcatccgggagcgtttgccttttgacttttcagaatataagcccactaccattctgcggcgtatcagacggcgtatggtatatctcgctttagataaggtggaagcttattatcaacacctgctggcgcatccccgcgaagtggaaacattggcccagagctttatgatcagtgtatctgctttcttcaggaatccggaggcatttgaagtaatggctgaaacagtgctgccggaaattgtacaacgaaaaaagaacggggaagaaataaagatctggatagcaggatgtgccacaggggaagaagcctataccatggcgatcctgttacatgaagaggtagaaaaagccggtaaagatattcaggtaaaagtatttgccaccgatatagataagcctgcactggagttcgccggtaaaggtttgtatggagagcatatccggaatgagctgtcggcagaaagactggagaaatattttagccgcgaaggtaatggctaccgtatcaggcaacatatccgcagaatgctgatcttcgcacagcataatattgtaaagaatccgccctactgtaacatggacctgatcagttgccgcaatctgctcatttacatgaacatatccctgcagaagaaggcgctttcaatgctgcatttcgggcttggccagaaaggatacctgtttctcggttccagtgaaaatcctgggatgttactgtcctatctcacagaaattagtaagaaatggaaaatataccgtaaccaggaatcggccaggtctgtaaggttcgatatatttacacctgtgatgatagccgatagtaatatggcgcctttgattccatcaaaaaaaaccggtagtgccggtaagagaagcattatgttggacgaggtaaatgaaatgttgctggaagaagtaaatgttgcaggaatatgtgtggaccaggataaccaggtaattaaatatttgggcaaggtagagcacttcctgttgcagcaaatcttcagtttcgacctggtagagctgctgccaaaatcgcttggggtagtatatgtaacagccgcccggcaagccagaaaggacaatgagcgggtaattgtaagtggtatcccggtggcagattacaacccggtaaagattgttaaccttacgatctgtccgcttcacgcgagggaaggagaacgttccctcttgctggtgcttttcagcgaaagcaaggaagaacaaaagaaggaggtaccaccttttgatgtacaaacatatctcaatgcaggcctgcaaagcctggaagaagaattgaaagatacccgcgaacggttgcaggacgccacagagaagctggaagcctccaatgaaaatatgcagtcgtttaacgaagaactggtttctgccaacgaagaaatgcaaagtgccaatgaagaaatgcagtcggtaaatgaagagttgcaaacgattaacaccgactaccagctgaaaataaaagaactcattgtgctgaacgatgatatggataattatttcaggagtaacctcaacgggcaattgtttgtagacaatgacctgaagctgaaaaagttttctcctgccgccgtaaaacatatcaatcttcaggaaggtgatatcggcagacccatccagaatattaccgtcaattttaagaataattccctggaagatgatcttcgtatggtaattaaaaatggtacagtgctgtcgaaggtcgtggaatcactaaatggtaactggtaccagatgatgataatgccttatatccggcagctggaccagaaacaggatggcgccattgtttcgtttaacgatattaccctgctaaataaagcccagctggaattacatcgttccaacctgagcctgcaacgtatcaatgatgacctggataattttgtatacgctgcctcccatgatttgttaggaccacttacgaatatagaaggattgatgagattgttgagtgaaaaactggatatgcaggacaaggaaactgtcagatatacagatatgatccagtcttctattgtcaggtttaaagaaaacctgcgggagctggcggaggtagggaaaattgaaagcgaatcactcaaggaagtacaggaggttgatattaacgccatactggatgaagtactttttagtatacaggacaaagtacaggatgccagggccttaattacaaagaacctggaagaaagccatctggtgttttccaggaaaaacatccgtagcattatctacaatcttctcaccaatgcccttaaattcaggtcgccggaccggccgctgcaaattcaaatcaatacccgtaaggaaaacggattcctgttgctggaagtaaaagacaatggtatcgggatagaacaggataaactccagacagtcttcaatatgtataagcgcctgcatccggaaatggaaggattaggcatcggattgttccttgtccggaaaattgtggatgcttccggcggcatgacggaggtgaacagcaagttgcacgaaggaagcgtctttaaaatcttcttcaattctaaataagaaggtgatcggagcggattttgtcttactcaggattacgctgattatactgattacctggatttttacttttggatttttttagatttctttgattttttaataataattaagggagataagagcgaatatatccgcttatatctcccttacttctttataaaatctaaaaaatctaaaaaaaatccaaaagtaaaaatccaggtaatcagtataatcagcgtaatcctgagtaagacaaaattcgctctaatcacgcattctcactcttcccttcgagccagtttttgaattcagaaaccctttcacggctaataataacatcagtatcaacatcgggcgctaattgaagaattaacctgctattgtaataagtggtgatctttttaatggcatctatctggataataaactgccggttgatgcggaaaaactggtgcttgtccagcaactgttcaatctggtcaagggagtagtccagcggcacccgctgattggtgacggtggtggcccaggtggcgccccgtgcaaactgcagccaggcaatgtctttcgcttttacatagatcagctggttgttgatccggccgataaaacgggcgctgtcgcggcgcaggaattcttctgcaatcctgctgatgtctacggtatagttattggctggcctgaactgttcgtattttttcagcgcattctttaaatcgtcaaggtcgataggttttaacaggtaatcgatactgtttaccttaaaagcctgcaaggcaaagccatcatacgcggtggtgaaaatgataggcgtgcgtacttttgttttgctgaatatttcaaagcagttgccgtcggacagctggatatccatcagcatcaggtctaccggctgctgctgttccagccagcggatgccttcttccacggaagtaataacggcagcgatctctatcgcggcattacacttgtgcagcaactgggtaagccgctcggcattatgcatttcatcttcaaaaataacgattctcatgagccactgataatgggtaattttacaataaacatctctgctgtttcgctgatttcaatattgctgttgctgatcagcgcatatcttttctgaatattttcgagtcctataccggaagatatttccgggtgaacttttggccgcttgtgattggacacgaccaggaaatggccgtcacttttaatcgtgatcagcagtgggtcctgcgcggaaaaccggttatgcttgatggcgttttcgatcagcatctgcagggttaccgggggaatcatgcctttggtctttatcttgtcaggaatgtcagcgctaaactgtatgctttgctggtggcggatctggatcaggaaaagataggcgtcaagaaaatccagttctgtttgcaccggcaccaggttttcaaattttttatcaagaatataccggtaggtttttgccagctgcgtaatataatcagcggaaaggtccgcgcttttatataccaggttggtcagcacactgagcgaattaaaaaagaagtgcgggtctatctggttgcgcaatgcgtcatatctcgcctggatgttttcccgcatcagtctttctgtttgcagctggtattccttccagccggaatagtaaaagatgatgccgttaaatgccagtatcagcaggtaaaacataaacgtgccgaagttgaggtcgtagctgaaatgccggaagctatcccatgcttcatagcggttaaatagcaggatgtcggtcactgaatagaaaaagccaaacaggaaggctaccagcataccgtacaccacgaggaccgccgacaggaacaccagtttgccggaagtatgtttgttcgctgtttttctctctgtggtgcgggccagccaggtcgcgccttcccaggcaataagaccaaaaattacatagaacaggctgaacatctgccccctgtaatccagtatccgtaaacctttcacgaaggtatggtcaaaggatttgaagatgatgctgaaggtatacagtatcagtatcctggaaagatacaggaatagtttactggagaacaatttttcattttcctggaagttcatctgatgggttgtatagtactaaatgtagttattttccttaaaccacgtaaatgcgccagtaacagctgcttctacgggggtgtaactgagttgcagttcccgctctgatttcttgccggaatagtaattgtccaggcacagcatataagccgtggtataatttaattttccggagatgcctggcagggaacctatgatacccgctgctttcaggataaaggcaggtatcggaatgagcagctgccgcttaccggaaatctttttcaagagccggaagaattctgcatagctgaggttctgaccggccagcaggtagcagtcgcccgttttgcctttttcaatagcgttgataataccgcggcatacatctttgatatgcacaaagtttttgcctcccggcggatagaacagcagccggtgttttagtccgtacaggatcagtttaccggagctgggcttcacatcatgcggccctatcataaaggtggggtttaccacgatgcccgggagttgcctgctggccacctgttcaagcacgtattgctgcgcgaggtacttggtgttgatgtagccggagttggcgttgaacagggtaaagccattcagttcgttacccggactgtttttatcgcccggcccgatagtgttggcggtgctgacataaatgaatttctgtacccggtgctcgaggcaggccgcggtaatatacctggtggcggtaaagttggtatgttcatattcggcaaacgaaacgccccattgtgcggtaatacaggcggcatggatcacaatgtcacagcccttcacggcttcatgtacatcgtcgttgttgctgatactcccgtaaaagatttcacagggaatgtcctcgatgcctttcatatcggccgaaggccggattaaaatttttatgtcaaaccccatgcgatatagttcccgtgttaaattggaacccaggaagccgttggcgccggtgatcagtacttttttcatgaattttttttagacagataaactataggggatctcttttttcacttccctggatacgatcctcatcctgaaggagagtggcagcaactgcatcagtatgtgattgagcttattcatccagccgggtatgatcaccgggtgcccggcaagcgttcctctcagcgcaatgtctgcaatgtcgggtgtagacaacaggcccatctttcctttcaatccctggctgatgatccgccgcgacgtgtgcgagttggtcataatagggccggggtatactacgctcacggatacactggtatctgccagttcttcttttagtccaagaaagaaagacgagataaacgctttggacgccgggtataccgttttataggcaatgggcgtgaaagccgccatgctggcaatgttcataatatagctctgcggatgcttcagcaggtgcgggatcagcaggtgggtaagtaaaacggtgcttcttacattgagcatcataatttcgtctatccgttccagtgaggtatgggtgatggaagaggtaccaccgatgcccgcattattaatgaggaaattaatgggatagtcgcggataataagctgcagttgctgcttcagtacatcgctgtcggacaggtcaaattcaaacacttttacgcagatgcggtattccagttccaggttctccgccatggattgaaggcggctgcccggcagggcaatgagaatgatgttcatgcctttcctggcgcattgaatggcgaattctttgcccaaaccggagctggcgccggtgatgagcgtgtatttattgtctggcatatgttttattttcaagcaggcttttaaattttgtcattgttttgaacaggttatcatgaatgatgggatcggatacccagcggggaattttcctgctacggtcggtggtgaccatataagtgatccgcagctgcccgttccccgaaggcgccatgatccattttccccgcgtgccggtaatccgtgttgttttattgtatagagggaagcgatgatccgtgatactttcaaacaccacttctgcagcgtcgtcggaaatttcctggtagcggtataacaggcagcagtcctggtcgtcgaccggccagggaatatcatatttaatataagtaatccagtggcggggatctggcgccgccgcgatcctgtattcgctggcattggtattccagtcgcggccatgcgcctggtccttgaacagcccgatcaccgccggtacggcgcatttcaccaggaagacggctttgatctcccttacattttcaccatctgcgccgggtatccacctttcatacagcgaaatggcgttatcctgttttaccagcttaaattcactggtatcaccaaataatgaccggacgaacatcatactgctgatcactaaaacggagagctgttgcatacatcatcatttacagcaaatatgccactggtaaatggactggccattgattacctgctgaactgtaggattaagctgttgacctgtcactaaaccggggatctgaataatggagaaatatttatatattattttatggagaagtactggtgatattttattattttggctgccggtgccctggttaagacagggccacgcctaaaaatcagctttgaacatgaaaaaatacctgctggccatcgccattgtattaactgctattcccgttgccgcacagcaaatctgcccggtgattccattgccggtaaaagcagacaaaggtcgcggcacatttgaaatcagcgcacaatccgttattagctgggaagacacttccctggttcagctgggcacctggctgcagcaggaactgcttcgccgttatcatatccaggtaccgttgcaacggaaatcaggcagcaccgttatcctgctgaaaaaaataaccggtactaacatggatgcatatacgcttaccatgaataagcaaacggctactatctcggcaggcgcacgggaaggggtgtttaatggcatcatcagcctgttgcagctcactgcacaggcgccggcaccggggaaagtgttacaggtgccttgctggaacatcacggatgctccgcaatacgcctggcgcggcgtaatgctggatgagtcgcggtatttttttggtaaagagaaggtgaagtcaatgctcgactggatggctttttataaactgaaccgctttcactggcatttgactgacatgcccggatggcggctggaaattaaaaagtatcctttgctcaccaccgttggcggtatcagcaacatcgccgaccccaaagcaccggcagcctattacacgcaagatgatatccgggaaatagtggcctatgccaaagcgcgttgcatcgatattattccggaaatagatatgccggggcatgccggcgccgccaacagggcttaccctgcattcgacggcggcggtactgcaaagtacccgcagttcaccttcaaccccggcagggaaggcacttactcgtacctggcggatatactaacggaaacggctcaactgtttcccgcgcagctcattcacctcggcggcgacgaagttacctttggcaatgcgggctgggaccaggataccggcatcatccggttaaagcaggcccacggcctgaaagaccgcaaacaggtagaggactattttattcaacgcatggccgacaccgttttgcagctgcataataaagtaatggcctgggatgaaatagccacggcgtccctgccggccgacagcaccatcgtatgctggtggcgccatgataaaccggaaaacctggccatggcatttcagaaaggatactccgtagtgttatgcccgcggctgccgttttatttcgactttgtacaggacagcacccacaaaatcgggcgccggtggaaagatggtgaattcaatcccttggaagcagtgtataatttctctgccgccgccattccggccacacaggggcatgaatccctcatactcggtgtgcaggcctgcctgtggtcagaaaccattcacagcaacaaccggctcgatttcctgcttttcccccgcattgcggcgctggcggaaactgcctggacgtcaacccaggcaaaggactttaatggctttaaaacccgtttaaaagcgcagttgccgctatatgcaaaggagcatctttattactttgatatcttccagccgggcaggcaccaggagtcgggtaaagcggccgccaactatatcgactgatgtgtcggttttgttctatttccggaaagggaagggaggtaatattgcaatgggattaaaaatacccggaacatcatgaagaattttgtactggcgcttgccactatcaccacggccctggtagcgggtttgttctatgcgtttgctgtttccgttaatgtagcttttgcgcaattaccggatgccgcttatataacggctacccaggccatcaacgttgccattgtgaaccctgccttcctggtatgttttttaggcgcaccggtgttattgccgctggccacctggctcagcgcccgaccggtttttacccgccgcagctggtacctgctggctgggaccgtggtatttgtggttggctcatttggggttacgataatcgccaatattccgctcaatgacaagctggcggccttccaggtaaacggggcttcggcggagcaactgcacagcatgcgggtggcatttgccacgccgtggaataactggcacactgtgcgcaccctggcaggcattatggccctggcattgctggtaatggcctgtttgcaacgcgataccaaaagcgaatcacgtaaagcttaaatgctttttgtaaatttaggatcatgcgttaccagacaattccaccaccgcctcatcttgcgcacgtcatccggttcttctgggtgctggaaggagaggtgggttacacgcattacaatatggcggatgcctgcgtagagctggtgtttcattatcatgggctgttcggcgaaatagcagataacggccatacagatacatcgtttaccgccggtgtgcagggcgttacacacaccctcaggaagtatactgttgatacaggcttcggtatttttggcgtatatttttacccacaggcagttccattgttgtttaatatttccgcggccgatctgaccaatactgccgccgaattaaggtacctgctgaaaggcgaaggcaccatcctcgaagaaaaaatcatgctggcgaaaaataaccgggagcgttgtgagattctctgccggtttacggagcagcggctggcagccagccgtgtggcggatttgccggtgtttgcggcgatcagggacatcattcatcacaaaccctccatgaatatacggtccctttcacaggcatactatttgtcggaacggcagtttgagcggcagttcaaacagtatgcaggactatcccctaaattgttttcacggattgtccgtttccagtcggctaccgccttttataaccggcaggtaatgagcctgggacgcctggcactggagtgcgggtattatgatcagtcgcattttatcagcgacttccgcgcattttcaggtatgcatcccaaacagtatttctctggccgctccggggccaccgactggcgcgactaacaagaatgtcggtttcttccaattttatcagggcatactgttgcaattttgtgcaagagacgtttaacctaaaaataaaaatgttatgaaattaccagaaaaacatcagcaggtaatgccctatctgatcctgaaaaatgcagaaggctttttcgattttaccagcaaagtatttggggcaaaagaaaaccaccggacctaccgggaaggcagcaaagagctgatgcatggcgaaatcagcatcggcggcagcgtcattatgtttggccagtcaaatgacaattggggcgccgacaacgcaggactattcatttacgtggaagatgccgacgccacttttaaaaaggccctggccgaaggcgctacagaagtaatgcccgtaacacaacaatcctacggcaagtccggcggcgtaagagatccgtttggaaatacgtggtggattacaacaccttaacgcggaggttgtcttactcaggattacgctgattttaatgattagcttgatttttactcttggattttttttagatttttagatttttttaaaataataattaagggagataaaagcgaatatatccgcttctatctcccttaatcctttataaaatccaaaaagtaaaaatcaagctaatcattaaaatcagcgtaatcctgagtaagacaaaattcgcgctattcccaatacttctcgcctttcttcattttctccagcgtggtctcgtagtttttcttttcgtcgccactggctttgttcagggctttttcttcccatgcgagggcatcgtcttttttaccggatttatacagcaggttggcgtaagtgtccatgaatgcaggtacttcgttgtctttgaaagagcgtttgctccattccagcgcctgttctatgcattgcatgtcgttgcatttttcgaagatggtccaagcatattcattcaatgcctgcggatctgctttgtggccatattttttcatataggcaacaatgttagccactgcgttatcggcatcttttacgtagctgaagtactgtacttttgttttcaggagcagttcttccgcgaaagcaggatattttttggtcaggccgctttcaagggtagcccagtcgggtttgctgccgtctttcttcatcagctccggatatacttcttcctgtgccacaatgcccattactttttcttcggccttaccggtgcccagtactttatttactttatcggcatggtgcaggaacatatcaaatcctacatctttactgctgttggtaaatttggcgatgaactggaggtttacaggtgtgtaaagatctttttgcttggcaagatattctttggaaataagagacgcattttcctggtcatatttattcagagccagcagtgccatttcgcggaggaaagcagtatccttttttccttttttataaaggtccagctgtgtgtaatactgtgtggccgggttcagggaagcagcgcatctttcaatgaactggtctgcttcggcgccgcctatctggcggtcaacgatatggccgtcgggtgcaaacaccaggaaggtaggataggcacggatggcatagtccttttcaatttgtttggcggcagcgtaccagcttttcacttcttcattgtctttgtccgtttggtccatctgcacctttacgctgatatatttatcattcataaagctgcctactttttcctgcgggaaaatattggccgacataaacttgcagggaccacaccaggtagtgaagcagtccataaagatgtatttgttttcagctttggctttggcctgcacatcggcccagctgctgccatgctcgaaatgaatgcctttgtcctgcgctgccgccagcaatggcaacaggaaggcgaggaggagtaattttttcataatgctgtttgttggttttgattagtaggctctaatttaatgcagttcaggaacaaaaccgggagggatgccaattaatttaacaggataagttggtgtaacggcgcgtttgcacaaaaaaagccatccggtgggacggccttttttgtgcaattagtacttaacctggtggatgttatttgagggaaaaaagatggtttccgtccacgaaaacccaatatggtgaacattcggcatccaattgcaaaatttcgtatttatctttagcacattcgtacctgtttttctgagttcggttaaattatactaacttgttgtagctaaaaacattagccatgccggtaaaacattttgtacagccgatagaccttacacatccgaagcaactacaacgcctggtggagaacaggcgggtctataacctgaatagctgtgaactgaatatatttgaaagttatcagcaggattaccgggtgccccttactttcggagatttcgttattaccagcatggtgcagggaaaaaagatcatgcatcttttcgatcagccctcctttgaataccagcccggggaaaccgtgattgtaccggccaacgaaaccatggtgattgacttccccgaagcctctgcagaaaacccgacacagtgtattgcgctgtcggtcgatgaaacttatatccgcagcaccctgcaatatctcaatgaatactataacagccagtatgccgataaaaacgactggcggctgcaattcaaccagtaccactttaataatgatgcagatctcacagacctgatcaataagttagtccgcatctgccgcagcaccgatctttccagggatatttacgccgatctcagtataaaggaactgctggtccgcatcctgcaaagccagcacctgcagctggtggcagaggaaaaagataccaacagcaacagcagcaggcttcattttgtgctgcattacatcaatgagcaccttactgaaaatatttcagtagatacgctttgccggaaggcttacctgagccgcaatgtcttcttcaaatggtttaaagaccagtttggcattacccccctccagtatattaaccgggaaaggttaaagctggcaaagcaactgctggcggaccgcaacaacagcgtgggccaggtgagtatgctttgcggttttaatgataccaactatttcatccgccttttcaggagcgcggaaggaattacccccggtacctaccagctgatctgctcccgctgatattttctttttagaaagatacctttcccttcctgaccaggacgaaaccttatgcgtctaccagcggataaataaatgcgagggaaacaattcccccgctaaaaactaataaaaaacaggcggtggattcagcgtgaggttttgctgctgatgccagtaaggataaatggtaggtatatcactcgcggcatccagctttttaagctgatcggtagtgaggttccaacctgtagcgccgaggttttgtatcagctgttcttcattgcgggcgccaataatgatgctggacaccgtggggcgttgcagcagccagttcagggagatctgcgccaccgttttgccggtttcagctgctatttcatccaatgcatcgatgatgttgtaaaaaacttcttcctttaccacggcctccggtacagggctgcctccctgcgctacgcggccgttttgtggcggcggactgttacgacggtatttacctcccagcctgcctgccgccagcggcgaccatacaatggcgcccacttgctggtccaggcccagtggcattagctcccattcatattcgcggttggccagtgaataatatacctggtgggccacgtaacggttccacccatatttttccgcgatggcctgcgatttcatcaggtgccagccggaaaagttggaggcggcgatataacgcaccttgccgctttgcacgagatcatccagcgtacgcatggtttcttccacgggcgtgttgccgtcgaacccatgcatgtgataaatatcgatatagtcggtttgcagccgcttcaaacttccttctatctgccgcagcaggtgaaaccgcgaagaaccctggttattgggaccctttccgaaagggaaagtggctttggtggagatcagcaactgctcccgcttgccggcaatggcttttccgagaatttcttccgaaagaccgtcagaataaatgtcggcagtgtcgaagaggtttacgcctgcatcaagacaaagattcaccatgcgcgtggcttcatccgccagtgtgctgccccaggctttaaagaaatcattaccgccgccaaaagtggcagtaccgaaactcagcaccggtacctgtaaaccggatgcgcctaattgtctgtattccatcagctaaattttatgaccgtttgttataaaaatataaagatcggggaaaagccgcaggctttatttgtattttcatcagtattttctatatttgcgtaactgattacgtaatttattacaatatggaattcttcaataaaacaggcaaggtagcgctcggaagcaggctgcgcatgctcacagaaaagatcacagaagatgccgcaaagatttaccagttgtataacatcgacatgcaaccgaagtggttcccggtattttatgtattatctgtaggagaggagaaaacaattacagccgtcgcaaaagaaattggtcattcccatccctcggtaagtaaaattatcggtgaaatggggaagaaaggactggtagtagagaaaaaagacaaaacagatggccgtcgtaatatcgtcagtctcactaaaaaaggactggacatcaccctcaaaatacaggaccagctcacagacgtgaacaccgctatagaagccatttctgcccaaaccacacacgacctgtggaaagcaatggaagaatgggaatacctgctggaacagcagtcgctgctcagccgtgtagtggaagcacataaaaaaagagaagcaggtaaagtaaccatcgtggattaccagcccaagtataaagcggcctttaaagcattgaatgaggaatggatctccaggtggtttaaactggaagcagcagaccataaatcactcgatcacccggaagaaaatattctcaaaaagaacggccatattttcgttgcgctttacaacgatgaaccggtaggggtttgtgcattaataaaaatggacgacccggactatgattacgaattggctaaaatggcggtatctcccaaagcccagggaaaaagtattgggtttttgttgggacaggctatcatcgcaaaagcaatatcactcggggcccggaatatttacctcgaaagcaataccatcctgaaaccggctatcagcctgtataataagctgggatttaaaaagatagccggcagggcaacgccatacgagcgttgcaatatccagatggagctgatattacccgcctgatttaaccggcagaggattggagtttataaaaatggaaatgtatattagagcttcggatgcatgctcaaaccatcattccacgttataaataaaatttaaaaactctgatcatgatatcacctgactccctggaacaggaagccttagaaaccactaaaaataccgcgtccacacccgcaaaattcacagagaataaatatgtcatcaccctcatattcgtgacttccctgttcatgtgctgggggattgcattaacaatgggcgatgtactgaataaacatttccagaatgtacttggattatccaaatcccaatccggcctggtacagttttctatcttcggcgcctacgcgctgatgggcatcccggcagggttgtttattaaaaagatgggatataaaaacggcgtgttactggggctcaccctgtatgccctgggtgcctttctctttgtgcctgcagccaatgccgcctcgtttggtattttccgcatcgccctttttgtactggcctgcgggatggctacactggaaacagtggcgcaccctttcatggctgctttgggagaccagcgcaccagtgatcagcgtatcaattttgcacagtcgtttaatgcggtaggcgccatagtaggaccaacgcttggttcctacttcctcctcagcgcaggccacgatgcaggcagcgaattgctgtctgtaaaacaattatacatttatatcggggcagtgatcgcagccatcgctattgcatttgccatggtaaaagtaccggcgctcaccgatccgcacgatggcccttcaaatgcaggtggcgtggctggtgtccgcaaaaaattattccagcagaaacattttgtgttcgccgtggtggcacagttttttaacgtagccgcacaggcaggtacctgggccttcttcatcaactacggacatgaagtgatgggcttctctgatcagaaagcgggttactttatgacggtgtttatgggtatgatgctggccggaaggtttgttggcacggcactgatgcgttacatcgcgcccaataaactgctcgctgctttcgcactcggcaacatcctcatgtgtatcctggtggcgcagggctggggctggacctccttcatcgccttgctgatgatcaacttcttcttcagcatcatgtatcctactattttcagtcttggtttaaaagacctgggcccgcaaacacaacaggcttcttctttcatcgtaatgggaatgtttggcggcgccatattcccttttatcatgggacgtattgcagatacgaatatcgctactgcctactacctgcccatcgtatgctacgtggttattttcctgtttggatataaattatataagctcaggtaacggatatccgttaccgttatacattacccgggctgctggttattcagcagcccttctttttgcccgcaagtgcgattattgttctgctttcatataatcaaacgctccttttctcaggttaatattatactcgaggtaagccttcaaacaggcaagaaaattagcccagccttccgtattgcctttcagccatttaattccttcttcattattttccatactgccttcagtaacctttaccagggtggtatgcccaaatctttcggaaaacaggatgtccacctgcagctgatgatctttgaccccttcccactggaaggagatgagcgcgtcctttttcacctgcaatacacttacaggaacaaccgtatcaaactccgggaatttccagatcacctgctttccttcttccatgggacctgagccggtggcgataaaatagttggacattttcagcgggtcaataacagcatcaaaaacttcggagatgggtttagagatctgtattgttgcgttggtttgtaatggtgccataagctgcggttttgagtgaagaaatggataataaagttacaaaaaagaggccatccgggccgggttgcggcgttgcagcccgctacggtagccggttgctgagatagcctgtaatgcgcctccctcccttgtactgcattgccccctttgccgtggcctcatcccaaaatccaatccacgcaaatgggtgctttttcgtaatattagtttgtccaatttagctttttggaccaatcttcaacgtcaggtaacatcataatataattccgggctttgtctgtagaacatggtaatatttgcaaactggttgttgtatccgcactgaataaccattactacgcttaaatattagatcatcaatcttttattcactttaaaaattaacatttatgtcaaatgctttaacttcctgcgtcactatcccgggaaagtctaagattaattcctgttttcaggatgttcagaatgataccttgaagtgggtacagcaatttgatattgccccaaaatttaaaccccttagttggtactccaaagcccgtttcgggttccaggcagccagggaataccctgatgccacctatgcccaggtaagtctcgccggagatttgctgtcctggctcttcacagtagacgacagctgcgaccgcggctctgccgacgcagcaactgcattggaaatgagacgtcagctggaaatattcatcgctatccttaatgatgaatatattgaggacgataatagtcttagtatggccctgaaagatatcctgcatcgtttcagcgacatcagcagccccttcttataccgcagatactgcatgcacatgaccgactatctcaatgaatgtttctttgagatcgatatgcagatagatggactcatgccgtccatcgaccggtattataaagaacggccctacacaggattctatatcatgtttccattggtagccatttttgaaaaactgaacctgccggatgaagtatatgatcacagtattatccgcgaaatagaactcatcttaaatctgctcggttgcctttccaatgatttacattcgattgtccgtgaagcaaaactggagaagccggggtttaacctcatctttatcgcccaaaaggaactggacctgggcagggacgaagcggtgcaatatgtaatcaatgaacataaagcgcacctgctccggtttgaacaactccgtgcgcaacttccctattggggcagggccgttaatgagcaggtagaccgctacatacagggcttatataccatcgtaagaggttacgacgactgggccgtgattgataccggccgctatgaaaatatatgatgaggcaaatactttgctaattcgagatgtaggtcgctgatgaaaaccggtttcgttatgaaaccgcaggcgcctgtcgctaacatctcatctttcaaaaaggcatctcctgaaatgatcagtacggggatgccttttaattcaggatcattttttatgtactgcaacaagtccctgccatcaaagcctggcatattcagatcagaaataaccaggttgggcttttctgtatggataacagcagtcacagacgcatgatccttacataacaccgggtctattcccatttccttcaggaatttgatcagcaattcagcgctcagcaggtcatcttcaatgatcaccactttcccgcctataaagcagccattcataaatttaggaggtagctgttgcctggtttttcccacgcctgcttcataagggatattgaaggtaatggtagtggtaaaaggagaggagggatcaataggggccagcgcaatttgtccgccgaaaagactgatcaggtgcttggtaatagacaggcccaacccggtgccttcaaactgttcgcgttttgatacaaacctgtcgaacattttgccggcaatgtccggatctaccaccccctggttggttaccttaaaaatgatctggtccgcatctttcgtacaactcagatggatcagggagttaccgctggcaaacttcaccgcattcgaaaggatattattcaggatcttggttaataaaagagggtcgctgttaatgggctcacccagctgcctgtcgaacgccatctcaatttttatccccctggatgctgccaggtagctattcaccgctatacaatgggatatacagtcttttaaactgatggcctccttcataacggaataaaaatttcccgattcaatcctcgacatttccagcacatgattaatgacattgcgggccaggtaacaggaggcaaacaattggttaatttcctttctttcggccatagaatatttggacttccgcagttcaaacaactggccgatagagaaaatggcattcatcggcgtacggatctcgtgaaatacctcccgtaaaaaaatgcttttcctttcagatgcctcccggagttgctgtgcagaagcaatcaaactcctgatctgcgccacataagacatcataacgcataatataaataccagcagcgccacggtggtcgaccacttcatggttaatgatacgtcaggcgaaagctgtatcggctggatgaagttataatgggaattggccaccatccacgcggcaaataccaccgttgcggctatacagcccagcagcgccccgcttcttttgtacaggaaaaaggcagaacttaaatggaatataatgatggtattgaatgccagcagtagctccagggaaatacttgaccccagtacggtagaccagtaagcaataaagatagcattggtactcagcatgagtaagttggcattaaaatattgccggacctggtttaaccggataactgccagaaagctaagcgtctccagcggaatcccgattaaaaagaacaccgaattcttaagaaaataaaaataactgccaaccccgacaaccagcgcgcttaacacaatggccatcgcgttgatgataataacaggacgtttttcttccgctttatcaaaatgctgggttccggcaaaaacaggtttgatgagtgtggctgtaatggtagcagctgtaggatagataccagttctcatgtatagttatttagaggattaggcagtagatttctttgggttaaggtaaatctagccagatatgcatcggaatgagttaattgaatgttaatataagcatatttttttttgaaaaaaagaatatcacgttatataaagtgaaaatatgtttggtccgggcctggtaagatatataaaccctaaaacctggaaagccttccgctaaaacatttttacagacttttgtcgtagtgtattcgctcatccttgccggctgacccgcgtactatactcaatatctgaatgtcaaccatttatccattttgatgcccttatcccggtaaaacccggcgggttccgtatgcagattcttttcacttaataaacattaaaaaacatggaaacacacaccctctacattcctgccctggaatttccaaccccttctgccataagcccgcttgcagaagatgtacaggtacacacttataaatgggcccatgaattccgcctggagtcgcccgaaaagctcaaacggtttaacaaaggtaaattcggctggtatgccgcccgggagtatcccgctgcaaactatgaagaactatgcctggtaggcgatctgatcacctggctgtttaccatcgacgacaaatgcgaccgcttttcttctggcaccctggaaggcgcctggctgcgcagcatgttgaacggctttatcgctattatggaacaccgggaaagcacggtagaaacacccctgaatgatgcgctcatcaacatccgcacccgcttccaacatctcagcccgccatttctctattccttgttctgcaaagagatggtgtcctattttgaagaatgcctgtgggaaacagaaatgcaggaaggagaatatagccccagtatccgggaatatctccagtggagacccaaaaccggcttctatattatgttcccactggtaagcatcttcggtaaaattgatttgccggaagaagtatatgaacactggctggtaaaaaaaatagagctgctgctgaacctcaccgccaacctggccaacgaccttcactccctggaacgggaaagggaactgaaaacgaagggactgaacctcgtactgatctatgaacaggagctgaatatttccctggaagaagccattcagcagatctcggatgaataccaccgcaatttgcttacactggaggagcaccgcgccagcttgcctttctggagcggggagatcaatgcgcagctggatgtgtacatcgacggattgtacatcgctatcaaggcttatttcgactgggcgctcatcgataccgaacgatacaaaggtaaagtttaggcttttacagatttagccgggagatgcttcatcatttcagcatacaggtcctcaaaagaaaagggcttattaaagaaagcgttcgcgcctgcctttaaaagctcctcggattcattactgtacttgttgaaagcatctcccgatataacgataaacggtgtatcagcaaacgaaggaatggcccgcaactgcagcaggaattcccggccattcatcaccggcatctgcgagtcagtgataatgatgtccggcttttccgccagtgtagcttccagcgcctcttgcccgttgctgcataacaacgcccttgcacctcctctggtcacaaatttttcgattacataccggttcatctcgttgtcatccacaatcaacaccttcatcccctcaaattcgtctttgctgatgtcaaatttcttttcgatggccgcctccggatgcgcagcgcggaagggaataaaaaactcgaagatggtatgatgatcttcactgaacacccggatactaccctccagtaaagtgatcagctgctgtgtcaggtgcaggccaatgccggttcccgatgtaatgtggttccgctccgactcataaggaagaaacaatttttcctgccgctcaggagatatctccccttcatttttaacacggaaacaaatctggtgatcatcccggaaaacgctgatcaccacctgcccgccgggggaagaaaatttcacggcattggaagtcaggttattgatgattttaatcagcacgatttcatcactctctataaattgctgcggtaactggtagtttaatacaatacggacattctgcagggcgccggtatactggttcattgccatacactgctcaatacaatcccgcaggtgaacagcccccagcttgatttcaaaaaatttgccggcctcgatccgtttcagatccagtacattgtttacaatgtcccgcgatagctgtcccgcacccagtaaattcttcaggtccggtcctatttcctccatgatgggcgcctgcttattttccttccgcaccatatccagcaactgtgcaataccgtaaatgctgttcagcggcgttttcagctcgtgaaatgtttcccgtaggaaagcagcatttgttgccagcactttgttcgatttgctgagatcctccatcagccggatgatctccttcataaactcgaagatgacaaacaaaatgaaagtaatcataccaccggtggtacaaagccgcataatataagcagaagtaggatggaggtctatcggtttaatgaatccaaaaaaggtattcacctgggttaccaccagcaacactacaattgccagcaataaacctattcttgccttgtgacgcttatataccaggaaagaaccgcaaataaggaagatcagtaaaaaaacaatcaccacttcaatcgggatggcattgcctaataaaattgtccagtaacccgccgctatgtaatggatggcaaacatgctgaagttggcgctgtcccttttacccataccgtttaatacaataaccgcaagcattccgataccctccagcaatagcggcagcaggatcagtaaactgtggaccagcaggtaaaagactcctccaagtataaaaacaagcatactggttagaaatgccagggaattaataatgaggatggtacgcttttctggctccgtggaatattgggtgccagcgtttttaataatattcaaaatatgcatgcgtcatttttgagggtagtaggcgtagaaaaggtgttcattctggtgtgtcttccgtggtaaattcaaaccaatatacgaattactggtaacatacgtgaaagacgcggtatagcaggggatatcctgtggcgcccctgggtcagattgtggcggaaaacccgttttatccctctaaaaagcgctggtgcaaaagttgtatgggaaaagaagagaaaccaaacagtccgatgttatgaaagcgcttaccgacaaaaaacctaaaaccaatttctttgaaacaatggccacaaaggtcatcgccgccaccggtagcccctgggccttttttatagccctgggagtgatcattatatgggcagtcagcgggcccgtattcggctactccgatacctggcagctcgttatcaataccggtaccaccatcattactttcctgatggtatttattatccagaagtcgcagaataaagacgccaaatcagttcagctgaaactcaatgaactcattgcagccaacaaggcagccagtaaccggctgattgacgtggaaaatttatcggaagaagaactggacgtgctgcacaaatactattgcgtgatggtggaagaaacgaggaaaagaatgagcatgacagaatcccactcggtggaagaagcgatcggagatgcattgagcaaacatgaggaagacctcctgacccggaaaaccaccaaaaagaaagcgccgcggaaataaaatgacaggtgttttggtgttattcttgatggccttcataaaaaaaaacttatgcaccatgtcgctgaaaaactgagaatatttacctggcatgtacacggcagctacctgtactacctgtcccagggcaactacgaactgtatattcctgtaaaggaaaacaaagaggaagggtattatggccggggagccacttttcccttcggcaataatgtacacgaaattcctttcgatgaagtaaaacattacacgttcgattgtatcctgttccagtcggaaaagaattacctcactgatcagtttgatgtgttatccgctacgcagcagcggctgccgcgtatttacctggaacacaacacgccctcgctccaccccgtgaaccagtcgcacgtagtggatgacccgatggtgctgctggtacacgtcacgcatttcaataaactgatgtggaataataatcgtacacccgttaccgttatctcgcacggggttacggattctccttatccttattgcggcgatcttccttgcggactggtaaccattaatcacctccggcaacgcggccgcaccctcggatgggatatttacgaccaggtaagcaggctggtgccgctggacctcgccggcatgggtaaccaggaaggggtgggagaagtgctgcaccccgatctgcctgctttccggagcaggtaccggttctattttcacccggtaagacacaccagtttagcgctggcagtttgtgaagccatgatgcagggaatgccggtggtagcgctggctaccacggaactggtaacggttattaaagatggtgaaaatggttatatccatacagatgtgaactacctcactgaaaaaatgcaactcctgttaaacgatcccgaacatgcgatgcggctgggagcgcgcgcaaaggaaacggccaatgcactgtttaacatcacccgcttcacaacagaatgggagcaggtgttccggcaggttaccggcgtggcgtggcaacctgaaagccttttttccgccacgcctgcactggacggacactaagcccggtgatacacccggtcatctgtacgcgccagcagctgatctgcttttatcagcatccggtcaaaatcattgtgccgtgtccagtcggtggtgcaatgaagatgcgtattcaacggcgcccagcgatgcggttcgccatccatgctgatgatcacgctgggagtcgccgtggcggctgcaatatgagatacgccggtgcagttggataccagcgccctcgatttttttatcagcaccgccatgcctcctaaactcagttccccggcggtatccactgcaggaaaccgcatataactttttacggccagcgtcaattcccgctcctcattactgccagtgagcactattttccaaccctgttctgccaggtgatcggcaatggcggcaaaataaggcggaggccactgccgccacgctgcccgtgagccgggatgcacacaaatatattggtagtcctcgcacggcaattgcaggctccggaacgaatcgcggtcggcggtagtcagcggaaattcaagatgagtgcctgccgccggtatacccagctgcttcagcaggtagaggtgccgctcaatttcatgaaggtcctccgggtacggaacaaacattccgctttcaggaacagtaccttttggtgaaaaaccaccggtgtatttcgcttccatagccaacaccagcgggttcaccagcgtgccgttaccctgcatctgtagtaccaggtcatacgatcgcttcctcataagattcataaactcgctgaaagcgaccgggtcatgcggttgctccggcaacccggggtaaccgggaaacaccaccatctcatctatatagtgagagaaccgctgccggaaagtgctggcccacggtaagcctatcagcgtgatatgtgcgttggggaacgtcgccctgagcgcacggaaagccggtactgcacataaaagatcgcccagctgtaaggcccttaaaatagcgatgcgttgaatatggctggttatcatgacgtaaaaattagctgtaacaattgttggacgctgctgcgctcaagatcttgtatcaatgccgtaatccgctcaccggtgctttcagatatccgcccctgcgtaagccttttgaacttttcctttggatcgtcccaggtgaaaggtgttgtgtaaaatcctttgtatgcttctttttccgctttaaatattgtaccatctttcatacggatggctacactacttttcagcttatcaggataggcggctgtgtaaggatccagcaaacccgccactttcaccggtttatgcaaaggaaatgcagtatgggtggttacattttgcaataattgctgtacgtccgtccgggtgatccgttcaggcgaaaattgttccggcgttacttcaccatccagcagggccacggcaattacataagccatactgtgatctgcctgttctttggtatgtaccagcgtacggttgccatactcgccgccaccaacaatatgatacgccgtaagaaaagtggttacttccacgtgccggatgtccgccgggttgatccggtgctgttcccttaattccacagctgcggctatagcagattgggtatgtacttccgcattgtaggttttcaggcagcagcgcggaatcagctcaaattgatctttggaccagtcatactccagcttcatcccgtaaatagcattgaatcctttttcgggaatctcaaacaattgcaccggtccggtaatatcttcctgtgccagcacacatatgttcatacaaccttcattaacaagagaagaagccagccctttccattgggtagtataagaggcacgcgaggtcaccaatggatgatagctgcagccggcaatgcctaaagcattcatcatttgtggcaccggcatttccagcagcttcgcaattcccgcggtggcggaaaacgccagcagcgtggtatggtcatgcccgctgatcattaccggcagctgctcagtaagccggcattccatttcataggctaaagccatggcagcgaggaagtcggcgccgctaatctctttcacatgggaggcggctaacaaggcgccaatattatcactggggtgacaggtagattccttggacaggaagttatccataaaatcaggatacctgatcagcgtggtgtaatactgcgcagcgaggttcggaggcagttgtaacgggaagtcggccgcttgtataccggataacctgccgagtccctgcgctactttttgtggaagatcttcccgggtggagaatataaaagaagccatgctgtcgagtaaatgtatcttcagctgttttgtgatcgccgcgggcaaggaattgaatcggatgctgtccgcgtattccgccatcattttgatctggttgctcatacaactttttaatggatgctgacgaccagaaacatgccagttgtactggtgcaatacttgtggttacttcacaaatcttttgttatgatacagcatctaaatgccactgtaaatggtcattcgtattcgctggacatccagccggatacttacaacggtcattccgtgtactacttactaaacgataacctgggtgaactgtttcatcatgctgtgcctgataacctcatgctgatggaaaacggcgacggctttacctgttctccccggcttacggaaatggaaggcgggtacattgttcagcagatatgggaggccataaaacagaacaacaaatcgtagcaaaaaaaatggatgcttaaatatgcatccattttttttgataaccgttttgaaacgttgtagagattaatgcttgttgtgtgaattttattctatcccggaaacgccccaatgcccgctcttgctatgttctacgccagcaggctatttttctttgaagcgctttacaaaacaggcgtttgaatcaggctcaggaaatccgcttatcatgccgctgaaaacgctaacctgttcactttatccggttggtgctattattgattttttgaaagtagcattcaactaattccttgataaaatctaatagtatgaaaaggatagcatttatcagcgagcatgcttctcctctggccatattgggcggagtagatgcaggcggacaaaacgtgtacgtagcggaactggcaagacagcttacacagaaaggctatgcggtagatattttcacccgcagggaaaaccgcgattatccccgctgtttacaatggcggcaggggatcaggatcattcatgtagatgcaggtccgccggaagtgatcgaaaaggaaaagctgctgccatatatggctgctttcagagaggacatgctgagatttatgaaggaagaagaaatcgactaccagcttattcacgccaatttctttatgtctgccctcgtagcaatggaaataaaaggtttattacgtattccttatgtagttactttccatgccttaggtcatatccggcaactattccagggagaaaacgaccggttcccgccggaacggctggcgatagaagaacaagccatgctgatggcagatggtattgtggcggaatgtccgcaggaccgggaagatctgctcaaatactacgatgcaccggcagataagattgccgtcattccatgtggcgtaaacctcgaagaactgtttcctattgataagcaactggcccgcattatgttgcggttacccaaagaggaaaaaatattgctgcagcttggccgtattgttccccggaagggaatcgacaatgtcatccaggcgttatcaaaactgagctgccgccagcataatgtccggctcattgtagtgggcggcgacgccaaccctacacaacataatcatgaagcccaacggctgaaaatgctggccaaggaactgggcgtaaccgcgggcatccagtttgcagggcacaaaaacagggatgaactgaagtattattattcggcggcagatctctttatcaccacaccctggtacgaaccctttggtatcaccccactggaatccatggcctgcggaacgcctgtagtaggcgctaacgtaggtggtatcaaatatagtgtagccgacggcgttactggtaaactggtgcccccgaaagacccggacgcattggctgccgccgtaagccagctgttacaggcgcctgagaaattaaatgaaatgggagagcaggcagtaagaagagtacgcaaattgtttacctggcaacaggtagcttccaggatgcacaaactttatggtgaggtgttggcgcgaagcagcaggagaagtgaagcagataccataaaaagagcagtatgaagaaagccatattcattgataaagacggcacattgatccatgatgaaccgtacaacgtaaaccctgaaaagatagcgctggaaccttttgcgggagagtctctccggaggttacgggaagcgggctttgcactgatcctggtttccaaccaggccggtgtggcacacggttacttccgcgaaattatgctggtaggtgttttcaaccacatcaacagcctgctccgcgatgaaggcgcctggctcgacggatgttattattgcccgcatcatcccgaagccacacttaaacaataccgggtcaactgcgagtgcaggaaacccaacgccggtatgatcctgggcgcggccaaagatcataacatccacttgccctcgtcctggatgataggtgatatcctcaacgatatagaagcgggcaaccgggcgggatgtaaaaccgtgttactggataatggcaatgaaaccgaatggcggatggatgtcaacagaacaccgttataccgggcaaactcctggccggcggccacggatattattatcgaacactcaaagaaccccgtttatggacttacttattaagcagatttgtgcagcggagaaaaaactatccgtactggtgataggcgacctgctgcttgatgtatatatgaaaggagaaagccatcgtctttgcccggaagccactgcaccggtggtggaagtcaacagccggcaatatgctcccggcggcgccggcaatacggctatcaacctggctggctttggcgtaaacgttacctgcctcggcatcaccggaaacgatgccgcaggccggcagctacaacaactgcttagcaggcatcacatcaatcctttactgttttcaccgcctgaacggcgcacgatctgcaaaacccgcctgttggcaggcacacagctgatcgcccggtatgataccggcacggaaaccaatatcagccgggaaaccgaagaccaggtaattgaccaactggaacggatatacgctgatttcgacgccgtactgctggcagattaccagaaagggttgttgacgccccgcatcatcagcgccctggaacgcctgcaacaacgctaccagccattccttgcagtagacgcaaaaaacctcagcgcttaccgcgacctgcatccatcactggtaaaacctaacagcgatgaaattgcgcggttgctgcaactccgcctcaacggaacaaaccggctggaaatcctgcaacaggccggggaagaaatattcagcgccaccggcgctggcatcaccgctgtaacgctggacgaagctggtgccctgatctttgaaagggatcaactcttgctgcatacgcctgctcaaaaaatattgcatccgcaggtatccggggccggcgatagttatatcagcgcatttacagtagcgtgcctgcatggggcagatgctgctaaagcagcctcagtagctggtatggccgctgccattgccgttagcaaagctactaccgctttctgtacctccaaagaattgctggcggccgcagcgctcaacggtaaggttctcacggatacggatacactggaagcgctggggaatttctaccgcaacaacggcagcaaaatagtatttacaaatggctgtttcgatatcctccacagtggtcatgttaattacctctgccgcgcaagggagctgggcgatgtactcatcgtagggattaataccgatgaaagcatccgccgcctgaaagggagcgacagacccgttaacaccctcgcagaacggatgcaggtgttgtcgggtctcggagcagtaacgcacattatacctttcggggatataacagacgacacacccgccgcactgattgcagctttgcggccacaggtgtttgtaaaaggaggagattattcactggaagatttgccggaagccaggctggtggaagagctacacggggaggtagtactgctgccattggtgaaagaccgctctactactgctattatcaggaaaatatctacccggcaattatcacatcccgcttaataattatgaatataaactggaacgactgtaaaaaaatcctgtgcatccgcctcgacaatatgggcgacttgctgatgagcacaccggctttccgggcattgaaagagtcctttcaatgtcacctgaccctgctcacttccgcggctgccgcaccggtaacagccgacataccggaaatagaccaggtgattgtatttaatgcgccttgggtaaaacacgatcatgtggctacaccggaaacctaccagcaactggtggaaaccctgcgcaaagaacattttgatgcggcgattatattcacagtgtacagccagaatccattgcctacggccatgctggcttttgaggcaggcattcctttaagactcgcctattgccgcgaaaatccctaccagctgcttacgcactggattccggacgaagaaccgctgcataccatccatcaccaggtggaacgcgatatcaacctggtagcgtttaccggcgctaaagtggtcagcacaaaactttccctgcaaacacatgaaacacactggccggccatcatcaaaaaaatgagactatacggcgctgaccacctcaaaccctggatcgtaatgcatccgatggtgcaggacgcaaaacgccagtataacttttataagtgggtggaaataggtaagcagatcattgcacaccaccagtgccagttactgattaccggcaacaccggcgaagaagcagatgcggaagcgctgaaagaagccattggcgaaggcgctatcaacctggcaggcgcattgtcggtcgctgaatttgcgttgctgatccgcaaaagccctttggtgatttctgtaaataccggtactatccatatcgcggcagctacggctacgccggtgattgtactgtatgcgttaacaaatttgcagcacacgccctggcgggtaagaagtgaagtgttatattttgatgttcccccgtcgctgcaaagtaaaaatgtattgttgcaatatgcttatcaacagatccctaagcatcaactgaaaaaagcaaccgtggaaaatgtgttgaaagcggtgaacaagctgctgcagccggtttaattactcacaggaagaaagcccggtatttaatgctgccgtaaaaatgccagtaaatagacagtatgggaatgaaggcagaagtataaagcatctccagcatatgcgatggctgccggctggtgtgtaataaccgctgacccgtaaaatataaccacgttgctatccagcaacccagccacagcgccgctgcaggtaaattctccaataacaaacaaatcacaaatgccaccaggctgccggccataatataatacttcagcgggggcgcttgtttgatccgggttttataaagggaggggtatttcctgaagagcagcgcattgaaaattcctttgcgctggtcccataagctgcttccccacgaacttttacgaacgggatgaaccacccgcgccaccggcaggtaacggataggaatgccatgccggagaaaattaaactccaggtcgctgtcttcccgccatgccatggtgaaccgttcatcaaaccctcccgtcaactccagcgctcttttagtgcaggcgcaattggccgtaataaattcagcttcggacaaatgagcggtattgtacgcgtggtccgtgatctcgccgggttcgggcatgggcaccaccactttgccggtgtaggccaccaggtcttcgtcctgccggtgatgctgccagatgcggttcagccattcagggtcgggccggcagtcgtcatcagtaaaggcaatgatttttcccgcggcatttttccatcccttgttccgggcagccgcagggcctcctttatgctgcaaactcaggtacttcaactgcagcaggccggtggccttccacgacgataccacttttttggtggcagcatccgggccatcacttaccacgagtacttcaaaatccgcccggtcgaaatgctgccgggccagcgcatgaatacattccatcagcagctccggtctgcgataggtgggaatcaccacggagatcttcatttctttcttcatcgtattatttatttttcaaccaggaaagagcctatcaccagcgcatcaaaaggcgatgaccagaaacattccagtgcatcccggggcgtacatacaataggcttacccaatgtgttaaaagaagtattgattaataccggcacacctgttttctttttgaatgcctgtaaaagctggtaataagccggatgctgggcttcatttacggtttggatacgtgcggtgccgtccacatgcgtaacggccggaataagggcctgcttgtcttttcttaccgggtatacaaacaacatgtaaggcgactgcctggctccctcaaaccattcagcggcatcttcttcggtcaccaccggcgctaccggccggaaatcttcccggtctttcacttcgttcaggcgggcctgcatatcctcatgcaggggagaagccaggatggagcggctgcccagcgccctgggaccgaattccatccgtccctggaaccagccgatgatcttatcatctgccagtaattgcgcggtttcctctgcaatattatccagcttacggtaggatgttttcgtccattttaaaaattgttcaatttccgcatccgcataagccgggccccagtaggcgtgatccattacaaagtcctttccttccggatgccgcatccgtgcatccagccacagggcagcgcccagcgcagtgcctgcatcgccggcggccggctgtacccacatgtttttaaagatacctgcatcgcggatggtggcattcagcacacagtttaaggctaccccgccggcaaagcacaacgtgtcgctttgtgtttcccgtttcagccaggaagccagcgaaagcacgctctcctgcaacacctgctgcatggaatgcgcaatgtcgaaatgatgcgccgtgaacggatcatttttccgccgcttcggacccaggatctctgccaggtccacatcatcaatctggtactgcccattatcagacagcgaaataatatcgcgtaacacatttacataaacaggtttgccgtatgatgccagcgccatcaccttgtattcatcagaagaatgaagaaaaccaagatgagtagtaattttttcgtacagcagtcccagtgagtgcggcatatttacctggctgatcctctccagcacattgccggacccggtactgaaagtagtggtagccctttccccgcggccgtctatcgtcattacagcggcctcgtgataaggagagggaaggaaagcgctggcagcatggcagaggtggtggtcgatatggtgccactgcccggggttactgttaccctgataaaaacttggctgcaggtgatgcggataaccatcattcaattgtcccctggcattaacaatcgcctgcagaaataaaggatcccagggcgattgccacttctctgcggtaagcgttcccgccggaaataaaggcagctttatctcttccttgctggcaacttccggttccatcaactggtacggatcaaaagaataggcaaagtgatctacatcgttgatatgaatgccggcggtacgcaaacaataatcaatggcatgaaaaggcagctcatatgctgcaaaaggaatgggtctttttccatgtttgatatgggtaaaccgctcgtcttctgccgctgcgatcagctgcccgtcttttaccaggcaggcggctgaatcatgaaaagcggcattaatacctaatgtatacatctccagaaattaaaatgaaaataaaaaacgggttagtaagggaagcaataatatcagctgccggactctttgtcctcgtcccattcaatattatctgcttcttcatctgaaagatcattttcttccaggtcattctcatctaatggcggatcggtgtcttctatttccagatccgcgtcttcatctgacgttaacccgctgtcaagatcctcttcttcacgggcattttgtgcggcagtactttgcgtattggcatgactgctgaatcctccgctaacctgtttgttaggagtgctttgttttgatgcttgcttttccatagtctgagttttttttaaaatcgttcaaagactacgccatgtgccggagcagcgcttccacatcgctgccgttatgcagttgcggaacactttacccattcaatgggaaatccggttacagagtgggagtaatttttcagcatgtaaccgcttgtattatttttttacgggagaataaggaagatgtaaagcatctttaaaaagtaataataattcgtgggtataatattgccgtatcgctgccggatctccgttatcttccgcttttaatctgccctgcgacatgggctggcctttgaagctgaaagcataataggcaaacagttcggtgatgcccagctcaggcacaggcgaagcatacccggtgatagcgatgccccagtcggccgagaataaaggccccactgctattgccatctccagcgctactttctccgatacacaatcacacttttgtccatgtatagggtcaatgttcaggtgcttcgttttctgaccaatattataagtggtaatacctccctggaaaaaatccatcgctttttcagccagtgaaagcgctacttgtaaatgcccggccgttacgctttctgctaccgccagggtttgctggttgctggtaagtaattgccggatatcacgcagtaattcagtatcagatacaaatgggtccatggttcattgcttttttttataaatcactaaagctgtgccattcagcaacacccggccccgtctttgctgccatttttaaaaatcattctatacacacttaattcatttgctatgacaaccgttaatgttaacaacagaaatgaatacgcattaattaccggcgctaccagcggtattggttatgaactggctaaactactggcggcagacagttacaatctcatcctcgtggcacggaaccccgaccggctgcaggaagtaacggatgaactgaaagcggcctatggggtggaagtaacgcccattacaaaagacctgttcatgccatctgcagcggctgaaatttatgcggaaacaaaagacatgggtatcagcatcgatgtgctggtaaatgacgcaggacagggagaatgggggcctttcctagaaactgacctgaacagggatattgatatcatccagttaaacatcattgcgttaatgtcgctcaccaaattttacctgagagacatgcataaacggaacatgggccgcatcctgctgctgggatcagaagcaggaaccacgccgatgccgctgttgtccgtatacgcagccaccaaagcctttgttatttcctttggcgccgccctggcagaagaactgcgtgacaccgatgtaaccgttacggtattgttgcccggcgctacagataccgatttcttccacaaggcacaccaggaagacactgttacctatcgtgaaaaatccctggctcctccggaagaagtggcgaaagacggctatgatgcactgatgaaaggagaacgcaaaattatttccggctcaaaaacaaaaatgcatgtgtggatgagcgacctgctcggaacttccaaagcagccgccaacgcccgcaaactgaacgaacccagtacagaagccctcggcgaaaagaagccgggacatgcagcttcccgcaaggaacgggaatatattaacgaagatagccgtcgcagtgatggtgatctgaaccaggacgtaaactgattccattaactttaaaaagacacaacttatgaaggctgcagtatttcaccgcccgggcaatatcagcgtagatacggttgacgaccccaaactggaaaaagacacagaccttatcctgaaggtaacgtcaacggctatatgtggttccgacctgcacatctacgacggcttttttccacaacccaaaccacaggtactgggacatgaatttatgggcattgtggaggaaacaggaaaggccatcacccatttaaaaaaaggagacagggtagtggtgccctttcccatttcatgtggcagctgctatttttgccagcatagtatgcccgtgcattgcgagcactccaaccccgaacactacggcccggaaggagatatgatgaaaggaaaaggcggcggcctttacgggtatacggatctttacggcggctacagcggcggccaggcagagtatgtgcgcgtaatgtacggcaacataaatccacgcaaggtgccggatcatttatctgacgaacaggtattattcctcacggatatttttcctacaggctggtcggcgatcgactggggccggctgcagggcggggaaacagtagccatattcggctccggccccgtaggtctcatggcacaaaaggccgcctggctgcagggcgccggcagggtgattgcggtagatccgctgaactaccgcctcgataaagcccggctggtaaacaaagtggaaaccatcaacccgcatgaaacagatgcagtggaagccattcgcgccatgacgggtggccgcggcgccgatgtatgcgtggacgccgtaggcacagaagcggaacgttctttctttgacaaagtgaaagcagtgatcaatgtagagaaaggcaccgccaaagtaatggaacaatgctttgaagccgtgcgcagaggcggcgtggtatcggtagtaggtgtatacggcagtccatatgataattttcccattcaccggatcttcgacaaaggtctgatcctgcaattcggacaggcgccggtacaaaagtatatcgataaactgctcggcctcatagagcaggaacaggtggtcctggatgatattataagccatcagctgcctttatccgaagcagcacatgcttatgatatctttaaacacaaagaagacgattgtgtgaaagtaatcctgaaaccctgataagtaaggtggcccgtataacatgcgggccaccttataataaacgctgtaatttgttcagcaccgttttcatattaatgccttttcccagcaaacctttcagcagatcgccttccgtcgctatccgctccggcatattataaatattaaagtccgacgttttcaaacccttcttcacttcctcccaccgcaaaggcgccgacacggtggctcccggcttcggccgcagcgaataagccaccgccatcgtttgtatttgccggttctgcataaagtcgagatagatctgtcccttccttttggccggtgttctcagcacgctggtgttatccggcagttgtttgttggcaatatttacaatcagctcggccagcatccttgattgctcaaagctgtatttcgcgcccagcggaataagtatatgcatgcccgtagaccccgaagtttttacaaaagaaggcgcaccaatttcatctaaaatatctttgatcaccaacgcggtgtcaactacctcgttaaaagaattggtatcaggatccaggtctatcaggcaatagtccggttcatcaggatgctgtatcctgctgtgccagggatttaattcaatacatcccaggttagccatgtacaacagtgtggccctgtctttacaaacaagaaatgattttgtttccccatccgattcgctggtgtaaggaaaagttggaatccagtcggcaaccttatcttccacattcttctggtaaaaattaaatcctttgatgccttcgggaaacctgttgagcgactgtggccggtctttcagatagggtagtatatagtcggcaatggctgcatagtaattgatcatatcccgcttggtaatgccttcatccggccagtataatttatcaagattcgtaaatttcagcaacttcccgtctaccttcatttctacctgtttctcatcgccgggtaaaaatatccctgtattctttttacgggaaggtatttttttcccggcaggaggggaaacaactttcacctctttttcatctgctgcttttttatcttcccgtaatcccataaataccggctgacgaagaatgccttcccgcgttacctcagcaaactttacttcacataccagcaccggttttagccaggtagccggcatattggtttgtggcttggttttaaatgggtgctttggtgccaggagcggctggaactttgcaaaaagttctttcagtagtttatcattaaagccgccaccggtatgaccaatatatttcagttcctttccttcgtactttccgaggataatggccccgaaatgcttgcggctgttcctgccggcggtatagccgcagatgatggcctccatccggtgactgtttttaattttcagccagctctccgttctgcggcccataatgtaggtgctgccggcagctttggccatcacgccttccagccctttgtcaatggccgcctcataaaatgcggtgccctgcccgctgatatgattgctgtagcggatgatgtcatgatccgccggtatgatctccgccaggatcgctttccgttcttccagtgataagtgcgtaagatctttgccgttataccacggtaaatcaaaaacgtagtaaacaagctgcgcacttttgccgtgcttaaaataattttgcagcgcctggaagtcggggttgcctttttcatctaccgccacaatttcgccatctgttactgcctttactttccattgttgcagcgcttctgtgatcaccctgaatttttcgttgaaagaaagctggttgcgggaaagcaggtccaccttgccattgttgagatacccgatggcgcggtagccatcccattttatttcatagagccagtcttctttatcaaacggtttggaagtaactgttgccagcataggcttcatctctttgggcataggagcggttttcccttttttcaacagcgcggtaaaatcgtctgctgctgccggtaccgcggcggcctttttcttggcgacagttttagtaacggtgggttcccggttgcttttccatactttatgtggattttttgcgatctgctcaatggttttaccggaaatcaccgatttgtttttagcggtaatatccgtttttgaagcgtaacggtcttttactttcatcagcagccaggcgttttctcctctgcctgcggccttcaccagtgcaaagctgcctttgagcttttttcccttgagcacaaattttagtttgccgctgtgcaattgatgcaggaggtcttttgtttgttgttttttatctgcgtcattatcgtccgccggttcataaacgccttcatcccaaacgatcacggtgccggcgccgtagttgccttcgggaataataccttcaaagtccttatagttatacggatgatcttctaccatcatggccagccgttttatttccgggtccatagacggtcccttgggtactgcccagcttttcagcacaccccgcatttccaggcggaaatcgtagtgcaggtgagaggcatcgtgcttttgtacaacaaagtgtagcagctgatcctcacctttcccgccggtaggctcaggggttttactaaaggttcttttctgacggtatttttccagactcatagccaacctgttttggatattatatataacgctttcaggagatatccagttgttccagtccctgatctgccggggtattcagcacctggccatcgataccataacgggcgccgtggcaggggcagtcccaggaatgctctgcgttattccagcttacatcacatttcatatgcgtacaggcaggtttcaacgcatgcaacttaccttcttcatctttatacaaagctattttctgatcttcatactctaccactttgccttcaccgggagcaatacctgccagcacttccagctgttcgccggaaaacaatttacccataaattgtttcactacatccgcattgtgggaaataaactggctgaatcctgccacaggtttaatccggttgggatcaaaaagcgcttcgtttttgggcttctgttccagcagtatccgcttcagtaataaagcggccacactgctgtacaccatcccgtttccgccatagccggctgctacaaaaatattatcctccacgccgggaagccgtccgatataaggtaatccatctaccggctcataatactgtgacgaccattggtattttatttccttcactttaaaatgttgccgcacatagctttccagccggagaaaacattgcgtggtattttcttcctgaccggttttatgatcttccccacctgcaatgaggtacttttgtccgtctacttcctgcgtacggtagtagtggtaaggatcatacatatcatagatcagttcatccgggtaacggtcgtcttccagcgtgacggccattgcatagctgcggtaaggtgtgcaccgcaggtgcagcaggttgatgcctggcggaatatgtgtggcgtaaatcaccgccctggctttaaaagtaccggcattggtggtaacggtaacggtttcgttattgtccacactggttacgcggcattgctgccggatggtaccgcctgctgtttcaaaggcgcgcgcgatgccctgtatatactgcaggggattgaactttgcctgttcgcccgctttcatggcttttgtaaaaggaatggatacgggtatagtgcctaccggcgtcatttcaagccccgcttcggcagaggcttctgcaatctgctccagctctttgtcctgttcctcattttgtgcaaacaggatagcatctgcgtcactgaatccacactcaattccccatctgctgatgttatgttttatcagcgcaatggcctctgaaacactggcatatacctgttgggcggcttccttgccaaagtttttacggatcacggaataaggaacgtccagcaaagtatttaaatgtgcagtagtgccgccggaagtgccatagccaatgttttccgcttccagcagcaaacagtttttgccttcatcctgtaaaagaaaggcggtgcttacaccggtaattcccccgccaataatgatcacatcgtatagtgtgtccgggtcagccgttttactcccttcaaagggcattgcgtgatcctgccagaggctgatggaatatgcatctcttgatatcatagctattggtttagtatttaaatcacatctaaatactatgccacggtagaggaggactccttacatacggctcatgccgctgtttatactggcatgattttgccgaaattttaagcaggaacatttgattttttaatgttttaaaaagacaggttatggaacagcacgatcagaataagcaaccggcacaaaaacctttttcaaaaaatgacctgttgggaaaacaggaacagtccgagccggcggagatccaatctgcggaggatgcggaagaagagaacacggaagagatagatggagagaaaaaggataccagcggagaacagtaaaattattttatgcagatacaagacctgaaaaaatcccgtggcgttaaaaatacatggatgttattcatggctacggttttatttgcctgcaataatcaacaaaagagagcgcccgcgtcggatagcctcgcggcccagcaaaatgtgccgggcgatacccttccggagccggatacgactaagtctgtgaaaaatttcagtcgtgttatcgggtggccgggaaacaaaactccggtagcgccgaaaggatttaccgtcactaaatttgccgatggtctcaaaaatccgcgctggatctatgtggccccggatggcgatatcttcgtggcagagtcaaatgccacccgcgcatttgtacagaaagtaggcgatgtagtatccggaaaggccgcatcagagaatgaacagaaaagcgccgaccgtatcaccctgctgagagataccaataaagatggtaaacccgaccagcggtttacgttcctgcaaaagcttgaccagcccttcgggatgctcatcctcggcaacagcttttacgtagctaataccaacggtctcgtacagttcccctataaaaaaggcgataacaaaattaccgcagccggtaaaaccatactggcattgccggccggcggctataacaatcactggacccgtaatgtgatcgctacgccggatggcgcaaagctctatgtgtccgtgggctccggcagcaatgtggcggagcatggcatggaaaacgaaaagcgcagggctaatatcctgcaggtcaatcctgatggcagcgatgaaaagatatatgcgggtggtctccgcaaccccgttggcatggactgggcgcccggctccaataccctgtggaccgtggtcaatgaacgggatgaactgggcgatgagctggtgccggactacctgaccggcgtaaaggaaggcggcttttatggctggccctattcttatttcggtcagcatgaagacccacgcctgaaaggaacgcagcctgactccgtaaaaaaggcgatcgtacctgattttccgctgggcgcacatacggcctcattaggacttgttttttaccgcggcagcgctttccctggcaaataccagcaaggcgcttttatagggcagcatggctcctggaaccgctcacaactggcagggtataaggtggtgtttgtgccctttcaaaaagggcaaccgtcagggcctgcggaagactttctcaccggcttcatcgcagatgcagcaacaagcgacgtatatggccggccggtaggagtggccgtagcggcagatggcgccctgctggtagcagatgatgctgccaacaccatctggcgcatagccgctgaataattattttttaaccttttaaaacggaatgttatgccactaaaagacaaaacgatcggcggacatggcgaaaccagtccggatctgggaaatgactacagccgcgatattacccgcgaagtaacatcggatgatacattgaaaaatgtagtacccgataaggaaaagaaaaaagaagaaaaaaaacaggaagaagaaaagcatacaaaagacacggataacgtatcagagtagttacaggtaaagaaaagccctgatttgccattggcgcatcagggctttttcttaggcggctgcactatttttctttgacgaagtttcctgcgttgtcaaagaatagtctttttttatcactgcctttatgaacgcccacttctatttgttgctctgttttatcaggccggatagtccttttaattttgtccgaatcaatcaggtatcccttatagtgctgcacaatataagtggatacattttgcggtaaccgggaattgatgatcagctctttggcttcaatcaggtgaccgctttcatcataagaggcttccaggttgccgcctcttttaccggtaatattgagtacatacacgttgaaatcgcccctgcttacctcgctgatgttgttttccgttacttcccagttcgacttatacgttttcaacggcatttttaatacttgtctcagggtcatgttggggaagttctttctcagggagtcccgtacagatttgggaacggcattgttgttgatctttttggcatcaacaattacttcctcgtcctgtgcgcggagggtacctgtagtacaaaataaaaatagcagcataaatgagaggtgaagtgctttcatgatatttgatttatgtgagaaatgtggatggtgtcctggttattttttttcaaacgatttcaggttgtacgcaagggtaagcataaatgtattgccctgtatcctgttctgtgcgcccatttcagctacccagcgcaggttgaataacatccggatgtgcggtgcataataactgccttccaggccggcgccaaagatctggtctttgtcggggtccaatgcatagctgcccgccagcggaattttatctgtagtggttttgaattgcatataatacactacgcccgcattgataatacgtggaaccggaccggcagcggcttttttataccatgtttttcccaagccgccttcaatactgaggttatcgcctgttttaacatcggaatctttcttttcggagttgaatgcgtaggacaataacgcagagaaatgaataagctttgttttatcaaagaaaacagtactgccggcagaaagctcatttgccagttgccccagcccactgttatcgtcacctcccatttcatacttcccactgggaaaatacaacgcatagccaaaaaggaaatcggcatgcttcgtatgccatcccagttgcaccggctgaaaataaatgtcactgaaagcaaagggcgatttggtagtcgttatagtagactccagccggttactggcaaacggaaacaataccgatccgccgtagttggcgcccagtattttaaaattggttacccagctgccgccgataccggtaacaaacatattaagatcaagattgtctgacaccacatctcccttgctgttctttaatttggaagcagcataaaaataggtgggtaccagcaatgcaaagcccggaggcgcttgtgtacctgattgcaaaccggcatcaccaagcaaatggtcgccttttagctgggcggaaagcggttgtgcagtaattacacataacagaaccagtaaagcaataaggagaggaatgcgcataatctctttgttcatcatcttgcagaagtttaagaaatgcaataaaagagatgagagagatttgtatatgcctggagaggaaaaattctacctgtaaattaagcagatatttttaaagtgccataaatttttttataaaaaaagaatagaattgtataacttttttaagcatcgtgatgttaatagaaatacaagcttacaacagttccttcctcggcatactccatacttggcaaatcatcttcactgtggcaaatcctttgctccgctgatgcaaatgaaaaaaaacacttatgaagaaaactgtattcatcctgatgttctgctggtacggtcacaccactttcggacaagctgctaatgaagacctgtcggttattcaaacagtatttggtaaagaaaagaaagccgtggtagaacaatatatgcaactggagaatagccagtcaaatgcattctggcaactgtatggcgcgtatgagtccaacaggcgggaactttcccgtgagcggctggtcatcctgaacgattatgcaaaagcatataaccagctggatgacaaaacagccctgtcactcgccaacagaactattacaaatgatatggcctacgataaattccacaaacgatacctgaaaaaatttacgaagatcattggcggaaagaatgcagttaaattctttcagctggaactttatttccagaacgctgtaaggtcctttatccttgatgaagtaccttttatagatgaactggaaaagagtaaaaagtctacacgtagttaatatacagccatcacgaagtaacctaagcatgtcaaagcaacggatggccggtcagcaacttaggaacagttgccatcgcctgagataattaatcaacaatacaggcagagccggtccggaagatcacggatggtagtggggttgtataaatcgtgcaggctccgggccgacactctgcccatttttaacacagatcagatatttaaacggtatataaaatgattatttcatcacgatataagctctttacaacccgccatcgtgattcattcctgtacggtttctcaatagtacactagcgtggaatctacaggcgatgaagattgcggggtgttctcaccctgcatgtttttttaaataccggttaatgtatggatatcacttttatacctgagtaattataatagtttaacggttgagtgaatgaaaacggcagggaatttttcccctgccgttatttttatgtttatataagaagaagatcagtaataataaaaaggctgcgtcttagacaagacacagccgttcctaagcataaacaaattagcaatcatcaattcttaagtatcattataagctttttagttgttcaggaataatccgatattgaagttgaagctcttaagattgtcgttttgaaacaggtcatttttattggtcgcataagaataagctgcgcccagtaaaatgccccagttgccaccgttaggacgtatcagcacacctatttcagggcgtacggcaaatccccagttgttttgcgtatcctcaaatatattgtagtaaatattctgctctgcatactgcgtacctatacccagtcccacataaggcatcgcttttttaccatagttaaagtagtaatgcgcagtagccataataggtacggtataaatcacccggtccatgtctgttgtgatagccgaattaccgtccttgtaagtgatcgtttgtgtggggatatattgctcgaaagaattccagcttacggcaacaccaaatgacaccggcgcctgcttcagaaaataacggtactccgctttgccgccggcaaaactggttttgtcgaggaactcgttgttggtgggaattgctatttcccaggataaaccaaacaggttattgatcctgccctgggcaaagctgctcccggcacccagcgtaaacaataatcccagtataatatactttttcataattttctttttaatggtaaaactattgggcactcaggtaaggcgactgggcaaatgcctgatcaataccatccagcgcacgttgcaggttggtggatgcggaactgcctaaggcgccgttcaggttcatcgtccacgcaacatccagcttctggttagcctgcgcattttttacatcaatgatctctgctattacactgccggtagtaacagagtaggtagtggcccatgggtaataataagggtaataccaaccccagtcccagggatcccaatagcccggatatccccaccagtaaccaggataaacaatacccacggttacatctttcacagctacggtattaatgccgagatccgggttcctgtttcggcctacataagtataacctcttgcttccatgttcttcctgatctgtgctaccagcgactttgcagtattgtccgtgaggatactgtcttttggattggagctgatataagcaacggtatctgaaatgtagaacgttttataagtattgaactgagcagccgggtccttgtccgtttgcacaacaaagttgcccgaaagatctgatagatccggctctttgcggcaagccgaaagtattaccagcgcagttaacagtagataattaaatcttttcattgcggttatttttgagtcattacaataactatcccttcggatgttgttgatccgttacctgtagaaatacctgctatcgttgtgtgcacaggtatgccactgtaattatggtccctgatggatggaagaagtaaaggtatttgcattcatagttatgctttgagttgtgaaaaatacatcagtcatttttttatccggaagaatggtcgatacgttaccgtatcttatcctttaggataaaagcccgtgttctacagatggccataacggctacaccctgattaaggcgatgcttgatgatgctacataactatgcttagggataatgctacttattgctttgaactcgttccgtcattcttttcgatggttaagtgcatttagtaatctggttagtgcctttggtaatttcgttaatagtactttggtgacagtacttccactctaactaacattgcgaatcgcggaaatgttcaaacatattgatttttattttttagaaataatttcggtgatttggatacccatagaaacagtagcagtaacagaattgtttagttgatgtttaatatttttattttttggcagatataaaagaagcgattatcttgcagctgttacctcgtttatttttctcctgagcattccgcataacagcaactcatcttcctttttaattagtgtttatttacagtaatgattccattccgtaggtggctgattgccttgtattatcgattgggtgggcattacaggtaaatctgaaaatacttcttttttcgtaacgtggaatttaaaaggtacacatgcggcgtgttcacacgctgcattatttttctctctttgcggattttcccgggcataagcgatacatcatcttaccgtatgttcctacaaatgagtcatcattttccggacatgaaaagcttttttcttttaacataaaacgaaagcaaaagcatatgatgttacaccgcatatttttattgatgtcctgcctttgcggcctcgccttttctgcaactgcgcagcaatggccgtatcatattactactcagcaaggtaccatcgtggtgtatcagccacagccgcaatcattcagtaacaataacctgtcggccatcgcagccgtgtcctttcagaaagccggcgcagacccggtgtttggcgctgcatggctggatgcaaaagtggaaacaaacagggatacccgcatcgttaccatgcaggaactgaaagtggcaaacgtgaagtttccaggtaatgcagataccacaaaagtgttacaactaaaacatttattggaacaggaattaccaaagcatgatctccacgtaacactggacgagctgctgagcgaactcgctgaaaacaatccaggcgccgctgccgatgccgcactgaaaaatgatccgccaaagatcatcttcaaagaacaaaattctttactcgttaccatcgacggagaaccgaaaacccaacccgataaaacactgggaatgttgcgtgtaataaattccccattcctgatagtgcaggagaaaaatggtcgcccgtattatttgtttataggagggagatggtttagcgcatcgcaccccaccagcaactggacctttgccaggaacccgccatccgctatacagaaagcagggcaaaaaataacggctgataataaggaaacgcccatcccgctggactcactaccacagattgtagtcagcaccgtacccgcagaactgctgcaaagcaacggtacgcccgactttgcacccgttgccggtacctcgctgctgtacatgagtaattctcccgataatatctttatgcagatctccacacaggagtattatatcctcctgtccggtcgctggtacctgtcgcgcagcctgcaaggcccctgggattatgtggcgccggacaacctgccaaaagactttgccaaaataccggaaggcaccaagaaagatattgtactcgccagcgtgcccggaacacccgctgcaaaggaagccgtgatggatgcacaggtaccgcaaacggccaaagtagaccggaagaaggccacaactaccgttacctatgatggcgcgccaaagttctccgcggtgtcaaatacgggcctggaatacgcagttaatacggcgtctaccgttctgaaggaagggaatacttattatgtggtggacaagggcgtatggtttacaggcaacaccccgaacggtccctggaccgctgctaccagcagacctgcagacgtggacaaaatacccgccagctccccggtgtacaatgtgaaatatgtgtatgtatacgacgtaacccctgaggtaatttacatggggtatacaccaggctataccggctgctatgtgatggggcctacagtggtatacggcacgggctacgcgtatgcaccctggtatggcagtatgtattatccccgacccgttacctggggattcggcatgtcgtataatccctggaccggctggagcattggcttcggcgtaagcgtaggattctttcatttcggtatcggctacaactttggcggcggctggtggggaccacccatttaccggcccccgttcttttatccttacccgcatgtatatggtcgcggaccggtagtgatcaataacatccacgtcaataacttttacaatcataccaacaatatttataaccaccgcaccgatgtggtaacaagagaccggaacctttccggcgctacacaaggccgcatttcccgcgctacccagggcaatttatcaggggccacccagggagcagtatcccgcgcgaggaacggcaacttatccggcgctactcaacacccccatatccaggccgaccggaacgggaacgtatttcaaagaaataatgccggcagctggcagcaaagggaaggcaatcagtggcgacccgcttccgatggcgcaggcagacagcaaatggagcaccagttccagcaaagacaacgcggctggcagcacaacgaaaacttccggcaatcgttccaacgcccgcaaggcaacttccgctccggcggatttcaaagaagacattaactctaaaaacgtagtatatgagaacactgatttcctggttgctgatgatgagcatcacgtatagtgttactgcccagaccgctaccgtagtaagtaataacattgtggaagatgacctggttacaaccatcttcgggaaaaacaggctttccctgctggccgataacctgaagatctcccggctggaagaaagagcgtttgaagaagccctgctggaatatgaaacagagaaaagtccctggctgtcggaaaggattgcgctgctgaaaatgtataatgaagaattcacctcgctcgacaatgcaaaactaaatagccttaccaaacaaatgatcaacaacgatcttgagtttggccggctgcagatgcgctacttccgcaaaatgaataaggtgctgggcgccacccgcgcagccaaattctttcaactggataactatatagagcaatctacccgggtgtatctgcaacggcaactgccgtttatcaaagagctggaatcagacaaggcaggaacggtgcaacatttaaaaagtctcacccgcaggtaacgggcattgtccggctaaaatgaaaggcatgcatacaacatcttccttcataaaaatcaaatggctgatcttcctctggctggtggcaggaatttccctgtccgcaagggcgcaggactctctttcaaaaaaaatgaaaccacccaaaaaaaagatcagcctccacgattcattggatcatgccattgatttcagcgattttatgatcgatgcaaatggattcatccccattcccatcctgatcacagaaccggccatcggcatcggtggcgctatcgcccccgtactcctgagaaaaagacaacagccggccagttacaaaaagcataagaacatggccgctatccccccggatataacaggcggattcgctttttatacggccaataaaagctggggcgccggcgctggcagaagtggtaccatcattccctggggaatgcgttataaagcatttgccgcttatattaatttgaacatggacttctacaaaacactccccgtaaaaggagaaacagagttcggcgttaacctgaaaagtatcccggtttttctgcaggtacagaaacaactcggcttctccaactggcacgcgggcatacggtacatgtttatcaaaacgaccgcgaaactggaaaagtccatcctgccggattcattattcaaaccaaaggaaatggataacctcagcagcattgcgggagtactggtggaatatgataaaagggacaatgagtttacacccggtaaaggcaccaagatgcatgtaggcgctaatttctccagccatattttcggaagtgatttcgattataccaacatagaagcatacgcttaccactacattcccatcggcaataaaaagaaatgggtatgcggcctccgggcggatatgcagcaggtgttcggcgacatccctttctattttaaaccatccatcgatttaagaggcattcccaaagggcgctaccagggaaacgtaaacatgctcatagaaacagagcagcgctggaatattgtgaggcgatggagcgccgtattctttaccggcgtgggcaaagcgttcgacgaatatgcagatttcggatcggcctcctgggattacagctatggtaccggtttcaggtacctgctggcgcgaaaattcggcgtgtacatgggcgcggatatcgcccggggaccggaacaatggggcttttatatacagtttggcagcgcatggttgaaatgaccgcttaaattttttatatgtcttacctgaaaaaatacagcctcgtagtattcctgctattaataggagggcagaccctgaaaggccaggcactgatcgcattactgtttggaaaaaaaatcacaaacgaccgcctgaagctgggaattatactgggcgcctcttccagctggctggaaaatgccaccgggcaacgcccccgcgtcgggttcgctatcggcgcctataccagttatgatctcaacgacaaatggcaggtggtgatggatatcgtgatgaaatcacccaaaggcgcaaaagacatccggtacgaaaatacatttatcacccccgatgatccgcagctgattggaacggaaatagaccgcaacattacttacctcaccgtggcgccgctgatccgctataagttcagtccctccttcggaatagcgataggaccacacctgggcgcaaggacaaacgcaaaggacatctatcagaaatcaatggaccagggcgatctttcgtatcggtataacagcaaagaccatacgcacctcgccgatgcaggcgccaccttcgatgtgcagtacgtactaatgaaaggcaaaggtctgcggctgaatgcacaattcaacctcgggttcgtgaatgcttataaagatactgacatgagcgcatataacaggcaggtactgctggcggttggaatacccattggtggtggcaataaatcaggaacgaaataaaacatctcatatgctaaacaacatcgtaggactgatcttactggtattgatctttcagggttgcaaacctaaagaggatcatgtacccaccgataaagaaattaatgacgcatatacgtatatgcttggtcgttatatagtactaagacaggagaacaacgacatcaatgtagaaaaagtgggctataataagatcaaatataatccgcttggctctgcacagttcgtaaatccgaacatggatgttgcctacctggaatgttggctggcggtggatagcagtcatgctgtaattttaaatgtaccggaagtaaaagaccgttactataccgctcagctgctcgatggctggggagaagtaatcaccaatatcaatgaacgcaattatccggatcaccctttcggaaagtttgcactggtgattaaaggcaccaatcccccaaacattggtgatgcggtaaagatagaactcccttctgccaaagcaaaaatgctggcaagggtggaacttaaaggctccccccaggaagccgtaaagctgcaacaggcattcacacttaacgtaccggaaggtattaaaattgatccgccggtaaaagtaccggaatttaccaacgctaaactgataggcgcagccatctttgataagccggatgccatattgaattcttatccggatccaatgccggaagctgccaggtatcaggcactcacaaaaagggtagcagcgtatatgcttacgagtgactctgctgctgcacatgtggaagaagttgtgcaaaaacaggccattccggctttcatggaaggtgctaaaggatttggtacccaaaaaggtggctggtcagtgtcttacgtggcaggtaaattcggcaacgatatcatggcccgcgatataatcaactacggcggcctgtgggccaacgtaatcacagaagcaatttatttcgtggggctcacggatagcggtaaacaattgctgcatggcgataatgtatatgaaattcgtttcccaaaaggggagtggcccgatgctgctgtgaatgcgttttggtcggtaacattatacagcgtaccggattatcatgtagttaacaatagtttaatgcgctacagcatcaacaatgtatccggcctcaaacccaatcctgatggatcaaaaagtatctggctcggatcaacaaaaccacctggtagtgatgacgtcaactggctgcccacacctgcagggaaaggttttgcactcacgttcagaatgtatgtatccaaacccgaagtactcgacggaaaatggttcccggcgccaatacaaaaaaaataaacaaaaagaaacattctggtgtttataacacaaagatccccttcttaagtataaaccaaattgcatcatctcatctttttattccatgctatgggtaaccctgttttatcccatgcgacggagattttgtgtacttaaacaaaggtttatatgaaacgcttcccaatctttaaccggctactttttggtgtaggcctgttttcagcgatgctctcgttccaggatgcatctgcgcagaagaaaccaaatatcctcgtcatcttcggcgatgatatcgggttctggaacctcagctgctggaaccgtggtatgatgggatttaaaacccctaacatcgaccgtattgccaccgaaggagccatgtttacggattattatggccagcaaagctgcaccgcaggaagggccgcatttattaccggccaatgtcctttccgtaccgggttaactaaagtaggtttacccggcgccgatgtgggattgcagaaagaagatcctaccattgctgagtttctgaaacctttgggatatgctacgggccagttcgggaagaatcacctgggcgataaagataaattcctgcctacggcacacggctttgatgaattctttggcaacctgtatcacctgaacgcagaagaagaaccggaaaataaggattatccgaaagatcctgccttcaagaaaaaattcggtccacgcggcgtacttaaatctactgccgatggtaaaatagaagataccggtccgttaaccaagaagcggatggaaacagttgatcaggaattcctggccgctgccgttgattttatgaagcggcagaaggacgcctcaaaacccttctttgtttggtttaactctacccgtatgcacgtaaatacccacctgaagccatcttccgatggtcgaaccggtttgggtttacaggccgacggtatggtggaacacgacgatatggtgggagacctgctgaagtttctcgacgataatgggctcacagaaaataccatcgttatttactctactgataacggcgccatgaaattagaatggcccgacggcggcgcttctcctttcaaaggtgaaaaagacatgaactgggaaggcgctttccgtgttccatgcgtggttcgctggcccggtcatattaaacccggtaccgtgtttaatgatatcttctctgcagaagactggttgcctacactcgtagccgccgccggtggagaagcagatctgccggctaaagtacggaatggcttctccgcaggaagtaaaaacttccgcgtacacctcgatggctataacatggtgccctacctcaccggccaggtgaaagaaggcccccgtacccagttcttttatttcagtgatgatggcgacctgatggcttaccggaaagatcgctggaagtttaactacatgctgcaggaagcaaaaggaatgaaggtatggcgtgaaccaatggataatttgcgcgcgcctgtattggaggacctgagagctgatccatttgagtatgcatatgatcacgcatcgaactattatgaaaaatggtttatggaccacgccttcctggttttaccatcagcagaagaagtgggcgcttacctcgctacctacaagcaatttccaccccggcaacggccagcctctttcaatgtagaggagtttaccaatgcgttgaaggccggtacaaaataagtgtgttgttcgttaatgtcaaaaaaagaggttgttccattaccccggaacaacctcttaattactttcaaagatgactacattagaacaggtaaaggaactcagaaagcgtataggcgacgacgtgattggccagcctgacgtcatagataaaatactcatcggcttactcaccgacggcaacgtattgctggaaggactgcccggcctggcgaaaacacgcgctgtgaaaagcctggcaaaacacctcgacagtaaactaagccgtatccagtttacgccggatctgctgccggcagatgttaccggcaccgagatctatcagcccgaagccaccgagaaatttattttccagcccggacccattttcagcaacctggtactggccgatgaaataaaccgggcgcccgccaaagtacaatccgcactgctggaagcaatggaagaacggcaggtatccgtggccggcaaaacccataaaatggagcccctttttatggtgctcgctacccagaacccgatcgaacaggaagggacttacccgctgccggaagcccagctggaccggtttgtgatcaagatcaacatcacgtaccccgaccaggaaagtgaaatcagtatcgtcaaactggtacgcgaagaatcaaaaggaaaggaagcggcaacagcagccatcccgcaacaggtgatcttcgacgcccgtaaagaaatcaacgaagtaaaagtatccgatgccgcggctaactacatttccgacctggtaaacggtacccgctacccggaaaaactcagcgatggtttagccaaatggctcaactatggcgccagccccagggccagtattgggctcgaccgctgcgcccgcgcggtcgcctggctcaacgcccgcgattatgttacgcccgacgacatccggtttattgtgcacgatgtactccgccaccgcataattctcagctatgaggccaatgtagcccgcatgaatgcagataaagtaattgatgaactgttaaaaatagtggccgttccataatggagaaaaagaaaaaacatatcgccgccgcatatcctccgggagtagtcattaccctcgatgaaatgatgcgttttgaatattatgtgcaggatatcccattgctgccacaacacccggtgtatagcatcctggccggacggcatgcctcccggctcaggggaaggggactggattttgaagaggtacgtatatacgttcccggtgatgatatccggaacatcgactggcgcgtaaccgcccgcaccggcgttacccattccaaagtattcaatgaagaaaaagaaagacccaccttcatcgtggtggatcagaccagcaccctgttcttcggatcacaggaacggatgaagtccgtggtagctgcacaggtagccgccctcagcgcattctataccgttcggcgcggcgacagggtagggggcatcatttttaatgaagatgacaacgaatatattccatctgccagaagcaaatcgcatgtgcaatatttactgacctgtattgcgaagatgaacgcacaactgccgctgcgcaccaacataaggccgcatacgcccgcgctcaatgaaatcctgcacaggaccggcacgctggtcacacacgattacgtagtaaccgtgatcagcgacttttctcaaatcgatgatgatacggtccggcatctccggcatattgccgcacacaatgatgtaatgctggtacacctcaccgatccgctggatgcacaactgcccgccggcaggctggtactcgccaacggtagtaaacagttattatggaataatgaatataaacacaacggtaacaggtatacggagaactttgaaaccatgaaagccacgctaacagaacggttcaggaattatcgtataccagtaatatttatggatacggcattgcccgtaaccagccagatcatgcacttttttggaaaaaccaataactgacaagttatgcaacaacctttacaacaattcggagacctgatagaaccggcgccggtgccgttcagttttcatacgccgggatggtatgtgacagaagtagtgttcatcctgctgctcttaatgggcgcatacctgtttgccaggtaccggcggcgcaacaggtatcgccggtatgccctgctgtggctgggcgaacggatgattacccttcatgcccaacaggaatacatgcagcaggtatacgaggcagatatgctgatgaaacgcattgccatgaaagtatacggacgtgaagaagtagccggcctgcgcggaaatgaatgggttactttcctgaaccagcgcaaccgtcgccgggatcagttttctgcggaagagggtcaactgctggcagaaacgttatacagtcattccaaaacggtggacaaaacagaaacggatcgctttatttcaaaaaccaataactggatacgctatcataaaaatgcacctggaaatcgcatataaatgggtatggttgctgttgccactgccgctgctggtatttgcactgctgccgccactgcgcaggcggcgaacggccctgatagccccgttctttcagcgggcagcagaagtgtccggtgaaaagccccggaaggctgcctggatcaccggcaaaagtatctggatgtacatggtgttgataggctgctggatttgcctgctggccgcagcttcttctccgcggtatgtaagcaaacccggcaaacgtcctaaaacagtgcgcagctttttaatcgccgcagatatttctttcagcatggcacaaaccgattgggtggtaaatggtaaacgcatgacccgctgggaagccgtgaaatcactcatgaaagaatttatcgcacaaagaaaaagtgaccagatggcattggtggtatttggcagcaacgcatatatccaggcgccgcttacgaccgacctgcccatgatcaactggctgctcgatcaaacagaagtaggcatggccgggcaaatgaccaatataggcgatgccatcgcctacagcgtgaagatattaaaacaggatacactcaaacaaaaagtcatgctgctcatcaccgatggtgtggacaccggcacagacctgctgccccaggacgcagccagcatggccggtaaagattcgattgccatctatacactcggcatcggcaaagcctccggcagcggaggctacgacctcgatgaacataccctgcaagccattgcccgcactaccggcggcaggtacttcaacgccctggatgaaaaaggactcagtggcgtatacaaagcactggaccagctcacaccagtggaataccaggaagacaactacgagcccgtaaccctgctgtattattatccactggcagccggcgttatacttgcgctggtattccagtttattgccggcagctatcacctcacccgtaaatggctgccctatgcatgaggcgcttgaacatacgcactggcccatcaactggcagcagttccatttcctgcggccggcagcactgtacctgttcatacccttgctgctcattgtcatcatactcatcatcggcaaccacgaaccacagaaatggaaacaattcatctcaccggtattacgtccctatcttttttcaccgggtagcagccgcgctatgtggttaccgcttattattttttcactgggaataagtatggccatcatcggtatcgcaggacccacctggcaccgcacggtgatccccgggcaaaaagtacaggcagtggtactggtggcaatggacctttcggcttctatggacgccacagatattcctcccagccggctggaaagagcaaaactcaaactcagcgatttcctggacgcacatccaggcgcaaaggccggcatattggcatatgcaggcacgccgcacctggtaatgccttttacaacagattatagcctggtgaaactgcaggccggcgcactccgcaccaatgaaatgcccgtgccgggcagcaacacaaccctgctcatgaagtacatcgatacgctcatgaaccccgtgctggcgcccagcaacatattgctcctcaccgatgaggtgaccgctgccgacgccgcactcttcaccaattacatcaacagctccattcatcacctcgaaatattactgatgtcgtcgccggcaggcgcaaaggtgccgggcttcccacaggccacctcccggcaggatgaaggcgtattgcaatcactcgccgccaacccgggtatccgggtgaaccgcctaaccctcgacaccacagatgtaggcagtatcgccaaacgcatccgcgaacacctcatctttgaaaaagatactaaaacggatgaaaaagcctgggatgatatggggtacctggtcatcatcccggtaggattgctctcactgctttggttccggaaaggctggaccattcaatggtgcatgcttccccttggcctgctgttcaccagctgcagcgtgaacagccgcgaagccgattggtggtacacaaaagattaccagggacaggtattgtataaaaatcatgactacgcccaggcggcggaacggttcacggatcttacgcacaaagccgcagcggcttataaggcgggcgactatgaagcggcagcggctttatttgcactcgacagctccgcggcagggcattataaccacggcctcgcactcgccagactgggccgctacgacgaagcgatgaatgcctttacagacgcggcttcgctcgactcgtccctgaaagcaaaagctggcaacagtatcagcaaagtaagcaaacaaaaaatgcaggtggattccatcatcaacatggatcagccggataaaaaaataaaggaagataaaaagaatggccccctcaaggaacgcaaacgcgaagcagaagatcccagcctctccgccgacaccaaagtgaaagacatgcccaaaaccggcgaacgcatgaccgatgaagtaaaatccaatatccaccaggcacaggaaggtcaatccggcgaacccggcaaagataccagcggcaataacaccatgaaaaacatcattctccgccggccaccggccgaccccggggaatttctgcataaaagatttgaactgcagcggaaacgtgattatcaacaggtaaaaccaggtacacaacgatggtgaaatattatataacggtcatgtatatactgtgcagcaacatgctgcatgcccagctgaaatgctttgccaaagtagagctggaccggaataatgtctatatccagcagccgtttaaggttacctgcacagtgctcactgccacctggtacacacagccgccggagttcgataatatccagatccccggcacatttgtggtgcctttcacgcattcgcaaaccggcaggttcacagatcagggtatcgaatactccggtatccagttttattatatcgttttcccttataaggaaggcatgttcagcgtgccatccatcaccatcaccgtagctacgccgctggaagccggtgccgccagcagcaaagtggtattgcataccacgccggtatcttttgtggtgaagccggtgcctgaaagttttccgcataatgaagaatggctggtggccggcgatgtaaagctcgccgaccactggagcaaaccattaagtaccctgaaagtaggtgatgtgattgaaagaacggtaaccacagatgcttccggcaccctcccgcagtttattccctcactgcccacaggcaaagtatcatgggcagaagtgtacccgggcaaggtaacgctgaaggatacacgcgatgagtatactgccaatggtgaacgcgtgcagtcatccacctggctgctcacaaaagcaggcacttttgaactgccgccggaaaaagtttcctggtggaatccatacgctgcccgcctgtatacacgtacattgcccgctgtgaaattacaggtggcagataatccgcagctggggatgctcaccaccctggaagatagccttgctaaagccagcacacctttgaaaccagctaagaaaggcccgcgcatgatagcaggcatgatctggtataaggcctgtttatatgcactcgccgtgttgttgctgatgtggctgctgtatagaaccggccgctatctcacaaaaaaaataaaataccttttgcagcaataccaccaaagtgaaagcttctggttccggcaatttatgaaagcgccggcaatgacttccctctatcagtggtgggaccgctggcggaaaaatggtgagtcccccgctgtagccgctacgctccttcagcaacaggaaacagacaccttaaaggatcttatcagctatgatatggccgtatatggtaataaacaagagaacaatgtcaccatcacgcaactgaaacatcgtttccgcagttaccggaacaaatggaaacacaaaaaagataatttcatacagcccggtaaccgtcaatggacaggaaactgaagtattatttttctgtatcagaacatttttcttttatgagatgttaatattcagacaagggaaactggttctcttccacgctgtagaaatccgttattaaaccagtcaacatacccgttgtatcctgagcatagcaagcaagcatcatcctgacattgattccttttagtgcagttatttgccgaaccggcatgccctgtcatgccataaacgccaggatgtccatgaaaaatttttctatcgtcataataataaaatcaaaggatacaatagttggcaaaacctatgtagccggcagggagttctctccctgccattcactttaattcataccagccatgtggaaatacgcactcatatcattttcattcatgctgctggaagctacggcaatggcccaggcaggagccggtatgaaaataggtaacaacgacaagcactataaagatagcctgcgcagggccggatatccctaccgcttccccatcctgggaagcaaggtggtggaaaaagggtttagcatccaatacccggtaggcgccatgctcaattttatgggcgggcaacaggaagtgaatatcaccgacctgaaggtgggcttcaacgatgtggagccggtaccgctcgactttatacagtttggcgatgtaaaagcccatatgcaaagcgccaccaccaggctggatctctggatactgccattcgtggatctctatggtattgttggattggtacaggcaaaaaccaatgtaaatattgttgaccctttccagttttccagcgaagccgatttcaagggatatacaatgggacttggaactaccttggccggtggttatcatggtatcatcaccatcacagatattaactatacctggacgcatctgaacaaactggataacgtagtaaaatcacttatgataagtcccaggctggggtataactttcagttccgggaaaatcccggaaagtcgatagcagcatggataggcaccaccggtttttttgtaaacaaaggcaccagcgggtctattgatctggcagatttagcacctacgatggaccccaaccaggcgcaaaagatcatcgacgaaacagagcaatggtacaaggaattgccccgcgctcaacaagtggtggtaaaacgtatagcccaggccgtaaaaaacaaaatggataatcttccggatgatatcacaatcaattattccctgaagaaaaacccggtatctaactggagccttatggtaggcgcccaataccagttcagtaaacggtggcaggtaagatcggaagtaggatttctcggtgggcgaaagtcgcttttattatcaggaaactaccggtggcgctggtgagatggatcggtatcatattattgctgacaggcatgctgcctgttgtcgtatatgcacagacgttacacccggaagaaagcgatgtgattgaatttatggatggagatcagatccggggtaaggtgaaaaaaatccagcgtggcgaactgatattggacccggataagctggaagacatggtaacaattaaactgagaaatataaaatcaattaccgcccgcagaaaattgtaccggatagaaagtgtggcgaacatcaaatacctgggcatcctggaacccgggcgtggcccgggatgggtaaagctcatagaagaacacgataccacggaactgttcattgaagacctggataacatagaaaacatggatgatgatttctggagacggctcgatggatcagccagtcttggtttttcgtactcccgttccagtaatataggccgtgtgaatgagagtcataatatgacctacagtacgaagaactggttgtttctaacatcgggagatctgatgtataccatcgataacgagtttaaaggaatagaaaaggctgatttgggggtgcaggcatatatcgaattctggaagcgatggttcgccataacgtctgttcagttccagcgcagcacggaattagggttaagtgcacgtatgcagctggcagaaggcgcgggtcctatattcatgaaaaccaggaggaacgacttaagggcagccacgggattttctatccagaaggaatacagcacagacagtatcaacgccggccgtgccgtgtctgctgaaattccgctgttcgtgaattactacctgtacgagctgggcacaccctatctcaccctgcaggccacgaattcactgttttttagcttgtcgcagaaaggccgctggcgcgtggaccagagcattacactgtactggaaaattgtaacgcacctgaacctgaacgtgcagttttatttcgattacgatagtaaaccaccggatgtaagcgcacagaaagtggattttggaacggtgttcagcataggatattcatggtaatacttaactcaattcaaatgaaatgcattaaaccactggtgatctgcagcatgctgcttacaccttccctggtcagggcacagcaggcacctgtacctggtgcaggcctgtcgcaggaagaaattgcgaaatccaataatcctctcgcggagctgaaccagattagctttcacgactttattaccatgcaccagcgcggtactacggaagtatccaacaccatgaacctgagaggggtaatggtggcgggccggcagattatccgtgccacagttccgtttaccacgctgccggcagataataagatgggctataattcaggcctcggtgatatccagatctttgacgcgatccgcttttctaaaaacggcgcatccaccgatctggcaataggcccgatgatcgtatttcccaccggcagcaacgattatctcggcaccggtaaatggcaggcgggtggcgcgttggtcgccatacatcacatccccggcggacatgtactgggttccctggttacgtaccaacactcgtttgcaggccagtccgatcgcgcagaagtaagcgtactggctgttcagccaacgcttacgttcaacatcgcagcaggattgtatggacgtagtgccggcgctgtctggacatttgactttgaaaatcaacgtaccctcatcccattcggccttggtgtgggtaaagtgttcaaggcaaacaatatgatggtaaacatctttattgaaccacaactcaccgtatacagcgaaggcgccggtcagcctgcataccaggtgttttttggaatgaacctgcagtgggcaaaaaaagctaaataattctttacaacctcatataaactgaatattatgaaaaaatcactcctctattctgcctttgcactcctgatgctggccgcctgcggacccacgttgaaggtaacctcagacgtgaacaaacaagccagttttgccgggtacaaaacttttgccctctataatcccgccggtcagaaaagtcccatcagcgaattaaacagggaccgtatcaacaacggtgtcatcgccgctatggtggcaaagggctatacacaatctgataccaccagcgctgatctgctggtaaatccaatcaccattgccaaacaaggccaaaacgtaacggctaataccgattattatggctacggtggtttctacagaccttactactggggtggcggcatgggcatgggttccagcaacaccaccttctctgtagataaatacatcgacggttccctcatcattgacgtgatagaccgcgaaaaaagatccctgttatggcaaggcgtaggcaatagccagatcgatggtccgatcaaagacccggatacaaagatccctgccgccgtaacaaagatcatggcgagcttcccggcaaaaatgtagtagcattttagatacagcaataaattaactgttatgttgacaacccacatgagaacatgttggtgtttatctgtcgcatggttcttttccctccatctgtcggcccgggagggcgcttgccctcctggaacgacggtgccgtaaagaagtgagtattgtcttttttgttatctgttaaagagatgtacaatgatgattaaaaaaaggtatttgccgttattgataatagctgtgtcctgcaaccagcaacaaccgcagcagcaggccgcggataaatcaggaaaggctgtttgctgcgccgttccctcaaggtatgcaaccgccgctgataagaaagatccgggtaacatggtgtggatcgccggcggacaatttatgatgggcaccgatgaaaaagaagcatacgaccaggaaagacctgcacatcccgttaaagtagatggcttctggatagataaaacggaagtcaccaacgaagaattcaaagcgtttaccgacgctacccaatatatcaccgtagctgaacggaaacccctatgggaagatatcagcaaacaattgccccccggaacgcctaaacccgacgacgacttgctggtgcccggcgcactggtatttgtggccccggatcacccggtaaacaccggcgatatttccaactggtggaaatgggtggccggcgccgactggaaacacccggaaggtccgggcagtaacctcgagggccgctggaaacaccccgtagtacaaattgcctgggaagatgccaacgcctacgctaaatgggccggcaaacgcctgcccacggaagcagaatgggaatacgccgcaagaggcggacaggcagaaaaacgctatgcctggggaaatgattttaaacccggcggccggtatatggccaatacctaccaggggcatttcccggataagaacctgggagaagatggatttaaaggaaccgcgccggtagccagttttcccgccaatccctacggactgtttgacatgaccggcaacgtatgggagtggaccgccgactggtacgacgcttccttctataaaaaaatgaatgtccacgccgtacaggtcgacccgcaaggcccggccggcacctatgatccggaagatcaatatgccataaaaagagtgaccaaaggcggctcctttctatgcgccaatgattactgcgtaaactaccgccccagcgcgagaagaggtacttcctttgactccggcgcctcgcacatcggcttccgctgcgtgaaagataaagacaacgggaaagagaaaactatattggtgcagaataaataatactaaaatacccatcatgaaaaatgtattaagtggcctgctaatgggcctggtcatattttcctgcaactctcagaaaaacactgcgccggcatcggacaacaagcaggataatgtggccatcagcgatccggatacagctgctgtatacgtagacaaggatattcccgccagaaaatccatcaataccctgtttgataaaatggactaccaacaagcagtacagtgctacctgtggggactacccatcgttgcttttgcggaatggcaacatgtgcattatgatgtattcggggcaaacagcaacgacctcgtattttataatacctatgaagataagctgggtatcttaacagcaaatgctaccacaccatatatcatggattttatagacctggccggaaatggtcccaccgttattgaaatgccccaaggtcatacagccggtggattagccgatttctggcaacgcgaacaggcggtcattggtgaaatgggccctgacaagggaaagggtggtaaatatgttttagtgccacccggacaaaaagattttaaagcccccggattttttatcgttccctgtaataccatgaatgtgttctttggtttccgggcactcgaccccgatccccaaaaggcagaagcattggtacacgccgttaaaatatatccttatgctcaacgagcaacccctacaccgacaaaagtagtaagcccctccggtaaaaaatattttggcggacaaccggatggattggcctactgggaacggctacacgctatcatccaggaagaaccggtagaggaacgcgaccgcttttttatggcctggctggataacctgggtgtaaagaagggtaaaccatttgcccccacagaaaggcaaaaaacaatattgatcgctgcggcagaaagaggaaaacaaatggccatggtaaattcatttgcaaaacgtttcgatagtgtgtatcactggccagaccggaaatgggattatgtgatgatcatcggcgacccctcccagcgcgcagccagttatgatgagttcttccagcgtacttcctatttttttgaagccgttacctactcaaaagcgatgatcaccaaaatagccaatgttgggcaggcttacctcggcgcctatgaagataaagatggcgaatggctactcggtgaccttaactatacattacatgtacccgctaacccgccggcagtaaacttctggtcgctcaccgtgtatgattccaatacccgctgcctgatagataacccccaacgaaatgcagacctctcgtccaggaaaaacctgatcaaaaataacgacggctcggtagacctctattttggtccaaaagcgccggaaggaaaagaaaagaattgggtacaaaccttacccggtaaacactggtttgcctatatgcgcttttatggcccaaccgccgcatatttcgataagagctggaagatggaggatattacaagagtgaaaaagtaaataacatctcaggtatataaaacaaaaaagctccgtcataacaacggagcttctgtaagctatttccccaccggtataattgatttctttacatcaattacataagtgtcggtccaccggtcgtgccatggatgacaccagccgccaaacgcactgaaagcatcgaatggaaccgcacggctcaaccccctcagaaaagcggttttagccgatatttcactcccatcttcatttactgcacgggtgcccgtgataagtttgccgagcgattttcccttaaatactgcttctatcacacccatataaatgccatacgccaccatggccagcaacctgtcgagatagtccattccgggcgaatccgcaaaatccagcaggtcgggataggcaatcgtaataggtattattaccactatcaggacaatataaaagctgaccaggtctatgatgtaattcgccagacgccggccatgaccggccatttcaagcgtggcctcatccgtaaagatggattcttgtgtttgtaattccataggttaaaaggattttaatagtaaattataaaataatcaggtggtttttatttttcccggaaaaaaagtcactttatctaaatcattgtcccgttcattttcaggcaaacacttatcaaagaaataactttgcaggaaattacaaccacgtaagcaatgcggaaacaaatgataacggtactattaatgctgatctggctttgccagctatcaggccgttatgtggtgatgctcgggttttatgtaaaccaggagtacatcgcgaaaaatttgtgtattaaccgcgatcaaccacaactgcattgtaacggtaaatgccacctggcaaaacaactccgcgaggaagaccggaaagaacacgaaagcccctggagtaaaacagataacaggagcgaaatattttatgcctgtcttcctgataataatattttaaaaccggcattcactgctgtaaataccagttacccggtatgtgatcatacaggtactcctgttgaccggccctcgtccgttttccgcccgcccatcgccccggtttcgcatatgctttaaaggtctgcagcccatgcagacagggccttctattgcccggatcattcattcttatttctttataacaccatttaacatgtaccgtatcaggcaaattatactcaccatcctggtgatcagcagcggcatcaccgcctgcaaaaaagacgacaccaccccggcagctaatgaaaccacgaaagcgacactatctattcagtttgataacatcgcaggcgataaaaacctccagttgaataccggtacttatgtgaatgcggcaggagaatcttttaaagtagaccgcctgaaatattttatcaccaatatcaaagtaaggaatgcaggcggacaagaatacaccgttcctaaagacagcagctatttcctggtatcagaatcagaactcgcctcgcagtttgtaaaagtgcgtgtaccggaaggtgaatatacttccctcagcttcatcctcggtgtggacagcctcagcagcgtaatggatgtaagtaaacgcaccggcgtgctggatcctgccggtggcatggacgatggtatgtactggggctggaatatgggctacatcttctttaaaatggaaggcacctcagacgccgctccaacagaccccagcgggcaacacaaattccgttatcatatcggtggcttcggcggatacagcgcgcctaccttaaacaataacaggaccattaccatcaatctcaccgctggcggcacggcaaaagtcaggcaggggagggaagccaatatccacctgatggcagatgtgctgaaaatgttcaacggcgctaccaccgtcagcatcttatccaatcccaccgtgatgtttggcgacttcagcgcaaaaatagcggataactgcagccatatgttccaccacgatcatacggaaaattaaaactaacggtcatggctaaacttagttggcgtatcctgctgatactccttttatctgcatgcggtaaaaatgatgaattaaaagatcccgccgatacatttaccggctttcagcagcccgcgggattccccgcgccggtgtataagctgatcagcaatcccattaccaaagaaggatttgaactgggtcgcaaactgttctatgagccgaggctttcccgcaacaataccatttcatgcggcagctgccacatacaaaccgccgccttcacgcatcacgggcatgatgtaagtcatggtatcgacgaccggctcggcagccgcaattcaccacccatcatgaacctcgcatggaataccaccttcatgtgggacggcggcgttttcgacctcgacctgcaaccggtagcccccatcaccaacttcgtggaaatggatgaaacaatgggcaatgtgctggataaactacgtcaaacaacgccctacccggcactgtttaaaaaagtattcggcacagaagaaataactaccgcccggatgatgaaagcactgtcgcaattcatggtaatggtggtcagcgatcaatcgaaatacgatagcgtagcccgtaagcaggccacgtttacaccggcagaacagcagggctacaccgtgtttcagcagaaatgtaacagctgccaccaggaaccgctgttcacggatcattccttccggaacaatggcatcggcacgggtccaaacaacgatgaaggccggtacccgatcacactaaacccggcggacaagtataagtttaaagtgcccagcctgcgtaacctcgcttacactgctccttacatgcacgatggacgcttttatacacttcagggcgtattaaatcattatgcagcggaagtggaggacggcccaacgctcgatccgctgctgaaaatgaacgcgaaacccggcatcacactcagcgcagcagagcagcaattactgctggtattcctcaacacgctgaacgaccggaattttgttaaagacaaacggttctcagaagaatcgcaataaaatgatacgacagatgaaaaaaatactattgctgctgctgatgatcaccaccggttgctacgaagccagggcctgtgatatctgcggctgcggggtaggaagctactacatcggcctgctgccggattttaaaaagaagtttatcggtatccgctaccagtacaaaacgctgcgttcccacctgggtcccggtggcgccacatcctatcttactaccaacgaaacctaccagacagcggaactctggggcggatggaatatcggcaaacgtttccggctgctggggtttataccggtcaacttcaacagccgcgaaaaccagggcgtcaccatgcataaatccggtatcggagatatagcggtggttggctattaccagctgctggataaacagcatactacccgtggcggcaaactgctggtgcaatcgttatggataggagggggcattaaagttcctacggggaaatatgagccaactgaacataaggaaaatgaagatacgcccaataatttccagctgggcacggccagcaccgactttaccttaaatgccatgtacgatgtgcggctaatggatttcggggtaaataccaacgtgagctacaaaatcaatagccgcaataaatacgattaccagtatggtaataaattcacggcaaacattctggcctattataaaataagggcagcggagaaagttacactggcgcccaatgcaggagtactgtatgaaaccgccgaaaaagatacggaaggaaaaaagtatgccgtggatatttcaggggggcattcactgctggctacaatgggactggaagccaccatgggcgttgtttccgtaggtggaaatttccaacccgttatttcacagcagctagctgatacccggattaaagcaggcaaccgcgtaatggtgcatgttacttatttattttgatgatgcccacgcaatagtgaacaggtgtaagccattttcaaaacggtagctttcctgccagccgtgcaggtggcagatctggcgcacaatcgccagccccagacccgtgccggtggtattgggggaggaagtgccaaaacgccggaaaagcattttctcctccaatggcatggcgccggtattggatatctccagcaggccctctttcagggtgatgatcacggtatctttcaggctactgtgccgcactgcattcatgatcaggttggtgagcagtatttccaccagcactttattaccggatattataacgtccggcgtaatatgcgtgactagctgcaattgcttgtcgtccacgaaatcctccagcaatgaaatatggttttccagcagcgcagataagtggatggtggctttcccggaaaactggctgttctctattttcgccagcagtaacaggtttttattgatgcgtgttaccttcgacaacgattgatgcgcttcatcgatgagcgccgattgctcgtctgtaacaggtttgctctggtgcagcaggtccagtttgaacttcacaatggataaaggcgtttgcaattcatgtgatgcattttgcgtaaactctttttgttgtttgtacactgcaatattgccggcaattaatttctccaggtgatggttcagtgtttcaaattcttcaatcccggttttttcaaattgaatagcatgttgctgatgaaggtcaaatgactggatcttttgtaagctgttataaaaaggccgccacagtttttcagatattttccggttaataaaaataagaccgcccagcaggatgaggaagaaaataaacgttacacccccaatagcaataatggtttcataggattcctccatattggattcctgcgtaagccggaatactttaccattaatggtgaagtaggtcaccaatccctggaacctgtcccagccctttgcaggtatatatttatttttacggtagatgttatacgtggaatccggccgtaatgcggcaacaggttgtaactgtgtttccggctgcagtttattccagagggccacactttcagcgagttctttatcagtaagagtaagcgcctgcaggttttgccgcgtggtagcgcttacaatgcggttatgttctttcagttcatgttcccagatgaaatctataatggcatagtaggcgggaatgctgcatgcgagcaccatcccggcatatagcacaaatgccctcatcgatttattaagcaacttattcatagccttgcaggatgctttaaggctgctaagataaactatacttcccacctgtaaccggtgccgtaaatagttttaagataatgaccgcacccggcctccgttagtttctttttcagatttttgatgtgggcgtaaatgaaattgtggtcgtcaagcataccggcaatatcgcctgaaagatgctccgccagcgcatttttagagataaccttatttttgttgctgataaaatagagtagcaggtcaaactcttttttggtgaggatcaccggcacattattaatgagcactgttttagccagcaggttaatggtgagttcattttgccggataacattattgttattaaattttcttcttctgatgacggaaaaaatccgggccgatagctccggtaaatgaaagggttttgccaggtaatcatctgccccggtttttaatccctgaatcttatcttcgtaagagtctttcgcagaaatgatgataatgccctcatctttctcccgtttttttatttcttccagcagcctgataccatcgccgccgggtaacatcaggtccagcaggatacattcatagtcaaacatttctatttttgccaatgcctgctgataggtacctgcatattcacatacgtaattttcacctgataaataagagataatgctttgtgccagctgtatctcgtcttctataatcagtaatttcatggcactaaattaaacttcaattctgaattaattctgaattaatccgctgccaataagggattaacgctataaagtaatcctgggtgtctttcttaatatattgtataacagttagttatgtgttggttggcactttatttatcttttagggagatggataacggtggtatcaccgcgtttagaggggttaatcacgatgtacaagggccatcgaacttttcccgatccgtctgagctaatcgacaggattgatttttctttgcacaaaattaatctcgttgaaacatttatactttattctcggcctcatttttatcaaccttactgtactggcacaaacaggtgtcattaaaggaaagatcagctccgccgacgggcagcctgcagcatttgtaacaattggattaaaagatactaaaaaaggtaccctgaccgacgaagcaggtctctttacattgaagaatgtaaagcccggtaattacacactggtcatctcttacaccggcgctaaaacactgaatcaatcggtaaccattggcgcagatgaagtaaccgcagtaaatatcgcactggaagcaaccgccagccagttgaacgaagtagtggtagacggcactaaaacaagaaccattaataaaagaccggtaagcatcggcaaattaccggtaccggtaatggacctgccacaaagcgtagccatcatcggtcatgaagtactggagaaccagcaggcacaacgcctcagcgacgtggtgaaaaacatcaacggcgtatacatggcctccatgagagccggtacccaggaaacattcaacgcccgcggatacggattttccagcaccaataccttcaagaacggcgcccgcgttaactccggcgccatgccagaaatgagctccctcgaaagggtagaagtgctgaaaggcagcgccgccatcctgtatggcaacgtttctcccggtgctgtgatgaacatggtcaccaaacaacccaaattcaatttcggtggtgaagtaaatctccgtgccggcagctacggattactgaaacccgccttcgatgtatacggtcccctgtcgtcaaagatagcctaccgcgtaaacggtaccttcgaaacagccgacagctaccgcgaccaggtacactccaaacgctattatgtaaatccttccttgttgttcaaattgagcgaccgcacggaattagtagtacaggcagattacctgaaacacgactttacccccgatttcggtacgggttctatcggcgataccgcattgatcaaagtgccccgcaatactttttacggcgctccatggcaatatgcacatacacaacaaaccaccgcatctgccaacatcaaacataaactgaacgataactgggcaataacaggcaatatcgcttattctaaatattaccgggactattactccatcgaaaggatccaggcaaaaggcgacagcacctgggcccgcccgctgggaagaaatggtaccaatgaagattactacgctgtacaggtggatttaaccggtaacgtaagaaccggcgccatagaacataccgtcctcgccggcgtggacgccgacaggtacctcacaggcacctatggatacaccgtaccatctatcaacaaaactaccggtatctacgatatcatcaatgtatacgaacccaataagttcccataccgtaccgatatgccggtggacacgctgaaaaccgttctcaatgcaccggtaaacaggttaggcgcttacgtacaggacctgatcagcatctctgaaaaaatcaaagtactggcaggcgtgcggttctcttacctgcaaacagaagccccggttacctataactttaaaggtggcaaaacagccggtaaatctaaatacgatcacgcattttcaccccgcttcggcctggtatataagccaatcgcttctaccgcggtattcgccagctactccacttcatttacacccaacagcggccaggatatctatggcgcaaacctgaagccatccaccatcgaacaatatgagctgggtgtgaaaaatgatatcctgaaaggacgtttgtccgttaacgttactgcataccgcatccgtaataataactacgcacaaatggcagcgtttttaagcgatggcaccaccgtgaatagcaacaccaacattaaaacactgatcggcgaaaccctcagccagggcgtagaactggatatcgcaggacatcctgtagccggtttggatctggtagcaggctacagctataacaacatgaccatcgaaaaaacaacaggacttaacggcagttccatagaaggcgaacgcctcgtaggtaaccccaatcataccgccaacgccagcgcattctataccttacaggaaacaaaactgaaaggtctgaaagtgggcattggatattactacctcggtcagcgctacgcaggctggaacaacacggtcaatcaaacacaaaaatataaccgcctgatttctgttcccggtttctctaccctcgacctgagcgccggatacgctttcaaacgctttgcagtaatgggtaaagtttctaacgttaccaacacctacagctactacgtacacgaaaactacagcatcaatccaataccgcctacgcagtttacgggcacagtgtcttacaaattctaaacgcgcggattttgtcttggctcaggattacgctgattttactgattacctggatttttacttttttgatttttttgattttataaaggagtaagggagatagaagcggatattcgcttttatctcccttaattattataaaaaaaatctaaaaatcttaaaaaaatccaaaagtaaaaatccaggtaatcagtaaaatcagcgtaatcctgagccaagacaaaatccgcgcaaacaatttcgcggcttagttgttcagtagggaaccgttttattcactcctcaagtacagcatgatgaacagagcaattatcacttgcatcctttttatatgcataagccagttattgtttgcccaggacgccaattattggtctggaaactatggccctggtggcttttttacgcccggtgctgttattgctaataataaagatagcggcgttcttttttataatcccgcattgcaggcgcttaccaaaaagaaaaccgcttctatttcaggaaccgtgtaccaggtggagtccatcaagataaaagatggcgcaggtaccgggaaaagcctgcattcacgtatcacttccagcgtgccccagatgttatccggcatcgtgtccctgggccacaggaaacccgtttatatcggctatgcacttacacatactgcggtgctgaattacaatgtatcccagcaacaggatacaaagctcaatgtggttgacggcagcgggagccccggactggaatattatcttggccagtacaattttcagaaccttacccgggaaacctctgcccttatcagcacaggatttaaattgtctgaccgctgggcaatcggttttatggcagaaggacaatcccgttcccagcactacagtgaaaccgtttccgcccgggcactgattggcagcaatacctccagcaccctgccactggccagtaacgagggcgcgtaccaggtggattatcatcacatcggcttaaaactaaaggccggtttaagctatgaagtaacgaaacatcatttcgggtttttgttgtcatcgccccttattcatatacgtggacggggaactttactgagcaacatggctattgccaatgtccgtttcctggacgaagatcccatcaacctgctggcgaacacgcggcagactaacctgaaaacaacttataaagtacccgccagtgcagcgtttggatatgcatatgactatcgcaaaggacaggtgtatctagcggcggaatacttcctgaaaataaaagactataatatcctcaccccgaggtctgaaatttttcaaagacccgacaccgggaatagtaattcatccgccattgcattgctggaaatgagggaaggcagaaaggccatttttaatatgtccgttggcgttagttaccagctgaagccgcagttaacaggctattgctccctcagaaccgatttcaactacgccagcagggaaaataccgatggcttttcgcctaatacgtctacatgggataactattactgccagctgggggtaaacatcaaaagaagacagtataatctccgcacaggcattttgttgggctacggccataccggcagttaccagcaacctattaacttcgatgatccgaaagagtctaatctcctaacaggtaccattggcgcggtgccggctacacgcgttacggccgctttgatgattgcctttattcataacctgtaatacccttagatcagccctttcaatatggccacactcttcgtcaattcctcgtttgaagaagaggcaaagccaagccgcacggcattggcatgatagttccggtattgatgagctttaccatccgaaaggaataaccccttgccaagggccctttgtgctaatttttccaggtcgatcgatgggtcaaattccgtccacacggtcatgccgccctcgggaatggtgaagcttactacatcacccaattcacggtgtaacaggccgcagaaaaggttgcgccttttttcatataccggtaaggcctttctgagatatcgttgcaacgtgccgtcatttaaaaggccggccatggcgttgtctaaaatatggtcgccctgccggtccagcaggatacggactttcgccaggtgttcaataacgttttctgcagccaccaggtaccccatacggaaagcaggcgaaaaacttttgctgaaagacccgcagtaaataaccatgccgttttcatcggcgcttgcaagcggtaataacgggcggtgtttatagtgaaagtcaaaatcataatcatcttcaaaaatgatgaaaccatattcattggccagccgcaacagctccagtctccggtccagccgcagcgatactgtggtgggataatgatgatgcggggttacatataccattctgacctttcttttcttgcagatctttttaagttcgtctaccaccaggccgttttcatccacgggtatggtaatatgtttcgcgccggcgtgagcaaagttaagttccgctctattccatcctggtatgcctgaaacaataacatcgccttcttcaatcagcgcgttacacaccaggttgactcccattaacgtaccccttaccgaaagaacatttttggctgtcgtctttaaccccctggtttcattcaggtaatgggataaggcatccctgtaaaaataggagccgtccgggtgactgtaactaccgaatttgtgataaagaccgcttcttgtcagctggttccggtaggcccggtacagttcttttatcggcgccaatgccgggtcaggaaatccgtcgtctaaatgaagctccgcactcaccagtgaaatttctgcataaagtttcggcgtaacagaaaatcctgcctttttttgaactgtcgctgtaccgccatgccgcaggacatggggcgccggttccgggatacgcgacgacacaaacgtaccacgccctacatagctttccagccaaccctgcatctgcagctcttcataagccttggataccgtaatcctattgaggcgcagcagggcggcaacatcccttgaacccggcagcttttgccctgaacgaagtttcccgttttttatcagcaataaaagggcatccgcaaactgaaggtaaacggccctgccggaagaagggtcgaaacgcaggccatcaaaaaactgtgctaaaattggactacccattttattctaattggactacaaatgtaatccaatttatgggtaattttgatccggaaaatagtacatatggagaatatcattatcagaaaagtaacgcagaccgatatggcgcaattgcaacaaatcggccggcaaaccttttacgaaacattttcggccggaaataccgaagaaaatatgactaaatatctggaagagggttttacgacagaaaagctcaccgccgaattgactaatgaaggctcgtcattttattttgcagtattggatgataaggtaatcgggtatctaaaactgaatatcgggcaatcgcaaaccgagttgcaggacgacaaagcacttgaaattgaacggatctatgtgatacaggaatatcatggcaaaaaagtggggcaaatgctttatgaacaagcgatgcaaattgcagcgcaggtaaatgcccactacgtttggttaggtgtttgggaagaaaaccagagagccatcagcttttacacgaaaaatggttttgtggcgtttgataagcatattttcaaactgggtgatgatgaacaaacagatatcatgatgaagaaaattttaaaataagacagatgaattttaatatacaacctacgttagaaaacgaaaaagtaatgatcctgccgttgcagcaggaagatttcgacgctttatacgccgtggcatcagatccggaaatatgggagcagcatcccaataaagaccgctggagaaaagaagtattcgaggtattctttgaaggggccatgcaaagcaaaggggcctttaaaatagtggataaagccaccgggaatattataggaagcacgcggttttatgaacataatgagcaggaaaacagcatatttataggttatacgttttatgccaaatcatactggggaacgggcgttaaccatttggtaaaagccaccatgctggagtatattttccaatttgtttcatcggtttacttccatatcggggtaaataatctccgttcacaaatttccattggccgtattggggcaaaaaagattgccgaacaggaagtgatttattttggagaagcgcccaggctgaattttgtgtatgaaatcagcagggaggcctggcagggacaaatgaaaaccgccgccagataacgggttctgcaaattggcactccgtttggaactataaggttataaataacaagatcatgaaaaagatattgattgtcacttgtttagctatagccggtttgttttatgggaataccggttccgcacaggtcgggataaatgtaaatgtgaatattggtaatcagccgctttggggtcctgttggatacgattatgcagaatactattatctgcccgatgtggatgcctattattacgtgcctgaacggcgctttatatacctgaacggcggaagatggatcttcgctccatcattgcccgccagctatcattacgatttaaacaggggttataaagtggtggtgaatgaaccaaggccataccttcatccggatgtgtaccgcagtaaatacaaaaggtataaaggtaattatggcaaacagcagatcattcgttatagtaacgacgaaaaatattacgtggtaaaaggacatccaaagaatggaaaatataaagaagggaaaggtaacaacggaaagggcaacaatgggagaggcaataacggaaaaggtaacaacggaaaagggcacggtaaacacgactaatttttcagcattattccggcatccattgttgttgtttattttttaacttttaaaacaacagttaacgcctatggcaaaacaaacagggttgctccgctttaccggtaagctgggcaatatcattggttaccggaggaacggaaattacttcgttcgcaccatgccggaagcagtaaggcaaactgccgctacccggaaggcttccaggaactttggcgttgccagcaggaaaggaaaactgatccggcgggccatcattccacagctgcatattcatcacgacgggtcgctcgttaaccggctaaacaaagccttgatacaaacaagcagtgatagtctccgcggcctcgaaggattccgggtaaaccgctacaccggaacggaacaattcttccctcatccaccagttgtttcaaaacaaggccagttaaaaatatcggcgcaaagtttaccgccgcagggtgaggcttcccacctggaagttacggtaacggccgtacgtatttgtttcccggagcgccggattaccggccgtagcagcaccaccgtcatgctcgacttacacgagcctttcaacggtttggaactggaagccaatacaccaggaaaaggaaccctgctgatcatcttgcaggtaagaagctttaatggaaccattgcaacgggtaaccgccgtttttttgctgcagatataatagcagtattgacacctgccgccaccaaacccaagcgcctgaaggctaacagcatccctgatgtaagaaagcgatggtctcttcagccggaatccatcagcattagttccaggctcctacatccggcgtctcaactgcagcgggaatgaagcaacgccgttctcttctcaaaaataattttttacgcaacgaagggccgctcttcgccagccctcatgcgcctatacatcaaattgcctggttccccatctgcttaaacatcacataccttcaaatactcacagaaacctgtcatttaagcctccttttcccccgctttattgaaagcatctcatcaaaagaacacctcctgatcaagtccacctcaacgacacgttaaaagtaatcctcctccatgtctctccctatcccacagtatctcccatctatctcacaataatcccccaaagtaaaaatcaagcaaataagtataatcaatgtaatcctgctccaagacaatttccgggccgccaaaggcgacccggtcatcaattatctactcgtaatcttcgtattaatggcactgtgtaccttttccagtaactcaccccctgagaagggcttcctgataaaatcgtcacccggacattcttccattaaggagtcgatatcttctgatgcggaaatgatcagtatcggtatctccctcgtgtcagcatgtgatttcaggtgcttgcatacttccagtatactatggtccggtaagtgactgttcaaaataaacagatctggtttctcaaatgacccttccaataataatttagcatcattcaagaaagaaatctggtaatgcttcttgagcaatgatgatacaagcaattttatatcaacatcgctttctgtgattaggatcttcctggtcatagcaatacgatttgatgtgcccgtatcttaaaccaatatcgcaccaaaatcggggattaaacttgttactgattgtttatcaattatttaagggtgatgataattttatgtttttgggtattttatgaagataattttctacactccgaggtggaaaccgggcgttaccggtacatggataccagttcctgcatgctcaccgcatgcgtattaatagctatctccgtttcaccggatgcaacatggcacacgtagccgggcatgatgggtaccgcgctaagctgccacgtgtgttgatgataaaaaaccgaatccttcataacgttaagcaggtgcaatgcttcattcaaacctgtgccggcggcttttaataccgcttccttccgggtccagtagcggtaaaagatttccggtgatgccggatcgttacggatagcatcccattcttccggggtgaactgctggtgaaagtcttcaacagataataacgtgggcttttcaatgtcaatacccacatctcctttgccggcaaccgcacataccacgatgttacctgcatgggaaatgttgaaatcgggtgcccctttaatgaacggccgcctgtgtaccgtgtatgcgatatcagccagtgaataaccgggaagggcatattgcagcagatgcttgcccagcaaaccggcatgggcatcttcccaacgtttgaaccggtgtatgcctgccctcataccttccggcagggcggccatcagccggttgaaagtatccgcgggcaggggtgtatcataacaactgtaataaacagagataagggtcttcggcatttttttatcaggttaagaaaaacgctcgcaggtgctgcacccgcaatctactccgcaattttcacattttttttgcaattgcatttaatatttcttgttaaattggccgccgtttaggaaacatcggatcactattctccaccgctgtatggagaagtaaatagctattatttcatcagaatataattattatttattaatcttatgttagcaatgtcagcaaggaacaaccactatcgccggcggattacgctgaatccgcattctcttttttgttttcttcttgtatccgttttattcgctaaacagggaattgcccagggaaacaatcattcatcaccaccttttacggcaagactcatcaacattgaagccgccaccaacaccacgtttacctacaacacccggcttcataacggatctgccgcatcccgtgtctatcaactttctgcaagcctgcccgccgggtggaactcctccttcaaagttgaaggcgtacaggtaacatcgctgaacatcgattcagaaaagacccaggacatcaccctggaaattaatccggccattgaaacaaaacccggcaagtataatatccccgtgctggccattaccggaacagataccgcgaagctggatctcgaggcggtagtaaagggaagctatgcggttacactcactacgccatcaggcaggttaagcgatgaggtcaccgaaggaaaccggaaagaaattcacctggtggtgaagaatacgggcactattacactcgacaacctcgacctctccgcacaggcgcccccgcaatgggaagcggcatttgttccctccaccattacccgcctggaaccgggaaaagatgcggaagttaccgctacactgagcgtgccggataaaacactcgcaggtgattatgtcaccaacttctctgttaaaaataccaatgccaacgccagtgcagctttccgtatgatggtgaaaacatctgcacttacaggatggctgggcgtattggtgatagtggcagcacttggcgccgtttattaccttatccgtaaatatggcaggagatagcagcttatggaacaaccaattattgaaataaatgggctgaccaaatactacggctccctgaaggccgtggacaacctccatctcaccattgggaagggcgaaatattcggactgctcggacctaatggcgcgggcaagtccaccactatattaatgctcctcggcctcacagaaccctccgcaggcgaggcgcgcatctgcggactaaacgcctcccggaacccgatcccggtaaaacggaaagtagggtatatgcccgatagtgttgggttctataatgaactcagcgcattggaaaacctcacctacataggacggctcaatggtatccccgaaacggaagtaacaggcgttgcccggaatatgctggaggaggtaggtctcggtgcagccatacacaagaaaacaggcgccttttcccgcggtatgaaacagcggcttggcctggcggaagtactgattaaacaaccggaagtgatcatcctcgacgaacccacgctgggtattgatcccacaggtgtgagggatttcctggaattgatcaggcaattaaaccaacgccagggcctcaccattttgttatcgtcacaccacctgcaccaggtgcaacaggtgtgtaaccgtgtaggcatattcgttggcgggcacttactggcagaaggtaatattgaaacgctggcagccaacttatttaacaccgcaccctatatggtgcaggtaactataaaaacgcccgtcaacgatgcaggcgcactggagaaggaactcctgcaaatgcccgccgtcggtaaagtaacagccgatggaaccctggtagagatctccggccaggagaatattacccccgacattgtacgtttctttgtgggcaaagggattgacgttaccggcgtacagcagaaaagctatggcctcgatgaaatctatcaacaatattttgaaaataatttaaaggaaaatacatccaatgaaaagtcaggtggcttatttcaacggtcttttttcggcaggttcaaaaagcgttgagaagaaaaacagcgcaacgaatccgttttttgtgatggtgcgcaaggaagtggccgatcagatacacagctggcggtttatcattttagccggactgatactgcttactttccttggctccatgtatgtgtccatgaccaatatcagcaaagcagtttccaatgccggcgaccccgacaggttgtttttatacctgaagctgctcaccaccacggatggtacgctgcctcccttccacgtattcgtgggtttcctggggccgttgctgggtattagcctgggctttgatgctattaactctgagcaatccaacggcaccctgatccgcctgatggcgcaaccggtataccgcgactccgtgatcaatgcaaaatttgtagcgtcactgatagttgtcagcacacttttcctgtcattgaacctactgatgatcggcgggggcctcattattaccggcgtaggaattgagccctcagagtttgtgcgtatcctgtgttttgtggtgttaagtgtgatctatgtatcgttctggcttaacctttccatcctgttgtcggtaaagttccgtcaaacggctacctccgcattaacggccatcgctatctggttgttctttaccgtcttctaccaggtgttgctgaatattattgtgaaagcattcctgccggacccggatgtattaagccaggaccagttgctggcctataacaggattattttaaccttcctgcgctttataccaagccagctgtataccgatgctactaccacgctgctgatgccttctgtacgcagcctggggccactcaccatggagcagatggccggggccattccttcgccgctgtccgtgcgggaaagcctgctggtggtatggccacaggtaagcggtttgattgccgccaccgtagtatgcttcgcgctttcctattatctttttatgcgaagggaaatacgtacctgagcatctgctgtattccccgcgtcactcgtccgttctgaagggtgatgcgggcaacagctcccggttatataaattagggttcaccgggttatcagaccatgcataacggacgtatttgggtgcactgatctcgtcgctccatactgtcactttattcccttctattttcgcattggccggaacgaatttcttatcagcgccggcaatctcaaaggtggatggcgcctcgccgtcattggtgatcagcccactgccggtatcagtgaagctgataacgatgctgttctccctggtaacagccaattggtaaagcggaccgctgaaggtaatattttctttgtaagccactttcatagcgccaaaagccaggcgttcacctacggcttttttattatcaggatgaacgtcgttccactcgcccaggtcaatcgccactgccatcgcggtattgggaaccgacaaggccttagcttgtgactccctcatcatcgcccaactgctttctgttggaaggtaagtgtagtccataaatcccgggagctgcacataaagaaaggggagaggcccctggttccatttagctctccagtcgctgatcagcgccggtagcagctttgcatactgcctgggctcaccggcattcgtctcgccctggtaccagcaaaaaccttttatggtataattgatttccgggaacaccatcgcgttatacaatgcagcgggttgattttgcaggttgatattcggggtagcgctttcacgtggtaagggcctgaaaacggcgcccactttatactgccagtcgccttttaaatcaacagtatcggtaccggagaaaatgaagtaaggcttatccggtacaaaccctcctttgccggcggtattggtaacacgcactacgaacaggtttttgcctgctttcaatacaccggccggtacctggtaccggcgttggggatacaggtaagtggtgcgtcccacctgtttgccgttgatgtaaagttcatccgcatccacaatccgtcccaggaaaactttggcaggcttgccggccatcgcagcagggagctctatttccctgcgataccataccacgccatttaaatccttaatgccctggtcttcccagtagccgggaatattaatcctgcgccatcctttcgggatatacgcttcgtcgtaccatttaccggttcctgccagtcctgcgtctgccggcggtttcaccgtatttcccggtggccgtttgaagctgttgagataagcggtgtctttatttttattcattgttgctgtggctgcaggaaattctttcaggccttcttcactcatccatgcttcaatcggcgttccacccacgctggcattaatgatgcctacaggtactttgtatttttcgtagatcttttttgcgaagaaataggcgactgcagagaatggcctggtatcttcgcctatggccggtttccagtaaccggtgggcaggtcggggatggggccggataagccggtgccacccggtaccaggaactgcctgatctgggggtagttcgcttcggcaatttcacgggcatatattacgtcatgaacattgagctgatgcgccatgttcgactggccactgcaaaaccatacatctccaaacaggatatcatgcagggtaattttattacccgcagtaatctccatgttgtaaggcccaccggctttagtgggcggcaaatgcacttcccagttaccattggcatccgccttcgcctggtatgttctgccattgaaacggacctgcacttttccatgattagcagcccatccccacaactttattttttcatccctttgaaggatcatactgtcgcggataagccggggcaatttcaactgtgcgaacccgctgaatacagcgagcaggaataactggaggaggattatctttttcatatcaggaactttaaaacgggaaagggatatcgttatttattaaaaattgtttccggcggaccaagatagctttctttcagatctccgaaatcgagcaccagttgctgcagtaccacaccgctgttgaccatccagtatttcaatgtatgtttaccggtggtggagagggtatgtttgctggattggatgatgatattgtcagctacccacttattccagatgctggtgtaagtaatggcatcttccttattgatactgatgatttgcggcgcttcgtcatcaatggataccgcatattgcaaaccatttttgttgctgtgaaaattcaatgtgggagagcaataggtgttgatggtaacttcccctttgctgtaagtataaaaatcatattccacatgcggcgcattgccaacaggttgctgttcttttgcggtaaccggaaaaggcgtgatagcggaaccggttctcccatgatcaggcaaaatcgtccacgtaataccatttgaatgaatggccctggtaaaatgatccgctgctatggaaacgcctttttcttcttcctggtaaaaaacgttaccggtaacaccgccgggaatgctcgcacgcatcagcttgtgcatgcccggtacttttctttcctccgctgaatctgccggaagatatttcacggcgggcattttttgtaccggtggttgctgccagttggtataaccgatatgcgtttggtccatcatatggttccatttccggttgtttaattgatgataagcaacggtgatcagcgagtcttccaggtagcatgcttttacccggtcggcataggtattggccattagctgtttattcttaatagcttctttgttgagcgctgtatagtaatacatctcattcaaattggcgcatgccttcaccggatgcagcactaactggaagtaggcgtctttatatgcagtgggtaacaagctatctatggcgctggcttttttcagcagttcgttgtaatcttttaccaccgttctccactcatcatagttaagacggtaagtattggcatccagcaactcgggtttccttctggcattaaattttgtataggcagctatgatagctgcgatatcttttgcatagggtgttccaaactgggctgcagcccattgtccggtatattgctgaaggtcgccggggccggtcttttccgggttccaggcataatccaggaagaaggagatggggaattccattggtttgatatctcccacatttacaatccagatctgacgggcattaaattcccaggcaaggtgcatttgctcccataccctggtaattgaattggtgttaagccatttgtaattcctgggcgcccctacataatcaaaatgataatagatgccatagccgcccttgcggcttctctctccgggtttgggcaatttccggatgttgccccagttgtcgtcgcaaagcagcagcgttacatcatccggtacgttcattcctttgtcgtagtagtcctgcacttctttgtataaggcccagagctgcggtgtttcactggcaggtttgccggttacatcgctgatgatttttctttgatcagcaacaatccgttccagcaaagccgtcgctgtttctctcgacatgggttcgtcgccgtcgccgcgcatgcccactgttactatcttttcattggtagcccgctgcaagccggtgcgccagaaggctttcagttttacggcattgctgtcgtaattccatggccctgttccatatcttctccattcatcgtgcgccctcatcaatggttcatggtgggaggtgcccatcacgatgccatacttttccgccatccggatgtttaacgagtcatcatcataaaacgcattgccccacatggccggccagaggtaattgcctttcagccggaggatcagttcaaatactttttcatagaagcggtgattaaagccgccaaacttttctttgctccagttagccagtgcgggcgcttcatcgtttataaagatgccgcggtacttcactttgggtgcatcgctgatcgtgatatgctgcttaacaaacagctgcgttcttttttttaccggcacatctgcccaccagtaccagggcgatacgcccaattgccgggatatttcaaatacgccgtaagcggttcccctgttgtcgcttcccgcaataatcaaacggttggcagtactttgtataaggtacccttcccactggtttttcagggagatgggatggatgtctcccgctgctgcaagcgcacgcaccagcgcggatctttcattggagccgataatgatcgcggggccggcgggaatggtcgctgatatcggaagctttatgccggtgaccatctcaatatcctgctgcaggcagctggccgattgcaacaccggctggccgtcgttcgggtccacgcaaatcaccgcgcgggtcagggcaaatgctgctttcgatgcattatcaacaatgatcgattgcgcatcacagcaaatagccagcaggcttgttattaagaaagatattgtccgtttcatcggctaagcgttgttaaaaaccaatactgtttccgccatctaccggcaatatcacgcctgtaataaattttgccgcatcgctggcaaggaaccaggccgcctcgccgatgtcggctggctgtcccatcgtccccatcggtgttctgccaaatacctttgcttttctttccggatcgctgtccaacgcttttgccgtcatgtcggaataaataaacccgggtgcgatggcatttacccgtatgcctttgggcgacagctcaacagccattgccctggtcatgccgtcgatagccgttttactggcagaataggcaatcacttttgggatgccatactgggcagccatggagctgatgttgatgatgcagccagcctgctgctgcaacatgtttttgacaacctcacggctcatcgtgaaaacggctgtaagattggtaaggacgacctgttgaaactcttcatctgttacttccgtgaaatcctttttcatgttggtgcccgcgttgttcaccagtatatctatggggccgtacttgtcaatcactgtttgtacaaaaccgggaacggccgaaaggtcggttacgtcacagttgatagcatgacagtgcgcgccgagtttttgttgggcggcatccagtctttcctggtttcttcctgcaatcaccacttcgattccctgttccacgaacttttctgcgatggccaggccaatccctgaaccgccgcctgttacaatcgctaattttctttttgttgatgtcatcttcttcgttgatttaatatgctgtggttaaatacccggtgcaaacgggaaccgcaggcttttatagtactccagtgttttgcctggttgttcgtacgacgccggtatgggcattttgctgaaggtctgaaaatacaatatacatgcatttctccaccagatcgcctcttcctgttgaattttcagcaacatggttacctgttcaaatctttgtggatctacaaatggctgtaaacttttccaggtatcctgcattttcctggcgcgttcagcccctttataatattgataacatagttcttcccataggctgttgccgcttttcatccggaaattccagggcacatgatgaaaccacaacaggtatttttcatcgcaggtttgcctgttttcccattgcgcccgcgctgccggctggtattgcgcaagggcattgctgccggtagcagtacggtcaaaaccgatgcccgcgctatccgccttgtgataataaacgggattccattccgggcgctgctggttatttacccagggcgcaggtccgtagtggtgactggtacccataatatgatgcaggccaagaggattggaatattgtacaatgatgtcgcggctttccagcatcaggcgggaggcggctttcaggaatgaaggattattgtagtaggtcatccgcagccattcgtctgcaacctgttcgctggacaaagtatgatcccacgcgaggcggccaagtgcataccagttggcctgcgcaaacggatgaccgcaccagttaatgtcattgccaatattcgccacaccggccatgcctgttaaggaatgatgatccaggctgccgtcgattaccttagcaacggtactgcctttgcccttagcgtaggtgtcgctctccagcgtttccttaaacaacggcgccaggaataccaggctggtagcctgacccaggtattcctgcgttacctggaactccatcatcaagggtgttttaggcatggcgccaaacaaaggatgaaaaggttcccgcggcatgaaatcaatcgccccgtttttcacctgtaccaatacgtttgaccggaaggtaccatccagtggaacaaaatcatcataggcctgcttatggcggtctaacgggttctcgtgactgtaaacaaatgcgcgccagataatcacgcctttaaaaggagcgatggcatctgcgagcatattggcgccgtcggcatgggtgcgtttgtaatcctgcggaccgggttgtccttcgctgttggccttcaccaggaagccgccgaagtccggcacataggtatatatttcttttattttttcctgccaccagcgcttaactgacgtatccagcgggtcggcggtttttagtccgccggtttccataggcgcgctgaacctggcggtgagatatactttgatgccataaggccggagcacatccgccaatgcttttactttttccaggtaaggtttggtgagcacaagggcattcgcatttacgttggttactacggtaccattaatgcctatggatgcattggctcttgcataatcgatgtaacgctgatcaatataaccaggcagcgtatgccagttccatatagaagaacccgcgtagcccctttctacagtccggtccaggttatcccaatgattcagcatccggagccggatcttcggtgcggaaataatatttaactgctgaatgggttgctccgtttgcagcaggcgcaggaaatgaaacgtgccatacagcactcctttttccgagttgccgctgatgaggatgcaacgtttaccgttcagtattttagagataataacaaatccttcttcaccggcctgttgcagcggtatggaaatcccggcgttgctgatcagggaagaggagcggggagtgccagcaatgatagcgccgttgcggttaatggcagcgccgtgagggatggtggtgtgcagcaaacccgacaagcctgccgacagttcattgcttacaatatccattgtagcggatgatctgccggtgatgatggtggtaatattttcgcggtaggattgcagcaatgttttatttgcaacaggtgtatatctcagccagagatcatatccgttttctccttttgtgatgagaaaacagcagaggcatcctatcaataacgtgagttttttcataccggcaataactattttatgttgctgataaagctaccggaatagctcatcatcatcgtggaataattctttcataacggttccaaaataacgcaaatagccgctttttacgcaccattttcgcaatcggttgcgtaaatatcataaaaaaaaacctattcccgtaattttttcagggaggaagcccggatcaccatttccgcgcggagtgtaatggcatcggtggtatacaggttgctgatccctttaaggtggttaattaaataggtagcggcggtatccccgatgctgttgccggaatagtccatggtagtgaggttgggctcaatcacccggctgatggggtcattattaaagccggcgaaggcaatatcctccgggatacgcaggccggcggctttaagggccagcatgcaatatacggcggccgtgtcgttggcggaaaataccgcatccgggcgctcgccggcgggcaggtccaggatatacctggcggcgtctgtccccgcctgttctgaaagcgtgctggttaagtaaagctttttgctgaaggcgaggtggtgatcgtgaagcgcctgcttgtagccgttcagcctttcctggtaaacgttccgcaataaatttcctcccaggtgcatgatccgtttgcagccttgtccgatcaggtgtttggtaatattataggccgcttcctggttattgatgccaacggaggtgctttcctcatgagggaacacgcggtcgaagaacacgaccggtatttttcgtttgaagaagggctccaggtggttaatgtcctgtgtattggaggaaagtgagatgaggagtccatccactcttttattaaacatggtagccgcattgcgtttttccttctccacatcttccagcgattgcgcaataatgaggttgtaaccatgccggttggcggcattttccataccggccaatgccgacgacatgaagtgactgttcagtcgcggtaccagtacgcccagcgtatgcgtatgcctgcttcttaaactactcgcaaatgtattggattgataaccaagcgattttgcagcctccacgatctttttccgggtgtttttgctgatcatgggattgtttttcaaccccctgctgaccgtggcggcagaaacattcaggtatttggctatgtcgtatatcgttacttcccggtcctctgacattttagtacagcttgtttctcaaaggaaatgaactttttctgaataaaaaaatgcaatcggttacgtaaatctgattttttcttatattcgtttcacagaacaaaccctgaccatcagccagcgatcaatttttttacgcaaaacgcccgttatgaaacaactgaatgatcaaccaaaatcaagaactgtagcgctcatctttttacgggcgtccctgatcactttatagcttaataaaaaggaacaaccacgatagacagattccatctcttccttttccattttttataattgtctaaacgacattaatcgttatgaaaaaaactgaaaaattaaagcacaaaccgggcatagtcaggctgtcgatcagccgcatattgacaatcgctctttttaccgcctgccttttagccaggccgcccctttcattggcacaggacaaagcgatccacggacgagttaccggcgatggcggcgaccccgttctcggcgcctccgtagccataaaaggcacgaacaaaggacaaaccaccaatgccaacggtgaattttctttggtagccgccaaaggcgctgtccttattatttccagcatcgggtacgccagccaggaaatccgggtggaagacaacaccaccataaaagtgcaactcaccgccgctacaaaagatatcggggaagtagtagtagtaggatatggaacgcaaagaaaaaaggacttaaccggcgccgttgccagcgtaaacctggaaacactgcgtgaagcgcccaacaccaatatcggtcagtacctgcagggaaccgtgccagggttaaacgtaggtatcgctaccgttgccggcggcaccccacccatttccatcaggggacgggtaacactcaacggtaaccagaatgtgctgatcattctcgatggcattcaatacaccggctccctttcttacatcaacccagatgatatcgctaccattgatgtattgaaagatgccagctccaccgcggtttacggcgcacaggcatctaacggggtgatactgattacttcgcggaaaggaaagatcaaccagaaaccacgcatcgcattttctacttcctataccaaccagtacccaaccgtaggcaacctgaaaccatacgaccgcgaaggatatcttaactatctgaaagaagcattttacgataaagcttacctgggtccggactatacaacacctaaccccaacttcaaaattgaagatgtagcagataacagtatccgcagcccgcaaggcggactgctgcccaataactacgattggtttggagaaggcaccaacaccggcaccatcggggaaactaacctcagcatttccggcggcggcgaccgcgttacctatttactgtccggcagcctggtagagcagaaaggttttatcatcaacgataagtttaaaagaaaatctatccgcgccaacatcgaaacacggcctttatcctggtggaaagtaggcctgctgtcctccgcagcatttatcaaccaggatggcgcagagccgtctttcggcagcctgcaacgtatgacgcccctcatcgttccatatgatacctccggtaaactgataccgtttcctatgaatacgctggagccaaatccattcactacctataacgtagacgactacgacagaacaaactattacttcgccaatatctacacagatatagattttccgtttttgaaagggctcaactaccggatgaactttggtaataactaccgcttatcaaaacactttttttccagtatatatgacgccggacaaacaggaagagcctacaaagaattccaggattattatgactatacctttgataatattcttacttattccaaaacttttggcagtcatgatatcaccgctacgttattatatggcgccgtaggaagaaagttcaacagcaccctttctgaagcaagaggatttccgcggctgacacttagctacaacaacctttcccagggcaatatccagctggcacagtcggatgcatgggaagagaacctggcttaccagatggcgcgcgtcaactataaattccgggataaatacctgctgaccgccatcctgcgccgcgatggcttttcgggatttgcaaagaataataaatatggcaccttccccgtactggcactcggctggatagcatcagaagaaaatttcatgaagggcgtaacgccgttcaactaccttaaactacgcgctggttacggcgtaaccggcaaccaaacatcgcgctatacttctatcgcacgggtaaccaccagcgcggcttatgtgtatggcgatggcggtaccaccgcttttggtcagcaggtagcctccttaggaaacgataacctgaagtgggaacgcacaaagggaatgaatgtgggcgttgacttcgccgccttcaacagcaggctgagtggcagtttggactattaccggaataatacctacgatttgttgtatagcgtggctatccccggcgtaaccggctttagcaatatttacacgaatctcggccagatccgtaacgccggctttgaagccgctttaaactacaacgtcatagacaaaaaggatttcaaatggtcggccacctttaatttctccgctaacaataacaagattgttacccttacaggcgtggatgccaacggagatggcaaagaagacgacctggtatccagttcattatttgtgggtaaatccatcagggccatatacgactacaaattagatgggatctatcagctcaatgatacgaggattccaggcttcccggtaggctcagtcaggatcgtagatcaaaacaaagacaatgatattacccaacaggccgacagggtatttctaggccggcaggagcctgcctatcgtatgagcttattgcagactttttcctacaaagcttttaccctcaccttattcctgaattcagtgcagggtggtaaagatggataccttggcaataacaacccgtcgtttttccgggaagacaacagcatcagagtgaataacctgcagggcatcgacttctggtcgccctccaatccaacgggtaaatatccaaggaatatctccggctcccgtgcgaaaattgaacctaacatgtaccaggacagaagctttgtaagactgcaggatgtgtcgctgtcctataacctcgccacttcgctgctgaagaaattcaaggcacaatcaatcaatctgtatgtgagcggcaaaaacctttatacgtggaccaactgggaaggctgggaccctgaagccaacgacaacgacggtaatccgatgggattgatcatcggcggaaggcccgttctcagaggtttcaccgtaggtctgagtattgtttattaatccacgttgtaaaaatattttttatgaagacattatatcggatatcactcatattaatgctttgttcacccgcgacttcctgtaagcatgatttcctggatgaaaaagcgctgtcgttcctcagtacttccaatgcctttaaaacaacggaagattttgatgcatcagtaaataacctatacgggttggttagaagcgagttttatacctccagcgactggcagcctatgcattatctctacagaacggatctggcggtggaagtggcagtaggtagtaatcctaatctttctgcagaatttggatcaaacggggtactcaccaataaccactggagccagctatataaaattgtagcagaagccaacaccattatcagccgcattcccgcttcgcagctgtcggatgccaacaaagtaatgtttgaggcgaaggcaaagttctttcgtgcattgggttacagaacgctggtatatttatatggcggtgtgccactggtactgaatgaaataataggagagaaaacagattttgtaagggccacaaagcaggaagttttaacgcagataacagcagacctgaaatttgcggctgccaacctgccagggattacggcggtgaaagatggtgaagcatccaacctcgctgcgcagcacctgctggcggaagtatgcctcgccaacggtaagttccaggatgcggtaactgcggcatctgtagtgattgacgatcccgccaccgatctgatgaaaacgcggtttggctcacggtcaaccgttacgcccggcgatgtatactgggatctgttccaggcaaaaaatcagaacaggaaaactgccaataacacagaagcgatctgggtagtgcagcttgaaacagatgtgcagggcggatctgcggtgtctaccgccatggcgggcaattaccagctggagcgcgtacacgtgccgttgtaccgcgatatgcgggtgaacggggtggcattgtttcaatggcctatcggcgattataccggtggcaggggtgttggttttttacagccctcaaaacattttgcggatgaagtatggcaaagtgattttaataacgatatccggaatgccaatcacaatttcgtaagagaagtggtggctaccaacccggcaagcccgtttttcggacaaaaaatttctacacaaaatcctcctccgggtgctaacatcacttttccttcaagggtgttttatccgtatcagtcgaaggcaaccacgccgtttaatcaccccgcatcactctacgtgaatccgggttcatctgatcctatcaagaagtatgagttgaaagccacggcaggcggcacgtttgccgaccagtatattttccggctggctgaaacctatttgctgagagcagaagcctaccttggcctgggtaatgccggcgccgccgcagcagatataaatgtagtgcgctcacgcgccaatgcttcacctgtactcgcaggagatgtgacgattgattatattctcgatgaaagattaagagagttaggagtagaagaaaaaagaatgctgacgctgatgcgcctgggtaaactgtatgaccgggtgaaaaggtataatcctttttacggagcgaatatggaaccacgctttaacctctgggcgattccacagggagaaattgaaagaaacagaagtgctgtactggagcaaaatccgggttacaattagtcgtatttttaagaagataaacctggatacatgcatgttaatttatggccggggatattccggtatgtgtttcgtagcactgtttatatgctgttattcagctcatggaccgggagcagctgtaaaagcgcccggttagtgcaggatgcaaacagcgtacgccaggaatcaacgtcgctcagagagcacattagcatcaacaacgactggaaatttttccggtataccggggagccggataaactgatctatgatgtgcgccccggggtgaccgaccggaacgataatgtggtagcagattccaggccaactgaatcagtggcggtaaacgcctcctcgcaggtattaaagaattggatactgccttccggcaatgactttattgccgatcctgccaaacaacatcagcgcccgcaaggcaaacccggcgctgattttccgtttgtgcaaaacaatttcgatgatcataactgggagtctgtacaactgccgcacgactgggccatcaaaggaccgttttacagcgagcccgatgccatcgtcggcggtggaatggggaggctgcctgttcacggagtggcctggtatcgcaggaaactggatatccctgctacagataaaggaaaagttatttacctggacatcgatggcgccatgtcgtataccatggtttggctgaatggcaacctggtgggcggatggccctacggctacaactccttccgcctggatctcacaccctatatcaatcccggcggggataatcaactggccatacggctggacaatcccactaattcagcccgttggtaccccggcggaggcatctaccgcaatgtgtggctcacgaaagtaaacccggtgcaggtggcacaatggggaacatttgttaccactaaaaatgtttctgcctcatctgctacggtcgatgtggtggttcaggtcagcaataaatcggaccatgagcagcagatcgaagtaatcacggacatcttcactgccggggaaaaaatagcgaccatacctgcgtcagcggttaccctgaaagccggcgccacgcacaagtcagcaggttccgtgatactgcaacatccacagctgtggggaccgccgccaacgcaaaagccccatctttatacagcggttacacatatcatctccaatggcaagccggtcgatgaatatcgcaccggttttggtatccgcgcacttacattcgatgcggtaaaaggcctcctggtaaatggtgcgcgggttcgcatacagggcgttaaccagcaccacgatctgggtgcattaggcgcggcatttaatgtacgggcagcagaaagacagctggaaatactccgggaacttggctgcaatgccatccggctggcgcataatccaccggcgcaggagctgctggatttaacagaccggatgggatttttggtaattgatgagatatttgataactgggaaaggaaaaaaacaccgctggctttccacctgatttttcccgactggtatgaacccgataccagggcttttatcaggagagacaggaatcatccttcggtgattgcctggagctttgggaatgaagtaggggagcagtatacagcggaacagggagccgcgattgcaaaaaagctgtatgatattgtaaaggaagaagatagtaccaggccggccaccgcatctatgaactatgcaaagccgggtatgccttttcccgctgtaatggatatattgagtttgaattaccagggagaaggaatacgcgatgcgcctgcctatcagcaattgcagggcatccgtacatcaccgctgtatcccgcctttcaacagcaatttcccggtaaaatgatcttcagcagtgaaaccgcctccgcattgagtacccggggcacgtatttatttccggttttcgaggggatcagtgcgcctgttggggaaggaacgggcggcagcggtaagctgcaacaggtaagcgcctatgagctttatacggctgcatttggtgcatcgcccgataaagtatttgcatcgcaggataagcatccttatgtagccggcgaatttgtatggtcgggttttgattaccttggagaacccacgccctattattccgcacgcagttcttattccggcattgtagacctggccgggtttaaaaaggaccgcttttacctgtatcaatcccggtggcgaccagactataaaatggcgcatatcctgccgcactggacatggccggagcgcgtgggcgccatcaccccggtacatgtgtttacatcgggagacgaagcggagctgttcctggatggagtatccctgggcagaaagaagaaaggtccttatacctatcgcctccgctgggacagtgttgtttataaacccggcgtactaagcgtggtggcctacaaaaacggcgtcgtatgggctgccgacacggtaagaacagccggtgaggcagcacagttgcagctgatcgccgaccgggataatatccgtaccgacggaaaagatctttcatttatcaccctccgtgtactcgacggcgcaggtgtactggtaccgcgggccggcaaccggatccgctttgaagtatccggaccaggcgaaattgtcgccaccgataacggtgatccggccgacctgcaatctttttcttctacagaaagaaaagcatttagcgggctggccatggtcattgtccgcgcaaagccgggaacaacgggaccaataaaagtaacggcgcaatcacccggcttaacgccggcacaggtgatattaaacgcgccatagtaggcaacatttcttgagtaaaatagcatcgctatgttaatgcatgaaaccatgcgctggtttggaccgcatgatatcgttagtttaaaagacatccggcaatctggttgtgccggtgttgttaccgcattgcatcacatcccggtgggagatgtgtggccggtggcagaaattcaacagcggaaatccctcattgaagccgaaggcatgagctggacggtggtggagagcctgcccgtaagtgaagacataaaacggcgcagtgggcattaccaggttcatatagaaaattataagaggagtttgcaacaccttgccgcctgcggtattcaggtgatcacctacaacttcatgccggtgctggactgggtccgcacggatatcagctacacgatgcccgatggaagtaaagcgctctactatgaacgtgccgcttttgtagcctttgatctttttatgctgaaaagaaatcaggcagaaaaggattacagcgcagctgaaattgaagcagcggaaagatggatgcatgcgcataccgaagcacaacaaaacgaagtattccggaatgcgttgctggggctgccgggcagcaccggccgcttttcgccggaagaaattctggcagcgctggaaacatataaagatatcgacgccgccacattaagggagcacttaatgtattttttgaaagaagtggtgccggtagcggaacaactggggctgaagatggccatacacccggatgatccgccttatgcggtgttgggattaccccgcgtggtcagttcagaagctgatttacttgacattgtgaacgcggttccgtcacccgcaaacggactgtgttactgtaccggctcactgggcgtacggcccggtaacgatcttaccgggatcattcagcgattgggcgcgcacatccactttcttcacctgcggaatacccggcgagatgaatccgggaacttttttgaggcagctcatttagatggcgatgctgatatggtgactatagtgcgtgaattattactgctgatgcaacagcggaatatttccctgccggtacggcctgatcatggccaccagatgctggacgatttgaacaagactacctatccgggttattcctgcatagggcgattgaaggggcttgctgaactccgggggctgcaaaccggtctagcccgtgtgctccagctgtaatgcgctgcttcgtatcttaaaacgaggggcgctctatcagtttgcaggggttttttaaatgctgtttctttttattaagcaccatgttaatgatgttggtccccatctttgtaaaatcagtggaaatggtggcaataccattggcagcaatttctttaatggggatctcattataggaaatgatgccaatatcttttccaagcttaaaggataatgcggtgatccgttttacaagatgcacaagatccccgtcgtgtaccagtatatatagttccccggttgccagtggcttattgccaacatgtgtaaccaccgctgagcggagaccggattcccggcagaaccgccggaagccattctcaatttgcttgaggttatagaaggcaggtcccattaccaggaccagcttgttgtacttgcgacggatctttgttaagtgctgctgcaacacctggtaaatatcttcatgaaaatactggcaaacagaaggatacctggcgccccagtcgcggtagccaagatcaagaatataaaccttctgctgcggcagttgctttaatgaagcggcaatgtctttatctttaataggcataataatgtacgccgtgtatttgccgttactttgcgccagcagtgtattaaacaatgccacgttgttatggtggaagtaaatattcactgtgcctttgccggctatcgtgtttttaatgctttcatatatttcttctttataggccgtcaggctgttgaacaatacaaagatgttgtgcctcgattgtgtatttgtgctggctacaaagaatcctttatactgcactgctgataccagtcctgcctgtttcaggctgcggaaggcctgcataacggttttaggggcaatgccggtgttgtcgctcacctggtttacagaagggagcctgtcaccgatctttaactggttgttgtcgatagcattgataatagattgtatgatctgttgatatttgggggcctcggaagtgtgatcgagtgaaataattgacttcatatgttgcgatgtttattcttcaaataaccaatccaggcgctgaacgctgtctgccgcggcaccggcgctgatctcctgtttgccatccataaagcccaacaccaggcaggcgcctttccccaatataagggtatgcttccctgcatcaaaataatacgtgtgcaggttcaccggtggaagggaagggatggttaaggcatgcgccatcctgatggcggcttgcccgtgatcgtcggcgctggcatctgtttccaggtcaggtggcctcaggtagtttttttctttcgtatcaaaatatcctattactgcttttaccggttgtgtattactgaattgaagcgtggtgcctttttcctgttgctgctgcatggaaaacggtaatgcctgtaagccggttaatgcctcgtcggcggtttgtatgcgagcgtctttgtctgtaaacggccgttgttgcgccaccggctgatagtacccgttaacaggttgtaagaagttgacctgcaccgggtgcaaccgggtaattatcgtgtgcccgttagcgttatcaccatgttgtgatatatttttgagtgaatcaagatgttgtttgaagttgcgtaattctgcttcgtaatatggcaggagctctacccatgttttattttttccgttatcaccgccaacaggcacttttctttgctgggtttgcatgctgttggcatagagataagtatcttttgtaagatctgccagctctttatagtgtaccacgctttgttgcagaaagggcagggctttctgcaggtcgttgttatcatgcgagtaccggtaccgcaatacatataaggccgcctgtactttcgcattaaagtaacgggccagcgcctggtagcagtacatatcattttttatgcgcgcaaattccgcggagttttgctgcaccgtggctgctgctttatcaatagccgccacggcacggtcgccgtgttggataatttccgtaataacctgcacaggtgtttctccggtatgggactgatgttgccattctttttccgcataggtagtcagcgtttctcctgcaggaccgtcggagtcatacaggtcggcccatacacgccacctcgaaggattcacgagctggctcatcagcatacccagtgtaagcgtttgccggttaccgttagtaatgccaaaacgccgcaggagcttgggggctatttcccccgcttgttcataggcttccagtatattcttaccggattcccggccgccgaattgcgcatccagtaagccgctccagtagcgattttcctcctcccggttgcggtggcagttccaggcataccgcgcccatgcctggtaccagagccagtcgcgatctacctgcaataaacgcggcgttgccttatccgcggtatatggccagtcccagtaagacgcctgcggatacaggtgcaggccgttggccccgtggatgctatgcatggcctgcacgcatttttgaatgaacgcggtggcgccataccggaaaggttccaggttggcgaggatatgtacattgtcgatgtcaacagtcaaccggctaagatcccggtgcatggcggcccatggtccccgcggggtataggtggttaatgcttcgccgttgtatttattttcggtatagaggttaggatataacggaagggctgcctgcattacctgttgcggattggtgtcatgtccgcgcagcacaatcggcgggagggtggttttacctaatgcgcgtaacccatcctttacaccggggataatggtttccgtaaaccatttcacgtcatcttcatcactcatggcttctcccaatgttaccagcaaccctacgttgggatactccgctacaaaggcggcaatggacttacgggtgtaatctgaaataagcggtgttaccggccgtttgcggtcctgtgtaacaagaccatgcttttctgcaaaaggtttggacaggataatattgtaaaacatctggatcacccatatgccgcgtttatcggcttccgttgtcaggaaatgatacatgtccctgttcttccggaaggtggcgctgtctacttccaccgcatagggataatctttcaggcgcaccaatgatgcaaacggatgaccgttccacaggtagagggaattcatgcggttggcggcgagcatgtccaggtattgaatccacaatgccttatcataaaaccacggaaattcctgtggcgtatagggatattcatatacattcctgccaggcaggtaggtggctttttgtatacctatgcaggtgccgcgcaataccatttccggttggtcggtgatgtttagcgcggtgggtaacgcccccgcagcgcggatcctgccggccatttcgaggcagccatataaggtgccgctgttgtcggcgcctgcaatcagcgtatgttgcttaccggtagtgatcacaaaaccttctttaccgggtgtgttgttaagggagaatttaaactggcgtatagccgtttgggtaagtgtatcaacaagtgcgcctattactatcgtggatgcacccgtaggcaggttgcgctgcgtgctggtttgtacatggtacccggctgcctgaagggctttgcttaattgttccatgccgtattgcaccctggcggcagggtgggggccggttaccagccatatggatttgtcacggcctgcctggccggaggcatataacggtaacaggcccacgaaaaagagaatgctgagaagtcgcttcatacctgtttagttcgtagtgctgatattatttcctatttcttccagtgcctggcggttcagttttacgcgaaccataccgatgggatgaaaacgtttatcattattaatggcggcgtatagtatggtatagtcgtcgtttccttccggtatcaggcaaagcggtgttctcatgatatcccaccacttttttactttggcctggatcggtaagtaacgtgcagcggtccagtgaaggccgtctttggaaagcgtatagcccatcatgttaggaaggtgtaatccgaacccttccgggccgccgtcaaaaatagcgatgtatagtccgttgggcagtttgcttacaagcgggttttcaacaaaccagggatgaatggaagtcacaggatttatgctgctgtccatgcgggtccacggcccttccagggtagaagaccgggcgaggccgatgaaccagcctttgcctgattttgcgggatagtcttcctgcctggcgtaaggataagcgcctgcataaaacgagaaccattccttcccaacaggatatggaaaaaaggaagctacgccctggcggccttcccagagttgtgtatccaggccgggttccatcacgatgcctttatccgtataaggtccgccaatgccctcaatgcctttttttaccgattctgcacgccagatccttccaaaggaatgattcggctcaatatctttatgcacagtataggcaaggtaatatccataccagcgttgatgtgtttcgctgtatacagggataaacgaccacagtgcagcgcggcggtcatttataggattatcgtctgctgtcagcgcatattgcccgctggcctggtaaagtgttttttgccgtttccagtgtacggcgtccgtgctggtccagtgcccgatgcgtgttttcacccggtcgtagtacggcggcatacctgcctgtcctgctctttcggtaggaaacaaatgataggtgccgttcaccttcacacaggcgcctccttcaaaaccgccctggatgccggttgtaccgggcatgccttcattgatcaccggggtatcgggaccgtctataatatcaaacagtggtgtttcagttttaaaaaaaggggaacctgcctgtgcatggttcccctgcgattgggacatttgttgcccgttctcgttcacgttatgattagagtctttaagtacaatcctgaaaacataggcgatgtcggaaggtatcctggttttcgcaggaatcgtgagtgccagtccctgttcctcgatgcggaaaggacaattctccagcgattttaatcccagcagttgaagggattgtatgccgccgcccatactggcgttgttcagcgccttcaggtgcaccgtcttgttatcgcccggccagtccaggaaaacagcatacagcgtatctcctttacgcgtgtagtgtacccgttgaccctctccggtggtttctccgtacacactgaaaggacgggtgccataaattgcttcgccattggcccacatccatttgcctacccggaacattacttcctgctggttttgcggaatgcggccgtcggatgttggagataagttcagcagcagttgcccgttcttgctcaccacttcaatgatcttatgcactatttcttttggggagcggatctccattcctgctgtatatccccacgacagggcaaagccggtgccaatggaataatcgcacagccagggttgggcgatgatgtggtctggattgctgttttcatggtccaccatcccgatgccttccggtatatcatttcctttgtaggtcattgtcacctcctgtccgcgttgcccggcatcattaaagtaatgcgccaggtatcctttgatgaattgctccgggatattttccagccaggagtcaaaatacatgatgtcgggatgatatttatccactacttcattacactttccctgccacatcttcagccatgcctcatgcggcatgggcgtgccatatagtttggcatattttggatctgccgcagcccatccgggtttgggctttacataaccatagttcagttcatgatgcaatgacacgaaaaacttcatgcctcttttacggatggctttttccagttcacctaccacatcgcggtgggggcccatttgtttggcgttaaaaggtgtcagttggctgtcccacatggcaaacccgtcgtgatgctcacctacaggcccggcaaaccgcgccccgctttttacaaacaggtcggcccattcatctgcattgaaatattcccctttgaacatcgggataaaatcatgataaccaaattttgacagtggtccatataatgcgatatgccgctgatacgtgcccagtttggaataacccgaatcggcatgcatatgcgaatagtaatgttcattattatatgcaggaacggtgtacactccccaatggcagtaaataccaaatttcgcatcacggatccattccggcacttctttatgttgctgaagtgaattccactcaggttgataaacaatatttttttgagcagatgataactggtaaaataagatgatcaatagcagtaataacccctgccggtatttaaacagcattgtattcttcataacctggatttaatgaaacagcagtcaggattgtaagaggaagaccaggttgataataaaaatataaatagtgaatgtgacgggtaaactttttttaatcacctcaacttttaccaagatagtgttttttatgaactatggtatactatggtatacttttttccaaaatagattcccggcaacgatgccggcaacgattgcgtaaaaaaaaacgggtgatataccttttttaagtaaatatttttctagcttgatcccaggatatactcctcaagaattccgggagtaattatcagaggggaacagcgtctctgattgtaaaggaaagaccataaaaattcctttgttatgaaaaataaaaattccattcctgtctgcaatgttattattgtctgatagacactaatctattctgtcaactcttattgtccatctaaatcattcaatcaatgattaatcagctacttcctggtaagccatttaccacaggggcgatcctattactgctattcttttatatatgtgcctgtatccctgctgtatctgcgcaagcgccagcccctatcaccgtaagaggaaaagtattatcagataaaggagaagaaattcccggcgtcaccgtccgcgttaaaggcgtttcaaaaggctccatcaccaatgctgatggcaattacaccatccaggtgcccaacggcaaatcggtgctggtgttttcttttatcagccacgccccggtagaagtagcggtgaacgaccgccaggtggtgaacgtcaccatgaaaaacggcaccacagatctctccgaaacagtagtagtaggttacggcacacaaacaaaaggacacttaaccggcgccatcactactatcaaagccaaagaggtggaagacctaccggtaggcaatcttggcgccgcactgcgaagccgcgtgctcggcctatccgtcagtggaggtaccgcacggccgggctcacaggccacattaacgatcaggaatcctgccactttcgcgaaagatggtggctccacagacccgctgtatgtaatcgacggcgtgatccaggtgaccggcgacggtaaaaatgatgcggaacaattcaataacctcgacccctccgaagtggaaagcatcagtgtcctgaaagatggctccgcagcgatttatggctccagggcggcaaacggcgtagtgctggtaactaccaaacgcggccgcgcaggcgcgccccggatcagctacagcggctcctatggtatcaacgatgaaagctaccgcaccaaaatgctcagcgcctacggctatgcacagtatatcaatatcatgaacggaccctatggtgaaaataaagacaccacagatcagaacgcgtttttctccgccgatgaactggaacattttaaaacaattaaccacgactggctcgatcccgtgtggcaaagttcttccaacacgcgccatacactgaacatcagcggcggcacggagaaatccactttttttgccagcggatcctattattcacagaatggaaatttaagcagtctcgattataaaaaatggaccttccgcgcaggcggggatatcacggttgcatctggactgaaggtaggattgcaggtatccggcaactggtcggaccaggtaaggacctataacaaaataggcaacgaaaacgaggaaaacgactaccgcaacctgctcctcgcgccccgctatatcccgtcttacgtagatggctacccggtaaaaataccaggcagtgataaactctccggctatcatttttacgaaattgaaagattgaagaatctctcagaaacaaaagataaaacactcgcggtaaatgcatacgcggaatatgaactcccttttctgcaaggattaaaggccagggtgaactatgcgcgctactttaccgggacaaacgcttcacagataggcaccacctataagctctatgacttcaaccgtaccggtacaaacgcacatatctatgatgacggggccacggtgaaattacccggcgcaacatacgaaaatggtaaccggctttattactccaattcaaacggagaatcagaacaggtgaacttcacgctcaactatgcccgcgcattcggcaaacataatatcagcggcctgttctctgttgaaaaaggagaagcctatgtaaaacaggaagatgtatggaaagaaaagcccatagccggtaccaatggccagtttggcagcgctttcggcgccatcgatggcagaacatcaggagcagaatccggtacactgggttatataggccgcgttaattacagctatgcagacaagtacctggcagaattcctgttccgcacagatgcttccacccatttcgcacccgaaaattactgggggtcattttattctttgtcagccggctgggtaatctccaatgaatctttctttaaatcttctatagttaattatctcaaattaagatactccgccggcctgttgggtaaagatgatacaaaggcatggcaatggcggcagcgctacagcttccagggcgggaaaggagccgtgtttggcggtaatgcagatgtaacaacaggtatgaagatggaagcctcgcctaacaggaatgctacctggagtaatgagttcaaaaataatcttggtatagacgcgcgtttcctgcaaaaccgcctctcccttaccatggaaggattctataacaagggaacggatttattgatggaaagaaccgctacggcgcctctcaccgtaggcggaagtgtggcggcagaaaactggggcaagatggacttcttcggctatgaagtaagcctgggctggaacgacaggatcagtaaagattttagttatggtgtggatgcgcgtttttcctggtatgataacaaatggaaacagggaaatttcgccgccacagatgcttactatccctggaataaacaacagggacaatcggatgataacggcatgtggggatacgattaccagggcatgttcaaaacccagggagatattgatgcttatgtaaaacaatataacattacttccgtgtttggcacagaagcaaaagatctgaagcctggtatgttatactaccgcgatgtaagaggagcgctgaaaacagatggcacctttggaggaccggatggtgtcattgatgaaaatgaccagatccggctggcgaaaaaagccaataaccactacggctttggcttcacttttaaagccaattataaaggcatcggcttcgattgcgtaatcggtggctctttcggtggctgggcagaaattgacggtgattccagggagaagatggataatgccatcgaccggaacttccagagcagaccggcttactgggaagatatctacgatccggaaataaatcccaatggaaaatatccaaatccaaactgggaaagtattagtctcgaccgcgcttccaccttctggaaagtaagcgctttcaggatgggaatgagaagcgtgaacctgaattacagcctgcctccgcgcgttattaaggcattgcgcatcaataacgcccgttttatcttgtcgatgctgaacccggtacagttcttcaatccgttcgactataaagcagcggaaggcgcttatgatgtttttccaaacctgagaacttattctttaggtgttaatctgacactctgattcgtttacgaattgatctataacgttatgataaataaaatcatgaaatatagtaaaacattaatcgccaccgccttcgtgttgtcggcgctggcagcctgtaaaaaagacttcctcgaagagaagcgtgatctgggtggtgtaaatgaacaggtattccaggattctacactggcccaggcttatgtggactacatatacggtatgttcctgcctgcggggaatgcgcagtcgctcgcctggaacctcgctaccaacaacaaccagtttacgcaaacaacagaggaattgccaggtgaaaccaactggaacaaattatggccggctgtttcttacctgaatgcgcacgcactgccttatttcggcgtgccgcttgcgtcaggcgttaacaacaacacctggaccaggatgaagcagatcaacctgttcctcgaccaggtagatcaatacggcctgccattgtatacccggaacaaactaaagggacaattatatttctggcgcgcctggcagtacttcgaccttgtaagactttatggcggcgttccgctggtgttgcacgcgcaggaccccattgtaggtgcaggagaaaacctccagatcccccgcagcgccacctcggcatgtattgaccagatctctgcagatttagattctgccatggccatgctgccgggcaaatggccctccggcgccgattggggaagaattaccagtggcgcagcagcagccatgaagggccgtgtactgcttacctgggcaagcccgcagtttaaccgtaacaacgacaaggcccgttggaaaaaatcgtatgatgccaatctcgctgcgaagttgttactggaagccaacggatttggcttatacaaaacaggcaacctgcccgatggcactgcctgggaaaacatgttcctggcagaagccaacaaccccgaagccgtactcgtgtttggatttaataacgtgatctccgaccaggtgcagaaatggaacggatgggaaaatgcagccaggcccaaagagatatttggcgatggttccctgagtcctaccaaacaaatgctggacgctttcccaatgaaagatggtaaaatgccgggacaatcctcctacacttacgaggctaaaaagttttataaaaacagggatccccgtttttataaaacattcgcttataacggaagcatgtggccattcaaggaaaattcaaagtacaggctgtggacttaccgctggtttgccaatgcctcggctgcaacaccggcttccaccacggagcagcgcggcactaacagcagcggcgtgtatatccgtaaagcaactacgggtaacgccagcaatgcagtgggcaactttaaaaccagcggcaccgattttatagaactgcgcttcgcagaagtaatccttaacctggcggaaagcgccatcggcatggataacatcggcgaaggactggattatgttaaaacgatcagggaaagagcaggcgtggaaaacctcgatggcgcctatggcttaagcggtatcgctggcgctgatccggcttttgcggctgtactgaacgaaaggaaaattgaactggcctacgaaggaaaacgtttctgggacctgcggcgctggttgctgtttaataatgataatggcacctgtgcccgtttgggcgttccgcctttaaatggcacccgcagaacaggcatttttatctatgtaaaaaataccgatggtacaaaatataccggcgccaacaaccaggacccgctttatacaccgcaacacggcggcagcggcaaagtgctggcagatcgtgaaccggccgctttcccgccgggcatcaacaaccaggatgagtatgtagattacctgtatgataattattttgaggtgatagagaaagatgacctggacccgactaagaacgactggaagtttacctggtataatcaatattatttcttcggattaaatcaaacgattcttaacaatgcaccatacctggaacaaaccaaggactgggatggctttacaggtccgggttctttcgacccgcttaaataaaggaaatcagctttaacaacaaccataacaacaatgaagaacagaaaagtatttttgctggcagtagcagcaatttgtgtatcggtacaggcggcacaagcccagtaccccaccataccaaagcgcatacaggactccagcgaggcagcactgaaagaagcgcaacggctctcggacgaagcctgggcaaaagcattacccattattcaaaaagatgcggtaaacggtaaaccttacattccctgggctacccgcccttatgatctgccgcaggcagatattccagcctttcccggcgctatgggcggtggcgcttattcctttggcggcaggggaggaaaagtatacgtggtaaccagcctggaagaccgtggccccggcactttacgggatgcctgtgaacagggaggcgcacgtatcgtagtgttcaacgtagcgggtattatccgtctgaaaagtccccttattatacgggcgccttacatcaccatcgcggggcaaactgcgcctggcgacggtgtatgtgtggccggtgaatctgtttggatcaacacgcatgatgtagtgctgcgctacatgcgtttccgccgcggggaaacctacgttggccgcagagacgacgcactgggcggtaatcctgtcggcaatatcatcatcgaccattgctctaccagctggggactcgatgaaaatatttctatctaccgtcacatgtacaatgcaggagacggatcacaggatcagaaactggcgaccgtgaatgtaaccatccagaatacgatctccgctgaagcgctggatacctataaccattcttttggcagcacattgggcggggaaaacgccaccttcatgcgcaacctgtgggcctgcaataccgggcgcaatccctccatcggatggaatggcgtgtttaacttcgtgaataacgttgtcttcaactggcgtcaccgttctgcagatggatccgactaccgcggcatgttcaacatgatcaataactattataaacctggccctatcacaccaaaagatgaaccggtaggtcaccgtatcctgaaacctgaatccggccgcagtaagctcggctatcatgtatacggcagggcttatgtgcatggcaatatcatggaaggctacgataaagtaacaaaagacaattgggacggcggcgtacaggtggaagatgaagcaaatgcaggaccctaccgcgacagcatgcgggtgaacaaacctttcccgatgccatcgttcccgatgatgtctgcaaaggaagcatttgactatgtattgaaaaatgcaggcgccacccttcctaaacgcgatgccgtggatacccgcattgtagaacaggtgcgtacgggcaagatccagtataaaactaattccgctaccgacgtgggcagcgagttcctgaaacgccggctcgataaagaatcctataaagaaggaatcatttcggatatcagccaggtaggcggataccctgtgtataaaggcacaccgtataaagacagtgatcaggatggtatgccggatgagtgggagaagaagcacggattaaatcccaatgacgcatcagacgcatccaggctggctaacaacggcaacgggtacacgaatattgaacagttcctgaatcactcataattataaaacctcctgaatgggccttaaagcactttcttccagaacatacgtctctgcattctccctgctgatgttcatcacctgtgctaaaatacagcacgggtttgatgaacacggcggaacagaaaacacggaagcattacccgcttttccgggtgcggaaggctatggtaaatacgccaccggtgggagaggcggtaaagtagtggaagttaccaatctgaatgatgcaggacccggcagcttccgccaggcattcctggaatatcccgatgatcccatcaccattgtgtttcgcgtgggtggcatcattgagctgcattccgccattaaagtacagcgttccaacattaccgtagcggggcaaacagcacctggaaacggcatctgcctgaaaggtcattcgctcatcatgaatggtgcacgggctttgagcaaaggaggtaaccacggcaatattattatccgttacctgcgctccagacccggtgcaacgctgtccaccggcgtttacggctttgatatggaaaactgccacaacgtgatcattgaccattgctctttcagttgggccaatgaagaatgcgccgcgttatacgatacaaaatataccacggtgcaatggtgcatcgtgagcgaaggactttacaatgccggccatgcaaaaggcgtgcgctcctatggcggcgtatggggagggcagtatgcgtcttatcaccataaccttatcgcgcatcagaacagccgcaccgtaaggtttaacggcgcccgtgcgcacgatacaaccgcactggtggactatcgcaataatgtgatctacaattggggcagtgcaggcgcctgttatggcggggaagtggaaatacccggaggaaagtccaccgtaaacatcatcaataattattacaaaccaggtcccgctactgcggccacccgcaaatttgtggaggccagttataccgcggctaaagcgctgggcatcggaaaatggtatgtagccggtaatatcatggaaggcagtaccggtatgaccgcggataactggctgggaacagacctcgcaaagatccctgaagcaaacaggggggaagcccggtcagcggcgcctttcccggttacagccgtgttgccgctgcaaagtgcaaaggacgcctataacgcggtgctcgcgaaggcaggcgccacacgtccccaacgggatgcagtggatgcgcgcatcgtaaaggaaacacgcactgctactgccagtggcgcaggttcatcagggaagcccggcattattgacctgccggctgccgtgggcggctggcctgcctacacaggtgcagaggcgccggcagatactgatcatgatggcatgccggatgaatgggaaaagaagaacggctcagatccgggtaacccggacgacaggaatgtcgtaaataaaaaaggatacaccaggttggaaatgtatctgaacagcttgtaaataatacacgtgatattttaacttgtggaaccatgatcaatactttggagaattttattaagaagagatacctgctgttgtttggagtccttcttttttgccaggtagctgtatttgcgaggcaggctaacacgcccgacgacacagcttatatccgcaccaccaatcagcgggcggataaaattgtagccaccctgggcgttgctaatgcagatagcgccctgctcgtacgggacgtgatcgcgcagcaataccgttatttaaatgaagtccaggcaaagcacgaccaggaagtaaagttggctaaagaacaatttgccaatgacaaaccggctttaacgacacaactgaaaggaatagaagatgccactaaccagcaactgaataaagggcatacggggtatttggaaaagctgtcggcttacctgaccccgcaacaggtaaaccaggtaaaggacggcatgacctatggcgtgctgccgcttacctaccgcgtgtataatgatatgctgcccaatctcaccactgagcaaaaagcgcagatcatggcgtggctggtggaagcgcgtgagcatgcgatggatgcgggatcatcagagaagaaacatcaatggtttggtaaatacaaaggaaggatcaacaattatctttctgctgccggcatcaatatgaagcaggcggaagaggaatggaaaaaaagaagtgcagctaaagctaaatagttgcggctggcagatcaaaacgaccgaatgaataagcgcccgataattagtttttgtttaatagcaataagcgccgttactaccgtttacgcgcaaaagaaatccaaaccggtaccgccggtggcactgaatgccactggcaaactggtatatagccccgatgcacagggcaaccggataccggatttttcttattgcggttatatggcaggagagcagcccattcccgatgttccggttcgtatagtagtgcctgttataactggagatgccactgcggctatacaaaatgcgttggatgaagtggccgtgttgccgccggataaccgcggcatacgcggcgctgtgcaactgcagaagggcaactaccacctttcgggtggccttgtaattcgtgcatccggcgtagtgctgcgtggcagcggtatgggtaatgatggcaccgtgttaacaggagagggccgcgaccggcaaacgctgatccgtattgcgggacagcccggccgggtaacggaagcgccggttaaaattacggatgcctatgtgccggtaaatgcccgtactgtacaggtagcatcggtacaaggcttcaaagccggcgataaggtgctggtacaacggccgtccacacgggaatggataaacgaacttggcatggaacaccagggcggcggcattactacgctgggctggaaactggggcagcgtgatattgcctgggaccggacgattgttggtataaacggcaaggctattaccctggatgcgccgctcactactgcattggataccgcctatggaggcggtaccgtggcagcatatcagtggcccggccgcatcagccagaccggtgtggaacacctgcgttgccgctccgcatacgacaccctttaccccaaagatgaagcccaccggtggatggcgatcacgctggagaatgtctgtgatgcatgggtgcggcaggtaacctttgagcatttcgccggttcggcagtggccgtgctggaaacaggcaaacgcattaccgtggaagattgtaaatcactggcgccggtatctgaaataggcgggcaacgccgctatactttttttacttccggtcagcaaacgcttttccagcgcaactacgcggagtatggttaccatgatttcgcggttggcttttgcgcgccagggcctaatgccttcgtgcaatgcgaagcgcacctgcctttcagtttcagcggcacgatcgatagctgggcttccggtgtgctcttcgatatcgtgaacatcgacgggcaggccatccgctttggcaacctcggacaggatgcacagggcgccggctggagcgctgccaacagcgtattatggcaatgcagcgccgcccggatagattgttaccgcccgccaacagccagtaattgggcctttggctcctgggcacagtttgctggcgacggctattgggagtcatccaatgaacatatcaccccacgaagtttatactatgcacaactggcagaacggataggcgccgatgtgttaaaacgggcgcagctgctgccagtggaatccgaagcctccagcagcccggcagcagaacaggcggcggaactcactgcacgcgctgtacaacccgcggtggtactatcagactggatagatcaatctgccgtacggaatcctattcctgtaaaaatcaccggcgttaaaacagccaacggtaccggttatacgaaaccggcttctcctgcaccacccatgcacatcgcaaacggctggctggtgcgcggcaacaggctattgaccggcaggcactacgaagtaccctggtggcgtggcaacacacggcccgatggtatccgggaagccatgccggcgatcacccggtttgttcccggccgcaccggtaaaggattaactgacgacctgcaggaagtagccgcatggatgacaaacgaacactttgtatcgctggagcataactatggtctctggtacgatcgccgccgcgacgatcatgaacgcatccgccgtatggatggcgaagtatgggctcctttctatgaacttcctttcgcgcgcagcggacagggaagcgcatgggatggactaagccgctatgatctcaccaggtataacgactggtattggagccgccttaaacaatttgcagacctggcagatgaaaaaggactggtactcgttcaccagcagtattttcagcacaacatcattgaagccggtgcacactgggcggattttccctggcgcaccgctaacaatatcaatcataccggcttcccggaaccaccgccctatgcgggcgacaagcgcatttttatggcggcgcaattctatgatattacagatcctgtacgccgcaaactgcacaccgcttatatccgcaagtgcctcgacaacttcgcggataacaatggtgtgatccatttgataggagcggagtttaccggtccggttacctttgtagagttctggatagataccatcctggagtgggaaaaagaaacaggtaaaaaagtacttattggcctgagcaccaccaaagatgtacaggacgctatattagccgatccggtgcgctcagctgctataacggtgatagatatacgccagtggcattatcagccggatggcagtttgtacgcacccaagggcggacagaacctggcgccccgtcaacatgcccgcctgctgaaaccaaagaaaagcagcttcgaacaggtttacagggcggtgcatgaatgccgcgaacgctatgccggcaaagctgtggtgtatgcaggcagcgcatatgaggagcagtcgtgggccgctttcatggctggcggctccctcgcgggcattcccgccatagccgctggtggctttctggaagccgcagccactatgcaacccatagtactccccggttccccgcagggacaatgggcgctgggtaataacggcaatgcctatattatttataccaataacaatgctccggtacagcttgatctgagcaaagccggtgcgtgcagtgtttattggattagtccaacagacggacatctgcttaaaaaagaaaaacagaaaggtggtaaacaggtcagcctcgccagcccgcaaccgggaccggttgtaatctggatcgatcgtaaataaataaacaaactggatgcataagatcgctattatattttttattacgttgctctcggttaccaatgccatacatgcacaaacaggtcgcattaccaaactgggcatctcttccaacggcaggtattttaccaccggtgggaatgcgcccttcttctggctgggcgataccggttggttattgtttaataaattaaccagggaagaggcggaaaaatacctggaagaccgccgtaagaaaggattcaatgtcatacaggtaatggtggtacataatcttgagcaggtaaatgcttatggtgattccgctttgatcaataaaaatatagccaccccgcataccacaacaggcaacgctttcacagatactgcacagtatgattactgggatcatgtggactatatcgttggtaaagcagcggagaagggcttgtatatggcgctggtgccggtttggggctccaatgtaaaagccggacaggtaagcgaccaacaggcacgcatatacgctgcgtggctggcagccaggtacaaaaacaaacccaacatcatctggttgaatggcggagatattaaaggcagcgatggcatggaggtatggaatgctatcggcgccacgctccacgcacaggatcccggtcatctgctcacctttcatccgcgtggccgcacacaatcatcccgctggtttcaccaggcttcctggctgcagttcaatatgttccagtcggggcatcgccgttatgatcaggacaccagcgcaggcgacctccactacggggaagataactggaaatacattgaagccgactaccgccaaacacccgccaaacctacgcttgatggcgagccatcatatgaagggattccacagggattacatgattccctcgaagcaagatggaacgacaaggatgtacggcgctatggatactggtcggtgtttgccggcgcagcaggttatacctacggtgataatgccgtgatgcagatgcatgcttccaaggataaaaaaggaagctacggcgtaacagatgtttggtccgatgcgatcaatgcacccggcgcacagcaaatggtacatctgaaaaatttattgttgtcaaggccttactttgaacgggtgcccgatccatcactcatagcaggcgacgccggtgataagtataaccgcgtgatggctacccgcggaaaacaatatgctttcatttatacttataacggccgcaacttccgggtgaacatgggcaaaattgccggcgacaccgtgaaggcgtcctggtatgatccccgcaacggccaggtaacacttattggcaaattccccaacaaaggcatcgccagctttgatccgccaggcacacaacaggatggtaacgactgggtattaatactggacacgtatgttcccggaaaaaaagtatacctgttcacttctttccgggaaccggctaccgatggattacgtttgctatacagctatgatggctatcactggatgagcctgggccgctctttcctgcaaccgcaagtgggagaaaaaaagctgatgcgcgatccttctatagtgcaggggccggatggtacttttcatctcgtatggaccagcggctggaaaaatgaaaaaggttttggttacgccagttcgaaagacctggtacactggtcggagcaacgcgctattgatgtgatgacacacgaacccactaccgtgaatgtttgggcgcccgaactgttttatgacaaagagcagcaacaattcgttattatctgggcatctacgatcccgcatcgttttccccgcgggcaggaagacgaagataataaccaccgtatgtactataccgccacaaaagatttcaaaacattttctcccgcaaaattatttctcgatcctgggtttagcgtgattgatgccaccattgttcagcaggccgcaggtaaatatgcgctggtgctaaaagataatacccgtcccgaaaggaacctgaagatggcgttcagtaagcatcccacgggtccttataccaatgtctctgccccgtttacgtcttcttttacggaggggcctgctacggtaaaagtgggcagcgaatggctcatttattttgatgcttatggagagaaatattacggcgcagtaaagacaaaggattttaaaacattcaccgatatatcagaccaggtgcaggtgccggaagggcataagcatggttctatcttccaggtaacagaaaatatactggatgttttacagcaacccgccgccgataccgtaagatataccgggcaaacccgcgttaatgtcgattaccatcacgggcagctaagtcccgctatgggagtgcataacattcaggtgttgcgggccaatcgcgaacatcctgaaaaggccgaaggtaccggttatacttataaccacgcaccaatgctggcttaccggaaccacactttttacctggaatacctgagtgatgaggtcagcgaaagtgtggcgcccgggcaaacactacttgccacctccaaagatggttacaattggtcaaagccggccatcctctttcctctctataaaataccggatggcactaccaagcaaggctatcccggtgtggcgcataacctgtatgcggtaatgcatcagcgcatgggtttttatacatcaaaaaaaggacggctgctggcgttggctttttatggtatctgccttgatgaagacgaccggcccaatgatggacaaggcattggccgcgtagtgcgtgaaatactccctgatggcagctttggtcccatttacttcatccgctataacgctgcctggaatgaaaagaatacgtcttacccacactacagtgccagtcccgataaggactttgtagccgcgtgcaacgaactgctggcggatccgctggtaacgcagcaatggaatgaagaagcagacaggaatgatccgctgataccgcttaaaaaacaatacaaagccctcagctattatcatttgcccgatggcagggtagtagggctatggaaaaatgcactcaccgctatcagcaacgatggtggtaaaacctggcctgaatcggctgtaagggcgccgggctttgtaaacgccaatgctaaaatatgggggcagcgtactgcagatggccgctatgccaccgtatataacccttccgaataccgctggccactggctatttctgtaagtaataacggtctcgattacacgaatatgttgctggtgcagggcgaaatatctcccctgcgctataagggatattttaaggattatggtccgcagtatgtgcgcggcatcacagaaaataacggtacgcctcccggcggtaatatgtggatcacgtacagtatgaataaggaagatatctgggtggcacgcatcccggtacctgtaaccgataaagcaaccgcacctgtaaatgatgtgtttaagcagatgttgccggacacagcattgcagcaatggaacatctacagccctgcctgggcgccggtaaaaatggagcaatccgcaaacggcccggtgttggcattgaaagacggcgatccatacgattatgcaaaagcagaacgcttgtttcccgaaacgcagcgggtagtggtggagttttccattacccctgcacaaaataatagaggactcctgcatgcggaattgcaggataccaaagggaatccctgcgtacggctcatgtttgaggcggacagtacattaaaggcaaaggccggcgccaaatttaaaaacattctgaagtaccaggccggcgctacttataatatccgcattaccctgaacactgccacccgtttttataccgttaatataaatgggaaggatgtattgacgcaactcacttttgcgccggtgcaaagtgtggcgcgtatggtattccgcacgggtatgccacggcatacgccggatgcagataccccggcagaacaaacttttgatctgccacacggaggagaaccggagcagccggcgatattttatatcgggtcattaaaaacaacagatcccaatcacagctaaactattctgtcgaaaacaacgcttatgactatacgtattttttgtacaacgattttattgttcgctggtttactgacacaaggtcaggctggaaattatcgcgccggcattgtcaccgacgaatttatatttgaaaaagcagcatttccttcatgtcatgcttctaccatcgcggaaacgaagcagggcctcgtagctgcctggtttggaggcacaaaggaaggacatccggatgtgggcatatgggtaagccgtaaaaagcagagcggtgaatggactgtgcccgtggaagtagccaatggcatacagccaaacggtacccgctttccctgctggaacccggtattgtaccaggtacccggcggcgatttactactgttctacaaaataggtcctaaaatatccggatggaaaggatggctgattacctccaaagatggcggcgctacctggtccgcgccggaagccttgccggatggttatctgggaccgataaagaataaaccggtactgttaagcaatggtacattgctttgtccgtccagcacagaaggagaccgctggagagtacatgttgaatcaacaaaagacaatggtaaaacctgggagaaaacggcgcccgtggatggtggtgacacttacaatgccatacaacccagcatattgttttatccgggtggaaagctccaggcgctttgcagaagtaagaaccgggccatactggagtcctggtcaacggataacggccgcacctggtcgcctttagcacctattgcactgcccaacaacaattcaggaacagatgcagtaaccctgcctgatggccggcaggtacttgtttacaaccacgtactgccaccggacggattggccaaaggtccacgcacgccgttgaatgtagcagtatcagaagatggcaaaaactggagcgcagcattggtgctggaaaactcacccatcagccagtattcatacccggcggtgatttatggcgcggatggatttatccatatcgtttacacctggagacgggagcggatcaaatatgtgaaagtcgatccgaagcaactacaattgaaagcaattaaaaacgggcaatggcctgagtaacctgtaactactatgaaccgtcgtcattttttaatcaatacaaccgccgctattactgcgggactgctgtaccgcaaggtatcgttcgccgcagcgccggcagcgcaacgttataagattgctgtttgcgactggatgatcctgaagcggcagaagctgggcgcattccagttaacgaaagacattggcgctgatgggctggagctggacatgggaggtttgggcacccgtgaaacgtttgacaacaaactaacagatcccgcgatcgccaaacaatttatagcagaagcgcgcaggcttaacctggagatcagttctattgccatgtcggggttttatgcgcagtcgtttgcagaacggcctggtgtagaccgcatggtacaggattgtatcaataccatgcagcagttgcaggtgaaagtagcgttcctgccgctgggcgtacaaggcgacctggtacaacatccggaactgcgccccgctattgttaaacggttgaaggctgcggctgcacaggcagaaaaggcaggcgtggtcattggcatagaaaccgcgctggatgctgccggagaagtgcagttgctgaaagatattggttctcctgctatccaaagctatttcaattttgccaacgccctggaagcaggccgcgacctgcaaaaggaattgcgcatacttgggaaagaccgcatctgccagattcattgtaccgataaagatggcgtatggttgcaggacaacccgcgtattcatctccccaaagtaaaacaaacactggatgagatgggctggcgtggatggctggtgatagaacgctcgcgtaatgcacaggacccgcgtaacgtaaaatggaactttggcgctaacgccgcgtatttaaaatcggtttttcaacaagtgtgatcggcgtcatgaaaaaaatagtaactactttattgctgctcgccactattggcgcccatgcacaggaaacacagctttttgataacgactggcgcttccatcgtggtggcgcgcaaggcgctgataaagcagcttttgatgatacgcaatggcgcatcgtggatctgccgcacgactggagtatagaagatcttcccggcactgcgtcaccttttaaccgtgatgcggtgagccaggcaagcggcgggtttaccaccggcggtaccggctggtatcgcaaaacatttacgctgcctgtaacccagaaagggaaacggatacaggtacagttcgatggtatttatatgaacgcagaagtgtggatcaatggtaaacggttgggtaagcacccttacggctatacgtcgttttattacgatgtcactgaccgcgtaaaattcggtgaacaaaatgtactggccgtaaaggtcaggaatgaaggggaaaacagccgttggtacgctggctcaggcatttaccgccatgtatggttaaaggtgatggaccccgtacacgtagcgcaatggggcacttatattactacgccggaagtaaatgccgctgccgcaaaagtacatgtacaaactaaagtgatgaatgaaaccagcagcactgctgcggtgaaagtaatcacccaccttatggatgcaaatgggaaggaagtagttacggcgacggatacacgtgaattaacaccgggcgcggttgccacgtgggaacaggatctcgccgtacgcaaaccggcgttatggtcggtgcaatcgccggtgctatataccgcggtaacggaggtttaccgccagcaacaattaacggaccgtactgtcacgccttttggtatccgcagtattaccattgacgccgtgaatggtttccgtttaaacgggcaaccgctgaaactaaagggcggctgcgtgcatcacgataacggcccgctcggggcaaaagcctacgaccgtgcagaagaacgcaaggtagaactgcttaaagccagcggttataatgcggtaagatgcgcgcacaatccgccttctcctgctttccttgatgcctgcgaccggctcggtatgctggtgatcgatgaagcatttgatacctgggaagatggaaagaatcctgacgactatcacctgtattttaaagactggtggaagaaggatgtagaaagtatggtataccgcgaccggaatcatcctgccatcatcatgtggagcaccggcaatgaaatccctaaccgcgaaaagccggaagtagtggaggtggcaaaggcgctcagtagttttatacgcacattggatacaacccggttcgtgacctgtggtgtaaacggcgtcacggaagataaagatgctttcctcgcaacactcgatgtggcaggttacaactatgcaagagataagtatcaaacggatcaccagcggctgccgcaacgggtgatgtttgcaacggagtctttgccgctggaagcttttgactattggatgggcgtggcagatcatccctgggtgataggtgattttgtatggaccgctttcgattacatcggcgaagccagtattggctggttaggatattggcaggagcagggcttctatccctggaaccttgcgtattgcggcgatattgatgtttgtggttggaagcgcccgcagtcgtattaccgcgatgtattatggaaagaaggacaggtgtctgtttttgtaaaaccaccgcagccgtcgtttgccactaatccgcataaggtggactggagccgctgggaatggcatgatgtattagctagctggaattgggagaacaccgcacaaccattggaagtggaagtatattcctcctgcgaacaggtggagctgtcgctcaatggccggtcgctgggaaaaaaagcaaccaaccgttccaataaattcacagccacctggcaggtgccttaccaggccggcacactgaaagcaacgggttataatggccgtaaagcagtaagcaatgcagtattgcaaacagccggtgaaccggcaaagattaatatggtagccgatcgtatggctatccgggcaaacgggcaggacttaagttacatcaccgtggaattgcaggatgcaaatggtgttcgtcatactaaagcagacaaccaggtacactttgatgtggaaggccctggaactattgtgggcgttggcaatgcgaacccgctcagtaaggagagttaccagttgccacagcgtaatgcctggcaggggagatgcctggtgattgtgaaatcttccgggcaggcgggaaatattgttgtaaaggcatcagcatccggattgcaaagcagccaggtaagcattgcagtgagatgatgttatcgcagcattacctggacatctttttttctttcttcaggaaatactttcagggacaacagcttaccattttttaaaacgccttctaccgttgtgttgtaaggtgcatgcagtttaaaatgaacgtcccatgcagccggccatgccgggaaaagataaaggtgtttaccgtcgttttgcagcagcatttcctgcaatccgatcatgcctgatccaccctggttatgatccggtgtccagtcgaaacccggcccccagaaagccgggaagcgcgtgctggcattcttcagtttttcgatagtataataggcggcgctgtcggtaaggccgagccgggcgcagaaaatattgtcctgcttccagccaacggcgctgcggtgtttaaccgcggtagtatcatacaaccaggtattaattgccgtatccagtcctggttttccgatgccatatatgccatagggaaataccgggtatagctgcggcgtttcctggttgttgatccgctcccaggattgggccggcgcaatggtcgtgtagccattcacgttacgataggagagtaaggggatacgttgccggaacaactgcagttgtgtacgcgtgctgtcggaaagatatttgcctggtagctccagcatcctgctggtaacggtacttagcccggagatggtggtggccgaattataggtcatcttgtacgtttctgctgccgagccgggatataacaccaggtggccgtttccatccagtgctttggagccgcgtaaccttgcgaggtattgataatgttcatcaaaaaaagtaagacaactttctataagcggtatataccgtgaaatatctttcccgctgaagcgctccatgtccaatatcatcaggcaaaattcaagtacggtatcccactcatattccagccagttgttgtactctacgcctttatcaaaccaggagggccgtttccatccatattcactggcagcaggcaaaccaaaatattccatttgttcggtgaagcaggcgccgttatgtccccagtaaaactggctcctggtggtggcatttttcagcgcacgcaaatagaaatcaaattgcgcagtcatcatatcaaagtcgccgcttttgagcatgggccagtataacaggcgctggttctgcgcggtaaaggtgccgcctccccagttgcggtgatccggtgtaaaaggaaatttttcatttacaaataccgggtcatacgtaaaaagcccgccattgaatttcgtaggataagcgccatatgcattacagccaagcatgtagcggaacaactggtagttccggcccgcctgccatacggcattggcagtatcaccgcccataaaaatatagctcctgttccagtattgctgccaccatgcggtggtttgctgaaaggtggttttttctgctacgctggctatccgcagttgttcctgcagtcctttgtaccatgcttcctgcgtggatgtttgcgctgtatgcagcagcacattgatgtgatgcgactttgaaggacggatgctttgcagctgccaggaggtgtacgcggtgtttatatatcgcccggtatctgtaccggcgggctgcatatcactgccccagacgaaaccaccaaacgtaagtccctgttggggattccatagttgtgcctttacggagtccaatccctgttgttgtaccgtgaaatcaaatatcagcgcatcattccggttgcggtgataaaacaacaccttcctgtcatcaaaagtaacttcatcatgataagccgtaacggctaccggtgcgcctttataaccggagcatgccagcagctccatttttgacattacacggtcgcccgttctccagttttcatagtgcacggtggccgttaccggctgacgggtgttcacgtccacatgcactaccgggtgatgcacatctacccatacccggatctgcgcctgctgctttcctttactgccggtaatagctatgtagccttcccgcagatgcaatgtttgccggaattgtgtacctgcttcaaaaggattgggcattaattttattcttagcctgccctgcttcaaaaaggtactgttttcatcaaaggtgccgctgcgcgacaggtaacataacaattccccgttttccatccatacattcagtcctatgtcgccgccgccacaaggcatggattccgccgcattccggctctggctgttccaggtaatattgtggttgtccagttccgggagctgggcaaaagaaggagaggtgtgaagaatagcggctgtgataataatatatcggaaaatagttttcatacagatagtgagaagataaagttaacagaacatttcctattatgctataccaccgcgttccggcaacgattgcgtaaaaaaatacttttttgcatagatatttctgtagcttgattgcggtaaaggagaacagaattccatgttgatgaaaatatttacgcgtagccttttactatccgataagtgttacttacacaattatttaacggctgccatactgattccatttattttattgctgccggccacaacggtatgtgcgcaagcgcctgccagtattatcgactggggcgcagataaaatgctgaacacctacctgatgcagcaaatgcaccggcagtatgcggggcgtagtaaccgggtgcagcaggccatgcaatcagtttccagcgtacaggcttaccagcaacagcttcgtgcttcctatcgccagctgttgggcgtattgccggaaaaaacgccgttacagccaacggtcacgggtatactccgtcaggatggctatcatattgaaaagatcatttatcagagtttccccaaacatcacgtaacggccagtttgtatgtgccggcaggtaacggtccgtttcccggtgtgctattgttttgcggtcatgaggcagaagcaaaggctacgccctcgtaccagcaaaccgctatcctgttcgccaggcaggggtttatggtattgatgattgatcctgtttcacaaggagagcggcatcagctgacagacagcaccggccagccttccacaagaggaggcactacggaacatacgctgctgaataccgcagcagccctggtaggctccagtgtggccgcttatgaattatgggataatgagcgggggctcgattacctgctgtcccgtaaagaagtagataccaccaggatcggttgcctggggaattccggcggcggcacacaaaccgcttatttcatggcctttgaaaacaggataaaagttgccgcggtatgcagctacatcaccacccgtgaaagaacgtttgaactgtctggtccattggatggctgcgtgcaaatacccaatgaaggtaaatacggattggagatcaccgactatatgcacctgctggcgcctaagccgttgctggtactggccggcagatacgattttgtagactataccggcgcagaacaggcttacaacgaagcaaaacaatgttatactaccctgggagcaccggaacgggtacagttgttaactgtagacgacgggcatggcatatcgcaacctaagcgcgaagccgcagcccgctggttcaggaggtggttgtaccaggatgataaaccggtacaggaaggggctcttgccgtgctgccagctaccgcgctgaattgtaccggcagcggggaattaaataatagtatctccggagaaattaccctgcaacaacatttcctgcaaaccgcttccgcgctcgccgcccgccgtacgcaatttcaacgcacggctactaaaaaagcgtttacagatacattgcagcaattactgggcatccatgtccggcggaataaagtgcaggtggaacgtgccggcacagggcagcaacaggaatgggcgtacgaaaagttattgttgcgcagcgaaaatgaaccgccgcttccttttatactgatgcggccaccgggcaatagtgcggtgcaaaaggtagtgatatgcatgaacgatgaaggcaagcgcacactgctggacagcactgtcctcctgcaatcatacctgcaaaaaggttatgcggtgttattgcctgatctgcgtggaataggtgaaacggccgatggagctgcattcaatcatccaaaattttataacagggagtaccggaatgtgatgtcttccctgcatattggccggccgttgatcggtcaacgtgtaacagacctgttgctgctgctggattacctgcagtcggaccaggagtttcagaaaaccaggatcgatataaaagcctccggcgctacggcgctggtagccctgcatgcagcggtaatagatccacggattaaccgcctgcaaatagaccaatacccggattcttttatcacgatgatccgccggataatgaagaaggatcaatacagtaacataattccgggcgcattgcaatattatgatgtgccggatcttgtgcggatgatggataagcgtgtagcttttctgtaagcagcgtagcaactttttttaattctttgataacctgtcaatgtcgatcagatctcttttattacaaagcctaaccatactaagtgtggcatcctgttcgtccggcagcaaaaatgccgttccgccggaaagcctgcccatggaggaaatcaacctggataatacgaatgcttttacggcaacggatcaccattggcgtatagccggcaacgtatatgcggaccggcagcaaccgcatcacatggaaattgcagccggcaaaggcatcctggtgtgtgacctttccggaaatacggcagacagtacggagctgcgcactaaactggtacatggcgatcttgacctggagctggatttcatgttatctgctgatgccgcagcaagtattcttttccagggaaaatatacattgcagctgaaagacagctggttaaaagacagcgttacgaacacagactgtggcgccattgaaggaagaccgcctgtattgaacgcctgcaaggcgccgggtttatggcagcacctgtcggtgaaatataaggcattgcgtccttcaacaccggatagcaatggtgtttactccgcaagcgaaagcggctttgcatccgtggaactgaatggccgcgcggtgagccggttgcagatcattaacacacacgacaccgcattgcgtgatgtaccaggaccgctgcgttttatcgtacacaaaggcccggtggtcttccggaatatccgctataaaacctatggcaatgatcgcgcaaaattagcagatatgcgtttccgtgtgtataagggcgtctataaaaatcacgatacgctgcaacagctaacgcccgtaaaatcaggcagcaccgattcactgaccttccataccggcgataaacgcgcccacttattagtggaaggaaaactactggtaccggtaacaggccaatacatcttcaggctgcaggccggtggtcctgtgcggttaatgattgatggaaatgaaatcgccaacaacggcggtacccgcgactaccagcgcgctttttacggtgatactacgctggagaaaggaggacatacttttcaactcagctacgccaattacgacgaaagcctggtactgctgtatgaaggtccgcatattccctttaccgcccttactacgcctgcttctgaaaggatggcagaaatatcgccacagatggaatatcctgttaggaatgccccggcagtacaacgcggttttatagaacatcgcggtaaggttaatccatacagcatagcagtgggtatgcccggcggattgaactacgcttacgatatggttaactatagccctttaatgacctggcacggccggtacctggatatcgctgaaatgtggcatgaacgcggtgagaagcaactggaaaaacctttgggcgctgccctggaactggcaggtacgccgtctattgcggagttgcaggccccggatgccccatggccggactccatacgggaagacagcagcagctatactaaccgcggatataaactgttgccggatggattgccggtgtacctgtataccttgcatcaatggtctgtggaagattatctgcatccccgcagcgaccggaaaggattgatccgcgaggtgacggtaaccaataacggaagcactaacgggaacgcctggtggttaatggcaagcggcggcgtcatcgaaaaattaccggatggcagttatgcggtagatgataaacaatattatatagaaacagccttgtcgccgcagatcgtgcaaagtaaaggacaataccgtttgttagtacccctgccggcggatagcaaaaaggtgaacattcattattccattatctggtaaaaattatgataagcaaacaacataggtcttttttgttgctcgtgtggagtatgctgttaccctacatcgcagctgcacaacaggagatgaaggccagggaaagtaaatattatgctatcacagacgtgcccataccagacagcgtagcgctggaggttggaggtctcacatttacaccggacgacaagctgggagtggccaccaggcacggagagatatggctgattacagatccctaccagaagaaatcaaggtatccgcattacacccgctttgcagcaggcatgcatgaaactctgggccttgcctggcacaacggttccttttacactacgcagcgctcggaattaacccgtgttacagatacagacaaagacgggaaagccgatctctttcaaacggttgcctcgtggcctttatcgggcaactaccatgaatattcctacggaccgctgttcctgcccaacggagatatgatcgttacactcaacctttcctggattgggcgcggcgcaagccttaccaagtggcgtggctggatgatgcagataaaaccggatggcaccatgaaaccttttgccggcggcatgcggtcgcccgcaggttttggattgtcggagagcggggatattttttttgcagaaaaccagggcgactggatcgggtccggaaggatcactcaactggactatggcgattttgcgggtcaccctgcaggtatgcgctggtccggcgaatacggatcaccactgcatttaaagccgcagcaatttcctgactccatcggtatcctgcacgattttgcccgtaaaataccgcacttcaaggaacccagcgtatggtttccgcatacactcatgggcacttctacgtcagcagtcatcaacatcgactcagacgcatttggtccttttaatggccagctgctggtaggcgatcagggacacagcaaagtaatgcgcgccttcctggagaaagtgaacggcaaataccagggcgcctgtttccctttcctggaagggttttcgtcaggtgtgctgcggcttgtatggggaagcgatcattcgttatttgttggtatgaccagcaggggatgggcctctacagggccggctccctacggtttgcaacgggtgaactttaagggcaacacgccttttgagataaaggccatgcgggcgcaaagcaatggctttgaacttgaatttacatctccggtaaataaaaaacaggcggtgaataaccgcttattccaggtaacaggatttacgtatagctatcacagtaagtacggcagcccggtgattaacagtcaaccctgcgctgttgtaaaaagcgaagtatctgatgatggccgccgggtaaggatctatgtagaaggtttacgcgagggatatattcatgcgttggatataaccggcttgcaatcgcaggttggtgtaccgctgttgcataatacggcctattacacgctcaatgctattccggctggaagtggcggtatgcctggttgtgctataacacccaaaagcgcggcagccaccgccaataataatactgcctgtggcagtgatccttcgaaatgcgtaaatgtgcagccggccagctggaccaaaggtcccgatgtggtcatcaaaataggtaccctgccgggtctgaagtttgacccggctgaagtgcaggtgccggcgggaagcaaagtgaaactggtgtttaataataacgatgatatgctgcataacctggtgatcgtaaaacccggcaaaggagatgtggtaggaaaactggcgatggatatgggattgaatggttcccagctcgcctacgtgccgcgttcagccgacgtgttgtttaacacctgcctgctgcaaccggaaacatcacagggcatttattttattgcaccggcaacaccgggtaattacccttacgtatgtacgttccctgggcattataccgtgatgaaaggaataatgaaagttgtaaagaaataaagtgatcatgcaacgatttttctatgtttgtttatggatatgcgtgtcggccaatagctgggcacaggacaggaaagctgtattaagtacagataaactgaagaaatatgttacgctcttcaaccgcctggacacaggagaagtgaaacaatacatcccggatgaccaggcagctgcatggcttgaaagcaatgtgccgttatttgattgccctgataacgtgatcgaacaaacgtactatttccgctggtggagttttcgtaagcatcttaaaaaaactcctgacgggtttatcttcacagaatttattattcctgtaaaacatgcaggcagatataatgcactgagttgcgcacttggccatcatatttatgaaggacgctggttgcgcgatacacagtacgttcatcaatatatccgctattggctggagaaggaccagcagcaggccaaaccgcgtttccaccagttcagcagctgggcggcggatgctatctataattattatctcgtaaatgcggaccggaattttgccctaagcctgctggattcactcgataaagattaccggctgtgggagcaggaaagaggtttgcccgacggcatgtactggcagtttgatgtgaaagatggcatggaagaatccatcagtggttcacgtaaggaaagaaatatccgtcccactatcaatagttatatgtacggaaatgccagggcattgtcgcagttggccgctatggccgggcgcgacagtctccggcagagatacgtgcaactggcagcacagctcaaagccggtgtgcaaaacaggctttgggatgataccgccgctttttttaaggtgcagttggccaaaggcccgttgtcaggcgtaagagaagaaatagggtatatcccctggtatttcaacctgccggacgatcagcctgaatatgcaaaggcctggcaacagttgacagaccgcaacggctttaatgcgccctgggggcttaccaccgcagagcagcggcatccggcttttcgtacgcacggtaccggtggttgcgagtgggacggcgccatatggccgtttgccactacgcaaacactaaaagggcttgcgaacctgcttacgcgttaccggcatcatgatggcatcactgcgggtgtatatttccgtgcgttacaaacctatgcgcgctcccatcagaaaaacgggcagccttacctgggtgaataccaggatgaaaagaacggctactggctgaaaggtgatgatccgcgcagcagctattataaccactccggcttctgcgacctggtgatcagcgacctggtgggactgaaaccacgggacgatgaacaggtggagatatacccgctgatacccgccggaacctgggattggttttgcctggaccaggtaccttatcatggccgtttgcttaccatcctgtgggataaaacgggtaaaaaatatcatagaggaaaaggcttccaggtatttgcagatggaacgaaaatatacagcggaaccaatcttacacctgtactaacgccactgccgcgaaaaaaagcagcgttaacgctttggtatgaccaccccgctgctaaatggaccgccgcaatacccatcggcaacgggcgcttgggcgccatgatctttgggggtgtaaatgaagaacacctgcagttcaatgaagctaccttatggactgatggtccgcgtgaacatgcgcgtgccggtgcggtgcagtacctgccaaagatccgtgcactcctcgccgaagggcggcaaaaggaagcggaacaactggcggaagagcatttcatgggacagaaaagcgcgccgccggtatcccgctatgaggcggattatcagccgttcggcgacctttggctacgttttaaagataccctgccggccgcaacaggttaccggcgggaactggaccttgctaacgctgttgcccgtacgacttatactgccaataacgtggaatatacccgcgaatatttttcgagtgcaccgcatcaggccatcgtcctgcagctgtcggccaataaacccggcagcatcagcttcaccgctgctttgaaaagtccgcagccattgtattccacccggaaaataaatgacagcacactggcgctttccctgaaggtacagcacggcgtgttgaaaggagaaagctggctgaaggtgagtgtgtcaaacggacgtgtagccgttacagatagcagcatcacggttactaacgcgaacgcagctacgctatatcttactgctgctaccagttaccgcaattataaggatgtttcagcagatccggtagcgctgtgcaggaaggttatacagccgttatcatcttaccaaaacatacgctccgcacatatcaaagactaccagcagtatttcaataccttctcggtggatctgggcgagggacaaacgcagttgcctacagaccagcggatcagccggtttaccgcgactaccgatcccgcgctggccgcattgtatatccaatacgcccggtacctgatgatctccgggtcgaggccaggcggacaaccactcaacttgcagggtatctggaacgatcagatgtcgcctccctggggcagtaagtataccaccaatattaacctggaaatgaattactggccggcagaagtgttgcatctctccaaatgtgcggagccgctgttcgccatgacccgcgaattatcggaagcgggccgccgcaccgcaacggagcattacggtgctcctgggtgggtgttgcatcataacacggatttgtggagaggaacagcgcctatcaatgccgccaaccacggcatatgggttacaggcgctgcatggctgtgccaccatctgtgggaacattatctctatacaaaggataaagtttttttacagcaacaggcttatccgctgatgaaagcagcagctgatttttttgtaagtttcctcgtgaaagatcctgccaccggctggttgatcagcaccccttccaactcgccggagaatggtggcttagtagccggtcctacgatggaccaccagttaataagagacctgttccggaattgtatacaagccagcgaaatattgcaccaggacgccgccttccgtgaaacgttgcaggcaaaatataaacagattgcgcccaaccaggtagggaagcacggacagctgcaggagtggttgcaggatgtggatgacccggaaaatcatcaccgccatgtatcgcatctgtggggcgtgttcccgggtaccgacattacctgggatcaatcgccgtccatgatgaaagccgcccgccaatcgcttcttttccgcggcgatgatggcaccggctggagcctggcctggaagatcaacctctgggcaaggttcaaagacggcaatcacgcgcttaccatgatcaacaaattgcttactcctgcagagggccctaccggcaaagcacacggaggatcgtatatcaacctgtttgatgcccatccacctttccagatagatggaaattttggcggcgcttccggcatggcagaaatgattgtgcaaagccatatggattatattgaactgctgcccgcgttgccggatgcctggccctcgggacaggtcagcggcatttgcgccaggggtggttttgtattggatatccgctggcaacaaggccaattgcagcaactaacggtaacggctacttcagatggaccttgtgaattacgctataaagaacaacaggtgaaatttacggcgaggaaaggaaagcgctaccagctacaaatgacagccggccggttacaaatgatcaagcaatgatttctctatgaaaacaatttatctttttacagcattccttttttttacatacgctgtgcaggcacaggaaataaaaccggaagctacggaggactggtccacgcaaccgccgcaggtgacgcccggtaaaaatgcaggccccccttccgatgccatcgtgttgtttgcaggggaaaaagacctgggcaaatgggagcatgccgacagcagcccggtgaaatggaccgtaaaaggaagcgaactaacggtaacgcctaaagcaaaagatatccgtaccaaacaggccttcggcaatatacaactgcacatagaatggaaaacacctgatccccgggaagatcgtggtaatagtcgtggtaacagcggggtactgttcatgggactatatgaactgcagatatacgagaactatcaatatcttcataaaatctattacaacgggcaggcgggcagtatctataaacaatatgcgccgctggtaaatgcctgtttgccgccacaaacctggcaaacatttgatgtagtttttgaaaccccggtattcaacgccgaccagtcgctgaaaacaccagcctatatcacggtatttcacaacggggtattgatacaatatcatgttgctatcaaaggaccaatggtgtatgccggttacccggagtatcaatatcatgaaaataaattaccgctggtattacaggaacataacagccgcgtgagcttccggaatatctggttaagggaattctaaaaatcatccatatgaaaaaaatattttacctgctacttattatatgctccgccgcaggcgcaatggcgcagcaaacatatccctcgcggttaacggtggctaaagatggcagcggagactataccaccatccaggaagcggtgaatgccgtcagggcttattctcctgtaccactcaccattactattaaaaacggggtataccccgaaaagctggtcgttccttcatgggtaacaaacatcaccttcatcggtgaaagtcgtgatagcactattatcaccaatgatgattattccggtaagctggtgggagataagaagttaagcactttcaactcctacaccgtatgggtgcagggcaatgatgtgaaaatagaaaaccttacgatccggaatacagcagggcgtgtaggccaggccgttgcattgcatgtcgacggtgaccattttgtgatccgcaactgtaatctgcttggcaaccaggatacgctgctgactgctaacagcaacagctgccagtattatgagaattgtttcattgaaggcaccaccgattttatttttggcccggctacggcgttgtttcgtcgctgtaccatccgtagcctttccgattcctatatcactgccgcctctaccacaaaggaacaggcatacggctatgtattcctggaatgcaacatcacagctggtaaagaggccagcaaagtatatctcggcaggccgtggcgtgcgtatgcccgtaccgtttttatccgatgtgaaatgggcaggcatattttgccggcaggctggcataactgggataaaaaggaaaatgaacaaactgctttttacgcagaatataataacacgggagaaggggccactgttgcagggcgggttccctggagcaagcaattgagcgccagggaggccaaaagatatgtggcgactaatatattgggagggtgggatcctgttaacaaagaaaaataactggtatgaacatacgaaagataagcatcttaatggccgcaggcataggaatagctgtacacgctttttcgcagtactcctggacgcggttacctgaaatagcatctcctgtttttaagaaagatacttttaatatcacccgctatggcgcggttccggatggtattacattgaatacaacggcgatcaataacgcgatcaccgcatgcagccggaatggtggcggcgtggtgctggtgccggaaggactctggcttaccgggcctgtggtcatgaaaaataatgtgaacctgcatctgaaaagtgccgctacgctattgttcacaccggataagagccagtatgcgttggtggaaggtctttatgaaggccgttccgccgcccgtaaccaatcgccggtaagcggcagcaacctgcatgacatcgccattaccggaaagggtgtgattgatggcaacggtgatgtatggcgcgcagtgggcaaaggtcagctaaccgaaagtgaatggaaaaagaaagtagcgtcgggtggtgtacttggaaaaaatggaaatgaatggtatccgagtgagcaatacaaagcggctaaggaacaaggcatgagcatgctgctggtgccaggcaagctactggaggagtatgccgtgatgaaagatttcctccggcccaatcttgtagcgctgaataactgcaaaagagtattgctggaaggtgttattttccagaactccgctgcgtggtgcctgcatccttctctttgcgaagatctcactttgcgtaacctgctggttaaaaacccggcttatgcgcaaaacggggatggcgctgatattgagtcgtgccgcaactttttgatagaaggctgcacctttgatgttggtgatgatgccatttgcatcaaatccggcaaagatgaagaaggacgccggcggggcaagccaaccgaaaatggtattgtgcgtaacagtattgtgtataaagcccacggcggttttgtgataggcagtgaaatgagtggcggcgcccggaacatttttgtatacaactgtacttttgtgggaacggataaggggctgcgtttcaaatctacccgcggccgtggaggtgtggtggaaaagatctatgcaaagaatatattcatgaaagatattgtggaagaagcggtattttttgacctgtactacttcgtgaaatttgctacagacagccagcgggatgaacggccacaggtaaatgaaggtacgccggtattcagggatatggagtttgataacattgtttgtaatggtgcaaagaaagcaatttttatccgtggcttgccggagatgccggtgaaaaatatccggatcagcaatagtgtctttaaaacaactatcggaaaagaattaacggatgccgataatattgtgcttgataatgtgcggatggacacacaagtgccgcgggatacgtctttcgccgtttggagtacttatcagaaacaacgtttgaagtttccatttataaaaattgcatcgccaacgccgcccgccggtatgaagcaggcaatggatgtgccttatcgcgaagcaagcggtcgcagtttattactggatgtattttatagtaaagaaaaacagcgtaaacctgcggtgttactgatctttggcggtggctggcattcgggcgataaaacccataaccatgcaatggcagtggagctggtgaaaagaggatacgtagcagtatcagcagaataccgtttgtccggggaagcgcaataccccgcggctgtgcaggatctgaaggcggctgtacgttggatgcgcgctcatgccggcgaatatggtattgataccaatcacattgcagcactgggttgttctgccggtgggcagctggctgcgttaatgggcgccaccaacggcgcaccaaagtttgaagagggcaacatagctcattcctccgctgttcaggcggccattgatatcgatggtatcctggcattcaaacacccggagtcggcggaagccggcgcggcgtctgaatggctgggcggcacctatgaggaaaagccggagctatggaaggaggcatctgcattaacttatgcaggaagcaatacggttcccatgctttttattaacagctccttttcccagtttcatgccggcaggaacgacatgatgcgtgtactgaaagaacataagatctattcggaagcccatgagctgccggatacaccgcatccgttctggttttttgatccctggtttgataaaacaatggattattccactgcatttctgcagaaggttttcaggtaaaacagctactttaagaaatgaaacccggttattttatatcacactcagcttctgcgatatcagttctgttactgcattgatggctttcgggaaaaccctgcgcaaatctatgtcctggctggtcagcaattgttgctgcaatgttttcataaaaatattttttgtttctgtggccaggttcactttggtgataccgtttttaaccgcttctttcagctggtcgtccggaacaccggagcagccgtgtaatacaagggcagcgggcgtggcggcatggatctctttaagcaggccgatctgcagatgcggaggtgatttataaaaaccatgcgcggtaccgatggcgacggccagtgcgttaacaccggtttcttctacaaattgcttcgcctgttccgggctggtgaaggcagctgtttgttcctgtccgagttttgcaatatatcccagttcagcttccacattcacatcataaccagcggctacccttacaacggcagtggtagtacgaatattttcttcaaaagatctttcactggcatcgatcattacggagtcgaagccggcatccaggcattctcggatcgtgtgtatgttgctgccatgatcaagatgtacccatccggttacgccatactgacgaagcgctaccctcgccatgttaacggcggagttgatacccaggtattgcaacgtgctttctgatagttgcagtatcaggctgcagttggctgctttggccgccatcagcaagcctttcagtgtttcgaaattataaaaattcacggccagcaaagcggagcccgactgtgaacattgctgtagttgttgtttcaggttcatgctggtaggtaattaaatttttgaatggcaatagcgtggaaggtatcaagactatgaaaagccgtggtgcccccgggcgcggtggtgttaatggcgccggccagggcggcgtattcagcgcattgccgcaacgaacggttacggatatactgactgataaagcctgcattaaagctgtcgcccgccccgatacaatcggcaatgtctgtttgtttaaaggaaggctggtggaacagcgagtgaccgtcccacacataggcgcctgcttccccatgcttaaccgctacaatattggcataggcgctgatcgtttgcaggcaggaggaaacgctgttgccgccggtgaatgcacatagttcggcgatgttgggcagaaagacatctacgtggggcaataatgtggggaggtcgatatcccactgttctgccgggtcccattgcgggtcaagagaggtggtgagtcccagcatttttgcccgggcaaaaagccggcacagatcaggtttcagggctggttgtaaaaatacagagcttacatgcaggtgccgggcgtttgcgagcgtggcatctgtaatatctgccatactcagttcttccatagcgccggggtacgtgatcatggctctttcctgctcatgactgaaagcaatgctgatgccggtaccggcggtccggctatatacaatcccggaagtatccacgcctttcgaggatagttcggacagcactttatggccgaacatatcattacctattttaccggcaaaggtaacggcagcgccaagggtactaaggttgcaggcaaagatggcggcgctgctgcccagtacgaaggtcatgtcttttgcgagtatttctttgcccagagcgggcaatgtgttaagcttgttgagtatcaggtcaacattcagttctccgaccaccaatacatcaaacgttgtgttgttcatagcggtgtttttatcaggcattgagcggatagatggcaacaccttccacaacgcgggtgatggcgccgtttacggaaggattgtccggctgaaggcccagggataaagaagtaaaaaaggccagcagttgcaggggcaatatactgcatacacataacagatcttcctccagcagcaacggctgatcgcccgtgagcagaatggtatccagttcaggcacttcgccgttagccggcagtatacccatttccaggagtgccttgttaccctgcttcatggaaatgacgaggtccttttcataatttaaaacgtagctgttgttcgagaatatatatacgacgagggtgttttcatcgatgatagctttcgggccatgccggaagccgaggaaactgtcgcttttgcaaatgactttgccgccgctgagttcctgtagtttcaggtgagcttctgtggcagtaccgtaaaatgcgccgtcgcccaggaataccgcgcgggtaaattttttgccggcgatagtgcggagcagggccgtgtaacgggtgagcagctgcttcccataggtgcacagtacttccacttgctgccgcatggcggcgatgttatgcagccgggtgatcagggcgccggtaagcagcatgccggtatagctgctggtcatggcgaggctcttatcattacattccggtggcagcaggatcatgtgttgcgggtgttggctctgccagccggccagttgcccgctgtgattgcaggtaatgatcaggtggtaacagcgccgggagatgttgtctgccagttccagtgcagcgcagctttccgggctgttgccggagcgtgcaaaggaaatgatcagtggtatcctgtcggaatgaaaataatcgtgcgggtgcgctaccaggtctgtggtgggtatagccctggtgataacgccggtatggcggaagaagctgcctgtgagcgaaagaccaataaaagcacttgtaccggcaccggtaagaatgatgttgtccactgtatgataggcttcttccaggaacgccgacagggcagtggcttcgccggtcagcccgttcatgatcttttcccatatgtaaggctgttgcgcaatttcccgggcagtatggaaggctcctttttcttgcaatgcggaaggttccagttcaagtactgattgcatagttaagatataagtgagtaatacaatacaaatatatcaaaaggtaaattactttcaaaacctttttattatttcggttaacttgttttaaatttcgtttgaaagagattgcacaataatttgtaacttagctggcttgtaatagtaaaatctcaaaataaataactgcaaatggaagagagccaaaacggatcaactgtaaacaggaggaaagaaatactgcagaagctgtataaaaatggccaggtgatcatcagtgaactaagcaaagaatttaatgtaagcgaggtgaccatccggaacgacctggaccagctggagcagaagaacatgctgttacgggccaggggcggagctatcaagctggagaataatgtgggagtggatcagcggatcagtgaaaagaacaaaattcattacgtcgaaaaagtggcgatcggcaaaagtgccgctgccctcatcagtgaaaacgataccatgattattgattcgggtaccactaccgcggagatggtaaagcatatgcagtctttcaaaagcctgaacgtcattaccaatgccatgaacattgtgaacatgctttccggctatccaaatatcaatgtaatcatccctggtggctatctgcggcaaaattccatgtcgctcgttggtccgctggcggaaaagaacctgcgcagtttccatgtagataaggtttttcttggggtagatggctttgatacccgcaatggtatttatacgcccaatatggaagaagcctacctgaatgaaatcatgatagaaatcgccaacgaagtgattgtgctggcggattccagcaagtttaacaaaaagagcctggcatttatctgccctgtaaataagatccacaccgtagttaccgacgccggtatttccgcagaagataagaagcggctggaagacctggacgtaaaggtgattatagtatagcattcattttcccgcaagccggaagccgcaaagacgatcataaaatagtcgtttttgcggcttctgtctttgtataccccgatgccttcgtttcctttgttatgcatcttcaaaatctttctaaaaaaatatttatcacttgttttctatttaaaaaacttatatttactttgttttaaaatgaaaaacaaggtttcgaaggttaaggcgccttgaaacaacaaatatccgcgtatgcacaaatcccggctttggcttttatataccgctatcaatactgtatttgtaggagtatggggggcttttatagaaatacctgaaaaagccggctttccggcaacgctcggatatattgtgtggacgctgactatgctgccctgtgctatcgcagcgttgcggatagtgaagtggcaactggaacatacgccgcgggatattttcctggggtctatggtgggcctgctcggtgccggaggacaactcattcttttccaggcattgcggataggaccggcctatattttatttccgctcattgcccttttcccgctgctcaccatcctgctgtcggtggtgttcctcggggaaacctgctcccgcaggcaatggctgggtattggcgtagcgttgctggccgcatttttcctggcctttcagccaggacagaataaacaggcgcagggctacacctggctgatcatggccatgctcgtgtttgtgatgtgggccacccagggctttgtgatgaagtttgccaatagccgtatgaaagcagaaagtatctttttttatatgacagtgtcgtctttactgctggtgcccgcggccattggcatgacaaacttctccggcgccatcaactggggatggaaagggtttgggctggctgttcccatccacctgttaaatgccatcggcgccctgatgctggtatatgcactgcgctacggcaaagcgattattgtaataccgctcaccagtttatcatctgtcatcacagtcattctttccctcattatttatggagtagtgccggatgcggtgctgacagcaggtttgctgctggcagcggtggcgatcttcatcctgtctgaataaaaataaatacgattagcaacataactgtccgggcgtttataacgcccgcgactatacggagtattgattttatttattgttcaccagcagtgcataaaaaataaaagcactggaaaaacctcacataatgaccacgctaacatggaaaaaattccttatcgccccggctatgatagccctctttgccggatcatgtaaagttgatccaaaaatactgtctgcagaagcatcactcaccaaaggcgccctgctggcagataccgtgaaaattacggtaaacaagaatgctgtgctgatgaccagttcgctcaagctgggtgtgacctatatgaaaaataacctcgacgcctggggtgatggcccctccattaccaggggtaccaatttgctgaaaggagcggttgtttatcacaaccagcatatattcggtttcggtgcagataacattgagccaagacccggtgtatttgactgggaatcactggacctccgcgtaaacatgatggccgcgatgcaatcaacaccggtgatcactcttgccacggcccccacctggatggtagaccccgactgggcgccgggaaagtatgaagacagcagcgatacggattggagcaaagtggaatgggcgcctttaccggaacatgaaaaggattttgcccacctgtgtgcattggtagcgaaacgttatcccgcggtaaaaaccttccaggtatggaatgagctgaaaagtatgtgggacgagacgaataaccgctgggattatgtgcgctatacccggctgtataacctggtatatgactctgtgaaagcggcacgcccggatgccatcatcggtggtccgtatatcgggatagattcctggcatagtgcgccaggcaacgcccatagcggtatcacagatcccacttacggagaactggataaacgttgcctggatgtagtaacctattggctgcagaacaaacatggcggcgacttcctctgcgtagacggaggcgtggattcaaaagacggggttgccaccaacgtgatcgcctctacgaagaagttcagggatgccagtaactggctgcattcgcaaactacactgcctatatggtggtcggaagattatgtgggcctgaacacagataccaccattcagccggcagcactgggttgtatgctgatacaccacgcattggccggcgatgccgcatcactgcgctgggcgcccgaacagcaggaaggggaagggaatgtaagcaactttttcagcagtaccctggtgccgaacggaggcaaaccattcaggaattattcgctgtacaaaaatttcaacacctattttccggcaggcactaacttatgcgccactacggtatcagatgaacaacgggtgatggtcatgtcttccaaaacaaagatcctgatgatcaataaaacggcggccatacaaaaaacaaagatcaacaacacattagcagtaaacctgaatccatacgaggcaaaatatgttacattaccgtaacgcctatatgaaaaaacagatcaacagggaatatccgggtattccgggtattccccatctggccttgttttcagcccgtcgcccggtaccatgactaaagtattttatatcctgctgaaaaataaactgacattttaaaaacagatgattatggatctcgacaaagtaaaaccaaagccattagcagatgtttcgtcatcaccggaacatatcagattacaggactaccggccgaagtcgatatttaaaacgccggaaacagccattgtaaaagctgctttcccggtgattgatatgcatacccacgcatggcagccggagctggatgtaagcaaatggattgcccgcatggacgaggcaaacattgaaaaaagcacggttcttacgtttgaaaccggcgccggctttgatgccgttacgaagcaatatgcagattatgccaaccgctttgatctgtggtgcggattcgactacaccggttacgaccagccaggcgacagctggattgatcatgcggtagcagaactggaacgttgccaccggatgggagcaaaaggcgtaggagagctgggcgacaaaggtcttggcgaattttattcccggcctgtagccggatacggcctgcacctggatgatccgcgcatgaaaccactcttcgaaaagtgcggccagctgcatatgccggtgaatatacacatcgcagatcccatgtggatgtacctgccgatggatgctacgaacgacggattaatgaatgcatacgagtggcgcatagaccacactcagccaggactcctggaccatcccacactgataaagacctttgaaaacgtagtcagggacaaccccggtaccattttcatcgcctgtcattttgccaactgcacctatgatctcagcatagtagggaaaatgctggatcgttatcctaacctgtatgtagataatgccgcgaggtttgcagaaaccgccaccattccgcgttttgccaaagcattttatgaaaagtaccaggaccggctgctatttggtaccgacctgggctatgatcctaaaatgaatatggagtatgccgctaagttttaccgtactgctttccggattatggaaacaacagacgatcatttttatgaacatgaaatattcacttatcactggcctttatacgggctgggattaagtgccgccatactggaaaaaatttaccgtttgaatgctttgaagttaatgcagttatgaagaatcagccagcgatcaactatttacagactacctaataccgtaagcgtatgtatttccaatgtatgaagaagggcccgttgaccgggccgtcaaccaaaagacagcgcaacgacgctaaaagaaaatacctgtattgtcatgtgtgcctgatcctgttactgcttgttttcagcggacaaaaaagcgccgctgccaatgcgcaactgcggcaggatacgctgatccccgtctccggcctgatcacggatgaaaaaggaaatccttttcccggtgtaaccgtatacgtgccttccctgaaaacgggtactgccagcgatgccacggggcattaccaggtaaaggcacccgcaaaagggaacctcgtttttaaggccatgggatatgcatcgcaggaaatgccggtgaatagccgcagcaggatagcggtgaagatggaagctgaaaatgccaacctgaatgaagtagtggtaaccggttatacttcgaaacggttatcgcagatctccagctctgtggccgtagtttccgggaaacaattaaatgatgtcacctccaataacgtagccagcctgttgcagggaaaggtagccggagtggtggtacaaaacgcctccggtaatcccagtgtagccgctaacgttaccatccgcggatccagttctatcaccgccggttccggaccgttgtacgtggtagatggtatcattggcggtaccgccaacccgaacgatattgcttccgttaccatcctgaaagatgccgcggcagcaggattgtacggcgccagggcatccaacggcgtagtcatcatcaccaccaaatcaggccaggccggtaaaacacagatcagcctgaattccagcgttggcttcaataaaatgagcatgggcaatatgaagctcatgaacagccagcagctgtatgattaccagaaaagttattttgctcccgccgattttgcaagggatcgtcctgccagcttgctgtcgcagaacaccgactggatgaaccttgcttatcgcacagggcttacccagaatcacctgttatctgtatccggcggatctgaaaaaacgcagttttatgtctccggaaattattataaagaagatggtattatcaggcataccagtaacgaagtatacaacctgcgggccaacatcacccatcgcatcaatgagaagctgaagctaagcaccaggatcaacgcagcttcccgcaattttgaaaatgaagcttccgggaattacggcgcactggtattgtcgaaaatcaatttgccctgggataatccctataacgcagatggctccataaagatggggactgaagaaggatggataggccgggaacacgacaacttcctccacggatggcaattcaattatgataaaggaaaacagctgatcacctatgccgatatcaatcttgattattatatcacaccacatctcaccttttcttcgtataaccgtgtaagttattccaacctgcgaagtgaactgtattatgatgtgcgctccaaagcaggcaggggactgggggaaatgtataacaactccagctatgaaaacaggttgatcacctccaaccgccttaattaccagcgcacctttggcgaacacgcgctgagtgccatagcggtggcggaaggagagaagaactattttgaaaacaacagcctgtatggcaacaagatcccggcaggattgcatatcatggatgcagcggctaacatccagaagtcgccctttggccccggcagcaagtctgagagccgttttacaaaaggactggtgcaggtcgattataccttccgcgaaaagtataatctcatcggtgcatacatcaatgagtcgtcgtcccgctttggagccaatcaccgctcggcgggcttttacacattaggcggctcctggatactgagcaacgaatcgtttatgaaagggcaacggttcattgatcagctcaagatcagggccagctatggcattaccggtaatgcggaaatcggcgactaccaatcgttaggcatttatgcatacacctcgcagtatgcatccaacccgggttctgtgccatctgttttacaaaatcctgatctcacctgggaaaaatcaaagacaaccaacatcgggctggatatagacctgttaaaacgtatatccctgaccgtagatgtatacgataaaaccaccagtgcgctgttgctggatgtaccggttccttacaccagcgggtatgcttatgttacccgcaatgtaggctctgtgcgcaacaggggaatagagttcaacctgaataccaaaaatataaatggcgcccgctttaaatgggaaaccagcttcaacctttccatcaacaggaacaaggtgctgaagctgaacaaccatgaagacattccttattcatccctgcagtggatcagcgaaggccgcgatctgtacagctggcatatgcgcaaatgggcaggcgcagatccgaagaacggcgacccgctctgggaagtagtgagcacagacgccaacggcaagcaaaccattggtaccactaattcatatgacgatgccaccttgcagtacatcggcagcgcttcgcccgattttaccggtggtatcaacaaccgcttttcctggaaaggaataacattgagcgccttcttcaattttgtaaacagcaaccaggtatatgaagaaaacacgaacgatggcagcgagcccacttccaattcaagggtactgcctaaaaaccataacaggtggcagaaagagggggacattgccacagatcccaaagcagtatacggcggcaataaaaactctgacctggaatcatcccggttcctggaagatggcagctacctgcgtttgcgcaacatcaccctttcttacgatgtgccggaatctttcctgcaaaggataaaggtgaacaatgcaaggatatttatcagcggcgataacctctggacgctcacccgtttctccggtatggaccctgaaatgggactgcgcccgtattcgcagccggcaggagaaagcggtaacaatttccagcagaacagcaccaaatatccgctggcgaagaaagtcctgtttggtattaatgtcaccttttaaaaacagcagctatgaaaagaaatctctttaaatattatacactcgctgccgctattatagtcataaccggcagctgcagcaaagacctggagccttataacggtaaatcggacgatgcggccctggaaacgccggaagacctgcagacagccacctatggggtttattccgggctggtagacaggatgtacactaaaaacctcaaccagttgggtgaatatcctggtgatgatgtggcattaagcggcgctacgggcgaccaggtattttatacctatacctatactcatttcccgggaatgggaaacaccgaacagttctggcagggcgcttataaagtaatctattctgccaatgccattattgaaagaataaatgatggcacttccccgcagctggaccaactgaagggagaaaacctgtacctgcgggccatggcgcatttcgacctggtacgtctttttggaagaccctacccgcagggcgcgggcaacaatcccggcgtggtgatcaaagacaatacaaaagatgaccgccctgcgaggagttccgtaaaagacgtatatgcgtttgtgatagccgatctcaaacatgcagccacgttaatgaaagaaaataaaagtgcggcctttgcatccagagaagtggcggaggcgttattatcgcgtgtgtacctgtacatggaagataacgccaatgccctgttatatgccaataaggtgatcggctccaaccgttatcgcctgatggaaacccagccttataaaacgtatttccgcgtaataccggaagaaaatcccgagacgatatttgctatcaggcatacggtggcagatgaccggggtaaagatgcgatcggctccatgtactataatgatccggttacacaatccaccggctggggagaggtatacgcctctcttgcttttgtaaagctgctggaccagaatcccgaggatgtgcgccacagctttgtagagccacagcgtgatgcgaatgggaacatgcaattacgcaaccagacgccggtatattttatcaacaaatacaactggcaggaaggagtggctaacctgagttcacctgtcatcctgcggttggcggagatgtacctgatccgcgcagaagccaatgccaaactgggtaatgcgcaagccgccattgacgatgtaaacctgatccgccgccgcgccggtttatcaggtgccgcgttatatactaccggcaatctgaaaggtcgcgcgtctgtactggatgtagtgctggaagaacgccgcctggagctggcgtttgaagcacaccggccttatgacctgtaccgcaacaaccgtcccatggtgcgtgcctatcccggctttcatggcagcaatcaatatgatcaaaccatccagccaacagacccgcaggtgatcaattatattcccgaacgcgaaaccggccttaatcctaatctcactcagaatccatgatcatgctgttatattgtaaacgggtattggtgcttgcagggatctgctgcagcatgtcattagctgcgcagcaacccgcggtgctgaaagtagccgctaccagcgactttaaggtaaccggcgagggcagtcatccgggttggaccaaggcggcatggatcacgctgccgcaacgcagcgggcagtcgcctgcatcaacaaaagtaaaggccctgtattcacccaacgggatatacttcctcttcgattgcgcggaccaacggatcagcgcctccatgcaggcagatttcctggatctgtggacagaagacgttgccgaagtattcctgtggccggacacgttgcagccggcttattttgaatatgaaatttctccgctgaactatgaactgcctattctgatatccaaccagcagggcgacctggtgcgctggcagccatttcattatgatgccgacaggaaaacacagcacgccaccaccgtacagggaggcaaaaagaaaagcggcgctgcaatcaaaagctggacagcagaattctttattccttttcaactcctgcggccattgcaaaatattcctccccggaggggaactacctggaaggcaaacctgtaccgggtagactacgacaaaggggaagcggagtggtcgtggcagctgaccgggaagagttttcatgacatagaaaaattcggttacctggtatttgaataaaatcaatttttaaatttttaatagtatgaagatgatgaaacaattagtagcctgtatcttttttgttatgccggttattgcctttgcgcaaaagggcaagctggtatggtcggatgaatttaattataccgggcatccggatcccagaaaatggcgatatgaagaaggttttgtgagacatcgcgaagcgcagtattacacaaaaaaccgctacgaaaatgcacatgtggaaggcgggaacctgatcatcagggcgatcaaggaagagccgctgcgtttgatcaagggcggcaccagcttcgttacttccgacagcgggggagagtttacgtctgcctgcctcaacacggaagatatttttgaatttactaccggcagggtggaagtgcgggccaaactgccacatggcaggggcgtgtggccggctatctggacactgggtaataacatggcctggggtcccggtgattctacccaggtgtattctgaaattgacatcatggaatttgttggacatgatcccaacagcatccatgccaacatccatccgggttatgatggcggcagccgtggcggaaagatcaccgtggaaaaaccctgggagaactttcacgtgtatgccattgagtggtataaggaccggatcgattttttctttgatgaccagaaatatttttcttacgaaaagaaagatgtacccgaaggcaaatgggcctatcatgtgccacaataccttttgctgaacctggctattggcggtgactggggcggagaacagggcattgatcctaccatcttcccggcagattttgttattgattacgtacgcgtatatgaactgaaatgacgaaaaaaaatgaacatgaaaaaaaatgtcagccgcctgatagcggtgcttcatttgttgctgttgcccgtgatactgctcgcgcaaaaaggcgaccttaaactgctcgactggcagccacgcagtcagctggtagtgaaacaaaccagcgtgatgaagccgaagttcccggtgatagatattcacaaccacctgggcgaattaaaaaataccgcgcactacctgtcggagatggataaagccggcgtgataaaatgcgtaagcctggatgcttattctgccggtgataaatacctgaatcatctgaaggcttcacaagccgtatcaaaagacaggttcctcgtatttttccggcccgacttcggccggatcgatgaacccgattttggtataaaagaggggaagaaactggaagcagccgtgaagatgggcatccgcggtgtaaaaattgccaaggaacttgggctgatcataaaggacaaaagcgggaagctggtgccggtagatgatccgcgcatcgatcccttctgggagaaatgcggtgagctcggaattccggtactgatacacgtgtctgatccaaaagctttttttacgccggcagaccgctataatgaacggtatgatgagctgggcgcgcacccggactggtccttttacgggccgcagtttccctccaaagaggccatactcacgcaacgtgatcatatcattgcacgtcatcccaaaactatttttatcggcgcgcatgtaggcaacctgccggaggaactggagcgggtatccggttggctggataaatatcccaatttatatgtggagatttctgcgcgcatcagtgagcttgggcgacaaccgtataccgcgcgcgatttcctgatcaaataccaggacagggtattgtttggcacagacacaccttgtgatgcagcagcctatcgtatttattaccgtttcctggaaacaaaggatgaatatatagatccgtcgcccagtcatcatatgcaggcgcgctggatgatttatggattgtacctgccggatgaagtattggaaaagatttataacgggaatgcttcgaaaatactggggctatacaacgggggaaagtaatctgaacaattcacatgcgatgatcgatacagggatggcaactgccatccctgtttttatatttttagtgattgaagtttaaaacgctttcaccgtttcaatgataacagtaatatcgcccacacttttattgtcagtggacgtggcgatacagtgaagcttaaaccggttatcaacatacgcttcctgtttaacatgcagtaccactgcctccccggaaaaccccaggttatcggccaacaacgtcatttccctgacatacatttttaatgatttgtcagcggtgatgtgatgaatatacctggccgccaggtccagcagcgtattcatcaggatagccaccggcatcgccgggaagtgagggaaatgccctgcacaataattatcctggattttacctaatgaggccgccgccgataagccggaaaactgtacatcaaaaagtggtttcttttgatgatacggatttgttacgccgaaatcaggtgtttctttatggaaattgtaatacagccgttcgaagagggcatggggcactacatggaaactggtttctattccacagataagctgattgtcttcatccagcaggcaggcttttatgctagccattcttttactaaaaaaagtacacgtggcggtggccactaatttctttcgggtgtaatgtattttctccgcggcccttttataggttccccggtgggcaagatagtagtgtttttgttttactgggttgatcagtgcacaacatacggatcccaggatggcaagatgcctgcatgcttcagccgcggcaataggggagatctcttctcccagcggttgttctgcttctattgtggcagttacaaaattatgttcatccacacgtacctctttcagggcgtaatagggctcatgaacatctatcagtttaaagatctcctcctttgataatactttgattgaatttccggtatgggttaacttaatcgctttggattggatctccaccatatcgtcacttttaattgtttgcaggctttccatagtttatatgtttcggttttaaatggttatctgaggatgcaaaaggatatcaccaccaccggatgcgggtggtttgccgggctgcaaaaatgcctggtagtttacgtgtataggaggaactattcccgtatacggcaatacagcatataagatagtttttggaaaccggtgaggcgctccatggttattaattgagtaaatgattacaaacaactggtttttcaggtaacggtaaatgtcttatggtaatgatacttttacagcgggtaaacatgctgtattatgcagccggtgaaggatgcagggttttaggaatagctatttacggtcgttacataggattcagtcgatatttaaaattaaatagttttgtcaaaaaaccaaaatgaaaacccggcgggaatcagaatgaataaaatgaatagctgtatccaaataacatctgaacgtaatatatttgtccgattgacaataatttatgaaattggctggtaaaatttagtattttaccagcacagtgactgttcattatcataagcagatggatattctgtcgcggcaaccataataataaaagggagtccatcttttcaagtcaaccaataaatgccggttaccatcctgttgttcctttcatggcgaataatcctaattaaaagaaggcgctcattgactgccggcttcgtggttattcatttttttagtatatcatataagcggggatgcagttgattaaatcgtttgaacgtgaccaaccatatggagaagcagaactgctgcaacggcttgctgttgccgatgaagccgcgttttctgttgttttcagggaatactatggtgttttgtgtgctttcgcacaaaaaattatccaggaagcaggcgatccgaaagacctggtaaacgacgtgttcctgaagttatggaacaggcgccaggcatttgaagacgtccggcacctgaaggatttcttgttcaaatctacccgcaatgcgtgtttcgattccataaaggtggccattcacagtaaagaacgccaggctgtatttctcggcgcccaggccgactgggaaaccgctgcagatcttgaaatgatccgcctggaagtattcaatgaactttatcatgaaatcaaccagctgccggaacaatgcagcaaaattatacgcatgggttatatagaagggttgaaaaacgatgaaattgcccgtgagctggggttatctgtacaaacggtgaaaaaccagaaatcccggggaataatgctgttaaaacgcaggctcccgcctgaaatttttgtcattctcctgctgatgacaactcattcctgatttttttttggatgctttggtacggtaagaatatcacgtcgtaataagagaaagcgccgtgccaatatggatgaaccaacatcaaatgccttttatatagccgccctgctcagcaagcatttaaagggaaccctgacgccggaagaggcggtggagctacatgcatgggtggcggataacaagcaacaccagcaggtatgggaggaaattaatgatgccgccgttcaacaggcggcagtaaagctgatcgcccagtacaatgagaacgaagcgctggcgcagttcctggccaggtattcaccaaacgcacaaccagtccccggggagcgcgttcatttcctgcaacgatggagatgggcggctgctgcagcggctattatatttatggcaggcaccttctattggttccagtcccaacgaccggctcctgccggttttgccggtaatgcgccggtaaccgacatcgcacccggaaaaaatggtgctatcctgaaattagccgacggttcccgcatagcgttggatagtctgcaaaacggtgtggtggccacacagaacggcacccggatcttatttgataacggccggctggtgtatggccctggcggaaaagaaaacaatgaagttgcctataatatcattacgaccccgaatggtcgccagttccgggtaagcttaccggatggtacgcaggtgtggttgaacgccgccagctctatccgctatcctacggtatttgaaggtaagcaccggaatgtggagatcaccggggaggtatattttgaagtagcacaaaatgcgcaaatgccattccaggtaaccgtgccggataatgtccgtattgaagtactgggcacccatttcaatgtaaatgcctacgcaaatgaagaaagccagcataccaccttgctggagggcgctgtgaaagtactgtcgctgaaaccacaggcgtcagacctctaccgcaagggtattgtgctccgcccggggcaacagctgcaattgtcagaaacccccagggtgatcagcaatgcagacatcgacaagatcatggcctggaaaaacgggctttttgatttcgatggaatggatttgaaatatgcaatgaaacaaatcgcacgatggtacgatgtagagatcgtatacaaaggggctgtgcccgatattaaattttatggaaagatcagcaggaacataagtctggctggcctgatcaaaggcctgaacagcaccggggtacatttgaacattgaagaaggaaaaagactggtagtcacacaataatcatcatcataaaaaagatcatcaaacagggttagtcgaaaaaacaaaaagccggaagcagtaggagcgcttccggcaggtagccggctaaacttaaaatttcggtgtaacgaattttttatcaaccaaaccacaaccaaatttatgcaaaaaatcgctcatgtagaacgaaagggatttctattgccggtccctatacaaatattgcggattatgagaattactaccttcttcctcttcgcctccttactgcacgtttctgcaaaatctttatcccaggcggtcactatttcggggaaggatatgcctctgaagaaaatctttgacgccgtttacaaacaaaccggtttcgtggtattcagcaacgaccggttgatggaacgtgcgatccctattaccattaacgccagggaaatccctttgcaggagttcctggaaaacgtatttaaaaaccaaccattaactttttctatcgacagtaaaaccatcttcctctctgaaaagccttatcagcaggagtctgccacgctttcagattctacggtgattcccctgctgaaaggcaggatcctggattccaccggtttgccgataccggatgttacagtggcggtacgcaatacaaagctcatggccgttaccgatatccagggggatttctcttttgtaaatgtgccccggaacgctacgttggtagccactaatattgcttatcagcgaaaagaattaaagctggagggaagaagcgcggttacattccggctttatgcagacatcagaaaactcggggaaatacaggtagtggtgaataccgggtatcaggcgcttccacaggaacgggctaccggatcattcggcgtggttaccgggaagcagctggcacaggtgccggtagtaagcatcctggagcggttgcagggcatggtgccgggcgtggaaatttccaccaaaaccacggcgggtaaaagccgtaacgggtcggtaaaaatccggggcctgtctactattaaaagtgagtacaccaaagtaagtttagatcctttgctggtcatagacggattcccttcgcaagtgtctattgccaatggcgcgctggacctgcttaatccagatgatattgaccagatcacttttctgaaagatgcggcagcggcttctatctggggcatccaggcagccaacggcgtaattgtgatcaccacaaaaagaggagtacgtaacagcaaaccggttttcagtttctccactacgatgggtaccagcagtaaacctactcttggatatggagaaatgatgtcggtatcacaatacgttgacctggaaaaagaactgctggataaaggaagatattctgatccggttccccgtagcacaccgggaagctattatccggagaatggcagccaggtgcaggctatttatttcaggaacaaacgcggagaaataacagatgccgagatgaacgcacagctggcggcgttaggcgcaaacgacaaccgctcgcagatggaaaaatacatgatccagtcacccactacccagcaatataacctctctgtttccggtggcggagtaaacagctcttactttctgtcgggttatttttataaggaagaccgtgtttacagaaataatacgaacaggggatattccctcaaagcagggaacacctccagtttgttgaatggacgcgttacaatcagtacagatctgactttcgggaatacaaaggataagataaacaacgccgctgtaaaggcaatgagcactgtgtcgggcggtatgcggccttacgatatgctcaaagatgcatctggtaacaatatttattatgatctgctgactattccgtcaacagccaggtaccttgaaaacaagggatatcttccgtttcgttattctcccatcgacgaactgcagtattccaacagttataataccgctaataacgtggcattgaatctggcggtgaacggtaatatcacgtcctggttaggagttaatatttcaggaaatgtaggcaggatgtttacggaatacgagcagtactgggaaccggacagctacgacgccaggatgctggtgaataaggctaccagtttgagttccacgggcacccgtgtgtatggcgtgcctccgggcggcaggctcgatctgggcaacggacagggaagaagttacaacctgcgtgggcagatcaatgtaaacaagaactggaaagaccggcatcagctgaatttactggcaggtaatgaaatcagggaatcctatagtaaaaacagcggggaaatgcgctacggttatgataagtctatcaacgcttttcgcagtgtgaatccttttgtcggatatacagatatctatgggatcacgcagagtatcggcgccactaccaggccggtcacagaaaaaaccaccagggcgctgtcgtactacgcgaacggatcttacacattcgacaataaatataccgtttccggaagtgcacgttttgatgactataatttactgggtgtggaacggcgtaaaagagccatccctttatggtctgccggcgcgaaatggaacctgggtaaggaagaatttctccgtaatattacctggatagatcagctgtcggcacgttttacctatggcttcagcggaaacgcgccacagggttatgcgccggttactactatcaatatactcggtgctgactattataccaactacccttatggtgtgattgccactcccgctatggaaaaccttggatgggaaaaaaccaggatgatgaactggggtctcgatttttccctctttaaaaacagggtattcggttctgcagaatattataagaaatatacgacagatatcatctggcaactgccgatcaacggtacctacggttttatatctaccttatttaataccgccaacctggaaggtcatggggtggacctgggaatcaatgtagtgccggttctcagcaaaaactggagatggacagccaccatcaatatgtcttataatacaaacattatcaaagatccacgtttcgaaaaaccgactacttactttgcgccggagatgctttattcaggttatcccacagattacctgtttacctacgcctgggcaggattggataataccggtcagtcattgatttataatggtaaagaccgttcaaagaaatataccgtaaatgagtatccgtatgaaaacgtccgtgtctatgccgggcggacgacttctccctggtttggaagtttcagtcactcggtgcaatacaaaggcttcgacctgaacgtacagttccagtgcgcttttggtggtgttttcctgaaaccttctatccaggatatcggattcagtaataacctttttgtaggaagaaacggggacctggccaatcgttggagacagccgggagatgaagcttttaccaatgttccgggactggaattcggtgacaatacctctttctataccagctcggcccgttacagggaatcagatctgttggtaagaagccgcagtaatatcaaattgcagcaggtgatgctgtcttatactattcctgctactttactgggaaaagcaggactgaaaagcctgaccgtttcagcgctcgcacgcaacctcggaatgatctgggcagccaataaggagaagctggaccccgattatctctataccaccgggaataactaccagcttcctccattaaccaattattctttcagagttgcactgagtttctaattcattaaaccgaaaagtatgcgtcactatacaatagttattgtttttttattactgggtgccggcatggtttcctgccgtaaatatgtggaagaagtgcccatacagggccagcgtgtgctggtgtatacagaagactaccgcgctttgatgaataaccgggatcagcaggagagcgcctttggttcagccccgcttgtgagctgtgatgacgtggagttccgtgcgccggagatccaggataatattaaaggtaacactgttcaaacggccacctatacctggcgtaaacccgtttacacggatcttatgcaggacaatgactggaattccctgtatgccggtatgtacacttacaacgtggtaattgacggcgtaatggacagtaaaggaggagatcagctgttgaagcaaacgatcctggcagaggcgctgatgcaaagggcctttacctactttaacctggctaacctgtatggaaagcagtatgatgctgctactgcggaaatcgatcctgctgtgccggtattactaaaggcggctctttttgtggatttaaaacgggccacggtgaaacaggtatatgagcaggtgctgaaggacatcacggcggcaattcccatgctgccactcaaacaggatattaatttcaggcccaataaggcatcggcttatgcgctgttagccaaagtataccttaacatgcgcgacttcaccaatgccgctgcttttgctgatagtacgctggcgttatcaagtaccttgtacgactataatttagccgttgccggaagtacctattttttcccttcccagttcaacgataagcagatcctgctgcggaaagtgccccgtggaatgtatagcgctccgcagttaagtcaggcaatactggacctgctcggaacaaaggatttgcgctaccagctttttgtaaaaaccggtacttcgttttatccttcatttaccgggttgggtttctggtcgcgtgaaaaatattcaggcgccccggataagcccgcagtgggcctatccgtaaatgaaacctggctgataaaagcagaatgccttgcccgtgcaggcaaaacagatgaagctgtgggtatgctgaatacactccgtaaattccgtttcctggccgccgattatgcagaccttaccgctgctactgcagcagaagcattgcaactggtagtggaggaacgccgtcgcgaattcttcggcaccggcctgcgttggtttgatcagcgccggctgaacaaggatccgcagtttgctaaaactgttaccaggtcattcaatggtaacacgtacacattggcgcccaacagcagcggctacgtatttccactggccaatatactcatcacccagaacccggaaatggaacaaaatccatagactgtacatctgcaaaaaaaaattataaaataaatggcatcaagtattctcagaattgaaaagttgtcccaccggtacagtacttcctgggccatccgtgatattaatatggaaataagcccaacaggtattgtcggtttgctgggctcaaacggtgcgggaaagtcgaccaccatgaatattgtatgcggggcactgaaccagaccgaaggcgatgtttatattaacggcgttaacatgaaagagcatccgcaacaggccaaaagggatatcggtttcctgccgcagcatccgccgctttacatggatcttacggtcgatgaatacctcagctactgcgccggtctgcggcatttgccaaaagataaaatgaaaccctccataaaagaagccaaggaacgttgcggggtggatcatttcagcaaaagactgatccggaacctttccggcggttaccgccagcgtgtaggcattgcacaggccattgtacaccagcccaaactggtagtgctggacgagcctaccaacggactggatcctaaccagatcatagaggtacggtcgctgatcaaagaaatcgcccgcgacagggccgtgattttttcttcgcacatcctgtcggaagtgcagatactctgtaaagaaatcaggatgatcgaaaacgggaaaattgttttctcagatacaatggacacgtttaacaactatgtagaaccacacagtgtgctggtgcatatggagaatcccccggtggaagcagagctgttaaaaattaacggtgttacccaggtggaatttcttacagaaagacaattgcgcatttacttcaatggtgaacaggagatcacggaaaggatcattgctgtgtcggtacataatggctggcgactccgggagatcagccttgataaaagcgcactcgacgaaatatttaagcagttatcccatccatcatcaaaacaataacggattaatgaagacgatattcagaatagccaaaacagagttacgcaccctgttttactcacctattgcctggtttttaatgattgtatttctcatccaatgcggggcaacctacctcggcgtaatggaagccatcgcaagggaccaggatgcgggcgggaaatttttcggcagtgtaggagaatttgttttcctgagtaacaggggtgtattaggcggcgtaatgcgcaatttatacttatacattccattgctcacgatgggcctgatcagccgtgaaaccagcagcggcactattaaactgttgtatacttcgcctatccgggtaagggaaattgtgttcgggaaatttttggcgatgatgatctacagcttgttgctggtgatgatctttgggatctttgttacttccagcatgttccagattaaatcgccggataccggtatgctgttcagcgctatgctggggctttacctgttgctttgcgcctattcggccatcgggttgttcatgtcgtgcctcaccacttaccaggtggtggctgcggtatgcacctttgtaatgataggcctgttatcctatgtaggcacactctggcaggatattgcatttgtgcggaacctgacttactttctgtctatttcagggcgtacggggaacatgctgctggggctcattacttcaaaggatgtgatctatttcctggccatcgtttatcttttcctcgggctcagtatctataagctgaaagccggcatggaatccaaaccggctattgtaaaaacaggaagatatgcttttgtgatagtgtccacactggccgttggctactttagctccatcccttcaatggtgggctattatgacgccagccgtggcaagcaaagaacgctgacacccaatgcgcagaaaattataagggaactgggagatgctcccctggaagtgacggcatataataacctgctgggacgccactgggacctgggcagccccgattcatataaccggaacctgggccgttgggaaccctatacccggttcaaacataacattgaacttaaaacggttttatattatgattcatcctatgaaaatcccggtatgtaccggtactaccagggcaaaacgttggaccagatagccaagcaatatgcagatagcagggatctttcaatggatcagtttaaaacgccggctgaaatgcggaaggtgattaacctgaaaccggagttgaaccggtacgtaatgcaactgaagtataaagggaaaacgacgttcctccgggtgtttgatgacaaccaggaatggccgggcgaaacggaagtatcggctgcatttaagcgtttgctgcaggcaaaaatgcccaaaatagttttcctgacagggcacctggagagaagtataaataagctgggagacagggaatataaagtgctcacgaacctcactaccttccgtaactcattgctgaaccagggttttgacgtggatacactatcattggagtcgcaggatattcccactgatatctccgccctggtattggccgatccgaaggtggccatcacaacggctggtatggagaaattgcagcgttatgtaaacaatggcggaaacttgctggtggccggagagccgggcaagcaagccatattgaatccttttctgcggcagctgggcgtgcaattgatggatggtatattagtgcaaaccagcaaagacctgcaaccggagctgatcacgccttatctcacagccacggtcgcatcgttttatccggcgctggcgcatagtcaccacgatagcgctatggcttccatgccgcgggcaacagccctctcttatagcgataccggcgcattcaccatcaagccattgctggtaacggatataagaaactgctggctgaagaaagataaccttgtaaccgattctgcggaagtggttttcttaccggaaaggggcgacgagcgcaaatcttttgccacagcggtttccctgacacggaagatcaataacaaagaacaacgcattatagtgaccggtgatgccgatttcatgggcaacgcggagctgcagcgttttaatttaagagccgccaattttgtttttaataccgctttgttcagctggctcagttatggcgaattcccgatcgatagcacccgccccaagccggaagatacagccgtactgttaacaaaagaccaggtgaagttcctgcggattatttacctgtgggtattgcccggcatcctgctggcattcggcgccatattgctcatcagacggaaaaggaaatagtcagggatagttttaattttttataagatgatttttaataccgataagcaaacccttactgatctcaatatactggggaaaccgggagctgattccatctacactgtttttaatcataccagcacacgtggtggcgccgctgtgctggaagatatgttcaggtacccgcttgcggaaaaaaccgctatcaacaatagaagcggcaagatccggtttcttcagtctgttgatgcccgtttccccttcagcagcggtttgttcgacgtaatagaaggctacctggccgtgcaggacgaccggacccgtttatcgccggagggcaataccctggcaaggaaattcaaccacctgatagcggccgatactaattttaaaacggtcagcgatggggtccggtcggtgatagaaatgctgcaaacgctgcaagggttttttattgatatgacaaaaatgtccgctgatcacccatacctgccggatatcgctgaaatgaaaaaactcctgcaagacccggcactggagccggtattgcaggagccggcgggaactaaattgccttacgacaaagtagtagcctatgatcaactgctcaggttccggttcagaaatgaactgggcaaaatgttgtcgctgatctatcacttagatgtatatatcacggtagccaacgtggcggcacaaagaaaatttatattcccggttgcattggatgccggtagtcatcatatacggctggagggcgtttaccatccccaggtagcgaaggcggtgcccaatacgatacatattaccccggaaagcaacgtggtttttttaaccggcgccaacatggcgggtaagtccacctttatgaaatcactgggcatagccatgttcctggcgcatatgggttttcccgttcctgcggagaaaatggagtttgccgtaagggatggtatttacaccactatcaatttaccggacgacctttcctccggaagcagccatttttacacggaggtattgcggataaaaaagatcgccagggagctgtcgaaagccaggaacctgttgctcatctttgatgaacttttcaggggcaccaatgtaaaagacgcctatgaaggtacggtggcagttaccgctgcctttgcagaaagagagaatggtgtttttgtcatttcaacgcatatcaccgaggcgggagaagtgctgaaagagcagtgccgtaacattcaattcatttttctgcctacccgcatggaaaacaacaaacccgtttatacctaccggttagccaatggtattaccaccgaccggcatgggatgattattatcaaaaatgaaggtatcctggatatcattggcaaaaagaaagataaaaataaggacgtatgagttttctcgcagacaaacaaacgcttgatgatctgaacattcccgggaggtacaacaacaaatccatttaccgtatattcgacaacgttataaccggtggtggcagaaagttactggatgatatgttccggtatccgttaacagatcatcttgcgatcaatgaacgcagcagtatatttcaatactttgacagcaaccctgctgtactgcctttcagtgctgaatcattcagcatagcagaaaattatcttaccactggcgccagtgctaccatgccggccactgcatggaacatagtatacaggaagttacttaaaacagtgatccgcgataacagctatgagctgcttgtaacagggctgggaaaaacgatcacattgttaatagcctttcgtgatttcatttacaaattagccgaaccgggcgcctatggccctgttcaggaacaggtcgaaaaaatccggcagatctttaacgaccggcggctgctgtggctccggaaagaaacagatgtaaagaatattccgctgccaaagcttataaaatacgactaccagttaagaacaggatgcctggaggagatgaagactgtgatagacattatttaccagtttgatgtatatatagccgtatccactgttgcgcggacaaagcacttttgttacgccagggctttacccaaacataaaaatgtaatcaatatcagcggattgtttcacccctcagtggagcatgccgtgcctaacgatatttcatttcatccggcatcgaatgttgcttttcttaccggggcaaatatggcggggaagtcaacatttatgaagtcgtttggcattgccgtttttttatcacatatggggttcccggtgccggcagcggaaatggagttctctgtaaaagacgggctcttttctacaattaatgtccccgataacctggagcatggctatagtcacttttatgcggaagtattgcgggtgaaaagtgtagcggagcaggtaggagcgtcaaaagatctcgtagttatattcgatgagctatttaaaggcaccaatgtaaaggatgcttatgatgctacgctcgctattactgctgctttttcggaacacaggaattgtttctttattatatcctcgcatattatcgaagtgggcgaggccctgaaaaaacaggatggaagttaccgctttttatacctgccaacggtgatggaaggaaatgtgcccaggtatacttatcaattgaaagagggtattacggcagatcgtcatggtatgattattatcgggaatgaagggttaatagcattgatccgtaagcgggagtgagttttatgcacgatcataaatttacgatatgtcgtatattttttattaaatagttttgcttatgatgttgattatgagatgattgcgaggtggcatctttgttgtcttaccgggcggaaactatttaatttatgaaaccgtcaccgaatctgttatcaccggagaaccacgcattagtattaattgattttgaaggccagatggcttttgccaccaagagtattccgctcagtgaactgcgtaccaataccgccattgttgccggcgcttcaaagatctttaatatccctaccattgtaacaacagttgccgaagaaaccttttcaggccctgtatttcctgaaattgaagaattttacccacaggctacttccgggtacatcgaccgtacctccatgaatacctgggaagatgaagctgcgtataaagccattaccggcgccggcaaaaagaagctggtacttgctggcctgtggacaggcgtttgtattgtaggtcctgcgctgtcggccattgaagaaggctataccgtgtatgttattaccgatgcctgtggcgacgttagccccgaagcgcatgaacgctccgtgcaacgcatggtgcacgcaggcgttaaacccattaccgctattcagtacctgctggaattgcagagagattgggccagacaggaaacgtatgtagcagttaccgacctgatgaaaaagtatggtggttcttatggcataggcattcattatgcccatcatatgcttaaacactgatttcttctgtaaaatcctctaccagctttgcgagtttccaatttctgtttatggcaaaagtcagcaatgctgatcatgctcctgctgatcagccatgcaggtttcacacaatcatttaaagggatgcgttttgatgagaattatgcctacctgcgtgattctgcacccaccttttatcgccaggtaaaatatacttccctctccgctgaacataacatctatgtttctttcggcggatcggcaaggtgggaatatgttgattttaataatgaagactggggacggctgggaacaggtcacaataatttcttattgcagcgctacgaccttcatgcggatgttcacctcggagaacgcatccgggtgttcacgcagctgcgaagtgcctgggaaggaggtcgtaaaaacggtcccaggcctattgatgaagatcacctgaatattcagaacctctttattgatgcacagctgtataaacgtaacacaaacagccttactgtccgcgccggccgccaggagctggactatggcagcgggcggctgatctctgtccgcgaagggcccaacctgcggctttattttgatggacttaaattaatgtatgccgccgcaggttttaccgcagacgcatttgcaatggcagcagacaccgtgaacacaggcgcattcgacaataagatcagcaaacaggtaaacctctgggggctatatgcgaagcgtattttcccccgggctggtaacctggatgtgtattacctgggtgtccggcgggatctggcagttttcgaagatggagctgcaaaggaagtaagacatacactgggcagcaggctttggaaatatggcggcggcttcatttacaacttcgaggcggcatggcagttcggaaaatttggcgttgcggatatcagcgcctggactgcttccgcagatatcggctatatgtttgaatctgtgaaaggccggccaacgatcaatttacgtaatgactacatctccggagaccgtaacaaaggcgacggaaaactgggcacctttaacccgctgtatcccaaaggaggatatttcggattcagtccgcaaataggcccggtaaacctcattgatatccatccttatgctactgtgaacccggggcctaaactgctgttgcaggcagatgtggtattcaactggcgttactccctgcaggatggtgtatatcgccccagtggcaattttaacctggcaggtgcttcttcagcaaaaagatatataggtaccgcttacctcgcaagtgcagtatacacactgaaccggtttatttcgctgaatgccggtatacaatattttaagacaggcgcttttgtagatgatctgatcaaagatcataaagacggattattcatcaacaccaggattgcattcaaattttaacaggaaaataaactattcatcatgagaaattataagcgtaatggaagtctttgggtaacaaaagtaagaagcctgttgccagtaatttttgcgttgctgctgggaaccacagcatatgcccaacaagcggcaaccgcggataccactgtgaagacaactgcgatcggcacttcaaagatctggggaaaggtagatgggatcgccatcgagggattggtccaggggccttcagccgctgaatctcctttacaggtggcttgtgtgttcgagtacacggaaggggatatttttaatcctcctgcattgcccgccgcgctgaacggcatggttcatttggatgaggcgctgcacggtcaaattacagcactgcgcaaaacaggcaggtttgccgggcatgcattggaaacgattctgattacgcccgccaaaggcgcattgaaatccccgcgtttattattgattggtatgggcaaccggaataatttcacgcccgatcttatgacctccgtggcaactgtggccatgcgtgaagcactgaatttaggcgtgaccagtttttctttcgccagcgatatcaaagatggcggtatcgattcaccgacggccctcgttgcaggtaacgtcaccaaaggcattattgaggcatacagaacgcagctgtatctccataaaaataatttagccgccccgaaaaaaataaccaaagtaatactgcttgcaggccccgcatttttcgtcactgccggcgaaggaatcaaagaagccattgcttcatttcataactaaaactgacgacgatgaaaaaggccgatttaattctttataacggtaaaatccataccgtagaccggcaccagccttcagcaacagcagtggcgatcaaagagggcaaattcattgctgtgggagacgacgctacggtactgaacggatttcaggataccggcacggtattgatcaacctgaaaaacaaaagggtgataccaggattaaacgattcgcatatccatttaatccgcggtggcctgaactataatcttgaattaagatgggatggagtgccttccctggcagatgcattgcgcatgctgaaagtgcaggtggcgctaacaccatcgccgcagtgggtgcgtgtggtaggtggctggactgaattccagttcgctgaaaaacgaatgcccaccttggatgaaatcaatgctattgcgccggatacgccggtgtttattatgcacctgtacgacagggcactgttaaaccgtgcagcattgcaggcagttggatttacaaaagacacgccggcgccgccgggaagccgcctggagaaagatgccaaaggcaatcccaccggactgctgctggcagcgcccaatgcactcatcctgtatgccacactcgccaaaggaccgcggttgtcgtatgaacaccaggtaaattctacccgtcactttatgacggagttaaaccgctttggcatcaccagcgtgatagacgccggtggcggctttcagaatttccccgacgactataaagttatcagtgaactgaatgagaaaaagcagctgaccgttcgtatcgcctacaacctgttcacacaacggcctaaacaggagcgggaagactttgaaaactggaccagctccgttacccttcaccagggagacgatatgtatcgtcacaacggcgccggcgaaatgctggtgttttctgcggccgactttgaagattttctccagccgcggccggacttgcccgatacaatggaggaggagctggaacgggtagtgaggctgctggtagaaaaacgctggcctttccgtttacatgctacctataacgaaagtatcacccggtttttaaatgtttttgagaaagtaaaccgggagattccttttaacggtcttccctggatcttcgatcatgcggagaccatcgatgagcgcaacattgaccgtgttcgggaacttggcggcggcattgccattcaaagccgcatggctttccagggcgaatactttgccgatcgttatgggcctgccgcagcggcgcatacgccaccggttaaacaaatgcttcaatcaggggtacccgttggcgcaggtactgatgccaccagggttagcagttataatccatgggtagccctgtactggcttactgccggcaaaaccgtaggagggttgcaactatacggcgatgcgaacaaattaagccgggaaactgcactggaactgtatacaaaagggagtgcatggttctccggggagcaacaaaagaaaggcagtatcagggtagggcagtttgccgacctggcggtattggaccaggacttttttgaagtggatgatgaagcgatcaaatctattgagtccatcctcaccattgttgacggaaaggtggtatacgccaaagacgatttcgctacccacgcaccgccaacaatacctgtgttgcccgactggtcacccgtaaaaaactatccgggttaccataaagatgctgcggttgttgccaaggcgccagctgccgaagcagttgctgctgccgggatacatagctgcaaaggcagttgcgacgttcacgggcatcatcacgatattgcccgtaagagcaacatccctgttaacaattacaccgcattctggggggcatttggttgctcctgttttgcattttaacgcgcatattatgaacgatattatcatctccatactttactccgacctgggcagcacctggaataacgccgctatgctggtattccgctgcctgctggcactggagctgttcagggtacatggcatgaaaaaattccgcgtagtgaacgggcaaaaagagcatgtacccaatccgcttcatttaccggaaaagctcaacgcactggtggctacgttttcagatacggtagtgcctttcctggtaatgctgggcatcggtacgcggctggtaattctgccgacgattggagtaaccgccatcggttactttgtggtacaccgtaacgacgacctggaggtacgcgatgtgccctatatgtacacgctctctttactttttttactggcgctgggcgccggtacctattctttggataccttttttattgcttcaattatttaattaaaaaagatgattacacgtattggtattaaaccagaacacctttctgccgtagcccattcgctgggaaaaataatggcagacgaattcgttctctacaccaaaaccctcaaagcgcactggtgtgtaacaggacctgattttcacagcaagcacctgttttttgaatcccagtatgggcagatggaagaaatagtggatgatgtggcggaaaggatccggtccctgggtcattttccgccggcaacgctgaaagaatttttaagcctgacgcacctcacggagcagtcgagggaaaaaaatgatgcaacagggcacatcaaagaactgctgtcggaccatgaaagtatactgatccgcctgcgggaaaacattgacggctacgtaaccgcattccatgatgcaggaaccagtgattatatcacagggctgatggaaaagcatgaaaaaatggcctggatgctaagggcgcatcttgaatagcaaaaaaggttttaaacaccacaaaattaaaacatgacagaagctacacacaatatcaattgggtaacctttttacttgcatgggtggcgggtttttgcgataccgccacctttgtatcgggagatggcattttttctgcacacgtgaccggcaattttattgtgtttgcggcgcaggtggcaacgggtggcgatcacatggagtcctggatgaaactaatcacctttcctgtatttgtattcgctgtaatggccgccggatgggccgttgagaaaacgcagaaaaagtataaaatactcctcgtggagggcatcgtactcatgatttgcggaattggcgctatcttgcagcctatgctaacgggagtggaagagaaagtaatgatctattcaattgtgatgactactgcagcagcaatggggctgcaaaatgcttttgggaaattatttgccaaagaaacacacggaccaaccaccatgatgaccggcaacgttacccaggcctcgctggatctgggaaacctgatcaggaagggccggagcggcgatgccctggcgtggaaggatttccagggccaggtgttcaccatcggggggtttttagccggttgcgtgatcggcgcaataatggctaaatggctgggactcagtgctatcctactgccgggagtggccgttgttgtttgttatttgcagggagaggtgctggcgcgtaaatttgcgccatgaggaaaatgatccgggggaaaatatggatatggatgttgctgggactggcggttaccggggaagcatatggacagtccgttgcgggccccgaaacaataggccggttggttcaaagcagtaaaggagataccgctactatcaccgcctggatgaagcggggagaatcgttcctcgacaaaccggggtcactggagcctgatatgaaaatggctttccagatcgccggccaaatggaaaaattaagtaaggagctgagatacccggcaggacttgggctgagtaaactgttactggcaaaagcctaccgggaatccggacgttctgctgaaggcagaaagataagtgaggaagcggttcgccttttaagtgtttatggaacacccaggctaaaggcggaagcaatattggagctgggcggcagctattccaattcggcggaagaccttccaataaagatcagtttatacaagcagggcatcgatatttatcaaagcttgggcgacagtctttctgcggccaaacttaatgagttcaggggagatctgctgcagctgaacggtcagtatacggaggcgctggaagtactcacggccactttatccgtttaccagcaaataggatacccgcgcttacagggaatttattcgataatgggtgaaatcaatcacgagttaaacaatttcactcaatcgctccggtataatttactcgccgtggaagccggaaaaaaaacaggggatacaggaccggtgatgacgaccgtatataaccgtgttgggctgaattactatagtattaaatattatgacgaggcaattgattacttcaataaagcattagtactggcccggagtaaccgggacaccggcagtattaaaaccatgcttgtcaatattgcagacgcctgccgcaataggggcggatacaggagaagcctcgacaccttgttggttagcgcgcaatatgggccgtctgcgagtgaaacggaacggatgctggaaccaatgatttatatgaaggactatatggcgctcatggagttcgacaaagcagatcattacttcaggaacctggtaagcagctatcagcagcgcaggatacctgacagaaccagccagcttttgcgcctggcgattatttattacctgcagtcggtgggccgttataaggaaacgattccctatctccggagttatgcccactataaagatagcataccactggcgcttgtacggaaggtggaaggagagtacctgttttacagaactgattcggcaatgggtaatatttcttcagctttcagccatttcaggcaatataaattgctttccgattctttaaccagtgttgcccaggcgaaacaactgggagtactgcaattacagtttgaaaccaggcaaaaagataaaaatatagaattacttacgcagaaaagtgcgctgcaggaggtgttgttgcaaaacgagaaagtattccgcaatgcatttgccgcaggtgtagccatgctggtgcttttctccgcattaatgtataaccgttaccggctgaaaaaacgttctaacctggagctggaaagtaaacaacgggaaataaatgatcagaacgaagtgctgaaaaagctggtggaagaaaaagagtggttattgaaagaagtacatcaccgcgttaaaaataatttacagattgtgatcagcctgctcaatacgcagtctgaatacctggataacgcagatgcaatagctgctatccgcaacagccagcaccgcatgtatgcgatgtcgctcattcatcagcggctttaccaggttgataatctcgggaaaatagatatgaaatggtacatgggagaattgattggttatatgaaggagtcatttgaacaaacagataagatttctttcactacggaaactgatccgttgctgctcgatgttatccaggcagtgcctattgggctgatcattaacgaggccgtgagcaattcgatcaaatatgcgtttccgggagaccagggaggcaatatttatgtttcattgaaacgtacaaacgaagccggttgtttgctgctgatttcagatgatggtattggctttttgcaggaacaggatccggagaacacatcgctgggaatgagcctgatgcacggcctttccggtcagcttgatggcaatttccgtatatcggctgctgtgggagccggcgtaagaatcaggttatcctttcaatgcaggacctttagtaccataaacagttaaaacgcccgcaggatgagtttaaaagagaaaatactgatcgtggaagacgaatttatcgttgccaatgatctgcgtattatgctggcgaaagccggttataccatgtgtgggattgcttcttctgtagagcaggcccgcgagttaattgcgcttaaagatcccgactgggtgctgctcgatattacgttgaagacgccggtgtcgggaattgaactggcaaaggaattgtttctgcagaaaaaaccgtttttgtttatctctgcaaatacaaaccaggccacattggaagcagcaaaaacaacgcagccatatggattcctggtgaagcctttccgcgagcgtgacctgctggtgatgctggacattgcccggtaccgttatagcgcggagcatggtgttgctgaaaataatacgaccgttgtaagcgatgacgacaacagctttcccgacattattggtaaaggagctgcattgaaaaaggccctcgaaaaaatccgtgcagtagcccgcagtaacagctccgtattgctgctgggagaaagcggaacaggaaaagaacggtttgcgcaggccgttcacaaagcttccaaccggaaaaacaaaccactggtaacggttaattgcgctgccttgccgttggctcttttagagtcggaattattcggtcatgagcggggagcctttaccggcgccggtcagaaacggattggtaagtttgaacaggcgggtggaggtaccatcttcctggatgaaatcggtgaattatctttagaagcgcaggtaaaactcctgcgcgtattacaggaaagggaaattcaccgccttggcggcgatatgcccgtgccggtagatgtgcgggtgattgcggcaaccaaccgcaatcttgaaaaagaagtggccgaaggaaggttccggctggacctgtattaccggctgaatgtatttccgatagcgttgccgcctttacgcgaaagggcagaagatattccgccgctgacagcttactttcttaaaaagtttgcactggcattgggaaagcaggtaccggaagtgagtaaggaagccatgcaatcactgctggaataccgctggccgggcaacatccgggaattagagcatgtcattgaacggcaggttattctgacgatgaacaatgagatcactgattttgatttgccggtacacctggaaaaaaatccgggttccacctcctttgaaacgatggagcagatggagcggaaccatattatgaacgcattaaaactatgcaagggccgggtttctggcgttaatggcgctgccgaaatgcttgggttacctgcgcaaactgtatactccaaaatgaaaaaacatggaattgaatcgggttacaaatagtattattttttgaatgccgtcacatggaaaaagaaacaacaaggatagaagctttcagcgatggggttttcgccattgccatcactttactggtattggaactgcatgtgccgttgatggaagaaaacgggaaaggagattcgttgttgaaaaagctggccgcggaatggccttctttcctggctttcagcctgtcttttttcagtattttcattatgtgggtcaaccatcataaaatcttcaaacagatctaccggcgcaataccccgctgatgttcgccaacgggcttatcctgttcctggctacctgcgtttcctatcctacggcattactctcccgttactaccatacttcctccgttcatattgtagtggccatttataccgctttatttgtatgcattaacctggcattcaacctgctttggtggatcgccagccaggaccggcaactgttaagaccagacatcaccgacgacggtattaagcgtataaaaagaaattacctgtatggcatcccggtgcataccctggcctttattctctccttcgtacaaccaacagccgcattgtttctttgtgtggccttatggatctactgggcttacacttccggtaagctcgatcttaaaggaaaatagtttcacgcttccccgtcttctttgccggtaacaaaatgttcttttttaatgcctaaccgctgcatttttgatatcagggtagttgccggcatctttaattttgtagcagcgccattgggccctgaaattcttcccctgcatattttaagcaccttcagaatatactcccgttctatttcttccagcggcaggatcttaaaagctttgtcatttaaactgctttctgcaccaatttgctcaggaagctggatcattttaatgatgctcttattagtcagcaataccgcgcgttcaataaggtgttccagttcacggatattacccggccaggcataggaaattaatttttccattgctttttgggagatgcccgaaatttttttcccggagttccgggagaaccgttctataaaataagaggtgagggcgggaatatcttcttttcgtttccgcaagggaggtaaggtaatagggaatacatttaaccggtagtataagtcgctccggaagcggttttgcgacacttccttttccaggttcctgttggtggcggcaatgatccttacattcacactgatggtttttccaccacccacccgctctatttctttttcctgcaatgcccttaataatttcacctggagctccggtggcaattccccgatttcatcgaggaacaaggtgctgttattcgccagttcaaacttcccgatacggcggtcggacgcaccggtgaaacttcctttctcatggccgaataattcgctttctatgaggttcgccggcaatgcagcacaattcactttgatcatgagcttcccccggcgcggagacgcctcatgtatggcacgggcaaccaactccttgccggtgccggtttccccgagtaaaagtacggtagcatctgatggcgctacctgcgaaattaaacggaaaatcttctggatttcaggtgaatgaccaatgaagcctgaaaagcggttggccgattgttcggctatcaggtaagccttttcttcttccagctgttgccggtaccggtctatttcctccatctgctgttctatcttttcattggccagcacattgcacataccagttcctaaaaggtctgccacaccagccagcaggttgaatttttcagatgaaaaggcgccttccttatttgagtaaagaaataacacgcccctgtcttcattggcattggtgattttaaccagcatcatttctttgatgccgagtttaaaccaatagtgaacatagggagcaatatctttctgttgggtgagtgcagcaagttgaaaaatcaccggctgatcagcggacaacgcgaggttaaaaaccccgtcattcacaggatgctggcggtgaataatgggactgtccaccttaccattttccagtttcttatcccggctatgcaaaaacggatagtgcgtcgtagcgtcttcagacaataaacataaagtataatactggctgttaaacaggtccagtatttcattattgatgatatcccacaggtcggcccggctgcgcaccgcagcaattctgccggctacgcaaagcaaactggcctgttcattttctttttgaataagttgattttcaaagatggcattcttgtccacatgactgccctgttccatatccaccggacccgtatgattggttttctgcatcatcgaaagtactgaatttcatagagccggacaagaaagcgatatcataatattacgacatgtcgtattttttaaaactaattaatttcataagaatttgattgttaattgattaaagctgggcacaccgtttgacttgcctgggcaaaacaaaccaataactatgagcacaaaagaaactacacagcaggtgcctgcggtagcaaatgatccggccatttcaaaagacgtcaaagcttttttaagtgtgctgaatgtaccgggtgcaccgggactggaaacactttccgtaagtgaagcccgccaggtgctgatcaatgcgcaggcggctgcggatgttgattattccggtattgaagaaagtgaaaagacgatcagcgccggtggtttttcgatcaaattaaatatcgtaaaaccagcaggaaacaaagaacaactcccggtattcattttcatccatggcggcggctgggtattgggcgattatcccacacataaaagaatggtaagagacctggtggtgttatccggtgcagcaggcgtttttgtgaattacacaccgtcacccgaagcccgctatccccaggcggtgaatgaaatttatgcagccaccaaatgggtagcggagcatggcgctgaaattggtgtggatggcagtcgccttgccattgtaggcaacagcgtaggtggcaatatggctaccgtaacagcgattaaagccaaagaaaacaaaggacctgagatccgtgtacaggtgctgttctggccgattgttgacgccggctttgaacatgatacctacaaaagattcggacaggaccgttttctgaccacgcctttaatgaaatggatgtacaatcagtacactacggatcctgcagaacgtgagcaggtgtacgcatctccacttaacgctacgatcgatcagttaaaaggacttcctcctgccttaatacaggtagccgaagcggatgtgctccgtgatggcggtgaggcttacggccgcaaacttgatgaagccggcgtagcggtaaccaccgttcgatacaatggaatgatccacgacttcggattactgaatgctttggcaaacattccccaaacaaaatcgctttttgtgcaggccgcagcagaactcaaaaaatacctggggttaaagtaaaagatcgccttttatccattccatcatctttataatatcataacatgagtgcttcttctgtaaaaaatatcgttattgtacacggcgccttcgcagacgcttccggctgggaagctgcctacaatatcttaaaatcaaaaggatataatgttaccctggtacaaaatcctacctctacactgaaagacgacgtgcaggcgaccaacgttgcgctggaccggcaggatggacccaccgtgctggtaggtcattcctggggcggtactgttatcactgaagcgggcgtacatcctaaagtagtgagcctggtgtatgtggctgcttttgttcctgatgtcgatgaatcaacgctggcccttgttcagtcggccccaatcctggaagtaaatggtattctgcccccggatgaaaaagggctggtgtacctggataaggataagtttaaccaaacatttgccacggggcaaagcaaggagaaatctgacttcatgtatgattcgcagattcctttaaccgtgacagccttcgttgataaagtaaccgcggcggcctggaaaactaaaccttcctatgctattcttcccaccgacgatggcaccatcaatcctgtactggaaagaaccatgtatcaaagggcgggcagcaaggtagtggaaatgaaaggtggtcatacactgttcatgacccatccgggagaagtggctgacgtgattgtagccgcttccatacttcagtaaacctgctgaaatcatctttacaaatttaaaaagaacattatgaaattaactttatcagttgctgcagtcctcgtgttttcgctgatgactgccgctacttccgctcaaaataaaccatctgccagggctgaatacatcgaggtagagcccaatgtaagattgcatgttaccgatctcggggaaggaacgcccgttgtgcttattcatggatatccattgagcgacgcctgctgggaataccagtaccatgccctggtaaaggccggctaccgggttattggcattactttgcggggatttggtttatccggcaagccttatggcaagtataactatgatcagtttgcaacggatattaaaacagtactcgataagctaaacattaaagatgccattcttggcggtcattcgatgggcggagcgatatcactgcattatgtcgccaaatttaatgcggcgcatgtaaaaaaactggtgttgtttgatgcggcagctccctgtcacacaaagaaagcggattatccttatccgctgttcaccaaagatcagatttccagctggattgagttgcacaacaacaaccgcccggccttatttgatgccgtagcggcaaagttcacgctgtcgccaacttcgctgacaccaggtttgggtaactggctgggaggtattgaagcacagtcttcgccatacgccacagaacaggcgcttattgcactccgggacgaggatctgcgatcagacctgcccaaaataaagatacctacgctcatcctgcacgctacgcacgacagcatcgtgtcgtacgcattggctgaacagatgaaggcaggtataaagaatgcaacactggtgccttttgagaaaagcgggcatgctgcatttatcgaagaaaaagataagaccaatgctgagttgatcaaatttatcaaagaatagcaacgtagttaatgtaacggggacaagccattgggcgtagtccccgttgcattaaacatcttctctgattgtgaaaaattctgccgggtttacgatatatttattataattgcagcactggttcctccttaccagcgtacgcgtatggttaattatagcaattattccgatcctgatctggtcttattacttaaggaaggagaccggaatgcctttgcagaaatttatcaccggtataaactggtacttcaccatcacgcctggaataaaacccgcaacgacattgatgcgcaggatgtgatccaggagattttctctaatctctgggtaaaaagagaggccattcagattgaaagtaatttatcaggttacctgtacagcagtgtgaggaatcatattctgaacctgtttgcgaaaaaacaacttcagcagaaatatattgactccatacaacattattcccaacatggaacggccgttaccgatcacaaggtgcgcgaatctatgctggcagcggcaattgagaaagaaatagccgaccttccgccaagaatgcgggaggtgtttgagctaagccggaaacagcacctgagccataaacagatcgctgaaatcatgggcactaccgagcaaacggtaaaaaagcaaatgtctaatgccttaaaacatctccgtaaaaaaataggtttctttgcttatctctacctgctctggatgctaaagcactaagtggggatggtccgcttaaaaatatttttctcccggctataccacttatagtcttcctgcctgtcttatgatgtataaagcacttttttaaagctaatcatcagaaaattggacaacagcattgtaaaagtatcacacctgtctcataaatacagccgggactgggccatacgcgatatcaaccttgaaatcagcaagctgggcgtactgggcttactgggttcaaacggcgccggcaaatcaaccaccatgaacatcctgtgcggggtactgagccagacagaaggtaccgtggagatagatgggattgatatccggcagcagccggaagcagccaaaatgaggataggcttccttcctcagaatgccccgctgcaccttgatctgacggttagtgagtacttaacgtattgcgcttacctgcgcaacatcgataaacggcatgtaaaggtggcagtagcgtcggcgatggaaaaatgcggggttgcccatttccgcaaaaggcttatcaacaacctcagcggcggctaccggcagcgggtgggcatcgctcaaagcatcatacaccggcccaaacttgttgtgctggatgagccaacaaacgggctggatcctaaccagatactggaagtgcgcaagctgatcaaagaaatcgccacggaaagggccgttatcttttcttctcatattttatcggaagtacaggctacctgcgatgatgtacgcatgattgaaggcggaagaatggtatttgcggataccatgaaggctttcaataattacattttgccaaattccctgcgcgtttatatgaacaatccgccgccaattgaaacaatggcggccatccccgggatcacccatgtagaactgctgaatgatggtggtttcaggatgcattttgacactacttcattggtgtcttctactattattcaactcgccgttgacgataactggcagctcacagagatcatgctggagaaaagcagcctggacgaaatttttgcacagttatcaaacaaaacttcctgaacctgttatgactaaaatatttaaaatagctaagctggagctcagcgtacttttttattcccctgtagcctggctcgtgctggtgatttttatggtgcaatcagggatgggtttctttggaatgctgggcagtttccaggagttgtttatgatgggagaaaaagcagataatttaacgcagcttctctttcccgctaccaatggactgttcgacaaagtgttgcaaaatctttatttatatatcccgctgcttaccatgggactgataagccgggaaatcagcagcggttctatcaaattattactatcgtcgccggtaaaaatcagtgaaatcattttgggtaaatacctcgccatgatttattacgcgctgatgctgatggctattttaggcatttactgtttgattggtatgtgtgtgattaaagatgcggatgctggattgatcggcgctgggttgttgtctttgttcctgttaacagccacctacgcggctattggcctgttcatgtcgagccttaccgggtaccaggtggttgctgccatcagtacccttgctgtatttgcggtgctgaagtatattggaacggtaggacaaagcattgattttgtaagagaccttacctattttctgtctttatcaggacgaacggaaagtatgttgaatggcctgattacctccagggatattatctattacctgctcattattttacttttcctgggtcttacgatgctgcggtttaaggtgagccgtgagtctgaaccattggccatacaggcaggcaagtatgttgcgctccttgcatttgttttgctggcaggatatttaagtgcaagaccctccggtatcttctacctggatgttaccgcgcaaaagtcccagacgctgacaccggccagccaggctgttgccaaacagatggaaggccccctcataatcaccacttacgtaaacctcctggaccagcatgtatacgccgggctgccggtatcacgaaacacggatctgtcgcgttttgaagatttccgcaggtttatacctggtatcaaaatgaactatgtttattattatgatgctaccgatcttgccagtaatcccaatatgatttaccagggagatattaccggtttgaatacaaagcaagtggctgaaaaagtggcggacaacataggagttgacctcgacgattttttaacgcctgaccagatccatcaaattattgacctggcgccggaggaaaatacatttgtccggcagctcagctaccgcggcaacaccagctttctccggctgtataatgaaaataaccagttcccggaagaagcggaaattacggctgctataaagaagctgatggcgccacgccagcagattgtttttatagaaggagatgatgaacgcagtatccggataaaaggggaccggagttacaatttgttcagtaacgccaggaaaaccaggaagtcgctgatcaaccagggctttgatgtagtaagcgtaaacctggatgtagcggatgtgccggaaagcacaaccctgcttatactggcagatccggccaagccattgagccaccatgccgactccagtgtgcgccgttatatagctacgggaggcgatatgctgattacagcagaaccttcgcaccgggaggtgatcaatccattcctgcgtcagtttggtgtgcagctgtccccgggcatgatggtgaaccccgataaaaatgcgcctgccgatcttatccaggggcgcattgccacagaaaataacgaatacctggatcagctgatgtacatgaatgcggctgtggccatgccttccgcggccatgctggaggtaacagacagtgttttcaccgcggataccgtgctgcaaagcagcgccctgggctggaacaggaagaatggatttgatccttcatcgtcgtcggtatcctatcaacccgagctgggagatctgaagggaagcaaaccgttagtcctgatgctcaaacgtaaaatagccaacagggagcaaaagatcctgatcagcggagatgccgattttatgagtaataattccattccgcaggcatacaatttcccatttattaatggcatctttagatggttcagcgatggccggttcccggtgaaggtgagccgcccggcgccgcaggacgatgccattttaaccagcagaaagcaattatcggtttaccggtcaggaacattatggggaatacctgcattaatgatcgcctgtgcagcagcgcttttgatcagcaggaaaagaaaataaaaaaaatatacctcctggggaggtgttgattgtcttacataatatacgcaggttatgagcgaactaactgaacaacaaatccgggagatgctggagcattacaggctgggagaggccaccccggaggaattggcgttgctggagtcatggtacctaagctaccgggaagaaggggtggccgctcctgatatgatagcgcagcttgctgccgttgaccaggtatgggagcggctggaaaatgaataccgcccggtcaaacgcctgtttggatggcggcgtaacctggtggccgcagcagctgttgcagctttcatgatcgggataggcgcttattttctttaccgcccggcgcatacaccggcaatttctgtcagccaactggcggagagtaagaatgatattcctcccgccacaaacaaagcaaccttgtctgttgccggcagtggtacgacggtgctggattcttccaggacgggtatagtggtgaacagcggcgatgtaaggtatgatgataatacaaagctcaagggggatgccgctttaagcgatggtatccggatgctaaccttgcaaacgcctaaaggaggtacgtaccggctggtattgcccgacagctctgtcgtttggctcaatgcagcttcgcgcctggtttttccttccagctttagtggacaacagcagcgggaagtggagttgcagggagagggctacttcgaagtggcaaaaaataaagcgcaaccctttgtcgtaaaaagccgtgggcaaaaagtggaagtgctgggaacacatttcaatatcagcagctataccgatgagtcgatcaccaaaacaaccctgctggaaggcagtatccgtatcggtaatgtagtattgaaaccaggagagcaggcgcagaaaagtgacgccggaattaaaaccatcctggtagatacagaggaagccatcggctggaaaaacaattatatcgttttccaggatgaaaagatccagtcgatcatgcgtaaaataagccgttggtatgatatggaagtggtgtatgaaggaacattgccaaccgatgattttggcggccgcgtaagcagccgtgcctacgtttcacaggtattaagaaaactggaactgaccaataaagtgcattttaaaattgtgggaagaacaattatcgtcaccaaataataagtcactgaagggcgaaaaatagccagatgtggttgcacacaactggctgacgcctggcagtattgtcaataaaattcctgattgtatcaactatcaaccaaacaagacaaatgtataaaaattatgcgatgaaatccggcatgcatcatttgtatgtccgtaaaatccggcggatcatgcgattaacgtcctgcttactgttcatcatgctcttcagcacgtcggcagcctttgcccagcagatatcactcaaggaaaaagaggtggctatccgggtgattattacaaagatccggcagcagagcaattatgaatttgtgtacactacccagctattggaaaatacccacaaagtaagtatcaatataaaagcggctgatatcagaaccgtattggacctggttttaaaagaccagccactgtcctatactatcgatgataataccattatactaagagaaaagccggtaggcgccgtcgcgccggcgatcaatttcgttgatatcatgggattcgtttccaacgaccagggcgtgggccttcccggggccaccatccggttgtcaggcacccctatatcagtggcaaccgaccagggcggtctgtacaaaatactcagggtacccgacgatggccgcctgatattctcttatgtcggttaccagtccgatactattgccgtaaaaggcagaacggccatcaatgtgttgctgaagcaagcatccattgaaatgaagggtgtggccatcgtttcaaccggtttgcaggaattgccgagagaaagagccacgggatcttttgaagtcatttctaaggagcagcttcaacacagcacggatcctaacctgatccggcggttggaagggattaccacctcgctggattttcgtaacgatcttcgtcctatcaattcagcttcgcctaatgccaggcagtctccattggccaaccttaccatccgtggtaaaaataccctgaatgacgcagtgaacgcagacctgaacggtaactacagcggccaggtgctggtggtgatcgatggtattgccagtccgtactctatcgaccgggtgaaccctaatgatgtagagagcgtaaccatcctgaaagatgccgccgccgcttctatctggggctcccgcgctgccaacggcgttatcgttattaaaacaaaacgtggggggtataaccgcgcaccacgggtaacctttaacagcaatattaatgtcaccgaaaaggtggacctgttctacaataaaacaatgagcgtttctgattacatcgacgcacaggcagcttattttgaacagcagaaccggccattgccggatctgagcatctcccacttatacgggcaggaaataaaatcaccggtagcagaaattgtagatgcctggaagtttaaacatacactgaccgacgcgcaggccaacgcgcaactggatgctttaaggaacaatgacatcaggaaagattatgataaatattttctgagaaatgcagttacccaaagttattccttaggagtagatggtggcggcgaacgctttaactaccgcttgtctggcggatgggacaagaccatcaacaatacaaaaaattcggactacgaccggatcgcactcggttattccatgtccgttaaaccactcaaaaaactcgaattacagggaaatatttcttacaatgttcagcaatacaacgaacaagccccgcaaaacaggatcaccggcgctactgatgccaccttttatccttactcacgcttagccgatgaccagggtaactacctggaacttgccaaactttaccgccagggctttgccgctgcggtggaaaaggaatatgccgataaatttttaagctaccgctatgtgccgctgaacgatatcaatgaaggatacaacaagctgaaatcgcagaacctgaacctgggcatcaacgccaattacaggatatcaaacgggcttaccgcacagctgacgtataattataacaccggcagaaataatgataataccctttaccggcaaaactcattttatatgaggaacctgctcaattatttcaccacttcgccggcgtctgtagatcccagaacactggaaccagtggagccttataaccgtcaactgcccttaggaggccagtacacgattatgcaaactacctccagcaatcataccttcaggggacagttgaactttgaccatacctggaaagaaaagcaccagttatcggccattgcaggttttgatatggcccagtcttatagtcttgccgccagcaacggttactacggctatgatgaaggcaccttgtataccaataacaagctggattttaaaaccatgataccaattgcttttgcagaagacttcagcgggtacaatggtgaatatattcctaatctttcaaccgggtttatcgacaataaagtgcgcaccctcagttactatgccaatgctgcctatacgtatgacgccaggtatacgctttcaggcagtatacgcaaggatctttccagtgagtttggccgtggcaccaaccagaaagggacaccattttattctgtaggcggcgcctggaatattcacaacgaaagtttttatcactggggcctggtgccttcactgaccctgagaacaacttatggttataacggaaacgtaaacccgctgattattgcgaggccactgatcacttactccacgctcaatggcaccaataatcttccgtatgcctatacttccttcggcaccggcatcaccaacagccagttgcgtccggagcggacaggcgtgctcaatataggtgtagacttccagtttaaaggcaaccggctttccggtaatatccagtactacagcaagaaaacgaccgacctgattgccggcggcgcgcttgatcccagcacagggtacaccaatatcaattacaacacaggcaacctgcagggacatggggtagagctcacactaaactcgctgaacgtaagcgcaggggcgttcaaatggaacagcaacctgttgtttgcctacaaccgggttaaggtaacgaagctgtttgccacggctaccagccaggccggcgcggcggtgagtaacagcaccggttcctataacgaaggctacgacctgtcacggttgtttggatatcagtgggcgggcctggaccctaaaaccggcgatccgcggggatacctggatggtaacatcgtaaccatatctaattcccccgagggcgacaacaattacaaagctattcagaatgccccgctgggtaccttgaaatattttggcagcgcggttcctgtgtattatgggtcattcaggaatacattttcctacgcttcttttgcgctgtcggccaacctgctttacaaactcggctactatgtacgccggcctttagcgcaggtggttaactatggcaacctgtattccggtaatagtttgcagggggaagaatataacaacaggtggcagcgccccggcgatgaaacaggcactaatgtgccgtcggccgtcatgtcgacgggtaaccccaacagggataatttttactattactcggccatcaatgtagtgaaaggggatcatgtaagattacaggagatcaacctgtcttataccctgaaagtaaagcctggatgccgtattaaagatccaagagtatatgccaacatcagcaacctgggtattatctggcgcgccaacgataaagggatagatccggaagtattcgattatcctttgccgcgtacttacagcctgggattttcaactaacttttaattgaacgagtcatgaaaaattatataaaatatattcttttgatagtgtgtgtgcttacggctaccgcttgtcagaaatatgtagacatcaaaaaaagtgggtcgcagtcttttattgaaacaacaaaagattgccagctgatactggataattatgatctgttcaacatcaattacccgatagacggggagattgccgctgatgattattatctggatgataaccgttataattcagatgcgattacactggaagataaagcgctgtatacctggcagcctaatgctattcgtgccgcgtcaactcagtgggtggcatcttacaataagatctatcattgtaacctggtgctggaagccctggaaaaaattaaggacacagaccagccggcagtgatcaataacctgcagggcagcgccttatttctgcgtgcctatgctttatggcctttggcacaagtgtatatcaaaccttatggcgccgctaccatgcaggaaccaggccttcctatccataagcgttcagatatcaacgatgttcccggcaggggcaccgtaaaagaaacttatgatgcgatcgttgatgatcttacccgggcggcgggtttactgaacaatacttccagcatatcttcccggccaaacaaagcagcagcactggccatgctcgcccgcgtttatttgtcgatggaagattatcccaatgccttatccgctgccgatgcagcgctgaagctcaaaagcggcctgcttgattataacacactcgagttgggcagttataatccttttccgcgtttcaataaagaagtaatattccattcagttattgactatcaaaacagtgtattggaagtaggttttggcgatgaaaacaaagcgctgatcgatcccgtgattatcagcgcgtatcagaacgatgatcttcgtaaacaattgttggtgaaggagaacctggatgtgccggtaccttcaggtacgtatcgctttgtcggtaactatgaaggagcagtgggttcatccgctttgtttaatggtcttgcggtaaatgaattgtacctggtacgggcagaatgttacgcacgcgcagggcaaaccgctaatgcggtgaacgatatgaataccttactcgccacccgttggtcaacgggaacttatcccggctttactgtaagcaacgcaactgatgcgcttcaaaagatccttttggaacggcgtaaggaattgctgatgaggggactccggtggacggatctgcggaggcttaataaagacacccgttttgcaaagaacctttcccgtaccgtaaatggaacggtatacagtctgcctgccaatgatgcccgttatacgttgctcataccgcaggaagtgatcaccaattccaaacttgcacaaaacatccgttagccaatgcttcacgtgaattcataaatttacgatatatagtatttttttgaaaaagggttttgtgataaagtgctgatttaaagggaaatatgcagtggtatgcttcttgactaccagtacatcattatgaacaacagtattttaggattgcaccatatcaccgctattgcgggaagtgcgcagggaaatttagatttttataccaaagctttgggtttaaggttagtgaagaaaacagtcaacttcgacgatcccggaacttatcatctttactatggtgatgaaagcggatctgccggaacgatccttacattttttccttgggaaggaattggacagggacgtgaaggtgttggaatggctactgaaattgggtatgcggttcctgccgggagcctggagttttggttagacaggtttgcaaagaagcaggtgaagaccagcgaaattgcggagcgttttggtgagcagtttctttctttccgtgatccggacggattgtcgctcagcctcattgttccaaaagcggaagataacagggtaccctgggaaacggacgagattaagaaagatactgctaccaggggttttcacagtaccacgcttaccttacggaaaatggaggaaaccgcgaaagtactgaccgatatcctgggttatcgttttctttctcaggagggtaaccggtaccgcttcattacagacaccgtaaacacagcagcaatcatagatctactggaagttccggatggccagagagggataaatgctgcaggaacgaaccatcatgtggctttccgtgtaaaagatgagcaggtgcaaatggagctccgggaaaaagtattaagcaggaacttacagattaccccaaaaattgacagggactatttcttctcgctgtacttccgggagccgggcggcgtcctttttgaaatcgctacagagaacccgggttttacagttgatgaacctttgaatgaactgggtacccacctgatgttgcctcatcaacatgcgcatctgagaggagatttagagaaagtgcttccaaaattagtatagttatgcaggaaatattgacagcaggaaagcgccttgatgtggcagagaaggcactgatcatggtacatggccgcggcggatcggcggaggatattttatcgttggcggcggagctgaatactgtggcatttgcacttattgctccccaggcgaaaggtaatagctggtacccgcaatcttttttggcgccaagggaaggaaatgaaccgtttctttctgattccctgaaggtattgggagatatagtggaagatcttgaagaaaaaggtttctcaaaatcgcagatcttcctgttgggattttcacaaggtgcatgtctgacactggaatttgcggcatccaatgcagcaaggtttggtggcatcgtggcttttaccggcggggttattggtgaccatgttgaccaccgtaattataatggtgattttgatggtacacccatttttattggaagcagtgatccggattttcatgtaccggtgagccgggtgaaggaaagtaccaccttattggaagcaataggagcgaaggtaaccgaaatcatctaccctaatatgggacataccatcagccgccaggaaatagcagcggtaaataaattgatctttcacgattaacgtaattacaaaaaggattttctaaatttatgaaccagggccattgaaccaaaattcaggaatagacgtttaatcattttatttaccctttagatccttttcctatgagtattttaggtattgtacacaccattatcgccatcgttgctttattatttgctgtagctgccttgctgaaagaaggtatcatcaaccctttctccaatacgggcaagatatatagcatactgacggtgatcgcctcggtcacttcctttgggctttccaaagcgggtggctttaatcccgggcacggtatcgggatactaatacttattttactcggagtggcctatttgctggggcgcaaagcgtccggcaaaagaagtttgttgctgatacaggtgctttgcatgacgcttaccctgttcctttccctgataccggcgataaacgaaaccttactacgtgtgccggtggggcacccgctgtccgatggacctacttcttcaattgtgcagaactgcattaaggtgttgctgggattactggtggtgggactggtactgcagttttttaaagtgaagcagccagtgaagtaaaccatagcgtcataaagcagtttctatagagccgccaaaaagatcataaaatcttaaagccttacagtattaactgtaaggctttaagattttaccagccatattggatcagcaagcggccgtcagggtctatgctgcgatgtcctaatacgttttatacatcaccttacaccctgttaccccgctcaaatgagcatgttctatggtgtaagtataagttccatgctggcgggtttcttttataatttctccggcctgtttttgctggtagctttcaaataaacggctataagcagcgcttcgttcgtcgtaatcagtaatagttaagggcaactgccaaccggtattagaatagcgccgtttaaacaacatgcggtccttttccttgttgaagcaggagtaatatacatttccatctttttcttccagtgtaaattcaaggccggtatttaactttttcttctggtaactttccggtgaaagatggtattcttcaatcaggaagaacgttttattaagcattttataaacccttaaccagttgggactatatgcaatgattgtatccatatggtaatccagcgacacattgcctgctttaacgggaatggtttgctggtatgttatggcatgctgccttgtatcaaacccgaaatttgcctgattgttatcggtgataggaacagttgaatatgcttccgcatcgaaaggaatatagcgctcccaatccctttctgcggaaggttgttgtctttttaataaaacagccgttaattgtccggctgtattaaactggtattccaatgaacgttgtttttcattatccgggcttatgaaaattgattgtgcgttggcgtaatccaggaattgaaggggaaggtaatgatcttcaaaaatatggtgaagtataaattcgttcatctggctgggtacaccaggggcaatgggattggttttagcaggatgtatataccgttctattttaagtgaatcgatctggaagcggtcatattcatatgaattgagcgctgttggccggttctgttgatccggcatctctatcattacatcggaagttgccgttgtttgcgtttgccagaaacgaatagtatactgtttcttatcatttccttccgaaggattgataaaacaaaaaacaaaccttccctccggatagggcgacggcggagtggatgataatgcggtattccgcttctccaggtaagcatatcttttttgcaggaatgttttgttgccaggaccttttgccagtgcggcgctgtcggtcaactgatagcgggaggtagcactgctcaataccacttttgccgttgggaaagaataagtttggaataacaacgcggtaacacgtccgtaataatacaccaggaggatcttatcaccttttgcattattggttactaccgtgtcttcgttgtaatcattattgtccaggaggtgtgcgtttttaaatcctttttttgccaggtattgtttaacgttctcgccggcattgaaagtactttccaggtcttttatggaaagcgtttgtgtgggggccgtttgggttttctgtgcaaagctctgggaaaacaaagaaaggatgccgaataaaataatcaggtgttttttcatagttgttaaaagaaagtattgacctaagctaacttaatagttaggattgcccaaaaaaaatttgatatacttcccggaaaagttcaccatgttgcaggtatggatttataatctttagatagtaaatttgtaaaaaagtaataatggctgatattggtaccaaacggataaaacggagtgaggaaataaccagtcaatacttcacgctgttggataagcacctcgatgacctggtgaaggggagagcgacggaaatgatggagctgaatgaaatcgcggctgagttatgcgtttcacataagcacctgaccgataccatcaggcaaacaatgggggctcatccctgccacttctacgatcagaaaattattgaaaaagccaaacaactgctgcaggaaaccaacgcgtctattgcgcatatcgccatcaccctgacctacgacccatctaatttttcaaaattcttcaaaaagtatgtaaagttaacacctgatcagtggcggaaaaataacctgccggattgaaagttccgaaaagttcaccatgataaacctgccggacctgcagatctttgccataattaaaaacaactcatatggcaagaaacgatttaaatggaaaagtggttttaatcgcaggcggagcgaagaacctgggcggactattaagccgtaattttgcagaaaagggcgccaaactggccattcactacaacagcgaaaacacgaaggctgacgcagaaaagacactggcggatgtacaatccctgggagcggaggcattcctgttccaggcagacctcactgatgtaaataacattgttaaattctttgatgaagccattgataaatttggcggaatagacatcgccatcaatactgttggtaaggtattgaagaaaccttatatagatactaccgaagcggaatacgacagcatgtccgacatcaactccaaagtagcctatttctttatccaggaagcgggtaaaaaattgaatgccaatggtaagatatgtaccatcgttacctctctgctggccgcatttacaggatactattccacttatgccgggatgaaagccccagtggaggacttcacccgtgccggatcaaaagagtttggcagccgtggtatttcagtaacggcggtggcacccgggccaatggataccccgtttttctacggtcaggaaagcgcggaggccgtagcgtatcataaatcagcttccgcattaggtggacttaccgatatcaaagatatcgctcccctggtggagttcctggttacggatggctggtggattacggggcaaaccatttttgcgaatggtggctatacgacacgataattttatcaatacaaatatgttctccggtattcgctgggcgtttgttctttaacttctttaaactgtttactgaaatgcgcccagcttttataaccactttcataacaaatatccagtatcggctgcgtagtggatgtcagcagcttacaggcatggctgatccgtaaatccctcaggaaatcgaaatacgtttttttgatatttttcttaaagaagcggcaaaagttaggcacgctcatgttggcaatagccgccacttcttccagggtcactttttcgagatagtgtttaaaagagaaatcaataattttctcaataaccgggttgagcacattgccggtgtcggtgaaatcttctgtcagtattttatattgggtggaatgacctatctgatgcaggcattgcagtaaaagcatcagcttatcaaaccctttttcgtggtgtatctgctgcatgctttccgatacgtcctttttcagggcgtgttccaattgtatgccgttgttcttttgcagcaacgattggatcgttttcatttctgccatttgcagcaacccttctccccagcaatccctggtgaaatgtataaccagggcggcccccctcattttaggatgacttttcctgaaccaatgcggaagattacccgccatgaaaaatacatcgttcaccgtgtagtcgcttacatagtcgccgatcatggcggtgccatgtccttttaatatcaggatcaattcgtattcaggatgcttgtgccagttggtttcaaactgcggcgtttcataaatacggcaggcaaaactctggctggagtcattggtgattttttgaagaatcgttttcatgcaggcttaagataacccatcttatcatataaatgactgaatttatcaaattattgataagatagcatattttctttcaaaaataacggttgataaccttttaaattcaggcaatatttgcgtattaaaacacggatatgaaaataattacaggaaagaaagaattttttagcggcattactgccgtgcaatatgaaggaccacgtacagataatcctttagcttaccgctggtatgatgaaaacaaagtcgtagccggcaaatccatgaaagagtggttacgctttgcagtcgcgtactggcattcctttaacggaaccggcgccgatccctttggcgaagcaacacatatttttgaatgggataaaaatgccgaccccattgagcgcgcaaaagataaggccgatgccgcttttgaactgatcaccaaactcaatctgccttattattgcttccatgatgtagatgtggttgattacaccaacaacatcgcagataatgaaaagcgcctgcaaacgctcacgcagtacctgaagcagaagcaggaggaaagcggcgttaagttgttgtggggtaccgccaacctgttcagtcatcgccgctatatgaacggcgccgctaccaatcccgatttccacgtgctcagccacgccgccgcccaggtaaaagctgcgctcgatgctaccattgcactcggaggagagaactatgttttctggggcggccgtgaaggctatatgagcctcttaaacacagacatgaagcgggaaaaggaacacctggccaggttcctgcaggcgtcaagagattatgcacgcaaaaatggctttacaggtaccttctttattgagcctaaaccatgcgaacctaccaagcaccaatatgattatgatgcagaaacggtgatcggtttcctccgtcagtacgacctgctgaatgacttcaagctcaatctcgaagtaaaccacgcaacactggcaggccatactttccaacatgaactgcaggtagccatagacgccggtttactcggaagcatggatgccaacaggggcgactaccagaatggctgggatacagatcagttcccgaccaacctcaacgaacttaccgaggccatgctgattatcctcgaaggcggcggctttaaaggcggcggcattaacttcgatgcaaagatccggagaaactctaccgatcccgccgacattttctatgcgcatattggtggcgtcgacagcttcgcccgcgcactgatcactgccgatgccatcctggagaaaagtgactaccggaaaatacgccaggatcgttacgcctctttcaatgttgatacagccaaagcttttgaatcaggacaggcgggcctggaagaactgcgcgcctttgcaattgcccagggagaaccagcagtgaagagcggcagacaagagtacctggaaaatgttatcaataattatctgtagaacgtttttataaaacaccttcctgactccgccggtattacccggcggagttttttttgcctgcaaatgagtaacaaacaaccggtcaaaacatttttacccttcatttcaacatttgtacctgccggttggaggagcgcggaattatcttaccactacaaaaaaccacgtttgtcaaatgttactaaaatctattgttcttgtctttttattttttagcctgacgatacaaaacgggcttgcccggcaaggcggtcctggcaggaagccgcccgctgaaacagattccacacgtttttattcggaggtaaatacctatgtcaaccctgttttaccgggagatcatcccgacccaaccctgctgaaagttggcgccgacttctatcactgtggctcctcttttcatttcaatccctacctgcccatctaccactccacagacctggtgcattggaaagtgatcagccgtgtattgccgccggtacatgccggtatggtggcagatcgtcccagcgctggtgtatggcagggcgccatcacttatttttatggctcatactggatctatttttcttcaggcggacaatggttttccaaagcatcgtcgcccgaaggcccgtggactgcccccgtgcgggtgaaggagaaccgggaaacagggccgctgggatatgataactccatttttgtagatgatgatggaaagccatacatggtaattaaaaacggtcagaaggtaaaccggctgcaagcgctggggcaggatggccagcttacagattcggtgatcaacctcgactggatcaatgcgaacctgcaatacagctgggcggaaggtcctgtgatgtgtaagcgtaacgggtattattattacttcccggccggcgatgtatccggcggacagtacgttttgcgggcaacggccctcacggctgattccaccaggtgggagcggttaggggattttttcaaaccaagtcccgacccggacaatacttttccccgtcctaatcatatttcagcgcccgttcaactggcggatggtacctggtggacgatcgggcagagttaccagaaaagaggtaacgacgactggtcaggtatgggcaggcaaacttctttgtaccaggtattatgggagggcgaccgcccctggggcgccccaccggtaagcggaccagtagtaaagcctgcactggataacaataacacaccctggcgcagcgtgcataccgatcattttaataccgacagcctgggcctttggtggcattttttaaccaggcctgctgctgcgcactactcactggcgcaccggaaaggttggatccgtttatctcccgacagcggcagaacgcacctgctgcaaaaggaaaccgaccatttctattcggcagtcacccgggtggacattggcgcgggcgagccggcagcacatggtggcatctacctcaccaatggcaaccaaagtgtgtttgcccgtctttattattccaacggacgcattgtatttcaattggattccgcgttgagggagctaccctataataaaggacgccaggtttggcttaaactggaaagattggaacatcagctgaccggctttttcagctccgatggtaaaagctggacacccgttggcggcgctgtcagtgcagtgcctttggataaagttcaacctaattataacagttgggtaggcaccagcattggtttgtttgcggagggcggtccggttgatttcgacttttttgtttgtaaagatggattttctgccctgccagctgcaggaagcagcaatcactatggaacctataaagtaaaacggggagatgattgggtagtcactaacgcttccgcacacggtggctggctgatgatatcaggagtggacttcggcgccgccggagatgccaaagcgattgaagtcacagctgatgcaactaaaagtggtgaactgaaggtatggatagatgacctgaagaacggccggcaaattgccggcgtccccatcaaacccggtaaactttccgggcatgctcctttgctgaataaggatatttccggtcagcacgacctctttatttggtttcccgcaggcgcctcacaggaaatatttattaaaagtatccggctgctaaaaacaggaaaataaacatcccgtttttttgtagcgaactgatttcgcagctcctgacagggccatctgcgctttatttagacattatttccatccttttggagattcgtgccattcatatatacatggctattgtagattcgtctgttgcttttcctttcagctccacctgataggcttacgcattaccgttatgaaaaattgtcaatttaacactaaatgattacttatgaaatttgaatgtcccccggggtaccacgtcccgatataatcattttcagttccatcacttaatgggtagcatccgataattactttaggggttctgctttttatcgcatctcattgttcccgccgggtgtgccggcgtgatagtcatgtactggctgtcagaacccctcattgccctaacattaaatattttgaattccatgtttaaaatgattctttcgcaaaagtcgtggaaatggcttgtcgtgacagcagtaatgctgtcaggtacgctcacctgtgcttccttacaggcccaggatacacgggtagtacagggagtagtgctggatgagaaaaagacgcctgttcccggtaccaccatacagataaaagaaacgaagattagtaccagcacagataatgatggtaaatttctcatccgcgttcctgccgacaaacacattcttattttcagttttataggaaaggcgccgcaggaagtaaacgtccgtaaccagtcgaccatcgccgttaccctgaaagacaatgtttttggtcttgaagatgtagtgatagtaggttatgggcggcagaaaaaggaaagcgttgttgccgccgtttcccaaactaccggtaaaacattggaaagggccggaggcgtgtcaaatatcggcgctgccctcaccggcaatgtaccgggtcttatcactgcccaaagtaccggcttgcccggtgaggaagatcctcaactgatcatccgcggtcttagtacctggaataacagtaacccgttaatattagtagatggtgtggaacggcccatgtccagtgtcgatatcggctccgtagaaacggtgacggttttaaaagacgcttcggcaacggcggtatttggttcacggggcgccaatggcgttatcctcatcaccacaaaaagaggaaagctcggcaaagcttctatccgggctacggtgaacaatgtcgtgaaagcgccatccaaactgcccggaaaggcagattcgtacgacgctttgcgtactgttaacgaagccatagaatatgagctggcattaaaacctgaaagctggaataactattacccacaggcaattctggataaataccggaatcccgccaacctggaagaagccgaacgttatcctaatgtggactgggcaaaaaccttattcaaggattatgctacgtcgcaaaatgctaatctcaatatcagcggcggtacccgtttcgtaaaatatttcaccagcgcagattttctgcatgaaggcgatctctttagaatatacgataacaaacgcggatacaaacccggttttggttttacaagattaaatgtccggtccaacctggattttcaattaacgccctctacactcttcaaggtaaatctctccggatcatatggtgtgcggaaaagtccctggggattttcgggtaatcagtatggttcctggatcgacgcttacactaccgcgccggatgtattcctgccggtatatgcggatggttcctggggctactatgcgccaaatgagggacgggcggagaattccgccagaagcctggcagtgggcggtattcaataccagaccactacacgcatcaccaccgactttaccgtagaacagaacctggatatgctcgtggacggactgaaactcaacgccaccatttcaatggataataccttccttgaaagcgacaggggagtgaatgacctttaccacgatgtacaacgcaaatggattgatcctgcaacgggaaatgtattttataagagtgcttttgacggcgtcaccaatttcgatttccaggaaggcatcaagtggacaccggcagcaggtgcggtttcggataatcaacggcgactgttttaccagttgcagttaaattatgcaaaaacgattgcggacgatcaccaggtaactgccatgggattgctgaaccgcaatgttaccgccaacggcagtatgataccctcgtaccgcgaagattgggtattccgtgccacttacacgtataaaaacaaatacaccctcgaatacaatggcgcctataatggctcggagaagtttgcacctgattaccggtttgccttcttctcgtcaggcggtgtaaactggattttatccaatgagcacttcatggaaaatataaaattcctggacctgctgaaattccgtgcctcttatggacaaacgggttttgacaacgtagcaggccgttttctatacatgacagaatgggcatatggtggacgctcgcggctgggaactacaggcgaaggtgcggagcaaagtccgtttaactggtaccgtgaatctaccgttggaaatccgaatgtgcaatgggagcaggcggagaaaatgaatgttggtgccgactttgaattattcaaaggtttcgtaaaaggtaaagtggatttcttcgaagataaacgttccaaaatattgcttgccaacaggtcgtcagtgccgtcttattacggcaccactcccccggtagcaaatcttggccgcgtaacatcgcggggttatgaggtggagttacatttcagttatcctgtcacaaaacagctgcgggtgtggtcagacctgaacatgactcataccaaaaataaggtgattgaagccgacaatcctgagctgctgccggcttaccagaaatcggagggcatgcagatcgggcaggcttactcttatgtgagccagggttactacaacacatgggatgaactttatggcagcaccatgcataataccaacgacaatcagaagctgccaggcaactattacatcgtggattataatggcgacggcgtaatcgacgcgagcgataacattccctatggtcatagcggatggcctaccaatacttacaacgccacgtttggcgtggactggaaagggctcagtgcttttgtacaattctatggggtgaataacgtaacccgccaggtggtattcaacagtttaggttcccagggccacacggtttataacgaaggcagttattggtcgaaggacaataccaacggagatgtgcccatgccacgctggctatccacaccagcaggctattaccgcggtacccaatatatgtacgacggttcctacctgcgcttaaagaacgctgaaattgcctacacactcgataaaggatttataaaacggataggtcttgaatcgctgagaatatatctcaacggcaataacctggccgcctggagcaagatgccggacgatcgggaatcaaattttgcaggtaccggctgggcatcccagggagcttatcctacagtgaagcgttacaatctcggcgccaattttactttctaaacatgacctttatgaataagtatacaaagatgttgttggctgccacagggatcgtaacgatacttggcctggcatcctgcaagaagttcctggataaggaaccacaatctatcgtgtcggaagaaaatgcctttaaaacctttatcggtttccagggctttaccgaagaactttatcactgcataccggattttaccaatgcctactggaccaattcctggaactggggagaagatgaaattcaatctaccgcacgtgatttccatttcatcataaaaatagataatggtgatttctggggctggcagtcgcagtttgacggctggcaggctggctggatggaccggaataataccagtaccaatgacgaccgttttgcaaagtcgatgtggaaactgggatggtacggtatccggaaagccaatatgggactggaaaatattgataaattaacagacgccacgcaggaagagaaagacctgattaaaggacagttgttgtttttcaggggatggtttcattttatgttcatccagtattttggcgggttaccatacatcgacaaagtacttccgggtgatcagaagctcaccttaccacgtctcaaatacagtgaatgtgcggataaagcggcggccgatttcagagaagcggcaaacctgctgcccgtaaactgggacaataccacagcaggtaaaagaacgctcggaaaaaaccagttgcgcattaataaaattatggcgctgggttacctggggaaaaactatttatgggcaggtagtccgctgatgaactatgtatctgccggcagcaaaacctacaacgcggagtattgcaaaaaggcggcagaagcatttggtgaattactgcaattgtgcgagtccggagaggcgccttacaagctggtagaattttcgaagtactataccaatttctatagcgccggtcagaactggttaatgccaggcggtaccgaagctattttccgtgggccttactatggcgcgcatggctccacttatggcaccgccaagcaatacggtccggctttgctcacagaagaagccatcacttttgtgcctacggctaattatgtggactattacggtatggctaacggcctgcccatcaaggacattacaaaggccgatccggagtcaggatacgaccccgcttatccgtggagaggcagggatccgcgtttctacaatgatatcgttttcgatggggttaaatgtgtacagggcgccactaccgatgaaagaaaccgttacgccaatctttatacaggcggcacttaccgcgacatcagcagcggcagccgctccggttacctgctctataagtttattcctatcacagccaacagatttgataatggctggacctacgacaaagcgctgaatatccacctgccgtatatgcgcctggcggacgtgtacctgatgtatgccgaagctgccgcacagggctatggcgccgccacaggcaaggccggcaactatgctaaaacggcattagatgctgtgaatgtaatccgcgaccgggcaggcgcaggacacgttgctgctgccttcaccgcctccctggatggctttatgagcgaagttcgccgtgaacgggccgtagagctgtcttttgaaggccatcgtttcaatgatttaagaaggtggatgttgctgatacaaagcccgtacacactgaaaaaatcggtggaatttgaccggtcgtcctcattcagtactgtagatccaatgaataaccgggtactcaatttacgcgaatccgttatcctggaacgcaggtatacagagaaacactactggctgccgttaaaaaattcagatgctaatatgtacctggaatttccacagaatccgggttggtaaaacgtgcaacccttacatgtatcgtttactgttaatttcaaaaattcatgaatcagataaaagcattaatagcctttgcagcgctgatgaacctgacgccggtttcgcaggcgcaggacaccacggcaaaaactaccactgttattcctcccggtaacccggtacaggtggccttccggaaggtggataaaaaagacctgtcaggaggcgtttcagtagtggacgtggcatcacaaatgaaactaaactatatgactaccagcctggaaaacatggacggctgggtaaatggttataatggaaacagtatgtggggcatgggtagctatctgctcgtcatcgacggggtgccccgtgatgaaggaaatgtagtgcccacagaagttgaacagatctcttttctcaaaggagtgaatgccgtagcgctttatggcagcagggccgccaaaggagttgtatacattaccaccaaaagaggtaaagcaggcaaccagcggatcgatatcagggccaatgccggcgtaaacgttcccaaagcgtatccccattacctgggatcggcggagtatatgacactttacaatgaagcccgccgcaacgacggactggccgagctgtatagccctgaaacgatctaccagttcgcgtcaggtaaaaatccataccggtatcccaatgtagattattactccgacgaatatcttaaacaatcctttggccgctatgatataacaacagagatatccgggggaaatgacaaggcgcggtattataccaatattggataccagacggccggttcgttgctcaactttggtgaggctgttagcaacggcaagtccgaccgcctcaacctgcgcggtaatgtggatgtgaatcttaaccagtatatttcctgtaatgtagatgccaccgcgattttctataccggtaggggcgtaaacaccgactactggcaaagcgctgctaccttgcgcccgcatcgtttttccccactcattcctttggatatgatcgagtcaaatgatgaagcatccaacgtatttgtgaagaacagcaatcacattattgatgggaaatatttgctgggcggaacgcagctggatcaaaccaacccgtttgccgccatttatgccggtggaaacaaccgctatatcagccggcaattccagttcaataccggcgtgaatgccgatctgagaaatttactgaaaggcctttccttccgctctgcgtttgctgttgactacaacacctcttataacctcgctttcaacaatacctatgcggtatatgcgcccacctggaatacgtattccggcgtggacctgatcagtagcctaacgcaatacggacaggatgccacttcaggtgtgcagaatgtaagcaacagctggtaccggcaaacgatctctgcttccggtcagttcaattatgtgaactccattgacaacaggcataatctttctgccgtgttactggtgaatggcttccagcaatctgaatcagccgtgtaccaccgtaccagcaatgccaatctcggtttgcaactgggctacaacttagaccatacttactacatcgatttcagcggcgccgtcattcacagcgcgaagctgcccgaaggaaaccgcaccgctttttcgcctaccgtgtcgctgggctggcggctcagcaacgagccctttatgcgtggtgtaaggggagtggatgatcttcgtttaactgcttccgcaggtgtgctgcataccgacctggatattgcttcttattatctataccagggtgtttataccacgcagggaagctggttcggctggaaagatggtaccggcgtgcaggccacggaatcaaggcgaggggctaacccggatatgcgtttcccaaaaagagaggagatcagcattggcctggaaggttctttcttccatgaatctttaaaactggatggtaacttctttgtcaataaaattaccggcaacattatccagcccaacgtgttgttcccttcttactacaccaccggctggccatcatcttctttcattccctatgtaaattataatgacgataaacggatgggagttgatttcagcctcagtctgaataagaagctgtctgatattaactattccatcgggctggtaggtacttactataaaacgattgccacaaaacgggcggagatttatgaagacaattaccaataccggcagggaaggccactggacgccatatggggactgcaaaacatgggcttcttccaggatgcggatgacatcaaaaattctccctcccaaactttcggccaggtaaaaccgggcgatatcaagtataaagatcagaatggagatggggttattgatacccgcgatgaagtatacctgggccgtgggggctggtttggctcaccgcttacactaggtgtgaacgtaagtgtgcaatggaagcatttctccttctttgcactggcgcagggtcgcttcggttcctatggaatgaagaacaattcctggttctgggtagatggagaggataaatattctgaagtggtaagagaccgctggacacccgaaacagcccagtcagcgaaatatccgcgactcaccactttcaacagtgacaacaattttcgcaattcggatttctggttgtacaaggctaatcgcatcgacctggccaaggtgcagatctcttatgatatgagcgatctgattggcaataaaaagatcgtgaaggagatgggggtgtatgtgagtggcttcaatttgctgacgtttgctgccgagcgtaaattgatggaaatgagtattggcagtgcacctcaaacccgcttatataacctgggagtaaaagctatgttctaatgatgcctttcacccaatcaagtttccactttatgaaaagaaatattatcatgctgctggcatccgttctgctgctaaccagctgcaaggatctgctgacaccggaaattgaaaataaccgggacctgaacccggcaaattataatcctaatgatgccggactcccgtttggcgtgctgctcaatggttacaaccgcataccaaccaattcatggtcgtttaatgatgtagccacagatgatgcggtaacaaatgatcagaacaatggcttcctgaaaatggccaatggccaatggaccgccaataataatccgcttaaccagtgggaaaatgcatatgccgctattcaatatcttaatatcacactgcgggatgttgataccgtgaagtgggccgctgatcctgctgtcagcaaactgtttggtatgcgggtaaagggagaggcttatggcctgcgcgcccttttctattaccacctgttgcaggcacatgccggcatgtctgaaagtggcgctgtattaggtgtgcccatcaacctggaagtgcagggatctaatgctgatttcaataaacccaggagcaattttgatgcgtgcatgaagcagatctacagtgatctggcacaggcggaccagctgttgccaaccgactacgaaaacattcccaatgcgtcccttatcccggcaaagtatggcacggtgaccaaggaacaatacgaccgtgcctttggcgctgccttccgtggatttcttaccggtcgtatcgtaaaggcgatccggtcgaaagcagcgttactggcagcgagcccagctttcagcagcggcaccactaccacctgggcagacgctgcgaattacgccggtgaagtaattgcgctgaaaggcgggataactgccttgtctgcaaatggcctcaactggtattccaacgcttctgaaattgcggggttagccgatggcgcaaatccttctgaaatactctggagaaataattatggcgacaatcgtgatctggaacaagccaatttcccaccaagtttatttggcaatggccgcatcaatccaacacaaaacctcgtggatgctttccccatggcgaatgggcttcccattacggatgccgccagcggttatgatgctgccaatccctacgtgggccgcgatcccaggctgcggatgtttattttagtcaatggcggcaccgcaggtccaaataattccgtgatctccaccgcggcagacggcgctaccaacgatgcgctgaacaaagtagaaacttctaccaggaccggctactacctccgcaaattgctgcgccaggatgtgaacctcaatcctaattcggcgaataatcaacggcattacaaacctcatatccggtatacagaaatttttctcaactacgcagaagctgccaatgaagcctggggaccaacaggcagtggcgccttcggattctccgcttatgatgttatcaaagctatccgcaaaagagcaggggtaggcactactaacggcgatgcatatctcgaagaatcaaaaggcagcaaggagcaaatgcgcacgcttatcaggaatgagcgtagaattgaactgtgctttgaaggcttccgcttctgggatcttcgccgctggaaggcaaacatcgccgaaacggccaaaggcgttagcatacgcaacaacagttatgctgttattaacgtggaaaaccgccagttccagccgttcatgatctatggtcctattccctacggcgaaacattaaagtttgggtcgttagaacagaacaaaggctggcgctaacagctcctggtacataaataattttctttgattttgaaattaacaaagatgaaaaagttcttaatacccatcatgctactcgttgtgtcaacagcatgcaataaagaggtagaattcccggattataaataccagacggtgtatttcgcctatcagtaccccgtgcgaaccatcactttcggggaagatatattcagcacggaactggacaaccagggcaaatgtaaaatcatggcaacaaccggaggtgtttactacagcaaaaaggatctgcatatcgggatcgcggtagataactccctgctgggaaacggcttgctgtttggcgccggcaaagatgagatcttagcgatgcccgctaactactattcgctggcggcaaatgagattgttatcccggaaggcggcctcacaggcggcgtggaagtacagctcacagacgctttcttcaatgatccaaagtcgatccggaatacctatgtgatcccgctgcgcatcaataataaatcgggcgctgactctatcctcagcgggaaagacttcatcctttacgctatcaaatatgtgaacacctggcatggcaactacctgcgcaggggaaaagatgtggtgtccggaagtgtaagccaaacaattgtaaggcacaaagaatatgttgagtcggatgaggtgaataaattgaacacgaagtccaggaaggaacttgagtttccggtagtgtataaagacaaagacggcaataatatttattgcacactgctgctcactttcgacgacaacggtaaatgcaccatttcgtctgccaccagcggtttcacagccacggggagcggccagtttgtaaaaagaggagaaaagaacagctggggcagcaaagaccgtgatgcattgtatctcaattaccaggtgtccttatcgggtatgcaggtgtctacatcagatacgttggtattaagggaccggtccgtaaccatggaaacttttacaccggtgagcaaataattttctgcctacaattaaagtaatttatatgcatcaacatcataaaatagcagttggctttatggcattcatggccattacttcctgcagtaaatataaagcgcttgattttaacgtggacaagcctgaaagtattgcgcttcaggaagacatagacgcttaccccgccctgaaaagctatattaaccgtgtggcgcaacccgggtttaaattgggtgtggcgctgggtttacaggaatatcttgacaaaggcgtgatgtaccggttagccaacaggaatttcgacgaggtggtgataggctacgatatgaaacatggcgccgtagtacaggccgatggcagtttaaacctggtaaaagtaaaatcattgcttcaatctgccggcgaagcgggaatgcaggtatatggtcataccctcatgtggcatgccaaccagaatgccagctacctgaatggattgcttagtcctttgctggtaacatcccccgcttatcagaatgacttaaatcttgcagccctgaaggataaaaccttcaccggttggtccctggccaatccgggggcgggcatttcaatagcggaaggtgaaggcatgggaaccgggaacaaagccattaagctggtgtcaaaaggcggctcgtcgtcagctgccgatctgcagctcgttaccccgcaggttggcgtgaacaaattgcataagtatgaagtagtgatgtatataaagtcggatgcagcgggtgaaggaagggtttcttttgaagggttaaataacaatacgccatcgatcgactggaccaaatcaggtacgccttccccgacttttacaaccgggatttcgtggaaagaaatccgctttactattgatgatttttccgccggtaatattaaactgcattttgacctgggctataaagccggcgtaacttattatattgatgtcaacaatttgtacatctacgatacgcaaggcgcacccgtagtaaacaacctggtggccaacggtgattttgaatccggaggtggctggggaggctggggcggcagctccacccgcggcgtaactgctgacggtatgggtgttggtaacaaaggcaaggctttttatgtgaccaatcctacaaaaggcgccaattactgggacgtgcaaaccagctatgattttgcagcgccgcttgctaacggagaaacttacgaattgagcttttgggtaaaaggaaccgccgatggcgtaatccgcccggaactgcaaagcgccaactattcgtctaatgggtacggacaggtggcggttactaccgcatggaagcaggtaactgtcgccaccacggctaccgcggccgaccggacacgattgatctttagctatggtgaatttgccggtaccgtttacattgatgatgtagtactgaaaaattccaaagcaaccggtggatccactaccatcgtggaaaaaacagccacagagaaaaaggctatcctgaccgctgcactcgataaatggatggatggcatggtgggagccggaaaaacagcagtgaaggcctgggatgttgtgaatgaacccatggatgacggtaatccatatgaactaaaaacgggtattggcaggccggtcatagcggctgatgagtttttctggcaggactacctgggtaaagactatgcagtaactgcatttaaaatggcccgccaatacggcaatccgggcgacattcattttatcaacgactacaatcttgagtatagcctggataaatgccgtggcctgattgcgtatgtcaattatattgaaagcaaaggcggaaaagtagatggcattggtacgcagatgcatataaccactactaccagtaaggaaaacattgccgaaatgtttaagctgctggccgctacgggcaagttgataaaagtttctgaactggatcttggtgtgggggtaaaaacaaccgaagctactgccgaacattacaaagcacaggcagagatgtataagtatgtcattgataaatattttgaactcattcctgcgaagcaacgttacggtattacgatctggagtcctttggacagccgggcgggttccttctggcgtccgggcgaacccatcggactttggactgaagggtatgtgcggaagctctcatatgctgcagtggcaaaggcactagaagctaatgcgaaataacaggaagccctatttttgtttttgataagcatccccggcaatagaagccggggattttttttgaagaacggttattcgctgctgttctcttttttaacctgcgctataaattcagagggcagcatattgtatttattcttgaacgatttagcgaagtagttaggcgtggaaaatcctacctggtaggcgatttcggcaatggtcatatcgcttttttgcatgagggtcatcgctttttccagccggtaggaacggatgtattcaacaggtgtttgcccggtgagctccagtaatttattatacagggagctgcggctcatgccaacctctttactgaggctttcaacagaaagctgggaatcggtgagcttctcttcgagatgacaaacgatcctgttcagcagtttttcatctgttgattctttctgcacttcgggggcatgcacttttatttgtttggtataggtgtttttcagggtatgattgagatgcagcaggttccggatcttcgcatgaagtatctcaaaattaaacggcttaatcaggtaatcattggcgccggtttccagtcctgagatctgttgttcttcattggtaagtgcggtcagtaatatcaccggtatatggctggttcttttgtctgatttcagtttttgcaacaggctgataccatccatctgcggcatcgtgatatcgctgacaatcaaatgcggatgcagtgccagtgccttttgccagccgtccttaccattagctgcttctattaccttgtagctgttgcggaggttgtctttaagatagaacctgaagtcttcattatcttccaccagtaatatcgttgacatctctgagaaactttgtgcggcgggcgatacgcgggatgcctccggtaacgcagtctcttcctgctggaatggtaaaactgtggccaggggaggtgtttcctgctcggctatttttaatggaagttgtataaaaaaggtagcgccttgcccggattcgctttccacttcaatatctcctccgtgcatctttacaaattcctttgtaatggataacccgatacctgtgccctggttaagtatggcggaactggtattggtttggaagaagtggtcgaatactttttctctcttatctttcggaataccaataccggtatctttcactgtaatgagcacccattgtaagccgggagtagcgggctttttcagcaactgcaattccaccgtcaccgcatcctcttcctgggtgaatttaaatgcgtttgaaagcaggttgaaaagaatacgttccattttatcatggtcgaagaaaacatacagggaggcaggtttgctgctgaaagtgaaacggatgtttttccgttcagcaaagtcactgaaagagtccgttacttcttttataaaagatacgagttctccttttgccagctgcagttttagttcgtgttcctccatcttccggaaatccagcagctgattaacgagattgagcaaccgcctggaattgcgcttgatcatattcagtttttccagcctgttgccggtttgttcactgccaatcaattgctccaccggcccaaggatcagcgaaataggcgtcctgaaatcgtgactgaggttggtaaggaatttaattttcatccggtccagctcacggacacgctttatctcctgtttttcctgctcggccaggaatttctttcttatcctggttatcccgcggtaccggctgtacaacagcagggcgcagatggcggagatataaaacaggtaggcataaatggttcgccagaaaggtggtcttacatagatctttatcgtggtatcctttgtattccataccccgtcgttattgctggctttcacgtgaaagatatactctcccggatccaggttggtataagaggcggtattgacggttccggtatagttccagtctttatcaaatccttccagtttataggcgtaataatttttcctggggatagtataattcagcgctacgaagctgagggcaaagttttgtttgtattcaagcctgatttcgctggtaaccgaaatgtgatctttgatgggactgtcttcccccgggatcactgatttgttggacacttttaagtctgtcagcagaacaaccggcacattcctgttcaccgttaacccggaaggggtgaagtaattaaagccttccaatccgccgaacatgatatccccgtcagacagccgtagcccggacgtatgtacgaagttattattttgcgcaccgttgtaatggctgtagttcctgattttttttgtggcagcattaaagctgctgatgcccgtgttggtacttaaccaaaggatgccgtctttatcttccaggatctggtagatggtggtattctgcagcccgtctttttcgtcgtaattgatgaatcgcccggtggctttatcgaacaggctcaggcctccgccataggtgcctacccatatatttccgcggctgtcgcgcagtatcacctgcactttatcgcctgccagctggctgttgctttgggtatagatatcccatttgttgttggcgggatgatagacgccgattcccccgccgtgtgaaccaatccagatgttgccttctgcatcttcttcaatggtcctgatgtatccattaaacgggagctttttttcttcaggtatgcctggtctgggatgcggactaaatctggcaacaactttttcatttcttaatatattcacaccctcaccgttggtacccacccaaacgtcgcccttactatcttcctttatacaaaaaacatcattggcgttcaggttgtccgggccggttccttttaccaggtgtttataattgccggcgccgttggaaatcagcagaccatgcgcgtaagtgccaataaacagttttttgtcctgcgtgtagtgaagcgccatgatggacacgttgttgtttgccggaagcgggatattgactggctgggctttcccggtattacgattgaactcgaacaaacctccgccatcggtgccgatcaggatattttccgcactcttttctgcaaaagcacttactatcgacgacttgcggtcggatgtatgaaagatagtgccgggcttgaaattgaagaggttcaggtttttatcgtatttattcacgccgccgcgaaaggtgcctatccagtaaattccctgccggtcgatataggtgcatctgatcgactggctggtaaggctatagatatttccattgtccggaagatattgatcaacggcttgtgtcctggtattaagcaccatgagtccttcctgtgtactgatccacaactggtcatcgtcgtcgggctcaatattgttcacctgcacattgctgatgggcgcattcccggtggatgcccggtagggggtaaatccggagccgtctggttgcaacatgcataggccggctaaggtacccacccagatctggccgtttttgtcggctgcaatggcctgtatatcattatccggtgcgctggatttcgctgctgtgttgaataccagctttaaggcgcctgttgatggggaatagcagtaaagaccaatggtagtgcctatccagatttgttgttttttgtcgaccaaaacacagcccagggtttttgttgcttcctggctgtcttttcccgtatcgagtttgatcctggaaatatggcgggtaacaggatcaagctgaaagaggttctcatactgcgctatccaaacctttcctgaagtatcgctgcaaatgtccatgataacagcgttggagggcagttcaggcgtattggcgtttaccgggaagtgaataaaagcatcctttttgcggtcatacaggctgagcccgccgccactggtgcctatccagaggttgccgtttttgtcttcatgaagtaccaatacctcgtttgccctgaggctggaagaatcaccgggattgtgccggtacgcggtaaaattagtaccgtcaaatttattcaggccatcatccgtggcaaaccacatcaggccgtagtggtctttgatgatgtagttcaccgcattggacaccaatccgtcttttgcggccagtgaggtgaagtttattttctttgtttgcgcccaacctatctgaaccaggaacagtaagcaacagaggaacgggaatttatatttaaacatatcaggcagtcgttaaaaaacaagatgttggttgaactttcgtacatggaactttgccgggactatttcatcacccaatttaagtattgtaaagcaatcttaaaagtgttaccggtgtttatctgcgccgcgccggtcccctggtagtttcttgcgcttaaaatgattgtctgtaagacaattgtgctatcaatttcaacaaatgagctatcaacagaaacatagtccgggtatttttgttttatcgctggtcaccatttgccgcgcttaaacgtaagtgactaaatgtctagtgtggacaaaacggcagccggtgatagtataattttttgaagatgcttatagatctaaccgcgaaaggtttgaaaagattcctcgttatggccctcttgtttacaggtaccgctctccaggcgcagcagtctgataatggagacggtacctttacaaatccgattatctgggctgattttccggacaatgacgtgatccgtgtgggagatacctattacatggtaactactaccatgtattttttcccgggtgttcctgtgctgaagtcgaaagacctggtgaactgggagtatgcttccaatgcggtggagcggtttaaacaacatcccttctacgatctaaacggcggtaaccggtatgggaagggccagtgggccagcagtatccgttatcacaatggaaaatttcacatcctctttcttacgctgaatgaaggcggctttttatgcacagcccctaaagccgaaggtccctgggagatacgaaagctggcaagaccttattacgatgcaggcctttttttcgatgacgacgggcgcacttatatcgcgcatggttataacaaaatatcagtcacagaagtagattccagcctggccccaattagcagggacagtgtggtgtttgacaaggtgcagagacccgggctggagggatcgcatgtttacaagataaacgggtactactatatctatgctacttatggtggtggggatggttatcaatgttgtctccggtcaaaaaatatttttggtccctatgaagagaagattgtgttaaaggacgatatgaaccttcatggcaggggtgttcaccagggggcattgattgaaacgcagaaaggggaatggtggagtgtgattttccaggacaggggaggcgtaggaagagtgcccacgctgcagccggttcagtgggtagatggctggcccatggtaggaaaagatggccgggcagtggttacctatgccaagcccaatacaggtactctttcacccgtgcgggtgctgcctaccagcgacgaatttaatacagataagccagccattcagtgggcctggaaccataatccaaacgacagcgcctggtcgctcaccgcgcgaaaaggttatctgcggctgattaccagcggtattgtaaccaaccttccgcaggcgcggaattccctggcccaacggatctttggtcccttctccgatgccaccacggagttggatgtgagccacatgcaggtgggagatgtggcaggtcttgcagtattacaaatccctcatgcactcattggtgtaaaggcagcagcaggtgcaaagtttattgtaatggaaaatgcagggaaaaccatcgatagtattgctttagggaaaaggaatgttatctttttcaaagcgtcggtcaatacggttaaagaccaggctcatttttcttatagttttgataacaaggtgtttgttcccattggcgatacgttgaacatgaagtttgacctgaagatgtttaccggcaacaggtttacgttgtttaactatgccaccgtgcggccgggcgggtatgtggattttaactggttccggatggatacccgccaggggccgcccaatctttttaaagcggcttcgtttgttcaggcggaaatgtatgatgaaatacacctggggcatgccaccgccagcaaggatttgggccatcccggtgatcaggatatctccaatttaaccgatggttcctggatcaggtttaaccaggtggattttgagaagggctaccagcagctcctgctgcgggtttctcccggacaggggcatgttaccgtgtatgttgacaaagattccctgaacccttatgcgtccatcacgctgccttccactacggctaaggaatatagcaccatctctataccagttaaaaaactgacggggaaacaccggctgacttttaagtttacgggagatgcgggatcgccggtgagtcttaactggttttctttcaccaacgccacacccggaaagaagggcaacgccgccagcgttgttcccgggttataactgcttatgttgaaattattttattcacttaaatcaaagaaaatgtattgtacaccgggaaaaacatcgtttaagtacctgttgtccgtgatagttattttttacatggttgcctgtagtccgccacgtgccggacgtgcgatcactgaaggaacaaccggaaaatatgcttcccggccactggtgtctcatatctatactgccgatccatcggcccattattttgatggtaaaatatttatctatccatctcatgatactgcaacaagtactacagagaatgataatggtgatcatttcaggatggccgactatcgtatcctttccatggattccattggaggaaaggtaacagaccatggtgttgccttgaaggtagaagatgtaccgtgggcttcgcagcaactatgggcgccggatgcagcgttttcacagggaacttactacctgtatttccccgcaaaggataagcagggtttatttaaaataggggtggctacttccccgaagccagaaggtccatttacggcagaaaaagagccgcttaaaggaacctatagcattgatccggctgtattccgggatgatgatggctcgttttatttatactttggaggtatctggggagggcagttgcagaactggaacaacaaccggtacgattcttccgcaaagctgcgtaataaagatgagacagcgattcttccgcgtgtggccaggctttcgccgggaatgaaaagcctggaaggggagcctgcagaaataaaaataacagacagcaatggtaacctgttcctggaaaaggacaatgacaaacgtttttttgaagccgcctggatgcataagtataatgggaagtattatctctcttactcaacaggggatacgcataatatcgtgtatgcgatcggggataatccgtacggaccgtttaaataccagggggtgatactgaaacctgttgatggctggaccaatcatcactccattattcagattggcgataaatggtatttgttttaccacgatacgcagctgtccggtaaaacccatttgagaaacgtgaaggtaactgagatgaagtataatagtgacggcactatccagcctttgagtgcatttaaataaaattggaataaccacttcatgaacaattttcatatgaaatataccagctttgctgctattactttgatcgttatttcggtgagcttttgttgcctcgcctaccgttcacaacccgctgctgctcccggaacgggcgggttgaaggattactacaaaaattattttcctataggcgtggctgtttccgcccgtgccctgcgaacagatgaagcgggattgcttatcagccagtttaatagtctcacgcccgaaaatgccatgaagatgagcgttatccatccccgtgagcaatggtataactggaaagacgccgactccatagcggcatttgcccgtagaaacggcatgaagttgcgggggcatacattagtctggcaccggcaggcgccggagtggatctttaaggatgccagcggacagcaggtgtctaaagaagtattgctgcagcggttaaaagatcacattacaacagtagtgaaaaggtacaaaggcgtggtgtacgcctgggatgttgccaacgaagtgataagtgatcagcgggatgaaatgtaccggaattcgccctggtaccagatctgcggtgaggaatttattgagaaggcatttcagtgggcgcatgaagccgatccggaggcgttgttgttttacaatgattataatgaaattaaccccgtaaagcggaaaaaaataatgcaactgttgactggcctgatcgccaaaggcgtgccggtgcatggtattggccttcagggccactgggcgatcaatgagccctccaaagagcagttggaaaagacttttgaggattttctcaccctgaacctgaaactacaggtcactgaactcgacatctctgtttacgcaaaggagcacgaaatgcgggaaaggcaaccgggtgacagcgcctttgcttttactgctgccagggaacagcggcagatcgaacaattccgtatgtgttttgatgttttccggaagtatagtaatgctttaaccggtgtgacgttctggaatatatctgacaggtacagctggcttgataacttccctgtacgtggccggaaagactatccccttttattcgacaaggatttgcagccaaagaaggcgttttggtctgttgtcaggttctgacaacgtagtttcctttgggttccgggaatctaccagcagtcggttatttagcccgcctgtgccgtagccgtgcactcgtcccaccaggccgatagcacggctacggtgtcttagtacagaaaagccttacagttgatgtattgaatacagaattagctttacattttggagattctttcagcgagcactttacagtagcagagcaatctcatccaggattcgccggggagatgtatttttgaggtagccttggttaaggaaccaggaagtaaaaggatgacgtggaaatgcttacctggcctaatatgcggtggtataaagccatagccggcacgcggccctcaaatcaaaaaaatgtaaattcgcattgttttatatacaccgttttatgaagcaatttatattacctgccggtcatcctactgccggttcacaaaatacgatggagcaggtggctgttatgctgtataacccggatgtggcaaatattaatggcaaaattgaattgcggcaaaacttattcagtttcctgctggagggccagaagagcgttcaatacgccggatcacaggtaaccataaacccggatcagttcttactgctttcatccggcaattgcctcatgagcgagaaaattgcagcgcctggtggtcgttacaggagtatcctgctttttgcggataataaagtgctggcagatttcttcctccgtcatccccaggccccggcgcaaagaaaacaggatgcacctttcctggtgtttgagaaagatgcattcctgataaacttcattgagtcgctgggttttattttagcttccggtgtgcctccatccgcggaattgaggaaagtgaaactggaagaattgctgctgtatttaagtgagcactatcctgagaaaatccaggggctccgcaatttcaacgatgaaactgacaacgatttgctgatccgccacgctatcacggcgaacatgtataatacggtgaccgttgaagagctggcctttctatgtcacatgagcctgtccacctttaagcgtcgctttgccagaatttatggtacttcgcccaataaatggctgcttgaaaagagaatgcagaaagcggctcaattgcttaaacaaggcgaatgcaaagtaagcgagatatattttgaacttggttacgagaacctgtcgagcttcattcaatcatttaaacaagtacacggaataacccccaagcaattccagctgtcaaattgaacgtttagcaacactttttgaacgttgcactatctgttgccagccctcttccgggctacctttgaataaaattcataaagttatggcaacactagcaacagctacggcacccggcggcggcgccctggcgcaggcattcaccctgaagagcaacgagcttggcggtcagttagcccgcaaacagtatttcaatggcatgggattctccggcgaaaaccaatcaccgcagctttattgggagaacgccccgaaagaaacgcagggtttcgcagtaaccatgcatgacctggacgctccaaccggcagtggcttctggcattgggtagttttcgatatcccggccgatgtgcacgaactcctgccggatgcgggaaatccggcaaaggatttacttcctgaaggcgccgtgcaaagcaatacggatatgggaactcccggctacgcaggggctgcgcctcctgatggccccgcacatcgttatgtgatcacggtttatgccctggacaaaaaactggaactggataaaagcgccaccccggcgttagtaggtttcaatatacacttcactaccctcgctaaagcctcgctgctggtatacggacaaaaacagtaagccgcattgaggtaaagagaaacatcaggaaaatggacaaaaagtattttataacgctggcagactacaacgtctgggcagataatattgctatgggatggctcaatcaaatcgatgaggagcaatggaaccaggctatcatcagcagtttcagcagcattcaacaaaccgccatgcatattgccagtgctgaaaaaatctgggtggacttctggagaaaggttcctgatccggtttatttatctgccgggtttaaaggcacgaagaatgatttaatagaaatttggagaaaggcatccgccggcctgagaaatttcatagaagaatatccggaagaaaattatctgcaaaaaatttcttttataaaaccgaatggcgaagaagaccagatggagtttgtgcaaacattccctcacatcattaaccattctacgtttcaccggggacagttagtaaccatgctgcgccaggccggcttcacaaagctgtcttcaaccgacttgtttaccttctatcgtttacactgctgacatagggttgtcacacggccggaatagctttgtactaaacaaaacgaagtacaatatgaatttatcttccatccgtattattactgccgatattaaacgcctggtgcagttttatgagagcatcaccggagtgccgtttaaatggtatactgatgattttgccgaactgcgaacgcctcttggggccctggctataggaagtacccgcacgttagctctttttggaggaaatgaggtggctacagcttcgagtaacaggtcggttatcattgagtttggtgttgacgatgttgatgacaaataccagcagttggccagtttgctaggcgaacaggtggtgcagcaaccaaccacaatgccgtgggggaatcgctcactgttattcagggatccggatggcaacctggttaacttctttaccccggtgacgcaggaggcaaagaaaagaaacgaaacaacagtgtagggaaagcctttgaactgatggtgattttcctggttttattaaaaggtgaaagctgctccctgagcggctttcaccttttaaattggcacattcaaactatactcactgaaaaccgggtctaaaaatagataattcccagttctccgtctgtttcaagaatggtggcattacctgcctggtgacttctgagtattttaacgggtggatttgtttccccgtagatgcctgtcagttgcgcatatttttcgccaccctgttctattattgaaacggagtttccatactcgtcgctgtaatcatctccatataccattttcatggtataggcagtagggaaaagatcgcctgcatgcagggtttgcagctggagctggcggcctggaataattgctgtaatcaacaacgagttataattataaggtgttgcctttattttattcaaaaaggtttcccggctgatattattcctgagataactgtcacttgccggtagaaagatagtgtaaggccggtcggtatgtgctatatacagcagcacggaatcgtagatccttttatggacgtcggcataattaccgccagcgagcacgggataaccccgtacgagcgtatccatataagagaacgcaggatccaggtgcagccaatcctttacggtattgactgcatagctggcctgcctgatagggaaagggacaggaaaagtatctgaagggccatcataagtatgccatgataaaggtccggtatctgcatttgcaggtagtttaacaagaaaggtatcactgcctctctttgaaacgatttttaatgctgcgtttccgatatagaagaaattatcactatcctgcctgctgaaattctccgtgtataaagcaatggtatctcctgcaaacgcatagctgggccagtagctttttattaacggggtggggtttaccgctatttcaggaccatctgcacttttaaattgctgattatggctgatcgttacccggatccggccattcagcactttggccggaattataatggcgatgctgtctgcagaccggttcagtatagcgccggggcgcccaccgataaatacttccgtaagcaggccatcctgtataagcaggtggccatatatcgttagccggtctccggtttgtgcaaacgttctgctgactttattgatcaccggtgtttgtatagccaggtcatctgccggaggctgatctttcttacaagcaatcagcaaaaacattaacacaatcccgggtatatgtttaagtaaaaaagttgttttcattattacggttgtaaggtcagaaattggtgatcgtagaaaggttgatggttttatttacattgccatctaccggttggcggtagccgcggaggatgactgtatagcatctgcctgcttccagtggtaccgatttgcggaccagtgttctttcttcacctgtaacatcatccctgtacatgatccggatggcgggcttgggaccgggggaaacggtggcatagttgctcacaccacggaaggcaatgtttttgatcgcatcaaccgcggtggtatcaatcttcatatatactgtgcccatatcaggcgtcagatgtaccagccttatttttgcatggtcaggatctggctgtacgtcgtcatgggtatagcgtatttcataaaaccccaggctatccagcaggtaaagcgtataatgttgatggttttcaaatttcagcagggtttccgaaattttatgcgcgttgtccggcagattggtggtatcagtaaatccaattttgaaaacaccggtatctgtgtaagtgtatttggaaaaattgaatgcgcccaccagtccattgccattatcattatagctacggggcccataaggtgtattattcaccagcaccatactattggcgccatagaaatccggtacaccattgtataccatcaggtacgcaagggtgggagaagctggtaattcattatccttcttacaggatatcagtaaccaccctgttgccaggaccaggagaagatatttttttatcattgttttttgactttaaatgtgtggttattattttccaatgactatttttacaattctcacatctgctccacagcacacattgtcataacctacatacagatcgccgaattgatcaaatacgatcctgtttggcctggcgagtatacaattattgccgggatgtggctcctgcataaaagcccgctgggacttatactccggcggaataggattttgcatgggaccgcctgcaatcaccgcgatcgtttccgccctgaggtccattttgtaaatagtggtgaacccaaaaacaatattcccatcgaaatcggtatcataggtagtgatcgtatagggcaaacctacttctttgaaggtgccggtctcgtaatcactgcgttgtccctccggtaagcctacaatggtggaggcctcccgggtatccaggtttatttctacaatgttagtgccccatccggcgccattactgagaacatagagtttgccattgcctgctattaccatgttagtagcgttatagaagcgtgcttcatcaccaaatccatcactatgttccatgagattgatgtacaatacaggatggtaggtaacgccatctgcgtcttcaaaatcaaatacttccctgctaactttacccattatcgttttaatagagccatcgggtttaagcacccggagcaatgtttccatatccagaaaatagagatttccatttttatcaaaagtaagcccgttgggagaagtgatcatcgctgaatctgcaggaccatcctccaatccacggtagttcattactgtattcgagtaataagcatctatactgcgtttgttattaccggcaaggatggttactttaccggtggcggggtctaaactctggatcagcgagtaatcggctggtttttcgtcaggcgttgcaggcgctactgtaaacaggttcttaaagtataatttgccgtcgggcccaggtttcatatcaacggtattggctgcactggggctaaaatcagttattcccagtttgagtttactaccagtggtggcaaaataatcatcgcctccccctgcaatggtggttaccattccgtttttgatcatccggatgcgtagggagttatcgctctgctgaaaatcgatgaagtaaaaggtttgggtattgcgatcataggtcagctgcttcactacgtttaccactgcctgtctggaaggaccgtctttcagctcaacagggaaagtgtattcgtatgccccgtcactgtttttcaggctatcggaatacgagaagaggtaaggtattactgttacctggtttggaataaggatgttcggccgttttaccacaaatggaagggcgggttttgcaagtccgttcacggagaagtaaatattacccggaccaatgtgagccgccttgggaacagtgatattaaaggtgtccataggtacctgcacatgttctccaattgatgttaaaagcgtactgttgcctttaccgtgggtgagtacctgggcttccacgtccgaaacgaatattttgacgactgctgccggatctcctattttggcatataccgtaatcgtttcatcgatctgtgcttccgtaatattgacaccagccttcactaccttaataatgccggattcgttgttttgaagatccagtttttccctgaatttattgcagcagcataagaggagcggcagcaggagcaggtatacagtgggtgattttatttgcatatgggtacatatcatgacaatcagagaataatgtttaaagcgagtgaatagtaaggatgctggtagtatctgcgatatataatgtctgcctggtcaaaagggattacctgcccaggctcaggtgcaataccttttaatttatcaaagtgatagttgtgtttccagtcctggtaaagcagtacaggcgtattcagcatattctgtacaccggcgcctatgctccacgttttattgatgcgttgcctccatgtcaggtccagctgattcctcgacttcatcatgatgtcggtatccgccctttttccctggttggcgcccactgcatagatgtagtcggccgcacggttataggtaatggaaatttttgtgccgaggccggggttttcgtagttgagagcagcattgatcaaatagggcgactggccctgcatgggcctggacctggtgccttcatagcccacatactgtggcatggaaggcacatctacattgcttttgaaccaggatccattcagaaccaccgataaattccggaagaaattgcctgaaacgaaatccaggttctttcttagttcggcttctatgccatagacgttagctttgccggtattcacatacacaaactggtcaaaaccttcactaaagatcatcctgaaacgttcaataggccggtcgagttgtttataaaagaagcctacatttatcagttcattactaccggcgccacggggataccattccagtcgcagttcggtgttatgaatatttactgttttcaaatccgggttaccgttgtaggtttcctggtccacgtagttaacatattgcataggcgcggcttccctgaactcgggacggttcagtgttttgccataaccgatacggataatcagggagctgtctgccttaaaagatgcattcacggagggcagaatgctggtaagcggctgatctacaataagcggatacgcagcgaggccgttttcgtaggatcccaggatacggaagtggttgtcttcaatcctcacgccgccaaatatattaagacgctcctgtaacaggttaatatcggtactgatatagcctgctttcaacgtattgtctgcatagtattggttattgggggttgttttttccaaccaccggtaaccggttccgtctgtgcggaacatggagggatcaaaataatgttggaggtatttttcttcaacgagctgaccatttcccattacctccccgttgtcgccatcatattttgaaccccggatggccaggttggggtcgtagaggtttacaccgtttacgataataaagatccggttgttgaaattcctcattcttgactggtaataggcgcctgctttaaacccccatacatccgtaagccggtaattcaggtcagtgtttgcctggtagcttttttcggtaatgtcattgaaagagcgggatagtgtatagaaagaaatcaattcagtgctgagggcccagggactttctccggtattggatagctgcctgttgaatgtatagtcgcggttgtctggctcctgcttatggatagtggaatagcctgcatttgctttcagttcatttcttttattttttccaaaaaggtatgttccggcaaattggccggagtacagggtattttgtacatagtaaagattggtatggcggaattcctgacccgggtaatcatccagtttgcggtaatcttctacagcaatacgctgattattcacgttgagaaaattatgaagcgccagtgtcagccggtcactgacctgcatttcattatcctgtattatggaaatcctggcggcatgaataccttgtgtgagctgcccgtcatagaatttatatagcgaacgttgttctgaaagtctgtgttcgtgggtgtttgaataagaaacggcgctaaggtttttcaggtatttccgtcctgttttccaggcatcgtagtaattgagattcagccgcaggtccggtaacgccgtgtaggttttatccaggacataaatatttttgaactgctttgagtatccggcattttctgcagggataagatgattgaaatttgcggctcttggtatcccggaggggagtttgcgcgtaccatcatcaaaacccaggaaatcatatttaccgcctgcataagaccagacattatcgaatgtagaaccggaacggtactgcgtagaaagctgaagatccacctgccgggtcatctggcttttcttggtatatatttttacaagtccgcctgaaaactctccaggcagatcaggagaaggagatttatacaccataatacggtcaattgcgttactactgatcacatcataggagaatgaacggctgtcagcatcattggcaggggcaattgcatcattgagataggtaaggttatatcttttgtttaacccacgaacgataacaaaattatcttctgaaatatttacaccgggcactctttttaccacttcagccgcgtcacggtcaagtgttctggctatttgctcgctggaaatgccggacactactgatttggcattgtatagttcccggatcagctgtgcatctgtggtattggccacccgtttccgtttaatagcagttaccactacggtgttggcagtagtggatttcacctgtagctttacatccaccgtattatttcccgcttctatccggatcatctggtgggtagtagcatagcccgtataggtaaccgtcagggcgtatttaccggcttgtatactattgatgttgtaaaaacctttatcgtcactgatggtgatcttggcggttccatccagtcgtaatgttgcaccgggcaagggctgcgcattttcgaaatcaacaattcttccttttaatataccttctgctgacgctgtttttttttgaggaaccgggctgacggcagcaacctttctcacagcaatattttttccggccacggaaaatgcaagaccataatgttcttccaggtattgtaatactttaccgaggttcgttttggtaaagtgcacgtcgcggatggtgatgctgtttaataccgctttgtctacagagaaagtatagtccgtttgtttttgtatggattcgagtaacgcggatgcgctgatggcggcggatgaatactcaactttagctgtaagcccggagaatttttcctgtgcttgtagcgtataaatggtacaacacatcagcaggcataaacaccctcgctttaattgtataggaaggaacttgaatagcaaaagaatttcatttgccttatagtacatagaaagcatacattaatttattttaagaatagattatagcggggatatggccccgctattggcgttggtttaaggcatattgtaaacggtgatatcctggccgtgctgttgtatatagcagttggagatgaaaagtatattatttaagatctcgctactgctttctttccggaagatggctgttatctttttatctgacagtgctgattgcgttccttttgcatagtgtataaccaggtgatatcgtgcggctactctttgtaccgcatccgtgagcggcagatcattaaacaccagtgaaccgcttgtccattcttgcggatcattgattttaatctgctgccgtttaaacgtatggctgcttttttcgtaatccatcacatcgccggggtgaagccttgtagccatatgatcggcgctgtcagcagatgcaaccgtaaccaggccacttaccaacgacactctcactgctgcttcatggggataagcttcaatattaaaggtggtacccaacacacgggtagccagcttatctgtatacaccacaaatggccgggaggcattttgcgccacatcaaaaaaagcttcgccatccagttttatactgcgctgccctttgccggtaaatggcgtataggataatttactgcctggcgccagccacaccttactattgtcaggtaatacggctagttcgggattgttatgatcattataaatggtggtccaggtaatgggcgtcgtatgattcctgttcgtaataagccaatatgtagttcctgttaccatgaatactacagcagccgctacgcgcagccagcttttccgccatttctgcgaagcacgttcaataggaataacctgctgcctcccataagttttcatttccagttgcatcagcatacgccgggtaatgtcttcgccaatattgccggcaggcaggtcatcccatgattgttccataagggaaatgaattcctgatggtcccgtcccgccaggtacttaagcacctgttgttcttcctgttgcgtgcatgttccgtcaaagtatttactaagcaaggctttatctatcatcatgaagtgcatttaagatctccgctaataataacacagcactggcataccagaaccctaccgcgaaaagtggagttaacatggagataacattggtgagtgggcatgtgaattaatcattatcttttataagagaagcggcagaaggtaaaacttttccaactttgtagctccccgataacgggaagtaccagcaatatggatatgcaatcacttcacctggaggaaaggtttaagcggatctacctggacaataaagaccgcctttatcattttgtaaaacgatatactaaagataccctcgtggtagaagacctggtgcaggagtgttttattaaggtatgggataacctgccctcgctgaaggatgatgcgatgatctatcccttgttgcgcacctatgtttaccgtataatagtgaaccacaatcagaaggaagcaaggcgtttgttacgggatattgcctttaatgagaagcaaccgctttctgtatctttcgaagaagacctgatatttaaagatggttggcgtagttttcatgaagttattaattccttaccggagaaacgccgtaaaatattcctcctgaaacaacaacatggctatactcaccaggaaattgcagatcagttaaagttgagtgtaaaagcgattgaaaagcatctaaacctggccaaccaggtactgcgcaagaagtttgttgcggataaattagtggtggtattgatattattgggaatgcaggcggagtttatgtagcgccggcaattatgtgcaacttatagacattgaatgaatagtagcttctcaccagcgttaaatacatttcatttcagagaaatgtataagttttaccgttaaatgttcaattgcgtgacgaaaggctgatggaactttgtgttataaaattcaatgattatgaacacaacaaatcagccatcaaaaatcgtcctggtgaccggtggcagccggggtatagggaaaagcattgcattaaatgcggctaaacgtaatatcggcgtcatccttacttacaatagcaatcctgaacaaggccaggcggtagcggatactatcaatggcaatggcggaaaagctgttgctttgcagatggatgctgctgaatttagctccatcaacgatttcgtcagccaggttcaacaggtacttaaaaaagaatggaaccgggaagacttcgactaccttgtaaataatgcagggatagcccagcgaacgctgattaaagacaccaccccggagattttcgaccagctcgtaaacgtaaatttcaaaggcgtatttttcctgacgcaaaagctgattcccttgatgaaggagggcgggcaggtgatcaatatttcatccggcctggcccgctttgcttttcccggtgttgcagtgtatggtgcgctcaaagccgggttggaaggattgaccaggtattttgccaaagaatatgcggaaaggaaaattcgttttaacagtgtggcgcccggagccattgacacggagtttggcggaggtaaaggggatgaaagtcaccgtcagcaaattgccggtatgactgccctcggtcgccttggagaggcggatgatgtaggcgcttttgttgcatcacttctttcagacgacagccgctttgtaaatgcccagcgaattgaggttagcggcggtatctttatctgattaacgacagcggccacctgtcagatggccgctatgttatcgatatctctttttttattaatttactttatggcaacaccaacgaagtatatcgacatcaaatcgatttcggaattgcatgatttttttcattatgataagccactgcacccgttgataagcgtggtggatttgtctaaagtggaccggtcgcaccggaaggcaggggcggcctaccggttggatttatattccattgcgtgcaagaaaatagaaggctcctttaaatatgggcgtacttcttacgatttctccgaaggttcattgatgttcacagctcctcagcaggttttatcgcccggcatagaaaataaagtggaaggctgggcaatttatatccaccctgattttttgcacaccagcaggggacaaaagctgaccggctattctttttttgggtatgataccaacgaatgcctgcatatttcggatgctgaaaaaagtgtgctggaagattgtctgaagaatatcagcagggagatctcgatgaatctggatactcattcacaccatcttatcctgactaatcttgaattgatgttatcctattgcgcaaggttttacgatcgccagttttttacaagaacaaaggcaagcaatgatattatagagaaatttgacaggattttgaatgactatttcgcccaggatgctccaatagcgtccggtgtaccggatgtgaaatatttcgcctcgcgtcttcatctctccgccaattatctttcggatttattaagcaaatataccggcaagtcgacacaggagcacattcatctgaagctgatagacaaggctaaatccctgttgtggggcaccgacaacgctattgcaacaatagcctacgagctgggatttgaacacccatctcactttacaaaattatttaaaagcaaaaccggttattcaccgagggaataccggaacttgaattgaatgaacaaggcccgttgcaaagcgggccttgttcattcaattatttaactatttgcatacatcaggcgctcaaatcaataggcagggtatagatgcgtttacctattgcggcataaatcgcattacataatgcaggggtgaaaggcggcacgggaggttcgccaataccggttggctgggcatcactttctatgatgtgcacatgtatttctttcggtgactccggcatccggataatctggtagccgtcgaaattgttctgttccacctgcccgtttttcagggtaatagcactcttcaacgcaaagctggccgaaaattgcgcacctccttcaaactgcgatttgatcctgtcagtgtttacggccgtaccacaatcgaccgcataatggacgcttggaatcgtgattttgttattcgcatctacctgtacttccactacgcaggcaacgtacgttaaaaaactccggtgcgcagcaaagccaagtgcagatcctttgggcattgtttttccccagccggattcctttgcaacccgttggataacgcctttcatccggctgatttcccaggggtaattggcgatatcctctccataattcggataagtggttttcaccagttcctggttgaaggtgatgttacggtcttctcccagaaggtcaatggcattggcaacagcgtccattcctcttgcttccgctacttcgtccagcatggtggtaatcgcaaatgcctggggaatgttacgcacggatctcagccagcctatacgcatgtgtgacttggcatcatgcgtttctatttgtatggcaggcgcgttataggggaagtcagaagcacccagcgccagctctccgtcactgggttgcaccacggaaatatcttctgtagccgaaatggaggggtaggcaatgtggtgattccagccactgagcttattgtcgtggtcaatggtggcaacaatgcgttgtacgcttaaagcatggtggtaatcgtgatggatatcatcttcccgggtccactgtactttgatgggaaggccggattcttttgcgagtatggctgcttccagcatgaaatcgggcttggacttacgtccgaaagcgccgcccagcagggtaacatttatctttaccttttctgcggaaaatcccaatgcttctgcaatggcatcccgcgctccctgtgggttttgcgtgcaggcccaaacttcgcaggtgccattttttaccactgcgagcgcgcagggtggctccagggtggcgtgggcaaggtgtggcgccacgtaggtatgttcaatcacttttttagctcccgattttgcggcgttaaagtcgccccgctttctgcgcaccgttccatttttcgcgacttccagctttaattcctcgatttgtttggctgaatcataggtagcattaggtcccaggtcccattccacttccagcagatcgcgggctttgatggctgcccaggtattttcagcaataaccgccacaccactcaggggttttgttaaagtagccggaagacccgcgcccttaatggcaataactttgatcacccctggtatgctgcgggcttttgtatcgttaaacgactttacagaaccgcctactaccgggcatctttttataaccgccactttcatgccttctgtcacggcatctataccaaaaacggctttgccacttacaatatcgtgcagatccacaatgggagttgctttgccaatcatattaaagcggctgcgatctttcagtttcacactggccgcaaggggaaccggtaaaaggttggcggcgtccaccaactcgccaaaacccagctgcttattcgattttttgtgaaccacctggccgttggccgtgtcgcattcctctacgggcacctgccatttttttgccgccgcctgcatgagtaaaagtttggcgattgctcctgcctcacgcatcggcttatagaacatccttatggaaaaggagccatctgtattttgattgccatatttcttttcatcgccttctgcctgcacaatctgaaccttgctccaatcggctcccaattcatctgctataaccagtgggagggaagtccggatgccctggcccatttcagagcggtgggcaatgataatcacttctccggccgaagtaatacgtaaatatacattgggagctaaagtggcaatcttttttcctttttcattacagctaaaaatactcacacccaacaccaaacctcctgcgagtaaactacctacttttagaaaatctcttctggaagctctgaagatttccgatgctacggcatcggtgttcttctcaaatggagatataaccttcatggatctgttctttttgaatgactgattaattagacagtagcagcacttagtatagctgctttaatcctgttgtaggtgccgcatctgcaaagattgccctgcatcgcctgttcgacttcctgttcggacgggtgcggattctttttcagcaaggctgctgcattcatgatttgcccggtttgacagtagccgcattgtggcacgaccagcttttcccaggcttgctgaacaggatgatccccttcttccgccaacccctcaatggtggtaatcttatcggcgccaactgcggaaacaggataactgcaggagcggatggctgtgtcattgagatgtacggtgcaggcgccgcacaaggctttgccgcaaccgaacttggttccctttaagccaatgatatcccgcagcacccataacaatggcatatcttctaacacatccacttcgtgtgttttgccatttacatgaattgaatatttagccatattgctttatttatttaatcttgatcttgcattggagggtatatagtacctggcaggtaatgatctgcactttaacatgaaaacaaaactattgattaatatacttaggcagttaagaaaaagaaacgaatgattatgataatcaatcaatcgtccttcatctgacaagcagttatatcgatattgaatataatgaaaaaaggcaacaatctgtattcttacaacaaataaggcggcgcgatatatccggagtctgaacaataacaaaaatcgtcgcacaggcatggccgcctgtcgttgccggagctgaacttttgatccgtggtaatacggaagaatcccggtggggggaaaatgaggggtggtccgaagcttcgatgattccttagaaatgaatattttataaaaaaagtatacctaatattttgaaaaataaaataattaagtacttttgcaccccatcgaatggggaaattaccggtaaaacgggacgtagcgcagcccggtagcgcgcttgcatggggtgcaagaggtcgctggttcgaatccagtcgtcccgacaagcctcaaaatctttattagtaaaggttttgaggcttttttattgctggcattttatacttccctgcgtacgagaaagtagctggaaagcacaatacttcacaaacaattaagccccgataaatatcggggccgtttgtctaacctacaactgattacactatatgtgttattgttacccataagtgttcagaaagtatacatctgcattatgttcaggaggaatgttggccaaacgcagcccataataccttagcaaccggcacctatcacgattcaactacaaaaattaaggttgcccggaatgaggcggctttcttgctgcttatgaagtaccctcgatggaaggctgcttacgatgacgggaaaggcggacaagtataccatccacaatcaggtacattgcgggtaccacaaagagcgtgagtatcatagaacttgtcagccccccaatgattacccaggccattccgtttttaatctcagctgcggcgccttttgccattgctataggtaacatgccaaaaatcatcgcgagcgttgtcattaaaattgggcgaagcctttccctgcctgcttctatcagtgcttctacagttccatgtccctcctctttgagtttatttgcaaagtcgacaatgagaatagcatttttagcgactaaccccaatagcataatcatcccaataattgtaaagatgtttaatgtttccatagttagcgccagcgccagtaatgcaccaaccagtgccactggtatcgaaaacagcactacaaatggatacaccgcgttttcataaagcgctaccatgataagatataccagtacgattgcggtgataagtgccagaccaaggcttccaaaggcatctgcctgattcctggaatctcccaggtactcaatattaaccccttccggcacctttatagattttgtcttagctttgatttcatcggctacagtacccgttggccgcccggaaacgtttgcctgcaccgtaatagacccgagccggtcaatacgctgaagagtggtttcccccagtgtttctttaacatccgcgaattgccgcagcagtattgtctgaccattagcgtttaccaccggcaggtccattatattgctgatatccgatttgctaaactgatccagccctgtcctgatatcatactcgttcccattttgtttgaactggttcttatcatccccgctaaaagcattctgtagcgcaacaccaacagcactcgcattgagtccaaggagactcattttttccctgttgagcctgatgtccacctcgggtttcctgtcctttaccgacagctttacaaactgcgctccgggaacatctgcgaccaccttcatatactcctgggcaacctgccgaacggcgctcagatcaacacctttgatggctatctgtatcggcgcattgcttacatttccggttattgaagtggaggcgactgtaaacttcacacccgctatgatagtacttagttcttgctgtagatacattccgagttcctcagaacttttacttctcccgttcttatcgaccaggccaaccgtcagttcagccaggttagcatttgcagatgctccagccacacttccactcacaaatcctatgctggagaagatcttcttcacctctggttgttcccggataatcttctccgcctgctgaaccttcatattagtcttgtaaatgcttgctgttggctccagttccatattcaggatcaaatcactttgatccgctttaggaataaacgcagcgccgataaaccccatcgggaccaacgcaattgatccaaaaatcaggcacattacaagtatcagtaaccatctcttttttcttaatactgctcttaataacctgccatattcctcttttatcatttcgataaagtactcgaacttcaaattaatccttccccaaatactttttgcagacagctgctccagtttaccaaacctgcttgccagcacaggtgtgatggtaaatgatacgaagaggctcatcagtgttgaaaaaataacgacgagggaaaattcccgtaaaattgctccaatcatcccgcctgctaatgccaacggcagaaacaccaccacatccaccaatgtgatagataaggctgtaaaaccaatctcatttcgtccttccagtgcagccttccggcgatccgcccccatctccatatggcggtaaatattctccagaaccacaattgaatcatccacaagtatccccaccaccaaagacattgccattaacgtcattaaattcaaggaaaatcccatcaggtacatggcgataaatgtaggaatgatagaagatggaagagcgatcagtacaaatgacgcacttcttatactatggaggaaagccaacattacaatacctacaattattacagccaaaaacagatcgaacataactgcattagctgcatgcaatgtatacacgctctgatccgaggaaacattaaacagcagtttctgccccgagtattgtttctctagctcacgaaagcacttctttacccgatcgcttactgccactgcatttgcgtcactctgcttaatgatttggataccaattgatggaatcccatctatgtggttgatggcggtaggctttgccgtcccatctgacacatccgcaacatctcctaactttatggtaccctgagttgggtgttgtaaaatgatcagattacgaagctccccgatcgaatccacatttgcatcgtagcggatggaaagctgtttgtttgttgtttcaatgctccctgcaggaaatgaaagattcgctttaccgatcgcatttgtcacctgcccaatagaaagcccataagccataagcctatcctgcattacatttacctgaatctcccgtttttctcccccgataatgttaacctgccccactccgggaacgttctgtaatattgggcgcaactggttatcaaccaggtcaaaaattttccgcggaggcaggttccccgtaacgccggccttaataaccggcgtttcatccaggttaactttacttatccccggcttttcagcatcaagtggtaactgactaataatttgatcggcttttcgctgtacatcacgttctgctttatcgatatcggttcccgatctgaaagaaattgtaattattgaaagattctcctgggaagttgaactaatttgatccaatccctcaactgaggaaaccgcatcttccaatttttttgtaacattggtttgaacttcagcagctgcagcccctgggtagattgtgctggcagaaaccgtaggaacatcaattttgggcaggagattgtaatttaaacccaggtacgactggacaccaaacaggatcagtacagtaaagatcacaatcagcagtagtggccgttttatggcgatttcagtaattgacatacatcttattctttacttaataacattaatcaaggcactgtctttcaggttaacctgaccagaaataaccaccttatccttgtcttccaaaccacccagtacctccagttcatccccataatttctacctacgctgatttcccgccggatagccttgccatttatcaccacataaacagctgcattagtagtactttcgattaaggcctcccgcgaaacaagtaatactttccgttcagttttctttgagaaatcggcgttaacaaatgtacctgcaagcagcggcatggatttatcattcggtgcagtaatctcaacctggtaattgaatgcctggttagcctggggactaatgaaagtcactaagccgggaataattcttcctggataaacagctgtggtgataccaattttctggcctttagccaccttgtaaacttcatcttcagtcaaatttacctgtactttcagcgacgacatattcactattgaagccacttccgttccggccgctatgaatatgccctgttcaaccggtttggaagcaataatgccatcatccggcgctttaatactcgcatcggctatctgttttcgtatctgttgagcaagattcaatgcgtcattatagctttgttgcatactctccaccttttcaagggtgacagcgtttcctgccaacagttccctgtaattattaatatccctctccaactttgcaacattcgtttctgccttttgcagatctagcgcaagcaacctgctatcaacaatagcgagtaactggccctttcttacatggtcgcccaggctgaacatcactttctgcaactggccgccggaagcagaaaacaccctggacgctcttaaaggcgccagcgcgccagttttcaccagcagttccagcataatctccgacttcacattggaggtagtgacaggtatacggatgtcttcaatgttagcaggcgaatttttctctgcaattttggttttattgtatgccaacttaaacacaatggcaattaacattgcagtaataaccagtatcaatacgattctttttttcatcccagttaaagagaatttaaaaatgttttcaatgtacccgcggctttctcaagatcaacccgagcctggtagtagttgtagatagcgttcagataattgttttgtgctgacttgagggaattctgggtaattaaccagtcattcaaatcagtagtgcctttctgaaattgaagatttgttaccttaaatactgattcggccaggtccatatttcgtttatcgttttccatattggtccgggtttgggcaactttcgtccgggcattttcaaattcaacgctgaacttactttcggaaagcttcaaactctcctctgcattgatccgattcaacacagcctgcttatgtctggcattacgtttatagaagtccaagattggaattgtaagttttaagccgactgtcgaatatggcaataattcatcaaaggcccctctcaatttttcgccaaatccaacagcgccataacgtgcatatcccgttaatttgggtagtccttcgactttaatgcgagcctgttctatctctaataatctgatattagcggatgatatccgatagtcaatccgggctgccggagaaaaacgcaccagcgaatcctccggaccagccagcggcgctatagcatcaaccagattaacgggaagtttatcatcaatgggatatcccatctcgaatttcaattgattctccgccaattgaaaattactctcagctaccctgatctgtgacatagtgttattgaaatccacggacaccttatccaggtccttctgtaatacaacacctttagccacttgcagccggtatatatccatctgtcgttcatatgttttgctgttaaattctaacagcagaatttgttgccggtaaaccagcaattgaaaaaaggcagcgctaatattgtagataattgattcctgactctgttgaatattgagatccgccagttccctattgaacttatttgctttaagccctgtcaacaatgactgatcgtataatacctggtcaagttgtgcaacggcattcgagttaaatttttgggtaagagacaccttgatttcattgggtccgagaactccggctggaataacattttgctgcaatttgagattgttgtccaacattgaagtaaggctcactttggggagataatctgcaagaacctccctggctttagcatcagcagctatcttctgattcgcataaatgctggcattccggttattttgcagaccatacgctatacaatgcttcaatgtccagctctcctgggcctcagctttgacatagatgcaaaagatgatcagcattagaaaatttttagccatacattctaacttattccttcgtctgtaaaaggatttctgataaaatgatgctaaaatagaccagaggagaacggcttaaattcattttataccaaaccggctggtttttatacaaaaggggataatagtaaccaatagggtgttgtgaagctatcgtatcgctaatcgggagggtaaagtttcatcaaggcttcttctggctgaaagcgccttttgatacagcagggaaatacgtatgctacctgttcgcaatcttttttgttacaaattcattgaaaaagaaatccctgtaagtatttccgatgggaatttcgtttgtacctatgtacactgtgttattatccacagaatcgatatgcttaacattaatgacataggatttgcttactctcacaaacatatcttttggtaattgatcgtagatagttttgatattcatcgccgtaatcactttctgattttcgctatgcatcacgacatagtcttttaaaccctgaataaaaagtatgttattaaaatagattttaaaaattctccggtctgctttcacaaagaaaaagtcgtctgctacctgttcaatattgttatcggcgtagtccgccttgaataatttggagtaggtgcgggctttctcaaccgctttttgaaaacggtccgattttacgggttttatcaggtagtcaatcgcatctacttcatagctgtcggtagcaaattcggaataggcggttgtgaaaatcacaaatgtttctttcggaatggttcgggcaaattcaattccgtttattcccggcatttgtatgtcaaggaaaattaattcaactgtattgttttctataaaatttttggcggtttcggggctgttgaacgaaccgattaaatctaaatcatcggtttggtcaatcaacatctctatggcttctcttgccaatggttcatcatctataataatgcagttcataatttatacgctttactatataacgaaattatcgtttgcgatatttgaatttgatcacgttcatcgctatcggatcgttattgactattatgcaagttatagctttatagttaaggttacgcaatacctttctgaatcatcttctatatttaaacgatgtgttgccgggaacaaaagttccagtcttcgtttgatatttgccagccccaatccgcctgtattattaacggatttaagcacaggtttggaattgatacatttaaagaaaagttcatcgtttctaacatcgaaatacaggtttacataagatgcttttgttgcatcattgttgtgcttcaccgcattttccacaaacgaaatgaacagcaaaggagggatttgcacgccgctcagatctccctcttttgaaatcaggaaatcaaaactatcccgccttactttctccaaatttaaaaaatcttccaagaaatgaatatccgaagtcaacaacaccttatctcttgcactgtcataaagttggtagcgaagtaaatcgctcaacttcattaaaacctgcgaggctttttcgggatctttctttgtcagaacattggcattgttgagcatattaaataaaaaatgcgggttgatctggtttttcaattgttccagttctgcatcagttttcgactgcttcagctcgtagatcaattgcttgtccatcattcccttctgaaacagttttatggaagatgacgctgctaacagcagtacagtaaggaaggaaaaaagtggaatattcagcgcattttctttattaataggattaaaaaaatagccacaaacagccattactaacaggatgatgatcactgataagcagtatttgatattcttattcctgaacaaaagctttggtaccagcacgtacatatttacataaaacaatattataaaatatacaaatatcgctatcgggttggcaattacggaagcgctgttgtacaatacactacctataaaaacaatgagcagcaaatgacggaatatcctgaggtcaggtgaaaccaggaaacgaaacagcacgttttcgctaataagctgttgatggttaaaatcattcatttataaaattgtatatagcaaacttaacaattaaagtgatggtttgatcctggttttatacgaaagtgtacgctttttatacgaaatcaggacgcattataaaaacgcataagacaagaaatatgttttgtagtaccccggtatactttgctataaaagataccgcgtttggtataattaaaaaaaggcggttatccaaagggatagttttgtagccaattacaattgttaaatcgatttttaaaagatgagatacaaaatcatttatacactgctgtttatcgtgatttcattcggggcttattcacaacagaaggtcacattgagcggaacagttaccatgaaaacaaacaccgaaacaataatcggtgcaagtgttttcatccctgaagcaaaagcctcggcagttaccaatgcctatggcttttattctatcacgctgccgaaaggagcatatacaatcgttatcagttgtataggatttgaaaatattgaggaacatatctctctgacagaaaacaccagggcaaatttttcgatgcttgaaaaaagcagaactttaaatgaggtagtgataaaggacatgagttcaacaaacaatatccggaatccggaaatgagtgtgaataaactctctatttccaccattaaaaagatgccggcagtgatgggcgaggttgatattttgaaagctattctgcagcttccaggagtttccactgcccaggaaggagcaaccggatttaacgtcagaggaggttcggttgacggtaatttgatattgttagatgaagccgttgtttacaatacttcacacctgttcggctttttctccgtttttaatgctgatgtgattaaagatctgaaattgtataaaggtggaataccagcaaatttcggtggacgtacttcgtctgttctggatatttatcaaaaagaagggaacaaccaggaatatcacgtaacgggtggaattggagcgatttcgagcagattactggcagaaggccctattgtaaaaggtaaaagttcgttcgtggttgctggtcgtacttcttatgctcaattgtttatgaaactggcagacaaccccaattctgtttctttttatgatttgaatgcgaaactgaattataacattaatgacaataacaggattttcctttcaggatatttcggcaaggataaaatggatttcagtaattttttcagcaacaattatggaaactcattctttaatcttcgctggaatcatatcttttccgataaacttttttccaatgcatcgatcatttacagtaagtacgattatggcctgaaaataaagtatgttggcattgattgggtatcggacatccgtaattataatctgaaatataattttaaccaccgtctgtctgataagctggttttgaattatggcatcaattccatctactaccaattcaatcccggcacaataaagcccatggacgataaatcgtctatcaatgccgaccagcttgaaaaaaaatatgcctgggaaaatgcgttgtatatcagtgccgagcaaaaactcaccaataaaatatcattgaattatggtctgcgatatagtaatttcatgcggttgggggaacagaacgtaaataattatgctaataatcaggcagtggttttcaatcccggcttacaaatttatgaggaaggaacgcctaccagtataacgcattacaataaaaacgaaaagatagttgggtttggaaatttagaacctcgtttggcagtttcttttgccataaatgacgaccaatccattaaggcgagttacaaccggatgagccagtatatccacttaatttccaacacagcttccgtttctccactcgatatctgggcgccgagcgaccagtttttgaaacccgaaattcttgaccaggttgcattgggctatttcagaaatttcaacaatggaaaatattctttggaaacagaagccttttacaagaaaatcaaaaataaagcggattacattgacggagccgaattgatcgcccaaaaagccatagaacaggtattgctaaacggggaaggaagggcttacggacttgaggtgatgctgaagaaaaataccggaaaactcacaggctggctttcttatacactttctaaagcagagcagcgcacaccgggaagaaacgcaggagaacctggcattaacaacggcgaatggtatcgtgccaactacgataaaacacataatttttcgcttacaggcgcttatcaactgacaaaaaaatggagttttggcggcatttttacctaccaaacagggaaagctgcaacttatcctattggaaaatatgagtatcagggaattacaattgggaactacggagagcgaaacgccaattcgcttccggcttatcaccatttggatttatcggccacctacacgccaaagcctgacagcaaaaaaaggtggaaaggtgaatgggtgttcagtatctacaatgtttacagcagaggcaacgccgcatctattatgttcgagcaaaacagggaaacagggttgagtgaagcaaagaggatatcgattttcggtatcattcctggtgtaacttacaatttcaaattttgattctaataattacaaaatgaaaaacatacttaaatacctgattgcttcatgttgtttttttcttctgtcctgcacaaaagtagtggaagtggatttggaaacggcagcaccaaaattggtaattgacgcatcgattgattgggtgaaaggtacaacaggcaatgagcagaaaattaaactctccaccacaacgggatattacagtgcgaaatttccaacagtttccggagccaatatagttataacaaattcagcaaatactgtttttagttttatagaaaatcccggtacgggggaatatatctgctccaatttccatccggttatcggggaaaactatgcattaaaaatggttttaaatggagagatttataccgcaaccgaaacttgtattggtgtgccgaatattgacaataatattgtacagaatgataagggcggatttgggggtgatgaagtggagatcacctactattaccaggataacggcaatgaggaaaattattatctgcaccgtattcaatcacctgtatcaacgtttccggattataaagctaaagacgatgagaacagtcaaggtaacctgataccggaatatttctctgacgaagatctgaaagccggagatccggtaaacatccggctgtatggaatttccaggagatattatgattatttcaggaaattgttagcagcatccggagctggtagcggcccgtttcaaacaacgccaggttcggtgaggggaaatatcatcaatcaaacccatttcgcaaacttcgcttatggatatttcaggttatctgaagtagacacaaaggattatacgataaagtaatgaattgcgttcacagacattgcatggtaaacggaaaagtgtagatttggaaaagataccatgttcacatcgaaatataaaaatatggccacttacgtttttttcaatatttcagcatatggtcatgtgaacccaacgctccccatcgtggcagaactaagtagacgtggccataaaatttattattttattggcgaatccttcaccggggctgtgcaaaaagcaggggcatcccggtcacattgtcaggaactttacgaagtcaaaatacaccgccaccgggggataaagagattgcgcttttaccgtttttaatggcgcgtgaatcgccacgtatagtgccggaaatagtagaaaagttaaaaagtatacgccctgactgtattgtatttaataccatgctgcttgcagccagactcgcagcacggatattgcggttacctgcgatcggcttccggccattccatagtcccagacaatcgcaaaagattatcgaaacgtttactgacccgaatttcaaactacttgcacatactgctaataaagcgcttgcagaagttaccacattgtaccagattcctgatcttacccttcaggagctgttttcagaagtgcctggattaacgttggtatttctaccaaaaatatttcaggttaatgccgcacaattcgacgagcgttttttgtttgtaggaccatcctttatggagcaaccaccagtcccatggccgatagcgcaaagcagcaaatcaccagcaatcaggatctatatttcattgggcacattacgaaataatgaacctgatttttaccggatgtgtttctctgctttttcagcacccggttggagcgtggtaatgtcggttggagatcaggttgacttacatacgctggaacccattcccgataattttgttgtaaggcgctctgttcctcagaccgcgctactccctcatgtggatgtttttgtcactcacggcggcttaaacagcaccatggaaagcctgtattatggtgtgcctttggttgtgctaccatccataaaggaacaggtaacaacagcagaacgtatacgggatttgcatctgggccttattcttgaccgtacagagtttactgctgaagcacttcgtgaggctgtcacaacagtattccaaagtgaatcgatccggtattctgtacacaatataaaggacacaatccatagtgcaggaggctatttgcgtgctactgacgcaattgttgcatttcagcaggaagtgcttcctccatgttgaagtccggccccattatttatctgccagatgtgcaccgccgtttggctgactgggtaaaaaagggaggggtgttgatttattgtggcagggataacgagccatttcaatccataatggaatggtggaataccaatggcatgcattgcaatgtaccgtctatgcatcttttcggcttgctgggtatccatccggattccagcaatggccaatcttttaaggtaacggtatatgtattgcggcaaaacctgaaagaggttgtgatgggagccggaggagcgctcaaacccccaggtattgatgaggatagttcgaagtgaaaatccttttagtgatcgttttttgggtttttgagacgaaacccaatcctggtcaatttcattaaaaagtaaaccttacaaacggcacagggaaaaacccctgctggtaattgtttacgacttgtccggtacgggcgttccaatcctgtctgaaaatattattgttattggtaacgttttgcaggtccagcgaaatttctaaagatgattttctgtattccttccggtaggatagctttacatccgagcggaaataagccgattgccttaatgaaaaagcctcttcttcagtaaactgtatttcgccgtctgcaatagatgctgtaatgtccacaggtgaaagatagcgacctccgacagcagagatcttcattgaaatgctgaaatatctttccctgttgaacttccattccttgcctgcaagggcattgattacataacccatattaaacgccgtatttcgcaataccccatcgcttccctggtatttggaatcaaacagggacgtggtaaacaggtaataaagcccttttgaaaaattcctttcaagggtaaactctacaccgaaatttcttcccttgccctggttgataagactgtcccgcaatgtaggagtggcctctgctccaagattgacggtcgaaaaagaagacggatgactttccacaggaaggtcatacaacgactggtaataaagttcggtcttcaggtttgtattattgtttaatttccagttgtgtgacaacacagcatggttgctccttataaaccctaaggattcatttgtatacaagtggccggagggagtggatgttacaaccgtgtaatttagcaggttgtccatttggctgtgcattccgaaaccgaagcctaaagtatgcctgttgtttattttagcatttagccctattcttggctctatgctttggctctgggaaatatccagatattggtagtgcatccctgcaataaatgtccacacatcgttcatcctgtatttccattgagcgtagctctgcaacaggtccaaatcgcgttgacggtcagcaattaccaggtcgtgcacgccggcgtagatccgtttgttgagaatggagaagttggtatagtcattgtaaacccctgcaataaagctatgccttgcatttaacttatgattcaactgaaaaacagcagaatattttcgcgtggagaatttccagtgccagtcgggagtagcgatatcgggttttaccgtactgatagaatccctgtcaaaccattcgtttgtactgctataaccgactgttattttcgcagtagtcttattgcttagcagatgctcgtaactaagtcctgtaatgttggtttcgtaatcggcaaaacgattggagtagctatttccataagcctgtccgccgggatcataatctttgcccaggcttacaaatgaacttctgccccaaataccgaacaaactcaggtttcctttcgccccgactgatgagtgtactttataatttacatcgtagtagtcgggttgccctccgccagtaccaaagttgagccctaactgccggaatacagaaagggtggaatatctggcatttacgagataggacgcttttttacctttcccggtcggcccctctgctccggcttcaaatccgttgaaacctacttgtcctacaaattcatgcttgtctttatttccatttcgcaaccgtaaatcaaagacgcctgcaacagcgttaccatattgggcggggaaagcacctgatataaaatcagacttggctatcaggttgttgttcagcatgcttacagaacctcccatactgttcagcgcaccgaagtggttaggattgggaatgttaagaccttcaaactgccacagcatagcattgggggaattgccccgtataataatgtcatttcttgtgtcattggtggataccactccggcaaagtttatagccatccgcgcagggtcgccaaaagagccggcatatcttttggtttcttccatattgaacgtgcggacgcttaccgtagccatttcattgttgggtgatttcctgttagaagcgctaatgaccacttcatccaacatcttaattttttcacgcattgccacattattaagttgaagttctttccctgcggtgatcaataaatcggaaagaaacaagggttcgtatcctacaaacgtaatgataatagattgcctgcctaaaggaactcccataagccggaaacttccaagcgagtccgaaaacgtatttatccccgggtaatttgccatttgtattgtcgcaccaccgataggagcgaacgaggcctcgtcaactaatttcccgtttatagtttgggtttgggcttgtacattgctgaaaaaggcaatgaggaacacagccaataaagtggccttataatagattgattttgctgccataattcgctatatttatctcaggaaattattttggacaaaaatccacaacaggatcttcctgttcattgatctgggtcaataaagaaagtatccttggaaaaacagtctattgaagccggctaagtttatgtttgaaaatattcatcagtattttttgcaatttttacccaacctttctgccggggcgtgggagcctcttactgagcttttggtagtgaagtcttacaagaaaggggaaattatcagtgatttgggtgctgtaaacaaatgggtgtcctttattgagaagggggcggtgatcgcatttgatttgtctgaccggaagaagaccgtctacgagttcttttttgagcatcaatttactggagattatgaaagttttttgacgtcccgtcctgctaattatggaatagaagccctggaagattgtgaattgtatcatcttcatttcaacagcctgcaaaagctgtatgaaagatttcctgagtatgaacgcattggcaggctcattgcagaagcccagtttttgcgtgttacccaaaaaaacgccaggttgatgggagaaaagcccgaagagcggtatttgaatcttataaaagaaagggaagagttgattcaaagagtaccgcagtattacgtggcatcttatcttggagttacgcccgaagcattaagccggatcaggaaaaggctggtttcaaaatagttgaaacaccatggtggataatggagacattggttggaagaaaattaagaagggtcctctccatgttttgcaaacacaacttaatccaataggaatagcggctttatttcattgttaataatttttgtgctgatttctgatggaaactatcaattctaattaagtctgccataagaaagttcgaattgtgtccggtttttctaacttaccactacaattgaaggtttagaacctaagaacagttttactattaaaaacacttaccttgttatgaacaatatatggaaacaataatcattgcagaacgcaagagaaaatatatagcagatttgatcatttttgctatattattggctggaggactgatttctattatacaatattcagcttcattaccatccattatttttatcgtctcattaatcatcccttcagttggaatagtgaaatatttatgggatgtaccatcacaaataaaactatcagaagacgagatggtcatatactatggcagaagtattttagaggatgtagatgcgcgaggcagctttgcttttccatcaattgtaaaacttaaatggggaaatatcgcagactttgaggtaaaatcctatacgtactgcatcccggataacggtggtgatagaggagccatcacaacgaactatgagtatcttatcataacccttagtaatatagataacctgaacccaaacagcaaccagaggtacacagtcgtattaaatcactttgaaaagacaccggaggaaattcttgccatttgtaaacaatttcaaatggcatggtcctgatcctgtaccgtgcgttttccattcctaatatcaacccacatctatacttctgcagtaaccttagcatatttgttcctgtattctataggcgttaggccggttacttttttaaatgcatcccggaaagctctggtatcggtgtaccctacatcaaacattacttcgctcacatttttccgggaagcctcaaagaagcgcttagcggcctctacgcgtactctttgtatatattccaaaggagtattgcttgttgcctgcctgaaccttcgctcgaaggtccttctcccggaattaactatggccgctaactcgtctatcgacattttctcgttgtaattcatctcgatgtaatcctggaccttcatgatttcttcatcggcatgtttcttttgccccttaaacactgtaaatacggcctggctgctgcggccaatatctaaggcgaagctctttgaaattaatacggccgtttccctgtcggaaaattcctcaatcaggtataggaccaaattccaaaggctgctggcacctccgctactatatatgtttcctacttcagtaataatagcgccatccactacctcaattccagggtaccgcgctctgaactcgtcaaggtaggcccaatgtgtagagcactttttgccgttcaacaacccggtctcagccagcaggaaagcgcctaaacacaaactggcaacgctacagcccttttcatacaatttcctgatgtgtggaatggcgtcagcatttatttctattccgtcagcaatattgccatatacaggaggaattattaataaatcggttttactcacatcccggagcaagcggtcggtccttatcgtgtattcaccgtcgtttgccgaaacaaacggggtaagaccaacatattcaacctcaaatatcgcctcttttcccagggccataagaaaatcattggctgtcttaaaagcacggtagggtggcgttaccgcttctattacgcccttctctggtgcaaaaactgatattaacatagacgttgtaagattaaaagtaaagataatacatccctgtcattttcacccccctaatttgacgcatttatgtatcctcagtcccatgtatttagaccacctttgtctcatcgaactaacaattaaaattacacatcatggcaaagaaaatctttatcaatctaccggtaactgaccttaaaaaggcaatggaattctataccaaaattggctttaccaacaatccggattttacggacgacactgccgcctgtatggtactaagtgaagaaatttatacgatgctattgacccatgacaagttctcgcagtttacaagcaaaaaaatcattgacactaaaacagacattggtgtgatcaactccatttcagtcgacagcctggaggaagtaaatgccatggcagatgctgccttaagcgccggtggaagcgagcccaattcgccaaaggactacggctttatgcagcaaagaagctttagcgatcaggatggtaaccattgggaggtattatatatggatatgagcaagttccccggttaaccatgatgtaggccgaaatcccagcccgttggttaacgtcgttgacatgtactatatcagtttgatattaagtgttcaaaaataaattatacaaaaatgaaaaaggctaaaattattttttgggtgtcaactgtttttatattcctgtttgaaggtatcatgcccatcagtaccttattgtttgcaccacagtataccaatgcaggaacgaagccacttggttatcctgactattttgcagttgcgctgatcattctgaaattttcaggcgcattagctatattgttgcccccgatcccggaccggttaaaggaatgggcctatgcgggacttacgttcaacctggtattcgctatcatcagtcatgccgttgtagatgggaacatagggtttatactactgcctgtgggtgtgatggctgtgctggcgctatcttattttaacagaaataaaatgcagatcgctaagagcgagagaaaggaggatggtgtggtaatgcgggaaagcatagcttaaaaagaatgttcccctaaagccatgcagaagtaagttcgaattttgtacagtagtcagggcgacaaagaaggagctgtctcataactaaatgaggcagctcctttttattttatccacgttcttcatacgggacagaaaaaaggccctgaatctatcttttgctaagtaatccattggttataaatattcctgccatccacggctgttgccttacattcccgctattcttcctcacgctggtttttaggatcaattcgacaaaaaactgaacaaaatttaaaagagatatttcatttcttcgcacgatctcagaactgaaatataccagcagcatacactggatgaagtatgaggcggtcgttcaaagcattggaaataatcactaaaatttaaataagttctacaaaaaaagcgttatgagtaaattatttttatcgttgctggcaatgatatcttttcagtttttgtttgcccagcaggatcatctgaccaaatttccaaagggagctacacctggcgaggtgggcaaacgattggcctatcactttgtggacggcaggcatgaactctatgcaggaaggtacattcactatgccgaagtttgtacctggaatggcgccttggactacgctataaaaacaaaagaccaaaagctgatcaggcttttacaggataaatttgagcccttcttctcccgggagaaagtattactgcctcccatgaatcacgtggactacaatatgtttggcagcgttgcgctgaaactttatcaggtaacaaaagacgaacgctataagaaaatcggactggcctacgccgatacgcagtgggaagtgccaaagaatgcgaatccggaagaaaaagcctgggcggataaaggatattcgtggcaaacccgtttgtggatcgatgatatgtatatgattactgttgtgcaaaatgaagcctataaagtaaccggcgaccgcaaatatattgacagggcggcaaaggaaatggtacgctacctggatgagctgcaacgcccgaacgggcttttctatcatgctccggatgttccatattactgggcaagaggagctggctggatggcagtaggtatgcccgatctgcttcgtgagttgcctaaagatcacaaagaccgcccgcggattatggaagggtatcttaccatgatgaaaagcctgaaggagcaccaaaggcccaatggaatgtggaaccagcttattgatgaagcagatttctggccggaaacatccggcaccgctatgttcacgtatgcttttattacaggcgttaagcaaggatggctggatgcggcggagtacgctccggcggcgcgaaaagcatggacagctatggtttcgtatatcgatgaacgtaataatgtgaccgaagtttgcgttggcacgggcaaaaagaatgataaacagtattaccacgaccgcccacgtaatgcgggtgaccttcacggccaggcaccctatctctggtgcgcagctgcacttttaggaaaatagttggagagttttataactgccgttggcgttggcgcccctgcacagggggcatgacgccaacggcttatcctgaaaagctgttttcgcgtacctgtgatttaacacctcccttttctatgcttccttattttggaatgattcgacaaaaagttgaataaaacgtatcaaaaaagaatttttacttcgcgttacagtattaatattaataattatccacaaatatgtgtgtccacttatgaattggccaggagtcgcgccggtgaatattccacgtatctcaaagaatgaaaactttcaaagaactacgtgccttggcggcgtatgtatattattctattaatctttttaacgattgtggctattaaaacaaccatgggtctctataacccaatacagcattataaatttcaccgcgataacgactaactgatcattatggagaaaaattatacagcaaccgggaaaagcaatgcctcttctttgtgtaagatgttcttattgcctggattattctgggctttattgttgctgctgtttcccttttgtgcccatgcacaacatcaaagtataaccggcagggttactgactctctcggtcatggaatagctgatgttacaatcgccgctaagggaacaaccgtgattgcaaaaacagatgtatcgggtaattttagcattcaggctgccaaaggagtgcccctgagagcatcacacgtaagttatgtcagcagagaggtgataccggatggaaagcctttgattattatactgcaacaagctaccaatgacctgaacaatgtggtggtgattggttacggtactatgaagaaaaaagatcttaccggggcaataacttctatccgcccaaataagattgcagacgagaatcctaaaacagttcaggatatcatacgcggaacacctggtgtgagtgtaggtttcgatgcctctgcaaaaggaggaggtaccatacgaatccgcgggcagcgctccgtttatacggatggcggacataatgatcctttgctgatactggatggtatgattttttatggagaactgtctgaaattaatcccgatgatattgatcagattgatatccttaaagatgcatcagctgctgctatttatggagcgaaatcagctaacggggtgcttatcatcactacaaaaaaagggaaaaaggggaagccgactgttaatctgacaaccaatttcgggctttctgatatggccgcaaacaggaaggtttttggccccgacggttatatgaaatacaggcaggactggtacatggctggtacctacggcatcaattcagcaacaggagcctatgaaccttatatatcagaaacggcaacagcgggtaaactgggatactatgaaatgcctaccgatgaaacgctgaagaaatacggtatcactatcgacgaatggagaacctattcaacaaacacaggtaacgcatctgataacgaaatccgggctaaacggttaggtcttcaatatacaacattggataactatctgaaaggtaaaaccttcgattggtatgaccatagtttccgtaccggttttaaccaggattataatctcagcgtatcaggcgccagtgataaaataaattattatttgtctgcaggttatttgtctaaccagggagtggttgtgggtgataactacagggcagtacgctccaacttaaaagtggacggaaaggtcaccgattggctggatattagtgccaatgttaattttcaggaccggtccgacggaaatattgcggttaactggggatcacagattattaataacagcccttttgcatcttataaagatgaggatggaaacctggaagtacatcctatgggcgatgaaatgactgccagtaaaggatataattttgatttcaataaacagtatatgaaattggaaagaggctatactgttctgaataccattctttctgccaaagtaaaactgccctttaatatcaagtactcttttaatgtttctcccaggtatcagtggtattataaccgctattttgaatcctcggagcatcctgactggctgccaattaatcatggtgttgaccggaactggggaaagcgtttcgactggtctttgaataatacgatcagctgggaagaaacttttgcccaaaaacataaggtaaatataaccctggttcaggaagcagaagaacggcggtattggagcgatgctattaatgcacgtaatattttaccaagtgatgccttaggattccacgaaacttctaccggcgatccgcttaacagcagttttaatacggacgattctcatgaaaccgctgatggtatgcttgcgcgcgtgttttattcgtatgatgaccgttatatgctgacagcctctgtgcgccgcgatggctattccgctttcgggacttcgaatccaagggctacttttttttcggcagctttggcctggacatttagtaatgaaagattctttcaatggagtccattgagcaatggtaaattgcgcttgtcctatggacaaaatggaaacagatcgcttgctaatccctatatagcattggcaaatcttgcaaatggtgcaaccactcagggatacgtagatgccagcggtaattatatccagtattactatttaagaattgaccgtatggcaaatcccaatttgcaatgggaaaaaactacagcatataatatcggactggatatcgctttcttaaataaccggatctccggtacgctcgattattattacatgcccaccactaacatgatcatgagccaatcgttgcctgatttttcaggatttacgagtattaccaccaacttaggggaagtacaaaacaaaggtttcgaaatttcagtcaacacacaaaatataagaacacccaactttacctggaataccacagtggggttttcgaaatataaaaacacgattaagcatctttattaccggtacgaggatgtgttagatgccaatggaaatgtagtgacttccaaagaatctgatgatatatccaacggatggtttatcgggcaaccggccagtgccatctggaactaccgcgtaacgggaatatggcaggtggacgaggttgcagaagctgctaaatacggccaacgtcccggggatcctaaagtagccaataattacacggcagatgatattaaaaatggtgatggaactacaacggcggtttataataataaggataaggaattcctgggccagactacaccacctactatgtggtcgttgcgaaatgattttacctataaaaacttcaacttctcattcaatatctattcttattggggcagtaaaagcttaagtacttcttacctgaaccaggataatagtgtttcgttggttacatacaatgccaatacctatcaaaaacaatattggacgcttgataatccgagtgatttttttgggcggttggatgcgagaggtccttccggagttgctgcccccagcagagtattcgatcgttcttttatcaggcttgataatgtaacaattggttatacaatgccccgcaaacttatttcacgggcggcgattgaaaacctgaagctatatgcaaccgttcgcaatgtagctgtctggagaaaagataaaaactgggattactgggatatagaaactggtgacattgcaccgagaatttacacgcttggattaaatgtgacattctaaaccttttacgaagggaaaataaaaaaaacaaaaatgaaaaataactttataagaaaagttttcttcctggtggtggcatcaacaatgattactgcctgtagtaagaaatatcttaagccggatcctttatctttttatgagcctgaaactactttctctaccaagtcgggactggatgctgccatagcgatgtgtgacaagcatttgcggagctattggagctacattacgaccagggatatttcggtacctattaacaccgagtatatgttgtcagacatggcggtagccggtaaaacagatgatggaagcatctttgcggatgtagctacacgtcttactccaactgacggcatgtacactaatgatgtgaacatgttgagctatttctggggggaaacttataatggtatcaagtatgccaatacaatcacctcgtttattgataaagttcccggcctggatgaagctacaaaacgtgaatatattggcagggcttattttcacaggtcctttcgttatctcgccctgtgctttcagtttaacaatgttccactgataacccaaatcccttcttctccaaagcaaaactataaaagcaccagtcgtgacgctattttagaaatgattactaaaaatatggaagatgccgtgcaatgggtgcctgatcagtccagtatgtcatatataggcatgattaataaaggcgcctgccgccagttattgatcaaatgctatctggctaccggtcagtgggacaaggcaattgcacaagctgattctttaattaataattcgggttattccttaatgacaaatacatttggtacgttcgaaagcccgctggaaggcacctggcatattacgcggaacgtgatatgggacctgcaccgccctgtgaacaaatgtatcatgacaaataaggaagccattcttgctatgcccaaccgtgataatacagatgccgcaataaaaatgcgcaccatgcggaattggggcccgatgtggaatatctctacattagtatcgcctgcaggaaaatttatgcaatgctacgcttcatcaagcagttcctaccgggccaacctcgattataactcggctgttggtcgtggtattgcaatgattagccctacctattttgcacaacacgatctttggaatgtaaacggaattaatgatgccggggatctgcgacataacagcagcgtgggcaactgggccagaatggattccctgaaatacaatgatccttcagacgcattgtatttcggtaaaaatttgcggctttacaatggaaacaaacttttatgtaccgatacggtgcgtaactggttcgattggccgcattataaagtttttgtaaatgatccggatcatattggcaatgctgcaagtaataacaataagggcggcgcggccgactggtattgctatcgtcttgcggaaacctatctgctccgtgccgaggcccaattttataaagggaatataggcgcagctgtagcagacgtaaatattgtaagacaaagggcaaaatgccagcagctatacactactattactattggtgatatcgcgaatgaacgtgcccgtgaattatggatggaagaatggcggcacatggaactaagccgtatgtcatatagcctggccttaagtggtaaagcagatgaatggggaaatacttataacgtgaatacgctttcagaaaacagttattggtatcagcgcatacagcattatagcaattattacaacaagaacaaagtaactgtaaagggcaggtcctataccatagcaccacataatatctattggcccattcctcaatcggcgatcgatgcaaatttgtatgggaaactacgccaaaaccccggttataacggttatggtcagagcgtggagatgtggacgaaatgggaagatgccgttaatgatgaaaataagaattaagaagagaggtacagccatggtcatctcccagggtaatggaaatacttggacgccttcatttgaaagcgtccaaggcttacttactctcttggcaatgaatcaaagtattcgagtggcgacattttgaaatacttctgaaagttgcgactgaaaagactttgcgagctgtaacctatcatctttgaaatttcgtaaaatgaaaactcatttttagcaattaaatcggcggcttttttaagacgcgtgatgtcgataagttcttttggagatagcgaggataaagatttgatcttgcggtataaggtggtgcggctcatgaacatgtgtgcggcaagcatgtcaatatcaatattggggtcttcaatatttgttttgatatattcatccagtttctttagaaaggcttcatccgtttttgaatgcgccattaccctcacatcctcaaaaggcgaactggcaaaatgatcttttattttacgacggtttttaagcaggttagcaatctgtacctgcagcaattctgatgagaatggcttctgtatataagcgtctgcgcctacctccagtccttcgatgtgagccttatacgtatttttagacgttaataaaatgatggggatatggcagtattcaacattggatttaatgagcctgcacaactcaaatccgtcaattccaggcatcataatgtctgatatgatgaggtgaataatttctttgtccaaaatggtttgtgcaatttctccattggcggcaagatgtaactggtaagcatctctcaaaaccatagataagaattccaggatatcttcattatcgtcaataataagaatattttcggtcatactattttatctttttccaactgcttaattgaaattcaaatttttgatgtatgggcagttgcagttcaaatataattaaatcagtttcgccggaaatcaatcgcagcgatccgttgtgcaactctgtgagcgattttgcaagcgacagcccgataccggtgcccggcttattatttccacgtactcttacaaagggttcaaatatctggtctttaaactcttctggtatgcctttgccatcgttgtgaaagctaatcttaaaatattcgtcggaatcgcttaccgtgtttatattaacggtggccctggtggctgcatacttaatagcatttgatattatgttggtgcatattttaatgagcgcctctctgtctacaaaagccgtaaggtgtttttccggtaatgcgatatccagttcaatattgttggcggcagcctgtgttttaaggcccgctaccagatcggttatcagcccggcaatatctgtttttacaaaattcaggctgaactggtccgcctccgtttttctaaagtcgagtagttgactggccagctctatcaggcgccgggtatttttttcagctatggcgagcgttttcttaacatctgggtctttatcaaattttttgctcaaccattctatggggcccgctatcagtgtaagcggcgtttgtatttcatgggtaatattggtgaaaaattctattttggcctggtaaatttctttttccttttcatgttcaaacaactgtagctttcgcaaatttttacgctccaggtattgacgatataggcggtccgtgatgaatattataacgcctaaaagcagcaggtatacaatatatgcgaagttgcttttccagaaaggtggaaggattttgatgatcagccgccgttccttgcccgtccagcttccggtgttgctttcagcctggacaataaattcataagtgccatgggtaagatcggtaaagtacgctttgcggttagtattgagataggtccagggctggtcaatgcctttcataagatatttataccgtgttgcttcgggcgaggaaaagttcaacgccgcaaattcaatactaaaattgttctgatcatatttcaatataacggtgtctgtgtataaaacagactgggagagggggctgttatgcccgccaggtattgcttctttgttattaatttggaaaccgatgatataggtaggcgggcttggctctctttggttaaataaaaccgggtcaaaaccaatcatacccttaacagagccaaagtacattttaccatcggtatgtttatacgctgagttgtagttgaattggtccgttatcagcccgttggcttgtgtgtacacttttacctgttctgtatgcaggtcaaaacaaataagacctttggatgagctgatccacaaatgttttgaattgtcttccaggatactgtataatacattgcctggcagcccgtttgcggttgtatatcttttgatggttttccggtcggagcttagttttataagcccactgccggttgtggcaaaccataaagcatggttgctgtcttcaaaaatattgtacacagggaattcgttgatggtctttcccttagtggtatcaccaaaatgtaaattcccgcggcggccggttttaggattataataaaatgcgccttcctttacactgcctgtccagatatttccttctgagtcttcaaatatatcataaacataagtgttgtatggtatctggctgatgcgcttaaatgttttgtgttgtgggtcatactcaaatagtcctgcattacggtatgcagtacccaccagtagtttattgttttttgtgcggtagattgaaattacaaaatcacttaccgggccgttcctgtcaccaataagtttaaaccggtctgtaaccaaacctttacgcatatccattatttccatgccctgtaaaaaagggccgataaataactcgttcccccaggatagcaggccatgtatattggagtaagagatgcttccttttttgcctgtggctgtatagtttgtaaatatgcccgtttttaaattcaatttgttaatacctgcatcttcggtgcccacccataagtggccgctgctgtcagcacatatttctcttaccgcatttcctgaaatagcattagcacccggtagcggataatatttttcaaatcgtgcattgaccttcgaatagtaatttaacccgccaaaaaaagtaccggcccacataccaccctggttgtccctgcatactgcataaacagcattgtctgccagggcataggggtcgcctggccgttttctcaggcttatgctcttgttggtggctaagtcgtaaatgtaaattcccgattcagtagctatccagtattgcccgtcgttacccgttgcaatatcgcggacaaatatgtctttgtttttatcggtatccagtgataaagatttaacgatgcctgtttgggtatgatagctttttaatccctgtttaaagcaacctatcaacagttcgttattattgatagggtatattttgctgatagaccgggcatttgcaggggcacttttatcaacgatccttatctttatgccaggctttgttttcgggttgtaaatatgaatattaccgtcattatctcccatccataaattcatatttgaatccagcgcaatacaggatgcttttgtttttaaatcctccacccggttctctgcctgtatgtatttgtatagagaaaactggatgagaaaccaaagattgttatccttgtctattacaagattattggtatattctttcgggacggtttccagttcagtgagtacttctttgtacgggttatatttaaaaatgcctttgccggtggctatccagatcatcctgtttttatcctcagcgatagaattgataacatcatttcccaggctgccgaatttatcgttattgtttttgtaggctttaaaagaatacccgtcaaaacggttcaaaccaccacgggtccccacccatatcaaccctttactatcctgtattacagcggtcactgcattgtgcaccagcccgtcatccacctggtagtgcttaaaataatattgcccataacatggagaaatggtgactggtaagaataaattcagcaaaacaatataaccgaggaatttcataatactgaattcaaatataaataatgatatcaaaatactatgggttttaaaataaaattgtatcacttgattgcggtgcatgctatatttggtacgattcgtcaaaacattgaacaatccggggggagtatggcaagccctggaatgatagttagaaaataggtataatacctaattttgattaagtttagttatagaataaaaatggttttcccgtcattctaaatcatctcttatgaaaatcaatgtaaatggcacagattataccctgaacgtgccggctaacaccagccttcttgatgccttaagagtaaatttaaatctcaccggtagtaaatacggctgcggagaaggcgcctgtggtgcatgcaaagtgctgatagacggtcatgctacaccttcgtgtattacccccgtagcaagcgtggaaaataaaattgttatcaccatagaaggattggaaaaagacggtcagctgcatcctatacagcaggcgttcctggatgaagacgccttccaatgcgcctattgcagctccggcatgatcatttcagcggttgccttaaaagcaagaaatccaacacccaccaggcaggagatcatagaagcaatgcagggaaatatttgtcgctgctgtgtttatccacgtattataaatgccatcagcaaggcttaacgttcaaaacccaaggttatgaaaaattcaggcacaaggcaaactcctgtggaaggaatcaacagacggaattttctgaaactgctgggcggcggtattgcggttgcccttacctattctgatctgaacgcattatcgaagcatacagctttcgttcctcccggtgatgacgctatcgccgcctgggtgcacatcctggaaaacggaacagtaaccgtttacaccggcaaagtggaagtaggacaaaacattcgtacttccttatcgcaggtggtggcggaagagttgtctgttcccgtgaccagcattgaaatgatcatgggcgatacccttcttaccccttacgaccggggtacatatggcagtctcactacacctactatgggaccgaagttgcggaaagcggccgcctcgttaaaagaggtgctcacggatatggctgcgaaacaatggaacgtagcccaacaaacggtgactgttaaaaacggccaggttagccacgccgcatccggtaaaaccgcgagcttcggcgatctcaccaaagggaagaaaatgctcttagccgtaaacgaccaggtgcagctcactcctgctgaaaaatggaccgtagccggtacacccgtggcaaaggttaatgcgaaaagcttcgtttcaggaaagcatcaatatgtatcagatatggtgatgccaggcatggtgtatgggaaaatgctccgtgcgccgtcttatggcgcatccctggttgctgctgatgtagaaaaggcaaagatctctccaggtgtaaatgttgttagagaagataacttcattggcgtaactgcccctgatccccagacagccactaatgctttggcccgaatagaggcccgctggaaaactaccccgcagccttccagggcggaaattttcacttatcttaaaacgcacgcacaagacaaggaaaaaaaagccggggaggccgttgataaagcctttggggcagccccggtgcaggtacaacaacattttgaggtgcaatatattgcccatgtgccattggagccgagggcggcgctggcggtgtgggaaaatgggaagctgaccgtatggaccggcacccaacggccttttggtgtgcaggaggaactggcggaagtattttccattccgaaagataatatccgtgtaatgatgccggataccggctccgcctatggcggaaaacacagcggggaagccgcggtggaagcggcgcgcctttccagggccgtaggtagaccggtaaaagtagtgtggacccgtgaagaagaattcaaatgggcttatttcagaccgggcggacttatagaagtagccgccgcagccagcaacgaaggacttttggcgtcctgggagtttcataattataactccggcggtgctggtattgaaatcccttatgaagtgccacacaagcacatccaataccatccatctgatacaccgttgaaacaaggctcttacaggggccttgccgctacggccaacgtcttttccatagaaagcgtaatggacgacctggcccggcaattaaaacaggatccattccggttccggcttaataatttaaaagaggaacgattaaaacaagtgttacaggcagcagcatccaaatttggctggacacggcaaaaggaagctggtcgtggttacggtatggcgtgtggatttgtaaaaaacgcctatgtaggaacctgcgcggaagtagcctataataaatccaacgggcagttgcaattgctccggctcgtagtggcttttgactgcggcgccattgtgaatcccatgcacctggaaaatcaggtgatgggttgcgtgttgcagggacttggtggcgctttatttgaagccgtggactttaaagatggccgcattttaaacccatcgctttccagctaccgggtgcccaggtttggcgatattccggaactggacattgtgcttgttgacagaaaggacatgccgtctgcaggagcaggtgaagcaccgattgttggtgttgcgcctgccatccgtaacgcaattgcggatgttaccggcgtaaagctgaatacgctgccattgctgccacatggaatgacattaaaaacctgaaaataatgcagaaaccattaagaaaacctaactttagatagtaaagggccccgcacatctcattcagaaaaaaaccaacttagggttgtcagtttggaataaaaatcgctgatcactttgagcgaaaaatccacgtataaaattgttcaccaaaaatcaaccaccatgacacagaaaattttgattacaaagtttaattacaatttgtctcatgccgaattgagggaccttcttcttaccgttgcaggagattttgctgcagtacccggctgcttatggaaaatctggcttatagatgaagggaaaaatgaaggcggggcagtatatctgttcaataacaacgacgcactggaagcatttaaagcaagtcctttggtgcaatcggtcatgtcacatccagctttaagtaatttcgattttcgaattacggacattgtagcgcaacccagtgtggttacaagagcaccactgacggcggcagttactatataaggcctgaagcaagggggatccagtgtttgggaaggccacatactaaaataccccatttgttatccaataaataattttaagtttacgggtgataaatcgcgtcttccggtatatagtatggaccaagttcaccatcgtatgcaaacaatatcagaccacacattgctcaatatgctcagaagtgaggacaatgcttcttttgaggtattgtatcaatactattttccaactattgccgcatatattattaataactacgggcaaaataaggatgcggaagatattttccaggaagcaatgattgtattgcttcaaaaagtaaggcaacctaatttcttacttacggcttccctgaaaacttatctttttgctatttccaggaacctctggctgaaacatctccgggataataggttattgcccgtagaggatgtatccctgtatccgtgcgcgacagcggactttccaacggaattacaccaggagaaaaccgaagatgaaaaagtacaaacctggatatccaggatcacagggcattgccagcgtatactaaaagccatctttttttaccgggagcctatggaagttttaatgaaaagaatgggctggaaaaacaggcatacagcagccaatcagcaatataaatgcattcaacaggttaggaaaatgaaggcaaaagaagaaagcatatagtttttgggtgataaatcttatgaacgggtattaataggaaatcacctttaaacagtttaattatgtctgtaaaaacaaaaatcattctttgtattgtctctttagtattaactggtatttgcctttatcatttctttggttgattaaaaaacagttagaatgaaaacagctgtcaatattcggggaataagggaatatgaaggagatggtaaaagctgccctgttgttcccgttcatctgccctggtataagaaagtggccctaacatttttccgcttcggggtatgtcccatttgtattactatgagtatatcgtataatatcggcaggttttttaagggaataaaaaagtgaaatgttgccgggtggcccatctgcaaacaatttttgtttatgaaggtgcaattgattattttttgtataaatagatgcatcccatatgtcatcaggcttcctcaaaatacctgtccctgccgcttcccgtgcagctgcaaatcaaacggttccccgtagtggaattgcctatccggccgttataacgccacctgtattacaacaacaggggatcatgcagctcaaaattgacaagttattggacaacggaagtgataagcaggcgattgaacgttatatgaaaggcgccgtgaattcacggggccagacttttgaacaggcggtggaagaagtgatggtattgttcccggcgttgagtgataagttggcaatctccaaaacctggcttttactaaaggaatccttgtctggtgaaaaaattgatgtcataacagactgcattatccggttgtctaaagacgtgaatacgatcttcatggaacatacgccctatcccaacctgagatctcatgacctcaggccggacaagccttttaccattccgcaaagcgagaaaagccaggagcgctcggagacactgtataaagagattgataaggaagcgaaacgcttgtttgaactggtgaaaaaggaagataatggggcaaaaacgaaattgggaaacttgctgcgttatgataaagagcacgacacctacaaaggatatatgctgggtgtacttattatggatgggcaggtgtttgctacctgctccggtggtcagtcggccggttttgagctcatcgccaagtcactggggatgcagtacgtgagctccgtaatgaatgtggaggaagcaagaggaattatcgtcaaagaaatagggccgcatagttttggaaccggagaggagaaaaacattgtaaaagaacatacggggagcgaggaagtgaaaaccgggcttgccggtacctgtgctgccccgaagctgatctggtctatcattgatggaggccatgtgaaattgcatcccaccactatgcagcatgcatccatgacggaaagatgggtgtctccactcaatgccgacagtacggttcctataattgatgcacatggcaagattataaaatatggcagtggtgatattgtaccttcctgtaaggcttgccagcatttaatgcatggactggaagaacgtctgcagcggcggctggcccacagtaaagaaatgaaatcactctgggaaaaggaaaattctgcagaaaatatagaaaggaaaagagtggaaaaagaacaaaaacaggcgctggacagggaatatgaaagccaaaccctgactggaaactcaggtgaagtacaggcattaaacctcgccttagagaatttattaaataccattataaaaggggacgattccattttgaaagacgaactcagtttcctgagaagcagcactgacagattagaagagttacgttttgacctgcgggcttttgcaaagatcccactgggcgatagcagggcagctgtattggataccctggaacggctgaaagaaggacaacgcgttattgctaccatggtggacggtatcaatcaattttgggcaacgcaggaaaagccggcggcagcatcatccggaaaaggtggcgcaacggagaaaaggtccggaaaaaataagaggtagccacaccagcttttgttttaaaaaaaaggggcatctcaaatacttttgagatgccccgtattactgttttacctttcttctcttaattatcccaccagacctttgtactctggatagctgtttgttgtggttgtgcattcgttaatatctcgttttgcggatataacaaccggcgggggatatctatcaatgctccatctactttctgcaattttggaaaacccgttcttctccagtcgttatacgtttcaaagttgaagatattagctactgctttttcctccatgatcagctgtagcgcatttccggcggttagtttgcggcggtttacataagcagtggccgcagcgctggcagtatcaatcccgagtttggacagatgggaattgatcgcatttacatataccggctgcgcagcggcataaccgctggtgatcagcagggcttctgcctgtatgaatagtgcttcagaataattgaagatgtaattggacgatgctttggcgccataaaatgcagcggggtaagagtacttagccaggtctcctgtgggcgtaccgatttttctgccggtaaacagtcctgttgccgtggcgggagcaatcatctttggcagccgcggatcattccggttgcgtaaggtatcgatcagtgtggcattcatcacgtaggtagttaccggtgtaaaggtgaggtaccagatgttttccgatcctgccgcgccggagtaggtgaacttaagatcatcgttgttggatgtcatgccttcttttaaagcagctattgcgctttcggcctgcaccttggcggtgtatccgggtgctttggtgagatgtatataatacctcgctttcagcgaccatgcgagcttgcgccaggcgttcatattgccgttgtagaagtagtcgtcacctgttgggctctttggactgctgtttttgtcgatgttggctatggcatcggtgagcaatgactggatgcttttgtaaatatcttcctgtttatcgtaaggtactgtgaaaacgccgctgacaaacgctttagaataaggaatatctccccagaaatcggtggcagtgccgagggtgtaagccgtaagtattttggcaatggccgcatagttccagttgttattcgcttccgcctttttattcagtgtgatcaggttgttgagtgaggtgacgtagaagttggaccagtcgccatccatatcaatattaaacagctggtaactgcccacataaggattcagctggttggcggctatgttctgcacatagttctgtataatgattcccgcattgccgccatggatattgtcagaaatgttcagttccgccggcgccaggatcagtgattcctgcacatctatcggattattgggatcggtgtttatatccaggaattttttacatccctgtaaacaaagaccggtgagcagcagtatataaagagactttttcatgttgataaattttagtggtgccggcatactaaaaactaaatttcaatgagaagttgattgagcgtgatgttggcgtggaaaacgcataaataccctgtgagctgttgcctgtgccataggaacttacttccggatcagcaccggtaaaatgcgggctgtagatccagagattcctgccggctactgccagggaagcggttttgaaaggtgttttagccacaaaggaagcaggcaggaggtaggaaagacttacattccgcaacttgatataagtaccatcctggatggtggattcgtattgcctggtctggtagtaggtttgcgcatctactgccacggtgttgggctttccgtctacttcgctgattcctttcaccaccatttggccgcgggtggcagttacctttgcagtgccgtagtagaaaccggctgactcaacatcattttgcacatcgccgccttttttcatatcgaagaaaaaggagaggctgagctgtttataacggaaggtattatccatgccggccagccaatccgggttaatatcgcccacaatgccttgttgcggatctactaccggtagtccaccggcgtcgatgagtagttccccgttgtcggcccgtttatagcggttgccaaagaagatgttatagggttctcctttgatcaaacgtcccagctggtcaacgcccggcgccagggaaagtacctcgtttttgatcttcgaaaaattcagggtaacattccagctgaaatcttttgtctttacaggagtagcgcccaacagcagctctattcctttgttggatatttcggcagagttaatagtagtgctgttgaaaccggttgaaggggggatttgtgaccctggaatgagcccgcttttggagcgacggctaaaataagatccttcaaaggtgatcctgtctttcaggaaacgcatttcaagccccgcttcatattcattgagccgttcattgatgagcgtggggttacccaatgcagttgtcagtaaaaagccttgctgtccctggaacgggaactggaaaaaaccggcgtttgtattcctgcctgcctgcacataaggggtagataacgcatacggacctacgccgtcgttacccaccgtagcatagctcaggcgtacctttccgaagttaatgacattggaggctttaggtccgaggaattcggaaaagataaagctggcagcggccgatccgtaagggtagaaatttttatcgggattgagcacggagctgccgtcgtacctgccggttaaagacaggttcaggaagcggttgtactcaatattagcctgggagtagaagcctacttttctgagctgggtgtaactttcagtacctgtgatagtggagccggacgataagttattaaagtcgttaatattgagcccggtgccgttaatattcatatactggctgtaagtagtatagatattattaccgactaacagatttacgttgaatttgccaaatgttttcgtggcgctgatgatcaggtcattattgaattgccggaagttgatgttctggttcctgatttgtcctgtgaggccaatctgcggacttggatgttctatatacttatcagactccgtgtagatgtccgcgccaagtctttctgtaatagtaagccagctggtaggagtgatgttggcggtaaataccgggagaaacctgttgactttagaatcattgctgatgttatcgagcgtccacagcggcatattcctggagtagcggtagccgcgctggctaccgtcgggcaggagcacagggtatggattccacgataccggttgtagcagcagcacaaataaaggcccgttgctggcgccttccggcagcctttcctggtcggagttgttgtatcccatctggaaagtagtgctcacatatttgcctattttggaattgtactttgcaaagaaggagtgccgcttaaaatcatttcccggcattacacctttctggttgaaataggaatagctgagaaaatagttggaattattggtactgccggaggcagaaatagtattgttggtagtaatacccgtgcggaaaaaatcgtacgggtcgtaggtaggtgcgggctggccgtttactttgagggtatccatgaggggaccccaggaaaggcttgtttttttgtcggcgtcctcaccgttataaaagataccggtggtaccctgtccatatatattttgccgttccggcaggagtggatgctcaaaagaagcatctgacgaaaagttgaataccggtttcttatccacaccgccatttttagtggtaatgagtactacaccccgggcgccggaagacccatacaacgccgtagcggcagcgcctttcaggatgttcacattttcaatgatagcgggatcaatatctgcgatacggtttacgccggagcccgcggctccgccgctgatattgccggtttccgtgttatcaacgggcacgccgtcgattacaaacagcgcctggttttccccggtgggagaagagttacccctgatcacaatgcgggaggaggcgcctgcattaccggaagaactggtaatctgtatgcccggcaccttgccggccaaagtattcaccaggttaggttccttggtttttaatagttcttctccgttcagctgctgggagctgaaggtaaggttgcgtttttcccgtttcactcccaatgccgttactaccacggcattcagcgccgaggtgttgctggctaaagtaatagcaaacgttgttttgctacccaccggtacttccgcactaagaaatccaacactggaaatgaccagcgaatttttttcgtccacggttaatttaaatgtaccgtcggcgctgcaggtggtgacggccttcccgcctttctccctgacggtggcgcctataacaggcatgccggacgaatcggcgacagtgcccgtaatcgctttcttctgcgcagatgcagacaaggagaagaaagcgagaaaacataccatatatagcggtacgaagcatcctgatactgctgattttgctgatagtgccatttgaataaacgtttggttgacaagttgagggctgcatagaatagttagcggaataaaagtaggtgtaagccgtaaacatggattcagaataattaaccgattgtaaacgtattttatcccaaaagccggtagagtattaatatgcgtctatgttaaatgtcatatcgacaataatatgaataagagagggtgtgtgggtttttataagcgttgttttgacactaattggggagatgtgccagccttggtatttaaatatatggtcagtttgcagttggttgtcttgaattagaataatatctgccgaccgggaattggatgattcaatatcagatgatgcaataattacccgatgtaaggaatggagtttatcctcactagccattactactattttcaaatatggacgaccaataagcataccaccgcagtgcaggaaattttttctaatggtgggagaggatccttaatcctaagtttcccttttaaaatactataaccttttactccgcagttgtaggatcaataacagtagccacctcactgacagcattggccggaaatcctccctgcttcgcgtgctcacgaaccatttcttcattaggggcaatgtaaacgcaataaattttatcagcagtcacataactatggatccattgaatttgcggacccatattgcttaatacgccacaggaagcttgtgaaatagctttcaactgttctcctgagagtttacctgcaccaggaatttcgcgttcgataacatacttaggcataatggtagattttagttttatcctatgaagttaaatcttgcttcttgccggggttttgacaggtagtggagtagtacgaatgtatatcctaaatataagcatttattctaagaaatcgttcaggtaaaaccgaaaaaagggcgcaggtacaacacctgcgccctttttatcaaaacagctcctttaacgtttatacacacccacttccgccagcgcagagaaatttccgttcttataatccgaccgcacaatcaccctgaaatacctgaaacttaccgtttccgtcaggtctatgtattgcttatccgctgcggataacaaggtaaacgcacccagcggttgccaggtggtattatcgtcgctcacttcaatttcaatcagtttcaatggtccgtccagcggggtacgttgtatgaaggtaaagccgtaggccaggttgatggtacccatatctactgtaatggtacgcggataagtaagacctgcaactttcgacatgtgccatacggtagatgctttgttatcgatcgcattggcgggcccgcggccggagggttcgtcatagtcagatgcggtggccgtccaccctgttttggcatattccaccggcggaccctttaccgcaatcgcctcgtaggccgttttaaacaagtcgatggcactggaatccggcaggtataccgtagtgtatgcgagatcggtattatcactgaaaagaaagttggacaaggtggtggtattggaatctaccggtacgcggatgtgctgcaccgtaccaccagcatctgtataccttatttctgtacctgttacgtgggtatctgcgcttccccaggtaatggccactttgccgtcggagtagagcgcgcttttaacaggtcggggtaacaacgagctgatataacgctcaccatacacctggccggtagtacttacttttatggacttgtttccctcatcatcaaaagtgtagatatcgaaagagtaagcgccttcggctataggggagaggatcacgttgatagtgtctacgtcatattgtcttttcaacaccatatccagggaatcacttttgttattccagtaaattttggctttagtgaccctgggatcgctgaccagccacgatagccggatccggttatcacccggaaaaacctttacggaatccactgagccggcgtaagggatttctccgtttttaatgaactgtttgtaggtgtcgtccattttgctgcaggcagcaaacaacaggagcagcgctaataaacaggcgttatatattttcatgaccagttatttgtgttagatgataacattttacttcacattgccccagaaggtaagttccgcgatgtagatatgatccagcgcgccccatactttgacggttttaaagcgcaggtatcttacaggtggtacatcgggcggaaaatcaaaatcctccccgtctacagtggcaaattgtttgtcttccgtggtgatggtgccatcgggcgtaccggagggttttacggattcaaaaccggatagcaatacccagttgtcccagctgccatcgctggatggattattactgccccagatctcatatattttgggatcgccgccggtataagacccgtcggcggtgctgccgtcacggtgatgcagcttgaagcggctcagcgtagcagtaacgcccatgtcgatcgtaaaccactgcggcaggccgctgcctggtttggtatggaagatggaggtaccggcgttgcccagcttgtcatcccagaggtaggggattttactgctgatatgccctgcataggtatctgtcggaagatctacttctttgaattttgttttttccagtttttgttcaaataaaggcgatagttcagcatacagcgtgtcggagtgattgttccatcggtcacgcacaaaggcggcaaattttcttttggtagtattaaagcccctggcggcaaacgtgccggtctttcttttggtataaaatgtttccgccggtaccaggtcgttcgtggaatcggccgccagtacggtaatcaccacatctgcttctgaattatttacgaagttgacccttacgccgccgaaggtagcagcaagcgtcagttgctggaatacttgttttaccggtggcgtaagtggctttacggagatggtgaccggctccgatatattttcgccacgactcacagcataaagttttaccgggtattccagcgtgtcgggaaatccgtctatggttagcatatgctggtagtaagatgcttttacttcccgctctatacctggccggatggagtacacggcttttatatacaggaggtctttgtctttcgggcgactataactgatattggcgccgccggcaatactttcggcgcgtacgttggtaaccggccccggcgcctggtctttgttaagcggctgaacgccttcctctttacagcagtataagccagcacaaagcagaacaggtatgatatattttttcatagttaatttctttttttgtaaacagattaccagccgggattttgattgatctttttattactcagcaactctgattcgggtatcggccataaataatccctggtggtgaaaacctggttatagatcactttttcacgataataagcggtggcgtcttcctgcgccagatcccacccggtaatgggtttgttaagttcgtccacagcttttttccatctccggagatcccaatagcgttgtccttcaaaggctaattcaatcagccgttcccgttggataatatcacgcatgccctcttttgtggtgaacttggcagggttacgcgcatagttggtccaggcgctttccacggatgttaagccagcccgctcgcggataagattgatataccggtatacctctgcgctggggccattggcttcattttcggcttctgcatataacaggtacaggttcgccagtcgcaaaataggccacggatagttttgaatagtgtaggtggtaccgtcgccgattacgttgttgaagttcaccagctttttgggccagtaaccggtaacggagtacgacgactggttctgcgcactggctggttgtccttttttgctggatacaaaaaagagattggcattgtcgttaaataaaccctgcccgtaccagatgccgccatcaaatcccaggtcggcataaaagcggggttcccggtcgaaatggagggctgcggtctgatatccttcctgcaggtcgtaccggtatgcatgcgtgccggtacgcagtttaaaacggccgttatagtcccatgtcttatcttctgtgatcggtacgccatgattggtgtaaaatagctgcgctattttcagggtaggggcgatgttgcccaccgtagcgctgttggccgttttagaaggatcgagtccgcgcggagtggcgctggcctgtatgctgccggccaaactattggtatggccccatataatttcgggattccatttctcacatacagcattacggatactgagttctatccgcgtggtgtcggagattttatattgaaagaactgcggattgaaggtatatagtttgtatccctgcgattcgcaaagcgtgagcgcagctttgcaggcagcggcggcgcgtacccatttctgcggatcattggtttgggcaaacagcaacctgccatcgggacctttaaaaccggcgtggtcggagttgccgttaaacagcgggctggctgccagtaccagcacctgtgctttcaccgttaatgcaatggctttggtaacacggcccagctctgatacttcattctctattttgtccggcagttgtgcagcagcttcgtccagctgcttggcaatgtagttcacacaggaatctaccggttctctggctggatatacttcctcctcgccggcgcttaccggcacattgtttttgatgagtggaacagggccatacatctggaacagccaaaaatgataataggctttcaggaattttgcttcccctgcccagcgttctttttcggtgctctccatatcgggcaccttaccaatgttttccaggaaaatattgcattgccggattccttcaaacaaatccttacctccggcagtaccctgccagtaattcatatagcagttcactacattctggttgccacgggcaatctgccaggcattggaggtattggtaacgggcagccagtactcatctccggcggcattagacggattgccgtcaaagttgcccagcgccggcatataggagtagcaggtaaaaagaaatctttcggcagtagaacggagccggaaggcatagtcgatggtggccacgttatccggtactatgtccaggtattttttacagctgctgaaaagctgtggtaacgtaacaatgaatatcaggcagatgatctttttcataacatgcagttaaaagaataagaaagcggatgtttagaatgtggcgagtgcgccaacgttgaatacccgttgtaccgggtaacccagaccgttaccggccatttccacatcccatagtttaaacttgctccaggtaagcaggttggtaccgttggtgtatacacgtaatgttctcatatgcgcccattgccgcacggtataacctatttccacctgcttcagccggatgaaagcgccattccgcataaaccacgtactttgctgggagttgttatcgttaccaatagcggtagtgctgagccgcggccataaagcatacagatcgcggtgctcttctgaccagtgactgtcggcgtatgcctgcagcagctggttctgtggtttacctgacaatgtttcattatcataataataggtcatgaaaggggcagtggcgcgtgcattgatccaaaacgattcccggcccagtccctggaaaaatgcagagaggtcgaatcgtttatagcctacagaaaaaccgaatccataagtgatttcgggcgtggtgggaaagcccaatggcacctggtcgagttgggtgatttgcccgtcgccgtttacatcatggtatttgatatctccgccgccatattccccaaaattctgacggggcgattttgcggcttccgcatcatctacaaaaagcctttctgcgatgtatccccattgctgggaaatggggtagttcacgtgcagtttccagggcgcgccatcgtacgaaggttcttcatatgtggtgaacttgctggtggcataggtgaagttggcccttgcctggatccagaagtgctggttgaaagaatggttgtaatcggctgagagatcgattccttttccttcggcggcgcccacgttggcgcggggttgggcggaaagtcccatagtggctggtgtggcagttctggtcatgaggatattactgcgttgttcctggtagaagtcggccatgatatccagtttgccaaacaggcccagctccaggcccaggttggcttttttagcagtttcccagctgatgttaggatctgcatatctcgagagtgaaatacctggccggctgtagccattgtcgcggccaaatactgcacttttgccggcgtcgttcatgtttacattggagaggtacataaagcggtcgtttggatcaccgatcgcatcgttaccggacaacccgtaagtagcgcggagccgcaggttggaaatcgcatttttataaggctcaaagaatttctcattggaaatgctccaggctacgcccgcagaagggaaaaatccatagcggtgcgattcatgaaaacgttccgacccgttatagccaaagttcagctccacataatacctgttctggtaagagtaggtgccgcgtcctgccaggcccacgttgcggaagggcagcgacgcctgcagatcagcgccgttgccggtaagattgttacgtaccataaacacaaacaaaccactcagggtatgatccttgtgaaaagtgcggttataattaagtgcggattccatataaaaactggagttcactgttttggcgccgggtacataattcaggtattctgtgcccagttcttcgttctgcagttccagtttaaaggtgttttgtagtttatcataagaacctgcctggtaccagaaggggctgtaggcacgggttacatcaaaataagtattgcgtgtcacatttaccatcgtccggaaattcaaaccttctgtcagcgccgataagttttgttttacttcaaactgcgccgccatcatagagcgggaataatttttatatccctttaccatgtcggcgtatggattcagcagataggcgttggtgccatcatcataattgccgaacataatatgctgaacatactggtggtctgcatcggccggataataggcggggaagtacacgggattggtgcgcattacttttttgtacaggtctgcgcctccgtcgataggaccggtgtagtcgtcgaaggagccgcttaaacgaaccaccatctcggtagatttggtgatgttcacgtttacattggatcggagcgaataatttttcaggtcgatgttgctgttaaaattattccgtttatctacgttcagtatgccattgtctttattgaaagagccggccacataatatcttgctgcagtgccgccaccgcttacattgaggttggcgcgctggttggtggtatagcttttaaaaagtgtgcctctccagtcggtagccggatacatgtaaggatttatgccggcaatggtgttatcaattttctgatctgtgtaaggtagctgcccaagtggatcgcgggtgagcacggcttcattattcagccgcatataagtgatgggatctgcgagtgccacattgcgggtgggggaggccagggaattttcgagccggacggtgatggcggctttcccttcttttccttccttggtcgttaccaggattacgccattggcagcgcggctgccgtagagggaggtggcggtggcatctttcatgatagagaagctggcaatatcatccggttgcagccgggcgaggtctgttacggtgagttctataccatctatcaatatcagcggatcttttttatagccgaaggtagttacgccgcggatgaaaaaatccgcgttatcctggccaggttcaccgctgcgctggtagccaatgacgcccgcaatgcggcctgccagggcggtagtcaggttgctggccggtacctttagttccgctgggttaatagtggttacggcgcctactacatccgtttttttctgtttaccaaaagccactactactgtttctcccagctggctgtaggaaggccgcatgatgatgttgattacttccctgccgtttaccgggatctcctgtgaggtgaagcctatcatggaaaatatcagggacgcgttgtctggcactttcaggatataccgtccgttgacgtcggaggcggtgcccacccctggcttgttctttacagcgatagttacgcctatcatgggaacgccgctgctgtctgttaccagtccccttacttccttgtcggccaccgggagaatggcgtcagcagaggcaggcagccggaataaaagcagcaatatggctactataccaacgtaaaatttgtctcgcataaattgtttttaaaagatggataaaattcgtgtatacgtttccgttacagacacagaaaggccatttccaccggtattttatccggtggatcagtggaatagcaactgcggtaatcacctttgttcaggagaatgttgccagtacgcggctatgcgccggatgttttcatcaggagataataattcataacggattttttgtggcggtcaatttttcttgtaatcgattgcaagcgtggttaaaaaaaacatacatcctttccggcggttgctgccggaatgttaatctcagtactttgtcttggtcattattcttttccccttaacaaacattgcttcatacgtggatcacaaataggggaatgtttatcatctggttgtgggcaggtgctgttttaagcatataggaactgttgcagcaccaaaacaaagattccataatattgcgcttaatgcaagttttgcgggttgtaaaatacaacctgtatagttgtgttttacaaacggcctgactgacaatcctgctaacttattgtatataaagtatttgaaaaaagcaccggatcagctattatttgattgtttgacgtacttttagaaagcaaaactttttttactatgaatattggtcagaaaattgcccgcctccgggaaatccggggcattaagcaggctgatctggcgcgtcggttaggcgttacacaacaggcgttatctaaaatggagaattgtgagtcgatggatgatgaacggctggagagagtggcttccgccctggaagtatcgccggacgtaatccgtaatttccgggaagacgtgatcatcaacaatgtgaatgaccagaataataccgtgatcaattaccagtttaatcccattgaaaaaatagtggctttatacgatcaactcctggccacagaacggaagcgtattgaattgctggaagcgatgttgaagcaggagcaggaaaaaaatcgctgaagcgtaataaataccctttaacaaccacatggttacctttaacaaccatcactacgataaacacccatgataacaacacagccttgtaacactgttacaaggctgcatttataaagctttagccccgcttgccgccgcggcttattaagaaaatgatcaggcccaccaccactgctacggctaatatgccggtccacacgcctgctttgaatattccgcctataacttcacaactgctgagtaaaagtaccaggcatgacagtaacaaataagtgaggtttttcatatcgttcagttttaatgttatatactaccagacatatcctgtaccaaaaaatatttgcaagtgtcagaataattaacaagctttagcagatcaaccagaatagtatgaatacagggaaagccttcagatcggggctgcacgtggtggcttcccattcctcactttggggactctttctacagggtgaccgccacgctttcgccggcatatacgatgcacacatcgatgacctctttcattatggcatgcatttctgccaggataaggaaagggtgaaagactgtttgcaggacctgttccaggatctctggatcagcagggaacacctgactgccaatatcgggaatatccggtattacctgatcagcagcctgagaagacggctgctccgcgcattgcgtaaagaccgccgctaccagcaccgcgaatcatgggaagcctttgaatttgaatataccctgccgctcgaaaaccagttaatccagcacgaaaccatagaagaacaaaagcgcctcctccaggaagccctcagcaacctctcacggcgccagcgcgaagcgatctatctccgctttttccagaacctgagctatactgaagtcgccgatatcatgtccatgcaggtagattctgtatacaataccatctccaaagccatcggcatcctcaaaaagaacctcccgctaccgctcctgttgctgcttttaggcaaataaaaaatattttttaaaaaagtgatgagattttgagcgttacgggctctttaggtaaaagcatgttctcttggcagccagtaactatttatcatacacggcccgggagtttgcgatggacgaggactttcagcaatgggtactacacccggagcaaaggaatgtattctgggaatcatggctcaggcaacacccggaaaaagaatcggtcatcagcgacgccaggcaactcgtgcaaagcatccgcttccgcgactattccctgtccgcaccggacaaggaacaactgtgggatgccgtgctgaatggactggaagaggaggaagaagaaacaaccatcccaatacatccgtctgtctggaggaatgtgggtaaatatgcagcagccgtaatactcggtatcctgctcactacagcctggtggtggtggaagcctgcagtacagcaaccggccatcctcagcacctatacccggctgggagaaaccaggcacctgatgttgccggatagctcggaagttacgctgaacgccgactcccgcctgctgtatgctgttgccggaaacgggcagcgcgaggtatggctcgatggagaagccttttttcatgtaaaacataccgcctccaaacagcagtttattgtgcatacctacgataacctcgacgtggaagtgctgggaacacagtttaatgtaaacagcaccggtaaagaaatagtagtagtgctgcagcagggaagtatcctgctcaatataggcgaaaccagtaagggaaaagccgcagcgctgtatctgcagccgggggaaatgctccggtacaacaaacaggacggcgactataccaaaaaaagtgtagatgccatacactacacctcctggcacaccggccggttaatcatggatgattttacgctggcagatgcagccatcttcatggaacaggtgtttggtaaaaaactgatcgttcgcgacacacaactattaaactataaagtatcgggctcaatgcctatcgtttataacgccgatactatgatgacacagctgggtaaggttttccgtatgcaattcaaccaaagaggcgacgaagtctggatccataaaccgtaacattcgccgctcaattttatagatgtcttattcttaatcgttaaaacctgttcaagatgaaaaaaggtttacgtgttttgctgatgcaagcattggccctgtatttcctgtcccaaacggtatcagctcaggaattggctgatgccggcaatcagccggttccccccgcaaccggtaacagtgcggaagcacaaccagatgaatcatccctgaaaacagttctccacctcatcgaagaacatttcagcgtatccatcgcctacaaaagcaacctggttaaaaacaaaaagatacaattgtcggtagctgcctgccagtcggcagaagaagccctgggcaaagccttgtcgccttttaaccttcacttcgaaaaggtgcgggaacacttttacatggtcacagaaaaagccattgttcctgctcctgcagaacccgccggcatacagcaacaacacccggtaaagggcgtggtaagggatgaaaaaggaaatcccgtggctggtgtaacggttcgcatcgcgggcaccagcatcggtactgtttccaatgccgatggctcttataccatttccgccccgggaagaagcagtgatgaactggatatcactttcatcgggtacgaagcacaacgtatacccgttagcggtagatcactcatcaatgttaccatgaaagagggttccagcgcattgaacgaaatagtggtcaccggttacaccacgcagaaaaagaaagatctgacaggctccgtggcggtagtgaacatcgataacctgaaaaagcaaccttccggccaggtaacagaacagttgcaaggacaggcatcaggcgtcaccgttataggctccggtcagcctggcgaatccccgcagatccgtatccgtggtgtgaataccttcggcgccaattccccgctttatgtggtggacggcgtgcctaccaccgatatcgcagacctcaaccccaacgacgtagccagcctgcaggtattaaaagatgccggcgctgcttccatttatggttcccgtgcctctaacggcgtgatcatcatcaccacccgccgcggttccggcaaggtaaaggtggcatacgacggctactatggccggcaatatccaaagaaaggtaacgtatggaataccctcaacccccaggaacaggccgacctacggtggctggcctacaaaaattccggattagatcccggaacagaactctatggcaacggtacaaaacccgttatcccggattacatcctgccatcgggcgcaatggaaggagatccttccgttgacccatctctctattatgtaaatccaaactatactgacctggacgattataacagcttttaccagatttcaaaggccaacaaagcaggtaccaactggtaccgtgagatcttccgcccggcgcccatcaccagccacaatgtagcagtgagcggcggcggcgataaagggaactatctcttctcccttaattattttaatcagcagggaactttaatgaacacctacctgagaagatatacggtacgctccaacacccagtataatatcacacccggtatcagggtgggagagaacctcgctttttccatgtcagaaaatccttcggtagatatcaatacgtcggatgccgctattggtcatgctatgcgcgaacaaagcattataccggtatatgatatcaaaggcaactttgccggttcctccggcgatgcactgggagacgcttttaacccggtagcgacgcagtatcgtacccggaataataaaggcctcaatacccgtttgttcgggaacgtatatggagaagtcgacttcctcagatacctgaccttccgcaccagcttcggcggagaagtagcctccggctggtcgcactctttcctgttcccgcaatatgagaacaaagaaaattccaccagcaattcctacacagaaggatctgtgaacgcacatagctggacctggaccaacacccttacctatcaccagacgtttaataaacacgacctgaaaataattgccggcacggaatcttttgatagccgcaaccgcgcagtaggcggtactacgaaagattattttactttcgatgattacttccccgacctgagcaccggcaccggcacacaaaccaactacagcaaccgggcatcagaaggactgttttctatcctgggccgcgtggattattcatttaacgaccggtatcttttaagcgctactatacgccgcgatggttcctccaaatttgtaaacgaccattacggcaccttccccgctattaccgcaggatggcgtatttcccaggaagaatttatgaagaagatcagctggatcaccgacctgaagatccgcggcggatggggaatcatggggaaccagctcaacctcagcgttaacaatggctacttcctctacggtggtaatcgcaactcttcctattacgacctggctggtgttaacaatggcctcaatgccggctttgcaggcacacaaatcggtaaccccgacgccaaatgggaaagcgatgtgaatgcgaacatcggtatcgatgccagtctctttaacggacaattagatttctctgccgactactaccgcaaagatatcaaagacctgctctacaatcctgaattgcccggacttgccggcacaggcgcccagccgtttgtaaatattgcccgcatgaaaaatgaaggattcgacttctccatcggctggcataaaaatatcaacaaagatctgcagctgaacatcagcggtacactcactacctataaaaataaaattgtgaaaattgccgacggcgtagactatttcgatagcgacggtcgccgcttcgatggcagcaacatcatccgcaatgcagtaggccaaccggtttcttctttctttggatataaagtgatcggtttctggaatgaagaatctgaaattgccgcagcagatgaacaggcaaagaaaataaccaatagcacagacgccatttaccaggaaggcgaagggctcggacgcttccgctaccaggatgtgaacggcgatggtatcatcacaccagacgaccgtaccttcctcggtaaccctaaccccgacttctcctacggcatcaacctgggcgtaacttacaaagggtttgatttcagcatcttcctctttggtacacacggcaaccagatctggaataatgtacgctggtggcgcgatttctatccatcctttgaaagcgccaaaagcaaaacagccttgtatgattcctggagacccgatcaccacaacgcaacagcgcctatccaggaagtggacggatctaccagcacacaaggcgtacccaattcctatatggtggaaaacggcgcttatctccgggccaaaaatatgcagctcggatataccctgcccactaaactgctgtcgggtatacacgtagaaaagctgcgtgtttatatacaggctgccaacgtattcaccattacaaaatactccggactggatcctgaaatcggcggttccgatatcaccgactttggggtagacgaaggcgcataccccaaccagcggcagttcctcattggcatcaacctgggtttctaacaattgctcatttaaaaaagtaggatcatgaaatcattatatcatatactattgagtgcggccattgcaactcccttcatctccggttgcagcaagagttttctcgaacgcaccccgcaatcttccctcgaagaatcttccctcaccaataaaaagggtgtaaatacgctgctcattggcgcctatggtgcattggacgggcaggattttaaagatggcgatatggtgaatatctccggtggcagcggttttgccgtatctcccgataactggatctatggcagcgtatgcggtggggatgcccataaaggcagcgatcccggtgatgctgccgctattttgcaaatcggcactttcgtggggaatgctaccaacggcttcttcaatgataaatggcgcgtaaattatgaaggcgtgcgccgctgtaactttgtattgcacatcctgccaaatgttacagatatgacggaagatgaaaagaaagaactggcagcggaagcccggttcctccgcggccatttctattccgacctgaaaaagatgtttgataatgttccctgggtagatgaaaattccaacagctataacaagctcgatgtagatgaatataaaataccgaacgacaaagacgtttggccgatgattgaagcggattttaaatatgcagctgaaaatcttaatgaaatacaggatgtaataggtcgcgctaacagctgggccgccaaagcctacctggctaaaacattgctctatgaaaagaaatatgcggaagccatgcccatttttgaagatgtgattgcgcacggcgttaccgccaaaggaactccttacgccctcactacaaagttccatgataattttgatgcttttacagagaataacagtgaagcagtgttctccattcaatacagcgccaacgatggttccggcggcaccggcaacgctaaccagggcgaaatgctgaactatccttacaacggacctttcagctgctgtggtttctaccagccttcacaagacctggtgaactcctatcgcaccgacgccaatgggctgccctacatcgacgactttaacagccatcctgtgaagaacgacatgggactagccagcagcgccgcttttacaccggatgcaggtaacctggaccctcgtctcgactggaccgttggccgccgcggtattccttttctcgactggggcaatcatcctggtatgaattgggtgcgcgaccagcaatccgcaggtccttatgccgccatcaaaaacgtgtacatgcaggctacccaggataaattttatgatggtaatggctgggcgcccggcaacgccatcaactatgtgctgatccgcttcgctgatgtgctgctcatggccgccgaatgccaggcacaggccggaagcctggctaccgcacaggatcatgtcaatactgttcgcatgcgcgctgcaaatcctgttggctgggtaaaaacatacctgaatccatcacacccgatggacggatataccaacacgcccgctgcgaaatacaacatcaaagcttatcctgccggcgcctttaccgccaacggcaaagcatgggccatcaaagccatccagtttgaacgcaagctggaactggcaatggaagggcaccgctactttgacctggtgcgctggggcatcgcacaaacagaactgaaccgctatttcagttacgaaaaaaatatcaccaccgacatcgtgaacggcagcttcaccagcaaaaacgtgcggttccctattccacaacgccagatcgatctcagtgttaaaaacggtacggctacattgaagcagaacgcggggtattaagcggagtttgtctttctcgctgattacgctgattatactgattaatttgattttgtttttttggattttataaaggattaagaagctgtctcataaataaatgaggcagctttttcattttaggctttaaggatggttttatccacaatttgcagttgaaaaaaagggaagttgtaagtgtttacgcaccagaagttattgtgtaa

SEQ ID NO: 9 - DNA, 317565 bp, Chitinophaga pinensis
  source 1..317565: mol_type = genomic DNA
cggggacgcatgaaattgttatcgccgggttgatttaattcaactccggaaattgtttgctcacataaccgatgaaagtccatatttccagtacctcttcaagggctacggttacggtttcatactgcgggttcagtgaatgcagtgataacgtaccgttttgcttaatgtgattgcctaccactttaaatacaatttcttcttcgcctcccttcagcacgaggatgcaggcggtattatcttttaaatgggaccagtcctgcaggtattgcgcaataacatggctgccatccggaatgggttccatggagtcgccgctgatgggaaacatgcggatggttttacccctgggcaaaccgggcagggtaaatttgggcagtgccgaaataaacgccgggtcgctgaagccgctgcggtagcctgcccgggcgcgtgcaggaacaaactccatgttttcctcattgctgttgtcgaccgtaatcggcaggatacgtatatgcctgcctgttaggtccacctttttcccggcttccagttccaggagttgttcttccgggagctgcgacaggtcggttttcaccatgaggtccaggtctattttaaaatagccggagatcagcgccaggtcgtccatccggggattgcgtgttttcccgctttcctgtgcggtgatcttgttccggttcagtccaagtaaatcagataggtgctgttgggaaatcttctttcgtgtccgtaataatttgagattagcggcccagaaaaggggctgtttgtccatgtattatatatttacgataacttatatttataattgacaaggacaaatgtagggctttttactcattctgtttattcagcaaactgtttaattgctggtagagtgcttccccggtgaggtctttattgaagatcatgccggtagaatctatgaggaagttctgtgggatggctttcacgccatataccctggcagcgtggtttttatctattttaggatcggcgaggttggtccacaccatgctgtcttctttaatggcttcgagcaaatatttccggtcggccggcggatcgagtgccacgctgataatggtaaagtttttatccttgaactgtttatagacttcctggatcttgcggtgttcgcgtctgcagggttcgcaccaggaggcccagaaatccaggaatacggttttgcctttaaagtcggagagctttaccattttcccattcatgtcgggtacttcaaagtcgggtgcatctgatcctactgtgaggctcctggcccgggcaatttctgctgcaaaggcttttccttcggtggtattgcgtatttcttcggagagtttaaggaagataggttctatcaggtcggggtttacatccaggccggccagttcttccagtgccatgaggctatagaatgagttgggattttcggcaatgtatttatgttgaagcagtttttgtgcttcgtaggacacgcggtactgcagggccatttgctgctggaatcctttgtcgtcttttttactggccggcgccctgttatattcctttgaaagctgccggatggatttcagaacagatttcatggatttattaaagttggcagcttcctcgttgatgggggaagagatgcgcgctttgcttacatgttccctgatcaacactttggtggttcccttttccaggaaaaagatcctggtgtccgcgtccggtggaagctgcatgaaatcgatgccgccacctttggtatggaggatgagcatggcacgaacgggaccttccacggaaccttcaaaacggaattcaccattttgtaccactgccgagtcaactaccagcacatcattcactactttgttcaggtacacttttgcggggccgttctgtttggtaagtttgccgttcaggacatattttgcgggttgggcatttatgaatgcgggcaaacacagtgctataagtgttatttttttcataagatatgctatcaggagcctaaactatcaacaaaatttattcatttgcaatacaggacttttgttaatcctgaataacatacaatacagcgttatggcaaatcaaagtaagtcgccgcacatactgaatacctctactaacctgctgggcttttgcctgatcgtattaacttccattaaagtggctcatttcaatcatgccaccattatagatgactgcaccgggatagcggccatcctgctgatggcgagttgcctgttgtcttttttatcgttgaaaagcaacgaagggaggaccagtgagcggttggaacaggtagctgattataccttcctggtggcattaatatgcataagtatcacaattgtttttgtatcttttaatctgctgagctagttgacgttgccggaatgcccgtcgatagccctttttagcaggtttgcttacggttttcattgtaatatctccctagtaccatgacgattcgcatatatgaagaaaccaggaaggtctggaatatactggctgagcgcaatgatccgccggatctggcgctggagatggaagtccataagaaagtgcttagttttttccaggtgggagcatgctactactttatatttaatgcggtaaggggagaactcgacttcatgcatccgggtgtatacgacgtgctgggttataacgcggatgaatgtacgattaccgagatgatgtcacgtattcacccggaagatgtggccagtttcctggagtttgagcaggcggcggtggatttcttttcccggctgccacccgaaaaagtattgaagtataaagtccgttacgatctgcgtgtgcggaaagccaacggcgaatatgtgcggttgctgcagcagtccacctgcatacagcacgatgaaaccggcgccgtattacgcagtttatgcgtgcatacggatattacccacctgaaacccaccggtcacccggtattatcttttgtagggctggagggagaaccatcttttaccaatgtggaaatccggaaaacgctcacacccagccgggaagtgttgaccaaaagggaaaaagagatccttcgtttggtgctggccagtatgcccagccgggagattgctatccatctaaatatcagtaagcttacggtggacaagcaccgtaaaaacatgctgaagaaaacggggatcaaatcggctgctgaactggtggtaaaggcggtgaaggaggggtgggtttaatgcagcggattttgtctttctgcctgattacgctgattataatgatttttattttttgattaaggaaggatggaggtaagatccggagagacagggcaacgtgactgatagatatatgtagatatattatcatttaaaatggataattgtttatattgatctttttttataacattgttatgtcaaccaaaagtttcacgataacaaccagaacaacaaggagaaccgctgattctcgttttttttgtccactaagcaaaaacgttttagcatacacatgaagatggctgagattagtgaatggcaggtgcagatagcgcgttatgatgatgaacaggcatttgcccgtttgttccgtcatctgtacgaccgtttattgcatttctgtatccggtatgtgcatgtaaaggaagcagcggaggaaatagtgtctgatgtttttgttaaactctggaaccgccgtaaggaaatagagcaggtatctaacctggaagtatatctttttgtggccgtaaaaaatcattcgctcaattacctggagcagtattcccacctgcgcattgtaccgctttccggttccgatacggccgatctgcgtaacagcatcgacctggaacgcgacctggaatggaaggagatgcgttttaaaatggaccagatcgtgtcctcgctgccggcccaatgccgccgcattttccagctgatcaaagaagacggcttcaaatacaaggaagttgccgaaatcctcaatatctctccccgcacggtggaaacgcagcttttccgcgccatgcgccgcctgaacgaagggctgggcgccatcggcaaaacgaaggaaatgctgccgccgctgatcatgctgctcgctatgtctgccctgctcgccttcggcgagtgaaattgtcttggagcaggattacactgattatactgattttctggattttttttctttggattttattaatgattaggggagatataagcggatagcttcgcttatatctcacccactaattctgttaaaatcaaaaaaatccaaagaaacaaaatccagaaaatcagtataatcagtgtaatcctgagtaagacaacctccgcggaaaatattttttccgcgcttgtaagtagttttccctccgccacctgtccttatacctgaacacgattccattttatgataaacgaagaacatttcgtcttactggttacccgtaaactggcgggagctgcaacgtctgcggaactggcggagctggacgccctgttggaacagtacccggtattgaaagaaaaatatcatcacttccaccactattttgaagatccgcggcacctgtcggccgaaaacacggaacaggccctgcagcgaacgatgtctaaaataaaacaacaaacgactaacatccatccgatggagcctaagagatccgggagatggaaatgggtagctgctgttgctgccaccatattgttaccggtcggcgtcctctggttttttaacgctacacgtaagataccggatgccggacgggaacaatgggtgaaacgcagtaacggcaaggctacccggtcgtttattgaactggccgacggcagtaagatctggctgaatgcagaaagcgtgatcacttacccggaaaaattccgcggcgacaaccgcgagatcttcctggaaggagaggccttttttgatgtagccaccaacgccaaacgtccttttattgtacacctgaaaaaaggaactattaaagtactgggtacctcttttaatatccgggcctatgaaaatgaaccggtgcaaaccgccgtggtaacaggaaaagtagccttcattccacgctatgaaggaaccaaaaagattagtgataccatcctggtaacacctgatgtaaaggtaacctataccgccagcagcggcaccctgatcaaaggcaataccatcgggtcggaagataaagcctggacagaaggacggcttattttcagaaatgccaccctggaagaaatcggcgccagcctgcaacgcaatttcaacaagcgggtagagtttgaagccaacgcaccaaaacagtaccggttaaccggggctttccataataactccctggaagatattatgtactacctcagtaaatcgaaagcgttccactaccgcatcaccgattcaacattagttataggagaataatcacatcaagccaacaccaatatttattcatttttaatcaccactacgttatgagaaaggtattatacaagccttcttttcgtccgcctttcctgtcgctgataatctgcttatcgctgctgagcgtgctggatctgcatgcgcaggtagcctatgcggcagggttacgccggcaggtgcaacatcagccggtaaaggaacgggaaagacctcccgctatgaatcagctgatcagcctgcaggttgacaatgccagtctcgcactggtactggaaaagattgaagcacaaacctccctggtttttgtgtattccaacgatgatattaaagcagcacaaaaaatatccctgaacgtaaaggataacaaactggatgatgtactgcagatgatcctgttgccgctggaaatcaactatgaattcatcgctaataaaattatcctgaagcgtagtaatcttactgctgataatgatcagcagcaggatattactattaccggtcgcgtagtggataacaaaggagaaaccattcccggcgccaacgttcgcgtaaagggaatgagtgtgggtaccgttaccaatgtggaaggcaactatacgctgaaaatccctgccagcgccgctaacggcaccctgatattttcttccgtaggatatgtaacttccgaaatagccatcagcggaagaaccagcatcattgccatgctgaatgtagattccaaagacctgggagaaatcgtggtaacggcttatggccagcagaagaaaacacaggtaaccgccgccatcagcaccattaattcaaaagacatcaccagcaggccggccgtgaatatgttccaggctttgcagggacaggcgcccaacctcatcatgcagcagaacactgccgaacccggggcacctatgaccatgaacatccgcggggtaggtagcctaaccggcaatgctccgctggtcatcattgatggtgtgcaggcaggaggcaatggtttgcagaacctgaacccctacgatgtggaaaccatttctgtactgaaagatgcggcatcggccgccatttacggttcacaggccgccaacggagtgatctatattaccacgaagaaaggtaagaaagacgaacatccttcagttagctacaacggtatgtatggctggcaaatgcccaccacactgccccggcagatggaagcatggcagtacatgaccctgaaaaatgaagccctcgtgaactccggcaaaacgccgcagtacacgccgggtgatatacagtcgtggcacaaccgtggctccgaacccgccatgctcaccgaaatgatccgcaaatacacgccgcagcaaagtcacaatttaagtttaaacggcggcggtaaaaccagcagttacctgttatcgctgggttacctcgaccagggcaatatgctccagaataaatatgtgccgcaggacttttactacaagcgttacaacgcccgcctcaacatgtcggtagatgtgagcaaatacgtgaaagtaagcggtaatgtagcttatacccgctccacttatcgcacacaggtatctgatatcggcttcctgatgcgcgatgcgatgcgtgtaccgcgtaccactgccgtgaaagatacgctgggtaactgggtggtgccaccactgaccagcaacagcgtaatggctttactggcacagagcggatacagactgagaacagtagataacctgatgggaggaatcgatgtagtgattacaccggcagatcattttaagatcaacctgaatgcgtccggtaattataacattgataataccgttacccgtattaataaattcacgtatgcaccttattatactaccgccacaccgccattgtataatgagatgcataattccgaatacaaggatctgacgacaaacgtatatggtaccgtagagtatgagaatacctttggcaagcattacgtaaaaggacaggtgggtgtgcgcagtgatgcggtgaatgaaggttacggcttccgggccgaccgttttggtactaccaacctggacaacgactgggccatcggtggcggctatatccctaaaccggatggcaccttcgattacagggatatcggcacctataacgatatgagcaatcctaacctgtatgcgctgaattctcttttcggaagatttaactacgtttataacgataaatacctggcggaagtgacctggcgttacgacggttcttccaagctggctccgggccaccgctggcagttcttcccggcattttcactgggatggagattgacagacgaagcatttatggaagaagtaaaggataagatcggcaactttaagctgcgttattcctggggacaggtgggtaactccaacatcggcggattcaattacctggccagggtacgactgacagatgaccgcaattctccgtataccaccggtagttattcgtttaataacacgcctgctattggcgctactttctctacttacaacgacctgttgcagtgggaaatttctaccatgagtaactatggtatcgatgcggatttcctgaagggtgctttaacagcgtctttcgattattttaataagacaacagacgggatctatcttttccagacggtaccgggaaccgcaggtactgccgctccgctggaaaacgtgggtaaggtaaataacaaaggctgggaactggccgtgaattacaggatgaccaccggtaaattccaccacaactttggtttcaacctcgccgataacctgaacaaggtgattaaattcggccaggaatctgttcgtggttccgatgtaacctttatcattaaagaagggtttcctatcgcttcttactatggttataaatccgatgggttataccagaacctggacgatataaagaatgcacctaaagtaccatttgcctacaaccagcaggtgatgccgggagatgtgagatatattgaccgtaataaagatggggtgatcgatgaaaacgaccgctacatctttggtaatcctttcccgcgttacacttttggctttaactacagcgtaagctggaagaacttcgatatgaccatgttctggcagggtgtgggcaagcgttcccagttcctgcgaggcgatatcgtggaggcattccataacaatgaagaccacgccatggtgcagcacctcgaccgctggacgcctactaatccgggtgcttcctatccacggctgaccatcggttctgctgatgccaacaacttcgcttattccgattactggctgtttgataccaaatacctgcgtctgaaaaacttccagctgggctacaacctgcctgcagctttagtgaacagggcgcgtatccagggtgtgcgggtatactttaccagccagaacctgataacgattatgcctaaacgcttccgtgaaataggcgtggaccctgagtttacgcagtttgatgataagttgtccatgtctaattacaaccctattgcaggacgtaattacccgaatgcggccacttttgcttttggtctggatgttaagttttgatgcctaaacaatcaattgtatgaagaaattagttttatcaatattaatggccggcactttgttcagttgccgtaaactggatcagccgatcacccgggagttcactgaaactgcctactggcgtgattcacaggatgccctcgatgcgttgaccgcctgttatgaacatctttcaaaagatgattatttctttggagatgaagcgctgagtgataatgcgtataacagcggcggtggcatgatgaatgtaaatgccatttccaacggcggttatgatggcgccaacgggcgtgtatcggatacctggtcgtattactatactactattcgcaggtgcaataccgttaccaccaatatagaccgggtacccaatatggacccagcgctgaaagcccgcatcctggcggaaacccgctttatccgtgcgtatgcttattttcagctcaccgcctggtatggtgatgtgcctttctatacggacctcatcaccattgatgcttcccgtaccattgcacgcaccgataagaacaccgtccaggaatttatattagcagaactggcggatatccagaaagacctgcctactaacacgcaacaggtgcagaacgaccgtggtcgcattacccgcggtgcagccatcgctatgagcgcccgtgtacacctgttccgcagcgaatgggcagctgtggtagcagattgtgagaagctgatcggcaaaacagacaatggcgcctatgccttgtttggcaactacagcggcctgtttaccgtagccaatgaatataacagcgaggtaatcctggacctgcaatatggtggtggcagaacatacgacaagcaacgttccttcatgccgcaaaccattgccgcgctgagaagtgtgctggtgcctacccaggacctggtaaatgattatatcatggctaacggcaaagccattggtgaagccggttccggttataatgagaacacgccgtatatcaacagggacccacgctttgaggctaccatcctgcatcatggctctaaggtgattgatttcgcaagagcggagcaaaccattcttacgcagccgggttctgtgcctgctaccaatacggtagacgaccagggcgcttctcccaccggttattatttctacaagtattatgaccgcgccgctaccaattatgcttccgggttgaacctgatcatgatccgttatgccgatgtactgctgatgtatgcagaagcaaaaaatgagttggggcagatgaatgcggccgtatggaatcaaacgattcagcctatccgtgtgcgtgccggctttaacgatgcaggcgccacgcagtttaatgcagcgcttaaccaggatcagcagcgtgtggtgatccgccgggaaagaagagctgagctggcgttcgagggactgcgtatttacgatgttcgtcgctggaaaattgcggaggtagtgatgaacaggccagtgagaggcatcaaagtaacttccggtgcattcaacaaagatccgaacggctacatcatagtggaaaacaggttgtttacaaatcccaaacactacctgtggccggtgccaaccgtagaacgcgatcagaataaaaatctttcacaaaatcaagactggtaatatccttccacctaaaactgtaataacatgcaaaaatatctgatcatcatactgagtgttttattctttagttgcaagaaagacgattattcactcaacaccaatatgcagccggtgccaaagctcaccgcgccgctggacaataaatacatcaagctgcagcctactaccagcgctacggtgagctttgaatgggaccaggcccgcgccgaagatggttccctggtgcaatatgaagtagcctttgacaaagccggtggcgatttctctgcccctgtggcaaagttttcttctgatggtggcggtgtgcagaacaaactgactttgtcgcataaagacctgaacagcgtggcgggtaaagcgggcattgcttccctggccaccggaaaactgatatggacggtgctggcatccaaaggatataatatccagaaggctgccgaaacaaaaaccattgaagtagaaagacctaatggttttgccgagatccctacagatgtgtacctcaccggtgaagctaccgaagtgggcgctgacctgtcgaaagccctgaagctgaaatccactgctccgggggtatatgaaatttatacatctctcaaaaacggtaaatatcatttcaccagcaggaacactggtacaccggatacctattccattaccggtaccgctgtaaaagaaggtggtgaaagtgaacaaaccgcaggtactaaaatatatcgcctgcgcctggatttcaataacgccgcagcaaccgtaacagaaataggcactattggtctttggtttgcgccactgaataaatttttattcgagatcaattatgccggtggcggtacctggaaaattcagagccagctgatcactttcaaacaggaatcatggggacgtgatgagcgttataaattccgtatcaacgtaaaagacagtgatggcaatgccggtgaagagtggataggaagttccaatgcagataacaaccgtccaacttccgctacaccgctgagtttctgggagctgcgtcctattaccaacaacgaccagtggaactactgttacaagttcgctaccgaagcagacaataagaattgtgatgtgaacctgtacttcaccacggataaaaattacacccacgaaatcatcgtaaaataatgaccgctatgaagctgatacgatattcccttttaatgctctccctggccttcactgcatgtttgaaagaacctgtagatgatggcccgggtccgggagccaacaaggcgcgttatgttttcgattgggcgcagatcggtgattcctctttacaggggctcaccagcaatttctggaaccaggagaaatattttaacgccaataatgcgggtaatgccacctttaattactggcccaatgcgcatgcactggacgtactaacggatgcctatatacgtaaaaatgacccggctatcaaagcccgtatggatgatttgctggcgggcatgaaaacaaagaacggcggtacttacatcaaccatttctatgatgatatggagtggatgaaccttgcctgcttacgcgcttttgaggccaccggcgatacccggtacaaagatgtagccgtattgctgtggaacgatatcaaaggcggctgggatgatgtatggggcggcggtatccactggaataaggataaatccaagaactacaagaatacgcctgccaatgcgcctgcgtgtattattgcctgccggatgtatggtcttacccagaacccggatgatattgcctgggcgaaaaagatctacgactggcagaaagccacgctggtagacccggttaccggtctcgtttgggatggtattaaccaggacggcagcggtcaggtaaccaagaactggaacttcacttacaaccagggtgtgtttattggagcaggggtggagttgtataaactgaccggtcagaatgtatatatcaatgacgcattgaaaacggccaacaacgccttagccggtggatttaccaatgccaatatcctgaaagatgaaggcggcggagatggtggtttgttcaaaggagtactggtgcgttacctgatgttgctgatcaccgatggcagtatcagcagcacggatgtggcaaagtatgccgctttcctgcagctgaacgcagaaacgttgtggctgaaaggcacgacgcgcccgcaggtgttatttaacaaggactggtccaccatggctgccggcagcgacctcaccacccagttgagtggcgctatgctcatggaagcggcggtgaagctgaagagtatgggactgatgaagtaatgaaaatgataaagatggggagaagaatagtgaggcttaccttttggtgtttgctgtctgccggcagcgtatttgcccaaagcaacaggcaaaaggcagagatgctgcagcaggcagtgaacaaatatttgtatgagcgcaaaacggggttgtatatccaaaccagcgaccgtacaaagaatcataatccgcatgccgacctgtggggcctttgcgggctcatacaagccaccaatgaaatggaacggatccatcccggcaaagtgtatatggcgccggtggtggaggcaattaaccagtattatgatcctattccacctgctccgggatatgcatcttatgtagtgaaggaaaggcgggaggataggtactacgacgataaccagtggattggcattgcgtacctggatgcgtatgcgcgtaccaggaagaagtggtacctgggtaaaggaacggagatctaccgttttatgatgacgggttacgataccgttagtggtggcggtttatactggaaggaaagagatctcaccacgaaaaatacctgttccaacggaccggctattttactggcgctgcaattgtataatgctgttcataaacaagcctacctggatactgctttgttgttgtacaactgggtaaacaggtatctgcgcagtgaggatggggtgtattgggatgccataaagccggcagaaaacaaccgtattgattctgcgacgtatacttacaatgccggcgttatgctggaggccaatgtaaagctgtaccgcattacaaagaatgcgcagtatttaaaagaggcccgtcatattgcagaaggcagctacaggcgctttttcagaaatggaaagtttccttcttcgtactggtttaatgccgtattgctaaggggatacgaagcgctgtacaggacagataacaacccgaagtatatccgtgctatgcaggagtatgcgggtaaggtatgggaacaggagaggaacagcagcaacaatatggtgggcaaccgtccggaaaaagagctgctgggacaggcggggatgatggaaatttacgcccggctggccggtatataaatcaaagaaatgaaattaaggggaggcccgtagcatttatttgttacgggctttttcgtggttacccgtgagcccgggttattattttgctataatattacataattccttaattttataatttttattattaatttatcccgggaagcattatttcctgaccatcttagaaaagagaagaagacaacctatcctatcctatgaggctgatgttattgctgctttttgctttcgtgccggtatctgttttgggacagacggcggcgccggcgggtaaaaaggggaatcgtgcaacggaattccagatgaaggagggcagttatctcagctttgcccaggttaatttaagtcttggtgaaataggcttccgcgtggaagtggcatcggagcacaaaaagagtaatgcccggctggagttccggatagataaacccaaaggtaaaattattggtacccttgacattccttatacgggagatagcacctatgcgttgaagttaacgggtaaccttcgtcatgccgaaggcgtgcatgatctgtacctggtagcgaagggcgggatgcctttcagcattacagcatttggctttatttttaattattaatataggcgttgccgttatttttttggaaaattaaaatagctgcttatctttgcgctccctgacacgatatcagttgcccagatggcgaaattggtagacgcactgtgttcaggtcgcagcgcctgcaagggtgtgctggttcgaatccagttctgggcacgagagtggacaaatcgagattttcctcggtttgtccatttttatttttatcaaagtccgcgtccagaccgtatattagcttgacggcttcattgagtcgggcggttcgataatgtaattaaatacttcatggcaagggcaattagggttgatctgaacttcgaatataattaattacatgaaagtgttattgttttttgtacccctagcctgtaccttagctttatcaaaacagtcacccaaataagttaatccaacaatgattttttttacgcaatgtcatgtaccttacctatataagatagtggacgttctacatattcgtgatttttttagtgcctatatctcctgtatcttatccccggataaatcccttgatactgtatgatattattaagatatcttgttgaatagcaattgcagttttgtacccttattccaggtcctggtatctatgatttatatgtttaagttctatgttattggtattttttgttcggtcaagctgctgatccagaaatccgacagaggatactgcatgctaaaagaggtacgaacggctacgtgattcaaacatccctaaaaatacctaataatgaaaaagcaatttttcaagaaacttcgagcgttactaacactcgccttgttaaccataacctctctggcccttgggcaatcagcattcagagttaagcaagatactgtcatggttgttggtgctgagctccaggtaaaaaatgcctccaaaaatgtacagggctttctgtataaccagggcgatggaaatacagtattcaaaaaactttccctggaaaatataggagacagtgctatcgctattgccggacaggatactatcgcggtaaggttttccggcggtggaggtgttagtgtgccggccgtttcgctggctgctatgtctattgatgccaacagtatgcagctgaaatggtggcagtcagacagggagctgtatcagtcgccgaagatagccctgattggagacagccagggggcggggagttatgccagtacaccggccaactccattgccggaaagctgcaggcttatatttatgcagtatcttccaatgcacggctgacgaactattgtaaagatggatataattcccgcaatctggcgcctacaggcagcaatagctttgtagactcgacgatgaacgtcaccaaggcaattgctgatgggaataatattattatcctcattaataccagtaacgactatgcatcccaggccagtggcggtgagatgtctacagaggaggcgctctctaataccttgctgatagatgaagcctgcaaaaaagctggtgtacagttgttggtaatgagcagtattcctcgtacggctttcggtgctccacagcgccttaaactgagacaaactgcagataacctgcgtaaaactttcggagccagatgcatctatgcgtatcacctcctggaagaccctgctaatcccgatgtattacaaccttcattgcagttcggcgataatatccatttgaatgaccaggggtacctggtaatgtttaatgcaatgaggaatgcactcgccagctattttacttccaataccgatgttgttaagtacattgtacaacggagcgcttatataaacggcctctataatgattttaaaactattacatcaccttatgaaaacacacttgctatcagccctgatagcagcttttaccgaatgcggatctatttccgggacgggtatttttccagctggagtaatgtagtcaaagctgtagttgatggtaacatcccaggggggccaggaggtaatggaataactgtcaatgcaggtttagatcaatatttaaatgaaaatgaaagtactaccaacttttatggaaacataaaaatcaataatccttctctttcagttgcttcctatcaatggtcagttatttctaatataacaggcgttacattttcaaacgtaaacggtataaatacaggagttacaggaattcctattgctgccaggtctacatatcgtttgactgtcactgataatcatggttcaacttacgctgatgatattgatgtttcagttgccagaccatcggatatgtttagttcaggaggttatttagacaacaaatatgattctaacaacccaaatttgaaaacatgggtttacttgccacaaggttatgattcattaaaaccaggtggttaccctttaataatattcttgcatggagttggagttaatggcgttgagaataacgatgatattaatcaattattactggaagctgaaggattaccatactttttgcataataagttgtttcctatgcagtgtgttgttgtttgtcctcaattgcatgatggactttggactttagcaaccgcacaaaaagcagttaattatgccgttaatggatatgcaattgattcaaataggacatatgtaactggtttgtcttctggcggcgcaggcacaactaacgttgctttaggtaatccaaatctgttagctggtggtatcgcttccaatacaacttttaatgatgtagcacttacagggaatggagatatagtaaaagatataccatttttgtttgtccattcttataatgatacaagagttccgttcacttctcaatattcaaccttagatgatgttaatagcatcaatgctgccaatccaaaaggtatataccctccattaatgttaatggcttggaatagtgaacatgataatggtacatggaataattatgtttatgataaaagaattgccccatttgattttgaaactgactttttactttttcacagcaaaaacttaacaactacctgtaataattatgttacaaaagcagaagaaaaattgaagttttatgattggtccagagcaaaattaattgtggataaattgaataatggaactgataaaacgggttttacaaaccgattgaatacagttttggatagtctgacaactgctaaaaatcgtaaatattatatgttgaatcttgggagcaattcaacttttaacttatatactatcaacaatgttacttcagctgctaacaatacaactgtatcaaatttgaaagacattaaaaatggtacaagtacaaaaggatttacagtagttagcaaccctgaaggaattacaactgatgggcttaatcataattacatgggcatgagtgctgatatgttcaaaacagcattcaaatactcaaatgttaatccagcgcaatggaagttaactggactggatgtaaacaaatattatgatgtaattatatacaactctaatacttcaaaagctttatttaattcgaataataaaactggtaccaggtcagaattgaacggcagtatcgctcaaagtagattagaaggttttaacacaatgtttacaactgaccattataatgttaaaccgaatgcatcgggagagatagttatgaatatgtccgctttagctaattttcaattcaatcagaacatatcctattatggtcaaaccgttgcaatattattgattgaaaaaacaacaacggctaatccaagagccaatttcggcaaatttaatttcgctagcacaaccgctgcttcccatcctgactgggcaactttaacaggcgacccaacaacatcagttcaaacagcaatagaccctgtatcaggttgggcaatcaatactgttagtactgatccaactcattgggcaaagtatagtggtaattatgggaatgacaatgaagctcctgctaacatttataccgatatttttccagcagttgtttctaaaagtgcgaggttaaattatgctttgaattttaatccagctacacaaaactataactatgaagtaattggtgtgcctggaatgggcttacctgccggcacttacaatgtgaagatactttcaagtactacagctgattttgcaccatcaaaaatttgggtaaaaatgggtagcagtaatggggtatgtgataatacaattgtaggtaaggataatgttaacaactatcttacttatacaggttatttaaaagatggagaaaccataaaaattggttgctatatgccggatgtttggggtttgtgttttatgaatgcagtgatcgttgagaaagtagattaatgtactaatgaggaactttttgtaaagacgttagctcataaactgtgtccctggtagaaatgtaacatcagatgcaaacgggaatatcaacattgcggtgtatcagtcggctaattctgccacatacggctctttttcattcctgaatgcattgatatgaaagaaaaataacccgcagcagggttgcttccccggatagcgtccctgctgcttcccagataaataatccctataccatgaaaatttttatatggcaaaagttatagcggcgtggtgtacctgtgtgctactttccgtcaccgttcatgctcaaacggtaaaagtaaatgcccccgttaagcaactggaggaatatgccaaaaaagctgggctgcctatgggtaaccctatgttgcagatgatactggcagactcgctgaacaaaaggtcagccatggcacaggctaaagcatatctccggcaaaatcttccggctgttccggatgtaggcgccggcaaatatctgcaggaatccgcccggcaggaattctttcagtttatcggtaattcagccggtaaacagcagctcgcgcagttgcagcaaggcatgagtaccatcaaagacactgcccgtatccgtcaatacatcgcggataagctgcggggcttctatgccttacgggatgaaacgggcgtgaataagctgttaaatgccggtgcgtatagtaacagccttaaagaagccagtgccggtgctttcgcagaaaatacgccgggcatgcctatgctgggtaccagcgttacaataggggatcagctgatgataaagaatatacccgttaacgtggagtattcaaatatttcaggacaaagtacctggaacaatccctttgcggatcagtcgctcgtgaagttttcatttgataaagacgcttacgtaaaacgcctcaatagcatagtcgaaaagaaatatgatctcaaaaaatactttctgaaagacattgatgtcaaaagcgcggtaaaatcctttaccaacagccggttggaagcgctccagcaaaaactcacagggctgggagaaaagcagtcagccgccttcggccaattgctcaacagcgatcatatcatccagctggattcgttacaactacggaatgagttactaaacaatagagctttcggcattacagcagaagaccttgagccggttgttgcggcattgcaggatagtatcttactggcacatccggtggccgacagcagcctcaatggactgttggaacacttccgtacagccagtgcagccagaaaatatatggcaggcgttttggcgctgaagaaagaagtaggagaaggcctgcaggctaagtccattatctcagacgaacgggtgatgggaggaaaaatcaacgggcaactggaagaggagagcaacaaaatcaggaacattaaagaactgttgccattgagcggtctgcaacgcctgttattaagtgccaaacaactcgacatcggtaacattgcggcttccggaagtaaaggtggggtacaggacttgtttatgtccggtatacagaccagttttctgaacaacaataaattcctgatgctgggtgccggaaagcgtatcgatggcggaacaataaaagaccttgcttttaattcatcgcttgatccgggggcttacagcatgcagttcctgcaaatgggcgccggtgatattacacagccacacagccatgccggggtcgtgaacgccaataccaaaagcgattcccgccgccagtatactaccctgaatttacctagaaatacttttgtaggcgctttttccgaagatatcagcctgggtggttatggccgtatcgccgcacaattatcaaagtccagcaaccagtttaaaaattcggcagtaggtaatgacccgatgctggccagtaaggctgctgcattatcgctgttcaacgatttctgggaaaccttgtcagtgggcctcgactacaacgggcaggtaaatgagtggaatatgaaccagcgcgcctacgtcagctattctggcctgggatataataacccggcgtctcccggagcaggaagaggaacgatacgttacggattaaaactgaaaagaaactggtataaaaataaactggtgctgggagtaagatccgatttccaggatatcagctcttcggccttgacttccagcaaatggaaaaacaggcagtttgctattgatggtcgctggaaactgaataagaagatcgcctttgatgcgcgttttaaccagtcggccatgaaaagcaccggtgaaaaggccccatcctttcagtatatgacccggcagttatcgctcgcttcacaggtgcagggaaaaatggccgcgcttccatacaacagcaatattatgctgggatatcagcagatcgatattttgccacaacacagcaccttactgaatattaatattaaccacaacctggtgatcagctcacatgtcctttcgttaaacctgttttacaataaagatattaagggtgaagcggtatatgccaacctccttacggttgaaacgggatggacctaccaggtgtggaagaaaataagctgtagcagcggtatgacctacctggataataaggcggtggtgcagcaactcggtttcaggcaaacagcaggcgccagtgtactgccccggttaaatgtgaatatgtatgttgactgccgtaaaaacctgttgaatacgccacagaactatctgttcggcaacttcagaagtgaactggctatttcttaccaattgaattaagtacctatgttaaagttttatcagggagtgatttttttgatgctgttctgtactgttcaactccgtgcccaggtgtcttttgtttttatcccagagctgcatggccgcacattggatggcctgttgcaggcaaaagtggccaataccggcagccagtcgcaattggtgagtctcaccgtaaaagtatctgttgccggcgccggcaacattgtaagtataaaaacacctgcctttcagttaatgcccggtaccaactccttaccgggtggattgattgccagatccgccatccgctttgcggaaaataaggtggccactgtttgccgccagtccggctactttatggaaggggattacgaatactgttttgaactgaatgccggtgatcagtcgcaccagggcgaaaccctgggcgaccagtgcttcgattattacctccagccgttttctcccttgctgctattgaacccggcagaagaagacaagatctgtaacaagcgaccaccctttttctggcaaccactattgccggctgttccgggtgtacaataccggcttgtactcacagaagtgaaacccggacaggcaaaggtagaagcacttaattacaatatgcctttgattaaccagctgggcattaattcccccatgcttttctatccttctctggcaaaagatcttatgcagggaaaaacgtacgtgtggcaggtaagcgcctacaaaaatgatatgctgctggtgaactccgagatatgggagtttactgtgttctgcgaagaggaaaccgcggcagtagtaccggaaagctttagggatattacggatctgacaaaaggtaatttttatgtggcccgcggaaaagtgctgtttgcggtagaaaatgtgtacgacaaagccccgctgaattataagatccgttgtatcaccaggcccgaactggaaatgcgtaaactaccggcgatcaaactgaatcggggaaataaccatgtggtcatacccctggcagagaacaggtcattcgtggatggctactattacctgctggagttgaagctgcctaacggtgaagaaaaacaattaagatttctttataaaagtgaaacggaatagcgatgaaatacttaataatatccgtgatgatagggttgttaatgtctgcctgtcattcaggaaagaaagaaataaaagctttttatgccaacaatggccaggcgctggttcaggaacaggatgcaggaggtatcggggtaagggccagttacctcccggtgcagtgggaacggatgctgggaagggaaaatccggatgcagcaggggaaatgacatttaagttaaacgttgccctaccagcttcctcccgggaagaaagccggaaaatgcaggcggtaagcgtggataccctgttttggctggtagtgggaagtgatacgctggcggcacagtttacgcagcgaattccgaatggaagtacctcttcagcagaatacctgaccacgttcaaaagggccgtgccggcaggaacagctgtattgtatttcgtgatgaatgattggatgtatacgcatcataagttggtgtttcccttccaggttgcacatatcaatagtattgactcattaagcagcaggttatgattccaggaaacataatattcagaaagtccattgcagttttttttctaggcttgcttaccttccagatattggtaccctgcgctgcatgggcacttacaaccggtccttctcaaccggaaagcaaacagtttgcggaagcaggtaccagtgaaacggtcgacatgtttaccggtgcatttaaatacaatattcctataatggatattgatggttaccccatcaatttaaattaccagtccggtgtaggaatggatgatgaggccagctgggtaggactgggctggaatctcaatgtgggcgccattaaccggagcctgagaggtattccggatgatatgaacggagataaggtaatcacggaacattatacggcgcctaaaacaacaaccggtgggcggggaacagtcaaagcggagttctttggcggggcgaaactgattggcctgaaaggctctttgtcgctcggtatcttcagtgatacttataccgggataggagccgagttcggcataaatgccggtatctctcttacacgcgggagtggtgccttaacgcccggactgggcgtgggcctgatgtccaataccagtaacggtgtggatgtatcgcctaatatcacgctggctttatatgataagtcgaatgaaaataagaccacaaacgtagggctgtcggccaatctaggttataacacccgccaggggctgaaaagcctcacactgaacgggtctttcggtattacaacgagagattgggataatcaatcgggttcttctagtttcgatgtaggtggcatcggattcacttataacacaccacctttttatccgcatatcggggtaccctataggtctaccaaccgtagctacagtatagatgtagggccttccggcgccggtgcttttgccggcgtaggacttaccggctaccggtataaacgcgaaatactgaacaggattaatactaatccggcatacggatacctgtatgcgaaccagggtaaagatgtacccaacgccgtaatggatttcatgcgggagaaagataatgcagtaattcccaatatgcccaacattgcgattcctatcgctacggccgatattttttcctattccagccagctgggaagcgggcaattccgcctgcatcgcggcggttcaggaacggtgtttgaccctgctgtcaatgacgcgaataacaccactacccttggagtagacctgggttttggattatactttcatggtggggtcacgttttataagcaggatgtatccaacaaaaccgggaagtggaaaaacgataaccgattcaatggagtagctgattataagaacatcgataataccctcgaagagcatgcctattttaagcagatggatgagaagaatgtggggagcaatgaatatgagacattgatcaaaggcgaagacgtagtgcatgtatctttggatggactcagcagtaaaagtgaactgaaagacggatataataatacttatcccatatccacatccaacccgctgacaaagaaagtaagacaggtaagacgtaatgccatttcctatctcaccgcctcagaaacctacaagggtggcgtgataagaatgaaagaagattaccgggagaacaaagtaactggttttacacccgcgctaccttccgcagtaacagagtcaagatatggtactcatctttctgaatttacgattacgggagacgatgggaaaagaatggtatacagcctgcccgtttataacaaggtacaggaggagtattcatttgctacagatccgaatgcggcgaaggatgaggacagaaacctggtaggattttcgctgaaaccagatggaggaatccagcataattacggcattgacaaatattttcataaggaaacgcaacctgcgtatgcgtcggctttcctgttgtctgcgatattgtcgcccgattatgtagatgtaacaggcgacggtatttcagatgatgacatgggtactgccattaagtttaactatacaaaagtaaacggtaattacaagtggcgttctccgatgaagccgaatagggcgctgtataacaaagcattgaatgcggatcaggatgatgataaaagtagcattgtttatggggagaaggaaatatggcttttaaactctattgagacaaaaaataaggtgatgtttttcctgttggacagcaggaatgatgcgttaggtgttaccggtatcaccggcgctatagacaataccgccaatggcagacagcgttgtttgaaggaagtccgcctgtattcgaaaaaagatctcactacaccgataaaaacagcggtattcaactatgaatacacgctctgtcagaaagtacccaaccaggctgttgccgatagtggtaaacttaccttaacgggtttgcactttacctatggtgcttctaccaaagggaaacattttccctatactttcaaatatacgggcaagaatcccgattatgagtatctctctaccgacaggtggggtaattataaagcggccaaatccggtttgaataatttaaataatgaccgcttcccctatagtacacaggataaggcgatcgctgatcagaatgccagtgcctggaatttgacgtatatcagtttgccaaccggtggagaaattaacgtagactatgaatccggcgactacgcttatgtacaggataagccggcgatgcagatggtggaactgacgcagttggtaaataaagacggtaacccggagccggacttcttttttgcccgtggatttatgatcaatattaaagaaagcctgaacggagcctccgcagaagagaaaaaaaatgattttatcaggcgttacctgaatggcgaaagggatttttacgccaagctatttgtgaacttgacggataaacccgacaatggcacggctgaaagtagttgcgattatgttccgtgttatggaaaggtgaaagatgtgatagaaaaatccggtggaaatgtagcggtcatattcgacaccatgggcgaagggaatgtgacttcgaatcctttcatttttgccgcctggcagaaaatgagattagagtatcccaagtatgcttatcctggctacaagaacaggatatccgacgatatgcctatacaggcagcattaggcgcccttgtgaactccatcagtaacctcagtgaaattacaggtaacttttataaaagagcggagcggaagaggtttgcacgaagcgtggatctgaaaaagagttttggacgtattgcaaaggtggatggaataaaactgggcggtgcggcccgggtgaagcgtgtcagaatatcggatatctggaacacgatcagtggagagcctttaacaggggctacctacggtcaggaatatacgtataccactacctggaatggaaaaacgatcagcagtggcgtagccagctatgagccgggagtagggagcgatgaaaatcccctgcgtttaccggtaccttataccgaagatataaaaggtggtctcaataactattactacctggagaaaccctttggagaaaccttgttcccggcaccggtagtgggttatagcaaagtggtggtaaaagatctgaatgcggagggtgtggtggaagccgcacctaaaacgggatgggtacaacatgagttctatacttcaaaggatttcccggtacaggtaagctatgatcaaagtccggacgcctataattatgattccaaaggttggtttagttttattggttccaatgtagcacatgaactggtgttatcccaggggtatgtggtgaaactgaacgacatgcatggcaagcctaaagcagaaagagtatttaaccagtcgggcgcagagattgccaacaccagttactacttcaatgcaaagccactgggggtaggcacgcaaacgctcgtgaataacgtggatgtagtgaacgaaaaaggagagattacgcagaaccaggttatcggtagagagatagaaatgatagtagacatgcgggaagaggaaaccagcaacacaggccggaccatccgcgcgggttttgatatgatacccggcttcccgataccgtgggtgatcccacactggcccatgagtcagaacgatgagtatcggttgttccgttctgcatcggtattaaaaaccgtgcaatattccggggtactggaccgggtagtgaaaactatcaatggatctaccgttacgaccaaaaatactttgtatgatgccgttaccggcgatccggtagttaccaccaccaataacgagtttgatgatcctgtgtaccaggtaaatatgccggcatactggatgaatagcgggatgtccggtgcttataaaaataacaatacccttatccggaatttcgagacagatgctcaggggaaaattccatctacgtttaccagatttgtgaccacaggcgatgaactgattgatctgaataagcaggattccatttactgggtggtgaaaacattgaccaagggagaccaggacctatcctataagcttatcaacaaggacgggaatgtggctaataatttcaagagcgacgtaaagttggcccgctccggataccggaaccaactgacggcccccggcgcttccgtggtgtgtttgaaaaacccggtgcaaaatggcgctttccgctttacaacagatacggacgacgaactggcttccctgggtgtgctggatgcgagcgtaacgctatacgatcagtcctggggctcccggcttaaaatggagggcatttatccagggtatgactatgagcgcccggacaggggggtgtatatcaggaatcctaatggaaacgaccgcatgtggccctattatgcacagtacaaagatagccaggatgggaatgacggaacgagcttttacgctcagaatggtgcggaatatggtaacagaaaaggatatttctggggagggaatggtaacaccggaagattaacggccattgggatgtatcccaggtataagaatccaaatggtaatgatttgtggtattcttacaacactgatataacactggaaccagctgccagctattctctgggtctgggtggaaatgatgaggtgtatgtatatatcgatggtgtggaagtgagaaagctcacggaagagaagctaagcaatcatagaaaatggcatgtttttgaattagcgaacatgctccccggtaaacataatttcgaggtcatgggtcgtaattccaagggtcaggaagccggttttgctgcggagatctataataaatcggcttatgaattatataacaccggtaattatacaaatattatcgcttattcatcagaagatctgatacattatcccgccgatgtagtggaacgtcagggggagttaggtacaccaataagtaatgagaagtataccttgcctataacctttcagatgaatcccttcttgtatggattcctcggaaactggcgcccggtagagcagaaagctttcctggtgaacaggaccgggcaacagctgtctgtccctgatatcaggaagggtggggtttatcagaactttactccttactggtatttctcagtgaccgataatttgtggaagcccacttacgtaaataatgaaaaatgggtcagcactggtactgccactctttttgatgctcagggaaatggcctggaatcaaaagatccactggggatttttaaaagcgcattgtttagctttaataatacacttaccgccgctgtggcctccaatgcaatgcagcgggaaatattttacgatggatttgaagattatgcatatcgggtgaaggctattccggaaaatagtaatccgaaagatagcttcaacatgttcgtgatgatccgcgacaagggacagtatacagactggctggataacaagattgtccacaccggtaaatacagcctgaaactaaacagcccactggtattatacacgcgtccgcatgaaaatgtacaccataccgtgccttatctggatttttctgacctgggagaatatatgcgtaccaccaggccctatgtttacccgatgggatttgctccgaagccctatgcgaactatattttttctgcctgggtaaaagatgcacagccatctggtaatacctccgatctgaaagtaagtgttaatggcgcggataagccacttacggtgaaggcttcggtagaaggatggaaactggtggagatgaatttctgggccagtgatcccggggtatccaccacgctcgcactcacggctggtactgcaacaaggatagatgatatccgcattttaccggtgaaaggtaacataaaaacgtatgcatatgatcccctgaaccagcggctcatggcgcaactggacgaaaataacctggccacactgtatgagtatgatgatgaaggtaccctgatcaggttaaagaaggaaacagaccggggaatcatgacgattaaagaaaaccgctcttcttacagggcgaaaaattaaccgctttaatattgaaagatgaagaagtatcatataagtggaaagtttatcattttattcatggcggcagtaatggtggttggatttgctataggcgccaggcccttgctgagcagctggtggccttctttgaaagaacaggcgccggtagcggaagaagcaacccattttcaacgggaggatgctgcgttgctcggacagatcattgctatttacagacgtatcgatacgttgtctgtgattgatatgggaggcagtatccggatcagtgatccggcggagccgacagaaaatgtgaatgccacatttaattattgcaggagaaatgcagaaatgtattatcagctgggcgataatgaaatgatccagctgaaagacgtgtgtatttcggctaaccgcggaattgagaaactatttgtttcacctcccaaagaggtagtggcggctccccagttaccgatcgacagtatcatttcactctgggagagcgacagctatgctatcaatactatacacaccgataatttaacaaccgtgcaactgctttgtgaacaccatgttacctgtaaggaattgaaaattacctatgatcgtagtaccgcgaagttgaacagcatctatatgcgtttaaccaacctggaagatccgctgaacaggaagatggacagagagatcaccacggttttcaataaatggaatgaggtgattacagatagccgccggcttagtttgtctacttacctgcagaaggaaggagagggctggaaacctgctgctgcctacagtaatttcagattaatatcaacgctttaagtgttaacctattcaccattaatgccctttacctatgggttatagaaaattaaatattctctgttacagtgtatgctgtgtactgttgctgttgctgggaacaattcatgttgccagcgcgcaggtagagtcctaccagaaacggctgcagggaaagataaaaaaaggagatacccttgttattaaggatgaaaaattccggaatgatgcctttgactggaaatcgatcaataacaagcttgtaaataatgttgttactttcggattgtaccgggattctacctaccggatcgataagcctttcaagtgtgagcttgatctgaaaatagagtactggagtcagcccgaccaggacgacccgattaccattgagcatgcgcggttgaatattgattatgatactgtgtggttggcgccctaccagggagaaaacatttattcctttaccaacggctataaggtaaaattaacggtcaatgatatcacgagtaaagagctgggtaccgatctgccggcaattttttcgttaaagggagacgtgatagtggaccggcagtatacctccaacaaggaagaggaattgtcgatgaccgcattttttaaatccggggaaacggccacggctccaaagaaacaggcgaaagcagccatggcgcctatgggcgctacaccgaatacgccgcctttaacgggtattataaacgttaactggaatgagattatacccgggcaggaatatgacctggagtggacctatatcgatgatgaatccaccaatgggcagttcatcactgcaaaccgttcttcgataacggatgcgcaactggaagcaatgttccggaataattccacccgtatcaccaccgatcagcataactacgatatcacgcttttgcatagcagcaaatacctgttgctccgtatccgttatgtgatctatgtaaatggttttcgggaagaacatccctgggtttaccaggcaaagctggcaagtggggaagtagccagggtactggatctaagctggcatcaacctgggtttaactggcaattcagcgccagttatgcggaagggggtaagaaaaaagaagtagtcgcttattttgatgggattttaaagaaccggcaaacggttaccatcaacaatacagataagaatgtagtattgcaggagaatgtgtacgacgagtatggaagggtagcggccaatattttgcctgctcctattaacgcaactgctttaacgtactatgggaggcaaaatctgaacgccctcaacaaagtatattcctacaaggatatttacaacaacagcacaggtgtctgtgtcgtaaagccagcgccattgggaacgacggggggcgccggtatgtactattcatccgccaatccttttaaagcgacggacgcatcgatgaactatgttcctgatgccagcggatatccttttgccattactgcctataccaatgataataccggtcgtgtgcgggtaaagggtggagtgggagatgtaatgcagcctaaccaggacgaagcattgaatcattccaccaggtacttctatggaaaacctgtgcaatgggaactggaccggcttttcggttcaagcgcgggaaaggcttcccactttttgaagaatatgaccattgaccccaatggacagatcagcatcagctatctgaattcttccggtaagccggtggccactgctttaagtgggggatcgcccgataatgtattgcccctggcttcaaaaggggtttcagaactggtggatgtgcctgtgctggaaccggaatcgtttgtgtttgatccacaggaactgaaactgaagggcgccgctacctatctctgcgcggtgccggatcataatgccagcatcaggtaccggatagataaactgatcaagaagtataaagagaatgcggtagagatttgcagtaattgttactatgaactgaagattgatgtgtatgatgattgtaataacaaggtagatgcgaatataacaccggttaagattggaagtcttgctcccaactgtgccgacgagggcagtgtagaaaacagctttgtggtagacctgggaaaggctggcgagtacagcatccgctttgaattgtcgctgaaccctgatgtcattgctgcctatactgatgactttatcaagcgtaacaccaatttacagccagagttctattttattatcaaccagttgagaacaactgatttcaccggctgcgtgagtgattgtcatacctgtgaagtagcgctgggtacaaaagcggaatttcaacaaagggtctggcagcggattgccgacaatcaggtgaatgctaccttgtacaccaatgacataaataactggagcggccctttgtatgacacattgaagatgaggtgcaccagtgccttgttgaattgcatacctgatccgtgtaaggagttaagagaaaccctgaagcaggatgtaagtccgggtgggcaatatgcgcagttcgacagttatggccggccgctggaactggcggtgaatatattatccatttatttcagaacagtatttccggtcgaagctatcggtggttcacgttatgaatcaaccaggatagtaaacgttgatggggtaagtatatcgccctgtgatgccagctttacactggaggacctggtgaagaactggagaccggagtgggcagatctgtttttgccatatcattgggaatattgtgcgctgcaaagctgtgagagcctgtctgccgtgaagcgttgggatgaaaagatcacttccctgtgtttaaaagcatccgaccttcctaaatatgtgggaagtaattatgaccgtactaatccgacctggttgctgaatgccgatccttttatgacaaacacggcggcgcagccctatattaatagttttattaacgatcttaacaactattccaggaaccggacgccttacaaaagcagcactttcaataacaagaatatctggcagtatgttgattatctgctttattgtgccgacagcacagggaacaccaatgctactgcagatgtgacttttgtatcccggtggaataactgtgtgccacaaacgcagtgccgggtacctgacagggaatggctggcttatgcggagtattatttccagttgaaggagatctattatcagcgtatccgcgatgcgagttgcggtgatatctgtaaaataggtcgtccgttgccgatgctgggagaaagttgtgccaccgtgtccgacttttcttttgcagaagattcattgggcaattgcagtgctggaacaaagcgggtgcgggttaattttgaaggaaaccgttttgctacggaaacgcgggtggctgttacatattccacagggacaaccaatacatcagagatattaatatttggtgcaggagatcgatataagacgatatgcattccacaatatcttcctttgagtgtgttaaaagtagattctgtttattgcaggaacagtggggctgtgtctttccctccgaaagggcccgttacgctgccatgcaggaccgattatacggtggaggtggatcaaataatacatagtacattaggttataagataacatttttgtctccgctatcaactgatgttgagtatatatttactctgaaaattgggacaaatccaaacaatatagttactgttaagatgaacccacctgatccggtttatattgggtcagtctatattggtactgatagtccaacgccggcagaacagcaaattacggtactttcttatacctgtaacgaccccaccggcggctgttctcctttattcaggaataaaacctcccgtatggagagaattgactatgatcagactttctccatgaatccggattctttaagaaacgatggttttgcacagatagcgaacctggtggcagataattgtgccaataatgcagatgtatggatgtcgcaattagaggaaggactgagtggctatacttctataaaaagagatgcgcttcgtcagaaattgattgaagtgtgcaaactgggtggggatactgctcacttaaacggtgcgagtgcggcagtgcctactgctactgcggagggttatcgttccttcaaggatgtgatgttgggtgtattgggcacaggtagtattacaatgaagaataatccctggattctttccgggccatatccatttaatgtgaaggcacaaacagcagaagcggttatcggcaacacgaacccggctatctgcgcccgtttgagtgcgttgcaggcaacctataacagcaatgctgcgggacgcacattcttaaaataccttacagatacgtatggcagtgcgatgaatctcaaacaggaggagttggatcagctgataaaaagttgtggtaactgccggtatctgctggccagccagcttacactgccggtattcctggaagtaaatacaaaaggatgtattacacctgctgagttcactgccggaatgacggctcttaaccaggagccatggtcaggtggactggataacacgaaggataactatgaaaccattgtagccacttatctgaaccatcgctggggcttttcgctcgggtatttggattatgatgactacaggcagaaggtaacggcgggtacttcggcgttgctctgtaatgagccggtgttcaggtcagtaacccctgatcctgctgaatgtttgatgggaatgatagatggagcaattgcgggtggtcgtcgtcgttatgtagtatatattgattctgtacgacaggatttccgtagacaatacgttaccgtatgtgccggtacaagggctactgccaacctgaaaacgcagcagcagctttatcatttcacgctttattattatgatcaggcgggtaacctggtgaggaccgtaccaccggaaggggtggatgtactgagtacagcgagactgaacaccactaccacggaagttcctgctgactttacctgtaattacaatggcgacaatgtcaatacaagtctgccattaacattaacggagctgactaacactctgaatattcaaaccggcgtagcagtagaaatgtggattaaaggccggccaacgggagctacccaggtgttgacacctacctccaataataattacttctttactacctgcattagcagtacctattgctatatctcgatttataagatgaatccggagactaatgctatcagtattgtaaacagtagtcatatagcggtgcccattacggcttttagcggtggcaactggctacacctggtagtacagggacctaatttgatggatggggtactgagtacctatgtaaatggtcaattactgaataatgatacgaaagcaccactggcaccttgcgcctgggagattgtggttggtacaggcggagtatctatcaccaatgatctcagtgatctgaagcacttaagaacatataaccgtcagcttaccgccgatgaaatatggatcaactcccaggagccttgtatggcacagatggcgggcctggacgctaagcgtttctggggtcgttttaatgtaccggctaacggtgcgccgggaacggtaggtggtccgaattccaatattgaagtacggcctatgccggtgcagcctcaacacaggcttgctaccgattatgcctatacttctttaaaccaggtatcgaaacagaagacaccggatgccggtgtcagcggtttctggtacgattacctgggaagactgattgcctcacgaaatgcaaaacagtgggcccgaaataacaattataactattcagtatatgatgaacttggccgtattacagagaatggcgaagtttttagtaacgccagtatttttgaacctggttttattataaactatggggatctattggagagtcccgtttcaaatcctgagcgcatttatactttctacgacagccccatgctgccctccagcctgggtacacaggataaccttaaaaatagggtctcagctcagtaccggtacgttgccgcctctacaggaggaactacgactgataattttgtttacagctatgatttgcttgggaatgtgaaaacgttctggcatgggaatgggttgtacgactacaaacagacagattacaattatgacctgatcagtggaaaagtgaatgcagttcgttatcagcccggaaaagatgatcagttctattatgcctatacatatgatgcggaaaacaggttagtagaggcaaaatccggtatcaatagcgtatctgtcgacaagtgggagattagtggtgcggttacagatgcctactatcgctactataaacatggcccactcagccgcatggagtatcttcgtaatgccgtacagggtatcgattacgcctatacgttgcaaggatggttgaaaggtgttaacggcaactacctctcgccagcatccgatatgggaagggatggtgacccttcgggaacgagactgcattttgccaaagacgtggcctcgtataccctggattacttccagggtgactatacccctattggcaagcctcccactgttacgaatccgttcgcattgaaatgggagagtaagaccgctgatattgcaggtcaggatttgtataatggtaacatcgcccgttcagaactcgccctgaaaggcattaacgggggaaatccaataggctatagctaccgctacgaccagttgaaccggttacgaaccatgcgtcagcatacactagcgggaggggccaccacctgggaaatgggtactactcctccaacaccctatgcagaagatattacttatgatgccagtggtaacattctcacgtataaccgtaataatatgagcggtgcgccgatggaccggctcacttataactatccgcggaatggtggtgggcagcttacccgcaaccggttgagatatgtgagggatgggatcacatcgccactttatccaggtgtcgatattggaaatcaggctccagctgtagaaacagcaagtgagattgggaatgtagcgggtgacgcctaccagtatgacgaaattggtaacctgataaaggatggaaacgacgtatctgaaatagaatggaatattattggaaaaatcaagagttttaagaaaggaacgcttaaaacagagtatttttacgatccggcaggtaacaggtccaggaaagtggtggaaacgtctgcgcaaaactttaccaccaccgtctatgaacgggatgtaaccggtaatgtgttggctacttacgaatacaaaacagggtcagcagatattacatggaaagagcagtatctttatggtagcagccgtctgggtgtgtggaagcctaatatgaaattgggctctaccgcaacaaaggatgccctatggactgcatttaataaccgggaatacgagattacgaatcacctgggaaatgtgctgaccacgattacggataacaagacaccaaccggtagcgtgtatgatgtgacgcttagcagtgccgtggattattcgccgtttggaatgcagctggttggaaggaagatgaatggaggtggttataggtatgggtttaacgggaaggagaatgataatgatgtgaagggagaagggaatcagatagactacggcatgcgtgtttacgacccacggatagggaagttcctttctacagatcctctatcgaaacaatatccacactataccccatatcagttcgcaggaaatacgcctattcaggcaatagatctggatggtgcagaggaatatcattttacacgaataaaagacaaggatggtaatacatcgcttcgttatttgggtaagactgatattaaagagcgcgtttttgttggatatagatttgttcatggttcattttatgatacgcctacaccagtttatgaaacccgtgttaatcagcgtgaggcatttactatacatgacacatacagggaacctgtagatagacatggggggcttgatccaaatcaatcgcaggagtggagggattttgatgtaaggacaacatatagatcattagaagatctttctgcagggaagaatggttcgaaatcagctgcagatatccttgggatgagattaacccagtttagtgcagcaataggtcctgagaatgcggctatgccggctttaggagcgggtaattctcctcaatttataaaagaaatagaatcatcagcgattagattctcacaaacgtcagttaatggagtggaagagattgttgcgagtatgaaagttaaaggatggaagggagctcctattgatgtagtacagatgagtgatggtttattgacttctgttgataatacaagagtattagcagcgcaattatcagggactagagtaaaagcggtagttcatgcttatgatgaattaattcctgcttctcaagcggggagatttgttctcaagaagacgggagatgtacctaagacctggggacaagctgtagaatacagagttcagaatcaaagtgcaacatttaggactaatactcctaatggtagccatgtacaacctaaagctaaaccaagcaccaattaataataataggttctataagatcctgttcatacaattctttattgtatgaacaggatcttatttatccggaatcataaacccaaatgtatccattaaatattcttcagaagatttatagttcgagagtcgaataataatttcttcatcccaatcaattaatgccagtttgtaagttgtgcctaatatatttagtgcagataatattttttgacagttttgagtttgagcaaatagttgggatagacatagccatatattggttacaaattctgcctcaaaggaaacaaaaatacctagcctctcaaatccaaaagcaacagtgttttctttagtttggatgttattgttgtatcctgtagttactttactaaagtaattaatggcaataggagatagtaaatcatagaattgattaaaggagatttttaaatcgcctaatttaatcagatgttcatctctgacaatggcattaggaaaaccatatttattttcatccttagagggtaggttctctatgtcaatgattgccttgaaataattttgctctggaacaagctctatctgtttgtaataatcttcatgaaagaatactgtatcaggcattgtatgttatttgtttatgtaagtttgtttagttttgacatctctgataaaggcagcgataaccctaagcaatgcagctttatcatcccctggtaaagtctcaatctctttaaaatacctgattacttccgcatcatgcaaagctgcattagctttatctccggtacttccaaataataaataatctacagaggtatcgagcgcctcagcaatcttctttactacttcagcaggaggctgcgcacctttagtctcgtagcgtccaatctgggcgtatgaaatatctactttatcagctagttccgtctgcgaccagcctttagctttacgtagttcaagtatacgtatgccgagattatttttttgagacataattgcctgtttaggttaacaaaaatagctgatctgtagcagttttggtgtgtttttgatactaataggggttagtgtgcgaaaaataagtttgtttgtgtgctacataaacgtttattttgctgcataaatgtagcaataaaatatttttccacatacatctattgagttaactaaaaatgctttttatgttggtcagtaataacaggcaaattaaactacaacccaaacaccgggatcaatcaggcaatcatacagtagtgccgtggcttaatatcagtggtgtgtggctggaggagttgggttttaaagtgggagatatggtaaagattaccacccgtgacaggttgctgattatagaaccactggaaggaacagagcaggtagcgcatgaatataaatctgccttacacgaaatgaagcagacgctgaaaaagctggcgcaatgaatatagcggagattaagcagcagcttacgttgtcgtctgtcttgcagcactatggcttaaagccagataagcatctgcggttacattgtccgttccatgatgataaaacgcctagcctgcaggtgtactataaaacgcatacctgttattgttttagttctaactgtaaaacacatggcaaggcattagacgtgatcgattttgttatgcataaggaaagctgcagcaagcatgaagctatccagaagtgcaaacaattaatcggtggccccgtatatcaaacttacgttccctcaccgcccggtatatctatactgggcaatatgtttatctattttaggaatgcggtatatcacagcaagccagcgcaggagtatatacgaagccgcggactggatgctactgttttagagatcggttataatacggcgcagttccatcatggtaaccgtaaagatgcaagctttatcgggccttgtgtagaagtggggttgttgtcgccgtggggaaccaatacccgtgaaggtggacaggcatataaaccttttgccaagtattgtattgtgtttgcgttgcgtgacagcagtaaccaggtgagtggactttacttccgcagtactattaacgatgaagaacagaaacacttttatttaaaagatcgtcggggtctttatccgggttatcctaaaccggacacgcagcgtttaatccttaccgaagctattatagatgcagccacattattacagcaatccgctatagcaaagaattatagcgtattgtcctgctacggaacgaatggttttacgaaggagcatcaggaggctatcaaatctttaccagctttacaggagattatttttgcctttgacggtgacgaggcaggtagtaaagccgtagctaaatatgctgcgcagctgcgggagcagctgccgcatattattattactacgcttatccttcctgttggcgaggatataaacagtatggcgctatcccatgaaccggatatttttgttcacctgcttagtgagcggaaggaattttttctttcatctgaaaaaataacaccagaatccgctacggtggctacagaaaagggggcatcacctggtggtctggatactacgaatccttataaactctgctatagcacggaccataccttttattatgtgcagggtggtatcagtaagcagctggatagtatgaaagtgacgttggtagtagagcggaaggataacagccagaaaagccgtaacaagctggatctgtacgaagataagcagctggataaagtgagcagggaggtaagcgaaaaactgttacttgataaacccttactggaagtggatttataccggttaacggatctgctggacgagtaccgagaaaaagatcttgtaaaaccgggcggggataatggatctgttatgggcgtgtacccgcttacgttacaggagcgcacagcagcagaaacctttttaaaggaaggtgatctgataaccagattaaatgatctgttagggcaggcaggtatagtaggagaggaaacgaatcgtttatttttactgcttattgccatcagctataagatgcctgaaaccttacacgcgctgatacaaggtagtagcggcagcggaaagacccgactgttaaaacaaatatctgattgcatcccgcaggagaaagtaacgaagctcacccgcgtgagtgataaagtactgtataattacccggaacattattttgtaaaccggttgttatgcctggaggatatagatgggttaagcgaagaagcggagtttgcatttagggagctacagagcaacggagagctgaacagcgccaccagtatcaagctggataacggacaaatcaccagcggccagaaaacagtaaaggggcctattgcttcccttgcctgtactacgcggggagaaatctatgaggacaatatgagccgtgtgttcctgctggcagtggatgaaagcggagagcaaaccagccgtattattaactatcagaatagtaaagcatctggtcagatcgacagtaagcaggaacaggacaccaaacactttatacaaaaccttgtacggtgcttacagtcaagaccggtagttaacccctatgccagtaagctacagttaccatcggacgcacataagatccggcgtttaaatgatctgtttttaaactttgtaaaaatggttacactggtacatcagtaccaaagaaaaaaggatagtaaaggccgtttaatcacagaaatatccgatcttgaaacggcggtagatattatgttcgatagtattgtgctgaaggtggacgagctggatggaagcctgcgacagttttttgaacagctgaaatgctggctgcgaaaggaatacagagaaaactataaaacggctacctttagtctgcgggaagttcgtcaggggctgcgttgtagtaaaatgcaggtgttccgttgttttaatgatcttagccgcttagagtatgttcgtcagcagggcggccatgctaaccgtggatttacttatcaggtaatctattgggataattacgaagccttacgggcaagggtgaagcagcacctgcaagcgcaaatcgatctgcttaaaaatgttacaccagctgcctctatgttacaccagtgaaacaccagcgaaacgccagaatcctctgccatagccaaaatgtgcgctggcgtaacgcgtaacaaaaaagtgttcaagccctactttagaaaaacggcatacttataccagaatcgccataccgttaacccttccttttattttatcacaaaataacatcattatttatgtacctgatcgtagatagttttaaaagctatctgtctgtattgggatacagcaggagtacgcaaagtatgctgcctgcgtgtatccgtgattttttggagtacgggcagtatagcagtatagggcggatccagccaatggatattagtatgttttatgagtggctgcatgaacggccgttaaagcgtggtgaaggtggcgctttaagcgaaatgatgatcagtcattacgtgtatgcgctcaaggtgttttttagctggcaacttgaaaccggaggtattaccattaacccggttagtgtgctcaggtttaagagtccggaacgtagctaccgggagcccttaacagtaggggagatacaaactttgtttgcagcagctgccacctgcagggaacatgctctgcttcacctgttttatagttgcgggctaagacgcagtgaggcggtacggctagggttatcagatgttcacttcaggccgcggttattgtatgtaagatcaggcaagggtgaaaggcgtcgggtgatccccttaacggacagggttgcggtcagtctggagcagtatgtattacaggagaggggcaaggcccggtgtaccggtactgcgtttatgcttaatagtaagggtagggccatgagcggtaatagttatgtaacgctgcttaaatctttactgcgtaaagctggtatggataagaatatcagcccgcattatctgcggcatagtatagccactcatcttttacaaagcggcatgagcatggagtatgtacgtgactttttaggacatagatgccttgaatccacacagatctatgcccggcccggcgcacatcaattacaagccttatgacattatatgaatatcttgaaaagcactatacgcctgctacggcggaaagttatcaccgggaaatatccatctttttaagtagttacccagctgcgcaggtggctggttatgcagagctgatcagctacttaagtgttttacgtgagcgttataataatgctgctacgttaaaccgcatcctatgcagtattaaggtgtactatgattatttatgttgtatcggtagccgtaacgatcatcctgcgcgttctatcctgttacgtgatcagcgcagccgtgacgtgcagttacaggatctgtttacgggggaagagctggaaaggttattagatcgaaaagagcgttatcagtcgttatcttaccgtaaccgggtattaatggggttactggtctatcagggattaaagccgcaggaaatggctcaaataggcattacagacattaatctggaagtggggagcatctatataaaatctacgcatactactaacagtcgtacgttatcgttaaagcccagccagatcctgttgttatatacctggttgcagcaggtgcgtccgcagctgctaaagggcgttgctagtgatgcgctgctgatcggtcacagaggaaggccgatgagtgcggatgatatagtcaagcatgtaatcaggagctataaacatgtgtatcctgaacggtcagtaacggctcaggctatacgaggcagcgtgatagctaatttactacagcagggctatgatattagtgtggtgcagcagttcgcgggtcataaatatccatcgagtacagaacggtataaacaaagccaggtggaaacgctgaaagctgctatagaacagtatcatcctatgaaatgaagaaaatgttttattattgttagctggttcgaatccgcttggaacctctgggagtgcctgaaaggtgttgggagttcgaatctcctccttcgcacctaagttagagctactgactcttaatcagtaggtcctgggttcgagccccagtggggtcatatccttcctttacaaaaatccttaatcagataagtgtatagagcaactgcgttctaagcagtaggccattggcttcaatccaatccagaaaaaggtggagatggcgggaatcgaacccgcgtccaatgctttttatcaagggttcgaatcccttcttctccgcaattaaaatgttaatccttctaaatcaatactttttagagcaaagggtcacaaatccggaagtcaaaccggaagtatccgtaaaaaatgcaactccactttaaactgtgccgagggttcgaatccctgactctccgcaagtactacctctttgtttatgatcatcagattatggtactgatgatcgtgttcccagaataggaaccgaacctgcactcattaataatgagcatctgactacggatcagaaggtgatcaagtccacctcagaggcagatcaagtccacgtcaaaggctagtgaaaggcaggtataaagcgtgttaaaggctagtgccattgcttcggaataagatgtccctgctactcaccataaagccctgttgtgttaaaaggtctcactacgggctaggtcggcaaaaaggcgcgccagtcctgcgcttgccccttgcgctgcgctacaggggctgcgctccgtcctgtcacgctttttgcgctcccttcgccctccgttcggccagctcccggtatggctaaggaggtgttttaatattggtcgcctttatgcccgccatcccttcgctgtccattttgtccgccccccgccgtcccccctggccttgcatttttgattttgccgtccgctggcgctcccggccagatataggtcgaaggcgcggcctgctgtggctccgtgcatcgccatgcccctccgctgcgctccggggcccggctcgcactcccgccccagcggccaggggggaatggcggtgtggggcggcagaccgtatgttggggcgataggatatagccatcagcgttataccgctgaccgggcaccgggagaataagactgcgcgaacaccagcgccagtaccccgatcagctgtagtactatcttgcttccgtcctggtagacagatgatgtggtcagctgtagaacataggctggacattagttctctggtcatcggcagcatataacatcagctgtagtaacacatcatctatctaccaggacggttgcctgccatttatccgcctgtatttttttctttcaaatggaaaaacagatgaaagaaaaagctatatatttatgagagttctttgagtgcgccaggttgcggatggtaggtgagtccgtggggtctgggagtggggaggtatatcgttatgggtttaacgggaaggagaatgataatgaagtgaagggagaggggaatcagcaggattatgggatgagggtgtatgatccgaggatagggaagtttttgagtgtggatccgttgactccacaatatccatggtatacaccgtatcaatttgcggggaataatcctgttaagtttattgacatggatgggttagagccagttaatgtaagtgttagtggtaatcagattgtatataacggaggatttattgttaatgcagctgatatttatagaataacatatcttaatgtagtgttggggcttaaactaccaagcaatttaaatacttcatctaatccatatgatgatagagatccttataatagggatacttgggagaaggcatatcaaaacgtttcttatttttttagtcaccatgcccctgcgtattcaagatcagaggctgcgacaagaactatacatacagccattgctaaaggtttgttgagtggtagcgattcggaggccgaaagtgctattgcacaaatagacaaatccgaagattatgcgtataggaactcacttgcaaaggatggattgttttatggaagtttggttaatgaccttagaacgcttgcggtaaaaacgatatttaaatcggatgataagtatgttcagatggcaatagatggaattgcgaaggttgaccctaatgctatttatgctgttgaggttctgattagaaatccaaaaacgggaatggatattacggattttgatatagtaatgaagaagttcattgttgaggtaactggaggcaagggaggaggtaagttggaacaggttgctactcagcgattgttagctcccaataaagaaatagtagtgtttggacccaaagtgggaggaactgttgaaaaaaatctgaaagaacaaaatgttaaattgtttagaaaggtcgaggatttggtgaaatatgtaacatcagaaaaaaaagaatagaatgaagtttgcttttgttataacagatgatttatttgaacttgatgattttattaaatcaaatacaggctcatttgaacttaaatttataaaggataatgagatagcctattggaatgagaaagaagagagaagtttggtttctcttgagaaaaaaaataaactctatgatttaatggaaccagaagccaaagcttatctgaatcagcaatttgattcgttcaatatatttttggtcaggttttttaactttgaagttgcaaagtatatcatttgtagtgctccgattgaaagaaagctattgatcgataatgattatggtggtatcttggaacgaaatgtattttgtcagatggatacatatgctaagtttatttcaataaccaagataccttattcttaattttaatggagttcccgataatgataaaaccctgcaactggcaggtttttatcatttatcgaaaattgcttcggtttgtccatttttaggagcaaagcccgggtttatacatgttcatgtttagttctgttaattttaacttcccatcaaaatagcaactattgcaggattcaatgtatgtaagtattcggctaacgcagttttcctgtcggcatcaattttcattaattcaaatttaggagccttgccctcaattcctgatgtactcacatatttgagggaataatcttcaagggacaggtgaatctccatatcagtgtcttttccacttaatataaattccttctttacccatttacctttagaaaaaaaatctgaaaagtatgttggtacatttattcctttatagattaaaagattggtcgcgatctctccgtttttttccagctccaggtaaatattgaagtatctcagtaaaggatggacaataacattcagtgaaagtgctttgtcttttggatgaacgaaagttttatatttaatcctaaaatcaaacggcctttcaacaatttcggctttaatcgaattcagtatttcaatattcagccggctatcctgtctagccagattgatgagggcgtcatgtatgatgttaaccatagtttgttgtataaaataatcatcttttaacgcaaaatcagtctcaagatcataacttattctgacatcgatattctttctattgccttcaaaaacaaaatcctggtccttttcgccggtatgaatgatgtgtatatggctataaaaggtaagttcattctttttcaacataccaccgtatattaatgaaatcccttctgcatatgaattaattacaccttcggtgattgatatcaatcttaacatctcattatattagttgcacaaacttacggctttatctgaggacctagcctttccttcaatccccacccccgtcaacattatcaaaagtttcccgcgcttttggtgtgaagctgtaacggagagaaaagatcggtccataataaatatcaaactgggttccattcgttcttaactgcatttgtgcaataacccctgcgagcgcgtggatgttctttgtaatgccggcgctgtagtaaatagattgtcggagaatatcaaacttgttgggggcatagtctttatccgcaaatttcagcatcagctccatatagtaggaaatgttggggcttttcaggaaggcttgcggattgttctgccggagaaagtgattgacacctactctggccctgatcctcggtaccacccttgctataccctgccggtcgtcaaaaaatttggtttcaaaccgtacctgctgaaagaggcttcctttgggcagtttctcagcaaaggagcccataacgattaaccgccgctcgagggtttcatagttgccggcttcctttatttcatatttcttattgcgcgcgtagcccagccacaacttcatatttttgaaccctgagtaagatatccagggcctgacaacaaaacgttgtgcataggcaaatggattgcctgtatcatatgagccttgggtaactatctgcaggtctacttctccgtcgagatgccatttttttatcaatggaaaggaaaaatcggtttcccctatggaagcaggaatgaaaccgaaggtatatggagggggagactgcgcaaaagtaccactgcttgcgaaaaagaatataacaggaatgatcagcttgcatgcaatcttaggcttccacctgcactctttggtatttgtatgcatttcaaattgcaatgactcatccctcctttattaaaggaaaaatttttacccgatgatattgttatgcttagtgaactgaagaagagagcgagaggcactgttaaccaattaaacgtttacgaagctggtttgttcaataatcgttcggttagtttttgaagcctggccggggcgacctgtttcctgatctatgaacaagagctcttttacccgggaaaaataccccctcagtcactgcctctttttctccaaatttttagtaactttcctaaagatgaccccaatatccattaacatttaatctaccccagaatgttctccaaaatacccaatcaatcaccagggattgcacgtccacaacataccccattttttactactaaaaatgatcccccgcaatctgcaaaacccaacttttttcagccccgtctaaaggtaggacaaccagatactgtgcaggaaaaagaggccgacgccgtagcggacgccgttacccagcctgccggcatggatcataaaataaatgctggccacaacacatccctacaacgaaaatgcgaggcatgcgaacatgaagaagagctgacccgcaaagagatcgacggcgctgaagtctccgcaccatccgcagacatgataaatgaagtgatttccactggcggacagccaatgaataacctcatccagcgggaaatgtcagagagaataggttacgacttcagcaacgtagtgctgcatacagaagataaagctgcgcagtcggcgcaggctgtcaacgcccgggcctataccgtgggcaatcatgtggtttttaatgaacaggaatacaaccctcattcccgggaaggacaacatctgttggcgcacgagcttacgcatgtagcgcagcaaaatgcagcagctccggccacggtacaacgccaggtagccggtacgccgggtgggccggatccctgctttaatttgctccaggaaatcattgctttgctggaagaagtggcacaccgtattatggatgccgaaaacgaccgccatggcctctttggcaggcgcaccccacatcccgagtatggaagctgggacggtcaccgcgatcgttttaactatgaccgtggccgtctgcgcaccaaactgggtgaatgggatattaacgacaggtgccggggctaccagctcaccagggagcaagcgcaggatttatctgaagcaagggaatttgctgaaagagagtttcccacaaggcctctccctgccatgcggcgggatggagagcctgtaacggcttcaccagacccggaattacggcaacgagtagagcggttcctgatccatatcgggatcccggctttcgcccttggaggaatggttgcattagtggtcgctgctttagcagaccccgaacctataaccaaattaggactgatcatcggcacggccgccgccgccgccctattaatattcctgggtggagattcatcttcctccacatccggaggcactgttgccagcgaagatcacacaaccggagacgacagcgccgctgcataaacttaaagcgggggtatctgaacatggatacacccgcttctcctattgacaaattatggaaggaatgatgtaaattagtaatcagcgacaggcttataccccgatagtttacattaccccaaagtattcaatccctttatgaaaacgttttatgtagcatccgtcatttgctgcttaatggcctgtaattacggccgcccgtccaaagaggtaaaaagcaatgctaataccattggttgcgcagttcctgccaccaccgacaaagaatggtatacatccggtaagaaagcgcctttatttgacgggttgcaaggcattcatttcacgatttcaacatccgtgaaagcagcacaaacttattttaaccagggaatgatgctctcctatggatttaaccatgcagaagcagcccgttctttctttgaagccacccggctggattccacctgtgccatggcctattggggctttgcgtacgtgctgggtcccaattacaatgccggtatggaatccgataattttcagcgcgcctacgaagctgttgtgaaagcgcaggcgctttcccatcagaacagtccaaaagagcaggcgctcatcgccgctttggccagcaggtatgttaaagatccaccggctgatcgcagcgccctggacagtgcctatgcggcagccatgaaaaaggtatacacgcaattccccgatgatccggatatcggtgctttatatgcagaagcgatgatgaacctgcatccctgggatttgtatgagaaaagaacacaagcacccaaagcatggacgcccgggataatagcagtactcgaacacctgatgcaattgcatcctactcatcctggcgcgcatcatttttatattcatgcactggaagcctcttcgcagccggagaaagctatgcacagtgcgaaattgctggatagtctggtgcccggcgccgggcatttactacatatgccttcgcatatttacatccgtaccggcgattatcatgaaggttcgctgtcaaatatccgcgcggtaacaaccgatagcgtttatacggtggcgtgtcatgcgcagggagcttaccctttggcgtactacccgcataactatcacttcctggcggctacggctacgctggaaggccattccgctctggcctggcaaaccgctgtgaaattgcagcaacatacctccgaagagattatgagcatgccgggctggggcactttgcaacactactataccatcccgttttatattgccgcgaagttatcgatgtgggataccatactggcgcttccagcgccggacaagcacctggtgtatccccgggctatctggcactatgcaaagggaatggcttatttaggcaggcatgaagtaataaaggcccggaaagaactggatagcctgcatgtacttgccgctgataccatcctgaaaagcctgacgatctggaatatcaatacttcggccgacctggtagaaattgccggaaaggtgttggctgcgggcatcgcagtgcggcaacaagcgtccggcacggctatttcattgttaaaagaggccgtggctatggaagaccacctcaactacaacgagccgccggactggttcttctccgtgcggcatcatttaggtgcggtgctcctcaaagcagggcaataccggcaggcggagacagtttaccgggaagacctgggaatatggagaaagaatggatgggcattgatcggtttatataacgcgctggttttacaaaagaaaaataaggaggcgaaggaaatattggctgcattcgaatccgcctggcaatatgcagatgtgaaaattaattcatcgtccagtataacccagtaagaccccttcatccattaaataaaacgaacggaacccaaatataatttatcttgtgccagcctgatatttaaaattatttttccttgttgaataatttcagaaagatgtttgagaacccgttgaaatggttggtagcagccacaattatttatactgtatttagttgcggcggaacagcagcaaccaaacaccccgtaaagcaatcccctcaccaggccttaccatctatacaggtaagggcgttttatcctggcgccgatgccgggaagttactggattcagtatccccgccattaaaagatgctttctcccggtatgccggaaacatggatcatataacctatacggccaataacgatggttcattcattgttacggtttattttaaaccaggtattgatctggactcagcagcaccgggtatatccaacgtggtggcagtagcttcgccacaactgccgtcacccgtagttcagtcaggcgttaccgttaccaggcaaaatgagtccattgttatgacggtgggcatgtatgcggaggataccggaagttacgatcaggcattcctggtaaattatgcggcaaccaatattgttcctggaatacggggaatccccggggttagtaatctgattacttttaacaagagtaaagattcggtgatgcgtatctggttaaatgaagaacacatggccgctgttcatctcaccctaaaggaaatattagcaaccattccggcagggcaactggaagcagtaacggagatgccttataagaaaagtaaatcatcttctgattatattattaagtgcagtagtaagcacaaccaacctgctgagtatggaaatatggttatccgcaaggatgctgataccatcctgagatggaaggacgtggcggcgaagattgaatttggcccttatacttatggaaacttttcgcgtatcaatggtaagcctggcgttaacatcgtggtaatgcagtgggcggattcaaattatagcgggattcaaccagcggtagaaaaggtgatggaaacagcatcagcacaatttccagtgggtataaaacacgtgatatcatataaccctaaagattctttatacatttcagcagagtaactagcctggatctttgcgttttttacgaaaagtaagggcagtcattcctgtttctttactgaaaaaccgggaaaagtaagagtggttttcaaaacccaggtcatcggctatttgttttacattcaggtcgctgaaatatagcagtcgctttgcctctataataatcctgtattttatccagaacgaaaccggggaaccggttattttcttcaggcactcattgagatacggctctgaaatatggagcatgtcggcgtaatccgaaggacttttgtgttgtcttatatgttcgccaagcaattttttaaatttgagcgacaggtaggctggccttgaactgccggtaccggcatccccggagacacgtacagtgtctgctgccatttcaaaaaaggagcgaagtaacgaatgaagtaccgttaaactgccaggagattgatccgtcattttgctatacaagatgctaaggagctggttgtagtgatgtgcatcgttgcttgataaagtaacaggttcctggaagcccgaccagctatcgaaagcatggcggcaggcgggatctatcaacgaaggatctgcagcgatgaaccacccgtttgctttgttggctttaatccggtagtgaatctgttccggcagaatataatagagttgatttgcacgcacggttttttcttcaaagtctaccacggctgtaccggcgcctttcagcatgatgaaaaagatatagtgatcatcccggtgcgcgcccggttgtgcgggcggtttatcatctgttcccttgtgagtgaatggcttcagcaggtaaccgcgactggtgctgtcctgtaatttatgtaccggaatattcttcatgagtttaaaagtaagtattttaacgcaggttcatgaagcctgtaaccggagtaatttatctgcatttccatgggcaatttttgctacctgctctgcgggaagctggatgttatttaagaactcgatgcccatctggttcgtgctgaaaggatagtccactgatagcataatgttgtcgataccaatcgtatcgagtgcaatctgaaggggtggttgtgtaaagaagccacttgtggtgataaagagttgctgccggaatgtatcgatcaatgtgcgttgattgcgcccgccattgccggggtgaaaagaccggttagatctcgcccacatcatgggtaacatttcgcccatgtgaccgataattatttttagttccgggtaaacatcaaaaatacctgccaccagcaggcgtagcacgtgaatagcggtttccgaatgccatccccatccccagcaggcaatagcatcaaaaggcccggtatcgtgtcctatgttgctgtaataggcatctatcaccggtttgggcggcaggcccgggtgaatgtagataggcacacccagcttttcagcttttgcaagcaccggcgcaaatttaggagcgtccaggaattctccgtttgtaagtcccctgatcatggcgccacgaaagccataagattttacggtgcgctcaagttcgtcggccgccgctgcgggtgcggtcattgggagatgtgcaaatgcggtgaacctgccgggatagttgttgattttctccgccagcagatcattgtattttgaagcaaacgccggagcgctggtggtgtccagcaggtttacatcggtgttttcaacggataatacctgcatggatatcccggattcgttcatggaatccaaccgttcaccggtaatgtcggccagctttggcatcatttgcattgccacggctgatggccgtgtattgctcagggtaccggcgggaagaagatgggtcatctccgggaaggatacatgttcttctaaggttactattctcattttgatgtatttgaacaatgcaaaggaaagatagtaaccctggaaaatcaatgttcatccagtggtgatgatagcacaattcgcggtaaaattttgcggtcagtcatttttatccgtactgtattcgttattttcttcatcttctgcgccgttccgctcctggtcatcgtcgagctctgcgccgggtacatccaggtctccggcttcattcagtgggtccccgtcgtcatctgcattatctaccacggctccgcgcatacgtaattcctccgaataagttggatctgtggtagatgcttcttccaatagttctttctcttcttcgcttacatctgcatccgcatctgccgttgtatcttcctccggcaaatcgtcttcattgagcaggtcttcgtttaagtcatctttattaatcataaccgttgttttatgggtgaatgataatctgttccaacaaaaggcagaccggatagcagcaggtgggcaatgcaggcggagagaagattccgggcgggtaaagttgatggaaatagtagggagatttggacaaattgtagaccagcctgatcgttgcggtgtccattttcagacaccggtgttcatatccggacagatacatgaaaataaaatattcgtagaatggctaccagtaagcatttcaggtgtggcagtattattgttttttcaatggcaaaccagttagctatgttaagaaatcatgctaaaattgcctggagaaatctgttgaaaaataaaactttttcgctcatcaatattgtgggactatctactggtatggcggtagccatgctgataggtttatggatatacgatgagcttactttcagtaaaaatcatgcgaattacgaccgtattgtatctgtgatgcagcatcaaacctttaacggcgtggtgggtacgcaaacggctaatccttacctgctgggagaggagatccgggataaatacggcagcgattttaaatacgtggtcatggcatcgtggcccaacaaacacctgctggcttacaacaacaatgtggtttcccaaaccgggaattattttgaaccggatttcccggaaatgttgacgctgaaaatgctgaagggaacccgcggcggcttgaaagatcctgcgtccatcctgctgtcggcttccactgcgaaggcgttgttcgggaatgcagatccggtagataaactggtgaaactggataaccagacgccggtgaaggtaacgggggtgtatgaagatctgccctataattcggctttccgggacctggcttttatggcgccgtgggaattgtacctgagcagtcagccctggatcagggagatggaaaacccgtggcgatccaattttacgcagacctatgcgcagctggcggatcatgccgaccttgaaaaagtatccgctaaaataaaagatgtaaaactgcacaaagtgcgcgcagcagacgccgcttttaaacccgaagtttttcttcatcccatgagcaaatggcatttgtacgccgactgggataacgggaagaatataggtggcaggatccagtttgtatggcttttcgggatcatcggtgtatttgtgctgttgctggcctgcatcaattttatgaacctgagcactgcccgttcagagaagcgggcgaaagaagtgggcatccgcaaggcggttggttccttccggggtcagctgatcacgcagtttttcagtgaatcgcttttgctggcggctatcggttttgtgggcgcgttggtgctggtgcaggtcggactgccggtatttaacgaggtagccgataagaaagtaagcattccggttggcagcccggtattctggctggtttgtttcggtatcaccttattcacgggtttaatagcgggcagttacccggcgttatatctttcttcttttgagccggtaaaagtactgaaaggtactttccgggccggacgttatgccgctattccgcggaaagcacttgtggtgatgcagtttacggtatcggtgatcctgattatcggaacgattgtggtgttcaggcagattcatttcgctaagaaccggcctacggcctacacccgtgaaggattgctccttatcccggtgtctaccggcgcattgaaagaccatttcgaggtgatcaggaatgagttgacatcatcaggcgccgttacggagatggcttattcttccgcgcctacaacagacgtggatgcaataaacaatggttatacctggaaagggatggcgccaggtgcacagggcaattttggcgcagtaacggttacacatgatttcgggaaaacgatcaactggcagatcatatcaggacgtgatttttcgagggattttgcttcggatagcacggcgatgatcctgaatgaatcggctgttaagtttatggggctgaaaaacccggtaggagaaattgtaaaaaaagatggccagccttttaccgtgatcggtgtgataaaggatatggtgatgcagtcgccatacgagccggttttccggactgttttcacactggactacaatgctgccaatgtgatcaatgcgaggataaacccggctaaacaaaccgctgatgcgctggcccggattgagggcgtctttaaaaaatacaaccctggtattcctttcgtttacaggtttgtggatgatgagtatgccgctaaatttgatgcggaacaacgcattggtaaactgtcgagttttttcgcggtgctggcggtattcatcagttgcctggggctttttggcatggcgtctttcatggcggagcaacgggtaaaggaaataggggtgcggaaagttatgggcgcttccgttttcaacttatggcgtttgatgacaaaggattttattatgctggttgttattgctttggtgatagcggtgccggtggcctgttattttatgaacaactggctgcagcgttatgaataccgtacggaaatatcgtggtggatcattgtggcttcttctgcaggagcgttgttaatcgccttgctgacggtgagctaccagtcgataaaggcggcattgatgaaccctgttaaatcgctgagatcggaatagctaagcgctatttatctttctataaaaaaaggagaaaatgaagtggattcattttctcctttttatgttaatttattttccattcgggccttacaaagtggcaggtatatccatgcggatgcttttggagatagtcctggtgttcttcttcggcgttccagaatgctgttgccggaaccacttctgttacaatgggcccgggccatttaccggaggcattcagttctgcgattaaggctttggctgtttcctgttgcgcttcgttctggtaaaagatagcggagcgataggaggtgcctatatcattgccctgcctgttgcgcgtggtagggtcatgtatctggaagaaaaattccaggagggagcggtatgataacacggctgaattaaaggtaacctcaataccttccgcatgggtgccatggttccggtaggtggcgttttgaacatcgccaccggtgtatcctaccactgttgagatcacgccgggtagctggcggatcagttcttccacgccccagaaacaaccaccggcaagaatcgctttttcaatattcatatgtctttcctcttttaatcatgtgaagttaagttatgctgcggaatccttggtgagaagcgccacatttttatgggtaatggctttccgcttattcagtatacgctgccggagccgcaggaacggcgcctctaccgccttattcaggatgaatgctcctaaaacggcaataagcaggcatagcaccagcatgaggcttccctttggagcgatgcctgtttgtgccagcaggggctgcaccaggtgtatcactcctttgtgcgataaatacaatgcaaaggatagtttagctattaaggtagtaacacggctgttgtactggtacaatatacccgttggactcaccgctgctatcaccatcaatccatatcctgccgccaccagcgggtaaccgaatatggaagcgtaaaaactttcctgttcattgcacaggaaccaggcgcctgtaagcaccagcagggatagtaataaaataatatttccccgtttggtgatccatgtttttgcagcaggtttgaatgcaaacagcgcagcaatggaaacgccggcaagcaggccatcaaggcgggtataagtggggtagtacatgtgccggtaccagatcacccagaaattgtcctgttctgcgtgaggggcaatcagggcgtaccagcagtacagccggataccgatacccaatataaacaacgccggcagcaggaatcccgcttttctccataccttgaaacggagcagcgtaaccagcaccagcgggaaaagcaggtaaaagtgttcttccacgcacagcgaccatacatgagagaacgtgccgtagtttttaatgtcgaaattgaagttctgcgtaaaggtcaggaacttccagagcggtggcagggcttccctttcgtggaatgccggaaaaaggaagtagatggtgagtaccaccaggtaagccggaatgatccggaagaaacgtttgataaagaactccggcagggagatgtttttccctgacgccatgtttacaaagaggggataggatatgagatatccgcttaatacgaagaacaggtctacgcctgtccaaccgaagcccatgatattatccagccattgcggatgttggaacatgcggtagtgatagaacaacaccatgagtattgccagcgaccttaaatgatccagtccggagagttttttaaccgttatgtcggtgtttgtcatgaaaaatgcctgtctgttgatccttgtaaaatacagtctttaaaagagatatgcaatggatgggggagcacatgccctggaatgccctatggcagggctgggagtaggggaatgcccggacgggaggtggacttgatcaggtgttgagttggtgatgacgctcatgcggttaactttacccggagcgtaccgtagtacctgttttacaccggccaggcggtttcctttgctggatttttgtttgttgaccggcagtacgactgctattatatcggcggccataaaccggcggtttagtgtaggggtggcgccgttaaatattctcacctggagcgtaacgagcaagattccttttccaggaacgttggcttccagtgtggcgccattaaatggttcctctatatttgtgaacagggaggagctgcggctgccggttacccgatgcgtaaccggattgatgcgaacggcgataacgctgatctccagcagatcgccggcggttgatggcgaccaggtttgtgcggggatcgccaatgtgccatccgtagacagcatagggagccgggagaagaatttctccacgccggtgtggcggttgaaccggaagccttcgagttgttgcaggcggtccttgccgccctgtatcagggctttattgaggcggtttaccagcgtaccatcgcggccaatgcttaattggggcgttatagcctgccggaccagtttacctgttctgctggcgacgccgaaattccgggatgactgccgtgtagcggtggtttgttttacttcttcgggcatggaacggacgaagtaacttccgttccttcggtaaccgatgaggttacccaatttccctgtaaaagggagtattcctgtttgttttgccatgggttaactttttgattaaaaatacgaaaaattgtggaggtgggaagggggcctaaatgcgatccccatgaaaatattctccgttgccttcgtatattgcggttgcaaataagtgaatacaggctatgcaggctccttacctaataggacaaacaaaaccattaaccccggctgaatttcagcagataaccgatacggtaccatttcttttgccggtgagctaccgggattttctttatacttacggactgggagccatcaatgaactgctgatgatccatcaacccgatgaagcgtatatccggtctaatttcggggagtatatggatttatgggagctgccggagagtgaagaacctgcagtgctgaatggactgaccattgcgactacgattgatggagatatcattgctttaattgacgatagccaatatccttttattatcttgccgcggcattcagataagatcctgcggtttgccgcctttgaggaggtgattgattattacgatcacacgtatcatttttcaggagatgtatatttcgacagttactatcactacgagcaggagaacattactttcgttaatggaccggccattgataaagcattgtttgaaaaggttcaccaggattttctcgcgcatgtgccattcgataaagtttataacgcggaaaggcagcctaaatatgttatccaggagatgggcggctgggtgtattttgataatatctatcagagttcagtgcggattaagtaccagtcgcaataccggccggcagccggtaaggtcatacaatttatccgggaccggatgaaatgatgttatttatttttcagcagcctgttgttgacgatcttctccagtaattcttctttctggtacttactgataggtacttcatgattgcccatgtgtaatacgtttccttcaatggcgctgatatgattgatgttaacgagataggatttgtgtggttgcaggaactgccgcgcaggtaaactttcctgtaccgatttcagggttgtatgggtgattatttttttgtctgcggtataaatcgccacataattgcccaaggcttctgcaaataaaatatcgttgaatattactttctccagcttattatctgtttttataaagaagtaaggttgttctttgctgatgtgctgggaggaaaaataatcaaatgctttattggaagctttgaggaagcggtcgaatgaaattggttttacgaggtaatccagtacatccagctcaaaaccctgtatggcatattgctcgtatgcggtagtgaaaatcaccttgggcggatggggatagcttttcaggaattcgatgccggtgatataaggcatttcaatatcgagaaacaacaggtccacaggttgttgcttcagcagggtattgagctgtatggcatcttcacaaacagctattacctgcaggaaaggcgttttctgggcataacgttgtaatccttctccggcgagcggttcatcgtcggtgataatgcagtgtatcgttaattggtccattatcgcgtagtgagttttagttcagccaaaaagctatcttctttaatttccgcggtaaacgtatgtttaccggggtacaacagttccagtcttcttttcaggttatctaacccgatgccttctttttcctggaagctaattttatcgggtattgaattctctacacaaaaagatatttcatgatcctgtttttttagatcgatgttgatatgaaaattaccaccaacatatttaaaggcattttccaccagcggcaaaaacagcagcggatatacctgttcatcgtgcagggcttcatcaaaaaatacgttgagctgcagcctgcgtgacgacctgatcttctgcagggcaataaagttccgcaggtattgtatttcattcatcacgcttaccgtttgctgctgatcgtacaattggtagcggagcagttctgaaaaacgttccactgtttttttagctgcctccacatccatatccatctggaaatatattgtgtttagcgcattaaacaaaaaatgggggtggtattgtgcccgcaggaatttgagttctgtttgcagctggtcgttggtgattttctccagctgcagccggttattgatatatgcctgtaaaaaggagttgcttctgcgtaccccatagtagatgaggcaatataacaacgggatcacattgatatcgatgaggtcgaacgattgcaggccgttgtcagtgaaggcggccatgggcgtaaaaatggcgttttgtataagttgattgatgataaagacatataataattccttcaggatgattttataagagaagccggcctggcttttttgatcgaaatagcggaacaggaggttgaagatccacacaaaaaggtagcccatcagcatactggatcctatttcaatcatgttaaccagtagtggccggtaccagaatttcatttctgttatgctgtccgtaagcaggcggatggtaaagtataccagcaggccatataacgggggaaagaaatatttccagaatattttcatgatagctgattaattatgccacttcaggttgtgccggtattaactttgtttctttggatctgcgatctttcccttcccgtgccggtggtttcatgccaaacaggaaacgcatgatggcaaagggtctgataaacaaatggaagatgaatatactgattaaaaaagtaaccagaacggtaaaagtgtatttcagtccaacgccatcaggtacctgcaccaggtaataagtaagtattacaataaccgtttgatgcaggatatagaacgggtatacggcctggttggcatatgccaggatgggcaggggtttattgagatatttttttgcgtagccaacaatcgccagtacccacatccaggcaacaatgccgcttaaagccatatatacgtaggtaaagggagcatgtttagcattgtcgttgaagagccagggttccattttattccagcgcaggtagttaatgatcataaggccggcgaaagcgatggccagtgaaaaccggcggttccgttccaggctgtccatgaacaggggattggcaatgcagataaatcctgccagtacataaaacaaccagtagaagaaatagccgtagtcgtgtaccagatcgccggtttgcgggaaccagatgagcagaaaggtgtgcaccagtgttcccgggatgatgaacaggtagatataccgtttgcttcccatccagtttaatttttgaagtagatttttgcctttgccggagatcagccatacgaaaacgggcgcaaaaatgatatcatataccagcaggtaagcgataaaccacaggtggtgccagctcatgttgccgtgcggataggcgccggtggtaaacatactggtgtagaagtcgaagaagttgcctttgaagccctgggtgaggcgttccatgtatacctgaggtggaacaataatcagtatgcccatcagcaacggaataaacagccgccggaaacgcaggccgataaagctgccgccggaattacgctgtagcataagatagcttactgtgccggaaacaaagaacagcaggggcatgcggaatcggtggaggaagtcgttcatttcaagcagcacattgctggtttctttattttttatatgccatccccattcagacacatagggcatcgcggaatggaagaacaggacgcccaggatagcgatgatgcggagccagtctaaatacgccagccgggaagaagatattggttgcatagataattgtttagtgcaaacctatctgaccggcggttttcaggaaaacatttttgacatgtggacagtttccggtgttgaaaagatcatttatgttaaaatacaataactttaaggctcgttccatctctgatattatggctgctacaccaatcgtccgtcaatcctaccgccttgagaaaatccccgggaaaggtggatggactttcgcgcgtatccccgaaattacgcccgataaagtgaaagcgttcggattggtaagagtaaaggggtttattgacgaccatgaaataaaaaaatgccacctgatgcctatgggcaatggggtgttatttcttcctgtaaaagcagctatcaggaagaaaataaaaaagaaagaaggcgattgggtggaaatcactttgttccgggatgatgatccgctggaaataccggaggagctgaaggcttgcctggaagacgagccctctgctaaccgtttctttgcatccctgtctgaaagtgagcagaaattttatatcgactggatttattccgccaaaagaacggaaacgagagtaagccgtatgactaaatcgatcatccggttatcgagaggactaaagttgtatgaaagggaggaaatgtaaactcagttaagaaaacgaaatggttaaagtatctttgataaccgttacgcctaaaggatacgggcccgttttatgagtattatcctgtcgccaggtaattattttggcaaagaacaacaggtcagcgagaatgcgtctttccggctgaacatcacggcataccagccggatgtgcagatccgtgagcactatcatgaaaatgcgtacctgagtttgctgatcagcggcagttatgaagagagaagtaaaaaaacggagagcggggtggttcccggcgaagtgcttttccggccggccggatacagccatgccaaccacttccaggcagtaggcggcaagtgtttgaatatagaatttaaaccaggcggattgcaggaactggaactggatcatttgcttccccgcaccgcggcgatctataaaaccggcacattcgattacctgtaccgcttgttgtatgcttttgtacaggatccgggcagttcattaccggaagaacatattatcaactggctgtgtgaatataccaatgacaaaatgcctgagcgcctgccctggcttcctaaagcaaagcagatcctggaaaatgaatttgatactcatcatactattcagtcgttagccgcgcgggtgtttgtacaccccgtttacctggcccgtgcctttaaagaaagggaggggattacgcccggcgagtaccagttaaagatgcgggtgcgaaaagcgatgaccttgttgttcaccactacgttgccggtaacagatattgcctttaccgccggtttttccgatgcttcccacctggtaaagtgtttccggttgttttaccgtgctactccccataaattccggacattgctaaaaagttaatccggtaccattttatttgtggcgccggccgttactttgtagaaaaagagtatgcgccgattgatcgtctttttatatttgttagcgccggcattattatcagcacagcgtaacctggattaccagttgcaggtaaaagcggacctggtaaagaagtcgttttttgtacagggcggatttagttttaaaaccgacacggctgctgccgactcagtggatgttgtcatcagccagggcgcaggaccggtaaggctgcagttacagggtgctgccgccgtaatggataccagccgcaaggcttccggggatattatttaccgctggcatttccgatcgccgctgccggcaggaacggccctgcactttacctgtgcgtatgagcggggtggtgcgccggcgttccagtattatctcgacagtaccttttgcatggctggcggctatggcgctgcgtggtatccacaggttacagatggcgcaggtaatcatacccgtggtaccggcaccattgctgttaccacttccgttaatttgatgcctgtaatggctgcaagtaaggtgacagtgaccgggcacacttatacattccactacgcacaaccggatattttctcactttatatcggtaattacacccggcaggaatataaagggcagtggtctttttatacttacagtttaagtaagggtgttgatggcaacgatctaagccgcaagtccgctgcggtgctggactacctgtcttcacaatttggtccgctggacattcccaacttttccattattgaataccccgactatgtggctgaaatcacaggtattggcggcgccagtattctaggtggtgtggccatgcctaccggggcgctgcgcgaatttaactatgcgctttttggtcacgagataggtcaccagtggtggggcaataaagtgttatcggccggcagtaaaggggaggccatgctctcggagggactggcacaatatggttctttgcaggtggtgagtcatttcgacagcgcccatgcgatggcctaccggagaaccggttaccccggttatatcagcgatcagtgtgggttgggctatcttaaaaacgtagctgccggtaatgatgaagcgttagtgtcgctgtcaggcaacaatggtcatactattggcgacagtaaaggttttcttgccctggaactattatctaacaccgttggtaaggccgtatttcataaagcgctgcgcacgatcggcgataaatataatcgaaccggcgttacgtgggacggcttccagatggaagtggagaaagcgcatggcagcagtttgcaatggttttaccgccagtggtttgagcagttgggcgcaccttcctggcaaagcagctggcagcaacagcaaaacaaactgcaactcagcattacgcaaaaagacagtatatatcatcttccgctggaagtgctgatcacgtatagcaacggaaccacttcactgcagcaagtcactatccgcgaccgcagcaatcagctgcaactgccggttaatggcgaagtaaaggaggtacaggtagatccttatttcaaagtgcttcactgggacgaagcgctaacaccggaggcgcttgcccaggcaaaagtggtgcgggtgatgaacctgcgccgccagcaaaaaaatgacgaagcaatgcggctggcgcaatcctatattaaggaaggtttcccggatgaccagtacggtgtggagtttacacttttttaccacatggggcgtattgctgcgatgcaaaataaaccggcggaagcattggcctattatgagcgtgctttgcaatgcgtatcacgcgcaccggacctgctggcttatacttattaccggatcgctacgctggctgctcaagggaatgacaatgcgctgatgcaatgggcggccgctaacgctgtgaaagcagatgctgcccgcaacaaatcagatgggatggaagcaaaggtggcggggttgttgtcatcggcagtggcgaaaacaaaatgatgagaaccaatcagatcagcgtaacaggatagggggatactttataggaggcgggggaaacgccggtgaaggatttaaattcccggatgaagtgggattgatcgaaatacccgcattcataagcaatggctgtgagggaaagtttgtgttgctgcaccagttccaggcttttctggaaccggtgcagttttgtataaaatttgggcggaacgccggtatactgtaagaagagtttatgaagataccgggaagatataagatgttgccgcgcgatactttcaatttttgcatcggcgtccggctgcttcatctggtggatgatattgcccaccatagcgatgttcagcggtttccggtttacttcctgtagcctgtttaacaggaattgtgccaccagttttatttgccggtccaggttttcttcttccagcagtttcatatgcaactggtgtatggacttgcctaacatatctgcagggtcgttcacctggtcattcagcagcatgatatcttcctgcataaaaaatgcggcggtatgggggtaaaatctcacgcccagcattttattatagctgcctgcggctttcacgggaaggggacgggtaatctggccccagagttcaattttaggggtgttttgaaagatattattgctggctgttttccaggtggctgttcccagattgaagataatttccatgtgaccgccgggaaatactacatcgtcgatagcagtgtctgcctcggattcaaaatggtagtaacattttacatatggttttaacagttgttccggaaggatttccctgtatatcattttggttgaaaattgcggtaactgcaatttaagtaaaataccggtttataaaaaacgctgttgtatcagttccatgaatgcgggccggaatttgtcgcttagcggaatacgtttgccggcgatgaacaggtgattatcctggattttatcgatccggctggtgtttacaatgtaggagttgtgtaccctgataaaaggcggcggcagctggctggcaatttctttcaggcgtttgtaaaccagtatttcttcccggagggtaacgatccgcagatattctttttctccttcaacgtatagtagttcagagagtttaatctgctggagagttttaccggtttttacaaaatagtaatcggcggaaggcgccggggcggcggtttccggcatacggggatgcataaacgctgattctattttttgccgggccgccaggaaacgtttaagggtaatgggtttcaggagatagtcgaccgtttggaaattataactggcggcggcatattccgtataggcggtggtgaacacaattttcatttccggcggcagcagtgcggccagttccatgccatcgagccggggcatgtttatatcaaggaaaatcaggtctgccttgttgcttttgaggaacgtcagtgcttccagcgcgtgatagcatttggcgatgagctgccagtcggtggtttgctgaatatgcagttccagcaaatttaccgcattgggttcatcatcaacaatgatacatttcaggctcataacggaatggataaaaaggcggtgaaataattttctgaccgggcggtttgcaggataaagccggcgccatacagcagggtaaggcgtttccggaggttgtcgatgccggaccccagcggatgattatgtaccggctgttgcggtaagctgttgcgggtggtaaagagtaacctgttttcctgtttcacgagtgaaatatcaatgtggttttgtaaactggttttatcgatcccatgtttgaaaatattttctacaaaagtcattagtaacatcggtggaatactgcatccgccgggtacctcgcgggtgaattgcaggtcgatatcatgccggatgcggatgcgctccaaagctatataattttccaggaagtttatttctgtggagatgtctacctggtccttcggactttcatctacaaaataccgcatgatatccgacagccgctcaatgagggcggcggtccgtggggcttccaggtaggcttcgtaatagatgttattaagcgtattaaaaagaaaatgcggctgcacctgtgatttcaggaggttgagtgctgctttcgtgttctgtaaaaccagtgcggcggcctgtgctttcagttcaaaataaacgatggccatccggaatacgaagctcagtaaaaataacatcgggatgccggtcatataccggagcattatttttacggtaacgggttcgggatgcgaagtgaaccaggtgttgtagatccagctgagaaagaagcccctggataatcctgccaccagtaaaaacagcagcacggctataacgtataccactatacggccttttaaataaagccgtgaatagagccagctgatattgccataaatgaccagcgcataaaaaagggtgttgaacaatgaaaaaatggcggcctgccagaagccatcttccggcagcatggagaaaaacatcatcaggaaaacaaccagccaaagcgcccattgcacttttgcggctgccggcatacgacttatcaattgcatgtctcaatttacgaagcttttgcgctcattagcccccgtcctgttcaggattcaataaataccggtaacggctcaacgggcaggcccggaaattcaacgagggccggtgatgtgtaaaaccgcctggttattaaaaatacaggggttgttattgaaatcatttttttgacagaccggaaaccgggaatctttgagcataattacacgtccgtatgccctccggcggcggatattgaaaactttaaattccctgatagatatgcaacctaaacgtttcctggtcctttcggtactgttagtcaccattgccatgctccctgcttttgcacaaaccgatacagttgatcagcaacatcaccggctgaatacagccttcctgaagccaggagtaaaacaatacctcgtgtacttccagatgccttcccgcagtaattggctggacctgagcctgtgggtgcgggagattgagaaaacgagccacaacaatgagccggtattccggatcacccagcactggtatgggagcgacactgcccggtatctcgaaagcatttcctataacagcgtggccgatttttcaccattatatcatgcacaaaccaggggcggggagcagcaggcttatcgctggacggttaatgggatcagcggtgacactgccaccatgaacaataaagcggcggatttcaagctggcttttgaccgtcccaattataactggaacctcgacattgaaacgtttgagatgctgcctttaaaggccggcaaaacctttgttatccggttttacgatgcggggctggaacctcctgcgtatgtgacatataaagtaaccggcagtgaagtgctgcagacattggatcagcggccggtggactgctggaagttgttaaccgaaggggattcgccacgggggcattactcgcaaactttctggatcagcaaagcggggcatgaattattaaaagaagaagattcctttggcggcttttaccggtacaaggtaaagctgccgggtgcagcgccttacctgcagccacgttttgtaaagtaacccctgtgaataatttgcgccccggaagtcccggggcgttttacatctcccgaaaacaaacaaataagggtaactggtgataatactgattgtcgtaacttgtatgcttcattccggacgcatgcaattacctcattaaaaataaacagtcatggatatccaacagtttgaagacaagggattggcgcagtactcttatgctatttacagtgaaaagtcgggggaagtgattgtgatagatccggcgagggatgttgcgccttacctggcgtatgcaaagacattgaatgcaaagatcaccggtgttattgaaacccatccgcatgcggattttgtgagtggtcacctggagctgcaccgcgttacgggagccactatttattgttccaagtatacccatgcagcttacccgcatgtaacttttgatgatggtatgcggatgatgctgggggatattgtgctgaaagcattgaatacacccggtcattcgccggacagcatcagtgtggtgctggtgtataaagcagagcccagggctgtatttacgggcgatactttgtttgtgggcgattgcgggcgtccggatctccgggagaataccggcaatgttattgtgagccgcaatgaactggccaagcaaatgtatcattcccttcatgaaaagctgatggtgctggcggatgatgtactggtatacccgggacatggcgccggtacgttatgtggtaagtcgctcggtgatgctgacagcagcacgattgctgccgagaaagtgagcaactggagcctgcagccgcttacggaagaagaatttgtggtggctttattatcggagcagccttttattccaaaatactttccctatgatgtagctgtaaaccgggaaggagcgccggttttgcaggcttcgctggataaagtggaggtcataaagggcacaccagcgtttgaagaaaatattgttataatagacagcaggccacagtccggttttaagcaggggcatttgcctaatgcaattaacctgcagaacggtggaaaatttgaaacgtggttgggtagcatggtggcgccggaggagccgtattatttgctggcagagaatgaagcggaggtgcaggaggtgatccgcaaggctgctaaaattggttacgagcgtaatatcagggctgcggcggtttatacaaaaggagccgaaatgatggcgcccataccactggcggatttccgggaacatccggagcagtatacgattgtggatatacgcatgccatcagaaatagaagaggaaccactttttgagcatgcgatgctcattccattggatgagctacgggaacgggcatccgaaattccggcagataagccggtggtagtgcattgtgccggtggctatagaagtgcggcgggcagcagtattgtagcggccgcattaaagacgcaaacgccggtatatgatctgggagaagcagtgaaagaatttatgtcgtaatacacccgttatttgccctgtttaccccctgtaactgtgatataatggtgatatatttatatctgcatatgcaatggagcaggccgctgtgcggggtttcactgcatttattcttcacctgaaaaaatcagttattatgtttgggaaaacaaaagcattcagcagtttttcggttaatgatctgcagcaggcaaagaatttttaccaggaaacgctgggaatagaagtagtatcagccggcaaagagccggtgatcacacttaaaattgcggggataccatcggtttggatctatgaaaaaccggatcatacacctgctacctttacggtgcttaacttccaggtgagtaatgtggaagaagccgtagaccagctgaccgcaaagggtgtaaagttccagcaatatgaaggggaacttaaaacagatgagaaaggaatattccgtggaggcggaccggtgatagcctggtttgctgatcctgccggcaatatactttcggttgtggaagaaggctaacccggtgttaacgtaatagccaattgtttttcctacttttgccgctcaaataaggaacatttatggctactaagattactgttaacaacaatggttcactgaagatagaaggtgaatttgagatcgtggataaagacggcaacaaatacgacctgggcggccgggaagcggtagggatctgccgttgcggacgttctgccaataagccgttttgtgatggttcacacaagggacattttgagcacgacgccgtggcttttgcgctcccgcctaaaaagtagggtcacaatgataacattcaggggctccatgcacgtgttgcatggagcctttttatatctgatctggtcgaaatgagcagaattgcatctgttttcagaaaataaatcaccgcatttttgtgttacaaattgcagtaacatatggaagtaagattttttcaggtagatgcctttaccaggcagccttttaaaggcaatcaggcaggcgtgtgcctcctggagcagatgccggacgatgaagtactgaaagccatcgccgctgagaacaatcttgcggaaacggcctttttattacgggcggagaatggctaccacctgcgctggttttcgccgctggtggaaatggcgctttgcgggcatgccacgctggccagtgcgcatgtattatgggaaaccgggctggtagctccggatgaaaccatttcctttaccacactgagcggcctgctcaccgccagccggcaaaacggttggattacgctcgatttccccgccagggaccatgaacccgctacgctgccggaagagctgcagccattgtttaaagacgaggtgacgaacgtggtgttcagcgtagatcgatatttggtggagctgaaaacgggggctgctgtggccggctttgtgcccgacaggaacctgctggcgccataccgactggtggttacaggaaagggtgatgaaggatcgccgtacgattttatttcccggtattttgctacgccggtgggcgttgatgaagacccggtaacaggttccgcacattgcagcctggcgccatattgggctgcacgtttgcataaaagtgaattctttgcttaccaggcatcgcagcggggaggtgaactgaaagtagtgctgcaaggtaaccgggtattgctgaaaggagaagcggtaacagtgatagacggggtgttccgtttttagcggaataaagaaacgccccaatagcccagggccagccatagcaggccttttataaggaagaaaagaaagccccagaagccgagcttttttatccatttgaggatctttgctttcctgttattttccggtgtcatagccctgcaaaattaagatttttgtgcagataaatgtatcttgcccgggtgaatatattttggctggcaattacgtgtatgcgtcggcgtaatcacctaatccctgtatatgattttcagagaagcaactactgcagatattcccggtttgcaacgggtacgtggcgctgtaaaggaaaatgtactgaataaccccgacctggttactacctcagattacatacaatatctcactaccgatggcaggggatggctatgtgaatctgccggtgttattgtggggtttgccattgtggatacacaccggcataatatctgggcgctgtttgtagacccgcgtacagaggcagtgggagtgggcagggagttgcagcgcctgatgctcgactggtactttgcggtgtatcagacatcgttgtggctgggaacctcgccgggtacaagggcagaacggttttacacccgcagcggctggaaaaatgcagggctgatgaaaaacggtgaggtaaggtttgagatggaccgggatacctggttgcgcatcgcaggtgccgtttcatgagccggcaacggctttcatgattgaataaatgatttaatacgtacttttgcgctcttttagcaacgatttttaaaagatgcgtgtagcagtaccgaacaataaactactgatatccctgttcctgggcctctgtggcagcgccactgcgcagcagcaggccgactctgtccttattacccatcacctggatgaggtgattgtgcaggaaaacaggctggccgcgcctgtaaaggcagtgaaccgtaatattaccatcattacccgccggcagatagaaaccatgccggtgtcgtctatcacggaagtactggcttacgtgccgggactggatgtgcggcagcgcggtccgggcggtatccaggcggatattggcatcgacggcggtacctttgaccagacgctggtgctgctgaacggggtgaaaataaccgatccgcaaacggggcataacatcatgaacctgccggtgtctctctccgatgtggaccatattgaagtactgagaggcgctgccgcccgtatttacgggatcaacgcactgaatggcgctatcaatatcgtaacccgcaaagccacccaaagcggcgctaccgttagcggcagcgggggcagcagcttcaaaaagaacgaaaacaatcacctttacggcgcttacagcattggcgctaccggcgcactggtaaagaatggtgtgagccagtcgctttccgccagccgcaaccagggcaacggctaccgctacaacacagcctacagcaactaccgtgcgttttaccaggccgcctttaaccgcgataccctgcaccagtacaacgtaatggcgggttttgtaaataacggttacggcgccaacggcttttatgcagcccccggtgatctgaatgcagaagaaaccgtgaaaaccgtcttcgccgccgtaagcaatacttcgcggatcaatcccaactgggtgatgacgcccagggtgagctaccggtacaccaaagatgattacatctacataaaaccggataaataccgcaatcttcataatacccacgtatttgatgcagagctgaataatacgttcactactgctgtcggtaccattggcgccggtgtggaaggacgttacgagcatattaagagttctaatcttggtaaccacgacagaaccaacctcgggctgtatggagagtataagtcggtagccgatcgccgctttagtttcacgataggcggttatctcaattacaacaccgtatacggctggcagtttttcccgggagcagatgtgggctttaatattacccccgatataaaactgtttgccaatgccggtactgcccagcgtttgcctacttataccgatctttattataaaggcggtggtattattggcaacgaaaacctgggaccggaaaaggcatcctttgcagaagcggggatacggaagttcagtggtaaattttcttttgcagggtcagtgttctacagacaggtcagcaactttattgattttgtaaaagataccgccggtggtgtggatccaacaaaggttccgtggcagccgcagaatttccagcgcgcagatatgactggtttttcccttaacagcggctataatactattttcaataatggttcgctgtttaacagctttggtgtaaatgccgggtacaattatctttctccatccttcaaaggggatgcgatcacaacgaagatttcacggtatgtcattgaaagtttgcggcatcagttcaccgccaatgtgcgtacggatatcggccatttcagtgtttctgctgcagcgcgttattgtatgcgggtaaattataaagattatacgctggcagatgcgcgtattgcgtataggcaaccacgttaccagatctatgcagatgccaacaacctgctggatgtaacctatgtggaagcaggtgcagtgcctatgcctggccgctggataacggtggggggcaaggtgagcttctgataataacgtatagaaaaaagctgtctcaaaaggaattttgagacagctttttttgcaatatcatttagcggacatatactgttgcctggattgttgaatgccactcatattagcgatggcccattgttcaagacctgtaatatgtggtaaaaggctttcgcccatagccgttaaggcatattcaaccctcggaggaatttcggggtacattttacgggataccaatccatcttcctgcagctttttaagcgttacggtcaacatcttttgcgagatatctccaatcatctcatgcagttggttaaaacgcatagttcctttctctcccagggtactgataacgagtaccgcccatttgtcgccgatccggtccatcagtgttctgaccgggcaagggatggatttatcaaattttttatattcttctatcatgtcaacagattgatttttagtattacttacccggaggtaattggcacacctgttagtgccttattgtttgataatcaattgtttaatagctttgacttaccaaaggtaactaacatacgattagtatgtaaaggtagttacatactggtattattaaaaatttaaaacttaacataatgattcttgtaacaggcgccaccggccatttaggagcagcggtgatcgattttctgctgaagaaagttcccgctaaccaggttgcggcattagtaagagacgaagcaaaagccagtggattaaaagaaaaaggtattagcgtaagggttgccaactatcacgattatccctctttggtaccggcttttaagggcgttgacaaaatattactggtatcttccagtgattttaatgatcgtgccggtcagcagatcaatgtgatcaatgccgctaaggaagcaggtgtgaaacatgttatttataccagcgttgcgaccaatgctccaactaccaccgttattcctatggtggtaggctcacacatcgctaccgctaaccaccttaaagcatccgggttgacctatacgctgctgaacaacaatctgtatgcagatgtattacccatgtttcttggagaaaaggtagtggaaaccggtgttttcattccgggtggagaaggcagggtgccttatgcatccaggttggatatggcagaagcggcggctaacgtgcttgccggaacaggacacgatgataaagtatataccattgcatctgatgttacttattcttttgctgatattgcacaattactatctaaactggctaataaacaggtggcttatgttgacgctccgcatgatgcgtatacagccgctttagcgaaagcgggcgtaccaccggagtatgttggtgttatgtcgggctttgcagaagcaattaaaaagaatgagttcaatctgccaggtactgaattggaaaatttgttgggcagaaaaccagcttccctggaaagttatctgcaaaagacttttttctaagcattggtttacttcaataacaaaaagctgtctcaaatttattttgagacagcttttttgttgcaggctacaaacttgtagtggagagtatgcctgcactcaccacgccctttgtatcggcccggataaataccgtatatattttcccggcttccaggtgaatattagtgagtgcctgctggtcaatagtaacaggcgccgcattttcaccagcgctaacgatcagcgaaaccgtacctgcgtttacgttagtgaacggcgcgctgtcgtatgcagcaccctgcaggttgctgccgccggcgctgccgtaggggattgtggtgaacagcggggtttccgtattgttttgttgtaaccgtacactcacaccggcaacgccttgcgccaggtgtacaaagcggagctttgctttaccggcggtgggagcagagaggtcgtcgtaaaaaaggagcagggtatctttggcggcattatactttgcggaggcggcaaataccgtatggtagtatccggcaatagggccgttaggtccgccggtggcagaatacacggcgctgttgccaaactgccgggaagctttataggcagcgccgccgccttccgtgaaattgatctgtacatttccgaaagtagtagctacatagggagatgcggcgcctgggagtacagcatccgttgttaccttttgtgtaaacgtccagaactggattccggcagcgggaatgcgggcatttacaaaacggatattagcggaaaggggaggccggtcgccggcatttacgtcgaggtaatctgttttattgcaggcgctgaaagccagtatggtgaagctgcccagcaagaggagattatttttcatgagtacattttttaagtattagaaacgggcgtacaatcttacaaacggctgaatgcctgcgctgccgttctgaatgcctactacggatggattgcgtaatcctgctattactttatcggagtaatcgcccagtacattgaaggcattgtttacgccggcggttacctgtatggctttgctgatatgatatcctactgagaaatcggtgacccagatgggtttcagctcctggaagtagtaatcgggccgcgggaagttagcattgagcgcggaagcggtggtaacggagccgaagtaaatggtacgcgcgaggaaggtgaagcggggcgtattcagtatagcctgcaacgttattttctgttgcggaatattggtggttaccctggctttttctgattcactgaagataacatatttgtattgttccagtcctttgggcgtatttacagccgttacttcatttttcacaaagttgccgccggccagcagttggaggctgttcctgtgcaggggaattttgtagctgccggtgaattcaattcctttggtgcgggtactgaaagcgttgtaaaaaaactttgcctgtgtggtacctgtttgcaggagcagtgcccttacatctgtcgggagattgggatcgttagcggagaagttaccggtattgcctacacggtttttaatatccacgagataggcgtctacgcttagttccacgttcctggcgggttgtgaggtgatgccggcggtgtatcctgtacttttttccggcgtaagggaggggatgccgagcgccctggtagcagcatttttattggaggcggttacctggtcgatggcgcggccctgctggaagctggtggaggtttcggtataatagaactgtgcgaggtcgggtgcgcggaagccggtattagcagatccgcggatgccgagccagggcgcaaagctgtacctggtggctattttaccggtggttacattgccaaagtcggagaagttttccgcgcggacggcggcggacaccagccatttttcggtgacgttgagctccacatctgcatagccggctacgatagcgcgacttacattcacttcattcgatgggcggaatcctgcgtggatctgtgatccgggcgaaaggccgttaagcgcgagaaggccgccgtcggtgaggtaagggatgccgttaacagaggtatctaccgagtaaatgggtcgaaggtcggctttactgtaggaggcttcttccccggcgatgatctggtaggtttcggtgcggtattgtgcgccgaatgcaacattgaggccatgcagtaccgaagggaagtaccggctgatatccaggctggcggtgttctgcgaggcgttgtatttaccggcatcgaaggtggttgggcttttcagccccaggctggcgttgagtgaattgctgatcacgttgccgaagtcatttttgccaaatacattggagatatcgaggttccattcacctgctttggctttcagcccgatggcgatggatttatcggagatactgttgtccatggcgggtaagaagccgtctgggtaaagaccggtgttgttgcgttccgtccagccgggtagacggtatactgcggtgaattgggagttgcggtgactgataccgccaaatgcgtacacttctgcatggtcaccaacgggaatggccgtattaaaaaacagcagtgcgtcttttgctttgttggaacctccgccgcgctggtcgaagaagtggcggtcgatgccccggctggcgagaatggcatcgtctatttctttggtataaatattatcgtatccgcgggtattggcgccgccgccataaatgggaccgttgtacaatccggcatcgtcgcggccgggttggagggacacggcttgtgtggcaaattcggcggtggcattgaggtagccaccacgatcgcctattttgatgccgtagttgatattggtgcgggtgctggccccatcgccgcggcggcggatgctgccggtggtgcttacgattacatcggccgtttgttttttcagtacgatattaataacgccggcaatggcatcggagccgtattgtgcggcggcgccgtcgcgcagtatttcaatgcgttcgatagcgccggcggggatggagttgaggtcgtagccggtggcgccgttgccaaggccgccccagttgacattggagcttttatggcggcgtttaccatttaccagtaccagcagttgatccacgcccaggcctttcagttgcgcgaggctgagggcagatcctgcatcgccggcgttggagccgtttacagaatggaaggagggcgacacatattgcagcagctgcgtgatgctggtttgcggtgctgcttcctggagtgatttgatatcgatgatatctaccggtaccggcgagttcagtttggtacggttggcgctgcggctgcctacaatttgtacttcacccagctggctggtggtatcggtgaggtgtttatcctgtgcagtaagtgttgcggaaaacagcaacaggggggagatgaccggcagtataatttttttcatgccctggttgatttttatggttagtgatgtgttgttttaaatcggtcgtcggtaagtgctacgagaaaggcttcgagatcttccatttcttccttgctgagattaagtggtttgttgagcgacagatcgcggttgatgccgtcgtgtacaatgttgttgggggtattgtaataggcaattacttctttgagtgttttgaacataccgttatgcatatatggagcggtaacggctacgttacgtagtcccggcactttgaagaagccgcggtgggagctgtctttcgttgtttcaaagcggccggcatctgtaagggtagttccgttataaagaccgatatttttgaagcgatctgccgtaaaatcttctcccgaatgacaattattgcaattggctttaccaataaaaagaaggcgcccgcgtatagccgatggcgttagtgcgttgttgtcgccggcgatgtaccggtcgtacggactgttggcggtttccagggtacgttcaaaagcggcgatggcctgcaggaggtttttgctggtaggcgggctgttgaacagctcctggaaatagcggcggtagctttcattgtcgttgaggcgttgtacggcttcttcgatgggcaggcccatttcatccgggttgatgataggttgcagcgcctggtcttccagggaagcggcgcgaccatcccagaagaagttggggcggccggagaggttggtgatgcctggtgtatttcttttggtgggcgtatgatgaatgcccctgctgaaagcgagggtatcggcgaatccaaattgtgggatatggcaggaggcacagctgatggtacggtctttcgacagcagcggatcaaagaatagtttttctccaagttgcgctttggtaggcggatcagtggtgttgaaacccgcgctgatggcaatggcgcatagcatgcccggtaaaatgagcatcatttttctcagcttcatggtggtaaaaattatggatggcatgaaatgcctggcagcaacttgggcgttgctaaaaagtaattggtcgattaataaaaaaggtgttgctgtaaggaggctgtaaaaagagaaatggttattggcattcccgggagcatgggcgggagtgcccgtgctccccaggaattatataatggggtagtataaacaagaacgaattatttggcagcggctaccagggttacatccaggtcaaagtcgtcgtaaatggctttgtcgccgatgccttcaaagaagcttttggaaccgtatttaatattgtatttggtacgatccactttgatagcagctttggcggtgagtttgttgcctgccaccgttaccgttgcggggaaggtaaccgggttggtgattcctttgatggttaggttgccggttacttcgtagttaccgccgcctttggaagtgacgctggtagtagcaaaagtggctgccgggaatttttccacggcgaagaaatcttcgcttttcaggtgacccagtaatttagcgttgccgccggcatctttgatatcggttaccgcgatgctgcgggtatccagtgagaagctgccacctttcagtacattgctttctacttccagtttgccgtcggcaatattgatggtaccctcatgttgcccggttacttttttacctgtccagcttaacttgctttctttaatgtctacctggaaaaccgttgctttcctggcggcagcagctttggttggtttttctcctttgttgacagtagcaggtgtggtgaaagacatcaggaagacagctcctccaataaagaataatgatgctaatcgttgcatatgtgttgtgtgtttaaattaggtgcaatttaagggtgacgggcggattagcgtttacgagatccggaaattaatgttaaaattacttttcagcgattaaagcatccaggtcctggttccattttgccacgtagtccttgtaatactgacctgtaacctcgccggtatagccggtatgtatttgccgtacttcgcccttgcggtctattataatagtggtggggaaggccatcatgcggttgagcgctggcagcttctctgatgccactttcttatcagcaatgccaccaaaaagaatatcatattgtatgttgtatttttcttttaatttccccagggtatactttgcatactccaggtcatctttttgttcaaagccgatggcgattgcttccacgccgcggtctttgtttttattgtaccacggtgaaaggaaggaggtctgatcggtgcagttagggcaccaggtaccgatgatttccacgatcactacttttcctttgtatttgtcgtcgctcagggaaacgttgttgccattgaggtctggcagggtgaagtccagttttttataaccttctttcaggaaagtaagtttgtaagggtctggtaattcggcggcggcatttttttctccatcgaatttgatgttattgtagatgcctaagctgatttccccggtaagggatttatcatcgttcacttttcctttgatgtagatgggactggggccggtgaagccggacagttcaaattcatcgccatgaacggtgccttcgagttcgcggctgtcgcccactacagacatcacaacaccggtgagtttgttgccgttttgtttcagtaagccgatgcggttaggggtgggttccttactgtaaattttaaggtcccatttaccgctgatatcgtaggtaggagcggcttccgtaccaggttccgcgaagcggtaggtttgtccgtgttccgcggtgaacggcagggcattgccacggaagttaggcaccaggctgcggtattcaccggtgatcttaccatctgattcaatcttcgctacgagtgcggcgtcataggtattcatctttataaataaagagtcgttgccaatgcgctgcacgtggaagtcgtcgcggcgggaaccgttgatcagcgtgaaaacggcgtgctcggggtctttccctttcagttcaaagttaaagggtacctgtgattcgctgagggtgaacacgcctctccagatgccttgttttacgaatggttttttaggggcagcgaacgagctgttgccgaataatcctgccaccatcaggccggttagaaataggtgcttatgcgttttcatgtttgtatattattggttgaacaatgcaagacgttgccggtcctggtggggcgacgaggtatgctacaaataaaactggtggtggagtactgatggagtggtggctttatcagtggtggtgaaacaaagataaaggggtcttttattatttccaaataaaagtctataaattttgtagactattagcgcggattttgtcttgactcaggattacgctgattttactgattaatttgattttgttttttgggattttacaagggattttgggagattgaagcgagttttgtctttctcaggattacgctgattttactgattataaggattttgttttttgggattttataaaggattttagaagatataaattggcttcattgatctgatccttttaatttaaaaaatccaaaagacataaacgaaaatatccgcttttatctcccaaaatcctttataaatcctaaaagtaaaatcaaattaatcagtaaaatcagcgtaatcctgagaaagacaaagtccgcgcaaaaagagctagatttgcggtttaaataaccggacttgaggaatactgtttttttaataacaccaccatttacccagctgaacacgccttacccggccactgcttatctgaaagggtttctgaatacaaagaatattacttccttccagtcggatctgggtattgaggtaacgctccgtttattttcaaaacagggtttggagcagttgtttgcgcatattgctgcagccccgccggtggcggcctcagagaatattgcgcggatgctggtgctgcaggacgattatatacagaccatcgacgccgttattttatttttacagggaaagaatcctacgctggcacatcttatctgtaagcgggattacctgccggaagcgtcgcggtttgcgcagctggatgaccttaactgggctttcggctctatgggtacacaggataaagcgaaacacctggccactatgtacctggaagatctctcggatctgatcatggaatgtgtggatccgcattttggtttcagtcgctatgccgaacgcctgagccgctctgccaacagctttgatgaactatacgccgctttgcaggcggaatatacttatatagacagtatcctgaccgatctcctggcgttgcatatgcaacaggtacaacccgcgatggtagcgatttctgtaccttttccaggtaacctgtatgccgcattacgctgcggacagtggatcaaacaacattacccggcggtaaaaatagcgatgggaggagggtttcctaacaccgagctgcgctcgctggcagacgcccgtgtatttgaattcgtggactttattacgctcgacgatggcgaagcaccgatagaaaatttgctgctgttcctggaaggaaagaaaacggcagaagagctgaagcgtactttcctgcttacggaagagaaagtaacttatgtgaacagcaaggctacacacgattataaacaagcccagctgggtacgccggactacagcaacctgttgctggataaatacatttccgctattgaagtggtaaacccgatgcacagcctctggagcgacgggcgctggaataagctcaccatggcgcatggctgctattggggtaaatgtacgttctgtgatatttctcttgattatataaagatatacgaacccattaccgcttcgctgctatgcgaccggatggaagctatcattgcgcaaaccgggcaaaatgggtttcattttgtggatgaagccgcacctcccgcgctgatgcgcgcgctggcgctggaaatcatccggcgcaagctcactgttagctggtggacgaacatccgttttgagaagagctttacccgtgatctctgcctgttgcttaaagcatctggatgtattgccgtttccggcggattggaagtagcttccgaccgtttgctggggctgatccagaaagggattaccgtggcccaggtggcgcgtgtaaaccggcatttcacagaagcgggcattatggtgcatgcgtacctgatgtacgggttccctacgcaaacagcgcaggaaaccattgacgcgctggaaatggtacggcagatgttccaggcagggatactgcaatcggccttctggcaccagtttacaatgacggctcacagcccggtaggactggagcctgcaaagttcggcgtacaaaaagaaacagaagagattggcccctttgccaataatgatatcctgcatattgatcctaccggtacggaccatgagacattcagctatggattgaaaaagtcgctgctgaactttatgcacggcgcctgcctggattacccgttgtccaaatggttcgacttcaaagtgccgaaaaccacggtgcatcccgatttcatcactaccgcgctgatggaggaggaagcgggcacggttaaacctacttctaaagtagtatacctgggcaaacagccggcgatggaaataattaccaagtcaaagaaagggagtacctgggaaatgtcttccttaactttccagggcaaaaaagagaaggtaaatatcagcgtgcaacctccccagggggcatggctcacggaaatgctgcaacagctggccgtgactaacgctaaaacatatacgctgcaggaggtgaaagacagctatgaagcggcagggctggatgattttgaattgttttgggataataagccggtgaatacccttcacaagctgggtttgctgaggttgtaaataaggaccgctgcaggtggaaagcagtattttacattaccggggattttcccggtatcagtcatgagcaaaaagtcaaatatttgtttccactaaactgacctaacatgagtgatcaaatgtcccttgcaggctatggctgtaatgaccagggctacctgaatcctatcaccgaacagctggactaccggatgccctttacagaggaccaggccgtgacctatggaatgcctattactgttgcggcatattttggtatgctgaataacttctacaaatttctgattgctaacccggggctgattcctttattccagggatcttactctgtggatttcagtaaagcctctcttttacgcatcctcagtcaggaaggttgcgaatacgtacgttttcattttgccatccccgagcctaacgagaagctgagcctggtagccgagggattaattttcgacagaagccaggtaggctatgcgcagttgttgcagaaagcaacggacaacaacatggtgcatgccggcggtgatccgaaaatagaggaaaggggcaatggaacaccggttcctttcccgccgttaaaacatttatttgaattactgaaaggacatggatcaccgttagctacggcagacctggaccagatatttggttaacccgattaaaactttttgtgccgatgaacggttgggtgtacgcatattatgctttattgatagcctgttttattatcagcttatttcacctggaacacagggaagtaaagttactgtgcgtattgctcgcagtatctattgttacggagataatagtagaattgatcggcacagaaggtttaggtttttttatagtgtatcatttttttgtggtgctggaatatagtctgattacaattattctccgatcggggatcagggattaccgctggcgcttactgatgggtatttccatttttgtgttttgcatggtgtcccttttctacagctttgtattgggcgggtggcgtgcctttccgggtatcaacatcaccatagaaagcttcctggttatttgctggtgccttttatcctttttttcaataaccccggatagtgaagcgtctatattccggcaccctgttttttggttaacccttgctttctttatttatttcgcggcttccgtgagtgtaaatgccttttataacctgttgctggaaaacgatactaccagggccaggcattttttcgcggtgttgaactcattatccaattacctgttgtatattatgctgataaaaggcgtcgtatgcttccggtcaaacaggatctctttgtagctgtgatttttatttcgttgctggttaccatcatgggactggtggtagtggcagcggtaataagttataagaagaagcaggatgcatatttacatcagcttaagttaatgaaagaagattacgacaaacaattaatgtggtcccagattgaaatgcaggaagaagcctttgcccacctcgggcaggaactgcatgacgatatcggccagctgctgagcagtaccaagctcctgatcaatgtaacccaacggagcatgaaggaaatcccggataccctgcaaattgcggaagataccctgagtaccgccattcagcatctgcgggcgctttccaaatcctttagccgtcagtggctcgaccagttcagcctgatagaaaacctgaaagcagaagtggacaggatcaattccagcagggctatcaccataaagtttacccatgaactaacggtgctgccattacaggcagaaccccagatcatcctgttcaggatcatccaggaagcgatccagaactgtataaaacatgcccgtccgcaggtaattgatatcagtatcagaaccgcgggccagcaattgatcctcattatcgcagatgatggttccggctttgataaagcagggatgtcgtctatcgggatgggcatccggaatatgcagcaccgcaccagtttacttggaggcgaaatccgctgggaggtaaccaccgccggcggtaccgccgtattgataacattaccccttgaataatttttgtttatgaagatcaacataggtattgcagatgaccaccagctgttcctgaaatcacttagtttactggtgagtggtttcaccggctttcatattgtagcggaagccatgaatggccgggagatgctggataagctggcgcaactgcctgtactgccggatatcctgctgctggatgtaaatatgccggtgatggatggcgccagggctaccgaggcggtgctgaaattgtatcccacggtaaaagtagtagcgttgtcgatgaaagacaatgacgccacgatcatagaaatgctgaaggctggttgctgtgcctatctcctgaaagatatccatcccacagaactggaaaaagcactaacggaaatttataccactggtcagtataacaacgatgcttccaatgttaactaccgccggttgctgttgcagtccgaacaaaagcaaacgcttacagagcgggaacgggagttccttcacctggcgtgcagtgatcttacctataaagctattgccgttaaaatgaacgttacagaaagaaccgtggatggttaccgcgaaatcctgtttaataagttgaacgtgcaaagccgtaccggtatggtattggaagctttgcgcaggcaactggtttctttgtagggcttagttttcccgcaggttttttacgggattagacagggccgctttcagcgctttgtaacctacggtgatccatgccatcatcagcgacagtataatggcggccgcaaatacgcccacgccaatggcggtatgataatagaacccggatagccagccttgcataaagaaatatcccagcggtgcagcaattacaaaggcgatacctatcagcagcataaattctttagagaaaaggaagaggatattgttaaccgatgcgcccagcactttacggatgcccacttcccttgtacggttggtgaccatgaaagaaaccagtccgtataaacccaggcaggaaataaatatcgcaatgcctgcaaataactggaacagctttgacgtaataacatctgccgcataaaaatccctgatccgctcatctaaaaagaaaaggtcatacaggtaagtagggtagatgccggtaaaggtttgctgcaccgatttcagcgtggcgcttacctttccgggatccatccgcacagctacatattcataagctgctgcctgggagccaatgaacatgggcacaatggcttcatgcagggatttgctgttgaagtcgttcaccacacctaccacgggataacttttatgatcaatggtgatcgtcttcccgagaatattttcgggagaggataaacccagtttttttacggtggtttcgttcacagtaatttcatgcagcgtatcgctggggtagggaagccggcctgctttcagtttgatgtcgaaggtcttgtagaagtcggcgtctgctgctttggcgcctattttaaagggttgtccttcgggattagtatcaaagtggaaattctgcataaatatccagtaagtggtgggagcatctgcacagaagctaacatttgtaacgcccggcagtgcagccagactggctttcagataattgtattttaattttaaagtactgtcgctgggcaggttgatcattacaacagcatctttgttaaagcccatcgactggtgtcttacataatccatttgcttcagtaccaccagtgttcctatgaccagcagctgggcaactacaaactggaatacgaccaggccgcggcgaagcgacacgcccccggttgatttaatactgattttgcttttaagcgctgttaccgggttaaaaccggaaacgatcatgcccgggtagaaaccagataaaagtgttaccacaatgccgcaggccaggatggcggcccatacacgtggcgttgcaagtaacgacaatggcagctgccggtcgatcaggttgcccgcataaggcagtgccacgatggtaataacgatggctacagcgatggaaagcaacgtaatgacacctgtttccgacaggaattgtgaaaacagctgcaggcggttactgccaagtacctttctcacgcctatttccttcgccctgtttacagacaaggcagtggccaggttaataaagttgatacaggctactatcaggaggaaaatgccgatgagcgtaagcgcccacaattccctggtactcagcgttgcattggtgaaattgggatagcgcttatccaggtgcatggcagtcagcggctgcaattttagctggggcaaccgcgtattatgaggcttgtaataccgtttggcaaaggcgggcaggcccgctgtgatggccgcggcattatccggttttttcagcagcacaaaacattgcccatagccaccgggtacagcgtcccattgtgcacccgcagtaaaatcttccggcaccagttttttcagggtgctgtaagatacacccacttgtacggggagatctgtatttgcaggaaggtctttgaatacgccggttacctgcaatggcaccctgaaggaccacatctggatagtgcgcccgatggcggcatggatgtccccgaaataggcccttgccactttttctgaaatgaccgctgtattcggggctgataagccatccgcgttaccggccagccaggaataatcaaagatgctgtagaaaccaggagaggtatagaagatgccattttgtttgaaacgcttttcatcagtggtgccgggggcaggaacgtacatctgcgctcccccctggaaagaaatgagcccggctttttccacgccggaaaaatcggtttttattttttccgggagctcccagttcaccgtactcagttgctctatcacttctccgttactgcggttcatcacgtcggtggtaacacgataaatcctgttggtgttggtatgataggtgtcgaagctgcgttcataactgatgaccaggaaaatgatcaatgcagcggcgatgccggcagacaggcctgctatattcaggatggtgaaagttttcttccgggtgatgctgcgaaaggctgttttcaggtagctgtttatcatagtggttatgccactgcaaaaagcaggtcagaaatgtaaggtactcagattcaatgtttttaatcatgctttattgtccggttctgaacaactgatttcaattccggacaattggctttcaccgttttatctccactgtttaccgcctttccggtggcattcaccggtttagccgcggtgatcaatctggttgttgtattttcggctgtacgtttaaactaaatgtgatcagatgatcaatcaacaacaggccgctgctcccgttttggctgtgaaccagctgaacgtgcagtatggcgctttccaggcagtgaaggatgtttcctttgaggtgcatgccggtgaaattttcggtttgctgggccccaatggcgccggcaaaaccagtacgctcagcgctattgagggcctgctgcatcctgcttccggcagcgttaccgtagcaggttttgatatcagggagaagccactgcatgcccgtgccaatatgggcgtacaattacaggctaccagttttcagcccgagctgaccatctctgaaatcatccggttgtttgccagtatttacggggtaaacttaaaggatgatgccgtgaagcaaaagctggcggagatcaatcttgaaacctcagcaggaaagaagatatcgcagctttcgggcggacagcagcaacgcgtatcgctggtcatttccactattcataacccgcagctggtattgctggatgaacccactacggggctggatccgcagtcgcggcgccagttatgggaaaggatggagtacttccgtgacaacggtcatgcggtattactcaccacccattccatggaagaagcggaagcggtatgcgaccgtattgcgatcattgaccatggccgcattatcgccatagatacgccggaggcgctgatcgcgcagcaccgggatgatccggcagtgctgggcgtagtgaggaaggggaaagttactttggaagatgtgtttattggtttaaccggaacggctgtccgttcctgatcaaattactacggatggaaacaagtgtaccaaaaaataggacggtaatgactgctttgttgcgggccgattttacaacgctgtggcgcaaccgccggtcgttcggactggtgttgctggtgtcgctcgttattttagtgtcctggaaggggctggtggataaactgggcggtgtgtttgtgctgtcgtcctgtattacgatcgggctgaccagtatcgggttaatggggtattccaatagcattgcccgcgaccgcgacaggggcgtgtttcagcgtttgagagtaggccctgtatcggcatggacgattatgatgagccgcctgattgtacaaatagcgatgattttgctgatgacgatccttgtttttgtggtgggttattttgtggatcatatttatgtttcgccggtgggttacatcgccggtttgctgatggcgatggtaggaggtttagtgtacctggggatggggcaggccattgtgggactcatcaaaaatcccgatacggttaactctactacccgtcttgtttactttatatttattatgatcggcatgttcggcgagtttggcgtgctgggtaagaagatagcattactggtgatctggtcgccgtatggtgtggtaaggaaagtactggcggcgagccttgatcctgccagctggagtatagataccacctgggcattactggcgtctgcagcttatactattgtatttgtggtgttgggggtgaagtggtttaagtgggaaaacaagtagtgaatcgccggtatgttcaaccaagttgaacataccggtggtgttttttatttcgttttgtttgtttttgggttgatgaattcccattcattgatatgtgcgtttcggtgttctttttttacgatgtcgttgaataccggcagcatggcagtatgtgctgccgccacatcgtgcgcttctgctttatcggtactgaggtcgtacagttcccagggtgcggcgggatttttcttcaggccgtttttaatggctttccattttcccatgcggatagcgatggcgccgcctttttcgggatattcaaaatagagatattttctttctgcttgttgggcatgtttgcccgtcatttccggcagcagtgaaatgccatcgtttggtggggcgggaatgcgggcaatggcggctaaggtggccatcaggtcgtactgaacggccggcagctccgatgttttccctgccggtattttccctggccagcgggctatgaaaggttcgcggataccaccttcgtaaaggtccattttaagccctttcagccccccggtgctattaaagaaggctgcgtccacgccgccgttaaaagtggtgccattatcgctggaaaacatgatgatggtattatcgtccaacccaagactggcaattaagttcataataatgcccacctgtgaatccaggtaagtgatcatggccgcgtaggccgacagcgggtatttctgcgggctgtagccctgctggccgtagtagggcttttcattgaactgcccgaggtatggctgtagggcgctgtcgggcacctgtaatgacacatgtggtatcgtgtaggggagatagagaaagaagggacgctgttgatttttcctgataaactgcgtggccttttttgtcatttcatctatggcataatctttccctttataatattcaaaatcggcatcggtagcagtggcgggcgacagtgacttgtgcacatcaatgaaagtattcctgagactgtcggctttgccgttttcccagaggtgagtaggatagaagctgtgggattgtttctggtcgaggtacccatagaagtaatcgaatccctggcggttaggatcgccggtgctgtattgcatgcccagtccccatttaccaacagcgccggtagtgtagccggctttctgaagcatggtaccgatggtaacggtaccttccggcagcggcatttgtccgccttccagtgaatcggcgaagccgcccatttcataattcccgcggatatacgagtgcccgccatggcggccggtaagcagcatacagcgtgcaggcgcgcacacgggtgtgctggtataaaactggttaaagtggatgccttctgcggagaggcggtcgaggtgtggtgtttttattttctgttgcccgtaagggcctgtttctgcataaccaaggtcatctgcataaataaaaataatatttggctttcgtgtttgcgcagtggaaataaggccctgcaagaccagtagtccaagcaggcatgtttttcttaccataccatcagattgtttgtgtcaagatagacatgttatggtagataaactatagtaaaagcattattgcgcaagcgtttgcgtacggatgatcacttcatcgatgcggtggtgatccattttttttatttcgaaggtcacctggttgagcattactttttcgcccggagcggggatatgttttagtttatcgatgagcaggccggcgatggtaatatcttctttttcatattcccgcagccattcaaagttcagtgtttcgcggatatagtttaaacgtgtatagccgtaggtaagccagcttttgtcgtcctgctgtacgaggtagcgctctgtggcgttgaatcccggcaggctgccgccgagtaagcctgaaacgatatcatgatacgagattattccttcgcaggcgccgtactcgttgatcactacgcccacattcgtgttttcgcggcgcagctgctggaagatatcgtatacggcctggtttaccgacaggaaagaaacggaggagagcagtgcttccagcggcttatcgggatacagcaggaattccttcgcccctaatgcgcccagcacttcctttttatcgctgactacggggaaggtgcggtgtatactgcgtttaatcgtgtccgttattacctccctgttcatttgattattgatgtaggtgatcatgctggccggtgtcatgatgttttccgctgtgaggtcgtatgcggagaacaggtttttgtgcagggtgaattcccctttatctatcagtccctgtttgtatgcggcagtgagcatgcttcgcaggtcgttttccgttaatttttcttcgcggatggtgtttacggaaaagagaccgagaatgaacttggtgctggcggtaaggagtttaataaagggataggtaatttttgaaaagatgatcatggatggagtgatcaggtaagatactttttcagggttcagcagggcgagggttttggggatgagctcaccaataacgatggtgaggtaggtgatgctgcctacgccaacgatcagcgctacgaggtgtgccatgctttcatgcaggccccaggaaacaaataccggttccagccacgcagccatgagatcgcctccgtataacccttccagtatgcctaccagcgtgatgcctacctgcactgcgctgaggaattcatccggatctttaatgaggtttagtacgttgagggcttttttattgccgttgtccgcctgttgctggaggaggggtttgtcgacagaaattaaaccaatctccgcaatggagaagtaaaagttgagcgcaataagtacgagtatgatgatgatagaagtcatagttagttaaacaacgggggggagttatttgtttaccgggctggttttcaggggagttgtggcggttgactgaaaaaaaatcccagtgaaattttggaaaaataaaatggctgcttatatttgcagccctgacacaatatcagttgcccagatggcgaaattggtagacgcactgtgttcaggtcgcagcgcctgcaagggtgtgctggttcgaatccagttctgggcactaaaagtggacaaatcgagattgatcttggtttgtccactttttattttcgggaaggtctgcgtccagcgcgtatattattcctgcgctaatttaaattatcgtcattattatttgagttcgggcagcttatatttaccatctaatatagattttccaggcatataaatacgtgtacatgtccagaatggctctgtaggaataatgagttcattgctatgttttcctttaccaaattcctcctttggtacaaagtacagatcaaaggttttgccatcggcgtttaattttatttcactgttactgatcgttgatccttcgtctgtcttcaggtattgatcatcaccgtatatggtgaccgagtaaaatcccaatttggggtctgcgagttccggtacattaaaggtagctttgtatgttttacctttttgcgcttcatgtttcgccgtaagataaacagcatctttgtcaggtaatagtccagtggctatggctacacctctgtttctcgcttccagggaaaccggattgtctgttgtgcccatagtaccctttacaccttccttctgtgccagttccacgtaatgattacggactttattaaactcgtccatattccaattggttaccttgaagctccttggtttataattattcaggaattctatttttaactggtcctggtaatcatttaccttctttatatctgcagggtcttttggattaacctgcattcttacatttgcatagaaaaagtcactgcttttggaagctggtataacatatctgccgggtccataaagcactttataagttgtatggtcatgattcatgacatgaagcgacatatatctgccgtcattctgcggaagtgtaattgctacatcgcctttaccatcaagaatagcaaatgaatactccgtatcccggttcataagtggagccggttgttcatccagtggcattggtttacggtgatggttccaggcattattggctccttgttcaaattctttctgcattgccaggtctgtcatggcaaaagcaaaattatctttagtaacgctcactgtgctatcactgtttgctaccgccgccccagtgctatcagtatttgtgttttttgtcgatgagttgcaacccaccagcataatggctgccccgcttataaaagcaaaggtgaactttttcagtatagttattttttgttgactaacgctgctcatggttaaagattttattttggaaagtgtattattaaaggatgtcattttactttcaaaacccggtgattttttacaaagtcctctttgtaagcaatcatagaaggtactgatgttggaagataacacctgaacagtgcgttccagtttttaggtaccttgatattgttaatatcggaatcggaaccattaaagttgagtgtaatagttccatccggattaggctttgcttttgcactgtttgtgttgaatgggtccgttaccacccagccttgttcatcatatatggtgattgaccaatatccagcacgaccatattgcagatcaggtttcttaaatgtcacgctactatgttcagcgttctttgctccttcatctccaggtactaccacaaaatagtaggcatgcttagcgggaagtccgccccagcctgccagatttatcatctgatactgaggtgtgagtgtatccttgatattgtctacgaatcctttttcaataacgccctcactaatggctctatgaataagttcattccggagtttattaaaagaacttacatcatatttaacagccgacacgtaaggattggaagctccggctgtaacgacaatggcatcctgtcgctttctcatttcttccattcctttttcatcataggaacgtggttgcgttctcataaataaatagacatgatcaccgtatgacaggtcttttttcccaatagtgagcgtttgcccaggatagcatacaccaaccgttacatggttttcatcaatcacctgaacaatctggtaaaggtcgtattgggggtttgtaatggtaattccaccactggcgtcgtaaactgcgtatgaatagataaggtcaaaattggaacggatgatggtctgatttttcagatcaataccgtttctttcatgtctgaatttattcgggccggcttctatggtttccgcggctaaatattttgcagtttctgcccggaccatgttatccatagtaactatctcaccaccattatcggtaaacgccggattctctgccgatgcttccccatttttaccaacgcctgtactcacttttgtagactgtgcgacaccgacagcatcagcattttcatttttggttttttgggtttccgcacatgaatagaagagaattatggatgagcagatcaggaagatgtttatttttttcatctttttaaaattttaagtataaacctgaaaatgtttatttaaggttgttaccactatttgccagccatgaattgtaagttaattcctgtaaacacctgaaactgtggctgcacgccatataccagcatcgaatattgtggttctacaaataaattaaataccgtccctccgagctttacaacttttccgatgcccaatgccaacggtacagaatatgcttcattcttaaaatcaaaagcccatataggcgcaccacgtaaataagtaccttttcccaattgccagaagtaaaatggttgcaatgccgccaggcttgttgatgttctgtcggcctgtccggcaaaggaagcctgccaggtaataagtcctccaaactgaaaaataggtgatttggcaataaaggcgacaagtgcaaagccaccttgccatttgccagcgcccaatggttgcgttgtagcactgggggtagtcaccattggcccgatgccaacggtggcagtaggtttagaaataaaattgtaagaaacgaaagcattttacatctcctaatccatttgaagtggtattggtcactgtgccattatacgtttgctgtatggacatggtgctcagtggagcggaggcacgtagcaataatttcccctttgcaaatggtttggcgaacctgatccaaccggtgttcatgtaggagccgctttctgcattactcagtttagcaacatagtagtcatggaagtttaaagccgtcatgttcgcaagcgggttattggcttgtgcggcagactgctcgttgtcctgtgcattgcttttattcaccgacagtgcaactgcaataatagtcgttaacagaattgccagaatcttcattataggtgtgtttgttatcattcgccgccaggttgtttgaaactcataaagtgtgtatgatataatcacaccccagagactgataacagatatcttgagcataaataataaggtttggttatagcaatacttatccctatttatgtgtttggattacacagaaatcacatctgaaaatcagtaccagtatattcgatattagtttattatacatatatccgatattacatataaatacaaactaaaattcaataccgataacccagttttgatttttgctaattacagtttgggagaatctcccgatagtgagagtaaatgatataacagtatataaagcggtattgttctggaaagaggtttttaaaatataatttactcgtttctaaacctcatccggcgagaaaaacataatgcttatttcacatgaattgtggatgcctatttactttaatcgactcgtttcttaatgacgcattcctctattttttggatcgcttcttcttttgcatttgtttaaatccctccgcggttagctcataaggtaaataattaggagtatattctgattgtaaaagcagctctaataagctactcaattcctgtattgcggggacaatcggcgaatgtgctattcgtgttgtttgctgggttagctgaagcattttccacgtaggcgtaagctttcagtggtctcttacattttccaggatgttattttttgctctgcctgttttgctgtcaattccggtcttatatttaaaatcctttctattttcgctaatgaaaacccaacctcactgccttttatttttacttttttatcatcaataaaagctattccccgacctttaattaccttatacttcaacacctgcattttttgctcaaactctgaattctattggggtgacagaaaggctcggggcttaaacttcctttaatttgtattgtttttccagtctccggcagagagtagccattctcttaaagctgttgctatcgttggctgtttttccattatagcctacctggttggcgacaatatgtatgtgttgttcgtttgtatccttgtgcaatacacaaatgtattggttgtctgctaccccgaattcattggcacattccctacctacctctgctaattgatttctggaaagagtttcaccgggagccaggcgaagtgataagtgtaacacggggatctctacccgtttgctcaatttagcaacatctttaaagtcttttgtcagttcatacttgttcccaaagcacttattataaaacaatacttctgcccgatccttatgccgaaggctgtctttttgggaaagttgccgcttctgttcttcggataatttgcttaaaccggtacgttcaatcaggtttaattcttccctgctgttacgttttctggcgatctggttgaggtttgctgccatgtggtttagcatggcagtgaagtttaaaacctcccatatctttatccaggaaaagatgcacttgtttatattgctccatccacaataacaattttgcttcgggttgtatcttttttttcatcagcgatgaaagccgggtgctggttattggtaggggaaggcgggtgaaaagaaagaatcaggtcagatggttggttggataggcggcatagcagatctgcaatactgcacttaaagtacagagtcccgaaatccaccagattgccacctttagcgattccgtggtcataccatacatttatttgcctgttgactttgaaggatggcgttttttcttcccgcagcggggacagataccaataatcttggtttcttattatttggggcaagtggcccaataaagccagatagtcaacgagatcaatctgttttgcttctgccgtccggcattggatgcagaattactgaacaatatgcgagttctcgtgttatctattaaatacccttcgcatcaaatagcattcatcaggttttaatattggccgccatgtttatgcatccaaggcatgtactggcgccaaattatataatgcaaaaagcaccctcatgaaaatgttatttagcggcaggctgtttctactagcacttgtaacttatagcctccatccccacccggcgtaaaggtctctaattcctattagctaaatactacttctttttcccaccaagtgcagcaactgccgaaaagttctggcgcaatagaagctggctatctgaggcattcttactattaacaatgacaggatgttcgtcgtataagaaaggcaaccggaagattaatgagcggttcatgattaggcgttgcccaacaaacgacgtaaaatctgttaaatacattctatgatgaaaaaaatatccggaataaaaatgaaactctacggtaaaatggccgtcacaggagtttggttagctgtaggtgtggtcattccgccgacggctaaagcgcaaaccgttaacaaaccaaacattctggtgatttttggagatgatatcgggcaaaccaatattagcgcatacacgcacggtttagtgggatatgaaactcctaatatcgaccgggtagctaaagaaggaattatgtttaacgactattatgccgaaaacagttgtacggccgggcgctctaccttcattacggggcaaagctgctatcgtaccggactgtctaaggtaggcatgcctggtgtagatataggcttgcaagcccgtgacatcaccattgcacaggcgctcaagccgctcgggtacgctaccggacaattcggtaagaaccacttgggtgacttgaataagtatctgccaacggtacatggcttcgacgaattctttggcaatttgtatcacctgaatgcagaagaagaacctgaggatcccacttatccttaccaggatagcgcatttgcaagatcgtatatggtaaggggagtgttaaaatgtaaagcaacaaacgtagatgacccgacagtcgacccgcgctttggaaaagttggcaaacaaaaaattgaagactcgggacctctgactaaaaagcggatggaaacgatagatgacgagacttttgcagcagccatcgattttatcaagcggcaaaatgcggccggaaaacccttcttctgctggatgaatgcaacgcgtatgcacgcctttacgcatgttcgtgcgtcgatgatcggacagagcggtatgcctggcaatgaatatgctgatggcatgttggagcatgacgctgatgtaggtttgatattgaaagcactggatgatctgggtatcacggacaatacaattgttatctatactactgataatggccccaatatgttcagttggccggatgctgcaatgtctccattcagaagtgaaaaagatgctaactgggaaggtgctttccgggtgcctgcatttatccgttggcccggccacattgccgccggtaaaatatctaatgaaattatgtcaggtttggattggttcccaactatattagccgctgcaggagacactaccataaaagaaaaattgttaaccggatatcaatcacagggcaccaatttcaaagtgcatttggatggcttcaaccagttgccatacctgacaggaaaacaaaaaaaatcggcaagaaccgaattctattattttaatgatgacgcagttcttgtatcgatgagaatgaacgattggaaaattgtctttcaggaacaaagaatgccaggtggttttgctatttgggcaaatccattcacaccgctccgcgttcccaaattattccatttacgaatggacccctacgagagagccgatattacttcttttgtgtacgaaaaatggtgggcgacgaaaatgttcattgtggcagaaggcattcaaaaaggagccatatttttgcaatcattcgtcacttatccgccaagtcaagatccggcgagtttctcgattgatgccataagtggaagagtaaaagatcaaattaaaatgcttcgcgcacaacaaaacgcaataaggaaatgatttttttgagactataacgtattatgtcaaatgtcgtttttatacgcttttacccgttttttcacactattagcgacacgtacttgacatgcgaaaattatcttctttttcctcagccgccagccagtcctgcgttttggcagaatggcaataaggctgttgtgtacgaaagaaaaatccttttcctattttcaccagcatcaaattacatatgtttcttgtgacggaagggggggcaatacggacgaatctggcggggatgaggatagttgcacgatcgataaacatttaaccctggtttttgttgttaatgatatcactttcttttccttgcataaacaaattaagttgaatgattttaataattcataactaattatgtttatgcgatttatttttcctctcagatcggcttatatttttctgttgctaattctgtcaatactccggagcatagcgaaaaaagccctctatccgttttttacagcgctgctttttgcaaattgcacacaaaataagcacacagaaaccaatcatactccagccgatagcagtgcagttgaaacagcaacttttacaccggctaatgtagatgaacgggcattatacagtcgcggttttaatgcagttgtgtggggcatgccggcggtaaattttgaattgtttatagaagcgcttaataaagcaaaaggtgattataaccaggtggtttattggtcggggcttgcgacttcaaaaaaccagacactcactcctaacccggatgtgatttatgtgaacccattttatgacacgcgaaaggggccggtagtattggaaattcccgcggcggcaggggtatcttctataacaggtagtttagatgattctggcaaacagctattgaagacgtagggccggcgggtgttgataaagggaaaggtggtaaatatctcattctgccgccggattataaagacaaaattccggcaggatatattccaatgccttcatccacttacgttggctatgcgatacttcgctctaatcttgcaaccggaaacaaagaagatctcgcaagggcaattgaatatggtaaaagcgtaaaaatctatccttacgcacaagctgccaatccgccgcaaacaacatttgtcgacttactgaatgttgattttaacactaccataccttacgatactcatttctttgaattgcttaatcagtttgtacaacgggaaccctggttaacgcgcgacaaagcaatgattgatcccctcaaatccattggtattgaaaaaggaaaaacatttaacccggatacacgtaccaaagaaattcttacagctgccataacagatgcgaaacaatggatcaataaaaaataccagggagtatttacaccgcctttttatgaaggtacgcactgggcactccctgcttctcctacagttgtaaaagaaataatgagcaactatgcggatgccaatgaatatccgatagatagtcgtgctacagtcttttcaatggcatatttcagtgcaaaacatttaggtacggggcaatattatttaatgacaatcagcgacaataaaggccagcccttggatggctccagattgtatcgtttgcatttgcctgccaaagttccggtaaaactgtattggtcggtaacagcctatgatggcaatacacatgcattaattcccggcatggcatattccagtcgcgcatccactacgccggggcttcagaaaaacagtgatggttcggttgatgtttacttcggggcaaaagcgcctgccggcaaagaaagtaattgggtaccgacacaacaaggaaaaccatttgaattattagcacgtttttatggccctgaaaaagcattctttgataaagtgtggaagatgggagatgtggaagaagtggaataggcagcgcccattcgtagcaaagcctccttccgggaatattggaaggaggctttctgattagtatcgataaattttcaccggccccaataaccccgatggctgcaaaggtgaaccggcgctgtaaaaaggcagggttgtataagtaatcttatttgtaacaccgggttgtgcatcaccgatcaaacggttcacccaaagattggtgacctttatttccagtttgttatctcctgctttgaaagcactggttgcatctacccggaagggcttcttccatagtatacccagcggttttccattgaccacaacttctgccaggttctttacatcgcctaagtctagccataatcgttcgcctttcatgatagcgtttgaagggagattgatatgctttgtataggtggctgtaccggaaaagtacttgatacctgcattgctgttttccgtataagaggtcagcctatcaaaagtggcactatccggcgcacctcgattgggttggaacatcacctgccaggaaccatctgtcgttgttatctccttttcagttttggcggggagggtaacggcattttttttggcatctgacaggaataccacaaacacagcgtcatttggcgtcagcttcaaggacacggtggtgcggttgtttgctattttgtaagatgccggttccatgcttcctgtctccggatgccagatctgtggcacttttccactgatccggaatatcgcttctactgcttcatcccggtcgttccggttgtttacccaatagatatcaccacctggtaatttgcgatgcacatatagcaggtgtgaattatttttcggtttggtatactcaaaatcaggggggatatttaaagaagaaaggacttctctcaaaggtttatttactgtaacgtttggatttgatgaggcccatatttcatgtaccagtgtattgaattcatttgggtcatcagccagacttggtgtggctattggttttacaccggtaatcgtggcgccggatcttacgagatcccttagtttacgcaatgccggcaatgtcattttaacagcgctgctatccagtgccagcacgcggtagctcatgccggccggcgtaattaatttaccatcttttaccgacaaaagatgaatgagtgcatctgtattgatgaagtcataatcatatccttccggaatgaccggcggttttctcccaaagaggttggtgatattatcatcttctccatagtaataagcaatatcggctgtaaacctgccctgctgcaataaatagctgctgcgggccagatagtcgttccatacttttgcctgttcagcccatgtttcatggcgggtataccactggccgaatggtccaaggccaagcccgggaattttggtatccgacggctggtggggcgaacaatgaatcacaaaacggtttacgccactggccagttccaggtctgcacttgattttaaattcccggggtaatacgcccacgcagatccgcccacacccaaggcggttaaggattccgcagctactaaattttgcccgtacaaatgcgctaccgatgcggattccctgatatcaatcgtatattttgtctgatcgttttgattgatgacggggttaggtgtccataacgcagacatagggatagctgcggttctttttacctccatgccatcgccgataaatgcgcggccatcttcatgcgattcggaatagcgcttcaagccgtatgctgcgagaatatcggtgagcgcatcgtaatgatatgcggccaccatttcccccaatgttttcctgaaatcaaacagaaacgcctcgctggcgtcagcgcttttcacgatggcgcctgttagtacaggtagccagggaataatgctgtaaccacggcgtttctgaaattccgctggaagatcagcagtccagttttgtgcgccggcttcccagctgtctgttacaaggtattgcagcgcgcctttaccgcccatcaggctaccggttgcatttttatactgatccaggtaagtggtgaagtatttttttatggcgaccgggtccagcttatccacttctaatcctgttgcggggtaggaggccgggtgatttattgtgccaagcaatgaatacccgaagcggataattctccattcgcctccctgaggggctgtccagttcagtgttccatctgcacgcagcttatccgtaatattaatcacctcatctactgtatcgctggtttcagcagtttttttgagatccaataaattgcctgccggtgcaaacgccgatttttcttcaaaccggtttatccggtcggcagtatatagaacgatttctgcaatttcggtgccgcctgcattttttttgctcttgtcggcgagtcccatagtggccgccctgttaaagggaggcggtgggttcttcacggtaatgcgaaaatattttgccgttgttgcaggcacagggatggtttgctgtaaaatggcgccaggtggaatataggtgatcaaccggtaattcacgccgtcgtcgcttgcttccaatgcgcggctgtctgccgggtctgcgccctgaccgtacatgccggggttgccaccgccaaccatgctgaccgctttaatcgtttgtggttgcggaaaggcaaattgtatccaggcatatcccttcaccgtgtctttcggtaaaagaatgcttgtatttaaatcgccatcggtaagttgagataaggtaaagttgttactaccagatgttacaaccgcgcccaagccacgtaatgatttgtcggcttgcggcactttgcaggcaagtactgctacatctttataaaatattatatttttagagatatcagtttttcgttcaccaaaaggctgaacaggcatattttgaaaagggccggtaataccgggtacaggcgctattttaataccagtggctccgccttttacacggacttctgtccacactatttttttcatcccgtcttccggctttacccagggaccgccggtttcactgaaccccggcgaagcggcgattgccatttctaatttcagggaatccgcaagtctggtggcgaatttgaaagcgtcgatccactcaggcgtcatataaacgagcggcttatcaactatctgcgactgctccgagcggccaagttccacttcaaaattatgaaagccgccgatacccacccgatgcatccattccaggtctttccggataccatctttggtgatgttgccattcatccagtgccaccacacacggggctttgcatcatttggcggggtaataaaatttttacggaggatatcgttgtttacctgctgcgcatttcccttaacaaagaagaaaagaagcacaaaaaatacgcttgtcctttgcacgaaatggagtttaaaattaacggatattacaaatgcacgaataggcagccatcacttattcctatggcctcattcgtgcatttgtaattatttaaactagaatttaaatgccgctgtcatgaaatatgctcttggcgcaatagcaacggttgagtaagggcggttactcttcacggcatcttcatacatctgttttgtaaatccttgcctgtcgagcgcttcgttgaatgaacccgggcggctccagctcattacaccataagtattgaagatattgttgacaataaaacttaaccggaagcttttagagatatcatagccggcgctgaaattgaactggctgaatgacggcagcagaaaagcattggccacatttgcctggcgttttcccatatatgaccaggtgaactgcgcgtagaatttatccaggttgtaggaaggagtaatattgatcatactcctcgcgatgttatccgtttcgtttccggagaaggtagtgaccagtgaatcatcctgcgggcctgggttgtttgccagccatgttttgaagtccagggcttttgacctttgcagggtaattacaccatgaatattgaaatgctttgcaaagccataatctgcttccacttctacgccataagttctgtatttattgtataccggtaatggattgtagttagtctgatccgcattttgaaatgtttgcaggttgggcacgtggctcagcacactgtaaaagggggttacaaataaactcaggttgcctgtttttgcttttatgccgagttcaaactggcttaccttctgcgcctgcggatctaatgtttttacaagaaaatcactggtggcattgatatacagatcaaggtcgggcgctttgttaccctgcgaataacgtccgtaaacggagaagtggttattaatcttataattcaggcccgctgaataagaaaaagtatttaagctgttgttgaagttgaaggtcgatggagtagtggcgtaagcattatcatacaaggtgagcttgtttttatctacgccaccggccgtatcctggttagcaacggatgggctgttgtagcctttcacgcgcactgtttcgtaacgcacaccccaatcgagatttaatgccggcgttatttgccagttgtgaccgaagaatagtgccagttggttttgggtaacatggttgattgtctggccaaccctgtttacagtcataacgccatttgaatttgtaaccagggctgtggtgccgtcaggattggtacgtgtaatacccaccacctgtggttgagcctctactgtgcccagcgcaaagcccagccgtccgttaagcctgtccagtttcgtagaaccaaagaatccgccgagcgtgaagctcatgttcttcatttttttggttaaagaaaactggtcaagatattcttttgctttattgctcacaaacaggagcggttcataaaacaaagagttaggaactacctcaccacctggcagattactctgggttaccgtaaatttacggccgtccaaagtttcaaccgttgccaggtcccggccgtttttcagatcacggatgtgataagtgcccggttgcccgattgtattcatgcgggtatagatcgcctgatcagtcagttgtattggataaacagagccattggtattccagatggtgcttttatcggagtaacgcatggcattactaaatgtccagccatcgccaaaccgctgttcccagttaaatcctgcagatttatctgttgagtgaatcaggtccttattgttgtaaatggcgttttgaccggtttgattgatactgaaattttgctgaatggagggcatcagcacatttgaagtttctgagaagcccggcgccggtttgggattcgtaaaaccaagcgttggtgtaaattcaaaccatccgttgtgatcgtttaaatatttcgcgtagaatttcagcgacccggatgaatatttttttacgaggttgccacggaattgtcctccgttgttcatcgggtacccggggtatcttgcaccttctgcgtaccggtaaaacccgccggcattccagaaccagtttttgcccagggggccgcccacattaaggtctgtacgatagaagctattcttgccatttccttccaggccgtatttggcgacaacttctccctgtgttttgtcgccgccttcttttgtgatgtagttgaagataccgcccggcgcattggcgcccagaatggatgcggtgccgccccgaaccgcttctaaccggcctacagtggcatcggcacgaaggaagtagtcgggcccgaaattactgcatgttatattggatacgggcaaaccatcttcctgcatactcacataataatacccagaagcaccatcattggaacccactgataccccacgggaataaacggtgttacggacctctccaagggaggagttgacataaacacccggaacatttttaaggatgtcggatgcgcttaccagtgccagtttggatgcctgggcagcagatatagtactgattgctactgatgcttccatctttttccgcttatcaaacacgccggtaacgaccacttctcccaggcccgtagcagatggcttcatgtcgacaaccaaagaaaaagtggcgcctccttttagtgtataaccagataatttttgtgactcatagccaatcatggtaacagaaaaactgtatggtccaccggcaggcacaccggaaaaggtgaaaacgccggcggtatcacttttggtgccggatgtaaagtttgttttgttgttgcggataataactgacacgcctgcaagaggttcgttatctgcgccatgcacaatacctttcactaaattggtaccttcctgtgcttttgcatagaatgacggaaggatttgtatgagcaatagaagagctaccagaacagccctgaatttaagcagttcaaatttcatgtggaattttttttaataaaaagtaaaggtctgtatcagtatgactgaaggttcatcctgcaggatgcaattattaacgtgttataatactacttgctgatgatgaaaacgctatcctttttggtgatcgttaaattgtgaaggatggcaatttcttttaaaatgttctctaaagaatctgttctattgtatttggctgtaaaatatatgttttgaatatccttcttcttatacactatttgcacattaaatagctgcgacaggtgatcaaacacttctgacagcaattgattgttgaactgataccacgaaccctcggtattttcaggcagggaaggcttatcatcagataactcatcattgatgatctgctcgggagcagccttgttgtttagtttaaatgacttcacattggccgcgttttgattgccgtaaacgaacgactgtcctggtaacaggtacacatcttcttccattttactgttcgatgtatctacggcctttactaccactttacctttatataaacggactatcacctggttggaattgccaaaagaagtaacggtaaattcagttcccaatgcagtagttgagatatcaccactggtcacggtaaaaggtcttgccttgtcgtgcgctactttgaagtatgctttacccaccagtgatatgtcgcgtttatccgtaaacgggtccgggtaagttacttcgctgttgttcgccagaacgatcaaagagccatctgctaactgaattcttttctctttaccagtcgtattcacttcatgccgcacaacaaaccttacgctttccgtcttttccggtgtatgtccggcaacaggattttctgcgttgttgttgcgggaaagcagccaacctacaccaattactaaaaggatggatgctgccacagctgctgcaagccacatgttgacaggcttggaaatttcccggacttccacctccgggaaattttgttccaagcgattccacttatcttccagtttcgtttcatccaccagatatgttaagtcgtgctttagctccgtaagttgccagacttttttcaaatgattaaagtagcgctggttctcttcacttgcattgagccagttttcaacaaatactttctcctcagcagtttcctcattaaacaagtatctgactaaaagctcgtcatattgattattatgttccatgtgcgctatattatttatacacctgatgatgaattcttccctacaagcgggaaaaaaatatttttacttttttaacaagaggctgaaaatcaatacaataataaagaggagaaacttcgacagcttttccttcaatttgatcatagccctgcttatctgggtgtccactgtttttacagatatatttaaccggctggctatttccgcgtactttaacccttcagattttctgagttcaaatatgatgcgcatctgttcagggagttctgcaatagcggcgtctattgcggaacttagctgctttaaatcaatactgttaaagtccgtttcagcaatatcttcagaagttgttctcaacagatggactgcatactgttgctttactttttcatgcctgagcgtatttaaactgagattgttaacaattttatacagataagatattggagatatgtcaggggcaagcgtttggcggatttcccaaagtttgatgaaacctgaatgaacaatctcctctgctgcatgaatgtcgaagccatatttcaacttacagtaaacacaaagaggtggataatgttgcttaaataactccttaaaggcagctttgtcgaaccgtggattatcaggaggtacgccatccggattgttttgtgtgtaattgatgctcattggcaagtgctcacctttaagtgaaaagataatttgagtatagcggttggatcggtaaaatgtagctccgacaataataataaatatatataacctgggaaataaaatttccaaaggcgatgtttgggatatcaattttaatggcttgcgaaaacaggtagcttttattgctggccgcgcaaaattttctccatctttctgcctttcgccaattcatctaccagcttatccaaatacctgacctgttgcgttaaaggatcttcgatgtcctccacacggtatccgcagatgacgcctgtgatgaggtttacgttgggattcagcgaagcctgttggaagaatgcagcgaaggttacattttcttttatcagctcctgcagctttttattgtcgaagccggtcagccaggttatcacctgatacaattcttcttttgttctgcctttcctttccacttttgcgagatacaacggatagacggaggcaaatgtcatttttgcgatacgctgattggcgttgtccatactgtctgtttagggtgttatgttatttttttaaaataatatgtgtggctctttctccgttaaatttttcgatttgatggaagcccatggcgggaatatcgattcctgaaaacaggtgttctcctgaaccgagaaaaatgggagcgaatgccaggtgcatttcgtcgatacagcccgcctgtaagaactggtgtattgttgaaacgccaccaccgatacggatatcttttccatttgccgccttttcagatttttcgagcgctgcttcaataccgccggtgacaaagtgaaaggtggttcctccttccatctcaaaagattcccttggatgatgggttaaaacaaataccggaacatgatagggtggtttttggccccaccagcctttccattcagcatctggccaggggcctcgaaccggtccaaacatattgcgccccattatccaggcgcctatattttccattgacttcttaacgaagtcatcatccacgccggtgttttcaacattactggtcctttcaaacatccaggtgtgaagttcttcgcccctgataccgagcggattttctacatcctgatgggctcctgcaccgaacccgtccagggaaaccgaaaatgcggctactttgaccttactcataacttatttttaagtatttcataacgatgcggtccgtggataaaatattcctgctagttgttcgtctactaatttacacatgtttttatctatatggccagaagacttttcctgatattattacttttcctgataggcgatacttatttctaccaggctgttattacacttacaccggatcccgttatccacctgagctactggctgattgatattttactgattgccgggattatatcggcgatatctatgctgagggcgcgtaagccggcgcagcgtctgctttccgggctaatgacggccatgctgctgattttcattccaaaattattctcttctcctattttgctggcagaagatatcctccgtttgttccggggcttcccgcctagaagcttttacatcagcgaggcggcgcttgcgctggccggcctgatttttcttatcatcgtttttggtgttacccgtggcaagcacttttacaagataagaaaggaaacgatctatttcccggacctccccgaggcatttgacggttttaccatcacccaaatatcggacttgcattccggaagcttcagcgatgctaaaggcgtacaaaagggacttgaccttgtaaattcccagaacagcgatttgctggtgtttacaggggatcttgtcaacaacatggcttcggaaatggatcgatggattcctatgtttacgaaactgaaggcgccttatgggaagtattccgtattgggtaaccacgactatggcgattatatcaggtgggacagtaatgcggctaaggaagccaaccttaaacgcctaaaggaaattcatgcggaaaccggctttaaattattgcttaatgaagcggtggaaataaacaagcagggagaacatgttgctctcatcggggtggagaactgggggaaaggcggttttcatcaatatggcgatctgaaaaaagcgaccgccagggtacatgataacgcttttaaaatcctgatgtcccatgacccatcccattgggatgaagtaacggtggaccatgaacaacatgtacatcttaccctggcggggcatacgcacggtatgcagtttggcattgaactgtttggtttcaaatggagtccgataaagtatttctacaagcaatgggctggcctttacaaacaggcgggtaaatatctctatgtaaacaggggctttggttttcacgggttaaaaggcaggattggcatatggcctgaaataacggtgcttaccctgaagcgggctggcgctgccttaatgcagtagtttgaagtgacgataactgtacggataatttagtatattagaatagcgtattctattttccgcgttaaccgttaatccgcttcgtccatgaaaaaaaaagcaccctatttgtttgcctggttatgccttgcactttgttccgcgtgtaaaaaaaataatcccgaaaagctggtgggccatcccctggctataggggctaatgaagtgactgaggcaaattttactatcgagaacaccttcaccaatccgctgataccacggggtgctgatccctgggtcacccaaaagaatgggatatattatttcatgtatacacaggggagcaaactggtgctttacaaaacaagcgccatgaccgaactggctttggcaactccgcatgatgcatggattcctccacagggcatgccgtattccaaaaacatctgggcgcccgagcttcatgaaattgataacaaatggtacatctattttgccgccgataacggcactaatgccaatcaccgtatgtacgtggtggaaaacagctccgccgatccaacgcagggatcctgggcattgaaaggaaaggttgctgattcgtcggatcaatgggcaatagacggaactgtttttaagcataacggacaaatgtatatgttatggtccggcggcaatgcgggcgctgcaccgcagcgtatctacatcgcccggatgagcaatccctggaccatcacgggcgcgaaagtagccatctccagccccacctactcctgggaaatgaatggcaatgccattaacgaggggccgcaggtgatcgtcaacccggacgggcgcctgttcattgtgtattcaggcagcggctactgggtggatacctattgcctgggattacttagtcttaacccgaacggtgatcccatgaacccggcggattgggtgaaaacatcaacgcccgttttttcaatgaacgccgatagtggtgcttttggtcccggtcataatggttttttcaaatcacccgacggtacggaagactggcttatctaccatgcgcgcagtgcggctggcgggggagcccggaatgcccggatacagcgctttacatggaaaacagatggcacgcctgatttcggggtaccggttaaaatcggctcgtttgtgcagaagccttccggtgaaccggtacggaagatgtataccaaagagaattggtcaattgccggattcagctcggaggagcttaacaacagcaggttggctatacgaataatagacgatgactcgtctacagtttggatagcccgctattccgcacccgccaccagctaccctgaccattggattgcagtagacatgggcgatacgcttgcagtagatgggtttgtttttatccagaagagtggcgaccggaaaataaaagagctgcagatactcgcgggcaatgataatcagaactgggaaaatttgggtaccgctgaactgcttaatctccatcctaataaacagtattttaatcttcccgccagaaagcatttcaggtattttaaactggtgccggtatcagggctcgacagtcagcctcaacccggcctggccgaagccggtacttttattattgataactaggcgaagttgaaattcatgtgtaacgttgtcgtttttttacaaacaggtaaaaacggtcgtttcttatctttacaaaaagcataagatctatggcagacacacattctgaaagcaaattaaaacacgagcaggtacagtatctcgaattcctgtcaaaagacatcagccgcgccaaagcattttataccaaaagttttggctggaagttcactgactacggtcccgactatacggcgtttgaaggggattatgtagatggaggattcaccaccggtaaaccggtgaaaggaactgtgttggttatcctttattcaaacaatattgaagcaacccagcaaaagattgtagcagcaggagggaccattgtaaaagacatcttcagcttccccggcggcaaacggttccatttcacggatcctgacgggtacgaactggcagtttggtctttgtaagcgtttgttccgttttgtacaattttaaagtttagggctatcctaattttacatcgtgaaacacaaaatcacctttaaactttaaaattatgaaacggaattttcgcggtataagtaaaatactcctcatcatgataaccgctacactgtggttatcccatgcaatggcagcgcccaatgatacggtactccgggtgttcagtcaaacattcccggatgcgaaatccacctcgtggatggaagatagcgagtattatattgtttccttcaccagaaacgatacgcaatgcaggatatggtatgataaagcaggcgcactggtttatgctttaaggtactgccaggagagtgaattgccgctgagcgtgctgctgacggtaaagaaagagtatcataataagcatatagaaggggttacagagcttaccaacaaaagcggcgttacatacgagcttttgctcagtgacaacaaaaagtggtatgtggttaattccacttctaacggtgacgtatatctgaaatatgcgatgaagaaacagccttagcagataaggtgttgtaccggaagcgcctcgcaggtttacctgcaaggcgcttttatgatttaacagaaatgaactgttttatctggccggcttggtggcactgaagccgctttcaccatgaaaccagcgaccagcctgaccggtaagccataaataatagtcggacgacagatctttttcaataccgacgaactttttatcgccatgtagtggcagttcgccttccctggcacacttgtaaatagcggtgccttcatctacttcgtcaaacatagctacgtataacgactgcgccccggatatccgtgcgcctgccacctgcttccataagaagtcgcctttcagccgcggaatggaattgtaggctgccacgtcgttctttaaattaccccagctgaagcccggaaacaccagcggcacataatctactttattcgtgttacaccactggatatcagccgccagctccgcgccggccacgttgttgtagctgttgttgtcgtaccggcctacggcccagggcataataatatcggaacgtttgatgagggaatgcagcagggaagaattttctgtatcatttttcagcgagcgccagtaataaggcacacccagcataatggataccttgttgccttttcctttgagctttgttaccagttgatctacattggcaatggtatacttcctgttatcattgaatcccacgccccagatggataacaacggtttgccgttgtgccttacataggaagggtgctttttattgtcgaagagggaaaataacgtttgcagttcattccagtcctgctcaatatacgccacatcttcactggtgcagccgctgaggtcatacatcacgcagatagcgcgctggtacttattggccgctttcagtgcattttccagcactttattgaaatgccgtttccctttcgggttggagtttttgatctccaccacaaaacgttgcatgaaaacgccgtcgatgccgtaatctttcatccatttaaagtgaaggtccacgctttcttcatcgtagggactgtacaaatatgcgtcggtgccatcggcgaagctgaaaggggatttatattttttcacatattcgcccatgtccggccagaaatcaattgcagaacaacctggcaaaaagccgccacagctgccattctgataatgataccatccgcggtcagacgcatcgcctgcggctgcaaaccagccctggtagccagccatcaccaggttcttgtaactcttgtacaaacaaccggtttcgtcatacactacattttccgtatctgatggaggacctggaggcggggtgtcaacttttttttcttttttggaacaaccgcaagccatgtaaagcgccaatacacaaaagagccaacttagttttttcataatatttatttttgagaacaacgattgatgaagtcccgcagggaggcggaacttcatcagtcgttataatgggttaaatatccagtcgaactgccgggcggtaattaggtttcgcttcaccggcatcaataagcgcacctacccggaaatagtatttgttgccgggtttcagtatagaactgttggcagccagatcaatctccagtgtatatacctgtgccggatcgcttaccgcatttaactgtatctcggaggccaccaggcgcataggttccccgacccttgcatcggaatgtgcatatagcccgattttctttacgttgttgatcacattctgttccagcttaaaggtagcggttaccttggtgccgttttttacaatatttacatccttcacacggatgtagggcgttaccgcaaaatcaagggttacctggccattgatgtttaccacctgcgaatccaccgggataaagttacccctcaccggtgtaacggtataggtgttggcaaagagcatggtgttggcgtaagtgccgtcggtttttacgatcagcggttgcggtgtgcgggaagcataaccatgttcaataatttcaatggtagtgcccaggatgatgtcctgttctatcagttcaccgcttttaacatcccggaagctgccggataatcctgcagtggggccatcgtagttatccttttcacaggacatcattcccagtgccagtgcggcgatgaagaaaaaatatcttagcttattcataatcatttttttagaatcacacattaatactgcgggttttggatcaagccatttgaaccgatacccggaataggtctgtaataggatttaggctggaatgttttggtattggtattaggtacgtttacgcggacgaagatgtatttcgtggccggtaatgcgcggaggtcccgtaatggtaacagcgagtgcagcatccggttattgaattcggtatgatactctcttctgcggatcaggtcccagaagcgtttgttttcaaatgccagctctacttttctttcccgctgtacgttagcggcggttaaggggatatctgtagtatgaccggcccttttacggatatcgttcagcgcctttacagcgatggacgcatcacctgttccgctttccacaacagcttccgcatagttgagtaatatttctgcgtacctgaagtcaataaagtcggtggtactctggttccatcccggtataataggcgcgttctgattcatgaattttttgaaagagaagcctgtgcgggtgttattgccgccgtaggtatcaaagccggaatacaggctggtgctggcggcgccgtatgtataataggtggtgccattgatggtgatgtgatcattggtgcggatcactgcggtgccatccggttttacgtaacctgcctgtatgatgatcgggatatttttccagagcgtagagggtaatatagcggttccccagaggcgggcatctttatttttaaagatgtcgttgggagaatcgaactggatatacgtcctggaagggttatagccgttatagtctgtcacgtttgcatctgtagaggtaacaacgggtgatgaatgaccgggattatcatagctttcgtaagtgtctacgagatccagcgtagggttcatcctgccgggatgcggccagccattggcgacctgggcgggctggtaccagatatcgtagttatgacccaggaatgcgccgggaagtgtatatccttttgcaaagatgacttccttatttccagggtcctggaacaggagccggtaattttctgctgctgcttcccggtttgccgggctagccgcatacagttcaaacttgttggcattcataatcgccagggaagcgcttttacaggcctcataataaccattggccagggaggcttcgagtcctatcagcttttcatttactgcttgtccggacataggcgccaggctgccgaattttgcaagcgaagcagcatgtaatgctactctcgacttcagcgcataagccgtccatttggaagctcttctgctcaccccatctccgaggttactgatcgcctgatcgcacaattccaaggtataatcccatgtttgctgttcggtgctcctgggcactttcaggctttctgcgtcaccggtatattgctgggatgctttaatgagcgatacgccgccatatctctttgccagggcgaaataagcgtatgctttaataaaggcgctttcgccaattaaagccgcacgttcctcttcacggatctttaatgttggaatggcatctatcaggaggtttacatcgcggatcagcttataagcgctctcccagcaattaaaatcaccgtcgccaacgaagtcgccgaactcggtatgcacggcttcatctgtagccatggcaggagcgaacccaccgttgttgggatctccgctgttccagttaaacccgttccggaaataggtaaagtcttccaccggtaactggtaatagagattggccatatatattttcaccccttccgggtcgccaaacagggcttctgcctggattttgtcggtaggcttcagatccagtactttattacagccggaaaagaggatgcctgtcaacagtataataaaagagaatttattggtagtcatgttgcgtgcttttagaagttgacgttgatcccgaaattgtaattcttcgtgaggggatagttgaagccggcgttgaagaggccttccagtctttcgggatcaaacgcttttacgaatggatctgcaatcgtgaagaggttgaagccgttggcatagatcctgatcttctggatgccgcttccacggagcaggttgggaccgaaggtgtatcccagttccaggctttttaacctgacataggaggcgtcttttctccacacggagctttccgcatacattttacctacgtcgccattgaatcgggaggctggccatttgcccggcacccattcgctgtttggatcatagggatctgccttatgccatctgtcgaagaagtaggcgggggtgttaccgcggaacgccagtatttctgcatacacttcgctgaaacgtacggtatacatggcagagccctgcagcagcaggttcaggtcgaagcctttgtaggcggcgccgatagaaagaccgtagtttattttcggatttttgccgcttggattttgattgtcgttgttacccacggcgccgatgaaagagggcgtcatatctttatcatccacaacgccatcattgttgagatcagcgtatttgaaatcaccgggcagctcacggatgttagcctgaccgccgttctgcaaaggccagttggcgatttcgtctaaattctggaactggcccaggtactggtatccccagatcacatcgttataccggtagtcgttaccatttctccatttgtcgtagctgttctggtaagcgcctctttctacatacagattttgtgcacggtagaagttgaagttggcagagatattataggagaattcaccgatgcggttgttgtgcgtgatggtaaactccacgccctgtacgcgatcgctgttcaggttttcttccggtaatcctgcgccaaaagtattgggcaatgatacatttctccgggcgggcagaccggtccgtgttttccggtaaacgtccgcttccagtccgagtttgttgttccataaaccgatatcgatgcccagatcggtggtagtgttggtagcccaggtgaggttgggattggtgataccgggagccgcggcgccgttggtaagaattccgtttgcaaattcatatcgtccaccgcctgaagtggagaatccctggatccattggaaaggctgaccggcatcttcgcccattttaccatgggaggcgcgtaacttcaggttggagatcgctggtatcttgtttttaagaaaaggttcttcagaaattctccagccgccggagatcaccgggaagaagccccatctactgttgctgggatacgcatagttgcccatgtaacggaaggcaaattctaccaggtatttggatttgtagtcgtaattgaaacggcccagcaacgactggtaggcagattgcccttcctggccggagttggtcatgccggcttctgaagcgccattgatctggtcggtggtataaaaggaatacagtcttctcaggtccgcattgcggctccaggattgctgctgctcaaatacgagggagctgccgatattatgggcgcgggcaatgctggtggaataattcagctgtgtttgtaacgtaagacggttaccattaccgtagccgttgctgatagcgccggcgcctacacgttgcggagccacgaggtattcgtcgtttacatacgtgtagagattataaggtttggatacgtctttaccctggtagctgttcatgtcataggctgccagtccttttaccgaaagtccctgcaggaaaggaaacgtgtaggtgagcgcgagggaagtctgcacactcctgttcacggtttcactgtagccggtggcgcctcgctgcgacagcagcagcggattctgattagaaggggttactaccgccgggtattcaggattgccgttggcatagggttgttccgtggggagggtaacgcgggtacctttaaagatgttgaagaagttttctcccggcgcttcttttttatcgtaccggccgccgatcaatacttctgctttcaggtttttggtgagctccgtagtgatattggaccgcaggttaaagcgttggtagttcaggtcgttactacgcagcaaaccgccttcctggaaatatcccaggcttacaaagtactgtgttttgtcggtgccgccggtggccgacaggttatgttgctgctgggtagcggctttcttcatggttacgtcgtaccaatcggtggtaccgtagcccggagccccatcgatgtatttttgtaactcttcttttgttacaaagggtgcgccggtacctaatacggctgcgtcgttgcgcatctgcatccactcggaggcactggccatgcggggtacgtctgtaggtttcatcatgcctacggtacctgaatagttgaaagcggtttttccctttgcgcccttcttcgtagttacgatgaccacgccgttgccggcgttgaacccgtagatggcggcggaagcatctttcaggaaggaaatgctttccacatcttccgggttgatacgctgaaattcggaggagccatctcttacaatgccatcaataacatatagcggcgttccgaagccacgtatattgatcatgttatcgaagttacccggctcgccgcctaactggcggaccatcaggccggctactttaccctggatcttttgcgcaaggctcacattggtggaggtttgtatttcccttgaagtgatattggacacagcgccggtaagggtttccttccgtttggtgccatatcccaccaccactacttctcccagctggtcttcgccggccgacaaactaacgttgatggtagtacgggcattgatcttttcgatggcgcctttcatgcccatgaaagaaaaggccagttccgtagcgcgggcatctacggtgatatggtagatccctgctgtattggtagtagcgccggaacggacaggagcattgtcgttcaccgttacgctcactcccggtatggggctgccatctttggcatccgttactttgccggtgatggtcctttgctgggccagcacacttaacggacagatacatattaaaaggaataggtagtagattcttttcataacgttactattgcattggataaatttgttttcgccagaaagtcgtcaggagaggagtgcctgatgattcttccgggattacggtggaaaaaaatgagtacaatacatcatatcaatacttgattttggttaatacgcgaaacaggaatatgctacctgatggcaggcaaggtgatatgcacaaacgaagctgaagtgtaaggatgttttctgatggctggcacgcaggagtaaaccaacacaaacaggtgtactgaaaggaatataagtcgcttcataatcgtggaatcgttttgctgcaataagctgctgcaataaatcggagagcttctaataaaccggttaatgaaccgactaactgaaaaattaattttctgtaagaatgataactagttggttttcactatattgtagtcgataaaaaataagacaaaaaatgggtcatcttcaatatttaaaaaaccgattattctttggattaattttataatattgcctcagggataatatgacaggaggatctgtggctgaaaacactgtgctgaaagcatcctggaggtagtttacctatgattatctctcatcaaccaaagtaaaagattaatttatcctgctggcgcaaaacagggcagatgctgtccgctggttaattgtttattgtaactgttcacgttgattaaaaattccgacattaattccaccagcgtattagccaggaaattattgtagtccttattagaatggatctaatgttaagatatatcttatgtatatgcggtgtgttgttagctggccacggggggtattgtcaatcacacggattgcagttccggagccatgaggtggtacaggagaaacggacatcccttcatctaacccccactgcccccatatgcctgcaacataacacggaaatatccttcgatcttacctttctgccttaccatgaaacttatttcgggtatatcatgcggctgattacccccaccaatcagagtatcgacctggtatataaccagcggctggcgaggttgaattttgttatcggggaaaactatataggggggtatgatatcgactctgctaaattattcgggaactggagccaggtccgtataagatttgatacagagcggcaggaagcttctttttatatgaatggccggctaatcagtaaaggcaaaggcaacttttccgccggtacctgttgcaatatctattttggcgccaacagttttgagggattccagatgctggatatccctcccatgaatatccgggatatcaggatcagtgaaaacgggcagctgacgcattatttccctttgtcagaagagaagggcaatgaagcccatgatgagatcgggaaaagggtggcccgcgtgggcaaccctgtttggatcagtcccaaacaccggaaatgggaaaaggcagtggactttgacacaaagggcgctgccagtattgccttcgacggtaagcgggaagtgctctatgtagtgtcggttgattccatttatgaattatcgttcagcaatatgcagctgaaaggcgaaagatttacccgcagccgtcacctgctgcctcccggcaaccagtccgtttttgatccggtaaataaccggttgtataatttttatgcagatgaaaaaaaggtaagcacattggatcctgccaaaccggagtgggacgttaactttaccacggattccctgaccgtattctggcaggtcaacaagttcctttctcccactgactcttccctatatgtgctgggcggctacgggcaactgcagtataaaaacctgttgcaacgctatcattttcccagtaaaacctgggaagtggttccctacggaggagaacgtcccatgccgcgttatctcaccgcacttggtatgaatgcggcaaaggataccgcgtatattataggtggctacggcagtaaatccggcgaccaggggatcaacccgcaatattgctacgacctgatggcttatagcatcagggaccggacctttcacccggtttttgaatttaaaaagccggaaagacaattctgttttgccaacagcatgatcaccataccggggaccaatgatttctatgcactcatttatccaacggataagttcaataccaccctgcagctgatcaaaggttccttaaactccccggaatatcagctgatgggagattccatcccttattccttttatgacatcgcctcttttgccgacttatattattgtccggttagtaaaaaactggtagccgtaaccttatacaattccaaagggaatgttaccaacgtgaaagtacatacgatctttttcccgccaaaccaggcaggcctgtgggcggccgttccggcaaccggcaggacttactggtggtacctgttgctgccacttgcggcagcgggtcttatattcctttattaccggagccggaaatctgctttcccaaaagccgcggagagtgccgtgccggctatggtgcctcctcccgtcagcagcagcgcagcgccggttgttcccgtaccggagccacccgccgctcctttgccggaggagaaccccgaaattgctgccatatttctttttggatccttcgaagtatttgatgccaacggtcaggatattacgcaacatttcaccccgctgctgaaagagcttttcctgttactgctcatttattcccttaaagacggaaaaggcatttctcccgaaaaactctatagtacgctatggccggataagttacagaaagacgccaaaaacaattactccgtaaacatcttaaaactgaaaaatctcctggaaaaagtaggcgactaccaggtagtaaaagaagcaggtaaatggcggcttgaaatactgaataactccatccgggtggattaccagcagtatatccagctggtgggcgcaaaggcgcctgttaaccgcgactggatattggaactgctgcgcatagcgggcaggggagcctttcttaaaacaagccagtacgaatggctggatcatatcaaagcagacgtttccaaccaggtgacggacgttatactatcttttattaaccatgctgatatgagtgcagatgcagagcttattgtgcggctcagcaactgcatcttctttttcgatacactgaatgaagaagcattggtgcataaaagcaaggcgttaatcctgctgggaaggcatggcaccgccaaagatgtttaccagcgctttgcaaaggaatacaaggaaagttacgggcaggattttgaaaggtcgttccaggaaattacggggcatccgcattgatacactactcccatccatgcaccagcgtcatcgtacaattttcagtagaacgccacctaatggcctttagcggctgatattccgggtcatggtaacattgcagcgcagctgcctccgacgggaatttaataatggcagtcatcttcttcaccgttccttctacagcgatggcttggaggtctgatgccagtacttccgcgccatatttatgcaataattgaactaccggcgggccatactttgcatattcttcttcattgatgatgtcgtagctattgatataatatacaggcatatgattttttatttgaaagatcagtaaacgtattcaggaggaacaataccctgtgtgcggagatagacagtcgcctgtccgcggtgatgcgtttgttaccgcaaaattaaccggaaggggaagcatctgtttaaggaaaattgctctctttaagaacgcatggcggagggtgattggccaaattgttttttataggcggcagagaaatgttcgaggctgttaaagcctgtggagaatgcaatgtcggttaccggtagccctgtgttgcaaagttgcagcgcagcttgtttgagccttacctgcagcaaataactgtagggagtggcggcggtgatctgtttaaaaagacggttaaaatgaaacgggctcatatttccctgcgctgcaagttgcggaagcgtaacattgtctgcatagttttcatggataaacgctttcaccttttctatcaccggcaggtaattccttttttgtttatcattcaatacgggcaggggatggcgcggatctccggcagacaacaccaggtggaaaagcgcggtcatcagctgctctgcccataaagaagggtagcgtgttttttgcagcaggctgaatatgcgctgatgcaggaactccatttccggcgtagcttttaccaggatggattggatgtcggggttattgaagaaccaggaaaagttggcagcatgttccatcaacaggccttcacttgcgggtgtaaaagaaaaaatggtgcattgatccggtatgttgtgcacgtgcgctacctggtgttcgtagccgggtttacagagcaggaaaagaccgctgtaagcatccagctcattcctgaaaacccggaagcggaagtttcctttccggatataagcaatggaaaatgtttcctggtattcttttgcagacacggaacattcctggcaccggcacagaaaattatgtacggtgcaaacgggagattgatagagtatttgaatatccgcctgcataatataaagttatcaaaaaaaagtgatcctgttacaggagaagccgttgtatttccttcatcagcgttttcttttctgcggttgattttgtaagatggatggcttgttgataatgcgcaaccgcttttgctgtattggtttccgcgtacagataacccagcagggaatgataatggctgttgttgtgtaagccaagtttttccgcttcctgtatgccggcggggtgtccgtaaacttttgcaaaggcaaaggttctgttcagtgcggtcataggagaatattcaattaatatcagctggttatacagctgcaggatatgcgtccatttattatgatcggtgggcgtggtatgccagtaggcgatgcctgcttcgaggtgatacttcgatatttcattgccggagcaggcatttacgaggtagtagttgccctgttggatgagttctttgctccacaggtttttatcctgttgctcatacagcacggtttctcctttgttgtctcttgcatccagcctggaactgtgaaagcacatcagtgccagcagtgcgttggattgagtggtgttggtgagcgggttttcggtgagtatcagcgccagcctgatggcttctgagcagaggtctttccggatgaggtgattattggatttagaaaagtatccctcattaaataaaagatagagggttcttaaaacaacgtccagtctttcttttatggttgcttcctgcagttgcctgatctggaagttgtcgttgcgcagattggcccttgcccggagcaatctttttttgatggtcgctgttttagaaagaaaggcatccgcaatttcttcgatgctgaatccgcacaggatctggagggcgaggcagacctgcgattcagtggagttagcgggattgcaaaccgcaaaaatcatggccagctggctgtcgctgatagtttgcggggtgaaatcaaagtcgggtgctatttgccattcgctggctgtaagagcgccttttacctgtgtttcgaagatggagagatgtttgagataatctttcgttttattttttgctacggtgtacagccaggcggtagggttttcaggggtgccctgcacgcgccatacttcggtggctttcagaaaggtttcgctcacaatgtcttcggctgtttccatatgcttcaagccaaaaagacggcataatacagccgtcattttggaatattccaacctgaataattgaggtaaaagctccgggtggggaggggtgcttgctgccatgggcgttagcttttctcttccggtctgagtatggcccttacttctacattgccgccggctttaagtaccgggttggcctgggcaaatgccaccgcttcttcaatattggctgcctttacaatcatatagccactgataaattctttgatttccgtgtaggggccgtctgttaccatatcgggcttcacggttttggcgtcgctggcggataaccggtttcctttatctgccagtttgttttgggcggcaataccagccagccagttcatcctttcctgtaactgttcgggagatgggttgtcgtgcgagttggtactgtttctgaaaattaacatgaattctttcattgcataatgttttatggtttcgttttagtaacgactgaatattcatgagggggacaaataacttcatttttttgtccgaaaaaaatattttccatccggtgtgcggattatgcatgctgttccatatcgtaccggtggagtcccggaccataagcatctttcgtgatgcgggtaaccacaaatccgagtttctcgaaaaaaggataaacgtgttgcgtagtgtcaagcctgatgctgcattgcgggcataccgaccggatcacctgtacgcggtacaggaataattgtctgccatatccctgtttatgtaatgcctgtgtgatgaggccccaggtcattgcagcttcctgttttgcagtatcgatataataacctccgcagccgattatctgttcctgcagggtggctacataatattgttcgttgttatttttttggggagatgcataccgtgcatcctgttcccggagccattcttcaaaatcgggtaattctgccggtgcaaaaaagccaggcatattacttttaaaagcagccatgcaggctggtttatcggagggcatatatggtctgatggtcatgctcattaacaacgataaaatgaataacgggaagttaagttttatataccagccggagaaaaaagaaccggaagcggagcggggcttttattgctgtcaacaaaaatataacaacaaaacacaggcatcttccggaattataaaaattaattgtcaaattgacgattaataaaatagttttattatttttcctgtcagaagtaagccggcgcacctgccaggcagctacaaaaattagtacgcgttatgaaaaagcatgtaagaaaagagatcctctttatgttctttattggcttgttgggtacacacctggcgggtgcacaaacgaagcacaaagccggcaaagctatttcccccgatctgttcggaattttttttgaagacatcagctatgcggcagatggcggcctgtatgcagaattaatccagaaccgttcgtttgagtatacaccggccgacaggcgggagtggcatgctttcacggcctgggaatacgtaacaaaaggcttcggctacggagcggtgaacgtggaaagtaaatcgccggttcatcccaataacccgcattatgtagtactcaccattgaggaacccggccaggaaggcatcgggctgcaaaacaacgggtttgatggcattgccatcaaaaaaggagaacagtataacttttctgtatttacccggctactgtcggcaactcctattccagtgtctgtgcagctgcgcggccggaaaggggaggtgtatggagaagtaagcatcacggcagatgcaaaggagtggaagaagagcagtggcgttcttaccgcacaacaaacagacgatagcgccgtgctggtactggtggccaaagcgaaaggcagcctggcgatagatatggtttccctgttcccggtaaatacttttcatggcagaacaaacgggctaagagccgatctcggacaggccatcgcggatctgaagcccaggttcatgcgcttcccgggaggttgcctcgtgcatggcgacggcctcgaaaacatgtaccgctggaaaaacactatcggtcctgtagaagaaagaaaagcacagcggaatatatggaactatcatcagtcgctcggacttggctacttcgagtacttccagttttgtgaagatattggcgccaaacccttaccggtagtacctgcggcggtgagctgccagaattccggcggcacctggcgcattggcggcaccgggcaaaagggattgccactggaagaaatgcccgcttatatcaatgaaatactggacctggttgaatatgccaatggaccagccacctccacctggggcgccaaaagggctgctgcaggtcatcctgcgccgttccacctggaatacctggccattggcaacgaggataaacaaacgcctgaattcagggagcgctttaaattaattgaagcggctgtaaaagaaaagcacccggaaattaccctgatcggaaccgtcggcccggctccggcaggagaagactttgaggcaggatgggcatttgccgacaaaaatgctttgcagatcgtagatgaacactattacgaaaaaccggagtggttcctggaaaataaaaaccgctacgattcctataaccgcaagaaatccaaagtatacctcggtgaatatgcttcaagaggaaacacctggttcaatgccttagcggaaggcgtatacatgaccgcgctggaacgcaacggcgacatcgtacggttatcttcctacgctccgctgctggcccgtaccggtcatacttcgtggaacccgaacctcatttatttcacgggcactacaatcacccgtacgcctaattattacgtacagcacctgttttcaaataatgccggcgatatctgctacccggatatcgttacgctgaataataataccaatacaggcgtatcttgcgtgaaagacagtaaaaccggtgatctcattattaaactggtgaatgccggtgaaaccggtgtatccgccaaagccaatgtggccggcctcgtagcccggcatacaaatgcagcagtaacggtacttacagaaaatgcaacggataaaaatgcgcccgcagttcaatctgctaccagtaatctcgaaattgacaaagtgattagttatgaagttgcgccccgctcggtggcgcttatccgtatcccggcgccgcgtagataagagcgggttttgtcttactcaggattacgctgattatactgattagctggatttttacttttggattttaagatttaataatatctaataataattaagggagataagagcgaatatccgcttctatctcccttaatcctttataaaatcaaaaaagtaaaaatccagctaatcagtataatcagcgtaatcctgagtaagacaacatccgcttattccaccggttgcagatactgcgcataggcatagccttcttcgcctgcatctgtgcggatcagccaccactgatcgctttgtttactgatcagcgaaacaatttcattgtgtgctgcttttcctacaacaggctggtcggtgccggggcccttgcggatattcaggttagttgattctgtgatcactttcagtttagcgcctgctacagcagtagctacattgatattcattactacgtcgccggtgaggaagttgggatcaatctttccgtagatgttccacagttggtcctttacggcgccggtaggtgcttctccttcgatatgcaatacgccatccagttcgtttactttcaggttgctggtgcctgcagcttgtgctgcatcaatcagctctttatatttatcctgtaatgctgccatgattattgtatttaaagagaaagattattttacttttaaaccggaagcatctacctttttaggcttcagggcatccagcgccattttcagttttttccaacggtctgctttctgttcgccggtaatagtaattactccgtctttaacatctgcctggataccagggaaatctttcacaatacttgctacggctgttttcagtgaatcgtcggcagtaacttctaccggtgcggctggcggcggcggaggaggggctacggtaacattgttaacaacactcttaacaccctggttcagcttaacagcagcttctgcggcatctttgtcagcctgggtggcaacagatccggaaagggttactacgccatccttcacatctgcactaacgccgggcgacgattgtaatgcagtggttactgcagcctgtatgtctgcatccttaggtttcgatttgcaggaaatcatgaacaatagtcccacggagaggatcactgtggtcaggtgtttcagtttcataatcatactgaggttttaatgatgaaaaaatactttcttaagttaagtatcttttttcatccggcaataagacggtaagagttgtttattttttaatacagacgtcccggtctctattaatgtgattttaattttgactgtcaggcgtattcaataatttaggcccagcaaaaaataatgcagtaaattccggacctatgaagaaatggtacctgttatcactcctgtgcatcctgctttgcacggcatctgcgcaacaaaatgatcagatagcgactcatttttttgagcagctcggtaaagggaactgggacggcgcaaaagaaaatatggatgccaccatgacggcaaaggtaacgccggacatgctgaaagggatctggcagcagatggaacagtcccatgggaagtgggaaactgttatctccctgaaaacagcaaaggaaggtgcatatgatatgatactggcggataacaggtttggcaaagccattatcacctttcgtgtggtgttcgacaccaatcaccggattgccggcttttttattgcaggtaccaaactcctgactaccgcactgttgccttatgaagaaacggatacggtgattactccggacggtggtatcctgtatggcgttcttacaaagcccgtggaaaaacaaccctggccggtggcattgatcatcgcaggttccgggccaactgatcataatggtaataatccattatcagcggctgccaacggtaactcttatcagcagctggcagcagctttagcggccaatggcattgcctctttgcgttacgataaacgcggcatcgggcaaagcaccggcttcaaaaaaagcagcagcgccacctcactcgacgattttacggatgatgccatcgcctggatagatcatctccaaaaaaatacgcagcaatttaaaagtgtggcagttattgggcatagcgaaggggctttaataggcctgatgtgtgccggccgcaggagctttaacagcctggtatcattatccggaccgggggaatgtatggataaagtattgctgacacagttaaggccaatgctggctgattcgttatatgatagggcgaccgtgattttaaatgaactccggcagggcaataatccgcagcaggtaccggcggtattaagcacgcttttcaatccttccctgtatactttctggaaaagtacttttcattatgatccctgtaccttgctacccgctgtaaaaatgccgttcttaattattggcggtaccagcgatacacaggtgccacctgtacaagccgatattctccatcactgtaagccgggttcgcagctgctgatgatcaaaggaatgacgcacgcgctgaaagacaccgcacccgttcccgcagggaataagacgccgttaccactgtcgccgcagctggtaccgtcgttggcagcgtttataaagcattagctataccggtcgtttctccaggggtaagcggtattggagtaacctctttcttcccagaagcccagcctgttggcagtgaggaattcaatgcgccgtatccacttggcgcctttccaggcatatagttcaggggtaatcattcttaccggtccgccatgttcttttggtaatggcgcgccttcaaatgtatgtaccagcagcacatccggtttcaatgcttcttccagtgacacgttggtggtgtaatcgtcgtatccgtaacagagtatatgcgtggccgtgtctttgggttgtaccagcgcggccaggtccagcaggcgaacgcccacccagttcatattcagcttcgaccaggtggtaacgcaatgaaagtccgaggtatcggatgtttgcggcagtgcgaggaaatcttcccaactcaaagtcaccgggtgttccacagcaccatcgaggacaagctgccattcttctttttcaatttccggctgtatgcccaggtccagtaccggccatttatgcgtgatggtttgtcctaccggtaatacgggcatgccatgccggttgggattgccgctgcctttgggtttattatcggctacagatggggtgagccgcatcttctcctcaaaacgggatttgagcttcattctcgcttctacgatacgctttagtttatccgcctcttccataaagtaatttttgggtctcagggcataaatatacggatttgcgcctatccgggcggtagggcctggtgtaccgggcgcggcattatctgaaaaaaagtaaccgtttggctatactttgttcatacaaagttgtatattgtacgaacaaagtaaacttaaataaaggcgcgttatggaggtcattcaaacggtattcaaggagatcatcgggttcctgggtatctcgcaactaatagaagtatgtaaaacggggaattataaggtgctgcttacgttaaacgggatcttctcggttatctcaccgctggtaccttttctgctgttgctggaaataggcagggctgttttttataagaaattcaagatcgaagactataaaatgcctttcctgatctttgtagccaaccggttcatttcccggttcatctctattgcggcagttgctttctgtatcgggttgctggagaaatatgcgttgatcaatacttcccttaaatggtactggtttatttatggatatgtgatctgggaattctctcactttatttaccattactatggacataaggtgcgtttattctggtgcctgcactctactcatcatgcgccgcaaaccatgaacctatcagttacttatgcgcacttcttcctggaagcgccctatgcagacgtaatccgcaccagtatctgcatcctcatgggcgtgaatccgccattgctttttatcattatgttcatcgacggcacctggggatctttcattcatgtgggtgaaaacctggttaaagacgggcgtcttggctttctcaataaaatcattctcacgccatcgcatcaccgggtgcatcacgcaaagaatcctttgtacatggataccaatttctgtaacctgctgaacatctgggacaaggtatttggcactttccagcatgaaaagagggatatgcagatcgaatatggtatttccagggaaatgaatcccaataatttcctggatgtttattttggtgaattgtacgggttgtggaaagatatacggaaagcgcctggcataaaaaacaagctgttgtacattgtaatgccgccgggatggagccatacaggggatcataaaaccgcgaaagtggtgaaacaggctttcctggaagaggtgcagcatcagcaaccattgcggcagcccacagcagatcaggtcatctgatcaaacaggtaatacagcggcgattcttcgagcaccacccgggaattcccctgcggtgcatcgtttttccatttgatcagccggatcgcgccatctgctatttcaatccccgtaatatcgccatcattgaaacagcaacagcccgtattgaaataagagggatgcgccattgtttttaccacctgtttaccggcatattctgcttgtctggctgctaatgctttttgtaagatggctatctcgccggtgtctccctgggcgcgggctttatccagttgtttcgtgagcttgtcgatatgatccagtgatgcaaataccggtttgtgggtgtgcccggaaatgaggaaggttttctcgtaccggatactccattcgtacatcatgatattgtggcggtcggccaggtcaaaggaatcggagagggtatccatccggatatcaaaaaagcgctgtacgggtgtccatatagcggctacaaaccatttactgaaagcattgccatcgctgcgcaggtcgccctggtggccatgtgtgagataaattctgtagtcgtggtcctggtagcgggtttgcaggataagtccttcataaactctcagtttcttcccgaagattcctttcagaaattgctgccggggtatggcataatgccattccaggtcatgattcccgaatatccggaaataacgttgctgctgcaggaaccgggcttcttccagcaatgtgtcgcggttttcccggatcacggtagccggcgtgcattcccacaattcctcgcaatcgcccaggttaataaatgtgtagcctttgtcgtagtaataacggagtgcagccacataattggcttctgcggccataaagtcgtccgcaccatctttacctcctttatgttgatcggagaaaataataaagcggctatgctcgtaatcaaaaggaacaatgagtcccttttgacggttgcctttgaggatttcctcgtgaagctgggatagggaggtaaatacctgggatttgtccggctgggaagaaaacctgtttgaaagccagataacaggacgctggaagaattttttcactggatgcggcacgctgtatttttttagaaaggtggctgagtaccttaccacgcacaaaaatgagcgattatcaataaccgctcagatttttttatttcaataaagccagacctgttacagtttagctttttacttctttctttacgttaaccgcacttggacctttctgtcctctctccacttcaaaagttaccttgtctttttctttaataagttcagtcagctggttaatgtgaacgaacacactatcctgtgtctgctgatcgataataaacccgtaacctttggactcattgaaaaatttcaccacacctctgcggatcagttctgctggttcctccggcaattgtctgcctggtccgagctgaatgtcttccacattgatttcccttttcctgcttggatcgggcggagtagaagagatattaccattctcatctatgtaagccatcatgtcttccagactctttccttttccgctttctctctttcgttcttcctttctttcctgtttatccagtctttgtttcgcttttttcttttctttttcttttttaccaactgtttcctgggatctagccatatttatgtatatattttgataccttacaaagatcggctttttttgcgtaaaaggcccggaatataaagcagcacagcctttatgcacaggtattttgccccaggactccccatagcggctattctatattttttgcacattgaaaataattcgcatcacgttgcagattatcatgatattttatttgtgaccaggggtaattatggtgtcatgggatttccatagattagcaaattggttttagtgcgcaacaaaattaaccacctggaagtggacccgtctaaaaaaatttaaaacgcttatgatgaagaaaacggccctggttttccttgctgctattgcaggaaaacaggcagtggcacaggtagacgccggcctgttccgctatcctgatgtatcccggtcgcagatcgcattttcctatgccaatgatatctggattgtcccgaaaacgggtggcactgccatcaaactgatttctccaccgggagtggaggccttcccgaaattttccccggatggcaacaaactcgctttcagcgccaactatgatggcaacgccgacgtatacgtattaccggtagccggcggggtaccgctgcgcctcacggaatacggcggcagcgaccgcgtagtggactggacacccgacggcaagcaggtgctttttgcctccggccgggaaagcacaaaagaacgcttcaaccagttctacaccatcccggaaaatggcggcgccgccaccaaactgccactggcctacgcagagtttggatcatggtcgcccgatggttccaaaatggccctggttactcgctcccagagcttccgcaactggaaaaggtaccgcggcggtatgaaagcagatatccatgtgtttgattttgccaaacaacaatcggaaaacatttccgcaaaaagtgacgcgggcgatgaatttcccatgtggcacaacaacttcatctacttcctgtccgaccgcggcgcagagaaaaggatgaacctctggcgttttgatgttaataccaaagcctgcgagcaaattaccagctacaaagactatgacgttcactttccctccctgggaccggatgatatcgtgtatgaagccaacggcaaattgtttctcctgtcgctgaacacacaacaatctaccgaggtgaaaattaatatcaccaccgacctcgcggcactgaaaccacgcacacaacgcactgctaaatatatccagtccaccgccattagccctgatggccagcgtgcgctgataagcgcccgcggcgatgttttctccgtacccgctgtaaacggctacgtgaaagatcttacccgcaccagcggtgtggcagaacgcttccctgtatgggcgccggatggcaaaaccatcgcctggtggagcgataaatcaggtgaatatgaactgtggctggctgccgccggtaaggaaaatgaggctaaacagatcacccattacggccccggcttccgctaccgcccgcactggtcgcccaacagcaaacaacttgcgtttatagaccacgacctgaaaatatgggtactggatgtgaccactggtaaaaccacggcggtcgacaaagcccttcactattcacccgatgtgctggatggcttccgtttcagctggactcccgacagcagatggcttacctatagccgcgacatggacaacggccatgaagccgtttttctcttcgatacaaaaaataaccagcgccaccaggtaaccagcggtttctatgatgccgcccggccggtgtttgacgaagaaggcaagtatctttatgtacttaccaaccagtcgttcaaacccacctacagcagtatcgacaatacctttatttacgccaacagcaccgtgatcggggttattggcctgcaaaaggaaacgccttccctgctggcaacccgcaatgatgcagtgaatgtagaggaagataaaaaggaaccggaaaagccggccgccaaaaaaggaaaagagaagaaggagaaacctgcgggcgataagaaagagacggccaccaacatcgacctggacaacatggaagccaggatggcactgctgccggtaccaggcggcaactactcccgcctcggcgccgtaaaaggcaaaatcctgtttgtgagcagcacaccacccagcgacgaggaaagcggcggtgaagccactttacaatactatgatatcgctaccaaacaggtaaaaaccatcatcaaagatccgggtcagtacgaactttccgccgatggcagtaaaatactggtcaataacgggccctatggcgtgatcgacgtggccgaaaatcagaagattgacaccgctatgcaggtggacgacatggaaatgaccgtgaacccggcagaagaatggaaacagctgtttatggacacctggcgcctggaacgcgatttcttctatgatccccatatgcacggcctgaactggaacagtgtaaaagataaatacctgcacctcctggaaggcgcccgcacccgcgaagaagtaagctttgtgattaatgaaatgctcggcgaaatgaatgcgtcgcatacgtataatttcggcggcgatattgaagatggcaagcatgaaaatgtaggctacctgggcgtggactggcaggcagatggtaaatactataaggttaaacgcatcatccgcggcgccgcatggaacgctgaagcccgtaacccgctggacgaacccggcgtaaacatccatgaaggagattatatcctggcagtaaacggtgagccgctcaccacggtgcaggagccgtacggcgcgtttcagtcgctcgcaggaaaagtagtggagatcacctggaatagccgcccttccctggaaggcgctaaaaccgcgatcgtaaaaaccatcggcagcgaataccgcctgcgccacctggcctggatagaaagtaaccgcaaacgtattgcggatgccaccaataaccaggttggatacatctttgtgccaagtaccggcatcgatggccaggatgaactgatccgccagtttaatggtcagtgggataaggcggcccttatcattgatgaacgcttcaataacggcgggcagattcccgatcgttttatagaaatgctgaaccgcaaaccgctggcttactgggctacccgtaacggtacgcccacacaatggccttcttacgcgcatttcggcccgaaggtgatgctgatcaacggctggagcggttccggcggggatgccttccctgattacttccgcaaggcaggactgggccccatcatcggtacccgcacctggggcggtttgatcggtatcagcaatacacccggcttaatcgacggcggcatcatcaccgtaccatccttccgcatgtttaataacgacggtacctggttccgcgaaggacacggcgtagatcctgatattgcggtagatgaaaatctcggcgatatggccaaaggcatcgatccgcagctggaacgggccatcaccgaaataaagaacctgctgcaaacaaagccttacaaggcgcctgcacagcctccttatgaagtgagataacggccttatataactgaccggtggctgtttgctttaactaaacagccaccggtttttttatttacgcggctgaaaattccatcgcagcccgccactgaaaaagtaattggtcgcaaaacgatgcatcggtttatccgcaaacatctcagataaattcttctccttaaaagtagcgccgctgtaaaggatactgccccccgacgccacaaaatcgatatgccggttcaggtgccaggtattctccagtcccacacttatttcagcataacccatcagccgttttttatccggcgcattctccacatcgtacgaagaaccgcgcatacggaatgccagcgccaggtccgtttgtttattcagactgctggatacacttattttctccgggaaattaacatctatcctgtacctgccggctgtttggtacttaatgagcaatgcaggcaatatcataggcgtgccaaaactattggtaagcatagcgcctataccataggagaaccgcttgttatgttgttttataaatattacgcccccgttaataaaaatatcttccccattgatctttttcatatcagtgaaaaccccggcagataacatactcagcatgccccaacggttaccgatactccggaaatgaaggagcgccagctgtgtttccagcagttcttccggaaagatccggtgatcataatcttcgctgaccagtttggtatagctgccggaagccgcgaggttccaggtacgcacctttccggtagcggtatccacctggttgctcagcataaatacagcgccgaaattataacgttgctgcgaagtagtggactttgttttcacactatcttccggcctgatataacgggagggtggtaagtaatccacgctgatcccgatgccgggaccattgagggaagtggcgcccagctgcgcccacaggcgttgcataggtgcaaaggcgaataaggcgagtaacaaacaggtatatattttcttttgctgcacgggctgtttatgtatgcgttgttgattcgtcatgagtgatatttattgctttagaggaagacaccatgcaccccatatacccctatgcctttaccggtatttattttcgggagataaaaaacacaattgccccatcccgtaaaatacaggcgtcattacaatgtcataattgggcggcagtatttccgtataaccattacagtaactaaattcaaggtataccacgtagaagagcgtacgaaaaaatctgtgagcccatttgtcttttttaaccaaacatacagtgcaatgaaaccaaaattatcgcttgcgttcgcattcggatgcctcaccctcgcgtcttgttcaaagaactattttgcctccggcgaatccccgaaagacagcctgtcacccgccaccgttaaagcttcaggcattacggatgttgccgtggcattggggagtaatgcctggttaacacaaagcagcgcaggcgctgcagaagtagtggtagactatggcctggccaactggaccagcagcagttccgtattcagcgcttactttcgcaccagcgctaccggcgcccttcacctcgcattgcgcggtaaagtaccgggtggcagcagccagctgaaaataaccgccgcgggccagtcgaaaactattaccgcctccggcggcaactaccacaccattgatgtgggcgattttaacctaacggataccggctatgtgaaagtcgatttccagggcgtatccaaaacaggcagctacttcgccgacctgtccgacctgtacatcagcggcgccgccaccagtggccggctcaactacattcaaaccgatgtatactggggcaggagaggtccctctgtacacctgggctatacgccgccggcaggtaaaaacgtggaatggttttataatgaagtaaccgtacccactggccaggacccggttggatcttactttatgtccaacggctttagccagggatattttggcatacaggtaaacagtactaccgaaagaagggtgttgttttcagtttggagtcctgccgatacagatgatcccaacagcatcccggattcactgaagattgaattactgcgcaaaggccccaatgtacaaacgggttcctttggcaacgaaggtgcaggcggacaaagttacctggtatacaactggcaggcgggaactacttatcgctttttaacgcatgctgtgccggtggccaataacaaaacggaattcacttcctggttttatgcccctgaaaccggcgcctggcaactgattgccagcttcagacgtccgcaaaccaatacatacctgaccgggttgtattctttcctggaaaatttctccaccgaaaccggttacatcggccggaaagcacagtacggcaatcagtgggcaagagataccaatggcacctggtatgagttaacaaaggcgcagtttacaggcgatgcaactgctgcatcccagtcgcgtatggactttgccggtggcgtggaatccacaaagttctacctgcgcaactgtggcttcttctctaactttgtaaaaatcaatacgccgcttacccgtacaccatcgggtactgcgccggtaattaattttaataccttaccataaacaaataaaaaggggctgtgactgcagccccttttttcaaacaatagtaaccctcaacgtggcggagtattatttacgctctccaccttatctttaatttcctttgaaggccggatgctcagcgcttttttccagaggatgttggcatttacagtatctttcctctccaggtaataatctcccatactatcatacgtattaaagctttccgggtaataatctatgttcagctgaaagaacattttagacttatcaaaatttttctgttgcaggtggtggtagccaaattcattaaaggtaggttcgtaggggcgtacccggtagcccatgtctttcgacaaaatatcgaaatgctgggtgataagtgtttttaacgaatccaccgggcagctgtcatcagtatagagataagtaggaaagcggtgatgaggaaacaggaatcttaatccgtcgtattctcccacgagcggtatcgagttatggtcatcatcttcataatatttataactccacctgagctggttaccggggaattttctcaggaaatcggttaagttaagaatagcgctggtatgaacggatccccgatcgttatcttttcttaattgtacagtatccagtccgggcttcatggtatgggccactgcgaggtagaggtttttacctttaaatgactgctgcaattgcctgctggctgttgcaagcacctggcctttattccaggaaatgctcggatctatggcaatataaccgttaaacaacgcaggatgatacaatagcgtgttcaccaccatcagtccgccgagggagtgtcctatcagcgtacggtagggggccgtggcgtattttttatcgatatagggaatgagttctttaccaaggaattcggtgaaagcctcgccaccgccggaacccggatacgcggagtcgcgtgtgggcgtaaggtcgcgcatccggttaccgccggtattcggaatgccaacaatgatcatccttggcagtgccgtattcccattaatggcgcttagctgcaggatcattgattgcagggaggagaagtgaaaatcaccgtccagcacatataccaccgggaacgccggctttgcagaatagctggtatccgccgaaggcgtatagatccataagggccttttttcttttagcacatcagaatatatgctatcgggttgcccgaaggaaaccaggctttggcttgtttgtgccatcacaccagcacgaccaccaccgcatagcaccaggaaggccaggaacaccagaaataccaggaatatttttttcataccgggttattatttcccgaaagatggaattttccgggcacgtatttccggagttgtgatgcaggcggggattaatgtgacggagtgggtgttttgcgtgacaaagcggattttgtcttggctcaggattacgctgattttattgatttaggggatttgaatactttggatttttaaatgattttgggagatataagcggatcttttataagatttttaaatgatttaagaagatataatcgatatacccgcttatatcttcttaaatcatttaaaaatccaaagtattcaaatcccctaaatcaataaaatcagcgtaatcctgagccaagacaacctccgctagaccttgcggaaaacgacgatgccgttatgtccgccgaagccgaaggtattgctcatggctacgttgaccgttttttctatggcggttcccagtacgatctgtaaggtggaagggatggcggcatccagttcctgtgtattgatagtgggagggatgatgcctttctgaatgctcatgacgctggcgatagcttctatggcgccggcggcgccaagcaggtggccggtcatggatttggtagcgctgatgtgcaggtgcgacggtgcggctccgaacattttgccgatggcagctatttcgctcaggtcgcccacgggggtggaggtggcgtgtgcattcaggtaatccacttcttctttattcagcccggcgtcttccaatgcgagctgcatagcccgcagggcgcccagtccttccggatgggtggcggtcatgtgataggcatcggcggtcatggctgcaccggctacttcggcgtaaatgtgtgcgcccctggctttggcatgttcatactcttccagtatgagtgctccggcgccttctcccatcacaaagccatcgcggtgcacgtcgaaaggacgcgaggcggtggtagggtcatcattgcgcaccgacatagctttcatggcacagaagccacctacagatgccgatgtaatgggcgcttcggagccaccggttacaattaccttcgccttacccaaacggatatacgttaacgcatccataatagcggtattggaagtggcgcaggccgataccgttgtataattaatgcccatcaggccatatttaatggagatcatgcctgatgccatattggtgatgagcttgggcacaaaataagggctgaaacggggattaaaatcgccggaaacatattcagtaacctgttcttcgaaggtttgcataccgccctggccggagccccagatcacaccggtatcaaaaggatccatggtactgaagtccaaccccgaatctttcactgcctggtcggccgctacgagcgcatactgcgtaaacgggtccgttttgcgcacttcgcctttgtcgagcaacgcgccggggtcaaagcctttcagctcgtgtgcaaactgtgtgcggaagcggctggcatcaaagtgactgatggtggcagcgccgcttttaccggtaacaagactattccagaaatcggtaacattgttaccaataggggatacggtacccattcctgttatgacaactcttttcatagctggttatttatgacgcagatcgtccaacagctgctccgcaatgtggcggaaagctgatggtcccatcaccctcgataaaagaagggaggcctgcaaattggatatgataatgagcgcacgcgtgttagcggcgcctttaaagtgaatgcgtttctttttccggccttcttcgaggcaccgggtaagccaggcgaggatgccgctggccatttcctgtactttcgcctgcatagccggttccagcgtctcaaaatccggggcgagagagcccatcaaacagatattgccttctttgctgtgccggcggaatacttccgtcagctttaccagttgttcttcttccggcaaacttttccacttgctcgtttgtgcgataaatttcgcaatgtcctggtctactatttccacgcccaggtcggctttcgccgggaaatgataatgcaccgccgcattttttatctccagcggtcctgaaatgtctttgtaactaaaggcgttaaatcctttggtcctcaccaggcggtcggccagcgccactattttatcttttgtttcagacatactttgccgtttgcggcacaaatatacttacttagtagtaagtaaacaaatgcacggcttttttgtaatttattggcttaaaaaaagcggggaggtttgatttcaaacttccccgccggaattacttatatgggcaacagtattactctgcctttaagctgttaatgggattcatcagtgccgcttttatactctggaagctgatcgtgagcagggcaatcagcatggcggccacaccggccagcacaaatacccagtaatgaatagagatgcggtaagggaatttctgcaaccactgatccatggtataccacgccaccgggaaggcaatcagcgcggcaatgcccaccagcttcaggaaatcggcagaaagcaggcgcgtaatgccggatacgctggcgccgagtaccttgcggatgcctatttctttggttctgcgctccgcggtatatgcggccagtccaaataaccccaggcagctgatcacaatagccagcgtggcaaacagccgggaaagctgctgcatcaacgtttcattggtaaacatctcgttaaactggtcgtccacaaactggtaagtaaatggataagccggattcaactccttcatcacatcgccgattttatgaagcgctgtttccttatctgtagccgcattcatgcgcacatacaggaggttggcgccatcaggaacacaatagaacactacaggatcaggtgagccatacatattaccataaacataatttttcactacaccggctacacgggaatgaatgacagaatcggcgctgaatggtgtgttaatagttttgcctacagcgcttcctttacccatcaactgttccaacgattcggtgatcagcacatccatgccattggcagcagccaccggtttaaaatcactgccggccactatcttcattccggtagtttgaatgaactcggggcttatgcgccgctgggaaacaaggattttatcagtaggcgattttccgctccagctgatatcgtcggtgttgttgccgccgtataaagtaacctggtccgccaatgcggcattttctatcacgccggtagccagcaaggctgttttaatagcggcaaagttttgcttcatcgttccctgaagctgcatggaaataagattatctttattaagaccgagattccgcttctttacatgctggatctgctggtaaatgatagccgtgcaaatgatgagcgtaatggaaacactgaactgcgcaatcaccaggcccttacggacaaaggcggcactgccggtcttcgacttaataccttttaacacaaaaaccgggttaaaggaagacaggtacagcgacggatagctgcctgccagtacgccgcaaatcagcgtaatccccagcaaccagataagatgcatcggttcattcagccccacgctgaggcgcttatctaccagcgcattaaatgcgggcagcaccaggaatagcagcagcaccgccatcaccgctgccagcatcgacataaacaatgcttcaccgataaattgcgtgatgagtctactttttcctgcacccactactttgcggatgcccacttcttttgcgcgtttttcactgcgcgcggtagataggttcatgaaattaatgcaggcaatgaataaaatgatccaggcaatcagggaaaacaaacggacatactctatgcggccaccactttgttttccgtcagtgaactggtcgcgcaaccgccagttgttcatactgaacaggaaggcctggttaatggcgccgggattgtgcgctgcaatgaagttttgaagtttatggttgatagcggtcagatctgcatggggagccagttcggcatatgtgtcaacagaattggcgccccagtttttcagataaggattttggttgaaaaagatctcaaaaggagctacccattcaaatttcagcgtggaattttccgggatatcttttattaccccggataccacgtatggctgcgcattatccaccgtaatggttttacccactacattctttgtgtcgccaaaaaatttccgggcggttttttcagtgaccacaatggagtataactgcggaaacggaacagccgcattgccttctgtaaaaggaagcgtgaaaatattaaagaggctggcatccacataaataccgccggcatacatttttttatctccgaacgtgaataacaggttggtcgtctgttctgaggtacggcaggtttgcgtaatacccggtatttctgtcttcatcgcatcggccagcagggcaggcgtagaggtaaatgtgcggatgttaccatcataattccagttttcccacacctggtatatcctgtcttttttcacgtgagagctgtcgtaggtaacttcatcttctacccataaaaaaattacaccggcgcagaccaggccaatggccagtccgaaaatattcagaaagctgtaggttttgtttttccagagatgtctgaatgagatcttaatataattttttagcatcatcatttgtacacatttgggagtagtgcgactagctccggccaagataatgccatagcattttatattgataatgagttatttggataattaaggttgtccgttttcacgggagaagtgttcatttccggacaggcagcagcacttattgccaggtggcagcaactatatgcccgggttcattgttaatttatcctggttcacacccccatttgcccggttcacctaaaaatattagttacggtgaacaagggaatttactttgccataaatataaatgtcgaccttatgaaacggtataaacaatggaaagtaatactgctggtggcgattggctgttttatcgccgtacagtttatccgcccgcgtattacccatccacccgttacaggcgaaccggatgttccgccggaagtcagcgctgtgttgcggaaggcctgctacgactgccactcaaatgaaacgcacctggcctggttcgaccagatttcacctgctatctggctggtggccggtcatatcacggaaggccggcgggtgcttaatttctccaactgggacagtataccgaaagaccagcgaaaaggaaaactgtttgaatccctcaaccagatgcagttcaatgtaatgccactgtcgcagtacacggccctccatcccgcggcacgccttacaaatgatgagatcagcatcctgaaaaactacctggccacacaacttgctcccctgaagccagacagtaataaaaccattgcggccaaccttcaatacgccgcctggcatccggacagccctgttgtaaaagtattgcccgtacctaacggcatcgcctatatgccggagtataagaactgggaagccatcagcagcacccagcgactggacaacggcaccatgcgggtcattaccgggaatgacatcgccgtgaaggccatccgggaacaccagaccaatccctggcccgacggtactgctttcgcaaaaatagcctgggatgaacttcctgatgccgccgggaacattactccgggggagtttaaacaggtagaatttatgatcaaagacagccataaatatgcttccaccaaaggctggggatgggcgcgctggaaaggaaccgcgctgaagccctatggtaaaaatgctatgttcaccatggaatgtgttaactgccaccaacctatgcgcaacaacgattttgtattcactacccctacgcagcacacggttgcctcactgccggatacgctgggcctgaagctaactgaatggaaggtgatcaccagcggtatccagaaagatcagaccatgagtaccctgtatggcaacgaacgggcagtagccagtgcaaggaaaagagcggccacttatccggcagatgccctgcttacattggtcacctggaaacagcaaccggacgatcattggtttggcgcagtcattccaggtatcgtggcatctgtagaacaggtgcagttccagccgggtaacatctcgccgttatataaaaaatataacggtagaaacctggtggccgacaaaaccagtgaagaggaaataaaaagcaggatcgcctacattacccgccagcgggcatctgtaatgccctaagaagttttctttgcttttttaagggctatcttgtatttatcaggggtaccggaaatgttgatgttcataaaacgcacctttttatctttatcccggtattcaatttcatccacctggtccacgttcacctcttcctgcttccggccaaaaagcgcctggaagcctacctgggtcaccatcttcatcgggatgcggaggtagtagttcatactcatgtccagcgactggttgcccgaaacctcaatatagccgagcgacgaattgatgttcatatttggaataacgagcgtgccgtttttcagggttagcttattgcgcagggtatcaaagcgtaccatgcggaggttcttatctttaaagtaaccggccatggcctgcataggaccaaaatccagcagggtgccattggtgatttcaatatccatctgcgattccgtttcactcagcaccggcgtaagatcgggatgcatgcgcacatagcttttgatattcccgctcagtatacctttcaggttgttgttgagcacaaagtcctgcccgaagttgtcgaacttgatgagcagtttggagatgtccacatttttgagatagataccgctccggaaatacagtttcttaggatcagctgcattgaacatgccacgcatggcaatatgtccgccggcaatattcatggcaatggtatctacctttattttctggtcttcccgcatatgaatattcgcaagcacatttttcagccacagctttttgtatttgatcttctttatatccacctgtgtttcaaattctgaaaaaggaatattgaatacattgaagccggtggcatgcagcgagtcgttttcttttacagtggtgcgccgcgcgggtgctgcgcctgccacgggatggtcgctgaaatcatagttcatcagttcatcaatatccagcatgtcagatttgaaccggaagtaattgctgcgttttaactggcgtttgcttttgccggtagcatagcgcatgttcaggttgaaatcggtgcggcctactttaccggtaagcgtatctaccacaataaagcggttattgccgtaccgtatacgcccggtcacattttccactttgataggatgttgtttcaatgtgccggaaatattggcgatgcgggcatctatccgtttaaaaacagtatcgtattttatgctcattttactccgcagccaaacgttgttggcttcttcataccaatatccctgcggaataaatttatggccgcgttcacttatcaggtcatttacagccaggcggtccgacttaaaatcgaatgccacttccgtgtttccttttttaattttatcaaaccagatgaggtagttatttaaccttcctttgagtgcaaagctggtgctgtcgatgtttccgctaaagttagacacccgtaaactggtgtcgttgatcatcactgccgcgttaaaatcatgcagggcgtgcgggtactgctggaatttggcgtacagcttttctaccttgaaggtgcctttgggcaaaggattgggatgcagtaattcttttaccgacgtttcaaacgccaggccgatattaaacccggtaattacttctttggataaaatgggatgagtagaatcaaatttgtacaattctcccagctgcaaacgcttgctggaagcgctgaaatttacggctaccggtttatcctgctggtgaaacagcgccggtacatcactgacggcgccctgcgccagtatatcggagctgcctatacgaaaagcaatggaatccagctgcagccgcccctgccgaatttgcgcatgcacattcatattgcgtaccggcaggtgatagccgggaatacggaattcaaggtttttaacagtgagctcactttgtacgccgtctttcagtttagctaaactttcttccggtatgcgcatatccactatttcccggaaattcatattcagcttgatttcaccgctgatctgttcaaggtctttgatgccgaggaactcgcccacgaagcgcaggttcagctcagaatataactgcatcaggatttgcggatcggtgaaatttttcatcacgaagttacctttgaatatgccgcttcccggtttggcgttgaagttcagtatatgcagttcggatgtttgcaggttatgcgcggcgccattggtataaaaccctttgaagccgagctggtctactttccggtcgatcttcttattctggaaccatacattttcgcagccaaaattaaattccattaaaggcatgatgcctttgccgatagcgcctttgataatgccatcgaaaaagacgcggccatcatgacggtatttatccagcatcacagccacgtttgccggcaccatggccagcaggaggttcagatccggtttatcgcctttaactttcaggtccacaaaatgttcgctgaccactccctgcagttgcagcgaggcctgttccagccggatagtaccgggaggcagggtcagttgtttttgctgcttgtcgtaaacagctgccagtttaaagttcagttgtttgtgccggaagagggtggtatcggatttcccggtgatgtctatttccagcttactgtccatatcgatggcgatatgggcggagtccatcgcgaaagctgtttttatcctatctatatgggtgttcactttcaggccggacatgccgtcgaaatagctgacgtcaatatttttcaggattattttcttcaggtccaggctcaggtcttcgctggagtcggccggcgcggcaggaccggtacttttgaattcatgggctttgatcaggtctacatcgccgttggcataacgggccacatgcacgcggccattggccagcacaataatgcgggcattgtagcgctgccggaggatatctggtaagctgaagcccacgtacaggcgttctacctggtacagtggctgtccctgcatttttttatctgcaaaaaaacgaacgtcgtgcagggcaatagaaatatatgggaagttgctgaatggagaaatactactttttgtgatgaccagctcccccgcaaactgcttattcaattccttcaccgccatctgcgtgagccgctcctgttgactgtataagataccgccggctattgtcatcaccaacaaaaaaacgcctgtgatgatcaggaatagcctgattactttttttccccgcttcatgtaaatgcctttctgaacgataaaattatgaaaaaatatagcagatatttttcatctcttaagaacggccagcgatttttattatttttaacgattcataaaatctggttacatgaaaagattgatagccctgttgttgctcgcaggaagtacgcatgttacaatggcccagcagaaaaagctggacaagttatccggaaaccccgtattcccgggctggtacgccgatccggaaggagtggtatttggtaaggaatactggatttatcctacctattctgccgcttacgaaaaacaggtgttcttcgacgctttctcgtcgcccgacctggttaactggacaaaacacccgcatatcctggataccgcttcggtgaagtgggccaaacgcgccgtatgggcgccgtccattatagaaatagcgaataagtattacctgttctttggcgccaacgacatacagaacaacgaggaaacaggcggcattggcgtggcggtggccgacaatcctgccggtccgtttaaagactatctcggcaaaccactggtggataagatcattaataaggcgcaacccatcgaccagtatgtatttcacgacagcgacgggaagtattacctgatctacggcggatggggacattgtaatattgcacagctgaaacccgatttaaccggcttcattccctttgcagacggcactacctttaaagaaatcactcccgaaaaatacgtggaaggacccaccatgttcaaaaaagatggtaagtactactttatgtggtctgaaggcggctggacaggccccgactacagcgtggcctacgccatcgctgattccccgatgggcccgttcaaaaggatcggcaaaatcctggaacaggacgccaccatcgccactggcgcaggtcatcactctgttatcggtattccggaggaaaaccgctggtatatagtgtaccaccgccgtccattaaccgaaaaagcggctaattcccgtgaaacctgtattgaccggatgtattttgataaagacggttatatcaaaccagtgaaaatcacccgcgaaggcgttaccaaagcggtgatccgctaaacatttccctattgcgtaaataaaattccggatacgattacattgccggtcttgcctgctccaattttgcaccatcaaaaaaagcaaaatatgatcaggcaaaccggcttagtttttttatttatcgtactccttttttcacccgtgtgcctgcgggcagaagaggagaatgctggtaccatcaggggaaaagtgatcaccacagatggtaagcctgccagtgatgtagtcatcctcttacaggaaacgaatgaaaccgcaatatcggaaacggatggatctttcgtgtttaaccgcataaaaccgggcagttatcacctcaccgtaacgctgatggggtacacccccatagaggaacaggtagtggtaaatgccgggaaaaccactaccatcaggttgcagctggccgttaccagcaaagccctgaaagaagtagtggtaaccggtaaccataataaactcatcaaaacctccagctacgatgtggcaaaaatgccgctgaaaaacctggaaaacccgcaggtatacagcaccatcacgaaagaactgttacagcagcaggtggtattttcagtggatgatgccctgaaaaatgcaccgggtcttacccgtatgtgggacgccacgggcagaggcggcgatggtggcggttattataacctccgcgggtttatcacccagagtaaattgcgcaatggcctggctggtaatgtgaccgctaaaattgatgcctataacctggagcaggtggaagtcatcaaaggaccgtctgccaccttgtttggtaacagtcttacttcctacggcggcctcattaaccgcgttaccaaaaaaccttacgatcatttcggcggagatgttacctacgcaatgggcagttacggttttaaccgcgtaagcgccgacgtaaatacgccgctggacaaggaaaaggacgtattactgagaatcaatacggcctataattacgaaggcagctggcaggattatggctttaacaaaaatttctccttcgcgccaagtttatcctatagggtcaacgaccgtctgtctttcctcttcgatgcagaatattccacgggacagaataccggtttgggtgtgtttttcttcccgtatatgcagcccatggctgatctgggcactaaccgcgccgatgagctgaagatagattacaaacgtgcctatgcaaagaatgacctgtaccagacttcccgtaataccaatattttcgggcaaatgaagtataagttgtctgaccagtggtccatgagcaccaacatcagctctaccaacagcttttcagatggtccttctccctatttttatctcctgtctgacgccgcggctaccggggtagctggcgccaaaggaagtaactatatttcgcgtaacgaccagtttaccgataacagcagggatcgtatcctggaaatacaacaaaactttaatggagattttaacatcggcagcctgagaaaccgtttcgttggcggattggattatttccatcataatgccgaccagttctttggtggcggtacctatgataccattccttctcacggcgatatccccacctattccaatttcaatcgccgtaacctggatacattgtacaataatcacggtttggcatttacgtttcctatccggaaccttaccaatacttacagtgcctatgtatcggatttgttgaacctgaccgataacctgataatcatggccgccctccgcgtggattattttgataacaagggcagttacaatgatgtaaaaggtatttatgaaggtggctacaaccaaaccgctttctctccaaaactgggtatcgtgtatgagcctttaaaggacaggatctccatattcggtaattatcagaacgggtttactaaccaggtaggcaccagtgctgcggggaaagcgtttaaaccggagcaggccaaccagctggaaggaggtgtgaaattacagttgttgaatggccgtattaacagtacgctcagttactataatatcaaagtaaaagatgtactccgtccggatatggcgaaccccaatttctctgtacaggatggaacgcaggtgagtaaaggatttgaggcagaagtaattgccaatcctttccagggctttaacattgtggctggttttgcttataatgattccaaatatgaggccgctgctaaagaggtggaaggaatgcgtcccggtactgctggcgcgccttcagtagctaacctgtggctcagttatcgtatatccgccggcgtagccgacggtcttggttttggttttggcggtaattatgccagcgacaataaaatagtgaacgacagaacggtcggtacttttatattgccatcgtacaccgtgttaaacggtagtattttctacgatcaaccccgtttccgcgtggcggttaaaatggataacattacggataagcattactggattggctatactactgtaaatccacagaagctgagaagctttaccggaagtttgtcgtttaaattttaataagaaaagcctgggcggtgtagcctcacagtccgggctttttcagttatgctgccacaccagcgcgacgatcctcctgtatttcgtagtggtgaaagcgtaattttttacgataataaacaaataccactgtagccacggcgcccgccaaacctgctacaaataccgttaaccgcggacctataaaatgtgccagcagcccggtgagcaaactgcccacgggaataatgccctgaaaagccatgatataataactgatagcccttgcgcgcatggtgggaatagcgtgtgtttgaatgtaagtattaatagacgcggtttgcgccatcatacccacaccggaaagcgccataaataccagtgccagcggcaaccagcccgacagcgacaacaatagtacgctgagcgaaaaaataagactggcagtaatgaggagctttacaagatcctttcccggctttagtttggccatgtaaatggctgcggcaatagacccaagaccagcagcactttcaaaccagctgaatgttttggcgtcgccattgaaaatgtctttggcaaataccggcatcagggtattgaagggaatcacaaacaggctgctggctgaaagcatgagcaggagcgacgataagtctttatcaccggcgatataatgaaaaccctcttttagttcggcccatatgctccggtccgaccggagaaccggcggcagtacaattttcatcatccataaagagatcagcaccggcacatagctcaggaagttgctgacaaagcagatatcttccccgaaagtactcaggataatccctgccagcgcaggccctgcgatgcgggcaaaattagacatcgtggaattcagcgcaatggcgttggggaggtcttcccttttttctaccatttccaccatcagcgattgccggcaggtaacatcaaaggcgttgataacgccttgtaccagcgatagtaagatgatgcccggaatattatagtaacgcaacaggatcatgagcgccaatgcgcctgcctgcagcatggaaatgatttgggtgatcatcaggatccggtaacggttgtggcgatcgatataactgccggcgtatggcgacaggagcagggaaggaattaagcttacaaaactcactacccccagcagcactgccgagttggtgaggcggtataccagccagcatacggctgttttctgcatccaggtacctataagtgaaactgattgtccgtagaagaataaccggaaattccgggattttaaagcacgaaaagcatccatttagaaatcatatttagggtattgatccgttattgaactggtgcaaatttcggtaagtgaagtatatttgttaaatagattgttttaatgatattgattgataaaaacgattagtgcatggaactccgtcaactgatgtatttcgtgaaggccgcagaaatggcgcattttacagaagcggcagcggcgctgtacattacccagtctactttatcgcaacagatcaagcagctggaaaatgaactgggcatgttattgttcgaccggatcggcaagcatgttcacctcacagaggcaggcggggttttcctgctgcatgcccggcaaatcctgctcgacgtggagaaaggcaaacaggcgatccaggatttgcagaatatgctgagcggcgaattacgtataggcgttacgtatgcctttacctcgttcctgttgccggcgctggccactttcccggtaaaatatcccggcatcaaaatattcgtggagtatggtactactgaacagctggagaataagctaagagcgtctgaactggacctggtactggcttttcaccaggatgcgttttacaaagacctcgaaactcgtgagctgttccgttcccggattgtagtggcggtgtctaaaaagaacaagctggcaggattaaaaaagatcaacctgcaaagtttaaatggtatggatttgatctttgcctcgcggggtttcagcgcccgtgattcgctggacgaagtgttacagaagaataaaattcagccttcggtgaagattgaaatgaatgatgtgcattctattttatcattggtggagaaaggacattgggctacgctacttaacgaaagggccttgctgggatggaaaaacctggtggccattcctattgaaggaaaggagttacaacgccgggcatatatcatctggcaaaaagaaacgtatcacaaaaaagcggcagatctgtttataaaggaattactgaaggagttgccgcccacagggaagtaaggcggcgccatatggcactcagcagcaacataagtgctgccgccgggtgaccacaggtaaggggttattgtgcggttcgcagttctgcgatattgcatttataatatttttcaaatacatctgacagttcttcccatccgctgtattgggtgagactggcaatatgcgtgagtgtacggtcggtttcaataagcattttaaatacaaatgccattttttcctgcaggatcagttcttccacagtgatgaggaattcctgttcaaatggtgcttccaggaattcggacgctacgctaaaccggtcgcagagcgcttccttgcaggtcgcttccgccggatgatgaataatataattggctatttcccgcagcttttcgcggtagtgttccatcagcatcagcgagggagggccttgcaggtaacggagataggtagcgtaaaagtcgatggcattacgccggaagaaaacgtctgccgtttcgcccactgctttgaagctgcggatccggtgcatgatctggtagttgacttcattaagatgataaggagcttttttaacgggctgtttgtctgcagccggttctttcagattcaacaccttgaacaggggaaattcagagaccaggtgtttcgccgacggcaggtgcagatttacgtgaaagttgatcgtaaattccttttctgtgatcagggtggtggtgtgagtggcgccttcccgggtattcatttcctttttgcccggtttcatcttcatgggaaaagccgccgcattttcagcaaaaccggaaatacaaacaggcagacaggcgttgtccggcgctaccgtggtaagttccacgccctgtttcagatgaaccagggcgtagtggacagacagttcattgagcgctatctcctgatccatgatcaccccgttttcatcaatatcggcaaagcatttggcattagggatcagttgcgactgcaggtagccgggaacctgttcgtaagtggtgcaaactcttttccccggattgatcagcaggtacttggttttcggttgactcatggttaatttcctttgatattgcctgttatttgaaatgcaatgtactatccgcggtaaaataataatcggtatttgtagtggcttttataccttccaggaggaagcctatcggtgtatttttatccagcaaaccggtgaaggttctgctggcaaggtcaggatgatccagggtagcgcgaacgccgtaccaccggaagatggcattacatatttcatccaggtgggtatcagaaaagcagtaaagccctttctgccagcccagttctacagtagcgttaaaaggttgtgtatccagggtagcggcctctttgttgaagatagcctgctgtccgggtttcatagtaacggtttttttaccggctttcatccgcacttttccgtctaccagggatactttcaccatgccactgtcgtagctgttgatattaaagctggtacccagtacttccacggtgctgttgggaagatgtacgaggaaaggtttaccggcgcgcttcgcgatattcaggtatgcttccccgttcagggtaatttccctgtcggcccccttaaaggtagccgggaaatccatggtggtagcagcattgagcgtaattacggaaccatccgggagggctacttcatagcttttgccgtgcggtactatcaatgagtgaatgccttgcggcaggtcgtctgatgcgttgagataaagggtattgtttttattgggaatcgttttaccgccaatagttacgttgccggctgattgggtcaggttgatggtgggctggccggtgatttccagcagcacatctttattgatggtggccaccggcgctggtttgggcgaggcgaaaaagtcccatttccaggccgaaaatgctacaagggccattaccactgctgcggctgcccagggaagtatggtgcggtacagtggctttttctgcttaaagtcaatcacttccagccacggggcaggaggggctgggatctgcatcatggaaagttgttcccacttctcccttactacttcgtcttcttcgataagttcttccagcaattggtcatctgctgcggaaattcttcccgcaagcttttccgtcattagcctgtatatttcttctgcgctgttcatgtacactattaaccgtttatttaatctggcggggtattaaaaaaggattttttttaaggatgcccttaaagttttcagcgcgttggctacctgtttttttacagtttcttcagtggtgtccatgaaggctgctatttcttttcgcgttttatgttcctggtaagccagccggaatgccatcgactggcgttccggaagctgactgatggcggtttccagctgctctttcagctcgttgttttccagcctgcttggaggaatcgtgtaggtttcaggcagcatgatttcctttaaccttttgttcctggtggcatctttggcaattttattcaaacagcggttacgtacgctgacaaagagaaagtttttgagagaaccggtggcgctcaggtctatccgcgcgctcaggtccttttgccagaagtcgacaaaaaagtcctggaccagctcctgggcctcggtttcgtttctgagtattgtgtatgcagtcatatacaaccattgacggtagctctcataaaaatactggaaagcggaaacactgcccgatttcagttgtgcaagcaattcaatatcgttgatagatgcactcatgctgggatttagttgataatcgcaggcctggcaacggctgctgttgtcaaatggttactgatacgcggttaggaaatacgtcagacagggcaggaaacagcatggctattttaagcaatgaggaaaaaccacccgtaagacaactgattttgatacaataacatgcacactacagaatatattcgatcagggggtatgggcggatttttaattagaagtaaagtttgttaatgaattgttattccgtcatttccggaagctgtctcaggtgtttgaaacaggaataggcaggggagcaggaggaggaaaacggagttattctgtgcagtctgcacaaaataacccgcctttactatttctttttggcgccccttttcttgggtttgccatatttcagcatcatcttttctttgtgggtcacctttttgttggtcttcatatttttagccagcttctggtgaaaagcagggcctacgtcttcccgcttgggcgcctttaccagcgtattccgcatatgtaccttcggtttttcatcttccgttaagacatcagaaattaccaagtcgtccggtaatggctgcacgggaatggcataattcatcaggctttctatccgcgccaggtcttctgtttctgcgtctttggtaaacaggatagaaattcctttcttatcagctctaccggttctgcctatacgatgaatatagttttccggtacttccggcgtatcaaagttgatcacatgcgttacctctgcaatatccagtccgcgggcaatgatgtctgtagcaatcaggaaacggtattcgttctgctgaaatttacggacagtattaaaacggtgattctgttccttgttggagtgaataatgcctacctggccggggaattccttctccagctgctcatgcagatcatccgccagttgtttggtggcggcgaaaatgagggttttggtcatggttttatcgtccgtgatcagcatttccaggaggttcacctttgtataaaagttgggaaccctgtatacgatctggtcgatgttttccagtggggtaccggtaggcgctgcttctattcttaccgggttattaaaatgtgtttcaatcattttctccacgtcttccgtaatggtagcggaaaacataaggttctgccgctttggaggcaacaggtccatgatatttcttaactgggtccggaaaccgaggttcagcatttcatctacctcatcaataataagacgctttaccagtttcactttcaaggcgccgctaaggataacgtcgtacaggcgcccgggggtagccacgagaatatccagtttgtcctgcaccgcctccatctgaggattcatattcacgccgccataaatgcccagcactgacacattcatgtaggtagtgagctttttaacggattccaccacctgtactaccagttcccgggtaggtacaatgatcagtacagtgggatatttttctttcgaaaatttaaactgccgtaatgtgggcaacaggtaagcgaaagttttaccggtacctgtttgcgcaatcccgcacacatcctgtccggacatgataacggaaaaggcgcgctgttgtatggtggtaggtcttttataacctaattcgtctatcgcgtttaataatggggtattcaggtttaaatcaccaaaagtcatgatactactataatatgaaccgcaaaggtaaagaattaccaattatggatttgccctttgtaattcttatttcaatacattagcataaaaaaagctatgaaaaacctccacataccggctattagtgttcaagcatatggaggccctgagcagttgcaactgcacgaggtgcccgttccggtgccggcagaagaccaggtgctgatcaaagtggtagccagcggtgtaaacccgattgactggaaaataagagaaggatttatgaaacatccgttgccctatatcccgggtgtagaagcctccggtattatcactgcagtaggcgagagtgtattcggcaaaaaaatcggcgatgaggtatatggttctgtagatggctcctatgccgcttatgccattgcgcagggcgaaggtttattccgtaagccacccggcatatcatttgaggaagcagctaccatggccggcgccagaacggcctggggcgcattgtttgatgtggccggcctcgtaaagggacaacgcattcttattcatgcaggcgcaggcggagtggggcatttcgccgtacaaatggcctataatgcaggcgcatatgtaattgccacggccagtgcagagaatctggatttcgttacctcgctgggcaccaatgaagtaattgattataaggctgcgccatttgaaacccaggtagcgccggtcgatattgtatttgatactgttggcggagataccacggaaagatcgctggcggtgcttaaacccgaaggcgtattattgtgtatcgtgcaaatgcctgacgaggagaaggtggctgcggcaggcgtccgcgcgctgtggggtggcaccaaaacactcgcttccatgaaggaggtgcatcaattgctggataaaggattgatccggccttacgtccgcaaagtatttcattccctgtcggccgccgctgaagcacaggaatacagtaaaaacggtggtagcggaaggggaaaaatagtactgaagatagcggaagaataaacgtcagccggggtcatcctccggctgatggtattatttgccgagtatttttttccggtgctgaatgccccatttctgcagggcaatgatcacactgtccagtgtagccgcataaggcgttaaggtatattctaccgatacaggctgtgtatcgtacacagttcgcttcaccagcttatgcgtttccaggtctttcagctctttggaaagcaccttcgacgttattttaggaatgctgcgctctatatcccggaaacgtttatgaccccgggaaacagcgatgataatgggcagtttccattttccgctgatcacatccagcgcgtcccttaccggcataatcactttatggcaatcggtatgagcactgctttccgccccgggtctgccacaatctatcgtgagttcttctgttttcatctgcatacagttggttaccttttgtaaagcacttactttaaggaaactggttactttctgatagcaaatatattaactttgttggtggaacttaaatttaaattaatgaaagtagaaatatggtctgatatcatgtgtccgttttgctacatcggcaaacggagatttgaagcagcactggagaaatttccggggaaagacgacatcacggtggaatggaaaagcttccagctgaacccttccctcaaatcgcagccgggaaaagatgtatatgactatgtagcagaaatgaaggggcagtcgcgcgaatggtcgttaaccgtacacgaacaactggccggtaccgcccgtgaagcgggtcttacctataattttgataaagcagttatcgccaattcttttgatgcccaccgccttattcagctggcgaaacagcagggcctcggcgatgcagcagaagaacgcctgttttatgcctattttacggaaggtaaagatgtgagcgaccatgccaccctgctggaactgggcctggaaatcgggctggataaagctactgtggaggctgtactggaaacatcagaaatggccgccgcagtgagcaaggatgtggacgaagcgcaacaactgggaatccggggtgttccgttttttgtactggaccgcaaatacggcgtgtcaggcgcgcaaccggtagacgctttcacacaaacactggaacaggcgtttgcagaatggaaaagcacacagctggtaactacactggataccttatcaggccaggtttgtacgccggacggagattgtcaatagtttgattttttataaggtaattggctggtcgatttttatagacgggcgactgtaataaatagaaatggcgcaggagattaaatcctgcgccatttctatttattgatttaattataaagacttcaatatcgtcataaagatatgcgcttgctccctggttttaataacctggttgagtgagcttacccctccggactttagggtaaccttgattttctgatcttcacattgctttgctttgagaagaagagcatctattttttttctggtttctttgtccataatgttaaagatatgaaaataaaataaattgatgaaataatggtcttagggctgatatagtttgaaaatgaagtaattatacagcttttcatatgtaagcgtaatctctttttgaatggacttgggtagtgttaatatgtcctccggatcaattggatgggatgaatcttcatccctttctttgcgcaaaattcttgcgtaataattaactccgaagattcggaaataccgggtgagaaaatcgtagttgttttgaatacagcgaaaatacatataagcccgggcattgtttgaaccatcaattcccagaaaacatgattgtttcctttccagaaatgtcaatgctgccagcactacagttgaaaataccctggaatggtgttggtgattgagtttaatccggtcatcaatttctccgttactattaatgggcccgaatgataaattatagacatcgggaatcaaaggatgaactgtatccgaaatatgaatgcctatttttgcagtattaccatctttcagacaagtttcaaagcaacaaagactaaaatccggctttagtatttccgtttcataacaatcgttaaaatttatctttaaatttagtgccattactttccttttctgcaagaaatcaaatttttacttcccaactgttaatcccacccaaacacgatcatcctgattcattattatcctcgcatttcttcttagctttacacctcaaatatccatttatggcgcttctgaaaagaatcaaccctttttccaggcaaaacgacgacaccggctttggtactaatgcaaatggctatggcggccggtttattaaccgcgacggaagctttaacatccgccgggaaggccgttcgtttatgcaacgttttaatatttatcacgccttattaagtgtacccgcctggcagtttgccctggtgatcctgcttttttatttctccattaacctcctgtataccggtatttactggtggataggcacggaaggatttcaggggattatcggtaaaaccggctgggaaaggtttaaagaagtcttctttttcagtacagaaacctttactacggtaggatatggccgtgttaacccggtgggcgacggcatcaactttgtagctgccattgaagcaatgacaggcttcctctctttcgcagtcgctacgggtcttatctatggccgcttttcaaagccacgcgcacacctgttgttcagcgatcatgcgctgattgctccttacaaggataaaacggccctgatgttccgcttcgcttcttacaaagaaaatcataccctcaccaacgtggaagtgctggtaacagcgggtgtccaggtgcaggaaaacggggaggccgtgtacaagttttataacctggccctggaacgaagcaaaattgaaacactgtcgatgaactggaccgtggtgcatcctatcgacgaaaacagccccttcctcgggtttacggcacaggatatggaagtggccgatgcggaaatttatgtaacggtaagaggctttaatgatgtgtattccaatacggtattgcaacgcacgtcttacacctaccaggaaattatttataacaggaaatttataccgatgtaccgggaaagtgataacgggaaaacaactgtgctggagctgcaccacctgaataaaacaaaagaattgaaatagtttatacccggatgcagtgatcatcactgcatccggatcatatcattagtctttacgggaaatcagcaataatcccaggaaagtaaacagcccgttgatgatcagcagttccagtcctatctggaatttaccaaaaatatgcgactggtagagatccaccaccaggcaaagcaacggcgcagctacgcaaacaaccggcaccagcgcatcctgcactttgcgtttggttaaaatgccaaaggcaaaaagtcccagcagcggtccataggtataagtagctactttcaggataacgcctatcatgctttggttattcacccattcaaataccatcacaaaaagaaggaagataaacgccatcatcaggtgaatacgctgacggtactttttcttttctgcttcggaccagtcggtgcgcttttgcatgtccaggatgtcgatgcagagcgaagaggtgagggccgtcatagcgccgtcggcactggggaacaacgctgagataagcgcaatgatgaagatcactgaaactaccggtggcatatgatgcaatgccagttccgggaataacttatcgccggtggctgttacctgttgctgtgcgccgtataaatgaagcaaaccacccaggaagaggaacaggccaattacgattaccataataaaagccagcgataccatgttcttcttggaatcttttaaagtttttacagagatgtttttctgcatcatctcctggtcaagaccggtcatggtgatggtgatgaatgcacccgccacaatctgctttatgaaaaagagtttgtcgtttggatcggtgttaaaaatttttgtcagccctctttcacccatggcggtgaagctttcaccgaggctaaggttcatggtatgcaggatataacctacacaaattaccagtccggccagcatacaggttgtttgcagggtgtcggtatatacaattgtttttacgccgccctcataggtatacagcaatatcataaataagatgatgatggtcgttaaccagaagggcacgccaaaactggagaggatggcgtcctgcagtattctcaccaccaggtatagccttgcggtagcaccgagtgtacgggaaaggataaagaaggaggccccggttttataggagcttcttccaaagcggctgtcgaggtaattatagatagaagttaactgcagccggtaataaagcggtatcagcacataggcaatcgtaatgtacccgataaaataacccagggtgatctgcatataggaaaaggcgtcgcgccccaccgcgccgggcacacttacaaaagtaaccccgctcagtgaggtgcctatcattccaaaggccaccagcatccagttactgttgcggttaccgatgaaaaaggagtcgttgttggagttccggcctgtataccaggcaactaccagcaaaatgataaagtaggcaatgacgaatgagaataataatcctggagacataaatcaaaaatcaaatttaatcaagatactactttcccgctaaggaacaaaaggacaaaaggacaaaaggacaaaggtaatcagtatatccctccaatcctgaaaaacacaaaatccgcttagatctccccgaatcatttaaaatccgcttagatctccccgaatcatttaaaatccaaagtgatcaaatcccccaaatcagtataatcagcgtaatcctgagaaagacaaactccgctcaagttacttgacaaaagcaaattaattatttgcttttgtcaagtaattatctacttttgcctggaaaacaagtaactatgactgtcgaatccccggttgtaggcgatatccgccgctttaaccgtttctataccggcatgatcgggttgctgaaccagcatatcctggacagtaacctgtcgctctccgaagtgagggttttatttgaaataggacagcttggaaaatgtaccgccgggcaattgattgccatcctgaagattgatggcgggtacctcagccgcctgctgaaaaaatttgaaaagaatgggtggctgaacaggcagcagtctaccgccgacggacgtacgttttttctttacctcagtgctgccggtaaaaaaatgctggccggcctggaagataaatctaaccgggagatcaggcagatcaccaatcatctctccgaaaaacaacaacaccaggtagccggcgctatgaaaaccattgaacaggtattgtctgcgcagccgggtgagcaaacttcggatatccatatccgttataacctgctgccgggggatgtaggctacctcatttacctgcacgggcagctgtatgcaagggaatcaggatataacctggagtttgaggcatatgtttgtaagacattctatgaatttcttcctgcctataacccggccaaagacaggatgttccttgctactgtaaacgatcagattgttggttcagtggccatcctgggatcttcccgccacctggcgcaattgcggtggttccttatccatcccgacttccggggcaaaggactgggaaagaaactgctgcaggaggccattgccttctgtaaggaaaaacattatcagaaagtatacctgatgaccaccagcatgcaggaaaccgccattgccctgtataagaatgccggcttccgcaaaacgggcgaaaaatatctgcagctgtggggacagcaactgtatgaacagcgttacgatatggatttattttaagcatacgcaaggtatgcccggattctttccccgttatgcatatttatgcagcagtacgatctgccccaggtgatacgcgtcatgttccgccagcccctgtaaataataaatggccttgttttctgttccgggaaaggtgtcaaacaattctttctccgggaacttccggatggtagcggctatttgctcaaaggaatgggtcagccggtgaatagtagcctgccagttttcttccccatggttctccggcatataaaaatcaggcaggtcgccatcctgctccggcgcttcattgtgcatatatcgctgcacccgctggtgccagaatattacatgattgacaatctcccagatgttattggattctccgaatgattttaccgcctgccgggcgtcaatgcgcgaaagatgttcctggaaagtaacatcgatccagggggtgccattgtaaagattttcaagcgatacggctaaatgctccagtaataaagacatacaataggatttttattttaaaagatatccggcttcaaacaccggtagccttcccgttaatcgtaatttactgaattctttcccttatttttaaagaatataaaaaccatcgttatggatcagcagcaattggaaaccaacaaaaatgaagatgctatgcggatggcaatcagcaccatgaaacaacgcctgggcgtaatagaacagggcggaggaaagaaaagcctggagaaagtgagacaaagaggtaagctcactgccagggaacgcattcaatacctcatcgataaagagaccccctttaccgaaatcggcgcatttgctgcctacgacatgtacgaagaatatggcggatgccccgcagcaggtaccgtaggaggaattggatatgtaagcggccggcaatgtatgattgtagccaacgacatgaccgtaaaggccggggcctggttccccatgaccggcaaaaagaacctgcgcctccaggaaatcgccatggaaaaccggctgccggtaatttacctggtcgacagcgccggcgtattccttcccatgcaggatgaaatattccccgacaaagaacactttggccgcatcttccgcaacaacgcccgcatgagcgccatgggtatcacacaaattgcggcggtaatgggcagctgcgtggccggaggagcttacctgcccatcatgagcgatgaagtgctcatggtagaaggcaatggctccattttcctcgcgggtccttacctcgtaaaggccgccatcggggaagacgcagatgcggaaacgttaggaggcgccgttacccatactgagatctccggcatcgccgattataaattcaagtctgatgaggaatgcctcgaccagataaaacgcattgtaagcaaactgggtcataccggtaatgccggcttcgaccggatagcgccgcagccaccggcaaagcccgccgatgaactggacagcgtgctgccggccgacagtacccggccctatgatatgctggaagtaatagaccgtattgtagatgccaacacactcgaccaatacaaacaggactacggcaaaagcatcatctgcggctatgcacgtatcgatggctgggcagtaggcattgttgccaaccaacgtaaaatcgtaaaaagtaaaaaaggcgaaatgcaaatgggcggcgttatctacaacgacagcgccgataaagcagcccgcttcatcatgaactgcaaccagaaaaaaattccgctggtattcctccaggacgtaacaggattcatggtaggcagcagaagcgaacattccggtattatcaaagatggggcaaaactggtgaatgccgttgctaattccgtggtgccaaaaattactatcatcgttggtaattcatatggcgcgggcaactatgcgatgtgcggcaaagcctatgatccacgctttatatatgcctggccatccgctaaaattgcggtgatgggaggagagcaggccgccaaaacattattgcagatccaggtggcttcgctgaaagcaaaaggacaggtgatcaccccggaagaagaagcccgcctgctgaaagaaattaccgataaatattacgcacaaaccactccttactacgccgcttccaggttatgggtagatgatatcattgatcccgccgatacccggataagaattgcagaaggtattaaagctgccaacaacgcaccggtggatcagccttttagtgtaggcgtattccaggtgtaaagaacggaggggaaagtgttcgatcccctccgcacttttccttatcttcgcgcttctttaaaattgaacatggctgaactggtagtatatacagatggtgcatcccgcggtaatcccggtccgggtgggtatggcgtggtgcttatatggggaaatgtcaggaaagaattatcccagggataccgcaaaaccaccaacaacaggatggaactgctggctgttattgttgcactggaagcactgaagaaagatggcgtaaccgtcaccatttttaccgacagtaaatatgtggtggatagtattgagaaaggatggttatggggctgggtaaaaattaattttaaagataaaaaaaataaagacctctggttacgctttatccccttgtttaaaagacaccaggtaaaaatgcaatgggtgaaaggccatgccagcaaccctttcaataaccgttgtgatgaactggccacacaggccgccgacagcggtaactggctgattgatgaaggttttgaaaacggattggcttaaagaataacacactccttaccgaaccaaccggcaatcataattgtaatataagcgcaaacttatattccgatggtgctctcctggttcacagatacgttgcagaaataccccgaaatagcagtgatgctaacccttctgacaggcttcctgataggcagggtacatataaaaggctttacactcggcactgttacaggtgttttattagtgggcattgccatcggaagctttcacatcaatataccctcagaaacaaaatctattttctttctcttctttttgttttgtaccggctatggtatcggtccgcagtttttccagggacttaaaaaagacggattgccattggcgctgttctcctttatagtatgctgcagcagtttgctattttgctggggattggcctccctgctgcgttttgaaacaggtaccactgcggggttaatgtccggcgccaatacctgttccgccattattggggtggcgtcaaataccatcggtgaacttaatattaccgacgatgaaaagaatacgctcatcaaccagatcccggtcgcttatgcagtcacctatatttttggtaccgccggtaccagctggttcctttctgtaatagggccgtggtttatgtctggcagccgtgcaaagctcatcgaagaaaccagggaaatggaagcgaaagtagcagaggccggtgcagaaggagaggagaatattaccaatgcctacgaccaggtggctttccgcgcttacctcgttagtgcagaacttaccgttgatggcaaaaccatccgtgaaatagaaaacctacttcacgacaagaaaaggttcctctatattttacgggtaagacgggaaggaaagctcatggaaacttcccctgattttataataaagccgggagatattattgcagtcagtggccagcgtgcagcggccattgcgtcagtatctttgttgggaaaagaagtagccgatgaggaactgctcacgttcccggtacagtcaataacattgatcattaccagcaaggacgccaataataagccgctgaaagcattttcaaaacatcccgaatttcatggtatcagcgtgcgtaaaattctgcgttccggtatggagatgccactgcatgcatctactgttatacagaaaggagatatggtagaattggtgggcatccaggaagaccttgataaggcggttgcgttgttaggttataaggaaagcagtggggtggaaacagatattgtttatctcgcagcaggcattgtggccggtactttatttggcagtttgagcatacatattggcagtgtgcctgtagagctgagtaccagtggcggggcgctgatagcaggtcttgttttcggctggatgcgtggtattcatccccggtttggttacatcccggctgcctcgcaatgggtgctgaccaaactggggctgcatgtatttattgccattgttgggctgagcgccagtgaaggatttttgcagggattgaaagaagaaggggtcactcttttcctggccggtgtggtgctaagcctgctgccaatggtgctggcactgttcctggcgaagtatgtatttaaatttcacccggccattggtctcggggcctgcgcgggagcgcatgatgaatcagcaccactgctggccatacaggatgccatcaacagcaaagtgcccgcactgggatataccgtggcatatgcagtagcgaatattacactcactacctccggcgtcatcatcgtgctgctgatgcataaaggcagttgatgttccccgctcatcacattttttaacaatgaaatccacgtctgtactgaaaacctgctctgatgaaaaatcttttcctcaacatttttaacaattcttttgtttttaattatgaaagcatatagctttgcgtcccattagtctataggaattataggataatagaacggaataatttaaagaattgcttatggagaatattacccaaccatattgtttaagcaactattgttgttgccatcattaagacgtaagaaatatttgtctgcttaaccacagcaggttacaacgatcaataactgtttccggaactccgtctgtaccggcgttaaaaacaatgggatacaaaactgcaatgcctgttcaataacagacaggggcaggtattgccaggaaaaaccagatcactgcaaaactctcaacattttactatgttacaacgactactcctctttctactgcttattggacccatggcagtatttgcacaaacacgtacggtgaccggtcgtgtttattccgcgaaagataattcgcccttaccgggtgcttcggtggtgattaaaggcactaccagcggcacggtgagtgatcctgaaggtaacttcagtctccaggtaactgatccggccgctactacgctcgtgatccgctacattggcctggaacaacaggaagtacccatcagcacatctcccatcaatgtatcgctccgttctttggggaaagacattgatgaaattgtagtggtagcttatggtactgctaaaaagagttcctacaccggttctgtctcgcaaattaaaagtgaggaactggtaaacaggcaggtatccagcgttaccaaagcattacaggggcttgcagctggtgtgcaaagcacgtctaccagcggtcagccgggctctgatgccaccatccgcatccgcggtatcggctccatcaacgcgtccgccgatccgttatacgtggtagacggtgtgccttacggaggcagcctgaatgcgatcaacccctacgacattgaatccatcagtgtactgaaagatgctgcctccagcgcgctgtacggctcccgtggcgccaatggcgtggtgattattactacgaagaaaggcaagaagcagggaagtaatatagacgttcgcgttagtcagggtttttcaaaaagagcggtcgataactacgaccgggtaagcaccgatcagtattttgaaatgtactgggaagccatccgtaacggtggcctcaccagtggcttatcgcccgctaccgcagccacccaggccagcagtagtcttatcagaagggtagggattaacccctatggcaccgcgtttccgcagcctgttggcaccgacggcaaactggtagccggcgctaaagccctgtgggacgataactgggacgatgccatgcaaagaaccgggaaacgtaccgaagcagatgtggccctcagcggcgctaccgaaaaatcgaggtactatgtttccgggggatacctgaatgaccagggtatttatcttgcttccggtttcaaacgctataacctccgcagcaatattgatattgatgccaagaaatggttgaaggtaggactgaacctgaatggtacgcactccgaacaggatgcacctccttcagaagacagccgctctgataactatgtaaactatggccgcctgatgtcaaatttctatcctatttatgagcgcgaccgggccaccggcgcctatatcctggatgccaacggcaataagatctttgactatggcagttaccgccccagcgctgccaatacaaacaccaacctggtggccacatccgctatcgataaacaccgccttacccgcgatgacttatcggcccgcctgtacggcgaagccaccatctggcgcggacttaaattcaaatcaagttacaacgccgattataccgccaaacaacaatatgattatacaaacccaaccctgggctttgatgcagaagtgggcggaacagtagaacggttgaacacccgcgtattcagctggacgttcaacaacatcttcacctacgaagaaacatttaatgaaaagcatcacctgaacctgctggcaggccaggaagcttataaatacaccactacctttttagatggtcagaaatccggcttctccctgccaggactggaagagctgtcggatgcctctctcatcaaggatctgcagggatatactgatacgtacacgctctccagcttcctgggcagggctgaatacgactatgtagggaaatatttcttatcggcttccctgcgccgcgacggatcttcccgtttcgcacccaatcaccgctggggtactttctggtccgtgggcgcatcctggaaattaacagaggaaagtattcttaagaatagttcctggcttaacctgctaacactccgcgccagctacggcggacaaggcaacgataacctcggtgatgacgcattttacaactactacccgctgctgaatgtaaacagcaaccttggtgaaggtggtacctatcgtcgccaggtatacaatccgaacctgcaatgggaaaccaatctgaacctgaacgttggtgtggatttcagcatgtttgaaaaccgtttgggcggtaccatagagtacttccagcgcaaatcacaggacctgttgtattccaggcctatggcgccttcagtaggttactcggcggtagatgaaaatatcggcgcactgaaaaataccggggtggaaggttccatacacgcagtgccggtgaaaacaaaagatttcagctggtccattgacctgaacgctactcactataagaataagattacggagctgccgcagaaagaaattatcagcggcaccaagaaactcatggtaggtaaatctatctatgatttttacctgagaaaatgggcaggtgtaaaccaggaaacaggtttgccaatgtggtacatcgataatgcagatggcaccaaaggtactaccggcaactattcttcggctacacagtattataacggttcctccctgccggatgtatacggcggtttcaccaacacatttacctacaagggattttcattgtcgttcctgatggtgtacagtcttggtggtaaagtactggaccaggattacctgttcctgctgggtaccgggacctccgcaggccgccctttcagcacggaaatgctgaaccgctggacgcccaccaacaaggtaacggatgtgcctaaactcactaccgtacaaaccaactggacatccgtttccgaccggttcctgtacgatgccagctacgcccgcctgaagagcctgaacatcagctataaccttcctaaatcattaatggataaagcacatcttaataacgtactcgtatatgtgcagggagaaaacctgttcacgatctataaccaccagggcctggatccggaacaatcagtaggaggtactacctactatcgttacccggccatcaaatccatttctgcaggtattaatctgagcttctaaaaattacgaccatgaaaaagaatatattcttaataataatcgcagctttggtattaggcgcctgcaacaaggacttcctggataccaaaccaaccaatgccgtacccgacgaccaggtgtttaatactgccgacaacgtggaaacggtgatcaacggtacctgggcatatatgtttgaagaattcttcacctttgcagtgccaggttataaatccattcatctcaccagcgacgccatgggcagcgatgtagcggtaacgcaatcgtatggcctgcgtgattcgtatggatatactgaaatgacggacaatacgaaaaaccgggtaaatgctttctggaccattctttacaaggtgatcgacaactgtaataatgtaatcgcgaaagtagataatgccaccggcgacgaggacaaaaagaaacgtcttaaaggccaggcatacgccctgcgcgccaattgctacctcacgctcgcatctttttaccagtttaacagaaccgggacagaaaaagccatcccgatctacacggaaccatccggcccggccactgcaggaaaggcaaaatcaaccgtagcagaagtatacaaacaggtaatcgacgacctgcagaaagcgctgccgctgttacagaattatcaacgcaacgctacccagaaatggaaaattgatctcaatgtagccaatggcttactggcccgtgcttacctttacaaccgccaatggacaagcgctgtcaccgctgccgtagcggcccgcaatggttatcccctgatgtcgggcgatgattataacaaaggattcagcgatatcaataatggggagtggatctggggacatgcacaaacgcctaatcaaagcaatgccagctataacttccatttcctggatgtttccagcccggcctcttactaccagagctttatggcagatccttactttaagaatttctttgatagtgcagacgtacgtttccgtttattcgactgggataccctgcctgaccaggaaggctacctgcgctataaaaaattccgtttccgtgatgccggcgcactggtgggcgacctggtactgatgcgctccgcagaaatgtacctgattgaagcagaagcctatgcccaaagcggcaacactgtcaaaggtgcggaagccctcaatgtattgcgtgcagcgcgcaacgctacgctttataaaggcggcggcagcctggtggataccatcctggtggaaagaaggaaagagttgtggggagaaggattttcattgtctgatattattcgtacaggcggtaccgtagtaaggaagccattcctttcttataacgggcaggatagcatcatcagtgtgccaagaggcgatggtacctttgtagaagtgcctgcacaggggcatcttacactgaaacaaccggatggaacaccgtttgtgccatacagtaaatattacctctttgccattccaattacggagttgcagaacaatccgaatatcaataattaaagcatataaaaaagcccccggaatttccgggggctttttttatgcttctatatttttatcgtaaaaagaaattgctaatagatccagggaataacccggctggtatgtttcatatagttggtgtattcttctccaaactgttcgctcagtactttttcttctatgttcatccggtaagcaaatgctataaaaaccgggatgaacacgatggctaatcccagccagttgttctgcgataacccgaatcccaggaaagataacagggaaccggcataggagggatgccgtaatatgctgtacagtccatcctttttaatgtgatggtctttccggatcgttacatttacggtgaacaacctgcccagctgcgcaatggccacaaagcgaaacaccattcccagcagtataacgctaaggcctatacgattcatatccgggccgggaagaatagggtaagctgtttttgcagataccaatacggaaatattgatgaacacaatgatcacgatccagataaacgccaggctgccctggtcctttttcttcttgtcttctttgtccttgccgcggagaatgcggtgcagcagaatctcagacaggaaccaggcaaaatagataatagtggatagcacgttcatatgcaaataaataagacgggttatattggtaatatatgttatattttctgattttcaaaaagtcgtaatttgtgattggaattaaaacttgtgctatggaaaaccttcaggcaatactcgcttcatcaaccccggtactgatcgattgttttgccacctggtgtggtccctgccagatggtgccgcctatcctgaaagaagtaaaggataaaatgggggaacagatcaggatcatcaagatagatatagacagaaaccagcaactggccgctcaatggcagattgccagcgtacctactttgttgcttttccgggaagggaaactgatctggcggcagagtggggtagtgccagcacaccagctgataccgctgctaaagcaaaagatataatcttcattacttcatggatacttcatccatgcctaaaacctgcgtatactatggaccatccatgcacttctcatgcacttctcatggactcctcatgcactatccatgcactatccatgcactatctatacactatgtcccttaaatcctgttgtaaaaactctgcagatcccctgccagctgatcataaataggccgggtaaattccataaataagtctgtaggcggcggtggcggcatatcccgtcctcccatcagctgcttgtcctcatcgctgagggccctttcgtcgcctttaaaggtaccaaactggttgagccaggtatagctgccggggatgcggtcggtgcgcagtaattgcccgttgccggtattggtgatgcggtaatccagtaaccctttcgataccaccgtttttttagtgataaaaagtgtggccttcaccgttttgtagatattgaactccttaccggtggagtctttcgtggtaccaaccacaatttcttttgaaacatcgcgctggatacggtctacatatgtttgacctaccacgaagtcaaaaaagcgcagttcaatatattcatcggggcggagattttcattacgaaccacccgttcgtcgtaaaactgcacaaattggttgatactgcgctgctgaaggttgcgcaccaggtagtcgcggaactgatcggcgctgaactggtaataaggtgagcgtacttcaatttcactgaccaccacattgatcacgcccatctggtaagcctcatcccgccgttgcttggtatcccggtaatcggggatcagcttcagtgcggcattaaattcatcaaaggccaggcgtgcactggctttatcgcctctatccagcaaagccatgccccggtcgtatcgcatttctgcggcgttttcctgggcgccggtgatcgcatcgcggtagtccttcggctgcaccagtttaagtgccgccggggagctgtgaatggcattgtagagcgtttgcaaagccctgtactcattccgtatattttcccacttgagttgattattagagcgaaggtatccgttaacgcggtcttcccgcaccagttgcgcctgtttataggcgtccggcagcatccgcgtggcggtggcatcctgcggtttacgttgcagcttttttacaaaagcggtaaccgcttcgtcgtatctgcctttattgtataatttttcacctgatttacaggagagaatacaggtgtagagaaggatggcggtaatgctcagtaacggcctgaatgctagttttttcaatggggaactgttttataaggatatgctttgcctgccggggctatgtttatttaaattgtcgtctgagctccctgtctgcttccctggccttgatagagtcgcgtttgtcgtgaagctttttacctttaccgataccaatttccatttttgccaggctcttatcggtaataaacatgcgaagtggtacaatggtgtagccacgttctttcatcttgttttccatctttctcagttcccgcttggtaagcagcagcttgcgttcccgcagcggatcatgattggaggaggtaccatgcgagtattctgcgatgtgcaggctcttcacgtataattctcctttggaaaaatagcagaaagaatcattaaagctcaccttgccggcgcggatcgatttgatctccgtacccagcaataccatcccggcaataaatttatcttctattgcgtactcaaaatatgccgatctgttctttaactctgccatttgcgctttaatatgggctgttagtttttagccttcaattgttagcagatgcaggaaagatccatgcccgtactaacaattgaaggctaaaagctgtttttctaatttttgaagatggtcagcaaacctgccaaccttgtcttaagttcttttctatccatgatgaaatccaggaagccatgttccagcaggaactcagcgctctggaaaccagcggggaggtcttttttaatcgtttctttaatgatcctgggacctgcaaacccgatgagcgcgcctggttcagcaatgttgaggtcgcccagcattgcgtaagaggcggttacaccaccggtggtggggtcagtcattaaagagatgtaggggagtcttgcatccgccagctgcgtgagcttggccgatgttttcgccatctgcatcagggagaaggcactttccatcatacgggcgcctcctgatttggagatgaccatcagcggcatcttgtgcagtatgcagtagtcgatagaacgggctatcttttcacctactacagagcccatagaacccccgataaagttaaaatccatacaggctactaccaggtcgtttcccagcaccttgccggctcctacggtcatcgcgtctttcagcccggatttcttctgcgcatccttcagcctgtcggcgtaaggtttcagatccttgaatcccaggaagtcggtcgggtatatatttgggaacagttcctcgaactgattgttatcaaatatgatctcaaaatactctgcagagttaatacggttgtgataattacacttatcgcaaacatagtaatgctctttcagatcctttacggtggtggtttttttacagttaggacacttgtgccacaaaccatccggtgcttctttcttttcactggtggtggtagagatgccttgtttaattcgcttaaaccagcttgacatattttactattagattagaaaatagtggtgcaagatacgaattatcgcataaagccaaaaacatatagggaaaagtataaagtttaagtcaaaaagcaaaaagccattgtagcggagataataacatatacatataatatatgatcacttttatctccgttacaacagctttttgcctttatatcttaagctgaatgcttaattatgcgttcctgttaatacagttcagatccctgaatgcttcttccaggcgcttaacaaaggtttcttcgcctttgcgcagccatacgcgcggatcgtagtattttttatttggcttgtcagcaccttcggggttacccagctgtccctgcaggtaatctttcttggcttcgtagaaatcgtgaataccttcccagaatgcccactgcatatcggtatcgatgttcattttgataacgccgtaacccagtgcttctgtgatctggtgctttggagaaccgctaccaccgtggaatacatagtaaacaggtttagctgcagttttatatttctcctggatgaattcctggctgttatgcaggattaccggacggagttccacattacctggtgagtatacgccatgaacgttaccgaaagcagcagctaccgtgaaacggggccctacttttgataaaatttcatacgcataagctacttcttcaggctgggtatacagcttggagttgtccacaccggagttgtccacgccgtcttcctcaccaccggttacgcccagttcgatttcgatggacatacccagtttgttcattctctcaaaatatttatgagaaatttcaatgttctctgcaattggttcttcggaaagatccagcatgtgagagctgtacagcggttgaccggtttgtttaaagaactgctcacctgcatccagcaaaccgtcgatccatggcaaccattttttagcagcatggtcggtatgcagtaccaccggaacaccgtaatatttagctacttcatgtacgtgtttagcaccggaaacgccacctgcaatgttcgcctgcagcttgtcgttcggcatgcctttaccggcaaaaaattgtgcaccaccgttagaaaactgaataataaccggtgaatttactttagcagctgtttccagtaccgcattcacggagttagttcccacaacatttacggcaggcatagcaaatccgttgtctttggcatcgttatacagcgcatccagctcttcgccgaataatacgccagctctgtattttcccatactctgatatgtgttttattttttaggaaagcaaatataaggagttaaatagaagatttatagcgaaaagtaagcgcttacgtattaattctaccaacagaaaaatgtattttaaccgatctcaatccggttttgtatgaaactatttctgtttttcatcgcaggtatattcctgaaagtgtctgctgctggtgcatttacagccaatgttgcggactccctgctatattatacctccttcgacagcacccgtattcattataccattgcaggtaccggcgccccggtattattggtgcacggttttattgtgaacggggattcctggaagaaaacagctttgtacgactccctgctggcgcatgggtatcaggtgatcaccctcgatctgaggggaaatggcgcgtcggatcatccgcacgacagcctcgcttatcttaatgatgcggaaacaaaagatattatgggactcatgacccatcttaatattaataattaccaggtagtgggctattcaaggggcgctattattgtttcccgcctgctggtgctggacgccagggtgcgcagcgccgtgatgggcggtatgggtatggcttttacagatcccgcatggccgcgccgccggcagttttacgaggcgctttcggggaaaaacgtgccggaactggctgcgatggttaaatatgtacaacagtccggactggatcagcgggccctcgccatgatgcagctgggccagccctctactacaccacaggagctggccggcgtgcatcagccggtattggttatcggtggggataaagacgaagataatgataccggaggctctctcgcggccatgatgccggcaggaatgcacggcacagtagccggagatcataattcagtagtgcgcacggtaccctttgcagaatgggtactcgattttctgcaaaaacattaactaacgctgagcacattgccatctaccttgatggtgtaggccgtcaacgcagcggtagcgggcccagtattcaccgcgccggtagtggtgtaccggctgccatgaccgcaaggcgcattacattcaattaatttggacgaattgttaaaggtggctacggtacagccctggtgggtgcaggtactggaaagggccgtgaaagccgctgcagtattgccggagcctgtacggataatgattaccccgttggagatcctgaaatcgcccacattggtgaggtcactgccgaggttcaatgttagctttgcattgccgccgccgggaggtgtggggtcgggatcattactgcctcccttgctgcaggcagccaaaccggctgtacataccaatgccagcgttaatccaatgttggaaacaaaatctcttctttccataaaatgcgttttagttgatcgttatcctgtttacgcaagtgaaaagaagaaagttgcctcgggaacatttaattttctatcaccgattgaaaataggcgggcgcctcagttaaacggctgccataccaggaaaacatttcaccgtctaccagctggattcgggcgtccggcaaaacagcctgcaactccgctatatgtttttctttgaaaggataaggttcagacgagagcaacaccctgcggcacccgctgctggccagctcagcggcggtaacagccggatagcggggcaggaggccaaatacattatggaacccgcataactgcaacatctggtgtatgaaggtgtcgccaccggctaccatccagggatcgcgccagatgaaataagcggtgggaacagcctccggaagcgggtgcagcgatgcaaagccggctttgatctgtgaaaccagatcagcggccgcttgcacccggtgggtgatagcgccgataccggcaatcatggcataagcatcttccaatgtctggatattactcacccacacccggtaatctttcatcagcagctccacatcagcggcgaggttttcttccttattggcaatgatcagatccggtgaaagctgccgtataataccagcgtgaatatttttggtgccacccacccgtgttttttccctgaaccacgttaacggatgtacgcagaatttggtaatacccaccacttccttttcaagtccgagggaatataacaactctgtttgggatggcaccagtgaaacaatccgctgtggcggatgttcaattgttatctgcctgttgagctgatcggtaaataacatgcggtacttttatctgcccaatgcctgtataatatcgtatttcgtaacaatgtggtgattgccgctgtcatcttttgtaagtacggcgccgttttcccggttgatatataccgaaagcttttcgataggcgtgtcctggcttaccagcgggaacaatggctgcattacctggcttatctgcgcatctttcaggttggcatcatcgatcaggcggttgaacaacccgttttcggaaatggatccaatcagttccccgccctggtctacaggtatatgttcgatgtcatattttttcatccgggcaatggcttcacttactttttcatcagcgctgatggttaccagtggctggttacgacggccattcactacatctttcactgtttttacatcgaggaaaccacgttccagcatccactggtcgttatagattttacctacatagcggctgccatgatcatgaaaaataacgactaccacatcggttggcttcagtccttctttcagctgcaacagcccggctatggctgatccggcggagtagccaacaaaaataccttcttctttggtgatgcgtcgcgccatcacggcagcatctttatccgttaccttttcaaatttgtcgatcaccttcatatcataattctccggcacaaaatcttccccgataccttctgtaatataaggatacacttcgctcatatccagctccccggtttcaaaatacttcttcagtaaggagccataactgtcgatcgcccatactttaatatccggatttttttctttcaggtatttcccggtgccggtaaccgtaccaccggtgccggtggccactaccaggtgggtgattttaccgtcggtttgttcccatatttcaggaccggtttgttcgtaatgcgcatcccggttagccaggttatcatattgattcacataaaatgaattggggacttccgtggccagtcttttagacacagaataataggagcggggatcttcgggttccacattggtaggacaaacaattacttcggcgcctaccgccttcaggatatccactttttctttggattgtttatcggtagtggtgaaaatacatttgtatcccctgataatggccgccagtgccagccccatacctgtattgccggaagtgccttcaatgagggtaccgccgggtttcagtaatcctttctcttccgctacatccaccattttcaccgccatgcggtccttaatagaattgccggggttaaaaaactccaccttcgccagcacggtgcaaggcagggaagccgttacgcggtgcaactttaccatcggggtattgcctatcgtttcaagtatattatcgcagtatttcataaaaaatgaggttgtatgattacgaaaatacggaattgcaccgatgcgaatgttgtctttctcaggattacgcggattttgtcttcctcaggattacgctgattatactgattagtttgattttactttttagattttataaggattttaaatgatttaagtagatctaagcggatatacccgcttagatctacctaaatcatttaaaatccaaagtgatcaaatccgtaaatcaatataatcagtgtaatcctgaggaagacaacattcgcgtatatttgcgccaatgagcgaaaggatttttattacaggaataggtacaggcgtgggtaaaaccactaccgctgcctgtatcacggaggcactaacggccgactactggaagccggtgcaaacgggtttgatggaaggcacagatacagatacggtattatccctgttgtcaaataaggtgtcagtttgtcacccggaagcgtggcggttgcaggcgcctgcctctccgcacctggcagcacggctggaggactgtactattgatgcggagcgtatcctggagctggcggaccagtaccagccggttgacaggccaatggtaatggaaggcgccgggggactgatggtgccggtaaatgaagagctgtttacgctggacctgatagtggcgctgaaagccagggtggtgattgtagcgcagaattacctgggcagcatcaaccactcgatgctcacggcaaggatgctgcaacatacaggcgtgcccgttatcggatgggtgtttggcggagattatcacagcaatgaagacgatgtggtaaagtggagcgggtacccgaaaattggccgtatcccgctgacagatacggtagataaggcattcattcaacaacaggcacagttgttgtcagcctcgctgcatagtttactggcatgaccactaaaaaggatatacgaaaacatttcctggagctgcggcttaacctggacgaacccaccgccctcgccctgaatgagcggttactggcgaatgcccgtcagcttgactacagcaacgtcaggaatgcgcatatctttcttcctatctctgaaaaaaaagaagtggatacctggccgctggtaaaatgggggagaacccaatggccggaaatggaatgggtgctttcccgctcggatatgaaaaccggcgagatgaatcattatctctggaaaaccaataccgtactggtgaaaaacaggttcggcatcccggaaccggatcatggggaagtgatatcaccggaaaatatagaccttgtatttgtacctttactggctttcgaccggcaggggcagcgggtaggatatggcaaaggtatgtacgaccgttttctgaaacaatgccggccggatgtgcgtaccatcggcctgtcgctgtttgaacccgttctgcagatagaagacgtggattcgtgggatgtgccgttgcatacggtggtgaccccggatcacatttatcaatttaaataaacaacagtgcttaaatacctgaatgttcttttatatcctttttccctgctgtatggcctggtgatgtggttgcggaaccggttttacgacaaagggctgctcactgcagtggaatttgatcttcctgtgatcgccgcgggcaacctgtcggtaggcggcaccgggaaaaccccgcatgttgaatatatgatccgcctgctgaaggatcatctgaaagttgccacgctcagccgggggtacaaccgccgtaccagcggctacatcctggcagatgaaagaagcactgccgccgatatcggggacgaacccatgcagtttcacgataaattcccggatatcaaggtctgcgtaggagaagaacggatgctggccattccgcagctgctcggagatgagcccgatacccaggtggtactgctcgatgatgccttccagcaccgctccataaagcccggtcttaatatcatgatcaccgattacagccgattgtttacccgggatcatgtagtaccttttggccgtttaagggaaggcagacagggatatcaccgggccgattgtattattgtatcaaagtgtccgcccgccatgagcacggaagagaagctggccctggaaaaagaaattaaaccattgccacatcagcggctctttttcactaccttgcaatacggcgccttgtccgatatgatcacccatcacccggtggccgtccctaaatcagcaaccgtattgctggcatgtggtatagcaaggcccgaaccattgctcgaagaattgaaacgacgttacgaacaggtatacctcttgtcttttcccgatcattattattatacggaaaaggatatactaaaaataaaaaaggaatgcagcgacctgcccggcacagaaaagattgtcattaccacagaaaaggatgcggtaagattacatctgctcaaaggaatgctggcagaacaaaacctgcagatggctgttattccagtagagattgcattcctcttcggggaagcagaattatttaataactttatttttgactacataggccggcacctgccagcgcccggtcaacaataacttacgactaacatgagtagaaaaaagaaaaataaaaaaggcggtaatcataaccctaacaacccccaacaaagccatagccagaagaagacctttaaaggcgtattggaagtaacaaggtccggaatggcctttgtgatcgtggatggccttacaaaagacatcatggtgaagcagaaaaacctgcataccgccctcgataaagatgaagtgctggtggatgtattgaaagcagcccataacgaaggccgcatggaaggcatcataacggacatccttaaacgaaataaaaccgaattcaccggtaccctgcaggtcagcaaaagctttgctttcctgatccctgaaaagggattgtttatgccggatatttatattcccgccaactccctcggagaggctaaaagcggcgataaagccgtggtgaaaatagtagcctggggagaaaaatcccgcaagcctgtaggtgaaatcgtggaaatcctggatgccagcgataccaacgacctggccatgaaggaaatccttatagaagcaggattcccgctcagtttccctaaagaagtaatagcagaactggataccatccaggaaaatatttctgaagaagaagtaggtaaacggaaagatatccgcaaaatccttaccatgaccatcgacccggtggatgccaaagattttgatgatgccatctctatccgcctgctgaaaaacggtttgtatgaactgggggtgcatattgccgatgtaagtcattatgtactgcccggcaccgaactcgataaagaagcggataaacgcgctacctccgtatacctgccagaccgcgtgttgcccatgctgccggaaaagatctccaatgagctttgttccctgcggccgcatgaagacaagctcaccttctccgctatgttccagatgaacgaaaaaggagaggtgaagcaacactggatcggccgcaccgtgatccattcggatcacaggtttacctacgaagaagtacaggaaattatagaaggcaaatctgagggtccgtataagaacgaagtgatgctgttaaaccgcattgctcaaactttgcgcaagcaacgttttgtacatggcgccattaacttctcctcgcaggaagtacgctttaaattggatgaaaccggcaagccgattggcattgtcattaaggaaagtaaagaagcgcaccagctgatcgaggaatttatgctgctggccaacaaaaccattgcggcatacgtgggcaagctgcggattaataaacagcccatcccgttcccttatcgtgtgcatgatacgcccgacccggaaaagctgaaagtgttcgccctgttcgccggaaaattcgggtataagttcgatctcaccacaccggaaagcatcgccagctccttcaataaaatgctggcacaggtaaaaggcaaaccggagcaaccggtactggaaacgctgggcatccgtacaatggccaaagccatttacacggtgaataatgtggggcactatggtcttggttttgaagactactgtcatttcacgtcccctatccgccgttaccccgatgtactggtacaccgtgtactggctgaatgtcttgccaacagcgtgcgtcccgacaagcaaatggagcagaaatgcaaacacagctctgaaatggaacgcaaggcaatggaagctgaacgcgccggtaacaaatacaaacaggtagaatacatgcagcagttcattggtcataccttcgatggtgtgatcagcggtgtggcgcatttcggcttctgggtggaaacagtggataccaagtgcgaaggactgatcagcattcacaatctgaataaaagagaagaattccaatataatgaaggggagtattccctggtgggccaaagcaccggccgcaagtttcgtataggcgaaaaagtgagcatccgcgtagtggctgccagcctggccaaacgccagctggactacgacctggaagatgaactgaccggcacgggcacacctgctgctgcgccattccagcataaacgccgggaagaccgccgcgatgatcgtaaaggtgatcagcgtcatggtgatcgtcgtgacgaccggaaaaagaagaaagacaaacaacgtccgtataaaccctgggaacaggaagggaaagcgccccacagagcgccggaagtatcgctcggcgagcctaaaccattaccggttgttgaccaggtgatagtggaaacgcatgtggtaccggtaacaccggatgtacctgtaacgcctgctgtaccagtaacaccggtaccagcacctgtgcataaaaagaagccgaagaaagaagtggcggaagaaaaaccagctcctgcaccggttgttgaaaaagaagtggtgaagaaaacacctgcaccagcgcccgcagttaaggcgcctgtgaagaaagccgctgctaaacctgcaccagcagcaaagaaagcagtgcccgcgaagaaagctgctgctgaaccggtagcaaagaaagcagtacccgcgaagaaagccgctgctaaaccggccgcaaaaaaagcagtaccggcgaagaaggcctctgctaaaccggtagctaagaaagcagtaccggcgaagaaagctgctgctaaaccggccgcaaaaaaagcagtaccggcgaagaaggcctctgctaaaccggtagctaagaaagcagtaccggcaaagaaagccgctgcaaaaccagtagctaagaaagcagtaccggcaaagaaagctgctgcaaaaccagtagctaagaaagcagtacctgcgaagaaggccgctgctaagccagtagcgaagaaagcggtacctgcgaagaaagctgctgcaaaaccggtagctaagaaagcagtacccgctaagaaggcagccgctaaaccagccgctaaaaaagccactgctaaaaaggccgcaccagcaaagaacaaaaagagtaaaaaataaaacacgagccaccagcaatgcattcattcaaagatttaacagcacagtttagtcagcattttgaaaaacaacagtttccggaacaacccagtaagttatataatgcagcgtcccacatcctgggaataagcggaaaaagaatccgccctgtactatgcctgatggggaacgagctatttgataatctgcgcccggatgcatttgaggtgggcagtgcgatagaactttttcataatttcactttattgcatgatgatatcatggataaagcgccgatccgccggggtaagcctaccgttcatacggtatatggcgagccggcggcgatccttgccggcgatgtaatgctcatttacgtatatgaacgcctgaacaaaatagaaccgcattataaacaaaagatcatatccgtatttaataaagccgccattgaagtatgtgaagggcagcagctcgacatggactttgaaggcatggaccccgaaaaggtgcagtacgatgattatgtgcatatgatcggattgaagacctccgttttacttgctgccagcctgcagctgggcgccatcattggcggcgccggcgaaggcaaccagcagcacatttattcctttggtaaaaatgtgggtattgctttccagatccaggacgactacctcgatgcatttggtgatcctgaaaaattcggaaagcagcagggaggggatatcctcgtcaataaaaaaacattcctgctcctgaaagcgctggaactgtgcaacccggaacaacgtgcagaattgaaaatgctcatggaaacatcacccgccgataaagtagaacgggtgctggcattattccgcagctgtaaagtggatgaatgggcggagaaggaaaaagaacgcttccagcaactggcgttccagagtctggataacgtggcggtgctgtctaaccgcaaggcagcgctgatggaagtggctaactacctcttaaaccgtcagcaataaggttcgtatttaaattcgcattatattcgcgctcgtctaaacgtaattccttagccaatgtcgtcaaactcgctgtttcggaaaaaatcacttactgccattattaaagatgccaaagacggtttgtcggatggtcatgaaacagggggaatgaataaggtgttgaaggtgaaagaccttactgctatgggaattgcggcggttatcggagccgggatcttttccactatcggggaagcttccttccacggcggaccaggcgtttccctgctcttcgttattaccgcagttacctgcggattctcagccctgtgctatgcagaatttgcgtcccgtgtaccggtatccggcagcgcctatacatactcctacgttactttcggagaactggctgcctgggtgatcggctgggcgctgatcctggaatacgccattggcaatatcgccgtagccatttcatggagcggctacttcaacaacctgttaagtggtatcggcctcagtttacccgattggctggccagcaattacgacagtgccacgccggaaaccattgcggcagcaccgcatattgccggcatacccttcatcgtgaacctccctgccttcctcatcgtactgctggtaacctatctggcgtatgtaggtatccaggaaagtaagaaaagcgccaactttatggtagccctgaagatcctggtgatcctgtttgtgattgtggtaggctttttttacgtaaataaggccaattggcacccttttatgcccaacggcttctcaggtgtgctaaagggggtatcggccgtattttttgcttatatcggctttgacgctgtgagcaccactgccgaagagtgtgctaatccacagcgggatctgcccaaaggcatgatctattccctgatcatctgtacggtattatatatcctgatctcattggtgctcaccggtatggtgccgtattataatttaaaggtaaatgatcccctggcatatgtcttcacacaggtaaacctgccctggatcagttatcttatttctgtaagcgccgtggtggctactaccagcgtactgctggtattccagatcggccagccgcgcatctggatgagcatgagccgcgacggcctgctgccaaaacgcttcagcaaaatacatccccggtttaaaacaccttctttcgctaccatcatcaccggtttcctggtaggtatcccggcgcttttcctgaacctcaccatcgttacggacctgaccagcattggtaccctgtttgcctttatcctggtatgcgggggcgtactcattctgccaagagaggaaaaatcagtggtaaaacggtttcagctgccatatatcaacgggcagttcattgtgcccggcatcgtggtgctgctcgttttcctgttcagcaaagaaatcatggcaaagctctcccccgcaggcggctgggaggtatggaaacataatatccccttctacatatttgtggtggttaccatcgccctttcctacttctcgctcacccgcaagctctccctgataccggttttggggatgctcagctgtttttacctgatgacagaaatcgcccttaaaaactggatcgttttttctgtttggctggcggtaggcttaaccatttacttcctctacagctataccaacagcaagctggccacgaaagcgtaaatcttcgtaacttcagggtagctctttgatcttaaaatttatattttatgaacatgctacaacgggttgaacactggggtgacacacatcacccaaattggctgagtgtggttcgcattctgctggggatatttattatgtatgtaggcatccggtttgtacaggacagggacgcgctgatttccatgattaatcaaaacccggctttggccacactgtccatattcctgggacattatgttgtatttgcacacacggtaggtgggctattcattgcgatgggactgttcaccaggatcgccgcattcctgaatattcccgtattgctgggtgctgtattttttgttcattctcccaccgggctgtttacagtataccccgtaatgggcatctccttactggtgctgttcctgctgatcgttttcctgattgaaggcagtggccgcatttcggtagatgactacatgcggcggcatcctgaaaaagcaaggtccaggaagtacgcggaataacttttcttcatatagccgtgcaggtgagtgttaccatttttaatggcaataaggagccatgtctccgccggatccggcaaatcttcaaatctcttccacgcatatcccttcaatattctatttttgcagttgaagaatgcaattatgaaataccaaaaaggcgacaacatcttgttgttgagttcaaaagaagaaggaacggttgttgacattgtgaatgataatatggtcatgatagaggtgaaaggaacgtcttttccggtgtacctggatcagatcgactttccctatttccatcgttttacccagcagaaactggtcaaggaaaagcccaaactaattcccggcgacgaaatcaaggtagacagaagcaagtatgaagtgtttaaaacagataagggaatgttcctgtctgttttgccggtataccagatggatggatatgatgaaaccgtgaagctgatgaagtttcacctgtttaatgatacgccgcatgcgatgcgtttttatttccagatatggctgaataaccagctggacctggaaatcaagaatgaaatacatccttataatcacttttatctcgctgatctcatcttcgaatcactgaatgataatccgcggtttgagtttacctttttcctgaaggagccacagcccaagctggccacttctgtaaagaaaacctggaagatcaagccaaaacagatgtttgtgcagctggagcagctgcgtaccaaagcagaagctaccatcacttacccgctgttcgataaatttccggagaaagaacccgagccgccggcgccggcagaacaaccgaaaaagaaggcgcctgttactactattggcggcggaaacttcgccagcctgttaagtaaaatacagctgcagcccgaaacatcgctggagcctaagcacgaagtagatctgcacatcgaagcacttgagaaaaactggaaagggctgagcaatattgccatccttgctatccagctcaatgctttccaacgttacctggaactggctatcagtcatcatcagcacaacctgatcgtgattcatggtatcggaaagggaaagctcaaagacgaaatacaccagatcctgaaacaaacgccggaagtagccagctttgtgaatcaatatcacgccaaatacggctatggggctacagaaataacgtttaggtaatatttttatttaccttcgcgcttcaactacaaaccgtgctatcgttccgctaacttgttggcgggaaggaaagtccggacagcgcagagcaacgcaccacctaacgggtggggcctggtgcaaaccgggaacagcaagtgccacagaaaataaccgtccgcttcggcagataagggtgaaaatgtggggtaagagcccacggtgcaggcaggtaactgtttgtacgggtaaaccttgcgtgctgaaatgccatgtatacggtcgattgagggctgctcgcccgatgaccgagggtaggcagatacagacaacgtgcgaacgttgtcgcagataaatgatagcagtctgtcccggcttgccggggcagaaacagaatccggcttacaggtttgtagttttttttcttctcttttttgatatcctaaaataagctgttaacttcccgcattatatttaatctatattttatgaatcagaaagatgaacgaacctggggagcgcttgttcacctgggaggaattatcgggatgctgatattacctaccgtcggcaacatccttggagtactgatcttttggcttatcaaaaagaacgaatctgcttttgtagacagccagggcaaagaagccatcaatttccagatcacattgagcatcgctgcggtcattgtaaacctggtcaataatattgttaccggtttttggtcgctcaccagcttctggcgccatgcaagaggagatttttataacgcctggggctggacaaacctgctcggtgtattatggctgctgaatgttatctttagcattattgctgccacaaaagccagcaatggccagtcttacaagtatccgctgagcgttcgtctcgtaaagtaattgtataaaaaaagggcgggaattttatcttataaagataaaattcccgcccttttttatatactgaatcagttctttttgatggcttttacttttgccttgtgctgttttttacctttcacattttcgcctttaacagtagccgccagctttaatgcttcataggcattgatcattccaccggtgatggacagatccgaaaaatttactttttcatccgcagcacctggtttatttacttccgtaataccaggtaatggtgtggcgcttttttccagcacatatttcaactgctttgcactgagctcaggataataggagagtaccaatgctgctacacctgctactacagggctggccatgctggtaccactggcgctgccgtatttgttgccaccgggaatggtggagtaaatttgtacaccgggagcaaaaagatccacgcttttcttaccatagttggagaaaggtgccaccttatcattgcccaggccggtattgctggcgcctacagtgatgacgttggaagcaaccgtgccatccaggtaattcgggttgggatagttggcaacagagtcgttgttgctgccgtcattacctgctgcatgtaccaataaaacgcccttttcttctgcatatttaaaagccgcatccacccagtctttatgaggtgaaaacggtttaccaaagctcatattgatgatctgtgcgccattatcaaccgcataacgaatggcgagggctacatctttatctctttcatcgccatcaggaacggcttttaccgccatgatgcgcacattatcggcgatgccatccatgcctacaccgttgttcctggccgccgcgatgataccggaaacgtgcgtgccatggaaaccaaaggtgcccatcacatcgttgttgccgtatttgttgtcattgatgtcgtcgaggttgtcgcctacaatcctttccctgttggcatttggcgctacttctgtgctttctgccttacgcttcagttcattcatgtactcatcaaactccattttgaactcgccgaaagtggctggttcatcaccggcgcttttcagcaaacggctcatgaaattacgtgccagcagtacatcctggttagtcgtttgaatgctgtccagctgcgctacattgaaatcatccttacccaggtaggttttcaggatagattcacatttattcacgttttcctggagcttcgacatgcttttgtattgcatcttgaactgggaattaggcttctccactttcgattgcaactgctgccagatggcatattctttggaatcctttgcgagtgcggaatccgggttgccataaaggtttttatagcggtagtattcgcgggcggcttcttcagagtcttctttcaggctgctgccgtctttgccacccaggaagttccagccatgaatatcgtccacatagccgttgtgatcgtcatccttgccattaccggggatttcacgggtattggtccacaggatacttttcagatcctcatgggtagtgtcaataccagagtcgatcaccgccacaataacgggcgtacttttcttcccttttaacaattccttgtaggctttttccgttgacgtacccagtatactgtcggtatcgtaactcagtaactgccagtttttaggtatctggggtttactctgcgctgtagtatttgttgtaaatgcagtcatcaatgcaacacaccctgccaggactgcaacctctcggcttaacaatttcatgttcaataattttccctataaaaaacaactaaaaatatcatgatgataagattaaaggtatagaaaaagcggtataacattaaatattaatgataaacgcgctatatattggttgattgggagattgaatgggtttctgcccattccgggccgcctttttccgcaggccattgttaccggttacttatcctgatttgcttgccagccatagctggtaaccacctgtcacaatcccttttgtaattgttgtcagccgtcttagctttaacctgttcttattcctcatacccctcatccgccagatctacgttcgggatttttacaggtatcgtatttcatttacttaaatttaccaatcatgttaaaagctgttctcatggccactttgctggctaccggcacacctgtgtctgccgctgaacctgaagtaaccacactcatttttgtgaatgctgcggaaatggaatcatcaccatcagcagatcccggtttgagcaccaccgggcaggaacaggccagccagctggcatcttccctggaaggaatggaaatttccgctatctacactacctatctgaaccgtgctgtgcaaacggtgacaccgctctctaaagcccaccagcaacagctggactacttccggttaaacggcgatccggagcaaacaaccgccacccttaaagacatgataaagaaaaataagggcaaaacaattgttatttgcagcgttcctgaaaatattactgctatgttgcagcatgcgggtgtaaagggcaaaatcatgaaaacactgtatgataaaggatccgggcaggttttagtagtgaaacacagtggtaataatgcggcagtagcacaaaagttgaatatgaatattcaaaaaaaagtctaatatttatatccggaagagtttctaatggcttcccgccatttctaacttttctcataagcatggtttccgtttaacgaaaagcggggttctctaacctcgctactatttttaaaaccttgccgccgtcggtgtatgtagagaaaagcaacgcaggttgcaaaacatttttgacacgtagttattttatcaaccgcttttaaaaatctgatcgggtagcatctcctgtcacgaaaattaaaagctccggggcaagcgcctcggagctggatgatccggaaaaatttacagtaaatatattgttgtcagctatccgttttcaggtatttgtacctgcaaaacagatagctgatttattattatcagagatcaaatttgatgccctgtgccagtgggagactgttggagtagttgatggtattggtttgccggcgcatgtaagctctccacgcgtcggaaccgctttcacggccgccgcccgtttctttttcaccaccgaaagcgccacctatttcagcgcctgatgtgccgatatttacattggcaatgccacagtcagatccggcattggaaaggaactgttctgcctcgcggaggttcagcgtcatgatggcggaggaaagtccctggggcacatcattctgcatggcaatggcttcggccagtgtggcgtatttcattacatacaaaatgggcgcaaaggtttcgtgctgtacaatatcgtaggtgttttccaccgctgcaatgcagggttttacatagcatccggattcataacccggaccggataatacaccgccttccaccaggaaggaaccgccctgctgctttacctgttctattgagttgagatacgcatccacagcggctttgtcgatcagcgggcctacgtggttgtgttgatccagcggattaccgatacgcaactgcgagtaagcttttaccagccttgcggtaaacgcatcatacacgctttcgtggatgatgagccggcgggtagaagtacagcgctgcccggcggtacccacggcgccaaacacagcgccaataagcgacatatccaggtcggcatcctgcgtaataatgatggcattattgccgccaagttcgagcagggaacgccccaaacgctcgcctacggcagcacctacggctttgcccatccgggtggacccggtggccgaaacgagcggaatccgcttgtcgtgtgccatccattcacctgcatcacgctgaccggttaccaggcagcaaacgccttccggtactttgttggcggcaaatacactggccgcaatatgttgacaggccaacgctgtcaccggcgttttttcagatggcttccagatacacacgttgccgcaaacccatgccagcatggcgttccagctccatactgctaccgggaagttaaaggcggaaataataccggtaatacccagcggatgccattgctcatacatccggtgccccggccgctcggagtgcatcgttaagccgtgcagctgcctcgacaggcccactgcaaagtcgcagatgtcgatcatctcctgcacttctccatatccttcctgcaaactctttcccatctcataggaaacaagtttgccaagatgttctttatgttcacggagcgctaccccgatttgccgtacgatttcgcctctttttggggccggccatgtacgccattcttggaaagcttcctgggccacggctaccacctggtcataatcttcccggctggcgcttctgacagtaataatcttcttattatttaccggcgaaactgaggtaatttcctccccgtgagccggcaaccagtgcgtgcccgtactgataccactttgtgccgcagtgatgccaaatgcttttaagatgtcttccattgttggtgtattaataaactaaattaggaacttttttttgtttgggcggcgtaggtactttcaaagatcttatcggcattgcctgcttcaaaaccctcacgccggtgttcccgccgtatttcactggcaggtaaatgcgcaaaggcaggaagtacctttctttcggcaaactccacataggagccggcaatggggaattcctccccaccggaaaaggttgcggtgatcattccggctaccgtggcgctttgcagcagtctgccatccggactggttttaattttacctcctgaatcattgagatgaaaaccatgtttttccaggaactggttgaaatcagcgaccgtattatatcccgggggcagattatgtacgctcacggtaaaatgattgaggtaataacggttatagatcacccaggcggcgtattcgctttctgcggccagcactttgtaatcggccagggtaggggtttgccacagtgcgctgtgaaggaaagcatccacggctttgctgtcgtcgaggtccaaggcattcaccgggtccgacttcacttcatctgtataatgatgaatgatggtttgcgcagcagggcttaattcggccacccgcagttcactgataaaaatacgcggatattgcggctcggggggagcataccaccatgcatccagcttcttggccggaaagtggtagtgatccattttcgtatagccgtaatggagaaaaattttctcgagcgactgcacgccaagctgtggaacgcccatcgtccggaaggcgatgtggtcattttctatatcatctgcctgcgcaataatgccttcctttatcatggcggcaataacggctccaacgtccggaaccctttgctgatagcgctccatcagcccatttaaaacatcttttaacatgacatacagcttttagggctagttataatataccgcaaagcggttgttgatcaggtcattaaatgctacatcttcctggcgcagaaagccattcgccggcagcagtccttttgcgtgcaggtctattactgcacaggcagcgcctgcggtggtgagttgtatggcggtaaagtccctgccggccaccgcctggttgtagatcttacgggaataggagcgttgcacagagcggccgttcaccattccggatacagacacaaaaaccaatactacatcctgctgggtgaaaggtatgctatcttccataatctccttcagcatttctctttttttattgagtttcagctcatttaaaagaattttcatcaggtggcagtggccgggataacgtactgttttatagtccaggttgtacactttatggtccaggatttcagcgagtgctccgagtccgccggaggtattaaacgcctcatattccacaccatcgagggcgaagcgctcgtagccttccatcggcattacttctttgcgttcgccttcgtagatggcatcgcagggattgcagtattcgttgatcagcccgtcggtgctccaggtaaggttatacatgagactgttggtaggaaactgtggcagggcgccaacacgcagccgcaccgcgtccagcgaatcgaattgtttggcgatatcatgggcggcaatactgatgaaaccaggcgccaatccgcattgtggcatgaagctaacattggcttgcgccgctatttcgcggatcgcgttggtagtagctacatcttctgttaaatcaaaatagtgggtgttggctttagctgctgcggtagcaatttttacgttgaggaaaaaggggcaggcgctcagcaccatgtcctggtcctgcaatgcgtcctgcagcgacgtggcgttgtttacgtccagcacggttttgcggatagctgtgtcggtacatttctgtaacagggcgtcgttgctgtcggccagcgttacttcatagtcgccggactgttgcagtaagaaggcagcggtttcgccgatcttaccggcgccaataatcattacacgtttcataatctgttttggaattatagtgaagagggaagcatgtgttgctcccggataaataataataaatgacgcttccctaaactacgtatatacgttactgttatacacgaacctaagcatttgcggattggttaaaaataaaccaatgcaaaatcatctgtcgtgatgaaagtcagtatggcagatacaatagcattacaagccgctaaacggcctacaggaaagaaaaagaagggaagtgctacctatggcacatgggagcaggtgctccgcagataggagagtagagaaagctgtatgtttaacaggtagttcattcaacttataaagtgcgaagcgaatatagggaatttatattaaatgcaaatgacgaatttgtatggagatattaatctctctacaaatccgtcatgcttattatttaatcagtactgattagtactgttcattttcattcgggaaatctttggattttacatcattgatgtatgcctgggtagcgccaaagatctggttgtaaaggtcgaggtaacgacggaggaaacgtggtttgaactccttattaataccaagcatatcatgcatgaccagcacctgtccgtctacatacctgcctgcaccgatgccgatgataggaatttctacgctttcggctacgatctttgccagggatgccggaattttttccagtacaatggcaaagcagccggcttcctgtaacagttttgcgtccttgatcagcttattggcttctgcttcttctgtggcgcgtacggcgtaggtgccaaacttataaatcgactgcggtgtaagtccgaggtgacccattaccggcacgccggcggagataatgcgttttacagattcaatgatttcttcgccaccttcaattttaataccgtgggcgcctgtttctttcataatacggatggcagatcccagggcttctttggagttcccctggtaagtaccgaagggcagatccacgatcacaaagcagcgtttaattgccctgaccaccgaagcggcatgatagatcatctggtccagcgtaatagggagggtggtttcatgaccggccattacattggaagcggaatctcccaccagcaggatatcaatgccggcatcatcaaaaatgcgggccatggaataatcatacgcagtaagcatggagatcttttccccgtctactttcatcttctgcagtatatgcgtagtgacacgctttatttctttattcacagacataagcagtgagcttttagcatttagctgttagcaataaccgcaaaggtggtaatataaaaagataaaaggaaatgttttttatgtacggccggggatcaggaactcactgcgatttcctcatagagggcatggataagaccatctgccagccctatcttgggtacatatatctccggggtatcagcccagcgcatgatgtttacatagatctgcagggccggaacaatcacgtcggcgcggtcttcccgcagtccgtacaggtgaatacgttcttccacggtgaaggcgctgaactccttgtaatagtctttcagcgtatccagtgaaaggggtttgccttcttttcgtttggagagagagaatattttattgatgttgccgccggaaccaatcgcaatcacggcgccgatgcctttgagctgatgtttcaggaaatctttcagttgctgccagtgcgcttcggtaacctgttgttgcagcaggcggatagtaccaatattaaaggactccttgaagatctgtttgcctgcgctgaaaagcgtgatttccgtgctgccgccgcctacatcgatgtagaggtacgactttgttttatccatgttctccgccacatggttttcgtagataaaagaagcttcttcctgaccggtaatgatccggatatcgatgccggtttgtgcttttacctgctggaggatgtcgatgccgttgctggcgtcgcgcatggcagaggtagcgcatgctttgaggtatttcacctcatacacatccagcagcagcttataggcccggatggtatcaataaggtgtgcggcctttttgtctgaaataacatgatggttaaatacatcaaagcccagccgtagcggtactcttaccaggtttagtttggtaaagtccattacgccggcactattgggcgatgcctcagagatgagcagtctggcagcattggagcctatatcaatcgcagctaatttcatctgtcagtcgttagatcaaagggcaaaagtataactttttagagttaatggtattgtttttcgtgcaggtatttatagatctccatttgtgtacggatctttttatcaccggctttcttatattcatttttctgctcgttatccagtatacgggccttcacattgccgctcagctgaatattcataatatcgatcagttctttgcgtatagccgggtccgttataggcgcagccgcttccacgcggtgatcgagattacgtatcatccagtcgcaggaagcaatgtataccttttcctggccgccgtggtgaaaaataaatacgcgggcatgttccaggtattcatccacgatgcttaccgcggtgatattctttttccattttttattttccgtataggcgcagcagatacctcttatcaccatcttcacgtccacaccggctttggcggcttcatacagcttggcaataagcgctgcatcagaaagcgagttcattttaacagtaatagccgccttctttttgtgttttgcattcttgatttcacggtccatcaggcgaaggaaggtatcgcgcatgttaaacggactaaccggcagggttttgcagccctccagtattttgatatcatgacgggtgttttccaggtaggaaaagatacggttcatatcggcaatgatagcgcggttggtggtgagcaggcagtgatcaccgtaaacccttgccgttttttcgttgaggttaccggtgcttacaaagccgcactgcagcgttttagtgccgatccgttttttgatgacgcacagtttggcgtggattttcatatttggtatacccagtaatactttcacgccttcctcttccaaccgtgatttccagtcgaggttggcggcttcgtcaaagcgggcgcgcagctccagcaccacggttacctgtttaccattacgtacggcattcaccagcgcattcactattttggaattacgggcaagcctgtacgcagttatttttatagaagatacgttcggatctattgccgcttcccttaacaggtcgatgatggtatcaaacgagtgataggggaagtgcagcattacatcctgctgttgtattacatgcattacactgggcgcattgaggaacagcggatgggtgaaggttttacggtgtaaatgaggggggaagatagattccgggaaatccataaagtctttgaaattatggatacgtgcgcccgggatcaggttatcctttccggaaagtccttgtctgcgcatgagatattccagcagcagcgggtctatgtccttgtcatatacaaaccttaccggcttgcccttgcgacggtctttcaggcctttttcaatctggtgaataagactgtcggagatatcgttatcaatatccagttccgcatcgcgtgttactttaatgatgtgtgcggagaatttatcgtaaccgaaataggaaaagatattgggtaagcagaagcgcaccaggtcttccagcaggatgatatcgtgttctccgggtttggagggcaggataataaagcggggaagtaccgtggtaggtatttctatgagtgcaaatttctgtcgtacggaattatcctgtcgggccagtacgatggccaggtaaatagatttatcgcgcaggatagggaactgttgtatgctttcaatcatcaggggaatgatgttggtgcgtacctgttcattgaagtagttgagtacaaatttctgttgctcgcggttgagttgtttttctgttcgcaggaagatgtgctgggcttccagttcttccgcgatatctttccataccaggtcaaactcgcgttgttgctcaattacacgggtttgtatttcgtccagtattttatccggattttcttcgagatgcattttaccggctttgccgaaaaacatcatgcgtttaagggtggctacccggaccctgaaaaattcatcgaggttattggaaaagatgcctaagaagcggatacgctcatggagtggaacggttttatcggctgcttcctgtaaaaccctggcattaaaggagagccagctgatatccctggcaatcatttttttcttctctgcaggggccttcttggttgttttcttttgtgctgttacatcgggcattgtcataatatcaaggttctcaccattcggcaaacgcatacgaacttatttacattcaaaaaaatcacatcgtctaaaccacgatgatacggctttcgctttaattgaagtattaaattaaagttaaagaaaatcggggagatgatcgccttcggcgatgcggattttgtcttggctcgggattacgctgattatactgattaatttgattttattcttttagattttataaaggattaagggagatagaagtggatattcgcttctatctcccttaatcctttataaaatctaaaagaataaaaatccaacataatcaaatcagtgaaatcagtataatcagcgtaatcctgagccaagacaatttaaaatcgccgaaggcgatccctccgctctacccgcgttttttgttgtaaacaggcaacgccaccaggctaatgaagccaagcaggatcacgagcaccgtttgcgccacccagatgatccagccaaaggcgaagccgatggctaacggaatgccatacagttccagcgatttctgtaccaggggctggtaggcgccgataccgccgggggtaacgatcatgcccacactaccgatcatcagtacggcgagagcggcgctgatacccaggtggctcgtttctttcaggcagaagaagccgatgtatacctgcgacaggtagcacgaccagatcaatacggtatgtaacaggaaccagcctttcttttccattttgccgatagaaagaatgccttccatgatacctctggcgagggttttaatagtgatggccactttggatcgggcaaactttttcagcagccagagtaacagcagcactataccggtgaggattaaaatgcctatgagcagctgtatgccattggcatgcgctattttattggataatggaacaaagatcgattcattgacataggagccgagaacgtccagttgggtcaatacagtgagggccatcagcagaagcaggcaaaccatgtctaccgcgcgttctgcgatcatagtgcctacgagcttatcggcaggtactttttcatattgcgccagtatcccgcagcgggtcacttctcccaggcggggtacagcgaggttggccaggtagcctaccatcaccgcaaaaaaggtgttcagggtagtgggttgatgccccagtggtttcatcagcagtttccatcttatggccctgaaccagtgactggcgataccgatagtcatggtggggatcagcagccagtaattggctttacggaaggctgtattgatctgttcccactgtgccgtggtgatatctttggtaaaaagccatatcaacagcaccccaatgccgaaaaagcaaataaacttaatgacgttcttaagcgttttgggcatcatccaaagttgtttagggcgttaattaaaaacaggtacagatacgggcttacagtttatttccttccttggggaaaatggcgataggcgtatattttttagcttcttcaaaatccatagtggcataggagataataattacaatatcaccgggggcaacaagacgggcagcggggccattcatgcagatcacaccggaaccacgttttcctttgatcacataggtttccaggcgttctccgttatttacgtttaatacctgcactttttcatattcgattaaaccagcggcgtccatcaggtcttcgtcaatcgtaatacttccaacatattgcagattggcttccgtaacaaccgcgcggtgaatcttacactttaaaatttcgatttgcataattatactggcttagcgctatagagcgtttgcaaagctaggaaaaaaatatggaagatcgaacaggggatgcagcagtaatgcagtgcctgccgcatcccttgcggaatgggctagaggctgccctgcagcaccatattatcgatgagccttacgccatccagccaggcagcaacggctacaactaccgtggcatttccgggtggttgatccaggtgaacgagggtgtcattatccagctggaggatatctacatattcgggttcgaagccttgtgttttgagtgcatcaaaagcttcatgggcgccttccataaagtggaggcctttcccgaaattgttttttatgtgaagaagtgcctggtagatgcccactgcctttttccgggcggcgggagagaggcgcgcattgcggctgctcattgccaaaccgtccttttccctttccgttggacataccaccagttttaccggggaatgggtaatcaccaggagccggcggacgatcaggcattgctgcagatctttttgtcccataaaaagctggtcaggttgcacaatatccagtaacttgtgaacaatacgacccacgccctgaaaatgccccgggcggaatttgccttcaaggatagtttccaggtcgccgaagtcataatgcagatcactttccaggccttccggatacatttcttccacggatggtaaaaaaagtatatctgtcgatgcattatttaatttttttatatcctcctctatggtgatgggatatttttcaaaatcttttggatcattaaactgagttggattgacaaagatgctgcaaacgaccacatcattttcttgcctggctgcctgaataagtgacaggtgaccggcatgcagggctcccatagtgggcacaaaaccaatgcttttgttactttttcttaccaggtccaggtgcttcttcaggtccgtgctgcgcttaaatagatacataaatcattgcttaaaaggatgttaaaactgacagattgaccaatattccgtaaaaaatccgtaattttgcaagccaaattaaaaattactgcattaataatcagcgttaaatgtccacaaagaaaagaattctttttattgcccaagagatgtcgccgtacctggaattgagtgattacgcggcaatggtcaataaaatggcaattaagtccaatgaggctggcctggaagtgagagtgatcatgcctagatttggaattattaatgagagaagacatcgtttgcacgaagtcgtaagattgtcggggatcaacattgtgattgacggggatgattacccgttgattatcaaggtggcttcgcttccaaacgcccggttgcaggtttacttcctggataatgaagattattttaagcgcaaaacggtgtttgccgatgaaaacgaagagtttttcgacgacaacgcggcgagagctgtcttcttctgcaaaggagccctggaaacggtcaaaaagttcggatggcctcctgacatcattcattgcagtggctggatgacctctctgatacctatgtatctgaaaacggcttataaaaaagagccggtctttgccaattcaaagatcatatattcgctgacccccaatacgttcaaggaaaagttaggcactacctttgttaagaaggccaccatcagtaaccagatcaaggaaaaagatatggaactgtttaaggaaggtaccaacactgcactgaacaggggagcagcaaaatacgcggacgcggttgtactggccggtgataaactggaaaagaaagtagtggatgaagtgaaagcggaaaaaggaaagatcattttgccgttcaaaaaagacaacgatgatctgggcgattaccttcaattgtataaccaattgctgggtaaatagccatcaagtccacctttaaagcgtggttgaagcgtatttaaagcgtattaaaagcatgttcgggcagtaaaaccaatactcactaacaacataacgcgtgaagatcaatttcaggaaccttagcttcttagctatctatattactctgctgtacggagcaaccggttgtaacaaatccactatcctgggaagtggcttaatccctcccggtgattttgtgaatgcacaggacacaacgctcacaggtattattgccaataacatactccggtatgactcctccattttaaacggacaaaacgcttataacaaaatcctgggatctgttaccactgatcctgtttttggcagaactcacgctttcgtatacacgcaggtatcattgcccaaaagtgcctttacctttgaaggtaccgggcaaacactggattctgttgtgttgtcgctggcctataccggctataccggtgactcttcgtcgcctcaaaccttccgggtgtaccggatggccgaaccgggatttacgatcgactccaactacgcttataacaaagcattggcttataaccccggagagttactgggtacggctaccgttacgccactgtcgctccgcgactccgtaagcatttacggcaccaaagaaactgcccagctgcgtattaaactgagcaccgccttcggtaatcagttgctgagccagaagtcggatggcgcttttgccacagattcctctttccgcgcctacctgaaaggtttcgctattgtaccggataccaatctgggtactaacaggaacatgatctatctgaacctgagcaatagcaataccaagctgacggtgttctataaaaacactacagacgattcgcttcgggccactatggcgtttgaccagtatgccagcgcccatgccaattactttacccgtaattacaatggttcccaggcatcgaggtttatcaataccaacaacccgaacggggatagtatcctgttcctgaacgccgcaccgggactgtttacgaatttgactatacccggactggagaacttcccgaatgtactgatcaataaagctgaactggtaattacacaaataacttccggtccaagtgatatgaataatatatttattgaaccaggaagcttatctttacgacagtatacaaacggtgataccaccaagatccccgcagattattatacaggaggaggcgcagcctattttggcggcacccgccaggtaattaccaactttggaggcgtacaggttgttcaatacacctttaatctcgccaataccatgcagcggtttatcaggaaactggacctcaataagggtttcaggctcgaaggatattcgccgttatacatggatatgaatcgtgtgaaagtgggtggtagtaacctgtcacagtataatatcaagctcagaattatttacactaaaccataaaactactaatcccagttttttatgccttatttatttacatctgaatccgtttcagaaggacatcctgataaagtagctgatcagatctctgacgctttgatcgacaactttctggcatacgacgcaaaatctaaagtagcttgtgaaacgcttgtaactaccggccaggttgttttggcaggtgaagtgaaatcagaggcatacctcgatgtgcaggacattgcaagagaagtaatccgtaaaattggttataccaagagtgagtacatgtttgaagcgaattcctgcggaattctatctgccatacatgagcaatctccggatatcaaccagggcgtagatcgtaaatctcccgaagaacaaggtgcaggagatcagggtatgatgttcggttatgctacccgcgaaaccgataactacatgccactggccctcgatctggcacataaactgttgctggaactcgctgttctccgtcgtgaaaataaagaaatcaagtacctgcgtccggatgccaaatcccaggttactatcgaatattctgatgataataaaccggtaagaattgattctatcgtgatctctacccagcacgacgactttgatgaagatgagaaaatgctggcaaagatcaaggaagatatgatcaaaatcctgatcccccgcgtaaaagcacagctgaaaccggaattgcaaaaactgtttgaaggtttcgatatcaatcaccatatcaacccaaccggtaaatttgtaatcggtggtcctcacggtgataccggcttaaccggccgtaaaatcattgtagatacctacggtggtaaaggtgctcacggtggtggcgctttctccggtaaagatccttccaaggtagaccgttccgctgcttatgcaacccgtcatatcgctaagaatatggtggctgcaggtgtatgcgacgaaatactggtacaggtatcctacgccatcggcgttgctaagccctgcggtatttatgtaaataccaacggtacctccaaagtgaaactgaacgatggcgaaatcgctaaaaagattgaagagatctttgacctgcgtccttatgcgatcgaacaaagattgaaactgcgcaatcctatttacagcgaaaccgccgcctatggccacatgggtcgcgagcctaaagtggtgaccaaagtattcaacaaaggcaagaaacacgagaaaagtgtggaagttgagctgtttacctgggagaagctggattatgttgataaagtaaaagcagctttcggcttgtaatcactccggaagcatatataattacaaaagggccgtttcaacttttgagacggcttttttgtttagagccttgtaccttttttattcattcgtgcctcattttttcacattcccctgatgtgggaaaagtttttcaattttattaaaaaaagttcaaaaaaagttacatattactgttaaaattatagtatatttaatagtaatattattgattggcctgcgtttcaggactggcaagcgcattatgggctcggtctatttcggaataaatgcataagggcttcagtggttttccagaaatccgttataactcatatagccctgtttctggcgtataatatttcgcggaggacgtccgttaagatgctgttttatatccaaaaatctggatattcgcagccataaattaaaatggaccgttaaattgtttccggagacaattgtatgcagtgcattatttattgaatgaccgaatccatatcacttgaatcaatttgcaatttaccaattgggtaattgtgagctttttattgaaaccatataatatctgaaaaaccatgaggcactacatcaccgcacgattgtctatgtttacattcgtatcctttgccctggctttagcgatcacaacagaaagttgcaacaaggatcaactaagccaggtattaccagaaaacaatccagctgaaacagccgtaaagcctactgttggcgggaagcaatacacacttgttcccgacaaggatggcagattagtagtggatggaagcatctacaaagcaggagaaattctgaatctgaaaggaacattttctgccgtcgtttttaataacctgaaaggcgcgtcaggcagccctatcattgttaaaaatgccagcggcaccgtagttaaaataggtaatccatcctggagcggtggttcctgggctacagccatcagtttcgtgaactgccattatgtgaaagcaggtggtgaaaaatcaaaatccgaatttgtagtagaaggaagcacccaggcaggcaaggaagcgtatttcgactttacgctgagccagcataccgataattttgaaatcgccaatgttaccatacataacggcggtacaggcatatgggctaaaaccgacccggtaaagggcgacttaagcacccagtatcctaactcctacatggacaacctgctcatccacgacgtggcgatcagcggtaccaacaacgaagcattttatattggtcataccgccctttactggaacctcactgccaacgcaccttactatggtgatccgtcagggtttaccagcggccagcagtacgtacagcccattaaatggcgtaatgtaaagatctataataattctgtttcaaatggaggagcagatggcatccagactgcagccatcgacaagctggaaatatatggcaacaccgttaccagctggggcggtcagcataattcaggtcataacggcggcatcctgattggcggccgtaccactaataccaacgtccacgataactatgtgcacgatggatggggtgaactgatccagttttacggatctggtgaaaatggcgcaacgcacattatccgtaataacctgttaagagataaccagggagatggggtgagcctgagaggaactgataaagcagtggttcagatcaccaataacaccattgcaagaacaggtggcgtgtctctccgtattaacggttatttcggtatgactgctgcgcagatcgtgaaagataacgcgttcattcaaccacgtgtaagtggcggtacaattgcgcctaacgcttacatatacactgaaaatggcgcctctgttatagaaggaacaggcacagaagccaattccaaatttgtatcagtagcagcagctggtgtggacaccaacaatttctatcagcctaaatccggttcagcattgctgaccaccggctatagaacaaactaatccgtactattccgcaacaggcgataataaaacagccgccctggttatccgggcggctgttttcttttttcaccgggcattactttttttcttcgagatacttccacatcatttcattcacttcctgtggttgttcaaaatgaggcatgtgcccggcgctgtctacttcatgtacttctaaagttgggtataaagcagtataagaacttaatttctctttggggaaaaaggggtcttgcttaccatagatgagtaacatttttccggcgggtattttttccagtaaataaagctggctctgattcagcatatgcatccaggacgatagcgtgatgcgcttgtaacccctgaaattcataaaatattttaaccgctctgcgtagttgttgaacagtggctgattcacaaactctttccgctgattttccaccgaacggggataccagtatccactcattaaaacgtctcttacaaccgggatgtgcaacagtttgctgggttgaagatctccgctggcagctggtccgagcaatataatctgtttcacccgtttggggtgactggccgcatagtccaatcctataggcgctcccatggacatagcgatcatatcaaatggctgacggagctgcagtgtatccaataaagcggtcagttgctccctgtacaggccgagatcataggctgtttccggtctgtcggaatagcccctgccgtaaagatcatatgaaagcacccggtaacctttggacaggagatagggaatattgtatttccatacctccatgccgctgcagccgcctccgtggattaataccagcagccgggcagtgtcggggccagccaggctataatgtacatttccctgtgccaggcgtataaactgccccggggcagatttacgcgtacgctcattaagcggcgcggtttcctgcccttgtttgatgaacaggaaagccgctgtcagcagcaatataatgccgcccgccagtgataatatccatttcatgcgcctggacatacctggttatcttttgaattgcaacagccactcgtaaatattcataccatcttcccggtaggaagggttgtaatattgttcccagcagcaatgtttatgatccccgatgctcagtttggtgagtcctggtttgtatttgttggtactgtccgcataaagtttacagttgccaagaaacaccggttcatcactaccaccgaaataccacacgtggatattgttcttggcagttatctgaaagtttttcaggttctctgcatcgatagtagccggcgacatgttcactgcagcagccacccgctttgccgttcttttatcggtaacggccattcctactgaccatccgcctgcactgtatcctgtgatataaatacgggaagagtcaatcggatatcttttcaatacatccgtaatggcagcatccaggtgttccgggccaagcgaccagctggtggccaggggcgccagcacaataaactcatatttcttgccgtccactttattgacagcatcaatattcttcccttcgtgcatttgccttgctacaccctgtctgaagatcttggtaatatcagtaccggcgatacttctgccatgaagacaaataagcaacgggtatcttttcccgcttttcagattgtccggcagcttcagcagcgctggaatatggtgccagggcgtaatctgtacctcaacctgtttaaatggtttcaagtcctgtgcagacaataacgccgtctgcagcattagcgtgataataagaaatactctcattcttgattttaattttcagtaatccgcattgccggatacgatgttcacaatccccgatattataaatgcagcaacacttcttccagcgaggtaccgataattgcttccagtaccagcttcgattgtcttacatctctttcaagatttaccttacgcaccatttctgcattatagatgcggtaagcatcattcaaaccttccacagcggtgttttgatctcctttggagaaacgctgttccacctgtttgtaatgattgtaggagtcttccagcaaaggcatttgcagctcatataactgtttgtttgctgcataatcttcataggcacgcaatacagcagattttaaggccagcttttcgccttctttctgctgctcgaacactttcccgttcgcctttgcagtttttacttcgttaggaatgctgatcaaatgaccaagtggcacattgacaccaaagttatacctggggtataatgtgttgttgctggtggtgccgcttccttttatggtaaattcattcaggttacctgaagcgacgatcatgtccagccaaccggctttagccctgttttcatcgtattttgtaatctgtttttttatgtccaatgctttgatctgcggattttccatggcaagttccaccagtcttgcttttagcctggtcactgtcggcaaatctgctggcaggcgcagcacaatactggtatcggctctttgcgcctttgccattgtacctgttaatgctactaataaaaagaatagtactcgtttcatgttgtgatatttggagatgataataaatattttaattttatagagatgccgttaagggcataataaagcaacgctgattcaataaggccggacgattcctgtgcgtaaatacttactaccagcgcgaacatcacacataggatgaccagtgtaaactgcttttccacttctgttctgctggcaaaataattggcaaccatatattgcattaccaggtaaatattgaccatgatcagtattaagcctatccatccctgctccagcgccgtacgtaaataaccgctgtcggggggaaagccatccagctcgctgcccgaacccggttcgcagctgagaaatccgccaccgataggatggctgtagatataaggttgtatacgatgcctgttcacttcccgcacattcagggaggcatcctctgaaccggaaaaggccgttctcatcctgataactgttgagttgccgtgaaacggcccaaacatcaataccaggaaagcaaatacaaataccagcgcaccaatcactgtattcctgttccgcaggtttacaaacaacatgatgataagccccatcggaaccatgatataagccgtacgggtaccggaaaagcccagtgccataaactgaagtgccagcgatatcagcaggaacacttttttgggtactgatatcattttattggagctggtgagcagtacaatattcatgatacagccgcaggccatgataacaccaaacaccgcaggatccgatacaaaggagaaaatccggataccggtgaggataatcacggtcttgaatttctccgggtatttggcgatgtatgctttttcaaacggcattaatccaaaccactgctgaatacacgcataaaaggccgcaacagtaagtatgatgatccagaatttcaggaatactttcaggtcgttcatgttacggatcattttcatgaccaggtacataaagatcatattgcggacaaataccctcgcaaaggtggtccagccatgccggtcgtatacaaaggcgggattaaaaaactgcaacaacacatagccgccgtagatgtaaaaagtgatcagcaccgggtcccggagaaagttaactttcttgatactatcgtctccggcctttaataaactaccgagtaatgtgatcagcagaatggcatctattaatacgcccacaggtatttccgtaccggacatcctttcgagcaaacgcacggtcagcgccactgtacaggagataaaataacctgcacggtaattcagaatggaaatcgcggcaacagtgattcctatcaccaacccgatcagcaacgcaatgtattttacctcctgggcgccgatataggctattgccgggatcagcagtacccaaccgataataataaatatgttgaaaatatttttcttcgcaatttccacttaggtcaatttataagaatactattttaatacccatagcgataatagtaagcgctataaagatgagaatcagcatctggtgaagatgttggtctattggctttttctttggttgcgttttcatataaaactatacgtcatgatttttccatttgaacggctggtaccaaactttcccgtaaacaggaaactgcatcctaattttaccagtaaacgataagcaataattgaaagcaatatcgaggatggtatacagatcagcagcaacacgatcccgttggttatccctatgcccagcagtaccgcgcgtaaccccgcaaaaacagtaatgtgcaggaggtagatgtacagggaatagtggccggttatgctcaggaactgcagcttgtgcagcttcgcaagccaggatgccagcatgattacaaataagcagccattgagtgcaatgagcattaacaggtacaggttcatttgttgatgatacaggtaataccattgcagcacacaaaacaccggcgtcaacatcagcaggttcaccgggttggataactgttgctgtatttgtatacggaaaaagtaaaccgcagtaatatccccgatggcaaagtagatgtagtgcagtgcgatgtcataaagcgcgctgctgctgtgcacatatggtgccacgccaagcagtaccagtcctgttaccacctgccagtactttttctctttgaacacccgtgatgtgagcagatacaacatggtaacattaaataatgcaaacaggtaccacaactgatccagtgttctgggctgaagcagtatattcaggaaatccgttgcggaccgttccgcatttgcgtatttcggaaataagatctgcaaactgatttgtatgactgcccaaagtatataaggatataatagcgtattgatcttcgatatcccaaagttcttggcacctcttttagcaatacttctgctgaaaaaaaatccggaaagcaggaaaaataaaggcatcctgaaactgtaaagcatgtcgtttgtggcaagtacttctttaggaagagatacgccccgcgccaccagaccatatgccagatgacggtaaaccaccagtacaatggctattcccttggcatagtcgatccaggcataacgcgaatcatttttttcgggccgcaaactaaatatgtctttaaagatccgttgatacatatttaaaagatcaaagctcaataaaatcttcttttacattattcaaaaccactcccaggaacttatcgccgagagactccaggaactcggaagattctctgtcaatttgtttcattttcaagcgggaggagaaaattgctaccacaccttctgcataggcagccagttcccggctatctgtgaaatcgttcagtggggcgccttccatcaaaatataatcgtagtgttttttcagttcaggcaggtaattgagcaggtggttgggcggtaaaatttctgatggcgtatagtcgccacctttacatccaataatttcaatacccggtgtttcgtaagtagtaacaatctcttttactttttcaatggaaaactcttccggtggtacagagaaatactccagggttggtttcgcttccatttgcacgcttacatcattgttacagaagttggtatcgatgatcaatacttttttgttgctcaggctgaggctgtatgccactgcctgcagcagtgtggttttaccctgctggggttctgtactggtaaacaggaatatttttttgccactgctttccaactcatacctgagtttacgtaaaagttcgcggaaaacattttgtcttttcagccattgtgcctcatccgttttacgttgtaatatttccagcagtttatatctctgaagattagtatgattgatggtagcaatcaacttcagattggagctgcggttgaatacagaaggggatttcagtgagttgtccataaactccctgaaaaggataccgatgcaggagatcataaaaacagccataccggacatgcccataatgacgagccgtttggatgattctggtgtgaaagccggttgtccctttaatgtctggcggaaattatcctgtggcacattccggttatctaaggcggagccgagtttttctttcagcttattatattcatcctgagccagttccacttcctgttgcagggaagttaccgtagcttccttattggcataagaaccaacggaagaacggagattacggatctttgcttccagggtactgatatttaatttagcggcgcttacctgtgcttccaatgcatccctgctttggatcagctcttcacgggtacttactttgcccgtagtagaagaagcatccagcaatatcttttgcaatttggcgcgctgcgtttttattttttctgccagtgcattatcagtggagccggaatttacatactggtcgttcagatcgttgatctgttttctcagcgtaactatttccccatttgaattggagtaggccggtttgccactggttgcctgggccaactgtgtgttcacgttgtcaagagaagcctgaaggttattgtagttcgccctttcgtctgatacagatttctcaaattgtttgatcagatcccattcgttgccgctggcggtttctacgtttaacacgccttgttgtgttttgtaacccctgagcgcttctactttctgctccagttcctgtttcttttggtttaccagtgcttcaaatgtttctacgttttcaacagagcgttcagaacgggagctgcggtaaaaacggataaactctttgtaaagggtattaacagtgtacgccgataattcaggattatctgaataacagatgatgttgatataatctgtacgggaaagacgtgcggcatacagcattttacggatagactcaaagtcgtaccggtaaatcttcatgaactccagtatttttctttcttccggctgggaagaagaaagtatctgcagcgaatcaattttctgacggcagatgcgcacaatttcttccttgttggcactggtataatgaggatctttcagatctttttctgaaagatgtctgaaaggtttagtggaggtgagatcgtgcaccatgaggtcacaggccagtaatccgattaccagcggggaattcatggtttcgataacgttatcgaatttaacatctgcttcaaagaggttcagattttcgtcccgcagtttgatttgttcattcgttgtaaaacctgtcgccatctgggcggtagaggcataaagtttgggtttgccgatggtaaaggcaaatgcagctgcaacagcggcaatggtgctgaacaggatccaccatttctttttaagcaatgcctttataaaatacacaatgtccatatagaatttttcctttaagctttaattgatacgcaggggtaggtatacgtaaatacacgtacatcggccttgtcccggcgtggtaactggtatgtcagaggagatggtaaaaaataagatgataatgtcaggcaagaagccctacaatatatcaggtttttggctgaggatgaggttaatggggagatatccggggagcaaagctatcctggtatatccggttatggctcaaaggtaaaagattatattaaaacacactttatttttaagcgaaacataaaaattagttggtaaccgctgaagtttggcgggtaaagcgattattttataaaaaaaccgttccggaacattgcccggaacggttttacttttatagtaatcattcagttacaactcagttctgcctgataagtttaacgctctttgtttcaccggtagaagaagtgatcctcaggatatatacacccggcagtgtcactgtacgctgtgtattgatccttatcaggtttttaccctgtggtacctctttcctggtttcgctgtaaaggcgcttaccactcaggtcattgatttcaatgagcattacaggtgctgttttctgcagtgtcatatcaatggccaggttatctatataagggtttggataaacgttcaccagcatactgctttttgcagtatttgtggtggtgatcattgaattacccgttcccatcagctgcgtattattgcccaggttctgaatgttggtggtggcaataatttccattgcattcagatagcctacctgaccgcccggagggatactaagcgtaaacgcaatttcaccgttagcgtctgctgtaaggttcgcgaaatctgcggtggtgctggtattgttttgcgcattcaatgttttgcttacaccattgatggtgaactgggtgctgccgttatcaggctgcggcgcccaccatttactgttggacaggaacttgatggtataagtggtattggcgcttaacccggtaaggtgaccgtgcataaccggtgcgcctgtaaagaagccggataatgaaccgaagtacaggtattcagccagtaccgcatccgggtacacaccgctgttattaccggtggtagctccttcaacgccggcagcccaccatgtttcgtcaaatcttaatcctacggaagtggtttgtccctgatcattcttcaggttggacgtagcgcctgtaatgttattccacggcgccggtaccgtattattgagcttgaagttcagtaacagtttgtagctgccactggtgttaggcgcctgggttaccgtgatattgaatgtagtggtgtcggcagcgccgtatgtatccttcacaataacttttacattattgtaagtacctgcatcgctgatagttggcgctacagaaagggatacactaccacctgattgtaccagggtaacaaaagaaggcaggttgacggtgctatacgtaatcgggttgttgtccgcgtccgttgccgttactggaacattcagactggaacctgcctccagactctggttggtaatatctgttattaccggtgcgtgattgactgccggtgctgaggaagtacctgcaaccacttcgatcgcattcaggtaacctacctgtccgcctgcaggaatactcagcgtaaatactatttcaccatttgcgtcggggctgaggtttgtaaagctcaccacgctcgcagaattgttttgtacatacagtgtctggctaacgccgttgacagtgaacttcgtgctgccattgtccggctgcggcgcccaccatttactgctggagaagaacttaacggtaaacttcttaccggcttccaggccagtaatgtggccggtcatgcttggtgcccctgtgaagaagcccggcaatgagccaaagtagaggaagtcgttgatcactgcatcggggtatacgccactgttattaccggtaatagcgccttcgccgttggtagcccaccaggtttcatcaaacaccaggctcgatgcagttgtttgacccttgtcgtttttcaggttggtggtcacttttccggtaacattattccacggtgctggtgcagtgctgttttgtttgatactgaggagcagtttatatccgctggtatctccacctgccggtgcatttacggtgaggttaaataccacggtgtcgctgttgccatgtgtatcagtaccaattacgccgatgttattaaactggcccgcattgctggtagcaggagccaccaggaggtaaggattactaccttgtgactgtactactgaaacaaaggcagggagattataaccggtgtacgtaatggcatcgttttcaggatcggatccctggagctgtacatgcagggtatctccggctgccagcgttttattcggaatagccgcaattacaggggctttatttaccacgacggtagtatcgccggctccgcccgcgtttatttccatcgcattgaggtaacctacctgtccgcctgcaggaacgctgagggtaaatttaatttcaccattagcatctgctgtcaggttttcgaaaactgctgtattcgtagtattattctgaacgttcagggctttggttacaccattaatagtgtactgcgtgctgccattatccggctgcggcgcccaccatttactgctggagaagaacttaatggaataagtcctgtttgtttccaggccggtgagatgtccgtgcatagccggcgcacctgtaaagaagccgggaagcgaaccaaagtagaggtactggctcatcacagcatcagggtatacaccactgttgttgccggtggtagcaccttctgtgccggcagcccaccaggtttcatcgaacgacaggccaacgctggtggttgttccgttgtcgtctttcagattggcggtagccccggtaatgttattccacggtgcaggcgccatgctgttcaatgtgaagttgaggagcagcttataattaggcgttggcttatctaccaccgttaacaggaagctgcgcacatcaatgccgcccttgttatcggttgcctgtaacttaacagtataagtaccggatgcaccaaatcctggttgcaggttgatgacacaggtatcattattactggtgatggtggcaaaagacgggatctggagtgctgtccaggtgtaggtattacccggattcagatcatgcagggatacctttacgttcctctgcgttccttcatccacgctccatcctgcaacagaatctattaccggaggatagttatcatttacgatgatattgaacaacgcggtgtcctttcctccgttagcatctgtggcgatcactccaacaccgttataggtgccctgctgcgctgctgttggcgccaggatcagggaagtggtaccagcgttctgctgcagggagaagaatgcaggtgcgttataaagactaaaagtaatcacatcattatccggatcggtagctgacagcggtatgctctgggtggtgccatagcggatcgtctgactgctgatgtcagctatcaccggtggattgttcagtgattttgcgattaccgctttggtaaatgcggagtaaccaccttcaccaaaagctcttaccttatagtatacaattgtattggcgacgagggaagagtcattgaacgttccctgtccggaagccacaggaccaaggcttttcagcacgctgaagtgcaggctgtctgccagggaacgctgaacttcgtagccagtttcaatggtgctgttatcagtccaggttaatttcactacctgggtggaaagcgcctgtgtaacgaggttggtgggtactaccggtggtaatggtttagctgctgtggtagcattggctaccgacgtgtaagcagattcaccataaaggccgatagcccgtatcttataataataaggagtggaagcgttcagtgcggtatctgtatagcttaccgcgttggcagctgcagtagccacaatggtataagtgccgccgctgctggtgctcctgtaaatttcaaagcctgtttcattattgctcttgtctgcccacgtcaggttcagtttactgtaattgtttacagctactgcgagggtggttggggcggtaggagcggtaccattcactactgatgtatcaacaaaggcctctgctggtatcagcgtgcgggtattaatgcctgccgcgctactggtccagtatacgcccattgcagaaccgccgctaccctggaagtaggtaaccgtgataggatacacaccggcactgataattacagtgcctgctgcataagccgccgcatgtgcgccatcgttgtttacggtagcggtagcagagttggaatatgctttattaaaatacagcttactgccatcatctgaatacgtttcaaatttataggtaccggtaacagggatacggatataacctgtccacattacggcgtagttggtggaaacaccggctggtacgatactctggtcaggcacataagccttgcctgtttgcgcaggcgtaagattggtgaagttgggcaatgtgctgtaagaaccggtataatatttataattaagatttgcctttttggttctcaccgttacctggttacttggagtagatgattttcccgacacatcttttgctttcacgtagaagttgtacaaggtgccatctgcgagaccggttacggttgcagtaagtactttgcctacggaggttaccaacacattgtttgcatagatatcatagccggcgatacctgcatcatctgtagcagccaaccagtttaatattacctggttattggtgtagctaccgagggttaaagacggaggggcagaaggagcagagctgtctgacgcagtggtgcctttcacttccgcagaaagaggcccggctgcattgtcgtttacaggacgtactttatagaaatagctggtatttggaatgagattgttatcagtaaaagtaactacgttggcattgtttttaccaacaagtatatatgggccacccgcctgggttgcgcggtatatttcaaagtacttttcgttgtaggccggtgtggcattttccacccacgacagcacgatctgtgttttggtgaaactgtttatagccaggctgctgataggatcaggcccgtttacaccagtgctgtttataatccggaaagtatcggagtaagtaccgatgcaatagttgggtgctgtaacccgcactacatatgctccgggagtagaagtagttaaagtgttagtggtgctgagaacggtagcgctgcctgcacgtatccattcatagttgagcataccggccggtacctgcatggtaagactggtagtgccatccgtagccgggagcacattgctggcaagggcaggggaggtagtaatggtttgcgcaggagaagcaggtttatagctgatcaccagcggggtaactgaccagccggtccagccggtagggagttgtcctcttacgcgataggtaccgggagtggtaaccacgattgagttggatgtgccggtagatatagtgacgccatctttctgccattcatactgcgaaaatcccggcgctatacctatggtaatagtctgaccaggacaaaaagtggatgaaccatataatggataaggattcagcctgttggctctcagcatgaagggaacaaaatctgcttcattccatgcatcgttccaggtattgtgttcatcgttgggataagtagtgagtttaaaattagcaccggcggcattaatcaatgccaccacctggttggtagtataaggagccgggttgccatccaggccaccctggaaaagccacatcggcgtaaatttgtaggtatcaatatgattgccgtagtctatggccatcgcactcattggcaacgaagccgccgttaactggggatagcgcatggtgaattcccatgtgccccatccgccaccggacaatccatttacgatcaggcgatcgggatcgcctttcgcactggtaacaatggaatcgattacttctttcaggttatcgtagtcgttggggccccaatagccaccctggctttgaggatatattaagtagccgtcgaactgaccattatcaacgcggttggcccatgtctggcctccccataataaatggaattcgttatcgtagatggtgcctttttcacctacaccatgaaagaacaggtagatgggatatttttttccatcattcacgccaggagcgtacgttttggggaatttcaggcgaaacgccatgttcttataaatgtagcatttataagaatctgtgttgtagctcatcctgactgttctcacccatttggtgatcttatcatactgtggatccgctgggggattggcaggattgtaagtgataacgggatcactggggtttaatgctgtttgtgccttcactgctgatagatagcagagacccaagagcattaaaaggagcatgcggtgtaaagttcgattcatggaagtatgttatatgttatgttatctggcagtcattcggctttaactgcagaaaaaaaagtataacaagcactgatccggaaagccggatatacttgcaattcaaaggagatggtaaaaattaaatacactccggatatctatccaaaggtgacgtggctttatcgaaggatgaggtcttagaaaaatggctgtaggtaaatcatcaattcactgatggtgcatttgtattctcagctcatttgtgacaaaaaatgattctacaattggtttttatattcaccgctaaagtaaataactgtatctatatataaggaatttttttgcaaacggcgtttttttgctggtaaacgcaaatttttatcgggtgaaataaaccggcactccattattgaacggcaatactccgttgtgcccgttcccaaacagcagattgccgcttcctgaagaagcgtatgcaaccgatgtaaacggctacgttcataaacacaaagtaaaaagggatatagaagtatttcgctttgatctgcttttgggcaagtacgtaaccggtaaatgcggccatatagaaaagcagctgtaatacaccggtaattatatatacagggccgccattgaacacgataagaagaatattggcaaccagggccagtaggagggacaagggcgcaagcgtccagcgcagcacccggtgggagatatactgccacgtaattttaggatacctgaaaggattcagcagcgggagcagccggcccatcgactgaaatccgcctgcgctgatccttactttacgcttatactcttcctggagggaagcagaagaggtttccatggcgtaggcggcaggttcatacattacccggtaacctttcatgtttattttaaatgaaatcatgaagtcgtccagtatggtatcttcctggggctgctcataaagcgcagtacggatcgctatcagttctcctgcagcacccattacactatacagttctgcatcccattttttcagtaacgattcatatttccagtacatgccctcgccctgggcttctgcaccgccggtagtagccattactttcttttcgccggccaccacgcccacctggtcatctgcaaagtgctgcataagcagggataccgcggcgggattcagcagggtattggcatcagacaatactacaaagggagtggtaaccattgccatggcccggtttaccgcggccatttttcctttgcgctgcggatcatataataaggtgatccggggatgctgcgaaatgatctcattggtgttgtcggaagatccgtccgtcacaaaaatgaactgtattttccccgcagggtaatccattgcgaggctgtttgctatcttttctgcaataaaatcttcttcgttataagcagctaccaggaaggtaacatcgggtacaaaaggtgcggccgcatcagcttttttgccctgtaatagccgtttgacgcggattacaagataaagcaacaaaccatatcctacgtaactatagcatactataaaaatgctcaaccagaaaatcacagacaaaattgacatagaggacaatacatttatggggatacgtatgttttcagtgcaaaagtatcataatttggatcatacgcaattgtatttttatattagatcgttgtttcatatcgttttattgacatcattccgaccgtttacagtaaaaattgcaacacttaccctccaaattaagtcgtttaccaaaaaaagtatctatgatatcctgaaaataatacttttgcttcatgttcatcagataacagatctggtaacgaacagcaaaaatgtaaaaaccatctttcctctctcatatccccatgttaaaaccgcagaaggtaatttacctgactaataattgaccacatcccatcaaaggccttcgggagtttgcaaaataatttgcacgtcccatattaacggttttaataattgtttgtaaagaaggtataaatgaaaaagaaaattttagtaatagacgatagcatgccgatgcgttatttgctggaggcagttttaggaaaagaatattcggtagtttccgcacaggatggactggtggcaatcacctggctgctgaaaggaaacaaagcggatcttatcatcaccgacctgcagatgccgaatatcgacggctgggaactgctggattatctgtcaggcagctatctctaccaggatacgccggtagtggtactttcgggattctatgccgataaaatgaatgatctttcaacaaaatataatagtgtgagagaagtgctgcaaaagcctttcgacccgatgcaattgttaaataaagtggattatatacttgagaaacaattaagtgctgctgctgtataataaatgatattgtcacctacgaatacactactaatttttaaccgatggatacctttactcaaaatttactgcaggtagaaagcatcagaggagtagataccggtaaaagctccctgtttaccaaaatgccggacgctgaaagtattttgctttttgttggcgccccgcataagggaatgctgacagaaaacgatcagttcagatgcatagtgaccgagaacgtagaagatgcgcaaaaagtgatcagtcagttgcagcacgtttttaagaaagtgcctgcggcaattatttaccgcttcgacagtgcctatgaatcggccctttctgaatgggacagctattttaaaacacaccagtttctttgctccattccttttttcgtatacacagaaaaaggatttgatgaaatgaaatcgctggtgaccaggcattcatttattgatgacatcatcacaatggaggcatggcatatgctgggtaacaaaattgccatcgtgagcaagtttaaacgtatgcgcaccttcccggtatataaaagtagcagtctccgtacccggctatacaaccgcaaattttacagcaatttcctgaaacgtacgctcgacgtaacactggccggcagcggcttaatattgctgagtcctgtattgctgacgattgccgtattgatcaggatggaatccaaaggtccggtgttctacgccgccaagcgcgctggaagaaattaccgcgtcttcaaattctacaaattccgtacaatggtacctgatgcggacaagcaactggataaaattaagcacctcaaccagtacgacgggcagacagacggaccggtttttataaaagtatccaatgatccgcgggtgaccaaactcggcagcttcctgcgcaataccagtttagatgagattcctcagctgctgaatgtactaaagggagatatgtcgctggtaggtaaccgccctttacctttatatgaagctaccacacttactacagacgaatgggtggaaagattcctcgctccggctggtatcacaggtttgtggcaggttagtaaacgcggaaagaaggatatgtccgtaaaagaacggattgacctggatatcaattatgcccataaacgctcactcaggtatgatatgtggctgatggccagtacgccgttcgcgcttgttcaaaaagataatgtataatgataacgattattgaagtaatactgtttgtttacctggccggttgtgtattgtacaatctgttgttagccatcgccggccgtttgagccggaaaaagaagattgcatacgaggaaactgttgattacgcgaggattgccattctcatcccggcatataaagaagacagtattattttatctactgtaaacagttataaccgcctgcgttacccgtcaaagcattttgaagtggtagtcatcgcagactctttgcagtcacggaccatggcagagctggcagcaacaggcataaatgtaatggccgttaagtttgataaaagtaccaaagctaaatcgctgaataccgcttttgaaaggttgggagacaattttgacctggcccttatctgcgatgccgataatatgctggaagcagattttcttttgaagatcaatcacgcttatcagcaggggcaccacgctattcagggacaaagagtagccaaaaaccttaacacgcctttcgctatcctggatgcagccaatgaaatcatcgccaatcacctttaccgcaaaggtgccaatgcgcttggattgtcctcttcggtaattggttcaggcatggcctttcactacccgctcatcaaacagatccttagtgaaatacaggccaccggcggatttgacaaggtgctgcaactgctggtgatctcaaaaggacacagcattttatacctggaagacgcctatgtgtatgatgaaaagattacgcatgcagccgtatttgaaaatcagcggaaacgctggatgtccagtcagctggtatacctgcgcacattctggagtaaaggatggtcggctttattcaaaggtgacatcaattatttcaatcttgcggtgtgccagaatgcgttgttgccgcggatgctgctgctggcagccttaacggtttgtaccgcgctttcattgctgctggagcactttgtaccggtttcagtttactggtggagcgtgttgtttatattgaatatagtgagtttgctgctgcctatcccggggaaattttttacaaaatatcttttcactgcggtggttacgttaccacgtgctatcggcatcatgatattattgttattccgcctgaaaggtgcagataaaacttttatacatactactcatacccaaacaggtattgacaatcctttattagatgcagccagaaagtaatacatattgtccgctggtatccattataaccgttaattataacaatgccaaggtaactgcggaactcatggcctcccttaacaggatcagctaccccaacctggagattattgtagtggataacgcctctgcagaaaacccggttgcggtgataaaaaatgagtacccgtctgccatcgtcattgaaagtaaaagtaacctgggttttgcaggaggaaataatctcggtatcaaagctgctaccggtgaatatcttttcctggtaaataatgatacagaatttaccgaaggattgatagaaggcttactggaagtatttggcaaacatccggatgccggtgtggtaagccccaagttccattacttttttcagaaaggaaccatagaatatgccgggtacaaagcagtggatacactcacgggaaggaacagtatgattggttgccgtgaagaggataaaggccagtacgatgcagtatcagaaacacattacgcccatggaggcgccatgatggtatctgcccgggcccttgcaaaggtaggcctgatgccggaagtatatttcctgtattatgaagaattcgattggtgcgaacaattcaaacgccagggatataagatatactaccagtacaaatcgctgatctatcacaaggagtccatgaccaccggaaagaacagcccgctgaaaacgtattatattacacgtaaccggatattattcatgcgccggaatgtaaagcttccagccagaatgtttttcatgctgtattttacttttcttaccattcccaaaaatacccttcagtttttactaaaaagggaatcggttcatatgaatgcattctggaagggaattttctggaatcttaaacaccctaaaccagataacatatgtgtggcatagcagggtttattgattttacccaaaaatcagacgcagacatcctgcgtagcatgacagatgtgatggcgcaccgcggccccaatgacgccggatatgaagtgtacgaacatccacaggcatctgttggcctcggtcagcggcgtttatccatcctggatctttcgaagtccggccaccagccaatgcactacgaacaatattccattattttcaatggagaggtatataactttaaagaaatccgcacggagctggaaaaactgggtcaccacttccattccggtgctgatactgaagtattgctgaaaggctatgcgcaatggggtgaaaagatcctggataaatgcatcggtatgtttgcctttgttatttatgaccgcaccgcagaggaagtaacgctgttccgcgatcgcgccggggttaagcctttatactactactggcatgatcgcaccttgctttttgcatccgagttaaaagggatttgtgaacatccggctttccggaaagagattgatgagaagagcttgtccctgttcctccaatacagctacattccggcgccgtacactatttacaagaatacccataagctgaaaccggggcatctccttaaattatcgctccgcgacgctgctatccgggaagtccaatactggaatgtactggatgcttaccgtcagccgcttacaggattatctgagcatgatgtcatcaagcatacagaggaactgatgcatagcgcttacagttaccgcatggtatctgatgtgccggtgggcgttttcttaagcgggggatacgatagtgccagcgttgcggcactgctgcagtccaatacttccagccgcatcaaaaccttcaccattgggtataaggagccgcagtgggacgaatcaaaagaagcgaagaaaatagcgatgcacctgggcaccgagcactacgaatggatagtaggagccaacgatgcgaaagacgtgttgcatcacttaccggaaatatatgatgaaccatttgcagataattccaccgtacccactacgttggtcagcaggtttgccagtaaagaagtaaaagtggtcctctctgctgatggaggcgacgaagtatttgcggggtataacaagtttaaccagtcgctccgctataccgggagtttcccaaagcccttacagcgcacgcttagcgccgccatgtctgtggtatcgccggaaattatcccttactttaacaagcaatataatttcgcgtcccggtacgaaaaaatgaaactgatatgggccagcggtaaaccgcagcacgccctaaaatatatcagccagtacctgacagaaaatgaagttaattattataccgccgtaccggcagatggttataaaaccaacttcgatatgaacggggagctggataatatgaatgatcccctgaacaggttgctggcagtggactataaaactttcctggtagataacaacctggtaaaggtggacagggccacaatgtcggtgagcattgagggacgggaacctatgctggatcaccgtttggtggagttcctcgcaaaagtgcctgctggtcttaaagtaaaggatggtatcaataaatatatattgaaaacaattgtacataagtacattcccaaaaccctgatggaacgtccaaaaagacctttcattgctcctttgcaggaatggtttaaagacgagctgaaagaacagatgcaatattatctgtcaggtgagcgcctcgcaaaatcagggcttttcaatgtgcctcatgtggagcagctgttggaaatttatttgtccggaggaaaggtgagtcaccagaaattatggaatatgctggttttccagttgtggtatagtcgctggatagaaaagttatagtatgggcaaaacaaatggtaaaacacgggtacttgaaaccatccgccagggtaaaattggcgggggagagagtcatgtactggacctggtagcctcgctggataaaaccgcgtttgatcccatcgtgctttctttcacagaaggccctatgataacggctttacagaaaatggatattcccgtctttgtaatcgaaagtgagaaagcatttgatatcagcgtctggaaaaaagtaaaaaaattcatgcaggaccagcggatagatattgtgcatgtgcatggtacccgcgcaaacacaaatgtgttgtgggccgcacgccgcctgggtttaccggtggtatataccattcatggctggtcttttcatgacggactgcatccactggccaaacgtctgcgtattgctgctgagaggtttattaccggtaaaactcaggtgaatatctgtgtgtcggaatccaaccggcaaaccggtgtcaaagcatttaaagattttaccggtattgtggttcgaaatggggtgaacctgcagaagtttaatcccgatcagtcttacccggacttgcgcgtggaatatggcataccggaagataaactcctggtttgttttatagcgcgcatgacctatcaaaaagacccggtatgtatgatcagggggtttgcgggagcgctgcaacaggcgccgcagctgcatttgctgatgataggagatggagaactgatggatgctgcggtaagcgccgctgcggaagcaggcgtggaaaagcaggtaactttcgccggcttccgccaggatgtacccgcagtgctgcatgcagcggatatttactgcctgccctctttatgggaaggctttcctatcggcgtattagaggccatggcaatggggaaagccgttattgccagcgatgttgacggtaccaaagaagcggtgaaagacggagagaacggactactggtgccatcagctaatcccgcggcattggctgaggccattgtgagggtggcaaaggataataccctgagggctacattgcaaagtaatgctaaagcggccattgcggcgaatttcaatgtggccggtatgacagaaaaaattgcggctgtatatcaacagctttgtaaataataacattttatcaatttcaatatgacaaacaccgtaatcacctacgaatatgatcggatcaccgatataaaaagactcaactttataacggatagtctgaaaagcaacattccggatgggggacgtgtattggatgtaggatgtggtaatggcgttatcagccggcatctcggacagtttggctatgaagtgctgggaatagatatcagcgagaaaaccattgccgttgcccaacagcgcaatacttatcctaatgtgaggtttgcagccatcagcgcagaagcgcttactgcccagggcgaaacgtatgatgccgtaatatgcagcgaagtactggagcacctggatcacccggggctgctgctgaacaccattcacgcatcactgaaagacgatggattattggttgtaacggttcccaatggtaatggccccagggaattgtgtgtaacaagacccatgctcaaagcgcgcaataaccccgttttgtggaagaacattaataaagtaaaaagtgcactagggtttaaaggtaccactgcacaatcccaggcagataacctggatcacgtgcagttctttacgcgtaaagacttacaggatctggcgcaggcgagtgatttcaaaattgtgaggtttgcgaaaacgaattttgtggaagatgtatttcctttttccctgttgacaaagcgccttaaattcctgcaaacgctcgattgccaggtagcagaaatattgccgtacaattttaccggtggctttaacaccttatggagaaaaagtgccggttgatttttgaatgttggtacaaatagagaaaggctgatcacggtgatcggccttctctttttacaggcggttggccgccgcatctattttatccagtagttccggcgttttatccatatcaaatttacgggccagtaatttacccgaccgcagtatagcaggaaggtcgctcatggtaaacgttttgggatgcgcatgtccttcggaccagtctatataccgctggtagttattttgtacgctgttcttaaagggcccgttcataataatggtctggaaaatgaattcatcccctccccaggtatatttgtaaaagcgctcaatctccgggtgatcctggatataccgcaggcaccaggtggcacattcctgtgtgaggctccaccagagcgatcctccatacacttccaggttcaggggatgacgcctgtggggcaatattttattgatccatgccgtgatcctgtatttccccggcaggcggagatcttcaaaatgataggaggtaattttgggcatcatctttttcagttcatccgcaggaagcagatccaggaattgttgtcctgcgcggttgctgaaaaaatcatagaacatattcatatccgtaagcggataatcctgtgcactgatgagatgaataaagccatattgactgcctgagccggcaataaattcgattccgttcaatgctgcctgtatggttccatatcccgcccaggtaacatttacccgtttttcaataaagtatacctgcggcatattcatcgcctcctgccagtcattgatatcagatttggcatcgaggtgtatataacaatcaatggcagggtgttgcagcctgttcagcaaccggcatagttgcgccgggtttttatgactcagtataataaaagcgagtttcataaactgaagattatttatactgtaaacggaacagttttatttttgacaataacattttgcattcaaaccagccgtagtgccatatacttttcaggttcaccgcgggaagataacgccgcaggaaaatatatccgaagatgaccgcaaataaaaggttcagggaagaagcaacagccaccgcacggatatctgcaaaaagcaataccagcgtgatatccagcacaatattcaggatcagtttaatgagatttttgtagaagttaatcagcggtttgttgatcatatccagtgtaaccccaataaagcggtcgataggatagaggatagccgagaacaggaatatccgcacaatatctgtggccggcaaataggctttggcggccagcaaaaggatcaggggtttggtaaagagcagcaatcctaccacaaaaggaagaatgagaatggtaaccgtaccggtatacctgcaaaaggcacgggatacttctttccagtcgttccggttggcagcggcagaaatagtgggctgtgaggtggctacaaaacttctcaatataatttcaattacctccatgaatttctggggaatactgtaaaccgctacggccgcaggattgagcattgttctgagtaccagattatcggaataattcagaaaagcagaagaaaccatactgcctactatcagccgcccgtaatggtacagttcttttacctggactttcgttctggcagccatcgttgttaaagctgtccaccggaatatcatgcaataaatgctggtgatcagcagcgataatgaataggtatacaatacgttgtgaagtgttacctgtttcatcaggaacaggccgccgagtaaaaccaggaaggacccgttttgcagcatacgtatctgtacaattttatcaaacctatgcgcagcctgtaatacccaggtggcaaagttaaaaggcagtgaaaataaagtcatgactccgagccatcccaggaaaaagtgccaggtggcgctgaaatacggataagcaacggcgtataccaggaaggacagcaggataaaagagatagtgagtaccagggaaatgtaccaggcagccccggtaacctgcctggtaacagcaatgtctgttcctgcgctgaacttaataatgccggattgcagcatggcggtgcgtatctgatccaggatattgtaagtggccagaaataacacccattcaccaaaggcgctcagggaaagcatcctcaccagtaatgcaaaggaaagtacgttgaaaaaagccattataacgtttcctagaagggaatggaaatgcctgttacgaacaacagctaaaagtttaaatgccatgaaccattaattacattcaaattgtatgaaaaacaatggtcttttacaggatgaggctaaaaaaaagaggaatattcgatgctcagaataacaaaggtagtttttttatttagaataaatagcatcgcaaggagagatagattgaaaataaacaaataaatatagatataaaatatttatactttatttattgtaatgatatatgttaatttttttcattatgtgaattaaaaaaaagctttctttgcaatagtaaaaacccctttttccgggaacttttaagtattgactatgaggatagacttttaaaaaccaattgcacaagccatatatttatatgataaaccatctgctattgctaaggcaatttttttgccgcggtatttataggctaggcgctgttatattattaatatcctgttttgggtcggtccctgttttcagccaggttcagacagcgcgttcgtttagtgatcctacgatgtccaatatcaaaggcttctatgaatatcttcccgccggctatacgcccgggagtggaaagaaatatcccctgattattttctttcatggcaacggggaactggccagctatggctctccgttatctgcagtactcagaaatggtctcccacgggtaatcaacgacgggaaatttcccaccaccttcaccgtaaacaatcaaactttttcatttatagtgatatccccccagtttaacacctggccgggttccggagatgtgacgctgtttaaaaattatcttcttacaaaatatgatatcgatccttcccgcatttatatcacaggcctgagcatgggaggtggactaacgtggggcacgctctgtgaagataaaaccaaggccaaggcttttgcagcagcagctgttgtttgcggcatgtatccacccaccaccgcctatgctgcggtagtggcttcaaataatacaccggtatgggcttttcataacgacgctgatccaacagtgccttccgactattcaaaaaactgggtaaaatatattaatgccaccgtgccggcccccaatccgctggcaaaactttctatttacagcgccgcttcccacgatgcgtggaccagggcttacgatcccgccacaaaggaagatggcaaaaatatgtatgagtggatgctgcagtatacgcagggtggaacagtacccaccacgccgccacccgttacaggagggaaacgtattgttgtaccaatgagcaacaccgccaacggacgtgcagaaatgtattatccggacgcaatgaaaacacttaacgtaaatcccggtgacacattatgtattccggccggagaatatgaatacctgcatctcggcaacctgacgggaactgcagcgaaacctattgttatcatcaactgtggcggacaggtaaagctgggcgtaaagaaccagggcactgcagccgtattcaatgcgccaacctgccggtttgtagagataagcgggagcggagataaaaattatgaatttgggtttgacctgaatggtacaaatataacaggccttaaaatattcggtcttacactgggtatgggcgcctccgattttgatgtgcataatgtctatatccacgatggtaacatcctgttacaggcaaaaaccctgcaaacctgtgcgcagcctcaatacctcgaaggcaactttgtaatgaagaatgtgaaactccatcacattaaatgccgcaactcgaccggtgaaggtttttatatcggtaacacgcattactactggacagaaggcacctgcgttgatatgaagtcgcactggattgaaaacctctgggtatacgacaatgacctggaaaatattggcagcgacggattacagatctccatggcgaagaatggtgacaaccgcgtattcaataaccggttggtaaattatgccacttcaaagaactctgcacatggttacggaatcctgattggttccggttccgccctgaaagtttataataacaccatcaccactggctatatgccaggtgttacggttttcggttcgggcgtaagcgaaatatataacaatgtgatctctgatattttttatgaaggaatcaacgtggcagataagattccggaaaacaccactctggatgtttttcctcctcctgctgccatcatctacaataataccattgttaatacagatgcaggtaagaacggtataaagatatttgcctaccagacacccatcgggcaccaggtgtataataacctgctggtggaaacaggaacagcctacgattatccttcaaagggaatgtatattaaaggagaccagcctattaagctgaccgccagcaacaatctttgttacacagatgtggcctccgccaaatttgtggacggagctgcgaaaaactaccggctgacatctacttcaacagcggtaaacactggcagggatatgactgacttttccctgaaaacagatttcgacaataccgcccgtccacagcagagcaaatacgatgtgggtgcttttgagttgaaaaccggtaccacttcaccacccgtttcaaatgcaggtggtgaccttaccattaccttaccaatagattatgtaaccctggacggcgcatcatcggccgcttcaggcggcagcaccattcaaagctatgcgtggaagaagatcagtggtcccaccgccggcaccattgtgagcccgaacgtcattaaaacaaatgtaacgggacttacacagggaacctatgtatatgctttgaccgtcacagacgataaggggctgacagatagcgacagcatcacggttaccgtgaaacccgctgccaataagccaccggtggccaatgccggaagtaatatccaggtacagttgcccgtaaacagtgcgtcactggacggcagcgcctctacggatgccgacggacaaataaccacctgggcctggacgaaaaccgccggtcctgccgggggcgatctttccgctgccaatgctgctaaaacaaatgtagccaacctggtggcaggcacttatacttaccgtctcatcatcacagataacaccggcgccaaggatacggccaccgttaatgtcaccgtaaccgccgcggctaataaaccgccggtggccaatgccggaagtaatatccaggtacagttgcccgtaaacagtgcatcactggacggcagcgcctctgcggatgcagacggacaaataactgcctggtcctggacaaaaaccgccggtcctgccgggggcgatctttccgccgccaatgccgccaaaacaaatgtagccaacctgttggcgggtacttacacttaccgtctcattatcacagacaacaccggtgcaaaggatacggccaccgtaaatgttaccgtaaccgctgctgctaataaaccaccagtagcttatgccgggaaaaatatacagatccagttgccggtaaacaccagtgcgctcgacggcagtaattccactgacagcgacggacaaatcgtgaactggtcatggcagaaaaccaccggcccggctggcggagacctggcaagtgccggcgcatccaaaacaacggtgagtaacctgtctgccggtacctatacctaccagctaacggttactgataataataacgccactgccacagccaccgtaaccatcctggtactggcagcagcgcccaatctttcgccggtagcagatgcgggcaatgacatagctatccagctaccggtaagcagcgcagccctggatggcagcgcctccacagatgccgacggacaaatcgttacctggctatgggagaaaactgcaggtcctgcgggaggaaatctttccgccgctaacgcagccaaaacaaatgtcaccaacctgcaggcgggaacttatacgttccggctgacagtcaccgataacgatggcgctaccagcaatgccactgtgaacattacagtaaccgcagcgccggtgaataatccaccggtggccgttgccggaaatgatatacagatccagttaccggtaagcagcgcagccctggatggcagcgcctccacagatgccgacgggcaaatcgttacctggctatgggagaaaaccgctggccctgcgggaggaaatctttccgccgctaacgcagccaaaacaaatgtcaccaacctgcaggcgggaacttatacgttccggctgacggtcactgataacgatggcgctaccagcaatgccactgtgaacattacagtaaccgcagcgccggtgaataatccaccggtggccgttgccggaaatgatatacagatccagctaccggtaagcagcgcaaccctggatggcagcgcctccacggatgcggatggacaaatcgttacctggctatgggagaaaaccacaggtcctgcaggagggaatctttctgcgaccaatgccgccaaaacaaatgtcaccaacctgctggcgggaacttatacgttccggctgacggtcactgataacaatggcgccaccaattcttcttcagtaagtattatggtactgcctttggaaaataaagcgccggtagcccaaacacagggtgataggagcattcagcagccaatgaattcgttcattgcagatggcagttcatcttatgatcctgatggtaatattgtgaagtatgaatggacacaggtagaaggacccgccaccgccaatttaaaaagccctgaccaggtacaaacactgatcaacggcctccatgcgggcaaatacgaattcaaacttactgtgacggatgacaggggcggtacggctaccagcaactttaccttaaccgtactgggcaacgatattatcacgcatgaggaagactcattgggtatattccccaacccggccacacaatacatccggttacggatcgtgcggagcggcgcaacgcctttgcaggtgaggattttcgacatgaatggccgcatgcagcaacagctgagatacaccacgcctgattcattccagacagaagtgaacatcagcaatttatcaaacggacatttcattatagatgtgaagtcggaagacagcagctacaataagaaaggccgttttataaaagtaagcaactagattttttcccaggtaccactggataactgatattgacggatagggcgggcagggttgcccgccactattgtaaaaggaggaacgtctttggtaaccacactgccgcccgccactacagaatggcggccgatggttacgcctgcggtaataacgctgttggcgccaatccagcaatctgcttctacaacaatttctccaacggtgcagggctgcaacgcaatcggaacatcgggatctttgtacccgtgattcaaacctgataatacaatgttctgcgccaatataacattgtcgcctatacgaaccgggccaatcagcacattgcctatcccgatccttacatggtcgccaataattaccgcgcccattccattatttacggtggcaaagtcttctatggtggagtagtttccgagagtaaaagtgttaaatggcaacacatccatccgtgtccgccttcttatcagggagccttttccttttttatggaggaagggattgataaacaaccgcacccacaggcgtggacgggcctgatgcttgggcatcagcaggtataaagccagtttcttcagccccgggtgttgtttcagtttgtcttttatactcataatcaattaccgctggaatttaagatcgcctggtaaatggccgcaacggaattctcccaggtatgtgtgcctgcaaagcggatacgctcagcggccagccccggatctgcgttatctgataaagctttttcaatcaatggaacataatcgtccggtgaaggcgccaggtaaacataatccctgaacagttccatggttttagtagcggttgctaccaccggcttacccatggcaagatattcgtcgattttcaacgggtaattgcctgctgtgacttcattgatgacttgtggattaagacacacatcaaaggactgcacataggcaggaagctgcgataagtccttatgccccgtaaaataaacgttgggtagctgatgaagcgctgacgctttgaagtcatcatcttccgggccaaccagcaccaacttccattccggccgttcgctggctatctttaccaaaacggaaatatccagtcgcagtgatttaagcgcccccacataaccaataaccggtccctgtcctgttggcacatcatccggaaccggatgtttatccgccgcattgaacagccggaggtcacatccctgtcccacataatagctggaagggttgtactgctgcagcatttccttgaggtataatgaattggctactgcggcatcggccttggcaatgtgctgcggttcaagccgcagcccgtgctttttccagtaaggcacgcccagcaggtagtccctgctataatatacataactggaaggctgcagcatttccttgaggtagaagccgcggaatatatcattatcattaaatagaatgatgtctttgaaattcatttccttgacagcatccataatactgtctgcaaactttctgttattccgcttgttaaaccaggagaataaaggggtgaaaggcagccagttaatagattcgaggatggcagaagggtagtagttccagaggttatcactgatcggcacaatggcaggtacctttttctgaatagcattcagctggtattgcacatgcggatcttccttcccggtcataagggtattcctgtccagcggagcgttaatatataataccctgttatgccgggcaaattcccgcgcaatatttttacagttgcttccaatagtagtgtaccattgttgcagccctattacaacgatatctctgttttgaattaaaggcacagtagcaaagtgtagatgatgtatatcggtttattgaattaatatgtgcaggtctgccgttggggatggttaaatattgaacttcttagctctaaatgcaaagtaaataaaaaaaatcgatattattggagtattagaataagaatcgttctttaaaaacagaaaaagaggctatgtcagaaacagtagaaataagaacattgaccgttgaggattacctggatcttaaagaatccatggtgtctgcctatgccgatatggccggcagctattggcgggagccaaccatacggcgactgatcacacttttcccggaagggcagatcgcagtgacggtaaatgacaaggtagtggggtgcgcactggccattatagtggactatgagaaatttggtgatagtcatacttatgaacagatcaccggttattatacgtttaatacgcataatccaaaaggcgatacactttatgggatcgaggtgttcgtacatcccgattatcgcggtaagcgactggcccgccgcttatatgacgcccgtaaaaatctctgcgaacaactgaacctgcaggggatcgtggccggcggacgtatacctaattttgaaaagttctccgaccggatgtcgcccagggagtatatcgagaaagtgcaggaccgggaaatttatgatcccaccctcacattccagttttcaaatgatttcacggtaaagaagatccttaaaaactacctgcctaacgatgaggcttcgaaaggctttgccacgctgctgcagtggtttaatatctattacgaaaaggacctggataccatccgctataacaaatcaaccgtacgcataggactggtgcagtggcagatgcgggattatggcagtcttgaaggtttcctgcaacaggtggagtattttatcgatgcagtaagcgactatggatccgactttgttgttttcccggaactctttaactctccgttgatgaaagagttcaaccagatggacccggcaggagctatcaggggagtagcccaatacacgcagcagttaagggaaatattccagcagcatgcggtagcttataatgtcaatatcatttcgggcagtatgccgattgtgatcgatgaggtactgtataatatttcctacctctgccgccgggatggtacctacgagcagtatattaagatccatcccacacccggcgaggtagctgcctggggaattaagggaggaagcgatattaaagtgtttgatacagattgcggtaaaatcggcatccagatctgctatgacgtggagttcccggaaccgtcccgtatcctggcagaacaaggtatgcagatcctgtttgtgcctttcatgacagatacgcagcatgcctataaccgggtacggttctgcgcgcaggccagagccgttgaaaatgagtgctatgtggccatcgccggctgtatcgggaatttgccgaaggtaaataatatggacctgcaatatgcgcaatcctgtgtatttaccccatcagattttgcttttccggtaacaggcattaaggcagaatcaacgccaaacaccgaaatggtggttatcgcggatgtggacctggtattattgaaagaattacacgcttttggaagcgtgcaaactaaaaaagatatccggcgggatctgtatgaagtaaattataaaaagaaggggtaattgtacatatagatgaggaggattttcgaattataaacagatgtaatttgatgcctgaaaataaatagggtaacggcttgcggaggcttgctgttatccttttttagttttaaattcagtgtaaatccccaaagttatgaaagatcaagcctattatccttcctggaggaatttatctaagtacagacagtatcttgcctattttagtgaatatatcaggtataacgactggaaatccctgcaagcgtcccttaaactcgttttattaaacaaaccctctctgaatgaatggaacgcaaaatcagccatgggacttttccggatccgcggaggcacaaccgacttccagtttattaattatgcatacgagaagcgggtacgcgacttcctaaaggagcaggtagaaaatgggaacatcgacggttttattgacattggcgcctgtatcggggagtatgatgtatggctgggtggaaaaggaatcccctgtgttgcttttgaacccgtgaattacaaagccgtgcaggaaaatatcaccctcaatcatgtggaagataaagtgaaactttacgcctgcggtcttggtagcaggcaggagaaggtgaacttcaatattatgagtactgttaccgggtcaagttatatcgaccgggatagcgataaagaaggcaatattcctattgaaaaactggatgacctgattcctgaaataggatttgacctgcgcagtaaaatcgttatgaagctggatgtggaaggaatggagacagaagtgctggaaggtgcgcgtaattttatcggcaaagccgatcatctgcgtatcatttttgaacgctatgaaggtgacaatactgtaaacgataagttgagctcattagctaattttactttcgacagaatagaccagtttaactatctcgctacaaaaatatagtccagctctttatgatgataaaggcaatacatgttcatttgtgtgttgcctttcgtagttttaccacccgacgggcggaataaacaagtcgaatggattgtttttatttgttatatataatgaaacgttcagtgattttaaatagtagtaaattataaaattatattctgtttaataattgataattaatatattgagagatttaactgaagtgatactataatgtaaataggctatttttcatgatcactaacaaattggccgcgaaaaatgatcatttcatttaaaccattactgtaagtattttgttttaatagattggtaaccataaaattaaaaagtaaataaaagatgagcaataagatcaatttagcccttcaaatcattccttcagtaccttcagagcaggtttacgcagtagtagacgaagcaattgcggtgattaaagattccggtgtaaaatacagggtatgcccttttgaaacggtgatggaaggcacctacgaggaactgatggaagtggtacgtaaaacccaggaagtatgttttaaggcaggtgcatcccagttattggtatatataaaaatgcagataagaaaagacggggatgttaccattgaagaaaaaacagggaagtatgatagcatataaccaattttttttatcttactcaccgaactaaaggagagccatatatatgagatacgctgccccgttggatgataactcgaagattgtaacgaacctggtcatcattattacgcttgtgtttttatgcagacagatgacggatgtttcgcatgatgcagttaccactaccatgtttttgtttatcctggtgccagccatcctggtagcctggtgtctgagcccccggtattacattctaacggctacgactatacttatcaagcgcccgctgcatagcattaccattcagctggaagatgtggtaagactgagaagcatcacggaagaagacctgggcacaagctcccgcttactgggattaggaggcattttcgggtacctcggtacctaccgttccagtgaaataggcaagtaccagcgctggtgtaccagccgggaaaacctggtgctgatagaatcgctcaacaggaaatggctgatcagccccaccggtgcagatgattttgtgaaacgggtgaatgccacgattaatgtaccagcttaatagctataaatgaaaaaaggaaggctgaatgccttccttttttcatttatagcataccccggtcgtttaatgaaagaaaagatagccgagtaatattgcgcagagcataccaaagaagtcggcaatcagtccggctgccagggcataccgtgtgagtttgatattgactgagccaaaatacactgcgagcacgtaaaaggtggtttctgtggtaccctgtataatgctggccagtttacccacaaaggaatccggtccgtgcgttttcaggatatccaccatcagggcacgggcgcctccgccactcagcggtttcataaaggccaccggcagggcaggaacaaaatccgtattgaaccccatcgccgcaaacaagagtccgatgccgttggtgatatagtcgaggcaaccggtggtccggaacacgctgatcgctaccagcatacccaccaggtagggaataattcttacagatacctggaaaccttctttcgccccctcaataaaggcatcgtatacgttgatcttttttaccatccctgccaccaggaaaatgataacaatgctgaaaatgatcgcgccaccgagggaagccgttttagggcctatctccgcaggtggtaaactgcggacccaaaaccataaggcagccataatcccggcaaacagggccaggaataccaggacagggagtttaaaaaggttgatcttttgatagatggaaaccacaaacatccccatgataaaggccatgaacgtggatatcagggtaggaatgaaaatatccgccgggttagccgcacccgcggccagccgtatggcaatcacagaagtggggatcagcaccacgccagctgtattcaataccaggaacatgatctgcggattactcgcttcctccggccggggattgatctcctgcagctccttcatcgccttcagccccataggcgtggcggcattatccagtcccagcatggtggcagagaagttcatcatcatagaccccatggccggatgccccttcggcacctccgggaacagcttggaaaagaaaggatttaccagcctggaaaaccggttgatcataccggccacctcgccgatccgcatgatgcccagccataaagtcatgatgccggccagtcccagggagatctctgcaccggttttggcgctggcaaacatgccgttcataatctccccaaaaatagacgcatcatgtaaaactactgacttgaaaagtgctacaacaaatgcaataagaaaaaatcccagccatacgtagtttaatgccattagattattggtttattcaatcaacaaataaactaaaataaacctatctttgcgcaaattttaaaaaatggctttgcaagttggaattgtaggattgccgaatgtaggaaaatcgactttatttaatgcggtgagcaacagcgctaaggcgcaggccagtaactaccgcttctgtactatagaacctaacgttggccaggtggatgtaccggacgaacgtatgcataaactggcagagctggtaaagcctgaccgcgtggtgcctactaccatcgagtttgtggacattgccggcctggttaaaggcgccagcaaaggggaaggtctgggaaacaagttcctggccaatatccgtgaggtggatgcgatcgttcacgtgatccgctgctttgaagatgaaaacatcctccgcgaagaaggagagatcaaccctgtcagcgataaggaaatcattgacaccgaattacagctgaaagacctcgacagcgtggagcgtaaagtggcccgtaccgagaaaatggctaaaaccggtggcgatccaaaagcaaagattgaattcgaaatactgaaaagatgccaggaacacctggagaaaggccgtaacatccgtgaactgggcctcagtaaagaagaaagggtagccattgccgacctgttcctgctcactgaaaaaccagtactgtacgtagccaacgtagatgaagcatcccttcataccggtaacaaattttcccaggccctccaggaatctgtgaaagcagaaaatgcccaggtaattatcatgaacaactccatcgaagcgcaaatctccgaaatggaggagccggccgataaagaattgttcctgggagaatatggactgactgaacccggcctgaaccgcttaatccgttctgcctataacctgctggaactgatcacctacttcactgccggcgtgcaggaagtacgtgcctggaccatccataaaggctggaaagctccccaggctgccagcgtaatccacaccgattttgagaaaggcttcattaaagcagaagtaattgcttatgaagattacgtaaaatacggatctgaagcagctgcccgtgacaacggccgtctgcgcattgaaggtaaagaatacatcgttgccgacggggatgttatgcacttccgctttaacgtttaaaaatacttctggataagatccatgaaggttacaacaaaaagacgggccggccatccggcccgttgctatgttacccctaacgtatatgcatatattaattatataacccccatacgccaaattcaaaattcttttattagcttagccacctatttttaatgttagctcatgcgtattgtcaggaacgtaaaactctttttccgggaaggaaactcggataagacctatgaaattgatctttgtgaggttggcccggaacagtatattgttaacttcagatatggtaaacgcttcggtaccctgaaagacggtaccaaaactgtaagccccgtaacattatctgccgccaccactatattcgatggtcttgaaaaagaaaaaagaagtaaaggttatctgggagaacaggaagctgttcaggacctgtcgtttaccccggtagatactaccctcgtggaaaacgtgaaacaccgcgctatcctgaaacgtttacaggatgcggtagaagggaaaagcagctttaaaactgcctggagcacttcccgcgtaatatggcgggccggtgaagaaaagataaaggaagccgttccctacctgatcaagctcgtggaaaaaggcgacggactgcaacgctatgcagctctctgggcgctgggtaaatcaggcgaccccgcggccatctcggtactccgctcttatgccgataacagctcccgccccctgaatatcaggatgctggctgccaacggcctgctactgctattgccaacggaagaacgggcggcacatgtgcgttcctatctccaacggctgcccgaaatattccagcaggcggttgccaaaggaagtacagaagaattgctcacactgttgcagcaacgggtcatcacacaacaggagcaaagctacccgctgctggaagacttatacatcgtagcctttgaacattccgccgtgagaattgccatcggcaacttcctcatgcacctgcctttcaggccatcctggttccagcatatccgccatatcttcaaacaggcggaactgcgcggcgatcagggaattgtagccatcctggctgcacgtttcgaaagggaagcccctatgtttaagaacccgggtacgagcatagattataacgataagccgtttgttccaaacacttatataccggaactgaaagaatctgtacaggcagataaagaactgaaaaggcccaccagtaaagttgcattttcagacaggacccgtaattaccttcattaccgcgtattccgcaacctgcgccagttcggtgaacaaaatgacgatcattatgttcgcctcgctaccgccctgttgctgcaatacgaagaaagcagggatgcggccaaagaataccagacccacgaacatacctgggtgaatggccgctatgaaagcttctaccgccagtttccggctaattcaaaactggtatacctcaactatatcctccgcggaaacgccgccaacctgcaattaacgcccgatcacaaggaatgggttttcaaagatgagggagcttctaacgcacagggacggacgaaactgacatcaggtagcaaccccgacgccgcgaaagacaaaggcggcctgctaaaaaaactcttcggctggctgggtggtgaaaagaacgcaccagcatcggccgtaccgccggagtataaggcatcaccggcacaaccggtgagcgatgtgccattcctgcaactgtggcaaaagttaccgcaggctttcatccagctgctcatatccgcacgcatggaagcgatccacatctttgccatggagcaactgaaagcccatccggattacagcaccctgaaagataaaatggatgaaggcgtgattgccgggctgctggctaacgcattttccattccatccatgttcgggttggaactggccaaagagagatacgatcccgccaacccgtcgttgcggctattatacatactggtgatgagcccactggatctggcccgtttacagggactgcagtggatcagcgaaaatgagccggtttgctttgcggacatggacttcctcatgcagctgatattttcgccctataaggaagtgcgcggctttgcccgtaagcaacttaaaccggcgtacctgccactggataaggcgagaatactctctgcaaaagcaattacttcgttgctggcattgaaaacatccacgccggcaggcaatgaaaacctgaatgatggctgtaatatcctggagcaacattgccgggaggcactaacggaaaccggcatgccggatatagaagcgttgctgcaaagcccggtggcggccaatcaggcattcgcggcgcgcctgctgctcctgaaacaaggagcgtttaacttcagcgaaatatccgacgcgatgctgaaacagctgatcagcaatgaattccagccggtaagagctgccggtgtggaagtgctggaagcaatgggcgtcgatgaattattgaaaagaccagaactggtactccatatattattaagtacgtacacggatgtacgtaatgcggtacgcccacttatcagccggctggtacagcaggataaacgcatggccgtttacctggtaaatgaactggtgccactgctcatgcgcaaggaaaccggggaaggcatgcatgccgatattgaagccaccctcagcaatgagctggttgactatttacaggatatcgacactgctaccgctttacgcctgctgtacgccaattacaggtcggcacaacaattcggattgctggtacttgataaatatattcctgcatcggcgctgtccgtgaaacaggtaattgctgccggtaatcatgaactgctgaaagtaagggagtggagctggcatttttactacaacaacgtcgcccgtatccgttttgaaagagacgccgctattggcctgctcgatgcgaaatgggacgatacccggcaggaagcaatggaatttttcagaacgcagtttacggataacgattggtcgccggaaacactggtggcggtggccgacagcgtgcggcccgatatccaggcctttggccgggaattgctgctgcgcttcttccgcgaacaggacggacaaacctacctgttgaaattaagccaacacccaagtgaaagcatgcagttatttgcgactaactacctgcagcaatatgccgctggcaacctggtgtttctgcaacagctggaacattatttccgggtggtactaagcagggtaaacaaagcccgcgccgccaaggaacggatcttcgtattcctggaaaaggaagccatgaagtcggaggaagcagctgcttatatcggtcatattattgcgcatatatccgctactgtagccattggcgacaaagcccgctgcattgccataatgcgtagtatccaggaacggtatgcggtagaactgccgattgaaatagtgccaacagcgattagagtatcttaaaaagtaatccatttatgttattcaattacagatacagcggaaactccaacgtgttcagcaatgccaccgctgcgggcatttcctttgcaccggatacccgtcgtgaccctaccttttttgtgggtaagctgcataaaaaaatagctttccgggaggccatctccgccctgcatgatgtagtggtatccgatctgcgctttaaaccgaaagataaaacagcctataaagaatgggccgcccagcaggaaacagtgtggctggcggagttcatgaacggctatgatgcgcaggcggccgatcagcggatagacgggctgagaggggaactcaatggtatttaccaggagaaggaaaaagtgatggcccctttttataaagcccgtaaaaattatttcgattatttataccagaaagaccgcgacgcctggtttgtactggacccggtgatcagcgtacatccggatgaactgttctttgaatgtttcagccaggacgaatctacctacggaaagctgagtgcgagttataatgttttcaaagaagtgaacgagtttgaatgcggcactaccaatattgattattctgcatcgctttataacgaattccagaagatccgtgattataaggaaacagattttaagattgatcccgccggcttccaggtgcaaacctcgcaggaggaactatatcatgaagtaaagatcgatttgcccgatagctgggtgaggggctttctgcaggtgagttctgcgatgacactgcccgccgcaacgtttgacctgcatcctatggatgtatataatttctgttcctggctgcggcgcttcaaagaaaaacacgggccacggtcgatccgttttatcctggaacccggtaaaccggtacgtgcagtgtttgagccatggaaccaggaaatcgtatgtgcaagatcgttatacaccggcccgcaaagcagggagatcaggatatgggggagaagacggttgctgatcctggaaaggctgattccaattgcgaagaagttcaccgtgcatcttaccggtaacgggttgccatccttttatgtagcggatcttggcgatatgcagtttacactggggctcagcggatggaccgccaacgactggtcgcgcgccgggcagtttgaccttatggcgccaagagcagacgtgagcgacgtagcaaagctcaccgtttttgaagacctgaaaaccaggtggatggctaaaccggaaacgattgttgccgccaccggccttgatagggctaccgtattgggggcactgggaatttatacccaggcaggcaaagtaatttacgatctgcacactggcttttaccgcctccgtgaactaagtcgtgagccactgccgctggaccagctgcgctttgccaatccgcaggaaggggaagccaccaaactggtgcaggccggaaaagtggaactgacggctaccgatatcccgggagtaggtttgcagctgaaaggaaatgtaaaaggtgtgcaacgtatataccatcccgttattaccattgatgcggatgaaagattaagtaatgcacactgtgactgtaatttttatagtacgaataaattatacaaggggccgtgcgaacacatgctggcactgcgtatagcgcattcggaaaataaagcggtaaaataatttaaggaggtgtttttatttccggagattattttctaccttgctgactcgttaataacaaagatctttgtaaagaggaattgattgcacttgcgcccgaaaagggacgaatgatgtttcgtcattcaggtattctgactatacatgcttcactaaatgcaatctttactttgggagggggctacggtacgcatatttccagtagaagccccctgggctgaaatatgcgtaccgtagccccctccctggagttgattgatttagtcaatggtttgcacgaaggccttttcctctttacagaattttgtttccccttctcagcagggccgtatcaccgcccattttccacccttttactggtattttattttagacgaccggatttttattacggataggctccgttgtcaaagtcatgaaacagcataaatacaaacatatttatcatgtccttaacccgtcaacaactgtacgataagatacgtgcatcctctaaagaggaatatatattacaggaaatgacacgcctgggtttctgggccgaaaatgttgcgcagccttcacctgcggctaccctcatccagaaggaaaatgaggtgcgccggcagttgaacgatctgatgaacgaacggcagcgataccgcaacaagcgggcaatgctggaagatatgcgcaaggcccgcatggcaaaagccaaactgaaaagggaagaaacaaaacaacgccgcgaaaccgcaagaaaagaaagagccgccgcatgggccatcaccaaagatcagcagatcgtatatcttggtgaggaagtatctgccggcttaaataaagtggtgccggatgtagcgcaactccaaaagttcggactgccggtatgggccgacgctaccgcgttagccaacgctatgggcatcaccatcggcaaactgaggtatttatcttttaaccggaaagtcgggcatcatacccactatcaacgttttcagatcccaaaaaaatccggcggcgcccgcaccatttctgcgccgatgccgcaactgaaagccgcacaacactggatcctggagaatattctctataaaataaaaaatgatgaatcagctcacggcttcgtaccgggcagatctatcgttaccaacgcagcgccacataccggtcaggatatcgtgatcaacattgatctgcgcgacttcttcccgtctattgaatacaaacgggtaaaaggactattctgtaaactcggatacgctgaacaggtagctaccatactggcgcttatttgtacagaaccggaagtagatgaagtactgctcgatggccgcaaatactatgtggctaaaacagcccggcatctcccgcagggagcccctaccagccccgctattacaaacctgatctgttataagctggacaggcgttttgcaggtttggcggcaaagtacggatacgcctatacgagatatgcagacgacatgacattttctgccaaaggcccggctgcagataaagcaggacaattgctgcgtgccgtgaaaatgtttgtaaaagaagaaggttttaccatccaccccgataaactaaaggtgatgcgtaaaggagataagcacgaagtaacgggcatcgtggtaaatgaaaagctgagcctggaccgtaccaccctgcgtaaattccgcgccttgctacaccaggtagagaaaaccggtttagccaataaaagctggggcaaaggaaaaaatgttatcagcagcatggaaggttacgccaactttgtatacatggtgaaaccggaactgggcgcaaagctgaaagccacactgggcgcattgctgcaaagggaagatattaaggcagaagcccgcagcctgtggacaggagaaagcacggctaaaaaaattacgccacaggtcaatgccataccactcaacaatccaaccaccccgtcagacaaaccctggtgggacgtagtataacaatcgacaaacaaatataaaaagccccgggtattattttctgacaagaaaacagtatccggggcttcttccttttataaattatagcctatagaaatatagccttgtgtgccaatagtgggattaccccacgactgtatatatttcttattcaggatattggcggcgcccagttttaccgtggttttagccttcgggaaaaacttactcaccattgcatccaatgtgccataggcaggaatttcgctaagaccagcggcatttaaattaggtcctacaaaagacgactgccatatgaaggagtcctgccatttccataatacgttaaacgcaaaattggaattggcaatgttgcggttaccgaaattcaggctgtagcgcacctttggtgtgttatacatcgtcataaatgaacccaggtccttttcattggtgagttcattataagagatgttaccaccggcggtgaaattgagcggcaggctgtaatccagtcccaatgcccatccccaggaatgcactacttcagtggcgcttaccggcacagagaagatattattctttgcaggatctgcggttggttgcaccagcacctgtgtaccattcatattcttgaaatcatttttatagatataggcatccaccagcaattgttttgcgattactgccttataacctatttcatatgcctggatcctttccggcaggaattcacggaaaacatactgttggggagcacccgcctgtaccgactggagagagaacaccggtcctttatccaggccataacgttcgcgcaggaatggcaagccgccgatcaggtgtgcctgcggcgttacgagatcgatatactgatcctggttgtgtggaatacggaagcctgtttgataggaagcgcggatattatgcgtaccgaggaacgtatatacagctgacaaacgtggactgaactggcctttaaagttcatgttcttatcatagcgcagggagccggtcagtttcacgtggtcctctataatctttttcatgatctgcacataaccgccatactcattgatacggaattcatcgccgttgtcatctactgcaaacagtgttttttctgagttcagcgcatagcggcggtagttgccgcctaccagtatttcagcaaagtgaatcaggttatggaagttgtacatgaactctgcctgatacaggttggttttatcggtgaacttagcgcccacaccggaagcgtctccggggatgggtttgttcttcactttatctgcggcagcatcaaactctggtgtgcctgggatcaggcggcccttgtcggcattggttctggcagcgccgataaagttggcctgctgtgattgaactgccgcctgggcagcagcaaatgcagcgggaattccttgtccgaggttattggtaaaagttgttttaaaaagattgcctgcggccagtccataggtaccgaagtattcactataccactgctgactggttttccaggcctcattgataccggcagccagggtaccaccggcgtagctgtcgcccgccctttcctgtgtagtgtataatcttacatagaagtcagggctcttcaattccactttatactggcccatgttgaagtttttcagggaatagcggtcagctcctgtgtacacggtagtaccggagccatagctgccctgtaaaatggcttcgagattggtagtgagccggtaatgcaatgcagcattcagtttgaggtttttggtagtatagtctactacgtccgcttcgttgtaaccggtgcgggttacgttcgacatattctgcggaggcaggatagcattatataactgatccggtgtgagggcgcctcccagttgctgcgacaatgcaaccatttgcggcatcagggcaggtttcaggccggtgtacatatttacggtattctcatctccatatacattcacgccattatagccttcattattagcgcgggtgccattttcgagggtatgaccgtttgccaggctctggtcgcggtgatcatatgcctgccagtccttcgcctgtaaatagcctacgttcagcttaaaggcaaccttgtcactaaaggcatgtgcgtaacgcacagatacatcgtaatacccggtagtggcggtagagcggcctgcatcattgaggaaaccggtttttacaagggcgctgagtccctggtactggaacgggtttttgctgttcatcaggaggataccgttgagggcattggggccatacaacgcggatgccgcgccagggatgagttccatgttgtcgagatccacttccggaatgcccaccatgttgcccacggcaaagttcagcccgggggcctggttgtccattccatcattcagttgcagcacgcgggtattaccattgctgttaaagccgcgggtattcactgatttgaacgttaagctctgggtgctcatttcaacgcctttcaggttggccagcgcatcataataagaaggtgcgggggaggccttcagggcgcgggcatccagtttttcgatggacaccggtgattgaaggatgctttcctgtgtacggctggcggctactactacttcctggccgagaatttcagtggagctgagttctattaccagtttgtccgccgcagaggagacttcccgctcttctgttttgaagcctacgtaggagaacaccagtgttaacgggaacgcatgtgtggttctgagggtaaaagcgcctccgctgccggtgatagtcccggtattggagcctttaactgctacggttacaccgggcatgacgttgccggaacctttttcgcgtacagtaccattaagggagacagggttttgggccgaaattatctgggtcagggataataaaagcaccaggcagccgatgaaggctttgattagaatgcttctcatacacgatggatttataaaaggtttagactcggtttaaataaatataaagaaaaaaaaccgcatatagccatcgggagtgcaggggattaaaataaaaatgcaacagggtcatcctgctgcatctatcttgttataataccttaaaaatcaatgtgctgttattgcatccattcctgtaaaatgctgccgatcttctcaaattctatcaggaaaccatcatgtccgtacgaagaatctatttcatgataagtagcgtgtggaagatgtgccgctataaactgctgttcctccggcgggcataaaatgtcactgctgatgcctatgagcagggtaggctgctgaatatgagaaagggtagtggtaatatcttcatgacggccacgggcaatattatggctgtccattgccttggtgagcagccagtacgactgcgcattaaagcgttttacgagtttgtcgccctggtaaatgatataggaggaagccctgaaattatcggtcttctctttatcttcatctgattgcgcgcgcacgaaggtgtggtagttgcgataagtaagcataccaatagccctggcggctttcagccctttcgatcctgcgctgtggttgttgtcctgccacgtatcatccgcttcaatagccagtcgctgcgcagtatggatggcaataccccaggcgctttccgcggctcctgtgcacagcaggaacagacggtcggtaacagccggctccagcaatgcccattccagtgcctggtagccgcccatagaaccgccgatcagcaggtggatacggggaatctgcagctgcttcctgagcaggatatgcgcctgtaccatatcccggatggtaatggtaggaaactgccgataccatggatggccggtttccgggtttacagtatgcgggccgctgctgccatagcaggacccaatgatattagcacacacaatgaaatgcctggcagggtcgatcgctttaccgggtccgattaagccagtccaccagtcagccgcatcactgttggcggttaaggcatgacatacccaaaccacgttgctgccatcttctttcatcgtaccatacgtatgatacgcgatatgtaatcccggtaatacttcgccggattctaaccggaatgctgtttgactgtgaaatacctttgccgacaatgcttcttcgaatttgcgcaaaactacaatatcagaattaaaaattgcaaaatagcgccggtgatttatgaattagggaggaatgacggccactgcataaatcctgatggttttatttatctttgttgaagataacctaataatcatgaagatagcattacaaagagtagatgacggatttaatatggaggcagtagatgaaggcggccacaaagtactgatggactcatctctggaaaatggcggtaagaataacggagtaagacctatgcaaatggtgatcatgggccttggtggttgttctgccattgatgtgatgatgatcctgaagaaacaacgccaggaagtaaccgatttccgtattgaaattgacgcagaaagagaaaaaggaaaagaaccttccctctgggaaacggctcacctggtatttcatctcaaaggtaatattgatcccgataaagcagcacgcgctgtggaattgtctatgaacaaatattgttctgtggcggaaaccctgcgtcagggtaaaacaaaactgacctgggaagtgaaactgaacgcataaatgctgtaactaccatatccatgagcaaagaaaaaaatcaataccaaccggataccaatgcggtaagaatgcagacgcctaaaacggaccagatggagcattctgtacccatgttcctgacctccagtttttgttttgataacgcagaagaaatgcgtgctactttcgcggacgaaacagacttcaatatctatagccgtttcagcaatcccaatgtagacgaatttgtacagaagatgtgcgcccttgaaggaggagaagccggctatgctacggcctccggtatgagcgcaatttttgccagcttcatggccctgctcaaaaccggcgatcacctgctgtctgcccgctctatcttcggctccacccacaccgtgatcacgaagttcctgccaaaatggggcattgaaacttcctattttgatatgaccgatcccgccggtattgaagccatgataaagcccaatacccggatgattttcgtggaaacgccgtctaatccaggtcttgagatcatagacctggaactgctggccggcattgccaataagcataatatcattttaaacgtcgacaactgctttgcaacgcctgtattgcaacgccctattgaatacggcgcccacctggttacccattcggctaccaaatggattgacggacaaggacgtgtactcggcggagtagtagtaggaaaggcggaactgatcaaggaaatccatactttttgcagaagtaccggcccggccatgtcgccattcaacgcatgggtgctcagcaaaagcctggaaaccctctatgtaagaatggaacgtcattcggccagtgccttgaaactcgccgagcgcctggaaaacaacccgcacctgctgtcagtgaaatatcctttgctgactagtcacccgcaatacaacattgccaaaaaacaaatgaatggcggcggtggtatcgtatgctttgaactgaaaggcggcctgcaacagggcgttcgtttcctggatgccttacagctcctttcactcaccgctaacctgggcgatagccgcagcattgcttcgcatcctgccagcaccacccacgcaaagctctctgaagaagaacgcgccattgccggtatcacgccaggactgatacggatttcggtaggactggaaaacattaaggatatcgtggaagacatagagcaggcactgaatgcgagtgccctgtagcggatgttgtcttactcaggattacgctgattatactgattttactttttggattttattaagattataaagatttaagagagactaaagcaattttattatttgttcttttttttaaaagaaaatcataaaaatccaaaaaatccaaaaagtaaaatcagtataatcagcgtaatcctgagaaagacaaaattcgcacaaatccgcattattctacttatattagaatcatgaaatcctttgcccattttctcctgatccttctcctgtcttatgtagcaggtatggtgctgccctggtggagcgttgcgctcgtggctttcctcgtaacgttgcttatgccgctgtcaccgggtaaatcattcttcagcgccttcatgggcgtgtttgtgttatggatgatcctggctttttatatggatgtaagaaatgatcacctgctcgccaaccgtatgagtgaaatgatattgaaagtacgaagcgcaccgcttatgggtgtagtcagttcctttatcggcggactcgtagccggcttcgccgccagctctgctgcgtttgtccgtgctgcaaaaaagcccgcctgattacttatccagggtgttaaaattctgataaaacagcttattcaaataacctgtaagcagttcgccgttacatttggaatatgaagaactacctgtctgccctgttttgcattttcatttccagctactgccaggctattgcggtgaaaggccgcgttacggatgataaagatcagccgctcccatttgctaccgtattcatcaaaggaactaccaccggcactactaccaacgctgccggccaataccagcttgatctccctgccggtcaatatacggtggtatgccagtatatcggttttaaaagaacggaactgccgcttaacgtgaatgcctcaacgcaggtactcgactttcatttgcagcctattaacatgcagataaaagaagtggtagtaaaagccaatggagaagatcccgcctatgctatcatccggcaagccattaagaaacggcatttctaccagcaacaggtgaaagaatatacctgcatgtcctatatcaaagggactatcggaatgaaaaatgtgccaggaagattcatgggacagaaaatagataagaacgacatgggagtggacagcaccgggaaaggcatgatattcctgtcggagtcagtaactaaaatatctgcaaggcagccggataaaataaaactggaagtcatttcctcccgcaaaagtggcggtggctttggcttaagcttccctgccatcatcagcttctatgataacaatgtttccgccgttatcacacaaatgggccccaggggttatatttctcccattgcagaaaatgcactggcctactataaataccggctggaaggcaccttcacggaagaaggcaaaaccgttaataaaatacaggtgattccccgccgtaaacaggagccactgttttcaggatatatcttcattaccgatgacgactggcgcattcacagcacagacctgatccttaccggtgaataccagctggaactgatggacacgctggagatccgccaaacccacgtacccgttaccgccgacatctggcgcgtaaaagaccaggtaatgcacatctcatttaataagtttggtttccgcatgggtggcagcttcgtcaatgtatactccgattataatgtacatcctcaattcccgccgaagttttttgataacaccttcctcaaatatgattctgcctttgataaacaaggacatacttattgggacagcatccggccggttccgctggaaaccgctgaggtgaaggattatcacgaaaaagacagcatcgctaaagcggcgcgcgactcctccttttcccgctatcacctcgattccctgcaacggaaacagaaaccggtgaaagtaacggatgtgctctggaacggtgtaaaacataagtactatttccgccgcgacagctccatacaatatcattccctcagtgtaaaaggactgctgaaatcactgaagtataataccgtggaagggctggtcattgcagtggagcctgagctgaacatctatacaggagaagaaagcagcctgcggataacacctttcttccggtacggattgagcaatactcacttcaatgcctatacgcaaattgatttcagtaacaggagtaaagtacagaagcgttatggccgcaacgactggtcactggcaggagggaagcgcatctcccagtttaaccaggacaatcccatcgataatatcgccaatgagttttataccctgttcctgaaggaaaactatatgaagctctatgaaaactggtttggtaaactgcgctacgcgcgtacgttccagacaaatgaccagttatcgttcgccgctacttatgaaagcaggaacccggtagaaaataccaccgactttgtaatctttaaaaacgaccgtaagcagtttacgcccaaccatccctatgagctggccaacgtgccctttgaaaagcaccaggcgttaatactggatgtggattttaccttccagcccggtcaacagtttgtggaattgcccgaccggaaaatcccttttggctccaaataccccacgttcaaagtaggctacagcaaagggatacccaatgtggcaaacagtattgttgatttcgacaaatggagtttctccgttcaggacaacatgaacttcaagttgttgggggaattccgctaccgtatcggcgccggcgggttcctgaacgaccggaacgtacaaatacccgattaccagcacttcaatggcaaccagactttctataacatgaaatacctgaacagcttccagctggcgccgtattaccagtacagtactaccgccccgttttatgctaccgctaatgtagaacaccatttcaatggattactcaccaataaaattccattgttcaaccgcctgaaatggaacctggtggcaggcgccaacgcattttatgtaaacagtgataataactatgtagaagtttttggaggtattgaaaatattctgaagatgatcagggtagatgtagtaacgggttatcagagtaaagaagatacccgtataggcgtccgggttggttttggaggtatcctggggaatatggtgaagtttaagaactaagaactgacagtgattccggggacctgttaccacctgttattgcttgccaggtaacaaaatccccgtatctcatcattcacaaaccggttctaaaatttcttcctgctctttatctctttcttttcatcaaagaaatatgccagtaacctgtagatccagataccaacaactgcataaataaagtaggtaatgtaaatactcataaaataacattttcgggttaaacaatattgcttctcttaatcaattttcaaaaagggtgccaatcggggttgtaacttatctgcaaagttatatacaataattatcaaatagttataaaaaaataaatattttttagatctccggtgaacctttggtggccttaattcgttagtaaggtaagtatatttggacaagcgctgtgcacattttactcacacgttggtgccaaaatgaaccgtcatcctttgaattaccggtatgagaaagatcgccctcattgcgctgttgtcgggaattatcctggccgcagccgcctatattacggaaacaaatgacctgcccggcgcagcagaactgagaacccccggctttatcggttatatcttcattatcagcgcaatagcctggttttccttacacgtcctgtaccagtgggcgaagaaatcagacccttctcattcctgatattcaatggattttgctacctttgctccctaaatcaattgttcttttacgattaaagagagttgattggagttttgttcgcgacgcaggcgtccttaaaatttcaagcaattatggcattacacaatagagtatctgccgccgaactgaaggtccggctggccaatgaaacgtttaaacgcgtcactgtttctttctaccagtacgcaaaaatccccgatccacaggcattccgtgatcagttgtacgaatcccttttccaactcggtactttcggacgcatttatgtagcccatgaaggcattaatgcccaggtgagcgttcctgagcatcactttgaggcatttaagcaacagttgtactcgatcgactttctacatggcatccggctgaatattgccgtggacgatgacggtaaatccttctttgtactgaaaatcaaagtccgcgataaaattgtggccgacggaattgaggaccccaccttcgatatggccaaccgtggccgttacgtggatgccagcaccttcaatgaacttactgccgacccggataccgtgatcgtggacatgagaaaccattacgaatatgaagtgggtcattttgaaggcgccatagaagtaccttcagatactttccgcgatcagctgccgatggcagttgatatgcttgcagataaaaaagacaagaatatcatcatgtactgcaccggtggaatccgttgtgaaaaagcatcggcttacatgctgcataatggttttaaaaacgtatttcacctggaaggaggtatcattgaatacaccaacaaagcccggcagcagggacttcccattaagttcaaaggtaaaaattttgtattcgacgaccggcttggggaacgcatcagcgacgatattatcagtcattgccaccagtgcggagcgccctgcgatacacataccaactgccttaacgatggctgccacctcctgtttatccagtgcgaatcctgcgcgaagaaatatgatggctgctgcagtgaatcctgccaaaccacccatgcattaccgccggaacaacaggcagaactgcgaaagggagtggagaaaggacttatgttcaataaatcccggcgaagaaaagtagaataaaaaatccgccccgcgttgtttcttctcggcagggcggagtagttgaccataaaattgaatcggccggatcactccggccttttcttttttacgaccattctatcaacctatatgcgaactaaaaatataagcgtatagtccaccacgttataacaaactaaatgaaaggactacacgcaatttcatcctcacatctgatctttcttatttttataggcgccatagaaaatgatcgggaacaccagcagtgttaatactgttgcggtaataagcccgccaattaccacgatcgccagcggcttctgtgtttcagacccgataccatgtgatatggccgccggaatcaaaccgatggcggccatcatggcggtcattaccaccggccgtatgcggctctgcacacctaacttgatcgattcattcagcgataatctcgcttcgaggttcttatggaatacagaaatgagaatcaccccattctgaatacagataccaaacaatgcaataaaacctacccccgcagagataccaaagttcatattggtaacatgcaatgccaggataccgcctatcaacgcaaacggcacgttcattaacaccagccccgcgtcctttacactgcccagcataataaacaacaccataaagatggcaatgatactgataggcactacctgtcccagtcgttgggtagcccgcacctggttttcaaattcacccgtccagccaatgctgtagcctttcggcaatttcactacccggttgatcttcgcctgcgcttccgcaatagtgctgccgaggtcgcggtcacggacagaaaacttcacgccgataaaacgtttgttactgtcgcggtaaatgaaagccggtcccgtaatggttttgatctcagcgatctctttcagcggtattttattgttgttgatagtaggcaccatcaggttggccaggtcatcttccgttttacgatagttttcatcataacggatacggatatcgaattttttctcgccttcatacagctgggtagccgttttaccgccaatggccatttcaataactgcctgggcatccccggtggctacaccatactgggccattttgttgtcgtcgagattgatgctcatttcaggctgaccaatattccggatcacgccaagatccttgatcccctgcaccgttttcaattgcgccactacctgttgcgacaatgattccagcttcacgaggtcgtcgccgaaaatctttacgccgttggcagccttgaacccggctactgcttcagaaacgttgtcgctgattggttgcgagaagttgaggatgatacccgggtatttcttcagccgttgttccatctgggaaatcagctcgtcctgcgtgatcttccgtttccattcttccttcggcgccaggtctacctggtattgtataaagtaaaaaccgttgggatctgtaccatcgttggagcggcctacctgtgataataccctttttacttcggggaagccgccgaggtcctgccggatatcatgcgccattttagtgctttccgtgagcgacatgctcatgggcaactccgtggttacccacagggagccttcattcagctgcggaaggaactctgttcccaggaatttggcggaaataaacgtaagtatcatgaaggccagtgccagcgtaatgctcaggcgtttattccggtaggtccatccaaaccctctcattacaaaacggtcaaagaagttcaccagtggattattcttctctttcacatttttgttgagcaagatggaacacagtaccggcaccagtgttaaggtaaagagcagtgcgcccagtaacgcaaatcccaacgtccaggccagtggcgaaaacattttaccttctactttctggaaagaaaatatggggatcagggagatgatgataatgagtttagaaaagaagatggctttggccagttctccaccggtttgcttgatccagcccagcttcgccattttgttgaaccgctccatgccgtatttgtgggctttatggtccagcatcacgaagatgccttctaccattaccaccgcgccgtctatgatgataccgaagtcaatcgcccccatcgacagcaggttggcgctcatacctttcatgcgcaggcacataaaggcaaacaacagtgccagcgggataatgatggatacaatcacggtagtgcgccagtcggccatgaacaggaatacgatcaccgttacaaaaatgatcccttccgcgaggttgtgcatcacggtgtgggtacagaactccatgaggttatcgcggtcatagaacgtttccatcttgatatcatccggcaaaatggtttcattcagctccttcagcttctctttcaggcgggcgagtacttctgtggggttttcacctttgcgcatcaccacaatgccttccaccaggtcgtcgttgctgcctatgcccacctggcccacgcgcggggcagaggcttcatgtacatttgcgaggtcttttaccagcaaaggcacgccgttgatattctgaacaatgatgttgttgatatcggggatgctgtttagcagcccgatgccacgcaccacgtatgcctgcccgttcttttcaatcacatcaccgcctacgttcacattacttttggtcactgcctggtataattccagcggtgtaatatcgtatttggccaatcgtaccgggtcagcggagatctcgtagatcttttcctgcccgccgaaggcaactacatcggctacaccgggcacgctccggatctgccggtctatcacccagttctgccaggtgagcagatcgcgggaatcgcgtttactgcttttcaggtagtaccggaatatttcaccggtaggaccgtagggaggctgtacttcgggttcggcgccctccggcaaactgatactctgcagcatgttgttgacctgctgccgtgcgaagaaatcttccacgtcatcgtcgaacatgatcttcactacagataacccgaacatggtaacagagcgcacactggttttcttctgcaccgcattcatggatacttctatgggcagcgttacaaagcgttccacttcctgcgcgctgcggccattccacttggttacaatcacaatctgtgtgttggtaacgtcggggaaggcttcaatgggcgtatgcaaaaaggaaaacacgcctgctgcgatcaaagtagctacgctgataaaaacaaacagtttgttcctcagcgaaaaagcgacaatatttctaatgaatttattcataagtcctgttctttagaatgccactctggtccttaatccgatgatatttaccggtccgcggtccccgttgtaggcagggtgcatcacaaactggtaatcagggcttagggctatatgtagcctggtaatgttacattgatagaaaacttcggcaatcatttccggtgcgtagttcaactggccgtcgccgatcatgaatccggtgccaccggcagcaaggtagttgcggtgctcttctgataatccgttcaccaccagcgccacaccggcgttatcctggttgcggtgccagcactggccgttttgcagccatccggcgctaacagagcggtctatttcggtataagcccaggtttcattgcggccatcattccacgatgctttcaggaaagcgccgccgctgttggtaagttcctggtctatattgataccaaaaccgtatttagtatgtccgtcccttcttacggaactgacgtccggcgtatcttttgcggcactcaccgcttcgttataattgcccataggagcctggttaataaaagccattaaccggacattcccttcatgcttattcagtgtatgcgtatgcgttacttctattacctcaccgttggatttaccgtattggtagttcaatttcggtccgttggcttcttccggctccagggaagtagctgcctgtaacagccagttatccttccggtactgaatggtcagcgccatggtatagccgcgtacatctgctgggtagtcccatgcggcattgctcatcagcgaccagttcataaactgggtgcggggatcgtggctatacgtattctgatcaaagaaatccgcgaggcagtatttaccgccaatgaaacggagatagtgggtaggcgtggcgccgcctacatggttcagatcatcaccatctgcttcggtattggaagttaacggtaatgtatacacgccataagccctggccaggtatattttcggtttgggatcgcccacgcgaaaggtttctccgttcgggaaacccgcaatgccggtggcatggctgagaccttcaccaccagcgagttccgggttcacatataattcaaagttcttccacgggcggataccggcataaacagtactggtaatagatgtagcccctttttcatgggtacggaaactgttggcgcctgagtacttcgcggagaaatcaggatgccattgcgttaccagtgtttgctgaaaatggaaagtgtaggggataatgctatccgtcttcttttcctgtgccagcaggcgggtactgcccagtgccagtattcctatggagaacagctgcttcatggcccgcttaatctttaagtgcatcgtagatgagcaattgatttttggaaatcactttctcttctgcggccaggccggaggagatataagtaatatcgccggatgttttagccacttctacctcgcgtacggctatattaaatttgtctttaaataccagcacataatttttgctgttatcaaagatgacggcggcagaagggacggctatcttttggtcgttatcctggtacttcacgtatacggtagcaaacatttccggcttcagcagcatgtttttgttatcgatgctgatccgtacctgcatggttttggtggcagggtccaggaaattgtagatcttatcgattttgccgtggaagggctcatcaggataacttaccgttaccacgtctgcttcatagccttctttgatacgcgcgatatctgtttcaaaaacattggccatcacccacacatcatccagttcggagatcgtaaaaatgttggaactgttatcggtacgtatctccatgttattattgatattcttctcaataatataaccggaaataggagcggttaccaggtaggtagcgcctttgcctttgcggtatatggtaaacagatcgttgagccggttaatttccgcatcagatttttgtacttctcctttggcgtttactacgtctttatctgtgttcaaacggctgtcgaacaggtcctgggctactttgaggtttttgtctgctacattgcggtcagactttgcctgggccagctgcttttcgtaatcagcaatttcagcactgtgtattacggccagtacctggcctttctgtacatagtcgcccagctgtactttgatatcttccacatacccgctcaccagtgggtatactttcaataccttaccgccattaggggtaaccttaccggataaacgaacttcgttcaccaccggctgcaggtatgccgtatcgatacggatatttttcagcatggtatcgctgagaacgaaggtggttttctcctgatcttctgcctggctgtgtttacaaccactccacagaatagttgccagcagcgaaaagccaataaaaaggaaaggctgtttcatgcgcttaatttttaaataattcttgtcctgttgcatagttgagttcttcgtaggcatttacccggttggataaaaacttgttgatatttttcgcgttatcgctataactgttgaagtaatcgatgaactgaagaagggagatatttcctttgctgaaattcttggctacttcagcaatcagggtatcaaattctccctggaaccggtgcaggtcaaatcctttgtaacgcttttccagtgctagtatacgctgataagcattcaatacttctgattgtgcgatggattgctgttgcagtagttgttgttgttctgcgccgatttgaagttgtgcggcgcggatatttccctggttgcggttccaggtgggtaaatcaattcccagtgtcaggccaacgaaattaggcgtgtaactaccttgtttatcgtaggtggcgcctacatgaaggtccggcactgccattgatttctggaggcggtagttgagctgtgcggtctggaactgcacgtcagccatccgtacatccggcctgttctgcgctacgctgtcgagtaatgattgcagctggatcttatccaggttatatgaagccaggtctgcgggttgcagccgggcctcataaaaaacgctggtatgtaacaactgttgtaggtttttctgtgattccaattcctgttgtttcagatcggcgaagtcgttttcaatgcctacctgtaatgcctgcagcctgacgagatccgcatgggccacgcttccttttttatcagctgttacatatgcatctacaattttctgcaggttatccagctgttcttttaacacggtttcaatctgttgctggtagtatacattgtagaagttttcccggagttgtaagcggagggtacgcaccagttcatcgaagttggcctcgctcattttggcggctgctgcggccagttgtatggttttattccgtttgcctgccagctgaatgagctgatcaaggttatattgtgtttcgccgccggcgcccacattaaacggtttaaagttattagtgctgccaaaacccagtacagtgctgaaggaaggattgtcccacatcttcgcctgccgtatcagcgctttggaggcgtctacctggtagcgttgcgccagtaataaatagttttttgtaagaaatgaatcttcaactgcctgcagtgttacaggttgagaagtgatttgcgcctgtgcatgttgaataaagcccaggcagtaaatacacgctgttaggaacagcatcctgatagttcgcataatgccagatttcatggcacaaagctcacaaaggggaattaaagcggcctttaaggaagattaaaaaaaaattaaaagaaatttatacgtgtgggaggaccacggagaatgtagtgcctccttcaggattggaggtaacagtaatatgcccgccatggatctgcacaattttcttacagatagataaacccaggccatggccgcggatttgaagcacattttgcccacggtaaaagggttcaaatattttgttaatatcgtccggtggaataccaatgccggaatcttttatctgtataagaatatttttcgtgaaaaaatctatcgacacatgcgcagtattattttctgaaaatttacacgcattatcgatcaggttcaggaaaagcaccttcaacaggctctcgtttccatagcaggtcacgagcaaatcattatcaggtacctttatgaaatggatctctactttactggaagttttttgtttcagccggatcagggtggtcatctccatcagtaactcatctatccttacattcgtcaatacaaactcctgctgccgcatttccgactgtgccagttgcaacaggccgttggaaagatcggagaggttttctgcatcttccagcacagaagtaagtagtgccaggtattcttctttgctccggtctttggataatgccacctgtaactggctgataatagccgccaggggagtacgcagctcatgggaagcattgctcacaaagcttttttgcaggtgaaacgactcgctgagacgttgcagcatagtgttgaagttggcgcccagcttggctatttcatcttttcctttcacggctacctgtgtatcctgcatgttgttggcattgatactatctacctgctgtaccagctgatcgattggctgtaccattttacgcgcaaaaaagtaacctacgcccaccagtactatcacggcggtaatcagctccagcagcaggatctggctgaggttctggaggttttgaaaaccatatttatcaaaggaagatacaatgacgatgacagatacgttgccttctgtataatacacgcccaccacttcgccaacgcctttgtcgtagctgtacagtttattttccttgatataatcgagtaaactgggatgtgtgcggatggtagtatctttcaggttgctgtacagcaggtcgtaattaggattgtatacgagtatggtttctttataaagatcctggaaggtggtccggtccagcttccgcagcaggtccacctttacgttgccatcttcaatgatcacgttggcaatggagcgggcgcggtattccagccgttccaggtattccgccttccgcgacttggcagagaaataataggccagcacggcaaatgcaacgagcatcagcgtagccgacagggtataataaagcgctattttatatttgattttcaaccggtgtgttattcttcagaaagataataacccatacctgtttttgtatgcaggagtttctgatcaaaatccttgtctatttttttgcggaggaagttcatatacacttcaatcacgttggtaccggtatcgaagtcgatatcccatactttttcagcgatggtgattttggagataaccttgcctttgtgcatggccaggaattccagcagctggtattctttggcggtgagggcaatctttttaccgccacgggttacatcttttttctcgcggtctatttcgaggtcggcgatcgtgattttgtactgggtgccatgcgtggcatcggagccggctcttttcaggaatacccggatgcgcgccagcagttcgcggaagtcgaagggctttaccaggtaatcgtcggcgcccagctcaaaagcctgcattttgtcttccacgccaccgagtgcggtgagcatgatcacgggaacgcggttgtttttgtggcggatcacttcacacagctcataaccgttgttgtgcggcaggttcaggtccaggatcaccaggtcgtaatcgttactggtagctaatcctttacccatacggccgtcgtaggccacatccacatcaaaaccgttttcctccagtcctttcttaacggcattggctactttaacttcgtcttcaacaaccagtatcttttgcatagaaagggtttaagtgttgttatacaggcatcctgaaagatacctgtataacaaaataactaactgataaggttcgcttccagctgcattattttctcaaataactgctcatattgctgattggccctgtccaggtacttctgaacatcctggtattcgctttctacctgggcaaatttagctttatcattgtagatttcaggagaaccgaggctggcttccaggccggccttacgttctttcaggctggccacctggccttctacctgtgaaaactgtttttgttgtttctgcagttcacgctgtacgtctttgttgatagcgcctttacctgcatctgcaaccggggctgctgcctgctggcggctttcttttttcgtatctgcgttattgttagtggctttggcgttgccgttttgttgctgggcagccattctctttttccactcttcgtattcgttgtaggtacctttaaactccttgatttcgccgtctacgatttcccagatcttattggctgtctggcttacgaagtaacggtcgtgggataccagtaccaggctgccatcatatttgttcagggcgtctatcagcatctgcacggagttcatgtccaggtggttcgtaggctcatccagcatcaggaagttcgcctggctgataatggtttttgccagcgccacacgggctttttcacctccggacaggatcttgatcttcttaaatacatcatcgccggtaaagaggaagcagcctaacaactggcgtaattccagctctgtacggccgctgccgaagttcttcagctcgtccagtatttcgctgttcatatccagtgattccagctggtgctgtgcatagaagctggttaccacgttatgaccgggtacgcgttctccttccatcggttccataccaaagatgatacgcagcagggtagacttacccttaccattggcgccgattaaggctattttatcaccacggttgatttcagcgctggtattttttaagatctctatcttgccgaagcttttactgatgttattcagtgtacataggatcttaccaggtgttttatctactgtgaagtttattttgattttagaagggccgttatcggtttgttccacccgctccagtttatcgagccttttggcgatactctgtgcctgggcggctttggacgctttggctttaaagcgttcaataaagcgttcctgctggcggatataatcctgctggttttcgtaagcgcgttgctgcatttcccggcgaagttccttttccacttcatagtcggcgtaagaaccggcgtagtggtgcagttgctgctggtatacttccacaatcttgttcaccatacggtccaggaagaaacggtcatgcgatacgatgatcacagcgccgttgtaacctaccaggtatctttccagccattcgatggagggaagatccaggtggttcgtgggctcatcgagcatcagcacatccggctgctgcaggataagacgagccaggagcacacgcatgcgccatccacccgaaaactggctgtacggccgctccaggtcggaggtggtaaagccgaggccttccagcacctgcgccgttttatgtttcatgttgtagccgtcgagcgcttcaaattcatgcagcttgtcactgaattcgtgcaacagttcttcggtctgactgtcttccagctcccgggtaatacgttcaatatctttctccagctccagtgctttgccaaaggccatcatgcctacggtaagaatagattcatcggtttcaaagctgagcaggtcctggttaaagaagccaatcgtcagacttttacttttattaacacttcctttggaaatggaatattccccattgataatgcgtaacagggtagatttgccggtaccattcaacccgataagccctacacggtcacccggttctatatgccacgaggaattttccagaataaccctggacccaaactcaaacgtaatgtcctgtaatgcgatcaacataaaaaataaaaaaattggataaaaaacgtgcaaagttaaggaaaaatgcggactttaacctactcaaattcagtactccaaagaaacaatccgctcattttatttagttttgttacaaagtgtaagattatgaattttaaagtatgcgttccggttggcttactgatgctgggtgtggccctgtttgcctgcaaccagcagaccgccccgaaacaggaagaagcggcagcaggcgcttccgccgcgttacaggcgccctatagccaggtgttttacgactcactgggcgccgccatgcaatcgtattaccagctttcggatgcgctggtacaggctgatagcactgccgccaataccgcagcagcgacactgaaagggcatgtggacagtttgccggtcaaccttttacagatggatagcagccacctggccaatattaccggtatcaccggcagcgtaagcgctgaattaaccggtctggcaggagaaacagggctggaaggcaaaagagccgctttccagatggtatccgatatgctgttcgaccttgtaaagaacaccggcctgaaaggtcatactatttatcaccagtactgcccgatggcatttgatgataaaggcgcgtactggcttagcgacaaagcagctatacagaatccttactttggccataagatgctcacctgcggtgaaaccaaagatagcctgagctataaataataagtaatcgttgaatcgtgcgcagtaaatcgtaaattactttcgctttgctgctcatgatttaacggtatgttcacacgatatagtccccttttattgttcttctttttgctgtgtttcttcaatgaggcagcgggacagcaatataccgtaagcggttttattaaagacagtaccaatggcgaatcgttgcccggcgccaccgtgcaggtgctgcattccaccaacggcgtacataccaacaactacggattttattctatcacgctgccggcaggcaattacatcctcctgtattcatttctcggctacgaatccaaagcagtggcgttgacgctggatgccaataccacccagcacctgcaactatacccgcgttcttaccaggcaaaggaagtagtgatcaccgacaaaagaaaggatgccaatgtgaaaaataccgagatgggaaaggccgagctgaccgcagtacagataaagaaactgccggcactgatgggggaggtggatgtgctcaaagccctgcagctgatgccgggggtacaggctgccggtgaaggcaacgccggtttttatgtgcgtggcggcggggccgatcagaaccttatcctgctggacgaagcgccggtgtataatacaggccacctttttggctttttctctgtatttaatgcagatgccatccggagcaccacgctcatcaaaggcggtatgccagccaattacgggggccggttgtcgtctgtggcagatattgctatgaaggaagggaataataaaaatttccagggagaagggggaatcgggctgatctcttcccggttatctttccagggacctttgaaaaaagataaggcctcttttatcgtgagcggccgtcgcacttatatcgaccttgtcacaaagccatttatcaataatacttcgtataagggttcgggttattatttctatgacctgaatgtaaagatgaactacgctatttcggagaaagaccatatttacctgagcggttatcttggaaaagatgtgttcagctttaataaccaggaccgttcctttgatgtaaagattccctggggcaataccacggctactttgcgctggaatcacgtgttcagccagaagttatttgccaacacctctctcatctataacgactataaatttcaattcagcgccctgcaaaataatttcgatatccggttgtcttccggcatcagcgatatgaacctgaaaacagattttgactattacgcgcatgtaaagcatcatatccgttttggcggcaactatatctatcacacgtttacaccctctactatcagcggggagcaggattccaccaaattctcccccgagaatgtgtttaagaaatatgcccatgaggtggcattatacctgatggatgactgggaaatatctcccaggttgcaattgaatgtgggtgttcgctacagcgggtttatgcagatcggcccttatacccgctactcccgtgatgcagcggggaataaaacggatagtgttgtataccggcgctggcagccgatatcccgtcatggtggctttgaaccgcgggtcatcctgagatggtcctggaacgaggtaagttccgtaaaagcttccgcaacccgtaactatcagtttattcatcttgtatccaacgcgggaactactttgcctacagacgtatgggtgcccagcacttacctggtgcagccgcagatttcctggcaatattctgccgggtacttccgcaatttcagcaacaatatgtatgaggcatctgccgaggtatattataaaagcctgcaaaaccagattgaatacagggaaggatacactccatcgctgaatgatccggagcaggacttcgtgttcggaaagggggaggcctatggcatggaattatttgtaaacaaaaagaaagggcggtttaccggctggctgggctatacactggcctggacctggcggcaatttcccgcgttgaatgatggcaaccgttatcccgcgaagtacgaccgtcgccatgatctggccctggtaggcacttacgacctgagtaaacgctggacggtgtcaggtgtgtttatttacggcaccggtaataccactacgctacctgaaaagttctattttatagaaggcacgctggtacagggttacggcagtatcaactcctaccggctggatgcctatcaccggctcgacctgtcggccatatatactccggtgcctaaacggcccaataagcgtgtgaaaggcagctggacattttctgtgtataacgtttacagcaggaagaatccttatttcatttactttgaccaggaggggagcgccgtagatggcacgttgaaggtgagtgcgaagcaggtgtcgttgttcccggtgttaccgtcggtgacgtataatttcaggttctagccgggattcaaaaggggtgatagtacctgaattcaaatgagatgatagtacatacaaatggggtgatagcgggggattacctcacgaagcagtacctgataattcctaccagggcagccactatagcaatgaattgcgcaatggcggcatagtgtaccgatttgatcagttctgctttaacgtcctggatagtgcccagcagctccgatttaaccttttggatgtccgttgttaattctgacttaaccttttgaatatccagcgtcaacccgttttttacaaccgatagctcttctttggtggccatcagatccatacgggtggcaagcttgtggatatcctgcttaagttcgtttttaacattcgacagctcttctttagtagccatcaaatccatacgggtagcaagcgtgtggatgtcctgcttaagttcgtttttaacatcccatagttcgcctttagttgccagttgttcaatttttgcggatgatttcctttcataatggtcatccagcgcatttacaacttcgagagctttgtcatccggcaaatgcaggtcattccggaagatgtcatacagtcttaagtttccgattgtcatatgtaatggttttatattacagggttaaaattaatttattctttatttcgatatcgtgataattacagatatttcttttaaatatatcaaagctgatggctgtttattattttgtaactgtgaataatattttgatgtaaataatctcaaaaaggcatccgtattattgccaggagcgctatatcagggaagtttttggggggcatagtgcattgggagtgcatgcctagtgcatggggagtccatgaggagtgcatggtaagtgcattgatactgcatggatgacccatgacatacgctggtttgaggcataggtgaagcaggggtgaggtaactgttatcttttagcttaacttcccctaaataagatcgtctcacccggtaaatcacatggattgtaatgttttatcattataaatgtgcatttaagccatttttcaactgtgttcacaccgctgtataaatatttatttttaaaatccttaagttcaacgacatggttatctaaaagctaacaaactatttcttaacttcgcaaacattttataaaggaaatatagcccatatgaaaaagtatggtgctaacagcaaaacgtatgataaatatcacttttccggatggcgcagttcgtcagtatgaatcaggagtaactgcattggacattgccaaatccatcagcgaaggattggcacgcaaagtattggcagcaaatgttaacgggcaggtagtggatgctacacgcccgattttgacggatagcacgctgcagctgctgacgtgggtggataaggatggtaaggcaacaatgtggcattcctcggcgcatctgatggccgaagcactggaagccctgtaccccggcgtaaagctcggctatggcccttcaattgaaaatggattctattacgatattgatttgggcgaccgcacgatttctgaagaagatctgaaggcgatcgaagcaaaaatggtggagttgtctaaacacaacagcgaatacgtgcgcaaagaagtaagcaaggcagatgccctgacttattttactgaaaaagacgatccgtataaaatagaaacgatcaatgaattacctgatggaagcattaccttctatacacagggcggattcaccgatctttgccgcggaccgcacattccgaataccggctttatcaaatccatcaagctgacgagcattgcaggcgcttactggcgcggcagtgaaaaaaataagatgcttacccgcatctatggcatcactttccctaaccagaaagagctggacgaatacctggccctgatagaagaagcaaagaaacgtgatcaccgcaaactgggtaaagaactggaactgtttgccttctctgaaaaagtaggtttaggtttacctatgtggttgcctaaaggcgccatgctgcgtgaacgcctgcagcgtttcctccaggaagcccagctggccagcggttacctgccggtagtaacaccgcatatcgggaataaaaatctgtatgtgacttccggtcactacgaaaaatacggaaaagacagttttcagccgatccatacgccggaagaaggtgaggagtttatgctgaaacctatgaactgcccgcatcactgcgaactgtacaaggtatcgccaaagtcgtacaaggatttacccgtgcgctttgccgaatttggtaccgtgtaccgttatgagcagcatggtgaactgcacggtcttacccgtgtgagaggatttacccaggatgatgcgcacctgttctgccgtcctgaccaggtaaaggaagaattccagaaagtgatagacctggtgatgtatgtattcaacagtttgagttttaccgagtatactgcacagatttcactgcgtcataaaacggaccgcagtaaatacatgggtaccgaagagaactgggagctggcagaaaaagcaattatcgagtctgccgccgaaaaagggctgaacaccgtggtggaatacgacgaagcggcgttctatggtcctaagctcgacttcatggtgaaggatgcactgggccgtaaatggcaacttggtaccatccaggtggattacaacctgccggaacgctttgaactggagtacatcggggccgataaccagaaacaccggccggtgatgattcaccgtgcgccatttggttcactggaacgctttatcgccgtgctgatcgaacattgcgccggtaaattcccgttgtggttagcgccaacacaggtgaagatcctgccgatcagtgataaaagccaggcctacgcagaaaaagtagcagaattgctaaaaaaagcagaaattcgcgctgagatagatgatagaagcgaaaagataggtaagaagatccgggaagcagagctggcaaagattccgtacatgctcgtactcggtgaaaaagaagcagccgacaatgtagtagccgttcgtcgtcaatcaaaaggtgatttgggaactatgcaactcgaacagtttaccaccatgataaacgaagaggtagcaaaccggaagccaattgagtaacatcgcataaatgtggaaaaaaggtatataaaacaatgaacattactcgattgaggtatgttaattgctgtaattttccccgtatttttgtaaagattgtttttggtccatggacgagatgtggaccatggactaaaaggacaattaattaattaattttatttttcttaatgcaacaaagacccagaccaagcagttttggcggcaacaaccggggaagaaaccccaacttccgcagggaacaacaacaagaacatcgcaccaacaggatgatacgcgttcctgaggtacgacttgtaggtgaaaatattgaggtaggtgtctacaaaacagaggatgcactgcgtatggctgaggaacagggtttagacctggtagagatttccccgaatgctgtgcctcccgtttgtcgtatcatcgactacaacaaattcctctacgaaaagaaaaagaaggaaaaggaaatgaaggcgaaggcgcacaaaagtgaagtgaaagaaattcgctttacgcctaacaccgatgaccatgacttcgatttcaaagcgaaacatgctgaaagcttcctgaaagacggtaacaaggtgaaaacctatgtacagtttaaaggacgtgccatcatgtttaaggaacgtggtgaattgatcctcctgaagtttgctgaaaggctggcagaagtaggtggcctggaaagtatgcctaccatggaaggtaagcgtatgatcgccatctttgcccctaaagcagcgaaaaagaaggaaaaagaacctaaggaaccgagagaaccccgggaaccaagggagccaagagaaccgaaagaagcaaaggcgcccgttacgcctccagccgctgatgcagcaggagatgccaacgcatagccgatggttatatcacattaaaaaagcagcacagcagggtattataccttgttgcgctgctttttcttttagcgtgtaacctgttattgtattgcttttagtactttccgcgccctggaacggatagccggtgtgggattattttccagctccgctgctatcagcagccggatctcgtttttgatgtcagggtaatcttttgccaggttagccagtaccgtcatggaaaaggctttcaccgccactgcttccagcggatcttccaggaacgcaaaacaactgttcatcaccggcccttgcagggattccgggactggcaggtattgcaatatcctcaatacatttctctttactgccaccggcatacccggttcctccatcctggctaccatagccggcaggtggggagcaagcaacgcggggtacttttttgccacaaagctcacaatccacgcggcccgttgtaccacgcggtattcgtcgtgcaggaacaagtgtatcaaggcggcaaaccgttccggatggggacctatccaggtcgcaatgcggagcgactgggcacgggaattttccgataaaatttcagtacgcagatccatagacctgcaatttaatacacacgagttaattattggcggaagtactgtttgccagcaggtaggcgagcgttttttcacgcatccgcgctacgtcttcaggcttcaccggcatatccgtttccttgcccatatcatcccagatgcggatctggatgtattggtggaataaaggatcattgcggaacgccagcgcctcttcttcattcataggcccaccctggtattcgagggtttgtttgctggcttcggagagggtatcgtaataggcgctgtccgaccaggtaagatagcgtttcgcggccacatgactgcccaccagctgcgccatgcgctccgggaagccgcattccagcaggaaagcgctgcccaggtcgtcgtgtgcgcgggtaccgaggccgcccatctggggcgcactttcaaaaaaatgaccaatgtcgtgcaggaatgcagcaacgatcatttcatcatcaaagcctgtgctttctgctataagggccgcctgcatcatatgcatcagcatggttacctgctcgccatattcctggtggccgtaagtattatacaggtcgaagattttgttgactactgattgggcatgtaattcactaccggtcattttcgtacgtttataagggttagtacagttttttcatagtatgccgtggcattatcgcaaatgtaatagctgcaactgctttatcagcacgcctcatgttatgtttttattaataccggagtggttttcaaacgccaataatcctttacctttgccctttacattacacaaaactgaaccattgctaaaaaaagaactgcgcgtcatactggtgtcgctgatcgttagttttatactaaccgtggcgaaattttcggcgtactttatgacccattcggtggcaatcctttctgatgccctggagtccattatcaacgtggtggcgggcggttttgcctgctatagtatttaccttgccagtcagccgaaagatgccaaccatccgtacggacatggcaaagtggaattcttttcgatcggttttgaaggcgccatgatctttatcgccggcgtgttgattcttgtgaaaacggcacagtattttatcctgccgcgtgaactgcaccagattgaaaacggtttatgggtattgggcgctaccactgtcgccaacctgttgctgggcctgtacctggtacgttccggtaagcagctttcttccatcactatttcggggaatggccagcatatcatgaccgatgtttacagcagcgcggggttgattgctgcgttggttgtcattcatttcaccggctggacctggctggatcccgcggtatcactggtgatgggcggattgatcctcagcaaaggatatcaattgatgcgccggtctatttccgggttaatggatgaaacggatatgaagatagtggacaaggtgatcactattttatcggttcatcgcaggcagaactggatcgatatgcataatatgcgtgtgcagcaatatggcaacaactatcacattgattgccatgtaacgatgccttactacctggagctgaatgatgcgcatgatgaaatgaagaagattgagaagctcgtgaatgaagggtttgccggcagtgaggtagagttttttattcatatggacccctgtattccttcctgttgccactactgtttaaaagaagcctgcccggtccggagccatgcatttaccggcgaaataatatggacccgcgataacgtgctacccaacagaaaacatggatagtaatacatcttgctataaaaaaaccagcataacttatacaagctatgctggttttttttatagtcagatgtttaactgtttattcttctccagcttcttcaccatcaccatggccgatgatatcgcgaataggttttactgcctggtaaataccgcggttgtatttgtttcctaagataacaagggtggtagaatcctgtatgaaacgatagaacacggtgttgttaccatgccaccagccgttgtgataaataatattttttgtactgtccggatataccataaggcgccatcccagcccgtaattgcggacgccgggcttctcattgctgtaaggcgtgtaggcagcctttaaggtagccgcattcaggaactggcctgaatagagggcctgatcccacttcagcatatcctgtgcgctgctgtaaatacctttatcgcccattacaccgtcgaagtaagtatccggttcaaactgcccgttatatttatggctctgggtttggtgcacgcgcacagcagaggaggggtcgtatacaaaagtgctggtcatatgcagcggtccgaaaatagtttgctgcatgaagtcggcatatttctgtccgcttaccttttcaataatagaagcaaggagcaggtaattggtgttgcagtactggaagtgcgtacctggcaaatgttgcatggcgggcttatgcgcttccattaatttgatgacttcgccgttggtaataaagttggcttcctctttccataaactgtcgcagaaataaaggtagttaggcaggccactccggtggttcaggagcatgcgtacattgattcctttataaggaaattcgggaaagaatttttgcagggaatcttccaggctcagtttctcattttgtaccagccacattactgctgcgccggtaaaggtttttgtaacagaagccagctgaaaggaagaactgtccatcaccggtgttttagtccgggaattttcatagccgtgatacttttcaaagataaccacccctttcctggccactatgatggcgccgttgaaaccggtacgcaggagctttccgttatagaatgcttccagttcctgttgcatttgtttagtacgcggtgatttaaggatggcttctttttccgcggccgatagtcctgttgtaaagcgtgccgaatctgctgctgctttccttttactttcttcccttcttgctgcattgctctggcagctggagataattgcaattcccgatatagttaagataatacttattgctttcaatcgcttcattagaggagttgtgactactttcttaattcaattttcgacccataaaatacaaagcgctcaatttagactcaaagtaaaagactgccaaataaaaacagtgatttcggattcttttaattgatttttaagcaaaaaagtgagaaaaactttaaaaatcatccccgatttccgtctttttttgataaaatcgaatttgattcccctgctatttgaatattcctcaacttcgagtaggtttgtgccctgtttccccgctatcagcaattattaagccaattgcaacacagagatacacatataacttagtataatattatggaccagcaaaagtcgacaagttatccgaaagagaagatcagcattttattattagagaacatcagcgatgctgcggtggcagaatttaccacggcaggataccatgtgcgcaagcttaccggtgcgctcagcgaagaggatcttatcaatgaaatcaaggacgttcatttactgggcatccgatccaaaaccaaagttacccgtaaggtactggaatcggccaggaaactgcaggctattggttgtttctgtatcggtaccaaccaggttgacctgaaagctgctacagagcacggtgtaaccgttttcaacgcgccttattccaatacccgttccgtggctgagctggtaataggtttgtctattatcctcatccgccgcatcgtggataaaaacaatgcagcgcataacggcatctggcttaaagaagccactggcagctatgagctaaggggtaaaacacttggaatagtaggttatggcaacatcggtagccaggtgagcgtattggcggaaggaatgggcatgaacgtaatttattacgacgccgaaaccaaattgccgctgggtaatgcagaacagcaacgcacgttgaaggaactcttcaacaaagcggatatcgtttcgctgcacgtaccttccagcaaaaccactacgaatatgatcactgcagaagtgcttgcagatgctaaacccggggctatttttattaactatgcccgcggtgaggtagtagacctggaagcgctgaaagatgcactggaaagcggacgtttgtccggcgccgccatagatgtattcccggtagaaccggaaaagaatggcgccgcattcagcacgccgctgcaaaaattatccaatgtaatcctcacgccgcatatcggcggaagcacggaagaagcgcagcacaacatcggactggacgtgagcagtaaaatgctcaactacctggaaaagggcgccagcttcggttctcatacggtacctgctatcagcgtgccgcctattgaaaacacacatcgcatcctgcatatccaccggaacgtgccgggcgtgttgtctgccatcaatactgctttatctgccaacaaaatcaacatcctggggcagtacctgaaaaccaacgaccagatcggttacgtggtactggacgtggatacgaggttatcacaagaggcgctggctttgctgaaggaagtagagcatacgattaaaacaagattactgtattaataaaagcaacaatggatttgcgggcgaacggttttagttccccgcaaatccgtgatgctcacccaccatatctccccgttcaccgactctttttactcatatacgttttttcttcccgtattttcaaaattctttgttaaccttgtagtgcaactgaaaaaattagcacatgaatatgaacagggtactgacagcaggagcaggggtaatagccggtcttttgttgtatgtaaatgcttccgcacaagatagtgaaccaaataaatgggcgccagcaaatatcaaaatcgacggacaggctactgaatggcccaaacccctgcagttttataacaacgttaccaagttattttacacaatagccaacgaccaggagaatgtatacgtaatcgttagtgttcctgatccgcaaagccagatgaaaattatgcgttccggccttactgtttccatcaaccctaccgggaagaaaaaagggggcgcggggattacatttccgctcacctataatgtgaacaccggtgcgccggatgtcccggaagaatcccgggcactcattgcaggtgaattgaaaaaacaactcctggcgaacgtaaaggacatcaaagtagaaggatttgacggcatcccggatggcaatattccggtgaagaatacgtttggtattcaaaccacctcctcatatgatgccgccggtaacctggtttgtgaactgggtatcccgctgaaggtgctgggtatccccgccggaagtgataagcccatcgcttaccattttaaggtaaacgccatgaaaagggaggataaaaaggaactggaggccaaacgtgccaaaggagaaaagcccccaatgccaggtgaatatgcggaccaattcgccttgtattattcagccgacttttggacacgtcaaacactggccactcaaaagtaagcaaccagactaccatcgtcttaactgtttttatgtataaaaaactgttttctgcgggaactaccaccatactggcgggagccttgtgcacaggcacttttatgtcttgccacaaagataaaccagcccctccgcctgttgacattacagacgccctgaagaaggactccctgaagtacctgatgtaccagatcatgcaggtaacttacggcgatggcggacgaacggtcagcaaaggattgcctacttactactggtattccagtgtaccgcagctagatcccctggccagcaagtatgcggatgcaaacgccctgctgacagagatgaaaggctatgccatcaacccggccaccaatgccgcatacgaccattacagcttcctggatgaagatggtaccatcaccaaccagctgatgaatggcgtatcggaacaaaatgccgccgccaatccctctaaactgggatttgacatcggttttgctgccggagcggatgccagtaaagtaagattatttgtaaagtatgcagataagaacagccccgccggtaaggcaggcgttttaagagggtgggagattatttccgtaaacggtaataccaatttttccagtgcctcttctgctatcaactcgctttataatacgatttcaacggcatccaccatcaccctgggatttaaaaaacaggatcagacttcggttacccttactatcaattccgctacatacaacataaacccggtgctgttcgataccatttacaccgttaagaataccgccaacataaatataaaggtgggctatttcgcgatgtatactttttccagtgtaaccaacgacgccggaaatgctaccgctaccaaaacggctttggatcaaacgatcgccaaattcaaagcacagggcatcaaacaactgattgtggatttccggtacaacggcggcggagccacctctacagcggaatacctggacaatgcttttgctccttcggctgccggcggtaaagtgatgtatacctacaagtataacgataagatcatgcagaacctcgcggctaccaaactggatgcgcaggtgaactttgctgctgctacaggtggtatgtcactggacaatatattctttattgtatccggtgaaactgcttctgccagcgaattaacactgaacaaccttaaaccgtacatgaatgtaaggctcatcgggaagaagacatacggaaaacctgttggctttattgattttaatatctccatgtatgataatgatcataaaccggtatacctcgctgacctgtacgccatcaacttcgaaaccatgaatgccaacggcaacggggggtactacaccggtatcccggtagatgcggaggcagcggactatgtaaacgttgcctggggcaacactacatcggatcagaacctgcagcaggccctgaactatgtttcaacaggcacttacctggatcttcgtaccagcgccaggatcagcgcagctgccggcaatgatttgcgcgcggctattcctggtattacgcctgccagagggtttaacggaatggttgatttcaggttaagcaagaaagtagcaggacttcaataacatatattctttaacgttagccggccaattcaagccgcgttgatcgcaagatcaacgcggctttttgcttcatagacaataaaaaagtccggatacgtatatccggaccagttagctgatggaggaagaagtatcagcggtgacccagtttccggatcatatcttcagacatatcctctgaataaacaccatacccatacatcaatacgcctttgagacctgatttcgtttcaatggcatacactactgcctcatcgccggggtccgtatctccttcaaagcgataggtttctgtaatgtcaaaatcctccggccgtacattcccgctgttacactgaatactgtcgaaaacaaggttgaaatcggtggtgtatccgcgtttacgcagatcttctatggccgctgttacggtgtcgtacactttcatataaaaacaatttccggtttgcaaatgaaacggcactaagttaataaatcgccggggatttgatggagttggatataaaaacaaaaagcataaagccggttggccttatgctttttgttttatgatcgcgtatccgttatcagcggatcacggtaacttctcctttcagtacgttggaggatccgccggctactttcttgtaagaaagccaccatacgtatgtgccaacatccaccggaactcccttgtatctgccatcccatcctttatgattgtcggacgacatgaagatcagttcaccccagcggttaaagatccgcagttcgtagtcgaacatttgtcccctcactactggcctgaacacatcgttacgtccgtcgccgtttggtgagaaggcgtttggtaaggttggtttaggttcacattctataaagcctacggtgatatcatcggtagcagatccgcaatcgttgaatacggttacggtataagtacctccgttggttacggtgagggatggtccgccggaaccgttatcccagcgtacaccggtaattccgccaccttcagcacgcagtatcagcgtttcacctttacacagggtggtatctcttcccaggttgataaccggtaagccggtgatatttactttcacgctgtcgaggaacacacgttgacagtatttatccatcacagctaatttatagctacctgcctgagagatctgtttaaccgggttaggatcgccgtcgttccagaggtaagaaatggcatccggattggttccgtccagggtaatggtgccaccagggcagatattcctgtcgggtcccagctccatagtgagcgctggtttcatccttacattcacggtatctcttaccacgcagttatccctgcttacggctacccagtatccgcctggcttgtttaccacgatagagttgctggtttcacccgtctgccatttgatacggccgccgttggaattaacggtgagcataatggactggtcaggacagatagaggtgtcgcggctcaggctgatgtctggcggaggattcacactcactttcacggtatcaatggtgatacatccggacttcatcactttcacccagaattgttcctgtgttcctaccaggatggaaggttctgtagaaccattactccagagataggagccaccatttacataagcatccagtttcacggtttggccgcggcagatggttgtatcagggatatcaaccagtggcgttggtaccagacctacatggatggtatcggtagtggcgcattcgccgttgcttacatttacccagtaggtgcctgcctggttaatattgacccgttgcgtggttgcgccggtagaccatttaatctggtaggcgaaattagcaggacctgcatccagcaccaggttgttgccaccacagatagtggtatcgttgcccaggttcaccattggtttctggatgtaactcagattgtaagtcacggtgtcagaggaacaacccgttctgccatccgtaatgatgaaggaagcagaagtagccccgttaaggttaaacacattgttgctttgtgttcttggcaatcctgttaccgcattggccggcgtaactgctaccagcgtataggaaggcaggtatacgttgccaactttgcgtaaagcgatcctgccgttgtctgaacagttggaaggcagggtagcttccagttgcggtttatcgcaaggcttaatgattacacgctggataacgtcgttggctttattgccgcaggcatccatgatggtccatcttcttataatcgtatatccgttacagatatcttccacatatggatcttctgtatagatagctcttttcgggaagctgttatcacagttgtctgttgcggttaataccggtgcagcagggatcttatcctgacagtagatttccacatctgcaggagcaggcatgatcactggtctggtggtatcttttacatttacgacctgtgtgatggtagtggtattaccacaggcatctttagcgatccaggttctgatgatgcggtagttgccggcacattctcctggtattctttctgtagtgatcctgcgggatacggtaagaccatttccgatgctgctgcaattatcagatacctgtacatcggtagcaggagcagggatgttatcacagctcactgttgtgtcggcaggaggcatcacagtgaataccggtttagtggtgtcctgaacggtgatgatctgctgcattacggttttgttgccgcattcgtcggtagcggtccaggttcttgtttcccggaagttagcggcgcagttacctggtaatttcacggttttgctactggtgaacacctggatgctgccgctgcaattgtcggtagcggtgatggcaggccatgccggtaccttatcgcaatctaccacggtatccttcggagcaggcatgctgaataccggtctgctggtgtcctgtaccttaatgatctgttgtactgcacgggcattaccacattcatcaaaggcggtccacttacggtagatcacgtagttgttattacagctgttcgggttgtgggcagcagagtctttcggcactactgtaattacacccggcgtacagttatcggttgctgtgagattaaatccggccgggatcttatcgcaatccactgtggtatcggcaggtgtagccatattgaataccggggcggtcatgtctttcacggtgatcacctgtttcagggtcacgccggtgttacattcgtctttcgcggtccaggtgcggatcagcaggtaattgttagcacagttgcctggcagatcctggcgaacttccactacagggataatgatttccccggcgcagtcgtcgtttgctttcaggtttattgctgcaggtaccttatcacaatttacggttgtatcagcaggcgctggtgtggtgaataccggtgctttggtatcctttaccgtaatggtttgtgaagcgcttactgagagaccgcatctatctgtcgctgtccaggtacgggtaatggtactgagacaaggcgaagtaaccacggtgacgtcattgtaagtaatggtcagcggctcgttgttgtaaggcgcgtgactgaacgccggatctccgaagagcgtggtgtagtctttacctctttcacattccgttgttatggccggaggagtgaaggtaacaatcgggctgatagtgatggccgtgattttcaccacgttgctgatgttgttgatacaagctccggaagctaccactcttctgtaccaggtgttggctgcaagcaaaccaggctggtaagtatcgctggtggcgccggtgatgttggtgaatggtccgtttgcaccggcagtgctttgttgccactggtaggtgtaagtgccattaccgccggtcagtgcattgctgcgtatagccattggcgtttctgttacgcaaactgtttgatcatcctgaatggtgttaccgagtattggtttacggttaaccagggtgacactggaactggaagcgtcgcacacgccgttgcttactacccatgttaattgggctgtttcgccggcaggaacggtgatggtagcatctttccggttaatatcactgatgttgatcagtgccgcgttgttgctggttacaatccaggtgccttttgcacctgctacaccaggatcgctggcgctcattttaaaggtggcatcatcgcaatgttcctgatcaatacctgcgttggcaggtaccggtaacctgtagttgatgagtgttacatcatcccaggtagcgctacatacgccgttggtcacagtccagcgtaaagtaaccgtatcacctgtgttgatgttcacattggaagtaggactgttgatagacctgatcgcagcatttcctttaataacagaccagaagccttttgcacttggtacagataccggatctgctgccagggtgaagtcgccggtgttattacacatttcaatatctgctcctgcatttgcagcagccgctgttttatagttgatcagtgtaaccgtgctgctggtgctcatgcagctaccatttgttacggtccatttcaggattacagtatcgccaaccggaacagttactgcggtattcgggtcatttaccgatttgataacggcgttacccggaacacggcttacatcggtccaggtgccttttgcactgggggatccgggttgactcgccttcatgatgaagtcggctgtagtattacatttttcctggtcaaggccggcatttgctgtgatggccgctttgtagttgatgatggttaccctgctgaagctggtatcacatacaccgtttgcgatagcccactggagtatcacggtatcgcctacaggcactgttaccgcggtagtcggactattaggtgatttgatttttgctcttccaggtattgggctgatgtcagtccaggttccttttgcagtgggcacgcctggtacatttgccgccatgatgaagtcgcctgtgttgccacagatggcctggtcaggaccggcatttgctttatttgcgttggcgtagttggtaagcattactgtatcataagtagcggcgcaggtgccattggtgattctccataccagttttacgctgacacccgcagcaacagtaacggccgtgttgtattgattcggagaggcgatagttacgccggtggtaccggctggattcgtccaggtacctgttacatgtaaaccggcaggtttgctcccatccaggatgaagttgatgtcatcacatttttcctggtcaggaccagccttggcggcagcaggtgttttgtagctggtgatccttacggtatctgccaggtctgctgcgcattttggattggtgatcttccaggtaaacaggatggtgctgtctgccggaacggtaacggaagttttcggatcgttaatgttcgacatcttcacagtggcagtcgctggtgagaagctccatgtaccaatagcacccagctcagtaggagcggtggcgttcatggtaaaggtggtttgctcacaggctattttattggtgcctgcatcacgcattaccggttttttcagactggtgatccttacggtgtcgatgttgtcagctgcgcatttcgcgttggtgattttccaggtgaacaggataacgctgtcggccggaacggtaacagccgttttaggatcgttgatattggcaatttttacagaagccgtagccggtgagaaagtccaggtaccttttgcgccaagctccgtaggggcggtggcgttgagggtaaaggtagttttatcacattccatctgatcggcgcctgcactgcgcatgattggtttaagcagactggtgattaacacggtatctacgttatctgccgcacatttcgcgttggtaatcttccagatcagctgcaccgccatattcgcaggaactgttacactggttttaggatcattcttattcacaaaggtcaccgcagcagtagcagggaggaacgaccaggtaccttgtgcacccagctctgtaggagcggtagcattgagggtaaaggtggttttctcacattccatctgatcggtgcctgcgctgcgcatcattggtttaagcaggctggtgatgataaccgtatccactttatccgcgctacatgtaccatttgaaatgctccagatcagctgtaccgctgtgtttgcaggaaccgtcacattagttttcggatcattcttatttacaaaggatactgcagcagtagcagggaggaacgaccaggtacctttggcgcccaattcagtaggagcggtggcgttgagggtaaaggtagttttctcacattccatttgatcggcgccggcattgcgcatgattggtttgagcagactggtgattcttacggtatcataagtaggagcagcacactcggagtttgaaatctgccagaagaggagtactgaactgtcggccggaacggtaacagtagtagtcgcgctgttgatgttagcaaacttcacagaagccgtcgccggagtgaatgtccaggtgcctttagcgcccagctctgtaggagcagtggcgttgagcgtaaatactgttttatcacaagcaatctggttggaaccggcatcgcgaacgattggttttttcaggctggtgatcctcacggtatcataagtagcagcagcacactgtgagtttgaaatctgccagaagaggagcactgagctgtcggccggaacggtaacagtagtagtcgcgctgttgacatttgcaaacttcacagaagcggtagccggagtgaatgtccaggtgcctttagcgcccagctctgtaggagcggtagcgttgagtgtaaacaccgttttatcacaagcaatctggttagaaccggcatcgcgaacgattggtttcttcagactggtgattcttaccgtatcataagtaggagcggcacactcggagtttgaaatctgccagaagaggagcactgagctgtcggccggaacggtaacagtagtggtagcactgttgatattagcaaacttcacagaagccgtcgccggagtgaatgtccaggtgcctttagcgcccagctctgtaggagcagtggcgttgagcgtaaatactgttttatcacaggcaatctggttggaaccggcatcgcgaacgattggttttttcaggctggtgatcctcacggtatcataagtagcagcagcacactgtgagtttgaaatctgccagaagaggagcactgagctgtcggccggaacggtaa
